European Patent Application EP 4 678 733 A1, published January 14, 2026. Title: Bacterial strain capable of oxidizing elemental sulphur and its use to promote plant growth. Applicant: AZUFRERA Y FERTILIZANTES PALLARÉS, SAU. The sequence listing filed with the application follows.

SEQUENCE LISTING (12 sequences)

SEQ ID NO: 1 - DNA, 1441 bp, Variovorax sp.
  source 1..1441: PCR_primers = fwd_seq: agagtttgatcctggctcag, rev_seq: aaggaggtgatccanccrca; PCR_primers = fwd_seq: gtaaaacgacggccagtgastttgatcctggctyag, rev_seq: ggaaacagctatgaccatgcggttaccttgttacgactt; mol_type = genomic DNA
  gene 1..1441: product = 16S ribosomic RNA; product (original language) = ARN ribosómico 16S
gctggcggcatgccttacacatgcaagtcgaacggcagcgcgggagcaatcctggcggcgagtggcgaacgggtgagtaatacatcggaacgtgcccaatcgtgggggataacgcagcgaaagctgtgctaataccgcatacgatctacggatgaaagcaggggatcgcaagaccttgcgcgaatggagcggccgatggcagattaggtagttggtgaggtaaaggctcaccaagccttcgatctgtagctggtctgagaggacgaccagccacactgggactgagacacggcccagactcctacgggaggcagcagtggggaattttggacaatgggcgaaagcctgatccagccatgccgcgtgcaggatgaaggccttcgggttgtaaactgcttttgtacggaacgaaacggctctttctaataaagagggctaatgacggtaccgtaagaataagcaccggctaactacgtgccagcagccgcggtaatacgtagggtgcaagcgttaatcggaattactgggcgtaaagcgtgcgcaggcggtaatgtaagacagttgtgaaatccccgggctcaacctgggaactgcatctgtgactgcattgctggagtacggtagagggggatggaattccgcgtgtagcagtgaaatgcgtagatatgcggaggaacaccgatggcgaaggcaatcccctggacctgtactgacgctcatgcacgaaagcgtggggagcaaacaggattagataccctggtagtccacgccctaaacgatgtcaactggttgttgggtcttcactgactcagtaacgaagctaacgcgtgaagttgaccgcctggggagtacggccgcaaggttgaaactcaaaggaattgacggggacccgcacaagcggtggatgatgtggtttaattcgatgcaacgcgaaaaaccttacccacctttgacatgtacggaattcgccagagatggcttagtgctcgaaagagaaccgtaacacaggtgctgcatggctgtcgtcagctcgtgtcgtgagatgttgggttaagtcccgcaacgagcgcaacccttgtcattagttgctacatttagttgggcactctaatgagactgccggtgacaaaccggaggaaggtggggatgacgtcaagtcctcatggcccttataggtggggctacacacgtcatacaatggctggtacaaagggttgccaacccgcgagggggagctaatcccataaaaccagtcgtagtccggatcgcagtctgcaactcgactgcgtgaagtcggaatcgctagtaatcgtggatcagaatgtcacggtgaatacgttcccgggtcttgtacacaccgcccgtcacaccatgggagcgggttctgccagaagtagttagcctaaccgcaaggagggcgattaccacggcagggttcgtg

SEQ ID NO: 2 - DNA, 378 bp, Variovorax sp.
  source 1..378: PCR_primers = fwd_seq: ggytwygaagtncghgacgtdca, rev_seq: tgacgytgcatgttbgmrcccatma; mol_type = genomic DNA
  misc_feature 1..378: note = Fragment of the 16S rRNA gene of SEQ ID NO:3; note (original language) = Fragmento del gen del ARNr 16S de SEQ ID NO:3
gacgtgcacgtgacccattacggccgcgtgtgcccgatcgaaacgcctgaaggcccgaacatcggcctgatcaactcgctggccctgtacgcccgcctgaacgaatacggcttcatcgagacgccgtaccgccgcgtggccgacagcaaggtcaccaacgagatcgactacctctcggccatcgaagaaggcaagtacgtcatcgcccaggccaatgcggtcctggacaaggacggcaagctgaccggcgacctggtctcggcgcgtgaagccggcgaatcgatcctggtcggtgccgagcgcatccagtacatggacgtgtcgcccgcgcagatcgtgtcggtggccgcctccctcgtgccgtcctgagcacgacga

SEQ ID NO: 3 - DNA, 4125 bp, Variovorax sp.
  source 1..4125: mol_type = genomic DNA
  CDS 1..4125: protein_id = 6; translation = MAQSSAYSYTERKRIRKSFGNRDSVVEIPYLLQMQKDAYTAFLQAGIPPKQRTVEGLQAAFDAAFPIVSHNGFVEMKFLEYNLAKPAFDVRECQTRGLTFASAVRAKVQLIIYDRESSTSQSKVVKEVKEQEVYMGEVPLMTEKGSFIINGTERVIVSQLHRSPGVFFEHDKGKTHSSGKLLFSARVIPYRGSWLDFEFDPKDMLYFRVDRRRKMPVTILLKAIGLNPESILANFFVNDNFRLMDSGAQMEFVPERLRGEVARFDITDKSGKVVVAKDKRVTARHTRELEQSATTHISVPEDFLVGRVIARNIVDADSGEILAKANDELTEALLKKLRTAGVQDIQVIYTNELDQGAYISQTLRIDETVDEFAARVAIYRMMRPGEPPTEDAVQALFQRLFYNPDTYDLSRVGRMKFNAKVGRDESTGPMVLTNEDILAVVKILVDLRNGNGEVDDIDHLGNRRVRCVGELAENQYRTGLARIEKAVKERLGQAEQEPLMPHDLINSKPISAALKEFFGASQLSQFMDQTNPLSEITHKRRVSALGPGGLTRERAGFEVRDVHVTHYGRVCPIETPEGPNIGLINSLALYARLNEYGFIETPYRRVADSKVTNEIDYLSAIEEGKYVIAQANAVLDKDGKLTGDLVSAREAGESILVGAERIQYMDVSPAQIVSVAASLVPFLEHDDANRALMGANMQRQAVPVLRPEKPMVGTGIERVSAVDSGTVVTATRGGIVDYVDATRIVVRVNDAEAAAGEVGVDIYNLIKYQRSNQNTNIHQRPIVKRGDKIAKGDVVADGASTDLGELALGQNMLIAFMPWNGYNFEDSILISERVVAEDRYTSIHIEELVVMARDTKLGAEEITRDIPNLAEQQLNRLDESGIIYVGAEVQPGDTLVGKVTPKGETTLTPEEKLLRAIFGEKASDVKDTSLRVDQGSQGTVIDVQVFTREGITRDKRAQQIIDDELKRFRLDLNDQLRIVEADAFDRIEKLLTGKVANGGPNKLAKGTKLDKAYLSSVEKFHWFDIRPADDEVATQLESIKNSLEQTRHSFDLAFEEKRKKLTQGDELPAGVLKMVKVYLAVKRRLQPGDKMAGRHGNKGVVSKIVPVEDMPHMADGTPCDICLNPLGVPSRMNVGQVLEVHLGWAGKGIGQRIGDLLQQEAKVAELRKFMEQLYNGSGRKEDLSKLSDTDLLEMAENLTSGATFATPVFDGASEEEIRGMLKLAYPDDIAKLKGLTDTRTQAYLYDGRTGDQFERPVTVGYMHFLKLHHLVDDKMHARSTGPYSLVTQQPLGGKAQFGGQRFGEMEVWALEAYGAAYVLQEMLTVKSDDVQGRTKVYESIVKGEHTIEAGMPESFNVLVKEIRSLGLDIELERS
  gene 1..4125: gene = rpoB; product = DNA-directed RNA polymerase beta subunit; product (original language) = Subunidad beta de la ARN polimerasa dirigida por ARN
  misc_feature 1681..2057: note = Fragment of SEQ ID NO:2; note (original language) = Fragmento de SEQ ID NO:2
atggcccaatcgtccgcgtacagttacaccgaacgcaagcgcatccgaaaaagtttcggtaaccgcgacagcgtcgtagaaattccctacctgctgcagatgcagaaagacgcgtacaccgcgttcctgcaagctggcattcctcccaaacaacgcaccgtcgaaggcctgcaggccgcgttcgacgccgcgttcccgatcgtctcgcacaacggttttgtcgagatgaagttcctcgagtacaacctcgcgaagcccgccttcgacgtgcgcgagtgccagacccgtggcctgaccttcgcctcggccgtgcgcgccaaggtgcagctcatcatctatgaccgcgagtcgtcgacctcgcagtcgaaggtggtcaaggaagtgaaggaacaagaggtctacatgggcgaagtgccgctcatgaccgaaaagggttccttcatcatcaacggcaccgagcgcgtgatcgtctcgcagctgcaccgttcgcccggcgtgttcttcgaacacgacaagggcaagacgcacagctcgggcaagctcctgttctcggcccgcgtgattccctaccgcggttcgtggctcgacttcgagttcgacccgaaggacatgctgtacttccgcgtcgaccgccgccgcaagatgccggtcacgatcctgctgaaggccatcggcctgaacccggagtcgatcctcgcgaacttcttcgtgaacgacaacttccgcctgatggacagcggcgcgcagatggaattcgttcccgagcgcctgcgcggcgaagtcgcgcgcttcgacatcaccgacaagtcgggcaaggtcgtggtcgccaaggacaagcgcgtcaccgcgcgccacacccgtgaactcgagcagtcggccaccacgcacatcagcgtgccggaagacttcctggtcggccgcgtcatcgcccgcaacatcgtcgacgctgactccggcgaaatcctggccaaggccaacgacgaactgaccgaagcgctgctgaagaagctgcgcacggccggcgtgcaggacatccaggtgatctacaccaacgaactcgaccagggcgcgtacatctcgcagaccctgcgcatcgacgagacggtggacgagttcgcagcccgcgtggccatctaccgcatgatgcgccccggcgagccgccgacggaagacgccgtgcaggccctgttccagcgcctgttctacaacccggacacgtacgacctgtcgcgcgtcggccgcatgaagttcaacgccaaggtcggccgcgacgaatcgaccggcccgatggtgttgaccaacgaagacatcctggccgtggtcaagatcctcgtggacctgcgcaacggcaacggcgaagtcgacgacatcgaccacctgggaaaccgccgcgtgcgttgcgtcggcgaactggccgagaaccagtaccgtaccggcctcgcccgcatcgagaaggccgtgaaggaacgtctgggccaggcggagcaagagccgctgatgccgcacgacctgatcaacagcaagccgatctcggccgcgctgaaggaattcttcggcgcctcgcagctgtcgcagttcatggaccagacgaacccgctgtccgaaatcacccacaagcgccgtgtgtcggcccttggcccgggcggtttgacgcgcgaacgtgcaggcttcgaagtgcgcgacgtgcacgtgacccattacggccgcgtgtgcccgatcgaaacgcctgaaggcccgaacatcggcctgatcaactcgctggccctgtacgcccgcctgaacgaatacggcttcatcgagacgccgtaccgccgcgtggccgacagcaaggtcaccaacgagatcgactacctctcggccatcgaagaaggcaagtacgtcatcgcccaggccaatgcggtcctggacaaggacggcaagctgaccggcgacctggtctcggcgcgtgaagccggcgaatcgatcctggtcggtgccgagcgcatccagtacatggacgtgtcgcccgcgcagatcgtgtcggtggccgcctccctcgtgccgttcctggagcacgacgacgcgaaccgcgcgctgatgggcgccaacatgcagcgtcaggccgtgcccgtgcttcgcccagagaagccgatggtcggtaccggtatcgagcgcgtttccgcggtcgactccggcaccgtggtcacggccacccgtggcggtatcgtcgattacgtcgacgcgacccgcatcgtggtgcgcgtgaacgacgccgaagcggcagccggtgaagtcggtgtggacatctacaacctgatcaagtatcagcgttcgaaccagaacaccaacatccaccagcgtccgatcgtcaagcgcggcgacaagatcgccaagggcgacgtggtggccgacggtgcatcgaccgacctcggcgaactggccctcggccagaacatgctgatcgcgttcatgccctggaacggctacaacttcgaagactcgatcctgatctcggaacgcgtcgtcgccgaagaccgctacacctcgatccacatcgaggaactggtggtgatggctcgcgacaccaagctgggtgccgaagaaatcacgcgcgacattccgaacctggccgagcagcagctcaaccgcctcgacgaatccggcatcatctatgtcggcgccgaagtgcagccgggcgacacgctggtgggcaaggtcacgccgaagggcgagaccacgctgacgcctgaagagaagctgcttcgcgccatcttcggcgagaaggcttccgacgtgaaggacacctcgctgcgtgtggaccagggctcgcaaggcaccgtgatcgacgtgcaggtgttcacccgcgaaggcatcacgcgcgacaagcgcgcccagcagatcatcgacgacgagctgaagcgcttccgcctcgacctgaacgaccagcttcgcatcgtcgaagccgacgcgttcgaccgtatcgagaagctcctgaccggcaaggtcgccaacggcggcccgaacaagctggccaagggcaccaagctcgacaaggcctacctgtcgtcggtcgagaagttccactggttcgacatccgcccggcggacgacgaagtggcaacgcaactcgagtcgatcaagaactcgctcgagcagacgcgccacagcttcgacctcgcgttcgaagaaaagcgcaagaagctcacgcagggcgacgagctgcccgcgggcgtgctcaagatggtcaaggtctacctggccgtcaagcgccgcctgcaacccggcgacaagatggccggccgtcacggcaacaagggtgtggtgtcgaagatcgttccggtcgaagacatgccccacatggccgacggtacgccgtgcgacatctgcctgaatccgctgggcgtgccttcgcggatgaacgtgggccaggtgctcgaagtgcacctgggctgggccggcaagggcatcggccagcgcatcggcgacctgctgcagcaagaagccaaggtggccgagctgcgcaagttcatggagcagctgtacaacggttcgggccgcaaggaagacctcagcaagctgagcgacaccgacctgctcgagatggcggagaacctcaccagcggcgcaacctttgcgacgccggtgttcgacggtgcctcggaagaagaaatccgcggcatgctgaagctcgcctatccggacgacatcgccaagctcaagggcctgaccgatacgcgcacgcaggcctacctgtacgacggccgcaccggcgaccagttcgagcgtcccgtcaccgtgggctacatgcacttcttgaagctgcaccacttggtggacgacaagatgcacgcccgctcgaccggcccgtactcgctggtcacgcagcagccgctgggcggcaaggcgcagttcggcggccagcgtttcggtgaaatggaagtgtgggcgctggaagcttacggcgccgcctacgtcctgcaggaaatgctgaccgtgaagtccgacgacgtgcaaggccgtaccaaggtgtacgaaagcatcgtcaagggcgagcacacgatcgaagccggcatgccggaatcgttcaacgtgctggtcaaggaaatccgttcgctgggtctcgacatcgagctcgagcgttcgtaa

SEQ ID NO: 4 - DNA, 5305463 bp, Variovorax sp. (residues 1-1,768,488 of 5,305,463)
  source 1..5305463: mol_type = genomic DNA
  gene 3283935..3288059: gene = rpoB; note = CDS of the gene; part of the gene of SEQ ID NO:3; note (original language) = CDS del gen; parte del gen de SEQ ID NO:3
  gene 2014365..2015895: note = From 2014425 to 2015865: Complementary fragment to SEQ ID NO:1; note (original language) = De 2014425 a 2015865: Fragmento complementario a SEQ ID NO:1; product = 16S ribosomal RNA; product (original language) = ARN ribosómico 16S
  misc_feature 1..5305463: note = Part of the genome (contig); note (original language) = Parte del genoma (cóntigo)
cgaaaggccccaccccatgcagaaactcaaactcgtgatggtcggcaacggcatggccggcgtgcgcactctggaggagctcctgaagctcgcccccgacctgtacgacatcaccgtcttcggtgccgagccgcaccccaactacaaccgcatcctcctgtcgcccgtgctcgcgggcgagcagaccgtggaggagatcgtgctcaacagctgggagtggtacgccgagaaccacatcaccctgcacgcgggcaagaaggtggtcgaggtcgaccgcgtcaagcgcatcgtgcgcgccgtggatgcgcagggcgccatcaccgaggccgcctacgaccgcctcctcatgtgcaccggctccaaccccttcatgctcccggtccccggcaaggacctccaaggcgtcatcgcctaccgcgacatcgccgacaccgactacatgatcgagaccgccaagacccacaagcacgcggtcgtcatcggcggcggcctcctgggcctggaggcggccaacggcctgatgctgcgcggcatgagcgtcaccgtggtgcacgtcatgccctggctcatggagcgccagctggacgacgtggccggcaagctgctgcaaaagtccctggaagaccgcggcctcaccttccgcatcggcgcccagacccaggaactcgtcggtggcgacgatggccgcgtcaaggccatccgcttcaaggacggcaccgaagtggccgccgacctggtcgtcatggcggtcggcatccgccccaacaccgagctggccgagaagatgcgcctgcactgcaaccgcggcatcgtggtcaccgacaccctgcagaccgtgaccgacgcgcgcatctactcggtgggcgaatgcgcggcccaccgcggcatcgcctacggcctggtcgcgcccctgttcgagcaggccaaggtcgcggccaaccacctggcccagttcggcatcgggcgctacctggggtcgctgacctccaccaagctgaaggtcaccggcatcgacctgttctccgccggcgagttcatgggcggcgaaggcaccgaggagatcgtcatgagcgaccccttcggcggggtctacaagaagctggtgatcaaggacgacaagctggtgggcgcgtgcctgtacggcgacacggtggacggcagctggtacttcaagctcttgcgcgacgggcgcagcgtgcacgacatccgcgacaagctgatgttcggcgaatccaacatcggcgacaccggccacgagggccacagcaaggccgccagcatgcccgacgaggccgaggtgtgcggctgcaacggcgtgaccaagggcaccatctgcaaggcgatcaaggacaagggcctgttcacgctggacgaggtcaagaagcacaccaaggccagcgccagctgtggttcctgcaccggcctggtcgagcagatcctgatgttcaccgccggcggcgactactcggccacgcccaagaagaaggcggtgtgcggctgcaccgacgcgaaccaccaggaggtgcgggaagccatccggaaggaacactacctgacccacgatgcggtctaccgcaacctgggctggcgcacgcccaacggctgcgcgacctgccgcccggcggtgaactactacctgatctcgacctggcccaaggaggccaaggacgatccgcagagccgcttcatcaacgagcgcagccacgccaacatccagaaggacggcacctactcggtgatcccgcgcatgtggggcggccacaccacgccggacgagctgcgccgcatcgcggacgcggccgacaagtacaagatcccgacggtgaaggtcacgggcggccagcgcatcgacctcctgggggtgaagaaggaggacctggagggggtctggaaggacatcggcatgccgtcgggctttgcctatgccaagagcctgcgcacggtgaagacctgcgtgggcagcgagtggtgccgcttcggcacgcaggactgcacgcagatgggcaaggacctggagcgggcgctgtgggcgatgtattcgccgcacaaggtcaagctcgcagtatccggctgcccgcgcaactgcgccgaggccgggatcaaggacgtgggggtgatcggggtggactcgggctgggagctgtacgtggggggcaacggcggcatcaagacggaggtggcgcagttcctggtgaaggtgaagacggcggccgaggtgatggagtactcgggcgcgttcttgcagctgtaccgcgaggaaggctggtacctggagcgcacggtgcactacatcgggcgggtcgggctggactatgtgaagaagaaggtcctggaagacgcggaaggccgcaaggcgctgtgggagcggctgcagttcgcgctggatggggagccggatccttggttcgcgtcgagccaggcgcaggtggatgtgcggcagttcacgcccgtggctgtcgtggacgaagcgacccaggcagcgtgagcgaaggagcaacagcaatgaacgacaacaacgaatggaaagtcatctgccgcgtcgaggacatccccgtgctcggcgcccgccgcgtggcgcgcccggtgggcgtggacgtggcggtgttccgcaatgccgagaaccaggtgttcgcgctgctcgaccgctgcccgcacaagggcgggcccttgagccagggcatcgtgttcggcaccagcgtggcctgcccgctgcacaactgggccatcggcctggacgacggctgcgccaagtcgcccgatgagggatgcacgccgaaatttgcagtgaaggtgactgagggcgtggtgcatctcgattcgaacgagctcgccacgcatgcggtggagctcgagcgcccggtcgccggaccggccaaccgcgcctgcctccaggccgaagacaccgccgcctgaactacagcagacgaaccatgagccttactctcacttcctcgtcgcgcagcggcgatcgcagcacgggcatgccgcccgcgcacggccgctgcacgctcgtcggcgccggccccggcgacccggaactgctcacgatcaaggcactgagggccatccagtcagccaccgtcttgcttgtcgacgacctggtcagcgacgacatcgtcgccatggcggcgcccggcgcgcgcgtgattcacgtcggcaagcgcggcggctgcaagagcacgccgcagagcttcatcgaacggctgatgatcatggccgttcgcgagggcgagcacgtggtccggctgaaaggcggcgacccgttcatcttcggccgcggcggcgaagaggtcgagcacctggcacaggccggcatccacgtcgaggtggtgaacggcatcacggccgggctggccgggctgacttcgctcggcgtgccgctcacgcaccgcacgcatgcgcagggcgtggtgttcatcaccgggcatgccaagcccggatcgccaaggcccgactggcgcacgctggctgccacggcccattcggcgcggctgacgctggtcatctacatgggcgtgtcgagcgcaggctcgatccaggacgagctgctgagcggactgccgccagagacccccgtcgcggtggtgcagaacgcgagcctgccctcgcagcggcacgccgtgggcacgctggcgacgctccggcacaccattgccgacaacggcctttccagcccctccatcatcgtggtcggcgatgtgctgcaggggctggccgccgcaagttctcccgcgcatgttgcgctggagaaggccgcctgagggggcggccctcccctcgcctgtctttctttcagcttctccaatcaaaaccaaagcaacgccatggcctatctcctgccttccgaattcgtcaccaagatggtggacgccggtgagtccaagatcttcatgtccacccgcgacacgctgatccgcgctttcatggcgggcgccatccttgcgctggcggccgtgtttgccgtcaccatcaacgtgcagaccggctactcgatcatcggggccatcctgtttccggtcggcttctgcatgctgtacctgctgggcttcgacctgttgaccggcgtattcgtactgacaccgctcgcgctcatcgacaagcggcccggcgtcaccatgggcggcgtgctgcgcaactggggcctggtcttcgtcggcaacttccttggtgccttcctcgtcgccgtgctgatggcgatcgtcttcaccttcggcttcacgagcccgccggacaaggtgggccaggtgatcgccaccatcggcgaggcgcgcacggtcggctactccgaccacggcgccgcaggcatgctgacgctcttcgtgcgcggcatgctgtgcaactggatggtgtccaccggcgtggtgggtgccatgatctccacctccgttaccggcaaggtgctggccatgtggatgccgatcatggtgttcttcttcatggtgttcgaacactctgtggtcaacatgttcctgttcccgtcggcactgctcatgggcggcaatttttcgatcatggactacatcatctggaacgagatcccgaccgtgctgggcaacctcatcggcggcctgtcgttcaccggcctgacgctgtacgccactcacgtgcgcacggcgcccaagcgcgtcgcccgctgattcccaatcgacagccatcgtcgcgccacgatgcgtcccggactcgcgatatcgatcggacagcactccgacaagggacgcaagaacgccaaccaggacttccacggcgccgccctgccggaggcgtccacccgccacgcgaagggcgtggccatcgccattgccgacggcatcagcagcagcgacgtcagccacgtggccagcgaggcggcggtccgcagcttcctgaccgactactactgcacctcggacgcatggagcgtgagccgctcggcgcagcgcgttctcaccgctaccaacgcctggctgcacgcacaaacccagagcggcggtggccgtttcgacaaggaccgcggctacgtctgcaccttcagcgccctcgtcatcaggtcggccacggcgcacgtctttcacgtcggcgacacgcgcgtctaccgctggcacgcggaggcgctcgagcagctgaccgaagaccatcgggtgttggtggccgacgggcacagctatctgagccgggcgctgggcgtcggcccgcacatcgaaatcgactaccaggccgtgcccgtcgagaaaggcgacgtcttcctgctgacgtcagatggcgtccatgaacacgtggacgccgccgccatcggggccgcgctggcggcccatccggaagacctcgatgcggcggcaagaaccatcaccgaggaagcctatcggcgcggcagccccgacaacctgacggtgcagatcgtccggatcgacgcactgcccgacggcgacttcaatgagctgcacgcacagcgcgcggcactccaactgcctcccgtcctcgatgcacgcatgcgcttcgacggctacaccatcgtgcgcgacctgcaccgcagccaccgcagccacatctacctagcggtggacgacgacacgggccagagcgtggtgctcaagacgccatcggtcgacctgcagaacgacgaggcgcacctggaccgcttcctgctcgaagagtgggtggcgcggcgcatcgacagcgcgcacgtgctcaagccgcatgttccggatcgcaagcgcaactacctctacgtggccatggagttcgtcgacgggcagacgctggcgcaatggatgatcgacaacccgcgccccagcctggagtcggtgcgcggcatcgtggagcagcttgcgaagggattgcaggccttccatcgcatggagatgctgcaccaggacctgcggcccgagaacgtgatgatcgaccgcaccggcaccgtgcgcatcatcgacttcggatcggcctgggtggcgggcctcggcgacggcacgcgggccgagcccggccagatactgggcacggtgcagtacacggcgcccgaatactttctgggcgaaggcggctccgcgcggtccgacctgttttcgctggccgtcatcgtctaccagatgctgaccgggcggttgccctacggcgccgaggtcgctcgcatccggacgcgcgcggatcagcgcaacctgcagtaccggtccgcgctggacgcgcagcgcgccattcccgcatggatcgacgaagtgctgcgcaaggccctgcatcccaacccgctgaagcgccacgaggtgctgtcggaattcgtgcaggacctgcggcagccccacccggattttctgaaccggcgcggcacgccgctcgtcgagaagaatccggtggtcttctggaaatgcgccaccctggtgttgggcattgcgctgatggtgctgcttggcgtgatcagcctgcggggctgagcccgcgtctcgtcagcctctgttcaggccggccgaggaaatcaaagcgcttctgtgccgccatggtttcgggcaacacgtagaccacgcctcggcggctgcccagcacgggcttgatgtaggcatcgtaaaaggcggccggcacgttgatgcagccgtacgaaatgcggttgtcggccacggtcggcgaggccagccgctgcaggcggcgctccgatttttgggtggcgcgcacgcggtgcatcgaaaccgccgcctcgtaatcgatccagacgatgtcctcgcccttgatgttgaggcccggctccgtctcgaaacggcccgcgggcgtcgtgcgctcttcaggccgtatctccgacaccgggcgttcgccgatgcccggcaccgaatcgtcaccgcgagccaggcccagcagcacgggcgatgaagcctgcagccgacccgcggcgtcgaagacgaagacgcgcgcattgcgcttgtcgatgaccgcgaaaggcgcgctacggttgtccgcagccgcaacggccgcccgggcgagccactgcgcatcttgcgccgcggccgccaaggggacttgggcgaacgcgagaacagcgacagcgagcatggcaagttgcctgctcgctgcgcccgttccgggcttcacggcattcatgggtgcgccgcgttcgtagcgggaggcagccgcgctcagttgcggtcggcgcgcgcgcgacgcatggcaggcgtgtcgcccgaggccgccatggtggtgctggagctgctgctcgtatcggtcgagccttgggccgtgggcggggtggtccgggtggcgccgccgctttccggggtcacgcccgtggtgcccatcgcgccgcccgaggggctttgctggcctgcagcggtggccggattgggcggcgccgtggtcggcgggttgccctgggcgaacgcggcgcctgcggcaccgagtgcaagtgcggcaatgagtctggaagtgctgttcatggtcgtgtctcctgaagaaagccggcggtgccggaagaaagaggccgtgccggaccgaatgcccgacttcaggaaagctaggtcgttgccggccgcggcgggtcagcttgcggcgcggcacggtgtaggagaagagaagcgcgaagtaaacggggctacctctaccctcccctacctcttggtatccgggttacgcgcctcctcggccttgtcctgcggcgccttcggcagcttgaccttcgtcacggtgacggacaccgggtcgctcgcggggaaggactcttccaccccgctgtccagcgcctcttcgctgggggcctgctcgaccggcttggccggctcgctggcgggcttgccgtggttcttggatgtgggaaagggaaatgccttgtccgatgtttccgtggtcatggggactcctcggccgtgccagctccaggcgtggacggctgctggtttgtgatttcgggcgactcgctcactcttcgctgctcctgttcagttgacgggaaaaggtaaagaatgcagccattctggaagggctcccaaagaccagcgtaggacgacgccagcgtccgtcagtcggagccatcctcgccccaacgccctttcggcgttgttgaatcctgttgggagcctgacttttgccgacgtgcaacacctggccggcagtgcccccgatttgttcggtgccacatgcacctattgacattgaatgtgataaattcacatttataacaatatgaaacattcattgatgggcccagctgaatgaaaaagcacttgtttttgcaaaagcaaaatggcttcacgctgatcgaattgatgatcacggtcgcgatcattgcgatcctggcgtccatcgcgtaccccagctacacgcaatacatcattcgatccaagcgttctgcggcccaggcacagatgatggagatcgccaatcgggagcagcagttcctgatcgcgaatcgcggctacgccgacaaggacaccctcatcgcgagcggctacacgctgccttcggatgtcgccgccaactatggctacacgatcaccctctcgaccccggttccgggcttcgttgtgactttcacgcctacgggaacccaggccagcgacggcaacctgacgctcgaccacaccggcgccaaaacgcccgcaaacaaatggtgaagcccagcacgcccgttgcccatgcccgcgcccagcgcggcgccacgctgatcgaagtgctggtcacgctgctgatcgtcgctttcgggctgttcggactcgtcggcttgcaagcccgcctccagtcgtcggaaatggagtcctaccagcgttcgcaagcgctgatcctcctcaacgacatggccagccgcattgcaatcaaccgccgcatggcctccaactacgtcaccactgagccgctcggcaccggggtcgactgcccggccagcaccggctcgcgccagacggtggatgccatggaatggtgcaacgccctgaagggcgcggccgaaacttcgggcggcaacaacctcggcgcaatgatcggcgggcgcggctgcgtgcaggacatgggcaacaacgaatacctgatcaccgtcgcctggcaaggcctggtgcccatcgccgcgccgcctgagggcgtgtcctgcggcaaggaccagtacgacgccaccgccgcgagcccgtcggcccccgcgccggcctgctcgagcgacaagtgccgcaggaccgtgaccacgctggtccgcatcggggcgctttcatgaggccggcccgccaagcgagcgccgggaggcatcctgcccgccctccccaggcatcccggctccagcgcggcctgaccctgatcgagctgatggtgtcggtcatcatcatgctgatcgtgttggcggcgctgatcgcgctgttcctcaacgtgaacagcacccagcgcgagatggtcaaggtcaaccgccagatcgagggcggccggctcagcgtcttcgtcctggagaacgaggttgcgcacgcgggcttctgggaaaactacatgcccgagttcgacgatctcacggtcagcagcgcacccacgaaggtgcctacgggcgtggcgcccgatccgtgcctggcctattcggcagctacgtggaccgacgactacaagcgcagcctgctcgacatcccggtgcaagcttacgacgccgtgcccgccagctgcgccgccctgctgaccaacaagaaggccggcaccgacgtgctggtggtgcgccatgccgagacctgcgtggcaggcatgcccaactgcgaagccgactcgctcggcaagctgtacttccagtcgacgttctgcggcacgcagaagccgtcggacttcgatctcagcacggcggggttcaccaccatgctggccaagaactgcacggcggcggcacccaagcgcaagttcatttccgacatctactacgtgcgcacctacgccgagacggccaccgacggcattccgaccctcatgcgctcgcgcttcgacctgtcggccaccggcctcgcacagcagccgccggttccgctcatcgaaggcatcgaaggcttccgcgtggagctgggcctggacacgctgagcaagaccggcgcggccgtgaactacacccaggccatcgcctgggccgatccggccaaccggtccacgcccaccaaccgcggcgacggaagccccgacggcaatttcgtccactgcagcacggcgtcgccctgcacgtcggaccaactgatcaacgtggcctcgctcaagctctacgtggtggcgcgcagcctggaaacctctcccggccataccgatgcacgcacctacaacctggggagcgcgaccatcggccccttcaacgaccactacaagcggcacgcgttcaccaccgcggttcgcctgaccaacgtgacaggccgcagggaaacgccgtgaagaagatgccgtcgacattccacaagcaccgccaaggcggcgcggcgctgatcgtcgggctgatcatgctggtgctgatcaccctggccgtcacggcggggttcacgctcagcagcaccaacctcaaatcggtcggcaacatgcagaaccgcaacgaggccgtggccgcagccaaccgcgccatcgaggaggtcgcgacctccttgctgctgcccggcgtcgacggctctccttctcttgccgcgccgcaacgcacccaaagcctggtcgacatcaacaacgatggcaccacagactacaccgtggacatcgcagtccccacctgcgtgcgtgccaccaagacaacggacaccggcggtagcacctccggcattggcggcatcggaggcaactcgtccactgcgggttccggcctcgcctccttgcccgaccaatacaactcggtatgggacatcagcaccaccgtgaccgacacccgtaccggcacttccaccgcagtgcgccagggcgtgcgggcgctgttgagcaaggcgcaattcgacgcgctgtgctcgtcctagccatgcccatcctccgaatgatcacgacgatgaacggatcgcaatcatgaaaaagaacctcttccggtcgctttgcgccaccgcgatgctgatgctcggcctgggctcggcgcaggcggaagacatcgatcttttcgtcggctacaaccagaccgtcacaggcaagccgaacgtgctgttcgtggtggacaacacggccaactggacgccgctcttcgccaccgagatggaagcgctggcagccgccttcgacggtctcgaggacggcggtttcaatgttgggttgatgctctttaccgaaacgggcaacggcaactcgaacctggatggcgcctacgtgcgcgccggcgtgcgcctgatggacgccgccaccaaggccaagtacagcgcgatgatccgcactctcgacgtgaatgccgacaagtccaacggcggcaaggccggcaagatgatggcggaggtctaccgctatctggctggacaggcgccactggccgggaacaacaagctcaaggccgactacaggggcaatgtctccacttatggtcagggcaacaacgaatccgctgggtccgtcgcgtccagggcggtctgggcgcttcctggcaatccactgagtgcattcggcggcaccacctacaccgccccgaacaccgccaactgcgtcggcacgttcgtcatctacatcagcaacggcgccgcacaggacaacagcagcgacaccacgatatcggccaatgcactgcgcttggccggcggggacgcgacgaccatcccgctcgaggtgagcggctcgcaggacaacatggccgacgagtgggccaggttcctgaagagcagcatgggcgtcagcgtctataccatcgaagcggccattgccaccggggggcaggggccgggctggaccgcactgctcgagaacatgggaaaggtaagcaatggcgggtactacaaagccgctggcgcgactaacctgggcaaggccttgagcgatgcgctcgacgacatcttcagcaagatccagtcggtcaacagcgtgttctcgtccgtaagcttgcccgtgagcgtgaacacgcagggcacctacctgaaccaggtgttcgtgggcatgttccggcccaacgattcggcccttccgcgctggaacggcaacctcaagcaatacaagctgggcctgcagaacaaccaactggtcttgcaggatgcggccagcgccaatgccatcaataaccagaccggctttattgacccgtgcgcacgaagtttctggacaccgaccgcgctcaacgactactggagcttcagtccttcgggcgactgcattcgcaccggggtgacaagtgcagccatgaaagcctcggacacccccgatggcaacgtggtcgaaaaaggcgcgcagggctacatgctgcggcaggtgcttgccgccaaccgcaacgtcaagacctgcacgccgggcgcctgttcggctctcacgagcttcgccaatgaaaacctggacatcactacagatgcgctgggcgcgcagaccgatgccgcacgcaccgcgatgatcaactggcttcgaggcctgaacaacaaggccgaagagacgaaagacgctgccggaaatttcacgacctccaccaccgcgatgcgcccctctgtgcacggcgacgtggtgcattcgcggccggtggccatcaactacggcaccgatgccgcccaacaggtggtggtgttctatggggccaatgacggcatgctgcgcgccatcaatggcaaccaggacacagccattggatcggcggcgcccggcggcgaactgtggtctttcgtgccgccggagttctacggcagcatcaagcggctgtacgacaacagccagcgcatcaattttcctggcgtccctgccacctcgagtcccaccgcacccaagccctatggcatggacggcccgatggcagcctaccgccagggcacgtcggcatggctatacgccagcatgcgccgcggtggccgcatgatctatgcattcgacgtatcaagcgtggcgtcgcctgtcctcaaatggcgccgcggctgcccgaaccaggacaacgacgacgaatgcggcaccggcacgaacgacatgagcggcatcggccagacctggtcggcccccaagatcgtgaaagccagcggctacggtgccggcctcacgcccatcgtgatgttcggcggtggctatgacaagtgcgaagacgtcgacgccatagaatcccctgctccctgcggtgccgcgacgaagggcaagaagatctacgtgctcgacgccagtacgggcgatgtcctgaagaccttcgacaccgaccgcgcggtcagcggcgaggtcaccatcgtgaacgacagcgcaggcttggccaagttcgcctatgcggcagacctcggcggcaatgtctatcgcatcaccattggcactgccataccgggcagctgggaaatgaccaagatcgcctcgctcggctgcgatgcccccgtgaccacgtgcacgcccaaccgcaagttcatgttcggccccgacgtggtcgaagacaacgggatgtacgtgctgctgctgggctcgggcgatcgcgaaaagccgctgcgttcctacgccggtgcgctcagcgtctccaaccgtttctacatgatggtggacaagcccagcgacaacacctggctcacgaccgaggccagcaagtgcgacggctattcgctgctgtgccacaactccctgttcggcatcacgggcacggcgacaccttcggcggccgacctcgaggcaaagaaggggtggtacctggtgctcgcggccggcgagcaggtggtgacttcgtcggtcacggcctatggcaacacgaccttcaatacccacactcccaccagtccgaccgtgagccagtcgtgccgggccgacctgggaactgccaacgtgtacaacgtctcgtatctcgatgcgggggggcagaacgacggcgcccgcttccagaacgtgatcggcggcggcctcgcgccttcacccgtggtcggccgcgtcatggtcgacggcactttgcgcgacgtggtgatcggcgccaaccccgactcgttcctgagcccgaagggcgccgcggtcaaggctgccttcaagcagcccaagggccgtgtctactggttcatccagaaataagggacaaggtgcagagcatggcaggaacgcgcacccgaggtttcacgctcgtcgagctgatggtcaccatcgtggtgctggtggtgctcgtgtcgatggccctcccctcctttgactacatcaagctttcgagccggttgaactcctactcgaccgaccttgtcgcaggcagccaggtggcgcgcagcgaggccatcaagcgcaatgcgcaagtgacgctgtgcgtctcgtccaacggcaccagctgcgccactaccggccaatgggagaccgggtggatcgtcatcagcggcacgcaggtgatccagaagcagccggccaccgccagcggctaccagatgcgcgacggggccggcctcagtgccctcgccttcgagccgaccggcgtcggcgccacggcggccaacttcacgatctgccgctccagccccgtgggatcccaggagcgggtggtcaaggtcagcgcaaccggccgcagttcgatcacccggaccagcaccggcgtctgcggcacctgaatacgtaagtgcggttttttgtgacatcctcggccacacgaggacaatagtgcaccaaggtgcatggcttcaaggccttgccggccggagccgccgcaccatgcactgcacaaaaacacagctttcacttcatggaacatcagttggactgggcacttgccgcctgcgcccgcatcctgcggccggtggtcaggctcgcccttgccatgggggtgaaacatccgcacctggaagtcctgctgcgtgacctgttgctggaggaggccacgcgctcctggcgcaagcagggggtggccaaacccaacatcagccagttgtccgtcacgacagggctgaatcgcaaggccgtgaccgccaaggtgcgcgacaccgcggacgccctgccccacaccgagctgtcggccgcggccaagactttcacgctgtggctgcagctggtgtcggaaaaccaggctttgcaacgcctgccgatcaccgccgacggggccggtgcgccctccttcgaaaccgtggccaagctcggcagccgcggcaacgtgcaccatcgcaccatccttgacgaactggtgcgcctgaacatggtggccgaagaggacggctgcgccgaactcaaggtcgatggcttcgtgcccgagggcgacctgcagtcgatgctggcctttctcggagacaatggccgcgaccacctgctggccgcggtgtccaacaccctgggcgaggagccgcggatgctcgagcgcgcggtgtttgcgcgcggcctcagcgtgcaggattgcgaaaatatccatcagatgatgcgcgaacgctggtctgccatgcaccttgaactggtgggcgaaatgacgcgcgcggtcgaccgggctccgagcggcgccaaggggcgtatccgcgtcgggatctacacctactatgaagacgaggcggcgccgaatgcgccggcggtcgctcccaagcgggaagaagaaagagaaagtacacgatgaaaacccaccaccgatggatgcgcagcatcctctttgccggagcgatagccttgctgctctcttgcggcggaggcggcggcgggggttccacggggagcctgggtaacctcaacagcagcagtagctcgtcgggcaccggaagcggcagctcggacggaacgggcacgggcagcactggcaccgatgggacgggcaccgcgggcggtacggacggttcgggcggcaccgacggcacgagcaccgcgggcaatggcagcgacgacgggtcgggcgtgggatcgggcggcaccggcgtgagcaccgccgacgcaaccggcgtcggctcggtcggcgggctgggcagcatcatcttgaacggcgttcgctacgacaccgacaccgcaaccaccagcctcgaagacaccaccgaactgcagatcggcatgagcgtgcgcatcgccggcaagatcgacagcgagttcaccgccgccacggcgcagcaggttgcttcggccgccgaattgcgcggtgccgtgtcggccatcgacgtgacgggcggcagcttcgtggtcatgggcaccacggtcaccgtcgacaacgccaccgtgtggagcaatgtcagcggactggcgcaggtcgccgcaggcgacgtggtgcaggtctggggcctgccctctgcgccgggcagcttgcgcgccacgcgcgtcgaactgaagccggcatcgaccgagccgctggtgaccggcaccgtgcagaacctggacctgatcggccagcgcttcacgctcggccagctcacggtccggtacaccggcgccgtgttctccggcggcatcgatcaagccacgctggctgaaggcgccatcgtccgcgtgcgcggcagcgtggcgccgattgcgggcttgttcagcgcaaccaaggtgcagggctggtatgccataccgacgcaaaacgccacagcggtgcagctcgcgggagtcgtcaccgattacaacgggatcggtgacttcaaggtgctcggtacagtgatcaacgcttcaaatgcgcagattccccccggccaactgacttcgatcggcaacggcgtgaaggtggaagtcgacggcttcatgagcaacggcattctggtcgcgaaaaagctgcgcgtccgcaacattccgggcgtcggcgggccggtggttttcactgtaattggcccgattgctcactatcaatctgcttccgacttcatggtgaaaggacagcgtgtgaatgccggcggctctggaacagtattcgaaaacggtacggtcgccgatctcgccaatctgccccccggccgccaaatcgctgtggttggcaacgccgtggtggacggcgtgctgatcgcgcagacagtcagcttcctcccgccttgacgaagctcgccggcccgacgagcccgaactcagtcgccggagaccgcatccgaactggtttcagcgcaccagcagcacgggcaccgtgcagcgcgccagcaccttcatggccaccgagcccagcacgaagttgctcagtgcgccctgcccgcgcgatcccatgatcacgaggtcgaactttccgttttccgcaaacgcggagatctcgtccgccgcatggccgaccttgtgcgcaaaggccgcctcgatgccgcgcgcggccagcgcggcgcgcaccggctccaggacgacgcgtgcctcgtcttggtagtagccgtgcacgaggtcgggccccgcgaatgcggctgcccggtgcggtaccgcaagcaccgcattgaagaccgtgaaggcatggcccgcatgcgaccattccttgtgcgcggccaggtagtcgagcatgcgcgcggtgtattcgctgccatccacggcaagaagaattttcatggtgtccctctggttgatcgtgttcgatggccggatgttcgccgccagcagaggagtccgccttgcgccagatcaagcctcggcgcccagcccgattggcgcgggcacgatgttcacgatgcggctgaagagcgcctcgtactcgcgctccgggggatatccggtgagcggatcgcggttgcggccgaatgcctcgtcgagctcgcgccagtcgtcggcagtcagcacgcgttcggcgagcggcaggatttcgcgctcctcgagcgccatgtggttcaggtagaaatccacgtattgctccacggcgttctcgaaggctgcgcgccgcgagtcgcccagcatttcgaaagccagcagcgcatgctcgacgttccggatctttcgctcgccccacgcatggtcgttgtcgagccggtccatcaactcgcgcgatatcggtgtcctggcgcgcagcttcggaaacagcagctcgctttccttgcggtggtggcgcttctcgggaaattcgtcgacgtagaacagcatggcccgaagtgacgtgaagtcgggccgggtgcctttgcggcggtgctgctcgagcagcatgacgatggagcgcagcatggcggccagtgccgcgtgctcctggcgaatgatgcgaatggtggcgtgggtcgtcatgaagggctcctgtgcgtcccccaagagtctcagctccaggcccgcgcaggcttgctgcagatcaaacgccgcgcatcccgttcgatcttttttcgccctttcggcgacgcattctcttgatcggcatcaagcggcgtcgcacgccggtcccgatactggccgaatcaccatcagaagcaaagcgaggacgccatgtaccagcgaattcttgttcctgtcgatggaagctcgacatccgcgcacggccttgacgaggcgattcgccttgccgaggtcaccggagggcgtctgcgcttgatgcacgtcatcgacgagctttccttcgccctggcgatggacgcctatgcgggccactcgggcgactggctccaggagttgcgcaacgctggcacccagttgctcgaagaaggcaaggcgaaggccgccgcggcaggcgtcgaggccgattcggtgctgtgcgacaacttccggggcgccgttcccgaccgggtcacggccgaagcagcttcatggcccgcggacctgatcgtccttggaacgcatggacgccgcggcctcggccgcatggtgatgggcagcagcgcggagcacatcttgcgaaccgcgaacgtgcccgtgctgctggtgcgcgcacccgaagcgcgcgccaaggccgacgcggagcgcttcgccatgccgaacggcaccgtggccagcgagtaagccggccggcgccgccgcgctctctcgctctctcgctctctctattacccgtccagcggaacaccgccgccgaagcggctggtccactggtcccacagctcctgctggacggccttggccgactcttgccaggcggcaagcattcccagctggatctgctgcgcctgcagcgcgctggtgccgcaggccgcctgccagtcgagcaccgagcgaaggtaagcatcggtccatgccgatgccaggggaacgttgctgtccatgtgactctccttgttcctgaaggtaaatcgtgcaagcaacacgcttgcaggttgcccctagcccatcgggccgccgcccggtcaagcgtacgaacgcaggcgcctggagaactcggccaatggcgcgatgccgctggcttcggcacgctggcaccagtcctgcaattgcctgacgagctgttcgcccgtggcggcggaacggctccacagcgcggtcaattcacggcgcatcgaatacatcgtatcgagcgcctgcgatccgcgcaaagccatggcgagccgcatgcgccgcgactcgtcgagcatgcgctcatccttggccagccagcgcttcacggactgcagcgaacgggcgtcggccggcgacaggcgccgcagccggccgaactcttccgcgtaagcctgcttcaaggagtgcgcgtagctcgaaagcacgtcgtagtggcaccggatgaccgcctgcacggtttccaggtcgacggcgggcttgggcgcggcaagccgcggtgtcggcgccacgtgcttcactgtggcaaggccaagggcctgcagcacgcggatgtagagccagccgatgtcgaactcgtaccacttgctcgacagcttggccgaggtgggaaaggcatggtggttgttgtgcagctcttccccgccaatcaggatgccgatgggcgagatgttcgtgctggcgtccggcgcgggccagttgcgatagccccagtagtggccgatgccgttgaccacgccggcagcccagaacggaatccacgcgatctgcgcaagaagaacgagcccgcccggcaccacgccgaagagcgccatgtcgagcaggcccatcagcacgatgccgaggatcttgtgctgcgagtacagctttcgttcgatccagtcgtcgggcgtgccgtggccgtagcgcgcgatggtctcggccttgttcgactcgcgtatgtagaggaacacgccgcgccacagcacccggttgatgcccagcacctgcgggctgtgcgggtcttccggggtgtcgcactttgcgtggtgcttgcgatgtaccgcagcccactccttcgtcaccatgcccgtcgtcaaccagagccagaagcggaagaaatggctggcgaccggatgcagatccagcgcgcgatgggcctggtggcggtgcaggaagatggtgaccgaggcaatggtgacgtgcgtcagcgccagcgccacgagcaccgcgccccaccatgggagatcgaaaaaacccgagaagaacaatgtttgcatgagtgccttttggtcatttggccttttgaacagtcgcggcattctgcaaagcggccggtgcggggactttgatgcaggtcaaggccgcggccgcaggcccgccgcaagatcgatcaaggcgccatcgggcggtttgcaggcatcgcgcttgccgtcagtacgcacagaccatggggtttcatgcggggtgcgttgacaaccacgatggccggctcaaactcgcgagaagcccgttgcagcgcgccccacacgtgctcctttttttgaaaggtttgaaatgaaccccgatattcaactcaggcacgaggtcttcgctcagctgaactgggacccggcggtgttcgggtgcgacgtcgacgtgcgcgtgaaagacggcgtggtcacgctgcaaggcaaggtcgccagcgaaagcctgaagctcgcggtcgagcgcgccgtgcgccgcgcggaaggcgtcaccaccatcgtgaacaggctcatcgcggcagcggacgcagccgactgcgcgaacggtgccgagctgccgggcgtcgaaagatgacagcggcggcggaacaatccgacttcgcactgctcgacgcctggtggcgggccgctaactacctgtcggtgggccagatctacttgatggacaaccccttgctgcgcgagaagctgagcctttcgcacatcaagccgcgcctcctgggccactggggcaccacgcccggcctcaacttcgtctacgcgcacatgaaccgggccatcaaggcccgcgaacttgacgcgctgttcattgccgggccgggccacggcggaccgggcgtggtcgccaacacctacctcgaaggcacctacagcgaggtctaccccgacatcagccaaaacgccgatggcctgaaacggctcttcacgcagttttcgtttccgggcggcattccgagccacgtggcacccgaaacgccgggctccatccatgaaggcggagagctgggctactcgctgctgcatgcctttggggccgtgttcgacaaccccggcctgctcgcctgctgcgtggtcggcgacggcgaggcggagaccggcgcgctcgcggcaagctggcattccaacaagttcctgaaccccgcgaccgatggcgccgtgctgccggtgctgcatctcaacggctacaagatcgccggccccacggtgctcgcgcgcatcggcgacgaagagctggcgcagctgatgcggggctatggctacgaaccctctttcgtctccggccatgaacccgcgcagatgcacagcctgatggcggccgcgctggacaaggcgctggacgacatccacgccatccagacgcgtgcccggaaggacgggttccgcgagcgcccgcgctggccgatgatcgtgctgcgctcgcccaagggctggaccgggccgcggcaggtggacgggattccggtcgagggcacgttccgttcgcaccaggtgccgctgaccggttttgagggcaagtcggagcacgtcgggctgctcgaagagtggatgcgcagctaccggcccgaggaactgttcgatgccgacggcgtgctgcggcccgagatcgctgcgctggcgcccttaggcccgaagcgcatgagcgccaatccgcacgccaacggcggcctgctgctcaaagacctagccatgccgccctttcacgaccacgcggtggcggtggccaagccaggagcaaccgatgccgaagccacgcgcgtcgccggcgagtttctgcgggacctgatgcagcgcaacgaggccgcccgcaacttccgcgtgatgggtcccgacgaaaccgcgtcgaaccggctcggtgccctgttcgaggtgaccgggcgcacctcgaccgcccggatactcgaaggcgacgatcacatgtcgcccgacggccgagtgatggaagtgctcagcgagcatctctgccaaggctggctcgaaggctacctgctcaccgggcgccatggcttcttctcgtgctacgaggccttcatccacatcatcgattcgatgttcaaccagcatgccaagtggctcaaggtgtgccgcggcatcggctggcggcggccgattgcatcgctcaactacctgctcacgagccatgtctggcggcaggaccacaacggcttcagccaccaggacccgggctttctcgaccacgtggccaacaaaaagtcggaggtggttcgcgtctacctgccgcccgatgccaacaccctgctctcggtggtcgaccactgcctgcgcagccgcgactacgtgaacgtgatcgtcgccggcaagcagcccgccccgcagtggctggacatcgaatcggcggtgcgccattgcacggtcggcctgggcatctggacctgggccagcaacgacgaaggcagtgcgcccgacgtggtgatggcctgtgcgggcgacgtgcccacgctggaaaccatggcgggggtcgacctgctgcgcgagatgcttccggacctgaaggtgcgcgtggtgaacgtggtcgacctgatggcgctgcaggcgccaaatgcccatccgcacgggctatcggatgcggacttcgacgccatcttcaccaccgattgcccggtcatcttcgcgttccacggctatccctcgctgatccaccggctgacctacaagcgaaccaatcacgacaatttccacgtgcacggctattgcgaagaaggcaccaccaccacgccgttcgacatgaccgtgctcaaccggctcgaccgctttcatctggccgccgatgccatcagccgcgtcgagcgctttcgcaacagcgcgggccacgttcaacagcacctgcgcgacaagctgctggagcaccgcgcctacatcaccgtccacggcaaggacatgccggagatctcggactggcgctggaaatcttgagcccgccgcatgcaccaaaggcatgcaccgccgcggcgtgcatgctacgcttgcacggctcccacgatgccgcggcgctcgcgccccactccatgctttccgaatgacatccgcctttcacatcgcggtcctcgacgacgaggtcgacatcacgcaactgctggccggttaccttcaaagccacggtttccgggtgacccagctgcacaacggcgcctcgctgatggcattgatgggcaccgatccggccgacctcgtactgctcgacctgggcctgcccggcgaagacggtttctccattgcgcgccgcatgcgcgaaaactggcgctgcgggctcgtcatcgtcaccggccggggcgacgcggtcgacaagatcgtgggcctggaggtgggcgcggacgactacgtcaccaagcccttcgacctgcgtgaactggtggcacgcgtcaaggccgtgctccggcgcttggcgcccagcaatgccgaagccgcatccatgtccgcagtcgcaccggtcaccccggcgctttcagacaagctccgcttcgccggatggcagctcgacgtcgccgcgcgcagcctggccaatccgcaagggcagaacgtggcgctcaccggcggtgagttcgacctgctgtgcgcctttgcgcgccatgcggggcgcgtgctgtcgcgcgacttcctgctcgagcagacgcgcgggcgcggagccgcccccttcgaccgcacgatcgacgtgcaggtcggccggctgcgcaagaagatcgaagccgacgcggacgatccgcagatcatcaaatcggtgcggggcgccggctacatcctggttccgcccgtcgctcgcgggtgacccgatgaacccgcccccgccctcttctccctccgtcgccgcgttgccggggctgccctcgggcgtcgaagaaagcagcgtcttccgttcgcttttcgtgtcctacccggactcgctgctgctggtcgaccaggcgggcggcatcgtgctggccaacccttcggcggccaagctgctgggctatgccgtcgatgaactggtgggcctgaacgtggacgtcctggtgcccgacagcatccggccgcgccatgccgcctaccgcgaagcctacggccaggcgccgcgcccaaggcccatgggcacgcagatggaactggtcgccaagcgcaaggacggcagcgaggtgatggtcgagatcgcactcagcccgctgcaaagccagggcctgcccttcgtggtggccgccatccgcgacattggcgcctacccgcgcgtgaagcaggcgctgcaacgcgcgcgctacagcgactatctcgcgcagctgggccgcctggccgtcgacacgcgcgacctgcaggtggtgctcgaccacgcacccaccatggccgccgaagcgctggaggtcgaagtggccatggtgctgttgctggacgacagtcgcctcgaatttcgcgtcgccagcggcgtgggcctggtgcccggcgaagagatcggcgcgcgcattccgagccacgcgaacacgccgcccggcttcgtgtttgcagaggccgcgcctgtgatggtggccgacttcgccaaggagcgccgctttgcggtgccgcaggcctatctcgacgccggtctggtcagtgcgctggccgtgcccttctacgatcgcggccgcttcatcggcgtgctgaccgtgcgctcgcgcgaggccaagcgcttcggtgacgaggagctccgattcctggagtcgctgtcgaacctgctggccaccagcctgcagcgggtgcagactgaagaggcgctcagccacgcgcagcggctcgaaagcgtcggccagctcaccggtggcattgcgcacgacttcaacaacctgctcaccgtcatccagggcaacctgcaggtgctcgaagagctgcccgccatcgcgaacgacggctacgcccagcagctggtgggcgcggcggcgcgagcctcgcagcgcggcgccgaactcaccggcaagctgcttgcgttctcgcgccggcagatgctgcagcccaatgcagtggacacgcatgccatgctgcactcgctggccgacatgctgcggcgcacgctcgaccagcgcatcggcatttcgatcgacagcgcgccgagctgcccgccggtgcttgccgacccggggcagctcgaatcggcactgctgaacattgccatcaatgcgcgcgatgccatgcccgacggcggcacgctgcactttcgaaccgaggcctgcggcgcgctgccgcccgaagtgcacaacgagctgagcgaccgcgatgcgcacggcagcttcgtggccatttccatcaccgacagcggcaccggaatgaccgaggaagtgaaggagcgcgcgttcgagcccttcttcaccaccaaggaagccggccgcggcacgggcctgggcctgagcacggtgtacggcttcgtgaagcagtccaagggcgccattgccatcgccacgcggccgggcgcgggcaccacggtgacgctctttctgccccagctggacgaggccgccgccccggccatggaagaggaagacatcgagcaggcgattccgctcggcctgcgcgtgatgctggtcgaggacgactccgaagtgcgcaaggtcgtgcagacctttctgacaaccctgggttgcagcgtggtcgcggccagcaatgccgagcaggccctgatgagcctggaaaccgatgcgggttccttcgacctgctgctgagcgacatcgcgctgggccccggcatgcgcggaacgcggctcgcggccgaagcgcagcagcgctttccggagctcgcgattctcctcatgtccggcttctcgtcggagttgctggaagccgaccgggaagtgccgcaaagctgggagctgctgcgcaagccctacacgcgggccgagcttgcgcgtgccatggccagggtgcttgcgcacccttagtgccgcgcgttcagcggcaccaggcctcgatctggtggccgatatccagccagagcgcctgcagcgccacggccgcgagcaatgcgccggccaggcgcgcgccccacgcctgcggtccgccaccgccgctccacctgagcttctgccagagccatggcgccagcaccagcgagaggccgctgcccgtggcgaacagcatcatcgcgacgccgccctgcagcggcccgttgcccaggctggccagcagcagcgccgaatagagcagcccgcacggcatggcaacccagagcgcgcccgtcgcgagcacgccgagcggcgagcttccggccagcggacgcagccgcgcctcgagcgtgcggccgatgcgctgtgcccacaccggctgccggccggagacggccagcatcgcgccccaggcgaacacgaacacatgcagcagcatccagagcggcctgagcgcggccacttgggtgctggcctgggccaggctgtccacgctcgcggcggcgatggcgcccgccgtggcgtagctcgcgatacggcccaggtgaaaagccgcctgcgccgggaacaccgcgccgccgcccgcgccccccgaggccggcacgggcacgatgcggatcacagcggccgatgccgcgccgcacatggccacgcagtgcgggccgcccgccaggcccatcagcaacgcggcaccggccagtgcggtctgcatggtcagaccacgcgcgaaaagcggttgcggttctcgcggcagtaccggtcgaacaccatcgcgatggcgcgcaccacgaaccatccctggggcgtcacgtcgatgtcgtggtcggtcatgcgcaccaggccctgtgccgccagcggcccgagcgccgcgaactcggtggcgaagtagtgccggaagtcgacccggtgcgcttcgcccatggcgtcgaaattgacgtgccccctgcacatcagggccatgatcacggcacgccgcaacaggtcgtcgcgcgagagcgcaagcccgcgaaccacgggcagccggccctggtcgagcaggtcgtagtacgcgtcgatggtcttcacgttctggctgtaggtggcaccgatgcggccgatggcggaaacgccgagcgccaccaggtcgccgtcgggctgggtgctgtagccctggaagtcgcggtgcaaccgcccttcccgcttggccaccgcgagcgggtcgtccggcaacgcgaaatggtccatgccgatgtagacatagccagcctcggtgagcgtggccacggcgcgcgcgagcatctgcacccgcgccgccgcatcgggcagctcgtccgcggcaatgcgccgctgcggcttgaagcgctcgggcaggtgcgcgtaggcatacagcgcaatgcggtcgggccggagttcgcagacctgcgccatcgtgcggtcgaacgacgtctcgttctggcgcggcaagccgtagatcaggtcgacgttgatcgactggaagcccagcgcgcgggcctcggccatcaggtcgaacacctggtgcgccggctggatgcggtgcacggccttctgcacgtcgggatcgaagtcctgcacgccgaagctcagccggttgaagcccagcgacgccaggtgcgcgagccgcaccgcatcgacggtgcgggggtcgatctcgatggactgctcgccgccgggaagaaagacgaaggcctcgcgcagcatggcaaggagctggctcagctcggcgtcgttcaggaacgtgggcgtgccgccgcccaggtgcagctggctcacggtggtgccgcgcccgagctgcgcaacctggagccggacttcgcgcgccaggtaggccaggtactgggtggccttctcgtggtgccgcgtcacgatcttgttgcacgcgcagtagtagcacagcgattcgcagaacggaatgtgcacgtacagcgagagcggcgccgccgaagcgcccgcatcgcgccggccctgcagcgccagcgcgtaatcgtcagcatcgaaggcctcgacgaagcgatcggccgtcgggtacgaggtgtagcgcggccccgcgacgtcgaactgccgcagcaaagcggtcgacaagggcgccgcggctggaacgacggggcggtcgagaaaggcggtggaagtcgaagtcattgcggatgctcgggagtgtcgcgggacggcggcatggccaggagcgcggtgaatgcgctggaagccgccgccatggcccagaaaacaaagaacgccagggtgtagacgccctggcgcgacatgcgcagcgcgtcgccgccccagtgcagatcggccggatcgaccatcgcgaagaccaggatctcgatggcgcaggccagcaggaaggccggccacaagacgccgatgagctggcgcgaccaggtcatggcctggcctcgccgcgcggcaccggcacagcttcttcgggcgtggccgcatggttcctgccggcgacggcgggcatcagcttcttgtccgccagggtcttgttgatctcgacgccgcggcggtaatagtcttgcgacaccagcgggtcggagcttccccaggcaaaccagaaggtcacgaagctcgcgaccaccaccagcgcgggcccggcaatcaccatccagagcagcgggtagcgccaccatggtttttcgcccggcgtctgcgtccatccgttcttcgttgcgttcatttcgttttccttgcttcagcgcggcaccaggaagaccgctttctcggacacttcggctccgccctcctcgtcccggatgtcgaagtgcaccgtgtgcgagccggagggcaccacgccgtagggcacttgcaggcgcacggcaacccagcgcgactgggccgcatcgatggtgacgcgctcgtcgggcgagacgcgcaggccttcgatgccgtgcgcggcaatgcggtagtggcgtgcgtcctcggtggcgttcatgatctgcaggcggtagacgttctcgagtcgcccgccctcgacgatgcgggccagcgatgcgcggtcgcgcaccacgtcgaccttcaacggcgtgcgcgcgacaaggctggccaggagccccgccaccagcagcgtgaggatggcggtgtagaccagcacgcgcgggcgcagcacgcggcgcagcagttggcggcgcgtccatccggcctccatgccgttttgcgtgtcgtagcggatcagccgcggcgcataggccatcttctgcatcaccgtgtcgcaggcgtccacgcaaagcccgcagccgatgcattcgtactgcagcccctggcggatgtcgatgcccgtggggcacacctgcacgcagagcccgcagtcgatgcagtcgcccagcgccacgctgcgcgggtcgaggcccttgcgcctcggtgcgcgcggctcgccgcgcttcgggtcgtaggtgacgatgagcgtgtcgcggtcgaacatggcgctctggaagcgcgcatacgggcacatgtacttgcagacctgctcgcgcatgaagcccgcgttgccgtaggtcgcaaagccgtagaagaaaacccagaacacctcccacgagcccatgcgggtctgcaaaaaggccatgcccagatcgcggatgggcgtgaagtagcccacgaaggtgaagccggtccacagcgcgatgccgatccacaccaggtgcttgaaccacttcttgaccagcttctccagcgacatcggttcggcatcgagccgcatgcgcgccgtgcggttgccctcgatcttgtgctccacccacatgaagatctcggtgtagacggtctgcgggcaggcgtagccgcaccacagccgcccggccacggcggtgaacagaaaaagcgccagcgcgctgaccaccagcaggcccgagagatagatcaggtcctgcgggtacagcaccaggccgaagatgtagaagcgccgcgaggccaggtcgaacagcaccagctgccgctcgccccactccgcccacggcaggccataaaacaccagctgggtcaggaagaccatggcccagcgccagcgcgcgaacatgccgcgcacggtgcgcgggtagatcttcttcgtggcttcgtacaggccgaccgagtcgctctccaccggaacgatggggatgatcttgcgcgcatcggggctggcagccggtaccgatgcagggacgggggtggatggatccatgatcagacagcggcggatgtcagggcccggtgacggggttcgaaagaccccagacgtaggaagcgagcagcttgatctgcgcctcggtcaggcggccttcctgcgccggcatttcgctgtgcttgccggcgttgacgatctgcacgatggcgctttcgccatagccgtgcagccagatcttgtcgctgaggttgggcgcgcccacggcctggttgccgacaccgccgatgccgtggcaggcggcgcacaccgtgaacttggacttgccgaggcccgcgcgcaccgagtcgtgcggcgcgcccgaaaggctcagcacgtagttcgccaggttcttcacttcctcctgcgtgccgaccgccgccgccaagggcggcatcacgccggtgcggcccttggtgatggtctcggcgatcttctcgggcgcgccgccgtgcagccagtccttgtcggtcagattcgggaagcccttgctgccgcgcgcgtcggagccgtggcactgggagcagttgttcatgaacaggcgttcgccgatggccatggccttgggttcgcgcgcaatgtcttccatcggcatgccggcgtagcttgcgtagacgggcgccagcgcctggttggccttggccacttcggcctcgtactcggcgctggtgctccagttggcctggccgctgaagctgcccaggccgggaaagaccaccaggtagccgaccgcgaagaagatggtcatcacgaacaggccgacccaccacaggggcagcgggttgttggactcgcgcagatcctcgtcccacacgtggccggtggtgttgtccgcatcggacgcaacgcgcttgcgcgccgtgagccacagcagcagcatgcatccgaggatgctcaggaccgtgccggccgcaacgtagttcgaccagaagttgttgacgaaatcgctcatcgtgggcccctctactcttcagtcttgctcgaatggcaggtgggcggcttcgtcgaagcgcgcggcgttgcggcgggcataggcccaggccacgatgccgagaaaaagcgcaaagcacagcacggtggcggcaacgcgcaaggtggtgatatcggtcatggtcgggtgctccttacttgagcgcgaggcccagcgattgcaggtacgccaccgtcgcgtccatctcggtcttgccgcggacgtcttcggccgcacgggcgatttcgtcgtccgaatacggcacgccgacctggcgcagcgcgcgcatgcggcgcggaatggcttcggcgtcgaccaggttcttgtcgagccacgaataggccggcatgttcgactcgggcaccaggtcgcgcgggttgttcagatggatgcgctgccactcgtcgctgtacttgccgcccacgcggtgcaggtcggggccggtgcgcttgctgccccactgaaaggggtggtcgtagacgaactcgcccgccaccgagtagtggccgtagcgcagcgtctccgagcggaacggccggatcatctgcgagtggcagttgtagcaaccctcgcgcaggtagacgtcgcggccggcgagctgcagcgccgtgtgcggcttcaggccctcgatcggctcggtggtcgacttctggaagaacagcggcacgatctcgaccatgccgccgatcgcgatcaccacgaggatcagcacgatcatcagcaggttgttggtctccaccttctcgtgggtgaagccggtgctcttgtgttcggggttcgggttcatgcttgttcctcaggcgtgggcaatggcaacgggcggaatcgatgccgcaaccgaacgcccggagatcacggtcatccacacgttccaggccatcaccagcatgccgcccagatacagcaggccgccggccagccgcaccacgtagaaggggaacgtggctttcacgctctccacgaaggtgtaggtgagcgagccgtcggggttgatggcgcgccacatcaggccctgcatcacgccggcgatccacatggcggcgatgtacagcacgatgccgatggtggcgatccagaagtgcgcatcgatggccttcacgctgtacatctccgtgcggccgtacatgcgcggaatcaggtagtacagcgagcccatggtgatgaagcccacccagccgagcgcgccggcatgcacgtggcccacggtccagtcggtgtagtggctcagggcgttgacggtcttgatggacatcatcggtccctcgaaggtcgccatgccgtagaacgacagtgccacgatcagaaagcgcaggatcgggtcggtgcgcagcttgtgccaggcgcccgagagcgtcatcacgccgttgatcattccgccccagctcggtgccagcaggatcagcgagaacaccatgcccagcgactgcgtccagtccggcagcgccgtgtagtgcaggtggtgcgggccggcccacatgtaggtgaagatcagcgcccagaagtggacgatggagagccggtacgagtacaccggccggccagcctgcttggggatgtagtagtacatcattccaaggaagcccgcggtgaggaagaagcccaccgcgttatggccgtaccaccactgcaccatggcgtcctgcacgcccgcataggccgaatagctcttcgtccagccggcaggaatctcggcgctgttcacgatgtgcagcaaggccacggcgatgatgaacgcgccgaagaaccagttcgcaacgtagatgtggcgcaccttgcgaacgccgatggtgccgaagaacacgaccgcataggacacccacaccgccgcgatgaggatgtcgatcggccattcgagctccgcgtattccttgcccgtggtgtagcccagcggcaggctgatggcggcggccacgatcaccgcctgccagccccagaacacgaatgacgcgagcgccggcgcgaacaaccggacctggcaggtgcgctgcaccacgtgaaagctggtggccatgagcgcgcagccgccgaacgcgaagatcactgcgttggtgtgcagcggccgcaggcggccatagctgagccatggaatgccgaggctgaattcgggccaggcgagctcggtggcgatgatcacgccgacgagcatgccgaccacgccccagaccacggacatgagggaaagttgccgcacgacggtgtcgtcgtacgccgctgcgggaggattgggttcttgcatcgtgctgcctcttgatggactggaggcagtgtccctgcgcacccgccgggtcggtttgatgcagatcaatcgtgacgcaggatgcggtcgccttcgatctcgatgtcgtcgaattgcccacgttcgatggcccaccacaggccgccgaggatggcgagcaccagcacgaccgacagcgggatcaggagaaagaggatgtccatcagccgcccgtcctggcgtcagcgttgccatgagccgccgcgagccgcgccgcattgagcaccaccaccagcgaactcgccgccatgcccagcccggcgagccatgcgggaagccagcctgcgatggccagcggcacgcacagcgcgttgtagcccgccgcccatgcgaggttctgccgcaccacgtgcagcgtgcgccgcgcctgcgcgatggtgcgcggaatggaagcgagcgcatcgccgagcacgacgaagtcggcccgcgcacgcgagagcggcaccgcgcggccgaaggcaaaggacgcgttcgcgcgcgccagcgaagggccgtcgttgagcccgtcgccgaccatcgcgacctgccggccctccgcctgcaggcgccacagcacctctagcttgtcctcaggcgtgcagccgccctgggcaaaggcaatgccggcgcgcgctgcgatctcgcgcgcggcgctgtcgcggtcgccggagagcaggcgcaccgtgatgccttcggcctgcagcgccgccaccgcggcgacggcatccgggcgcagctcctcggcaagcacgaagctcgcgagccagccctgctcgtcgctgaggtgaacctgcggcgcttcgacctgcagcggcggcacgttgcaatagcccgcggagcccagccgcatgcggcgggcgggcccgtcgacgctcgtgtctcggcgcagcaggccttcgaggccgaggcccgccagttcggccggctgcgtcacttcccaggcgggcggcgagcggaactgcgcattccatgcattcaccagcgcgcgggcaccgggatgcagcgaatgcgcgccgagcgcggcgccaatctccagcgcgtcgccggggcgcaaaccctgccggcagtacacgcgctccaggcgcggggtgtcgccggtcagcgttcccgtcttgtcgaagaccaccgtatcgaccgaggccagcgcctccagcgcctgcaggttcgacgtcagcacgccgccgcgcgccagcgcccccgcgctcgcgagcatggcggccggcgtggccagggacagcgcgcaggggcaggtcacgatcagtaccgccaccgccaccatcaaggcctggcccgaatcggcatgccaccagaaagctgcggccccggcggccgacgccagcaccaggatgagaaacggccgtgcgatccggtcggccaattgcgccaggcgcggcttgctcagcgccgcgctttccatcagtcgcacgatctgcgcgaagcgcgtgccctcgcccaccgattcgatgcgcacctgcaccgtggccgagaggttgtggctgcccgccagcacgcgctccccgcgcgctcgcggcacgggacgggattcgccggtgagcagcgcctcgtcggtgctggtgccgccgtcgatcagcacgccgtcggccggaaaggcctcgccggggcgcacccgcaccacgtcgccggcggcaaggcggcgcacggccacgcgctgccagccgccatcggcctcgagccgttcgatgctgtcgggcaggcggttcatcacggcttcgagcgaaccggccgtgcggtcccgcagccgggcctcgagccagcggcccgtgagcaggaagaacacgaacatggtcagcgagtcgaaatacacctcatggcccagcgcgcccgcgttgtcgaaggtggccgcggtgctgaccgcgaaggcaatggcgatgccgaaggccaccggcagatccatgccgatgcgcccgttgcgaagatcgcgccacgcgctgcggaagaacgggccgcaggaaaagaagagcacgggcagcgtgagcacccacgaggcccagcgaagcaattgcgccgcgtccgcagtcatctcgccgggctgcgcgatgtaggccgggtaggcatacatcatcacctgcatcatgcagaagcccgacaccagccagcgccacagcgcaagccgcagctcgcgcgaacggcgctcgcgcgcggagctgtcggcggccggcaccagccggtagcccgccaccgcggatgcctcgaaccagcgggagggccgcgtctgtgcggcggaccacaccacgcgcgcacgctggctcgcggcattgacctgcacttcgagcacgccgggcacgtgcagcagcgccgtctccaccgcaaggccgcaggtcgcgcagtgcatgccctccacggcgacctgcgactcccatcgtcccgccgcggccgtgccatcgtcgagcgcgcggccgaacgccggccattcggagggatcgtcgagcacctgccactcttcacggggtgcccgtgggagcgcggcggccggggagaaagaggcgagcgcggcttgcatcgggcaaggctaagggccgcggccgcgccgccgtttgatctgcatcaagcgatgcgcgtggccggctgcctaagctgggggcacatttcctccaatgagagaagaccatgttcaagcgcattctcgtggccaccgacggctccacgctctcgaagaaagccgtcaccagcgccatcgccatcgcggcccggaacgaggccgacctggtggcgctcaccgtggtaccgcgctacccgaagagctacttcgacggcgccatgtccttctcgcccgaggacattgcgcgggtggaaaagcagtgggccgacaaggcgcagggcatgctggatgcggtggagacgcgcgcggccgcgagcggcgtgcagctgaagacggccatcgccaactcggatctggtggccgagtcgatcgtcgccacggcaaagaagcacaagtgcgacctgatcgtgatggcctctcacggccgcaagggcatcaagcggctgctgctgggcagcgagacgcagcacgtgctgacgcactccacgctgcctgtgctcgtgctgcgttagtccgcagcgggctcttctcgcgtcaggcggcctgcaccgacgcggcgccgagcgcgtcgttctgggcttcgctgagccagcgccgcttgtcgcgcagcggcggcgcgccgaacatgcggctgtattcgcgggcgaactgcgacgggctttcgtagcccacgctgtgcgccgcgctcgccacgtccacgcccgccatcagcatctgccggcgcgcctcctgcagccggagttgcttctggtattgcagcgggctcatggcggtcacggccttgaagtgatggtggaaggacgacacgctcatgtgcaccgcgcgcgccatgtcctcgatgcgcagcgactgcgcatagttgacgcgcagcgcgctgatggccttggccacgcgctgggtgtggctgtcctgcagcgcgatctggcgcagccgcgcgccctccccgttcaccagcaggcggtacatgatctcgcgcttgatgagcggcgccatgatcggcacgtcttccggcgtctcggccagccgcaagagccgcagcaccggctccagcaccggcatggcgatgcggttgacgtacatgccgcgcgatgcgggcgcgttggccttcgcgggcagcttctcgtcgccgatgagttcgccgatgtcctcgatcgcaagctccagccgcacgccgaggtagggttcgttgtcgctcgtcaggcgcacctggccgcacaccggcaagtcgaccgaggtcaccaggtagtgcatcgggtcgtacacatagatgtcgtcgcccacgatgatccgcttggagccctgcgcgatcagcccgagcgccggggttgcgaaggcatgcttggggccgtcgggcttgctgatgcagaacacctgcaggccggctaccggcgtttccacggtgccgtcctggccgcgcgtgatgcggttgatcagcgccaccagttccttcctggcttcgtcgagttgcgggtccagcggcatcggctgggcaagggcggcagcgatttcgggtgtttcgtcggacatgttcaggaccttgtcacagggtgattcacggcgccggggcagcgtggaggatcgggtggttcaaagcttagcgccgcatctgccaatctgcacgggcaccagtggaggtctggagaaataggcaaagactttgcaggaacgcgctggccgccctgccaccgccggccggatacttttgccaggccctccggggaatctccgaatctccatcacccagcaaaggaatgcgcgatgcaataccgcaaattcggccgcaccggcctgttcgtttccgagctctgcctcggcaccatgaccttcggcggcgcgagcggcatctggggacacatcggcaacctccagcagtccgaggcggaaagcctggtgggccgcgcgctggacgccggcatcaacttcatcgacaccgccgacgtgtactccgaaggcctttcggaaaccatcaccggccaggcgctgaagaacctcaaggtgccgcgcgagaacgtggtgatcgccaccaaggtgctgggcgaaaccggcaagagccccaattcggccggcgcctcgcgctatcacatcatggacggcgtgaaggccagcctgaagcgcctgcagctggaccacatcgacctgtatcagatccacggcttcgacccggtgacgcccatcgaggaaaccgtgcgcgcgctggacaacctggtgcggcagggccatgtgcgctatgtgggcgtttcgaactgggccgcctggcagatcatgaaggcgttgggcatcgccgagcggcaagggctcgcgcgcttcgaatcgctgcaggcctactacaccatcgcgggccgtgacctggaacgcgaactggcgcccatgctgcagagcgagaacgtcgggctgatggtctggagcccgttggcgggcggcctcctgagcggcaaatatggacggaactctgaagccgagaaaggcagccgccgcaccaccttcgactttccgcccgtgaacgtcgagcgcgcctacgactgcatcgacgtgatgcgccagctggccgaggcgcgcaaggtctcggtggcgcagatcgcgctcgcatggctgctgcaccagcaggtggtgaccagcgtgatcgtcggcgccaagcgcgtcgagcagctggacgacaacatcgccgccacggccatccggctcgatgccgacgcgctggccgcactcgacaaggtgagcgcgctaccgtccgagtacccgggctggatgctcgaacgccagggcggcgcgcgggccaagcgcctcgccgaatcaggccagcgcggctgaccggcggcgcgcggcgtgggccgcggtggcgcgcaatgcgcgcagatcgaggtgccgcgccgcagttgccgcagagggctcggcaaggtgcggcaccacgccgagcaagggcgcaccgagccggccgcgcagcgtctggaggttggcctcgggtgcccgcatccgcggctcgatgacgctcgcgatccaccccgccagcacgaggccgcgcgcccggatggcttccgccgtgagcagcgcgtggttcaggcagccgagccgcagtccgaccaccaggatcaccggcaggcccagcgccacggccaggtcggcgctgtcgatgtcgtcgccgaacggcacgcagaacccgcccacgccttcgacgaccaccgcatcggcctgctccgacaacgccgcgaaggccgacagcagcggcggcaactcgatgcgcacgccctcctcccgcgccgccaggtgcggcgacatcggcgcgcgcagcaggtacgggcagcgcagggaaagtggcgcatcgacattgccggccgcgcgcaactgctcgacgtcttcgttgcaccacacaccgttgacttgctccaggcccgcggccacgggcttcatgccgaccgaccgcaggcccgaggcggccaacaggctcagcatcgcgctgctggccagcgtcttgcccacacccgtgtcggtgcccgtgacgaaccagcggcggtgcgtcatgcgtacttcctgggcgcttcgaacgcctcgcccaaggcgtccagcagccgcgccacgtcggcctcgctgtggctggccgacagcgtgatccgcagccgcgcggtgccggcgggcacggtcggcgggcggatcgcaccgacgcgcaggccgcgggcatcgagctcagccatcgcctgcatcgcgcgcgcgttgtcaccgacgatcagcggctggatcgcggtgggcgaatccggcagccacgcgctgccgtcccgcggcaggatcgcctcgaggccccggcgcagttgcccgatgcgcgccttcagacgggcgcgccgcagcttgccctcctcgccttcgatcagcgtgaggctcgcaagcagcgcgtgcgcgatggccggcggcgcggcggtggtgaagatgtagggccgcgcccgctgcaccaggtagtcgatgacggtgcggtgcgccgccacgaaggcgcccgacaccccggccgccttgccgagcgtgccgatgagcaccagccgctctgagcagaggcccatggcctgcagcacgccccggcccgtggcgcccagcacgccgaagccgtgcgcgtcgtccagcacgagccaggcgtcatgccgctccgccagcgcaagcagttcggccaccggcgcgatgttgccgtccatgctgaagaccgcatcgctcacgatcagcttgaccggcgcgtcgcaggcgccgagctgcgcatcgagcgcggccacgtcgcagtgcggatagcgctcgacccgcgccttggccagccgcgcaccgtcgatcagcgacgcatggttgagcgactcggaaaagatcaccgcctcggcgccgcccagcgccgacagcaccgcgaggttggccatgtagccggtgcagaagaacaggctccgcgcctccgggatgtgcggcgccatccagtcggccaggcgctcctcgagctcggcgtgcgcgcgcgagtggccgaggatcaggtgcgacccgccgctgcccgtgccatagcgcgccgcgccttcggccattgcggcggccagcgccggatgcgcggccaggccgagatagtcgttgctgctgaagccgagcatggtgcgcggcgcgggcgcgccggccagcgtcagggactgctcgggtgcacaggccgtttcggcgatctgccggcggcggcgcagcgacttcgcgtcgagcgccgtgatctcgtcctgcaggcgttcaagcaagcgcggcatcgcggcctccttctgcgtggtcttcgtggtctgcgtggatgggggcggccaccgcttgcagcgtggcgagcgtgccatcgaccagcaggtcgatctcgtcgtcgccgatcgcatagggcggcatgaggtagaccgtcgcaccgatcgggcgcatcagcagcccgttggcgcgtgcggccatgtgaaagcgctcagcaaatcgcacaccgggctcgcgcacgtcgaaggccgtgatcattccgcactggcgcaggtgatcgacgggcatgccctggtggagcccttcgcgcagccggccgatcaaccgctcggcacgcgcgaggttccgccgcagcgcgtcttcgcgctcgaacaggtcgagcgtcgcgagcgccgcgcggcaggccagcgcgttgccggtgtaggaatgggaatgcaggaagctgcgcgccacgtcgtcgtcgacgaatccgtcgtagatcgcatcgcgcgtcatcaccagcgcaagcggcaggtagccgccgctgatgcccttggagaggcaaagaaagtcggaccagatgccggcctgctcgcacgcgaagaaagtgccggtgcgcccgcagcccaccgcgatctcatcggcgatgaggtgcacctcgtagcgatcgcacagcgcgcgcacgaggcgcaggtattccgggtcgtgcatcgccatgccggtggcgcattgcaccagcggctcgatgatcacggcagcgatggaggcgtgccgctcggccagcagcgcttcgagttcggcggcggcgcgctgcgccacggcggctgcgtgctcgcccggccgtgcggcccgtgcgtcgggcgaggcaacgaggtgggcattcgcgagcagtggcgcataggcgtcgcggaacaccggcacgtcggtcacatgcagcgcgcccagcgtttcgccgtggtagccgcgccgcacggcgacaaagctttgcttgccgctgcggcccgcattgcgccacgcatgaaagctcatcttcaatgcaatctccaccgccgaggcgccatcggaggcatagaagcaatgacccagcgcatggccggtcaacgcggcgagccgctcggccagctcgacggccggcgcatgcgtgcagccggcgagcatcacatgcgagagcgtgtcgatctggtccttcagcgccgcattgatggccggatgcgcgtggccgaagagattgacccaccacgaactggtcgcgtccagatagcggcgaccgtcgtggtcgaacagccagacgccctcgccccgcgcgatgggcagcggaggcaccgcttcgagccggatgctctgcgtgcacggatgccagacatggcgccggctgcgctgctgccagctggcgtttttcgacggtgcggatgtcgagggagaagcaatcgttggcggcattcgcgcattcttttgggggcaaggcgcgggatcgtatcggcgcaaatccggcacggcaaaccgctggctcacgcgtgaaaagcaccgtacttgaacgacgttggccggcgtaggcagaacgttcagatcaaccccgcgcaactggacggtttcgcgcgcgagggcgggttgatgaggggcatgcaagttgtcttgcagacgataaagatagcggcggaatatcgagttctcacacgccaaggggtggcaattcttgttatcggacacgcggatggcagatctcgaatattggcgaatctttggcctcacgcgacgtccgagccttgcacggcgcgaggccaggacgacgcgtgccgtgggtctattcccacacccgcggcgccgcactgcgccgacaaatgaatgtccatccattccttcgaaggagcacttatgtccaagacgaaccccaacacgcccgacgagcgcggttcgttgcctccccagcacaacaaggccggcaaccaaagcccgaccccccgcaacgagccacgccggaccaccgagagccgtcacgaccgcgatgaccatctcggcagcagcaaccagaaccaagcccggcgcggtggtgccaaaggtgcctccaatcactgagcccggaggcgcctgaacgcccggcacaccgttgcgacaccgtgtcacatcgcaacgaagccacagccgcgctgaacgccttgagcgtggccaccgacgcctgccgggagtgcccgctgggcgcgcgtgccacgcagtcggtgtttggcgagggaccggtcgacgcggtgctgatggtggtgggcgagcagccgggcgacaaggaagacctggtgggccgccctttcgtcggccccgcgggcaagctgttcgaccgcgccgtggccgagctcggctggtcacgcgagaagctctacgtgaccaatgcggtgaagcacttcaaatacgaactgcgcggcaagcgccgcatccacaagacaccgggccagcgcgaggccgaagcctgccaccactggcttgaaagcgagatggaactcgtgcagccgcgcgcctgcatcgcgctgggcgccacggccgcccgctccctgctcggccggcctgtcgcggtgatgaaggagcgcggccagtggatcgaagatgcggcgaccggccgccgcgtgctggtcacgctgcatccctccgccctgctgcgcggcgacccggcgcaacgggaggccgcctgggaggcctggctcaaggacctgtccgtggcgtcgagcctgatgaagaaggctgggggtaaacagcccgcggcaaagcagcgtgcaccgcgttccgccgcaggtcacgcgcgccggcgggtgcgcatggtgatggagtagcgcaacgcctctgtgggcgcgatgctgtgctgccatgcccaccgcgcttcgccgcgcagcatgtagatggaacgcggctcgatcagcaattgaagactggcaggtgcgctggcgctggccggcgggtacggccgcagctgcatcacggcgctgctgcgcagcgaaacaccgacgatgtcttcgaagtcgggcacgtcgcggtgccagccgagcggcgtgccgggcctgtattcggacaacagcacgtgcgtgaaatcttcgggcgccatgtccatccacgcggccacccgttcgcgcagcggatgaagcgcctcgggcagtggcgcgccgggccgcagccggtggttgtcgaagtcgtagctgccgccaaagctgatgccgcggcggcgcgcggtgtattccttgtagcgcatttcgcggagctgaaagccctggacgatgcgcagcagttcgtgttcctcggtgcgcgagagaaattcgcgctcgtaccgcagcccttcgatggcggccgtgggcgcctcgccgaacaggtcgggctcgtcggcaaaccggacgtagctagcggaccgcatcgacgtcttctccttgcttgggcgcgcgcatggggccgcccaggcgcagctcccaccacggcggcagcaactcgcggatctcggcgcgcgcaaagcggtcgtccagcaggtgcagcacgccctggtcctgctcggtgcggatcacgcggccggccgcctgcaccaccttttgcaggcccggataaagataggtgtattcgtagcccttgccgaatcgcgcctgcatgcgctcgcgcgtgatctcgttcagcgcgttgtgctgcggcaggcccaggctcgcgacgaaggcgccgatcaggcggctgccgggcaggtcgatgccctcgccgaatgcgccgccgagcacggcaaagccgatgccgcggccgccctcttcgaagcgcgccagaaattcgtggcgctcggcttcggccatgccgcgcgtctgcgtccacaccggcacgccggggtgcctggccaggaaggccgcgcaggctttctccaggtaatcgaagctgctgaagaacgcgaggtagttgcccggcaggcgctcgaactgggcgccgatgatctcggccacgctgcgaagcgatcccgcacggtcgcggaaccgggtcgatacgttcatggccacctcgacgcgcaattgccggccctggaatggcgaggccacgtcgagcagcatcgtttccggcgggaggccgagcgcatcgcgatagaacccgaagggcgacaaggtgcccgaaaagcaggtgaccgatgcagcctcggcaaagcgtggttccagaaacggcgcgggcacgaggttgcggatggcgaggctgcgctgctgcgggccgtcggcagggcccagcgtgcgctcgaataccgaatggtcgtcgaaggaatcggccagccgggcaaactgcagcgcgtcgaagaagaagcgctgcagcggcccctgcgccgcgtccggcgtggccgcaaagtactcgcccatggccgtgttggccgcctgcagggtgcgcgcgaagcgttcgggtatctcgtcggcggtgtcgtaggcctcggtttgcgattgctgcaccgtgtcccattcgcggtacagccggcccagtgcgccgcgcaccgatgcgggcgccacgcggtgggcttcttcgagtgccaggccgtcgagctgggcggtgtacatgccgcgggcgcgttccagcaggttgtgcgcctcgtcgaccagcaccgccgcgcgccagccatcgtccttcatggtggcgtagagaaaggcgctgccgtcgaagtagtagttgtagtcgcccacgatcacgtcggaccagtgcgccatttcctgcgcgaggaaatacgggcacaccgtgtgcgcgagcgcaatttgccgcagcgcctgccggtcgagccgggcggctcgtgcggcctcttcgcgtgcggcgggcaggcggtcgtagaagcccttggccagcggacacgagtcgccgttgcaggcccggtcggggtattcgcaaaccttctcgcgcgcggtgagctcgagcacgcgcacctgcgcgcacccttcccccagcacgcgcaaggcgtcgagcgccaccgcccggcccgaggtcttggcggtgagaaagaaaatcttgtcgatcttccgcgcggcgcgcgccttcagcagcggaaagatggtggccagcgtcttgccgatgccggtgggcgcctgcgtcatcaggcagcgtccgttgaccgcggcgcggtacacggcctcggccagttcgcgctggccggcgcggaatttgccatgcggaaaatccagacggcccagcgcatcgtcgagcacggcatggtgtgcggcttcgctctgcgcccagacgctgtagcgtgcgcacaagagttcaaagtgcgcctgcagcgcagcccgggtgtgctgctcttccagcacggtttcctcgccggagcctaggtcgaggtacaccagcgcgacagtgatgtgcgcgtagccgtgcatctcgcacagcatccagccgtaggtgcgggcctgggcccagtgcagcgcacggtggttgccgcggatggcatcgaagtcgccgcgaaaggtcttgatttcttcgacgcgcggctcgcgcgggtcgtgcccgtcggcccggccgcgtactttgagcgggccgcaatgggagacgagggccacttcgctctggtaggcctcgccgcgccgtccctgcaccagcgcgtggccggccatgccctcgagcgcgctgggcgcgggcacgaagcgcaggtcgaggtcgcccgccttcgcgccgaaggcgcacagcgccttgacggacactgtgcgggcatcgggcgactctgcctgcggcgttgtggaaagatccgtggtcactgcaatgctgtatgaaacaacagtatagcgacccgctccggcctgtgccgcagaatcgttgtcggggccttctccgacacgaaggtcctcggctttcggcaaaacttcaaaagttttgcttacaaatcctctgtgaatgaaaacccccactgcgatcgaccccgatgatttcgaacgtctgctgagccgcaacctgaagtggcctctgctgggcgggctgatcggcgcgctggtgttcgtggggttgatcgtgttcctgctgtcggccatcagccgcgtcgagcaaaccgaccgcgtggtgcgcaacgcgagcgaactgcagcgccgcaccatcgacatggaaaccggcctgcgcggcttcctcatcaccggcgaggaaagttttctggagccctaccagagcgcattgccaaggatcaagggcgacatcgaggcactccagggacaggtttcggacaacaggcagcaaggcgagcggatcggacgcatcgcggcgctgcaaacggaatggaatgaattcgcgcgcgagatgatcaccgcgcgccgcgacggcggcgactaccaggcgctggtgcggcagggccggggcaagcggctgagcgacgacatgcgcgccgagttcacggccttcatggacacccagcaaggcctgcgcttccagcgcaacgaggaggccaaccgcaccagctggctggtggtgggcgtgttcctgcttttcacgctggcgttcaccggcatggtggcctacttcggccggcggcagctcatgcggctttcggacagctacgacgcggtgctgcgggagcaggccgcgcacgccgcgcggctggcgcagcaagcctggctgcgcagcgcgcaaaccgagatggtgggcgagctggtgggcgagctcagcgcgaacgacctgggccgcaaggtgctcgcgttcttttcgcggcgcctgggcagcgcggtgggcgcgctgtacgtgcgcgagcggcatggcacgctgcgccgcgccgcgagctacggcttctcgatggaggccgaggcaacgccgcaggtcttctcgcccacccagagcctggtcggccaggccgcggccgagaagcgccgcatgctgatcgaacccattcaagccgactacctgaaggtcaattcaggcctgggcgagatggcgccctcggccgtgctgctggtgccggtggccagcgacggcatcgtgaacggcgtggtcgaactcggccttcccggcgcgcccgacgggcggaccgttgaactgctcgacctggtggccgacgacatcggggcttcccttgcggcggcacgctaccgcgaacagctgcaggacgcgctagcggaaacgcagcagctcaacgaagagttgcaggtgcagcaggaagagctgcgcaccgccaacgaggaactcgaggaacagtcgcgcgcgctgcgcgcctcgcaagccatgctggagaaccagcaagccgagctggagcagaccaacagccagctctccgagcgcaccgaagcgctggaccagcgcaacgccgccctgcgccgcgtgcagcgcgacctcgaagaccgcgccgacgaactgcagcgcgccagccgctacaagtcggaatttctcgccaacatgtcgcacgagctgcgcaccccgctcaacagcgcgctcatcctggccaagctgctcggcgacaacccgcagggcaacctgagcgccgagcaggtgaagttcgcggagtcgatctactcgtcgggcaacgacctgctgacgctgatcaacgacatcctcgacatctcgaaggtcgaggcgggcaagctcgaagtggtgatcgaagacgtggcgcccggcaagctcgcccagagcctggagcgcaccttcagcccgctggccgccgagaagcgcctggacttcaagctgacgatgcatccggatgtgccggcgtcgctggtgaccgaccgccaccgggtcgagcagatcctgaagaacctgctgtccaatgcactcaagttcaccgacagcggcgaggtggcgctggtggtttccgccgcacccgacggtggcgctgtgtttgcggtctccgactcgggcatcggcattgcgcccgagcagcaagagctgatcttcgaagccttccgccaggcggatggcaccaccagccgccggtatggcggcaccggcctgggcctgtcgatctcgcgcgatctgacccgcctgctgggcgggacgctggcgctgcagagccagcccggccagggcagcaccttcaccttgcagctgccggcggtggcaccgcaggcgtcccggcaaacgcccgccgcgactgccgcagctgccgcggctgccgccaaggctgcttcggcgcgcgggccctcctccccatctcccgcttcgcgtgccgttccagcggcgccggcgccgccggtggtgataccgccaccccagttttccgacgaccgtgcactgccgcgcgaccaggtgcgccgggtgctggtgatcgaggacgagccgcagttcgcgcacatcctctacgacctggcgcacgaactcggctaccgctgcctggtggcgcacggcgcggccgacggcttcgatctggcgcagcagctcctgcccgacgccatcctgctggacatgcgcctgcccgacagcaccggcctggacctgctgcagcgcctgaaggattcgcccgagacgcgccatatcccgatccacgtggtgtcggcggccgacgacgcgcaagccgccgcgctgcacatgggcgccatcggctatgcgcagaagccggccacccgcgccgagctgacgcaggtgtttgcccggctcgaggaaaagctcacgcagaaggtcaagaccgtgctgctggtcgaggacgacgccgtgcagcgcgaaagcgtgatccggctcatcggcgacgaggacatcgagatcatcgccgtgggctcgggcgaagaagcgctcgccgtgctgcgcaagcgcgtgttcgactgcatgatcaccgacctgcacctgcccgacatgcagggcggcgaactgctcaagcgcatggcggccgaagaaatcgtttcgttcccgcccgtcatcgtctacaccgggcgcaacctcacgcgggaggaggaagccgagctgcagcgctactcgcgctcgatcatcatcaagggcgcgcgctcgccggagcgcctgctcgacgaggtgacgctgttcctgcacaaggtggaggccgagctctccagcgagcgccagggcatgctcaaggccgcgcgcggacgcgaccgcatcttcgagggccgcaccatccttctggtggacgacgacgtgcgcaacatctttgcgctgacgagcgcgctggagcagcgcggcgcggtggtcgagatcggccgcaacggccgcgaggcgctcgaaaagctcgcgcaggtgcccgagatcgatctggttttgatggacgtcatgatgccggagatggacggcctggaggccacgcgccggctgcgcgccgaccggcgcttcgagaagctgcccgtgatcgccgtaaccgccaaggccatgaaggacgaccgcgagcaatgcctggccgcgggtgccagcgactacctggccaagcccgtggatttggagcgcctgttctcgcttctgcgcgtgtggatgcccaaaatggagaggctgtgaaccgcaccgccgcgccctcgcccctgccctctccgctgagcaacacggagatcgagctgcggctgctgatggaggcgatctacctcaagtacagctacgacttccgcgactacaccgttgcctcgcagaagcgccgcgtgctgcacgcgctggcgcagctcgggctccccagcatttcggcgctgcaggaaaaagtgctgcgcgacccggggctcttcggccggctgctgcaatacctgacgattccggtgagcgagatgtttcgcgatcccgcctactttctggcgctgcgccagcacgtggtgcccatcctgcacacctacccctcggtgaaggtgtgggtggcgggctgcagcaccggcgaagaggtgttttcgctcgcgattctgctgcgcgaagaaggactgctttcgcgcacgcagatctacgcgaccgacatcaatcccgcttcgctcgagaaggcgcgccagggcatctttcccatcgagtcgatccggggctacacggccaactaccagcgcgccggcgggcgtagttcattctccgactactacacggccgcctacgaggccgcgcgtttcgacccctcgctgtgcgctggcgtcatctttgccgaccacagcctggccaccgacagcgtgtttgccgagacgcaattcgtttcgtgccgcaacgtgctcatctatttcaaccgcgagctgcaggaccgcgcgctgggcctgtttcacgagtcgctgtgccatcgcggctttctgggcctgggcgccaaggagagcatcgatttctccagctattcggaacgtttcgatgcgcatgcgaagccggagcgcatctaccgcaaggccacatgaaaccgaacgccatgcaatctccgcccaggcgcatcgaggccgtggtgctcggcgcctccgccggcggcatcgaggcgctcttgcggttgctgcacgaccttcccctgccatggagtcttccgctggtggtggtcctgcacctgcctgaagggcatgagagccacctggccgagatcttcgccgagcgcatgcgggttccggtgcacgaggccacggacaagatgccgctcgcgcccggccacatgtatttcgcgccacccggctaccatctgtcgatcgagcgcaaccggcgcttttcgctcagctgcgagccgccggtacgcttttcgcggccttcgatcgacgtattgatggcctccgcagccgacgcctacgggccggcattggccggctttctgctgaccggcgcgaacgacgacggcgctgaaggcctgcagcgcattcatctggccggtggcaccaccgccgtccaggaccccaacgaagcccagatttccaccatgcccgaagcggccattgccctccattcccccgatcacgtgcttcccttgcgcgagcttcgcgccctgctcttgcaactggagtccgcccatgtccattgacgtcgaaagcaagctgctgatcgtcgatgacctgcccgagaaccttcttgcgctcgaggcgctgattcgcgggccgggtcgcacggtgtaccgtgcgacctcggccgaagaggccctggcgctgctgctcgaccacgaattcgcgctcgccattctcgacgtgcagatgcccggcatgaacggcttcgagctggccgagttgatgcgcggcaccgagcgcacgcggcacatcccgatcatcttcgtgagcgcggcgggccgcgagctcaactatgccttccggggctatgagagcggtgcggtcgacttcctgcacaagccgctcgacccgcatgcggtcacgagcaaggtcaccgtgttcgtcgacctgcaccgccaccgcaaggcgcttggccaggagatggaaaaactcgcggccgcccactacaagcaggaagaactggtggagcagctgcggcaaacgcagcgcaagctcgaacacgctgtgcgcatgcgcgacgatttcatgtccatggtttcgcacgagctgcgcacgccgctcaataccctctatctcgaaacgcagctgcggcaaatgcacctgtcgaagggcaagctggagcccttcgcgccggagcgcctgcccgcgatgatcgagcgcgaccagcggcagatccgcaacatggtgcggctgatcgacgacatgctcgacgtcacgcgcatgcggcgggatgcgctctcgatccagccacagccggtcgaccttgccgctctggcgcggactgtggtcgaagggctgcggcagcaggccgaggccgcgggctccatgattgcgctcgaggcgccgggcgaactgcggggcgtgtgggacgagttccgcatcgaacaggtgttgaccaacctgctgaccaatgcgctgcgctacggccgcggcaagccggtggagatgatggtgagcgaggccggcggcatcgcgcacatcaccgtgcgcgaccagggcatcggcattgcgcccgaagaccaggaacgcatcttcgagcagttcgaacgcaccgacgacagccgcaagcacgcctccggcctgggcctcgggctctttatcacgcgcaagatcgtgggcttgcaccacgggcgcatcgaggtgcaaagcacgccgggccagggtgcgctgttccgggtcgagctgccgcttcaggcggaggcaaagactgcaacacaggcgcgggcgtaggcgccctcctactgcatatggggcgacggaccgggatactcgaaggttccttctctcctgatcaaggcgtgccccagtgaatgtgctgatcgtcgacgacaacgtagccgcggcagacctgctgcaggagcttttgacactgcaggaccacaccgcccgctgcgcctacacggcgcaacaggccctggatgctgctgcggcggagcacttcgatgcggcgctcatcgatctcacgctgcccgactttccgggcaccgaggtggcgcggcggttgcgctcggccacgggggaaggcagcccgaagctgcttgtcgccatctcgggattctcggtggaagacgctgccggcgcgggcgcgcgcgagctgttcgaccaccatctgcagaagccgatcgacatcgccgaactgaccgcgatcctttcttcagcgccgcagtgagcaccggcggcgcctagcgcgcgatctcgcggcgcgagagcagtacctcggcaccggcggtattgaaggcgatggtcggcgcggtgaaatcgctcagcggcgcgcccaggccgatctcgccgctgccatgaaggacgcattcctcgcgccgcagcgcgatttcattgctggggccgccgttgccatgaaaccggacccaggtgccgtaggtgctgagatcggtcaggacgcagctgccctgccgcagttcgatgcgcgcatgcagccgcgaaacacgcggatcgttgaccacgaactgcgcgtcgttcacccgacccagatggatcgggagctcttccgtacggaacatggaacgcacgtcgagccatgccagctcgatctgcccgaaggacgaatcgggcagccgaggcggcgtcagcgcggccggcaccgtcaggaacgacgtcagctcctcctgccagtcgatacggtggacggccgacatttcgctgcgcccgcggatggtgatgaggcccaggtcgcgatgccgcaccaccgcctcgctcaactgcgcgatgacggcgtcggtcgcccagatctggccaggcccggccaggtcgctcaggcgcgacgcaaggttgaccgcatcgccgaagcagtcgccctcgacctcgagaacttcgccgcttgcaacgccgatctgcagcgccatgcgcagcggcaccggccatgccatgaggcgcttctggtggtagcgctgcagttcgatcaccgcatgcgtggccgcggcggcattcgaaaagattgcgaatatcccgtcacccagcgacttcacgaccctgccgccgtgggcctggcagatgcttccgatccactgggtaaggcgcgtcaccgtttccgtggcccgggcatttcccatggcttcaaaaaccctggaactcccggtcaggtctgcgaaaacaattgtggaattgacacccatgctttgaaggaactcgatggtggcgtagcggctcgtggttaggtattagaagccacggaatgaaaggcgcaacgggttctcccgcgaaccccttgcgccatggcggccacacgccagcaaatggttatttcctatcacttttgtattcggttaaccacatccgcccgaagtgaagcgtaaagtgtgttgtttacaaacaagaaacagtgttccagatcttgtgaattgccgaactgaggcttaaggtagcaaccgttctggtttccggcaatacgcttttggtgctcatgtcgtcccttcgtcgctttctccgccttttgggaattcccggcctggggtctggccgcgtgggagaacatcaacttggccgcatccgcacagccatgctgtcggtgctgcaggcgcatgggggccattcggtccagcgcatcgcccagcgcgtgcggtttgcaaccgacgtcgaggcactctggtatttgcgccaggacgtgatggtggcgctgagcgccatcgacggcgaggccgcggcccgtcgccagatgaaagccatcaacagcatgttcaagggcggcctgccccgttcgatggggccgcgagcccaccagcgcatcacgcactgagcccaccggggccgcggcagctttcggctgccacttttgcattacccgttcttttcctggtgcccgcagtccgcctgctcaatgggcgtgcgcgtggccatggtcgtgagcatgatcgtgctcatgggcatgccgatggccccacaccatgaagacatcgcggccttcggcagccagttcgaccttggcgcccacggggagcagcaccttggtctggacgtggccgaacggcaggccggtgaggaccggcaccttgagcgcggcgcgcagccggtcgaccaccgaatcgaatccgaagccgcggtcgtagcccggcaccttgcgcatgccggtgaactggccgaacacgatggcgcgctgccgtcccagcacgccggccatgcgcagttgctcgagcatgcgttcgatgcggtatggatgctcgttggtgtcctcgatgaagagcacgcccttgtcgactgccgggaagtaaggcgttcccagcaggctggtgagcacgcaaaggttgcctccccacagggtggcgtcgtgcacgggcttgaccttgagcccggcatcgcgcaccggcatgcgccagccggtgccttcgccctgcccgctcacgaggtcgtcgaaacaggcttccatgatgtcgtccgcgccgccttcggcgccgaagtcttcgccgaccgctgggccggcccaggtcacggccccggtcttggcgagcagcgcgctctgcaaggcggtgaagtcgctgaccccgacgaattcggttccgtgctggatggccttggccacggccttgtagggaatggcgtccaggatgcgcgtgagcccgtagccgccgcgcgcgatcagggcaatgtcggcaccgctggccgcggcgcggccaatggcggcgagccgcgtcgcgtcgtcgcccgcaaagcgctggtatacggcaagcgccgcttcgtcgatttcgacttcatagcccagggtcttgagtcttgcgacgccgcggcggaaggcggctttgtcgcgaatcgcgctggcgggggaatagatgtagatgtgtttcttggtcacggcgccgagtatcccattgcgctgcgcacctgcccggcaagcaacgccgcctgcgcggcgctcggccccgaggacgacgccaaggggccgagcgcgcgcagcgcggcctggtagccgcggtccgggaacggcgcccgccaggcgtcgccaacctgttcgccgccttcgggagccaggagcatggccgcgaaatggcccggccttgcgccctgcagcagcgcggcgagcccggtggccgcggtgctgtgcaccagcaccacgggcgccggtgcgatgcggtcgagccattcgatcaagacctggcagtgccattcgagccgatgcgccgcttcgcgcttgggcttgtcgctcttgccgaagccgatcaggtcgggcaccagcgtgcggagtccgggcataccggcgagatggcggaaaaagtagccccattcgccggggccgtgcaggcagacgcagcaggccgtctgcccgtcgcggggggcaccttcgtcgacatagtgcagtcgccagccgttcagggcgggcaggtcctggacgtagtgcggttcgaaggcgtagtcgccaagcgcgccgaagcgttcggccggcgtgcgcagcgcgtcgtcgcgcaagggctcggcctgctcgcgcgccgtctcgcggcgctgctggaaaaattgctgcagcaccgcgctgcactccgccgccagcacgccgccctgcacttgcgtgcggtggttcagccggggttcggcaaaaagatcgagcaccgaaccggccgcgccggtcttggggtcggccgcgccgaacaccacgcgcgccaggcgcgaatgcagcatggcgcccgcgcacatggcgcagggctcgagcgtgacgaacagctcgcagccgtcgaggcggtagttgccgagcgccgcggcaccggcgcgcagcgcgttgatttcggcgtgggcactcgggtcatgctgcgcgacgggcgagttgcggcctgttgcgatgacctggccatccttgaccagcaccgcacccaccggcacctcgccggcctcggccgcccgccctgcctcggcgagcgccagcgccatccagcgcgcgtcgccggtggtctcggaaggcgtcttcggctcagttgtcatccggcatcttgcgcgcctgcgccgcggcgtcgagcgcgtccttgacctgcttttgcacctgctgggcctgcgtgcgcgcgtcggcaggcgcctcgcctggcgcgggcgcggcggcaccggggaccggcggcaatacgggggccgcggcggaggtcagctgcttcttcgcgaccatccccacgatcacgagcgccagcaccaggccgagcaatccgaacatgcgcatctcagcttccttccgccacgctcgcgtccgccgtcgtcatgccgaggcgctccatccacaccgccagtgccttctcgtcgggtgtgccggcgctgtagacggcatgcatggcggcatgcgattcgcgccgatgctggttgagcttgaccttgcactgcaatgaacgcacgcgcagctcgaagcccacgatgccggccagcatcttgagctggaattcctcgcccaggtcgcgccactgctgcgcgtagccgggctcgtgctcgccgatgagcttcttgagcagcgcatccttggccatgggctcctcgatcagccgggcttccacggtgcaatgcaccaccaggtaattccacgtgggcacgcgcgcgagatcggggtagaccgatggcgacaggtacgaatgcgggccgagaaaagtggcgaccgcctgcggccggtcctgcaggtagcgccaatgcgggttgggcttggcgcagtggcccagcagcaccagctggtcgccctcctgctgctccgcgaccagcggcaggtgcgagacgaacggcaggccttcgtcgtcgttcgagatcaggctggcgaacggatgtgcgcgcatcagctcgagcgcgatggccgggtccttggcgttgaactgcgggggcatgtacatgggtcggtttcctcttggcgagccaccgattgtccccgagccgccgctatcttgtcgggcgcggcgcttccagcagcttgaccatggccgtgtagccgcgggccttggccagctgcagcggcgtgttgccctggcgatcggtcagcttcaggctggcgccggcatcgatcagcgcagccagcgtgcgctggtggcgcgggccgccgtcgccgagcacgatggcttcgatcaccgccgtccagtgcaggttgttgacgtggtcgagcggcgcgccggccgcgatcagccggcgcacgacctcgtcgtggcccaggtgcgcggcagcgatcagcgcggtgccgtcgtagcggctcgtcacctgccccgcattggccccgagcgacagcagcagcgcgagcgtcgcggggtcgtcggccaccgacgcgatggtcaccgcgtcgtagcggtcgtcttcgagcgcatcgaggctcgcgcccgccttggccaggagcgtcaccgcctcgcgctgccgtgcatgggtggcgacgtgcaagggcgtgcggccccgcgcatcgcgcgcatcgaggttggcgccggacgcgaccaggctcttgagcttcggcaggtcgccatgccaggcggcccggtgcagcccttcataggccagcacctcggccgacagcggcggcacctgggcccacgcgccggccgatgcgcccgcgccgagcgcgaccgccaacacgccggaccagataccgcgtttcatcatcatcagcccagcaggcccttgaccttttcgagcgccgcgttggcacactggtcgtccaggtggccgccgggcgcaccgcccacgcccacggcgccgatcacgtcgttgcccgacttcaccggcacgccgccgcccagcaacaggaagcccggcaggtagacgaggttcgcggcgccggggttcttctgcgcgccttccatcatgggctgggtcgcgctcttggccgacgccgaggtccaggccttgcgctcgctcgacgccagcgtgtgcgggccggcgttgtcggcacgctgcacggcgcgcacggtgccggcgcggtcgaccacggtggcggccacgttgtagccgttggcggcgcaggccgccacggcctcggccgcgatctggttggccagtgcgagcgagatgttcttttcggtgcgcacggcgggcgccggcgtctgggcttgggcagccgatgcggcgagcaggacagcgaggccgccgaggcgaagaatggaacgcatttttgatttctccagtggatgcagggtgattgcgccggcaagttgccggcggctgcgccactgtagaaaacaccggcggccgaggccattcgtacggctacgcccggtgctccgtagaactacggagcaccgggtttcagtcttccccggccaccagcacggcgtagcgccggatcagctgcgcgagcgaatcgcagtcgagcttggcaaagacattggcgcgatgggtctcgaccgtgcgcggcgacagcgcgagcgtgcgcgcaatttccttgttggtgcggccctgcgcgatgaaggccagcacctcgcgctcgcgctccgacagctgtgcgacccgctcgcgcgccgcctggtcggcctgcgagcgttcgcgcgagcgcacatgctggcgcaccgcctgctgcagcgcctcgagcagttgctcgtcgtccaccggcttctcgagaaactcggccgcgccggccttgaaggcgcggcggcacatctcgaccgtgccatggccggtcagcatgatcaccggctggtcgacaccctgcgccaccagccggtccagcacggtgagcccgctgatgccgggcatgcgcacgtcgagcacgatggcgcccacgcccgcacggtcgaagccgtcgatgaaggcttgcggatcggcccagccctgcacccgcaggccgaccgtgccgatcagcagcgagaggctttcgcgcaccgcctggtcgtcgtcgatcaggtgaatgagcggcgactgcggctcatgggtggccgaggcattcatgccggatgccccgccgaccgcgccaccagaggcagcgccagcgtgaagcgcgcaccgcgcggcgccacgttggcggcgctcaggctgccgcccatgccgctcgccagcgtctcgctcaggctgaggccaaggcccaggccgccctcgcgcgtgctgaagaagggctcgaaaaggcgcggcagggcttccggcgcaatgccgcggccgttgtccgtcacggtcagcacgccctcctggccgttgcggccgaccgaaaccgccagccgccgctcggacgcgggcacgagttccagcgcctgcaacgcattcatcagcaggttgtgcacgatctgctcgagcgccacggcgtcggcctgcacgcgcaccggcgcttgcgcggtggcgtcgaactgcgccgacaccgagcgcttggcgaactccggcgccagcagatgcatcgcgctgcgaaccagctcctgcagcacgagcgggcgaacttcaccctcggcctcgggccgttcgatgacacggcgcagccggccgaccacgccggctgcgcggcgggcctgctcgaccgcctgccccatggcatcgcgtgccgtggccaggtcgggcggatcgtcgtcgagcaggcggcgcgcggcctgggcgttggcgagcaccgccgtgaggggctggttgagttcatgcgcgaggcccgccgagagttcgcccagcgcgttgaggcgcgccacctggccgagccgcagcagctcttcggcgcggcggcgcgcaatgcgctgccgctgcgcggcccaaagacccgccagcaacaagcccacggccgcggcccagccagccatgctgcgccagggcagttcgccccagcccacatggcgcgcagccaccagctcgaaaggctggctcggtgatgccagtgccttcgtgagatcgaagcgccagccgccgccttccgccggccggccgggctgcagcaccagttgctgtccgtcgcgctgcaggccgaggcgcaccgggctgcgctgcggatccatgggccagtcgcgccacggcacggagccggccaagtcgatctcgagggcgtagctgaacggcgtggcgccgatcacgagctggtagcggccgcgcgcaagatcgagcgccgccagttcggcgcggcgctggctgcgcgaacgcgcttctgcggcggccaatgcgccggcctgcttgtcgtcgggccagggctcgtcgcctccacgccgctgcacgcgcaggatcgacggatagaccgacggcaggcgctgctccggatggtccgcgccggtgccgggctccagcagcgcgaccgtggccagcaccgcgtcgtactgcaccacctgctggctcatgatgcggtgggcaatgcgcacgtcggagccgaaatcctgctgcatctgcgcgagttcggcacgcgcaagccacaccgcgcccacccccgtcagggcaagccatgccagccaccatccaccctgcgcgcgcaaccactgtttcatggcgcggattgtgcctctcgctgcgggcccggccgatgttggccgagaatgcgggcccagacatggctgaactgcaggactccctttttcccgatcttccgcgcccgcccgaggcgcccgcgcccccgccgcctctggaggccgagccagccgccgagccgccggcccgcaagaagacacgcggtgccgccgtggcgccggcgccggtcgatccggcactcgtcgaattggccgccgcgctcccgcccgggcttcggctcggcacctcttcatggagttatcccggctgggccaatctcgtctgggacggcgactacgccgaaaccgtgctctcgaagagcgggctcgccgcattggcgaggcacccgctctttcgcaccgtgagcctggaccgcaacttctaccgcgccctcaccgcgagccagtacgcacgctatgcggccatggtgccggacgacttccgcttcgtggtgaaggcgccgagcctggtgaccgacgccaccgtgcgcgacgaaagcggccgcggaacgcaggtgaacccggtgttcctgaacagcgagatcgccatccaggagttcgtgcagcccgcgctcgaaggcctgggccaccgcatcggcgcgctggtgttccagctgagcccgattccgtcgcaactgctggccgaccagcccgccctcctggcgcgcatcggcgacatgctcgaagcgctgcccggtctgaagccagccgcacccgacgccgtgattgccgtcgaagtgcgcgacccgcaattgctgtgccccgccttcgccgacatgctgcgcagcgtgggcgcgaccttctgcatgggcctgcacgcgaagatgccgccgatcgaagaccagctgccgatgctgcgcgctctctggcccgggccgctggtgtgccgctggaacctgcaccgccgccatggccgcttcggctatgaagatgccgaaaagctctacgggcctttcgacaggatcgtcgatcccgaccccgagacgcgcgcggcgctggccaaggtgattgccggcaccacgcgtgccggccagaacgccttcgtcaccgtgagcaacaacgccgagggatgcgcgccgctgacgatcgcgtcgctcgcgcgggacatcgtcgatctgctgccgcgttccgggtagacaggaaatcctattcacgtagcatgaccgtgactcccacacaggaacacttggtcatgagctccctgtcattgctccgcacccttttcaactaccgcgcctgggccaacgacgaactgctcgaaaagatggagggcttcgatccggagcgacacggggacgcgcggcacgccgccctccgcctgatgaatcactgccatgtggtggaccagatcttcgcggcgcacctcaccggcaggccgcacggctttgccgcggacaacacgcaggacacgcccacgctgcaggaccttcgcgcctctgtagccgcgctcgaccgctggtacctcgactacctggaatcggcgacgccggaactgctctgggaacgcgtgcgcttcaccttcaccgatggcgacaagggtttcatgacgcgcgaggaaatgctggcccatgtcgtcacccacggcggctaccaccgcggcgaggtcgggcggctcatgtcgcagcaatcggtcgggctgccatgggacaccttcgcggtgtacctgcacagcaccgacccgtcgcgccggcttcaggccgcgtaggcctcaggccgtgtcgcccttggcggcgaccgtcatctccagctcgacgctcgcgttcttcggcagctgatagacgccgaccgcggtgcgcacatgcacgccggcatctccgaagacgcggtgcagcaggtcggatgccgcgtcggccacttcgctctgctgcgtgaaatcggcgctgcagtgcacgaagacgccgacgcgcaggagcttgtcgatgctgtcgagcgaaccaagctcgcgccgcagcagcgtcaggcagcgcaaggcgcaaatctgcgcgccttcgcgggccttctcgagcgacacctgctcgcccacgcggccggtgacgaccaccgtggtgcccacgcgcggcacctggccgctggtgtagagcgtgttcccgtcgcgtacgacgggtgcgtagtggccgccggcgacaagttcgccctcgaagctgtgacccagctcggcggcgattcggtcggccatctggtctctggtctgcgctgtcatggaggctttctcgaatgaagcctcattgtcgcgagccgtgttgcgatgaacagatacagattgcgcggactcggcacgcaacagttggcccggccttcacgattttgcggaagggtccggaatgggccttgcaggcggccaccgccccaaaacttcatggacgctcttgcccacgcggctgtcgaccagcgcaaacgaatcggcggcccaccggatgggctctatggcatgcggatcgatctcgctgggcgtgtaggcaagagtcatgtgaggcgtgaagccgcgctcgggcttgaaccccgcttcggccaacgctttgcccaggcgctgcctgaacgcggccagggctgaagtgccgtcatgcccgcacagcacgaaggccttgctcttttcgaaacgcatcgcttcgtcgaacaccacgtcgaaggatggcggcgccacggtggcggcagcctcgagggcggcctgcaccagttcgcgaggcacttcggcaaacctgccgagatgatgcagcgtgacgtgcaggcgatgcaccccggtcatctttgctttcagcgcatgctgtgcaccgaggcgcgcaccctgcgcggcgatgcgctcggcatcggcgtgatgcggaaagatcgcaaagaagagcgagtgagccggctgctccctgcgcggtgcggcgctctggggtcgacgcggcggcgggtcttcgaacatttgcaattctgcatctcctgcaaataggatggctgccctgaagcggcgcggcgaatggtccggccatcacaacatcacatgaatgcattgatcaatggccccgacggccacccccgctgccgctggtgcgcaaccgcacccgaattcctggcctatcacgacaccgaatggggctacccggtggcagacgaccagcgcctgttcgagaaaatctgcctggaaggctttcagtccgggctgagctggcgcaccatcctggccaagagggagaacttccgcgcggcattccacggtttcgacttcgacaaaatcgcccgcttcaccgcgcgggatgtcgaacgcctgctgcaggacccgggcatcgtgcgccaccgcggcaagatcgaggccgtgatccacaacgccgcccgggcgcaggaactcgtcgcccttcacggctcgctggctacattcttctggagccatgaaccggatgcggggcagctcgcggcgccgcagaccgcttcgacctcggaggcgtccattgcactgtccaaggcattgaagaagctcggctggaagttcgtcgggccgaccacggtatacgctttcatgcaggcgatgggcctcatcaacgaccatgcaaccggctgcgtggtccgggccaaggcggcacatgcgcgcagcaggttcaaaagtccggcgcgctgacattctggaggagcggaactcgcgcctgcggcgcggctctgacggaccatgaacgccacacccgaacacggccttccccggcgcaccgtcgctgcagcgctggttgccgcgcccgcactctggctgggcgcccgcgcgcagccggcggcggcccggctcgcaacgccttcgcagaccgagggaccgttctatccggtccggctgccgcaggattccgacaacgacctgctgcgcaacggcacgctgagctatcaccgcggccagccggcctgggtcgacggcaccgtgaccgatctggacggcaagccgctgcgcggcgcccaggtcgagatctggcaatgcgacgaaaacggccactaccaccacccgggcgacggcgaccgggccgacgccgcttttcagggcttcggccgcgtcgccgtgggcgaggacggcagctggcgctttcgcaccatccggcccgtcgcctacagcgggcgcacaccgcacatccacgtcaaggtgaagctcggcacgcgcgaactgctgaccacgcagctctatgtggccggcgacccgggcaacgcgcgcgactttctctggcgcaatctcccccaggccgcgaaggacgccatcaccgtgccattcgagcgcgggccggacggcttgcaggcgcgcttcccgatcatcgtggcggcctgagggagttcagtctccggctgagtctgccttccacatccgaacaggtggtcgattcaactcgccgatcgggcctagtccctacccgtcttgcgggagtcatacaggcgtcatccaggtcgggatcaatgcgcggaaccaatcacatgcaggccgtctgcgcgcggccgcctttgccacgccatgaaccccagccaccctgttcacgtcctcttcctctgcaacagcaatgcggcgcgcagcctgatcgcgcaggcgctgctcaatcacctcggcaagggccggttcgtcgcgtattccgcgggccatgcgcccacgccggacgggaagcccgatccccgcaccatcgaagcgctgaagggtgcgggcctgccgaccgatgggctgcgcagcaagagctgggacgaatacggcctggcctcggcgccgcacatggacctggtcgtcacgctttgcgaccaggctgcgggcgaaacctgccccgtctggcccggccaccaacccgccgcggcgcattggtcgcatccagacccccgcggcgaaagcgccggtgacgaggtcgatgccttcgtgaagacgatgcatgcgatccgccggcacgtggaactgctggtcaacctgccggacgagcgcatcgagcggctggtgatccagtccgaggcgcggcgcatcggcatgtctgccggggagcacgcctcccctaccccgtagatcaggcaggaagcttggtgtcggtgaagcgccggatgggctgaacgaagctgatgtccgcaccgtcgagcacatcgcgcccttcgaggctttcaaatttgagccccgtctcggcttcgatgaacgaaagcgggcgctgggacgtagcgaagtcctccaggtcgcgcgccacccccgaatcgagataggtgccctggctcatcaagtaggcgatggcggtcagctcgcccgtcgcctcgctgatgaacccaacgactttccagaactcccgcggaatctggatgccgaatctctcggcatcgtccgaccggagaatgggccctgtgaagacgctgatgcgcttgtcgtcgccctgggcgttgccgaggatgtagtcctcgaggtcgccccacagtccgtcgttgaaaggctgccactgggggcatgcattggttgcaaagaaggtatcgatgttggcccgctgtgcggtcgccagcgaaccccagttcggatcctgcctgcgcgtcatgtggccgcgggagaacttcctgtcctgctcgggaccataggcctcccgcagcatctggtattccttcttgatgcggccgtcgtagttccaggtatcgtggcgcggaacgttcttcgacttcgacccatcgacgttgcatgcggaataaagcggcacgcggcgtgaaatgcactgcaccgtactgaagtgctggtacttgagctcgaaggagccgtcttccagccttgcgatatcgtccatcgatatggcgtcgctcatcgacggcagctccacgcggttgtcggctccgaagaagtcaggtgcgtagccttgccggcccctgaagaattccggcggtttgggcgttgcggcaacgcgctggattccggtccatgagttgctcacgacctggacgtctgtatcggacatggaacttcctctccaaaaaacccatgaccaccagcggccatggacgcctcgcgactatttgccgagcttggcgcgtgcgtttttcagattgaagacaggcttgcggatttccgcaaaagtcggttgagtcacgacccattcgggattctgttcaagcgccgccagttgcgcgtcgtcgtcgatctgggcctccaccagggtgcccgtcttcggcgtcagcacgacacccggcacgcaacgccgcagccgcgcctcggccgacgacttctggtcgggactgcctgtgtaggtcaacaccacgcttgtcacttcagaactccaaacccttcgtactcggccgaccaacccacctttcgggctgcctgcgacagcatcttgacgatggcgtcggccttttcaggacctctgggcatgttaagcaggttctgatcccctgacaacagacgggccgccatgcccgatgtgaacggtgtcgccatcgaagtgccggacatcatcgcgtatcgcccgccgggaaaagtcgacagaacggcgacgccggggccgatgaaatcggtcgaaagcccgtagttcgagaactcggcaacgaactccttcttgcggcggatctcgctctcctgaaagctctcggggcaatccgccggaaacgttccgtcgcggccgagcgcgccgaccgccagggtgtggctgtaccgggcgggataacgcagcagcgactgcccgtcgttgccggtggctgcgaacacggcaatgccggcgttgcgcgccttttcgagaatgtccggcatctccggcatcggctcgaggctgcccatgctgatgttgacgatgtggcagccgtcgctgatcgcgcgttcgagcgcgctggcaatgtcgctggatttcgcacgcccgcgttctccggttttggggcacacacggtaggccagcagacggcaggcgggcgccaggccgtagatcccggtgccagcggccatcttgcccgcgatgatgccggcgacgtgggtcccgtggccgatgccgttgtcgaggaaatccgctgcatcgtcgccggtgacgaagcatccgccgcccgccacggcgatgtcggcatgcggcccgacgccgctgtcgatcacgccgaccgtgacgcccgctccggcctggggatcgtaaggcgcgtagttcgccagcagttggaaggtatcgggtgccagcgccgtggtctggacatccagccgcttcggtgccgcgacgcggtcgaatcccttcaagaagaccgaccagtgcgtgtgttccggctcaaccaggatcatttccactcgcgggtagagcacaggaattccaagcctcgcgaccccctggctgtcggtcaccgcgggcacatgtgcgccatcccaatccacgagcgccttgacccgaatacccggcacaggtttgcccagcgagtcggcaaggcgcaattcgaacctcttgaccttggcccccgccgcaacctggatcgcgatggattccagttcctcgcccagcggccggatgtattggaggtatgcccatgccgccggtgcaacccgcagtccgggcgtattccggcgcatcgccagcaaggcggacgaattggccttcatgaccgacacgccgtccagctgcttgacgagattcatccggggagcaccccggccttgcaccccctgcccgagcacctcttcggcatggcccaggttgatggcgcccagcgtcgccagctcggtaccaccgggcgccgcgctcttcgaaggccatacgatgacgtcgtcggaaaatttaggctccgccgcgatgcggcgcagacgcaattcctgcagcagtcgctccattttctcgccgtccgacttcgacatggcgccttttgcgtgctggtaggcacgctcggttcgacgcggcgagccggccagtctcaggacatcttgtcgcttgctcgctgcagccatgcgttctctccttgttgccccgacttatcgcaccagggcgtttcaagtcgatgaatttcgcacgcagggaagagtagacggccttgggcgcgaaggcccagtgcacacattacgttggtggaccgggcgcacggcttggccgggccggaccttggatcactcccactcgatcgtcgccggcggcttgctcgacacgtcgtaggtcacgcggttgatgccgcgcacttcattgatgatgcggcccgacaccttcttgagcagcgcgtacggcagctcggcccagtcggcggtcatgaagtcgctggtctgcacggcgcgcagtgcgacgacgtagtcgtaggtgcggccgtcgcccatcacgcccacgctcttcacggggaggaacacggtaaaggcctggctcgtgaggtcgtaccagctcttgccgctctcgtccttgaagttgcgtagttcctcgatgaagatcgcgtcggcgcggcgcagcaggtcggcgtattccttcttcacttcgccgaggatgcgcacgcccaggcccgggccggggaacggatggcggtacaccatctcgggcggcaggccgagcgccacgcccagttcgcgcacttcgtccttgaacaggtcgcgcagcggctccagcagcttgaggccgagctgttcgggcagcccacccacgttgtggtggctcttgatggtgacggccttcttgctcttggcgccgcccgactcgatgacgtcggggtagatggtgccttgggccaggaacgtggcgcccttatggccaccatcgcccgctttgagcttggcggcctcctgcttgaacaccgtgacgaattcgccgccgatgatcttgcgcttggcttcagggtcgctcacgccggcgagcttgccgaggaacaggtcgctggcatcgacgcggatcaccttcgcgtgcagcttgccttcgaacatctccatgaccatgtcgccttcgttcaaacgcaagaggccgtggtcgacgaacacgcaggtcagctggtcgccgatggcgcggtggatgagcgcggcagccacgctcgaatcgaccccgcccgagaggccgaggatgacttcttcatcgcccacctgctcgcggatcttctccacggcttcggcgatgtggtcgcgcatgacccagtcgggcttggcttcgcagatgccgagcacgaagcgctcgatgatcgccttgccctgcaccgtgtgcgtcacttcggggtggaactgcagcgcgtagtagcggcgcgcctcgtcggccatgccggcgatggggcagctgtcggtgctggccatgagcttgaagcccggcggcagttcggtgaccttgtcgccgtggctcatccacacgttgagcatgccgtggccttcgggcgtggtgaagtcggcaatgtctttcaagagcgcggtgtggccgtgggcgcgcacggacgcaaagccgaattcgcgcttgtggccgccctcgaccttgccgccgagctggtgcgccatggtctgcatgccgtagcagatgcccaggaccggcacgcccaggtcgaacacggcttgcggcgccttgtcagtggtctcttcgtagacgctggcgtggctgcccgaaaggatcacgcccttgaggtggccgtcggccgcatattcgcgcacccattcgtcggtgacgtcgcagggatgcacttcgctgagcacgtgcgcctcgcgcacgcggcgggcaatgagctgcgtgacttgcgagccgaaatcgaggatgaggatcttgtcgtgttgcatggagaagactcggtcagagcgttgaaatgtcgaacagcttcacgcccgcttgcggcgcggcctggatgagttgctcgtcgaaagtggcgagcgggagattgagcgagcgcgcgagccacagatagcccgcgtcgtagagcgacacaccggcgtcgatggccacggccagcacggccttgtgctgcgcgggggcgagttcatgcagctcgacgcgatggcggatggcgtcgagcacgctccacagcccttcgaccgccgacgcgggaatgcggccgctgcgcacgccgttggcaaggatgttggcgcactcccactgccaggcattgggcgcctgcggctcgacctcgtcgcggcgaatggcggcgtagagcttgcgggtgtgttcgctggcctggtcgggcagcagccaggcggcggtgacggaggcatccatgacgaaggctgtcacgattggcgcccttcgtcgagcaatgcgcgcaccgaaaggccaggctggatggtggcgtgcagcgcgtcgatctggccgagctcgcgctcgatctgctcgtcggtgatgaccggcttgcgccgcaccggcagcatgcgcacgacttccttgccgtggcgggtgatgcgaacctcctcgcccttttcgaccaggtcgatcagggcggagaagttgttcttggcttcggcgatgccgatggattgcatttgggccagaaagtttgaatctggcccaaattctaatgctaatctggcctgactttcaaggtctggccagattgggcttactcagcgcgatagttcggcgcttccttggtgatctgcacgtcgtgcacgtggctctcgcggatgccggccgtggtgatctcgacgaactcggccttgttcttcatgtcctcgatggtcgcgcagccgcagtagcccatgctggcacgcaagccgcccgacatctggtagacgatggacaccatcgaacccttgtagggcacgcggccttcgataccttcgggcaccagcttgtcggcgttgggattgccggtggtggattcctgaaagtagcggtcggcactgccctgctgcatcgcgccgatggagcccatgccgcggtagctcttgtagctgcggccctggaacagcacgatctcgccgggcgcctcttcggtgcccgcgaacatgccgcccatcatcacggtgctggcgccagcggcgatggccttggcgatgtcgcccgaatagcggatgccgccgtcggcgatcagcggaatgccggtgccctgcagcgcggtggccacgttgtcgatggccatgatctgcggcacgcccacgccagcgacgatgcgcgtggtgcagatcgatccggggccgatgccgaccttgaccgcatccgcgccggcatcggccagcgcacgcgcggcatcgccggtggcaatgttgccgccgatcacgtcgacctgcggatagtttttcttgacccagcgcacgcgctcgatcacgccggcgctgtggccgtgcgcggtgtcgaccacgatggcatcgacgccggccttgaccagcgcctctacgcgctcttcggtgcccgcgcccacgcccaccgccgcgcccacgcgcaggcggccgctcgggtcgcgcgcggcgttgggaaagctggtctgcttggtgatgtccttgacggtgatcaggcccttgagctcccacgcgctgttgatgaccagcaggcgttcgagcttgtgcttgttgagcagcgccttggcctcggccaaggtggtgccgtcgggcacggtgatgagcttgtcgcgcggcgtcatgatctcgctcaccggcacgtcgtagcggttctcgaagcgcaggtcgcgccccgtgacgatgccgaccaccttgccgccgtcgagcaccgggaagcccgagatgccgagttcgtcggacagctgcatgacctgcagcacggtgtgcgtgggcgtgatcaccaccgggtcgcgcagcacgcccgactcatagcgcttcaccttggccacctgcgcggcctgctcggctgcggtgaagttcttgtgcacgatgccgatgccgccttcctgcgcgatcgcgatggcgaggcgcgcctcggtcaccgtgtccatcgcggcggagaccagcggcagattcagcgcgatgttgcgggaaaaacgggtggcgagagaggtgtccttgggcaggacctgggagaacgctggcaccaacaacacgtcgtcgaaggtgagcgctttgccgagaaggcgcatgggtgaagctccaaaagacggattgtagcgatgctcggtacttacccgccctccagggggcttcagccggcctcgttctggccggcaaggcggctgaacgtagccaatttccaactcaccgcgagcgaaaagccgcagtccggatgttgccaaacgtaaggcaacgctaaactcgctgcatgaaattcgcgcattggctcgtactgggatgtgtttgcctgctgccgctcgcggccagcgcgcaatggcaatggatcgacaagaacggcaagaaggtcttcagcgaccaggcgccgccgccggacgtgcccgagaagaacattcttcgccgctccggcacgccgccgccgcgcggcggcttcacgcaggcccctgccgaagccgaggcgccggaggcggcagccgccaaatcgcgcgaagcagcggccgcgcccaaaccggcgggtgtcgacaaggaactcgaggaaaagaccaagaaggcgcaggctgaagaaaaagccaagcaggcggccgaggcggagaagaacgccaaggtcaaggccgacaactgcgaccgcgcgcgccagggcaaggccacgttcgacagcggcatccgcgtggccaaggtcaacgccaagggcgagcgcgaaatcatggacgacaccgcgcgtgccgccgagcagaagcgccttcagtcgatcatcgagagcgaatgcaagtaaccccagcaagcgggccggtttttcagtagccggccttgccgcccttgcggcggttggcaaaaaggccggtaccgcgcgcgccctggcgctggaagcgctcgcggcgcgccaccttgggatcgacggtcaacggccggcacagctcgacgcgatcgccgtccttcagcgcctggtcccagcccacctccctgccccagatccccggtgtcatggcctcgcgccagtccagctgcggaaagcgctgcgcaaggtcgctggccttcacggcatcgtccacggtggcatcgggcgccagccgaaggacttgctcgaacacctcgcgcggcgcgggcgagcagctcagcgtgacttcgatcatcaggaagcgccgtagacctgctcggcgcgcttgacgaaggcttcgaccaggctggaggcgatggtgtcgaacaccggccccaccagggcctgcagcgcgaagttgctgaagccgtagctcatgtgcagctcgacgcggcaggcgcgctcgccgggttcgcccacgggcgcgaatttccagaggccgtcgagattggagaacggcccgtcgacgagcttgaggtgcacttcacgcccgggcacgtgggtgttgcgggtggtgaagctctggtgaagaccggcgaaagccaggccgacttcggcagtcattccggcttcgtcttcctcgatgatccgggacttgtcgcaccacggcaggaactgcggatacttctccacatcggtgacgagcgcgtacatctcttcggcgctgtaccagatgaggacggacttgttgactgttttcatagaatcgggacagcgtgcgcgacggattgtattgaagccatgcgcccccatcttcccgagccatggccaccaagaaacaagatacctcctcccgcattgccgacaacaagaaggccgcgtacaactacttcttcgaagaacgcttcgaagccggcatcgtcctcgaaggctgggaagtcaaatccctgcgcgaaggcaaggtccagctgaccgacggctacgtggtgatccgcgacggcgagctgttcgtcgtcggcctgcagatcaatccgctcaagagtgcttcgacccacgtcaaccccgactccatccgcaccaagaagttgctgctgcacaaggaagagatccgccgcctggtcggcaaggtcgaacaaaaaggctacacgctggtgccgctcaacctgcactggaaagccggcaagatcaaactcgaaattgcgctggccaagggcaaggccgagcacgacaagcgcgacaccatcaaggaccgcgaaggcaagcgcgaggtcgagcgcgcgatgaagagccgcaaccggtagttcttttttgcccggcatggaataaaacgcgcggtgcaggcgtttgtgcggtgtcatcggatcgtcggtgccaccaacccaggagtcattccatgtcgccttttcgcgcttcctacgccggcattgccgccgcgctgctgagcagcctgctcgcgcttcccgcattcgcccagcccaaggccgccgacggcgcgttggtcggcccgaacggcatgacgctgtacaccttcgacaaggacacggccggcagcggcaaatcggcctgcaatggcggctgcgcggccaactggccgcccttcatggccgccgacagcgacaagccggccggcgacttcaccatcgtcacgcgcgacgacggcaagaagcaatgggccgccaagggctggccgctctactactgggccaaggactcgaagccgggcgacaagaccggcgacggcgtgggcggtgcctggaaaaccgccaagccctgaccgcgacgcaccaatcgcctttccgtggacgcccgcctgctcgccgaacagattccgagcctgcgccgctacgcgcgcgcgctcacgggcgatgcatgggcggcggacgacctggtgcaggacacgctcgagcgggcctgcggcaagtggcgtctctggcgggtgggcagcgacctgcgcgcgtggctgttcacggtcatgcacaacatcttcgcgagccagcggcggcgcacgccaccgccgcacagcgtcgtgccgctggaccacgccgagcacgagctgcacggcgccgtcgacccgggccgggacctcggcagcggcctcgacctgcagcgctgcctgatgcagttgcccgaagagcagcgggccgtgctgctgctggtgacgctcgaagacctttcctatgccgaggtggccaaggtgctcggcgttcccgcgggcaccgtgatgtcgcgcctctcgcgcgcccgcgcccggctgcacgaattgatggatggcgccgccgcgccgaaccgcaccggcctgcgccgcctcaagtgaaacctttcgccgaaccatgaaccgccccgccccgccccccaccgacgacgagctgcatgccctcgtcgatggccagctggcaccggaccgacggtccgaagtcgaagacgccgtggcacacgacccagccgtcgccgaacgggtcgcagcgtggcggagccagcgggacgccttgcgccggctgcatggcgacctgctcggcgaacccgctcccgcccacttgatgggcgcactcgatcgcaaccagccccggcacgctcggcaagaccgatggatgcggtggggcggcatggcggccggcgtgctggtcgcctttgccgccggctggctcggcaatggccaatggtcggcgcagcgcgccgcgccggcccaattggccaaggcgcccgcgatgcgcgagttcgtgcacgacgcgtcggtggcgcacgccgtctacgcgcccgagaaaagacacccggtcgaagtggctgccacggagcagcagcacctcgtgcagtggctgtcgaagcggctcgacaagccgctcaaggtgcccgacctggcatcgatgggctacacgctcgtcggcggccgccttttgcccggggaaagcggtgcacgggcccagttcatgttcgaggacgctgccggcgagcgcgtgacgctctacatcggcacgctcgacagccgagccgccgccggtacggccgcatcgcgcgaaacagcgttccgctttgcatccgaaggcccggtgcccagcttctattgggtggaccagggcttcggctatgccgttgcaggcaagctaccgcgcgatgttttgctgaaactcgcgacgcttgcctaccgcgatttgtcttgagcccggcataaactgccgggtcgcgcaaacacatggcttgttatcgcgttttatcaactgaaggagaaactgcatgaaattgctcagcgcctcgatcctcgcggcggcattgctcgccggctgcggcggcatgtccaacaagagcgccagcgcgcccgacacgcccacccgcaccgccgatggtgtgctcgtgggaccgaacggcatgacgctgtacaccttcaccaaggacacggccggcaccggcacctctgcctgcaacgcccagtgcgccgccaactggccgccgctccccgtggccgaaaccgccaagccgatcggcggctacaccatcatcattcgcgaagacggcaagcgccaatgggcctacaagggctggccgctctacttctgggccaaggacgccaagccgggcgacaagaccggtgacggcgtggccggcgcctggaagatcgcccgcccctgatcgcgtggtttcctgaatgcaaaggccccggcagacgtcggggcctttttcttttccgctcgcttaatgtgcgctgggaagcgcgccgtcggccaccgtggcgcggcgcccgcgcagtgccagcagttcattgaacaccagtgcgccgatgaccagtgcaccgccggtcagcacgctcacggcgggttcttcacctgcaccgatccatgccagcgcaatgccgaagatcacttcgagcaaagccagcagagcgacctcgggcgccttcagcacccgcgcgcacagcaccgacagcacgcagggaatggccagttggaacacccccaggaaagccagcaggccgaggtcgcgtgcgtttgcctgaaacggcaatgcaaagggcagcgtgaacagtgcgctgagcaccgcgccgatcagcaccgccggcaccagatcgatgtcatgccccttggcatgcgcatgctgaacgacagtccagttggtggcgccggccagcggcacgcacagcgccaccagcgttccaagcagcgagccacctgccccgccctgcatcagctgcgtgccatacatccaggcaatgccgagcccggccaccacgatggcgagccaggtccgcgcgggaagccggtggccgatgaagatccgcgcggccaacgcggtgagcagcggcccgagcgccatcgtgaccagcacgctggcggtggaagccagcgtgagcgccaccatgaaggccgtgaacatcacggtccagcagacgcccgagatccacagcgcccggccgccatgccgtatctgcgagaacacggcccggccccgccaaagcggcaagatcaccagcaacgccagcatcgtgaagaggctgcgccagaaggtgatctcgaagctgtgcgcctgtgcgaggtgccgcgtgacgacgcccgccgtggcccacatcagggtcacggcgaccatcagccacacagccccgccgtgcgtcaggcgcagcatcggtcgatgatggcgatcagctcgccatttcgcggccggcccgcttgcgctcgtgctctttcaggtagcgcttgcgcagacgaacgctcttgggcgtgatttcgaccagctcgtcgtcctcgatgaattccacgccgtattcgagcgtgagttcgatcggcggcgtgatcttgatcgcgtcttccttgcccgagacacggaagttggtcagctgcttggtgcgcgtggcgttcaccaccaggtcgttgtcgcggctgtggatgccgacgatcatgccttcatacaccggatcgttggccttcacgaacatgcggccgcggtcgtccagcttgcccagggcgtaggtgaagatttcaccgtcgtccatggaaatcagcacgccgttcttgcggctgccgatgtcgcccttgtgcggttcgtagctgtcgaagatgttgctgatgaggcccgagccgcgcgtcaggttcaggaattcgttggtgaagccgatcaggccacgcgccggaatgcggtactccaggcgcacgcggccgcggccgtccggttccatgttgaccagctcgcccttgcgctcgcccagtgcctgcatcacgccgccctggtgctgctcttcgatgtcggccgtaaccagctcgatgggttcgtgcttctcgccgttcacggtgcggaacaccacgcgcggcttcgacacggccatttcatagccttcgcggcgcatgttttccaagaggatggtcaggtgcagttcgccgcggcccatcacctcgaagatgccttcttcgtcggtttcgttgacgcgcagcgccacgttgtgctgcagttccttctgcaagcggtcccagatctggcggctggtgacaaacttgccttcgcggccggccagcgggctggtgttgacgcagaagttcatggtcagggtcggttcgtcgaccttgagcatgggcagcggcgccgggttggtggggtcggtcacggtcacgccaatgccgatgtcggcaatgccgttgatcagcacgatctcgcccgggccggcttcagttgcctgcacgcgctcgaggccctggaaagtcaggacctggttgacgcggcccttgacggccttgccgtccggaccttccatcaccaccacgtccatcatgggcttgagcgtgccctggctgatgcgacccacgccgatgcggccgacgaaggtcgagaaatcgagtgccgaaatctgcagctgcagcggtgcttcggggtcacccgtttgcgccggcacgtgcttcaggatggtgttgaacagggccgacatgtcgggaccccactgttcgccggcagcgccttcttcgagcgacgaccagccgttgatgcccgaggcatacacgaccgggaagtcgagctgttcgtccgtggcgccgagcttgtcgaacaggtcgaaggcggcgttcaccaccttgtcggggttcgcaccgggcttgtcgaccttgttcacgaccaggatcggcttgaggcccagggccagcgccttcttggtcacgaagcgcgtctgcggcatcgggccttcctgagcgtcgatcaagagcaccacgccgtcgaccatcgacagcgcgcgttccacttcaccgccgaagtccgcgtggcccggggtgtcgacgatgttgatgtgcgtgccttcccaggtcacggcgcagttcttggccaggatcgtgatgccacgttccttttcgatggcgttgttgtccatcaccgtgtcgacgactttctcgtgctcggcgaaggtgcccgactggcgcagcaattggtcgaccatcgtggtcttgccatggtccacgtgggcaatgatggcgatattgcggatttgcttggtactcatggtgtcgcttcggtctgttgtgcgttcaaaagaatttgctggatttcgatggggttcagcaagcgccccgggatcagttcgttggcggcgacatgcgccgtgccgaggaaggcggtaggcgcttcaccgaacaccgccacgtggtcggcatcgggccagttgccgcggcggcgcaggccggacagaaagcgccctgcatcttcgctgcccagcgtgacgatcgtatggccctcgaccagggattcggcaggcaacaaccgggccagccgctcgtcctcgcccatggcttcgagcgcttcgagcgtgatgcactgcgccacaccgaaaccgccggtggccgtacggcgcagcgacgtgaggtgggccccgcagcccagtgcctcgccgatgtcttcgcccagcgtgcggatgtaggttcccttgctcacggaagccactatttttatcgcattgcccgccgattcggccgctgcctgcgtgatcttcaatgcatgaatgaccacgtcgcgcggcgcgcgctcgatctcgatgccttcgcgggcgtactcgtacagcgccttgccgtctttcttgagcgcgctgtgcatcggcggcacctgtcggatcgggccggtgaattgcgcctcgacgcgggccaggtcttcaggcgtgacgtgcaccggacgctcggcgatcacctcgccctcggcgtcgccggtggtggtcttgatgcccaggcgggccgtggcctcgtaggtcttgtcggcgtcgagatgcagctggctgaacttggtggccgcgccaaaacacagcggcagcacgccggtggccaacggatcgagcgtgccggtgtggcccgctttttcggcgcgcagcaaccacttggccttctgcaaggcctggttgctggaaagtcccagcggcttgtcgagcaacaacaccccatgcacagggcgccgctgcaccctggtgcgtggcgcgttcatggctagtcgtctttcgaacgcgaagcgacggcctgcgcgatgagcgcattcatgtcggccgcacgctcggtggtgcggtcgaacaggaagtgcagcgtcggcacggtgtggatgtgcaggcgcttgaacaggccgttgcgcaggaagcctgcggcctggttcagcgcttcggtggtctcgtccacgtcgcctgtgagcatgctgaagtacaccttcgcatgcgcatagtcgggcgtgacctcgaccgcctggatcgtgaccatgcccacgcgcgggtccttcaactcgcgcgcgatcagctccgtcagatcccgctggatctggtcggcaaccttgaacgcacggttgggggcggcggcttttcttttcggcatggtctctctcgcatcgaacgcttacagcgtccgggcgatttccttgatctcgaagaattccaactgatcaccttctttgatgtcgttgtagttcttgagcttgataccgcactcgaagccttcgcgcacttcgcgaacgtcgtccttcatgcgcttgatcgagtcgacttcgccggtgtagatcaccacgttgtcgcgcagcaggcggaaatgcgccgtgcggttgaccgagcccgaggtgatgtacgaacccgcgaccgtaccgatcttggaagccacgaacaccgtgcggatttcggccgagccgatgatttcctcgcggcgctccggtgccagcatgcccgacatcgcgaccttgatctcgtccacggcgtcgtagatgatgctgtagtagttcagctgcacgccattgccttcggccagcttgcgcgcaccggaatcggcgcgcacgttgaagccgatcacgatcgccttcgaggcgatggccaggttgatgtcgctttcgctgatgccgcccacgccggcgtacaccatttgaaccttgacctcttcggtcgccagcttgagcagcgactgggccagcgcttcctgcgagccctgcacgtcggccttgatgatgatgcgcagcgtctgcacttcgccggccgagaggtcggtgaacatgttctgcagattcgcggcttgcagcttcgccagcttggtattgcggaacttgccggcacggtaggtggcgatttcgcgcgcacggcgctcgtcggccatcaccatgaactcgtcgcccgcttgcggcacttcggtcaggccctggatctcgaccggaatcgagggaccggccgacttgatggacttgccgtcttcgtcgagcatggcgcgcacgcggccataggtcgaacccgccagcaccacgtcgccggtcttgagcgtgccggactgcaccagcacggtggcgaccgggccgcggcccttgtcgagctgcgcttcgatgaccaggcccttggcggcagcatccaccggcgccttgagttccagcacttcggcctgcagcagcacctgctcgagcagctcgtcgatgccctggcccgtcttggcggacaccggcacgaacggcacgtcgccgccgtactcttcgggcacgacctcttcggtcaccagttcctgcttcacgcggtccgggctggcatcgggcttgtcgatcttgttgatcgcgaccacgatcggcacaccggcagccttcgcgtgcttgatggcttccttggtctggggcatgacgccgtcgtcggccgccaccacgaggatgacgatgtcggtggcctgcgcaccgcgggcacgcatggccgtgaaggcctcgtgacccggggtgtcgaggaacgacaccatgccgcgttcggtctgcacatggtaggcaccgatgtgctgcgtgatgccgccggcttcgcccgcggccaccttggcacggcggatgtagtccagcagcgaggtcttgccgtggtcgacgtggcccatgacggtcacgaccggtgcgcgcggcagggcttcggcggtttgcgccgacacgtcctcgtcggtgaaggcttcggggtcgtccagcgcggcaacgaccgcgttgtggcccatttcctccaccaggatcatggcggtgtcctggtccagcgactggttgatggtcgccatctggcccagcttcatgagctgcttgatgacttcctgcgccttgacggccatcttgtgggcgagttcggccacggtgatggtttcgggcacgtgcacttcgagaatgcgcgcctcgaccggtgcggcctgcacatgctcttcatggcctccacggtcgttgctgccacggcggccgcgcgggcctccgcgccagttgccgcggccaacaccaccgctggcatcgccgcgggtcttgatttctttcttcttggccggatcgccagcccagctcgacgagagcttggccgacttgacttccttgccggcaccggcggcgccaggggctgcggcagcacccggtgcggctggcgcgccggggcgtgcggccggagcggctggcttgtgcagcgttcccttgaccgcggccttttcgggctgcggcttctcgggcgccttgtgcggcaccagcacgcgggccggtgcgttcatcatggcgcgaatggcttcggcttcggcgagggccttgcggcggcgctcgtcgaggtccttggcgcgggcggcttcttcgtcggcacgagccttcgattcggcggcggccttggccttcgcgtcttccttggcttgcgtggcggcggtttgcgcagccagcttggtgtcagcggcttgctgttcggcggcggctgcagcggctgcggcaggcgcggcaaccggcttggcggcttccttcgggggcgcggcagcggcttcggcagcggccttcttctcggcggcgatgcgtgcggcttcctgctctgcctgttcggcgcgctcggccttttcggcctgctcgcgttcgcgcgcttcggcttcctcgcgcaggcggcgcttttcgaccagttcttcttcctggcggcggatcagctcggcctggcggcgcgcttcttcctcgcggcgggccagttcggcttcgtcgacgcggggtgcggcgggtgccgcggcgggcgcttcggccaccggttgtgcttcgggcacggccgggtggccgtcgtcgcgctggatgaaggtgcgcttcttgcgcacctcgacctggatggtgcgggcgcggccggtggcgtcggcctgcttgatctcgctggtcgacttcttcgtcagcgtgatcttcttgcgctcgggctcggcggtgccgtggctggctttgagaaagccgagcaggcgctgcttgtcagcctcggtgagtgcatcggtgggtgccgctttgggcacgcctgcgctcttgagctggtcaagcaaggtttcgggagtcttcttgagctcgttcgcgaactcggcgacagtggtactggacatattggtttcgtgcctccatgaccatcactcttggccggcgaaccaatgttcgcgggctttcaagatgagggctttggcgtcatcggcgctgtggccggtgatctcggtgagttcatcgaccgcgaggtcggcgaggtcgtcgcgggtgtgcacacccgcctcggccagcttgggaatcagctcggggtcgaggccttcgaggtcgcgcagattctgcgagacggtctcgacgccctcttccttggcgatttccatggtcagcagcgcatccttggcgcgcgtgcgcagctcattgatggtgtcttcatcgaaagcttcgatctccagcatttcggagatcggcacataggccacttcttcgaggctgttgaagccctcggagatcaggatgtcggcgatttcctcgtcgacgtcgagcttttccatgaacagcttgcggctggcgtcggtttcgctcgcctgcttctgggccgattcattggcgtccatgatgttgatcttccagccggtcaggtcggaggcgagcctcacgttctggccgccgcggccgatggcgatggcgaggttttcctcgtcgaccaccacgtccatggcgtgcttttcttcatcgacaacgatggaagacacattggccggggccagggcgccgatcacgaactgggccgggtcttcgctccacagcacgatgtccacgcgctcgccggcgagctcgttggtcacggcgttgacacgggtgccgcgcacgccgacgcaggtgccgatcgggtcgacacgcttgtcgtgcgagagcacggcgatcttggcgcgcgaaccggggtcgcgggcgcagctcttgatttcgagcaggccttgttcgatctcgggcacttcctggcggaacagctcgatcatgaactcgggggccgagcgcgacaggatgatcggcgcgccgcgcagcgtcaggtcgacctccatgatcatggcccgcacgcggtcgccgttgcgcaggttttccttggcgatcatctcgctgcggcgcaggcgcccttcgacgcggccggcctccacgatgatgtcgcccttgtccaggcgcttgacggtgcccacgaagatcttgtcgccgcgcgacatgaagtcgttcagcagcatctcgcgctcagcgtcgcggatcttctgcaggatcacctgcttggcggccatggcgccgatgcggccgatcggcaccgagtccaccgattcctcgatgtattcgtcgacctcgatgtcgggcatttcttccttggcttcgaacaggaggatttcctggtcgggcagctgcaggccggcctcgtcgggaacgacgtgccagcggcggaaggtttcgtagtcgccgctgtcgcggtccacggccacgcggatgtccacttcgcccgcatagagcttcttggtggcttgcgccagtgcggattcgaccgcgccgaagaccacgtcgcgctcgacgttcttctctcgcgagatcgcatccaccaacatcaacatttcgcgattcatgccaccactcctctagtcagtccggaacattcgttccgtcgtcaatatccgaaaaacccggttgggttttggccctgcggcccttgaaatccacaattggcgcgagccgcgcatcgcgcagctcgtccagcacgaagccgagcgcatgcaactttgcaggcgcgcgcttcttgctcactttttgtcccggtttgggctcgggcgcatcgctccagacgatttgccagcccggggctgcgtcagccccttccgctgtttcagcacgctccagcgtgccgcgaaatttcttgcggttggcagacacctgccccgccgccgcggcacccatcggcaccttgagcgtgatgtcgatcacctcgccgacaaaacgctcgaaatcctgctcattgcgaagcggacggtcaatacccggcgaggaaacctcgagccgcttgtaatcgacaccatcgacctcgagcgcaaactgcagctgccgcgtgaccttttcgcaatcctcgacggtcacgaagggctcgggaattcccgcagccacagcttccgaggtgggggccgtccagggcaaatcaatcgtgacgcgcagcaatcccccggccgatctatcgatctcgaccaggtcgtagccgagtccggccacggtttgttccactgtctgctgcaatgccacgtgtttgaaaatgccttgtaaaaatgcctgtgcgaaatgcttatgcgcgccgcccgcttatgcgcgccgcccgcttatgcgcgccacccgcccgccacgggtgccacgcatcgagaatgcatagaccaaaaaaaacgggcggttggtacccgcccgtttggtcgtgagcctcgaattatatgctattcgtgtgagaaatgaaggggcttcggcgctcaggcgggcctaatacggcgagatttcgaccacaccaccgcaaacagcgcggccccgagcgccagggccgcagccgctaccagcagcggcacctggaacgaaccggttcgctgggccagcggcgcggcaaaaagcggtccgatgatctgcccgacgccgtaggaagcggttgcgtagccgatcagcccggcggcggcattgccccgcagccggcgcgcatcccgcatcgcaaaaagagtgatggccgtgaacggcatgccgagcagcaggctgccaagcgcaaagccggcaatcgtgggccacgccaccgacagcagtacgcccagcgcctgcagcgcatacgccgccgccagcagcagccggttgtcccaatgcaggggcgcacgggcgccgatcagcgcgcccggaatgatcgccaggccgaaaagcggccagaagaaatcgggccagggcgagcccggcagcgcctggcgggcgatcacgggcagaaaggtcgccgtgatgatgtaaccgaagccggccaggccgtagagcgcgaccagccagaccgcgtcgctgcgcgccgaggccgccgaagccggtgtaccggccgcggctgcgggtgtggcggcagagccggccgccgccggcagctcgccgtcatcgaacacccgccagatcgccgccaccagcaccaccgccagcaggccgaggccgatccacccggtttccgagccccaccgccccagggcgccgccgagcaggccggtcatggcaatgccgatgccgggccccgtgtagatgacgccggccagcgccggagaattggtttcggccaaccggcgcaggccccatcccgacgcgaatacgaagacccaggcactcatcacgccggctgccgcgcgcaggatgccccagcttgtgaagctgtggagcacgcccatgccgaccagcagcacggctgttgccgccagcccgccgcgcaccatggtcttggccttgatgccgatggccgcgcaactgacggcgcccagaaagtagcccaggtagttgagcgacgccagcacgcctccggcctcgagctggagttttccttcatgcagcatgatcggcagcatgggtgtgaaggcgaaacgccccagccccatggccacggccaaagtgaccatgcaggccagtgccgcgcgccaggccccgcgccggccttgtccgattcccgacattgctttgaattccgttgttctattccagcagcgctgcggccaccagttttcttgtgtaggggtgctcgggtgcatcgagcacgcgctcgacgaggccggcttcgagaatggcgccatccttcatcacgatgacctggtgcgccatggcgcgaatcacttcgacgtcgtgggtgatgagcaggtagctcaggccgcgctcgcgctgcaggcgctgcagcagccccagcacctgcttctggatcgtcacgtcgagtgcgctggtgggctcgtcgagcaccagcagttgcggatcgacgataagcgcgcgcgcaatcgcaaggcgctggcgctggccgcccgaaaactcgtgtgggtagcggtcgagcagcgacggaaactgcgcctcgctcaatcccacgtcggccagcgcggccagggcccgtgcccggcgctgctcggtgccgagctcgggtgcatgcacgcgcaggccctcgccgacgatctgctcgaccgtcatgcgcggcgagagcgaagaaaacgggtcctggaaaaccacctgcatgacccggcgcaaggccaggtcggaaccccggtcgaccgcccagcccttgccgtccaccttgagcgcaccgcgatatttcagcagcccgagagcggccagcgccagcgtcgacttgcccgacccggattccccgaccacgcccagcgtttcaccaggtgcgatgcggaagtcagcgttctgcacggcgatgaattcgcctttgcggaaccagccggcaacgccgggccgggacaccgggtagctcacgcgcaggcccgtggcctcgagcaccggccgtgcatcgctgcccgcggctacggcactgacgttgcgctctggatggctgtcgatcaacttgcgggtgtaggcatgcttcggcgcttcgaaaaccgtggccacctcgccctgctcgacgatgtggccatcttccatcaccgccacccggtcagcgaaccggcgcaccaggttcaggtcgtgggtgatcagcagcacggccatgccattcttgcgctgcaggtcggcgagcagatcgaggatctgcgcgcgcacggtcacgtccagcgcggtggtgggctcgtcggccagcagcaggcgcggcttgcaggcgagcgccatcgcgatcatggcgcgctggcgctgcccacccgagagctggtgcgggaacgccctcgcccgccgctccggctcgggaatgccggtgtcggcgagcagccggacggcggcggcctgcgcgtcgcgtgccgagagcccttcgtgcagttcgagcacctcggcaatctggtcgccgacggtgtagagcgcattgagcgcggtcatcggctcctggaagatcatcgcgatctccttgccgcgaatgccgcgcagttcgcgctccggaatcgacagcaggtcgcgcgcattggaagaggcctgggggtcgaacagcttcgcaacacccgcgaggtcggcgttctgcgccaggcgcagcagcgccagcgccgtgacggtcttgcccgaacccgactcgcccaccagggcgagcttctcgccggcggcaatgcgaaagtcgatgccatgcaccacttccttgccgccgaacgcgacgcgcaggcccttgacgtcgagcagcggcagatggggggtcgtcatttcgctcacgtgtcggccttccgtggatcgagcgcatcgcgcagcgcatcgcccatgaaggtcaggagcatcagcgtcacgaccagcacaccaaaggtcgacaacgagatccaccaggcatcgatgttggccttgccctggctcagcagttcgccgagcgacggcgtgcccggcggcacgccaaggcccaggaagtcgagcgaagtgagcgccaggatggccgcgctcattcggaaaggcaggaaggtgacgaccggcaccatgctgttgggcaggatgtggcgccacatgatctgcaggttgccgacgccgagggctcgtgcggcgcgcacgtagtccatctgtcggttgcgcaggaattcggcgcgcacgtagtccgacaggcccatccatccgaagaggctcagcaatatgagcagcagcgccacgctgggcgagaagatcgcactgaagatgatcagcaggtagagctcgggcatggaaccccatatctcgatgaagcgctgaaatgccaggtcggtcttgccgccgaagaagccctgcacagcccccgtcacgatgcccagcaccacgccgatgaccgtgagcgccagtgcgaacagcacgctcacgcgaaagccgtagatcagttgcgccagcagatcgcggccgcggtcgtcggtgccaaaaaagttgtcacgcgacggggccgacggattcggcaacttggcaaaataattgagcgtctgtgggccataggtgttcggcgcatagatggcccagttcttccccgcggtgatccgctcgcggatgaacgggtcgaggtagtcggccggcgtctcgaagtcgccgccgaatgtcttttcgggatagtcgcgcagcacgggaaagtaggtttgtccttcgtagtgcacgacgagcggcttgtccgtggacagcacttccgcaaagaggctcaggaccacaagcaccgtgaagacgacgaggctccagaacccgagcggattccggcgaaaacggcgccaggcgcggcgcgccgggctcagcgaaacgggcagcgcgtcagtcaaatttcaccctcgggtcgacccagacgtagcaaaggtcggaaatgagcttggtcaagaggccgatcagcgtgaacaggtacagcgtgcccagcaccacgggatagtcgcgccggatcacgctttcgtaactcaacaggcccagcccgtcgagggagaacagtgtctcgatcagcagcgagcccgtgaagaaggcgccgatgaaggccgccggaaatcccgtgatgatcgggatcagggcgttgcggaagacgtgcttccagagcacttgccgctcggccagccccttggcgcgcgcggtcagcacgtattgcttgcggatttcctcaaggaatgaattcttcgtgagcatggccgtcacggcgaagctgccgagcaccattgcggtcacgggcagcgcgatgtgccagagatagtcgacgatcttcgcgccccagccgagcgtttcccagttgggcgaggtcagcccgcgcagcggaaaccactgcaactggccgccgaagatcacgagcagcgccacccccagcacaaagccaggtatcgcatagccgaccagcacgatgagcgtggtcacgaagtcgaaacgcgaacccgcgcgcaccgccttcgctacgccgagcggcaccgcgatcaggtagctgatgaagaaggtccagagccccaggctgatcgacaccggcagtttttccttgaccaggtcccacaccgccttgcgctggtagaagctctggcccaggtcgagttttgcgaaggacttgagcatctgccagaagcgctcgtgggccggcttgtcgaagccgtagagcgccttgatttcctcgatgcgttgtggatccagaccctggcggccacggtagccggcgccggtgctcgcagcgcgctccccaccagaatcgcggccctgcaactgggacaccatctgctcgacgggcccgcccggcacgaactggatgaccacgaaggtcagcagcagcacgccgagcagcgtgggcaccatcaggagcaggcgtttgaggatgtagctggccatggcgtgcgcgactctctatttgttcgtgggcgacgcccaccaggtggtcatcgcccaagcgtcggcctggtaatacgggggaacgacatcgggcagcacgacaggccgcggccggtagccgaccaggaaggcgctcccgtagtactgcgggatcgagtagtagccgtgcgacagcacgcgatcgagcgcgcgcaccgccgtgcgcagttcggacctggttgtggcactgagcaccttctgcaccagcgcgtcgacggccggatcggcaatgccccagatgttggaggagccatgggtctcggccgccttggacccgaagaagtcgagcaactcgcctccgggcgcggtactgcccgacaagcgcaggctggtcatctcgaagtcgaaattgtccatgcgctgctgcgacagcgagaaatcgacggtgcgaaagcgcatctcgatgccaagcttctgcagcgcactctggaacggcgtggcaacccggatgagcgagggctggtcgttcaggaactcgatggtgaacggctcgttcctggcgttgcgcagcgcgccatcgcggtaggtccagcccgcctcggccagcaacgcccttgcgcggcgcagattctcgcgcaggcttcctggcggcgcggtgctgggggagatcacggccggcccgaaaacctcggggcgcagcttgtcgcgcagcggttcgagcagcgccagctcgtcgggttttggcaagccttcggcgtggaactcgctgttggggaaataaccctgcacgcgcgtgtagagcccgtagaacagctggcggttgagccattcgaaatccattgccagcccgatcgcctggcgcacccgcacgtccttgaacttgtccttgcgaaggttgaatacgtagccctggaaatcgccggggttccgggtttcgaaagcgcgcttgacgagctccccgctctcgaattgcttgcccttgtattggcgcgcccagttgcgcgaagtgaattcgcgcatgaagtcgaattccccggccttgagcccctcgaagcgggaggtgtcgtccaggtagttcttgaaggcgacccggtcgaaattgaactgcccccggcgcaccggcagctcggcgccccaatagcgcgggtctcgcacataggtgatgtcgcggcccagccgcgcgctcgagggcttgtaggggccggaggcaatcggcacctcgctgatgatctggtcgaaaggcttgccgccgccccaggcgcgactgaacaccgccatgccgccgaccaccaaaggcagctccggattgggccttgcgaactcgaagcgcactgtgcgttcgtcgagtgcgcgcacgcccttcacctcggcatagagcgttcggaactggggcgctgccagcttgctgttgagcgtttcgaaggaatacaccacgtcggccgccagcaccggcgagccgtcgttgaaacgcgccttggggttgagccggaatgtggcggaaagcttgtcggctggcacctcgacgtcttccgccagcaggccataggctgtggtcggctcctccgaattgcctgcgagcaggctttcgaacaccagcacgccctgcccatagggcgccgtgcccttcagggtgaacgggttgaacttgtcgaagttggtgggccgggtcggcggcaccatccggatctctccgcccttgggcgcattcgggttcacgtagctgaaatgggtgaagccgggcggatacttgacatcgccgaattgcgcataggcatgggcggcccatgaaggagccgcccagagcatcaggagaaaaagcagccaagcccgcatgcgagaattctgcccaagattttcacgaggcaacttcatgggctttctttccggcaaaaaactgttgatcaccggcgtgttgagcaatcgctccattgcctatggcattgccaaggcgtgtcacgaacaaggcgccgagcttgctttcagctacgtcggcgagcgattcaaggaccgtatcaccgaattcgccgcagacttcggctccaagctcattttcgactgcgacgtgggcgacgatgcgcagatcgacaagctctttgccgatctggcgcagacctggcccaagttcgacggcttcgtgcacagcatcgggttcgcgccgcgcgaggccattgcgggcgactttctcgaagggctgtcgcgcgagggtttcaagattgcgcacgacatcagtgcctacagcttcccggccatggccaaggccgccctgccctacctcaacgacaaggccgcgctgctgacgctgacctacctcggcgccgaacgcgcactgcccaactacaacaccatgggcctggccaaggcctcgctggaagcttcggtgcgctacaccgcggcatcgctcggccccaagggcatgcgcgtcaacggcatcagcgccggccccatcaagacgctggcggccagcggcatcaaaggcttcggcaagatgctgtccgccgtggccgaggcctcgccgatccgccgcaacgtgaccatcgaggaagtcggcaacgtggccgcctttctgctgagcgacctggcaagcggcgtgagcgccgagatcacctacgtggatggcggcttcagcaacgtcgtcgcgggaatgggcgaataaaggctcgccccggcaccttccgcagaacattgcgtcttcatcgattggcagcggcgtcgtgctgacccgacgttccctcctgcttgccgggctcagtgcgctggcggcccgcacggccgtcgcacgcgagcccgcaccggcactgatgctggccgaggtctaccgcccaggcatgtcgctggcggactactgggtcagcgaaaaatacgacggggtgcgcggctactgggacggccagcagctctggacgcgtggcggcgagccggtggtggcgcccgcctggttcacggcaaagttgccgaggcagccgctcgatggcgagctgtgggccggccggggccagtttgcgcacgccgtttccaccgtgcgcagccagacacccaacgacaccgcctggcacagcatgcggttcatggtgttcgacctgccgtcccagggcggcgatttcacggcgcggctcgctgccctgcgcaaactgctgccggtcaccgacgcgccgtggatcgtgcccgtgccccaggaacgcgccaccacgcatcccgagttgcaggcgctgctcgacaagaccgtgaagatgggcggcgaaggcctgatgctgcatcggggcggctcgctctatcgcgccgagcgcaacagcgacctgctcaaggtcaagctccacgacgacgccgaggcccgggtggtcgggcacgttccgggcaagggccggcacggtggccggctgggtgcgctgctggtcgaaacgcccgagggcaagcgcttcaagctcggcaccggcctcaccgacgccgagcgcgagaacccgcccgccatcggcagctgggtgacctaccgcttcaacggtaccaaccccggcggcctgccgaggtttgcccgcttcatgcgggaacgcatcgacctgccctcctgaagcgcggcgcgcccacggcgcgcaccactctcgcttccctgattattttttcttcggcgcggccacgcagtccgcgtagtagcgcttcttgccggtttcgtcgacgcgcgccaccaggccgtggatgtcggtctcgaagcccgggcactgcaggttgaactcgcgcgagaacttgaggtagtcgacgatcttcttgttgaacacctcgcccggaatcagcagcggaatgcccggcgggtacggcgtgatcaggctggtggtgatgcggccttcgagctcgtcgatttccacgcgctcggtcttgcggtgcgcgatgtgggcgaaggcgtcgctcggcttcatggccggcgtgagatcgctcaggtacatctcggtggtgaggcgcgccacgtcgtagcgtgcgtagagctggtggatgtgctggcacagatcgcgcaggcccaggcgttcgtagccggggtgctgctggcagaactcgggcaggatgcgccacatcggctggttgcgcgcgtagtcgtccttgaactgctgcagcgccgtgagcagcgtgttccagcggcccttggtgatgccgatggtgaacatgatgaagaagctgtagagcccggtcttctccacgatcacgccgtgctccgcgaggaacttggtcaccacgctggcgggaatgccggtctcggcgaaattgccttccagatccaggccgggcgtcacgatggtcgacttgatcgggtcgagcatgttgaagccgtcggccagatcgccaaagccgtgccagttgcgcggcgacttcttgtttttcggcttgccgttcttctcgcccgtcatgatccagtcttcggcgcggccgatgccttcgtcgacgagcttctcgggaccccagaccttgaaccaccactcgtccttgccgaactcggcctcgaccttgcgcatggcgcggcggaagtcgagcgcttcgagaatgctctcctccaccagtgcggtgccgccgggcggctccatcatggcggcggccacgtcgcagctcgcgatgatcgcgtactgcgggctggtggacgagtgcatcaggtaggcctcgttgaacaggtcgcggtcgagcgcgcggttctgcgagtcctgcaccagcacgtggctggcctggctgatgccggccagcagcttgtgggtcgactgcgtggcaaacaccagcgactccttcggccgcacgcggcgcttgcccatggcgtggtaggcgccgtagaacggatggaaggccgcatgcggcagccatgcttcgtcgaaatgcagcgtgtcgacgtagccgtcgagcatgcccttgatggtctcggtgttgtagatcacgccgtcgtaggtcgactgcgtgagcgtcatcacgcgcggcttgaccttgtcggggtccacgtcggccagcagcgggttggccttgatcttggccttgatggcgctctgctcgaactcgctcttgggaatcgggccgatgatgccgaagtggttgcgcgtgggcttcatgaagaccgggatcgcgccggtcatgatgatcgcgtgcaggatcgacttgtggcagttgcggtcgaccaccaccacgtcatcgggcgccaccgtgtggtgccacaccatcttgttgctggtgctggtgccgtttgtcacgaagaagcaatggtcggcgttgaagatgcgcgccgcgttgcgctcgctggccgccaccgggccggtgtggtcgagcagctggccgagttcttccaccgcgttgcagacgtcggcgcgcagcatgttctcgccgaagaactggtggaacatctggcccaccgggctcttcaggaacgccacgccgcccgaatggcccgggcagtgccatgaatacgagccgtcttcggcgtagtcgatcagcgccttgaagaacggcggctgcacaccctccaggtagctcttggcctcgcggatgatgtggcgcgccacgaactcgggcgtgtcctcgaacatgtgaatgaagccatgcagctcgcgcaggatgtcgttcgggatgtggcgcgaggtcttggtttcgccgtagatgtagatcggcacgtcggcgttcttgcggcgcacctcgccgatgaagctgcgcaggctcagcacggcgggatcgaggtcggggccgaccgtgaactcctcgtcgtcgatcgacaggatgaacgcgctggcacggctttgctgctgcgcgaactggctcagatccccgtagctcgtgacgcccagcacctcgaagccctcgctttcgaaggcctgcgcaagcgcgcgaatgccaaggcccgaggtgttttcggagcggaagtcctcgtcgatgatgacgatggggaagcgaaatttcatgagcagggctccggacaggcaatgaggcgcgaagtgtacggaattcggatgaaggtttccgtcaccttttgactcagaatgtcgggcgtccatcaaagaggagaagacatggcgaattccaccatctggtggctgatagcgggagccgcgatcgtgctcgagttgctctcgggtacggtctacctgttgctgctggccacgggcttcgcagcggcggccatcgcggcgcatgtgggcgcgggaacggtcgcgcaactcgtcgtggcggccgtggtcggcgtgggtgcggtcctggcctggtatgcggtgcagcgccgacgcccgggcccgccgcctaccggctcgaatcgcgacgtcaacctggacatcggcgagatcatccatatcgaggcatggaaccccgacggcacggccaccgtgcgctatcggggagcccagtggaccgtggttccgcgcagcggtcacgccccggccgccggcgagcaccgcgtggtcgaggtcatcggcagccgcctcgtggtcgagaaaacctagtcagaacattcaagaggagaaacatcatggaattttcagttcccatcatcatcctggtcatcgcggtgatcgtcatcagccagtcggtcaagttcgtgccgcagcagaacgcctgggtgcgcgagcgcctgggcaagtaccacagcaccatgacgcccgggcccaacttcctgatcccgttcatcgacaaggtcgcctacaagcacagcctgaaggaaattccgctcgacgtgccgagccagatctgcatcacgcgggacaacacccagctgcaggtcgacggcatcctgtactttcaggtgaccgacccgatgcgcgcgagctacggctcgtcgaactacatcgtggccgtgacgcagctggcgcaaacgtcgctgcgcagcgtgatcggcaagctcgaactcgacaagactttcgaggagcgcgacgtcatcaacgcccaggtggttgcggccatcgacgaggcagcgctcaactggggcgtgaaggtgctgcgctacgaaatcaaggacctgacgccgcccaaggaaatcctgctggccatgcaggcgcagatcaccgccgagcgcggcaagcgcgcgctcatcgcggcctctgaaggccgtcgccaggaacagatcaacatcgccaccggcgaacgcgaagccttcattgcccgctccgagggcgagaagcaggcccagatcaacaacgcccagggcgaggcggccgccatcaccgccgtggccaccgccacggccgacgccatcgagcgcgtggcggcagccatccgccagcccggcggcgaacaggccgtgcagctcaaggtggccgagcgcgcggtcgatgcctacggcaaggttgcggccgattccaagaccacgctgatcgtgccgagcaacatgaccgaaaccgccgcgctcatcgcgtcggccatgcgcatggtccaggccggcaagccatcgaatccggcctgagcgactgctacaatcgaaggctcaggagcggtggatgagcggtttaagtcgcacgcctggaaagcgtgtgagggttaatagccctccgcgggttcgaatcccgcctgctccgccagagattgattgttcgtaaccgttcacggacatgagagccagaataaaaagcccaggttgccttccagcaccctgggcttttttgtcggcgcgttgcgccctggcaacgcgcatccgactgccccgccgccctcaactggcggtacgatccaaagtcttactttcacgcctgcaaaggagcccggatggccggacaaccacaacccaccccgactggcgatacgtcgctcgaacagacattggagaagaccgaagcggttgccgccgatgtgcagcgggcgtcggacaaccttgcggtcgtgaacacggtcctcgaacaggagctgcccgaggaaatccaggtgggtgaagtggcccaggccatcgagcacaccagccagctcgaagaaaagctggccaagtcggccgagacattggccgaggtcaacgccgccttgagcgaggaaatcgagaagcgcctggagatcactgcccagcgcgatgaaagccaggcagaggccgaagaactcaaggcaaggatccaatccggcgcagcggactgatcgtctccacggtctttccagccggtacggatcgctccttatcccttctcctacgctgcggacgcatccggcacgctacgctattggttctcaaagcgaaaccacggcatggccctcatcacgttcctcgtcgaggacaacaagaccatcagggacaacctggtcccggctctcgaagatctggtcaacggccagatcgtcggcttcgctgaaaccgagtcggccgcgctcgcctggctcgcctcccatccccacgattggcaattgctcatcgtcgacctgttcctgaaagaaggctccgggctgggcgtgctctcgggctgcaagacacgcggcccgggccagcgcgtggtggtgctgagcaactacgtgacggccgacatccgtgcacgttgcgaagcactgggcgcggacgcggtcttcgacaagtcgcgcgacctcgacgccttcatcgactactgcaacaccgaccggccttcgggctttgccagattgaactgacgccggttgccgccagtgaccgtcctgaaatgcgttgacacccaaatagccggcctcagccgaccacggacgcccgatgcacgacatcgggcgtttgcattttgagcgacaaatggggccgctcgtggttgtagatctgcacggactcagccaccagtcgcctggcttgagccaggtcagttggctggctcagcaggaattcggtcttgaggatgccgttgatgcgctcggccagcgcgttctggtagcagtcgtagccgtcggtcatcgagcacttcaggccatggcggcgattcgcatcgcgccccaactcgatgccctggcgctgcaacggctcgcgcaacaggtagtgcagcttgcgcgtgcccagtctcggctggcgcatgcgctgttccttgaccaactgcaccaccgtttcggcgcgttcgtggcgccgggccgccctgtgctgaccttggtagtacgcctgacgagttatgcccatgtggtggcaagcccgggtcacgctcagcccttcgacgaggccttgcgcgaggacttgtccgaaggcttttttacgacacgcacgccgtgatccttcttcaggacctccagcaccgcttcgaacaaccgggccttttcctgcgctctggccagttgcgtttccaattccttgatccgctgttccggcgtcggtgcaatggctgtcttgtcgatcggcatagccgccgatgatgccgcacgaccccacccctggcgaccgtgcttgcgcagccagttcaacactgtcgagttgccctggatcccatagcggctctgcgcctggccgcaggtcaactcccctttttccacttgctcgacaacagccaatttgaaggccatcgtgtagtcaccctgcgttctcttgacgcctgtgtccattgcgctttttcctttcgctgatgaaaggtgtcaacgctgggcaggacgggtcaaagccaagaaaaaagggcccgaaggcccttttcctttttgcgccatggcgcagcggtttgcaatgaaaccgatcagcgcaccacggcgatctgtgtacgcacgccacccttgtaggtgaagagcgtcagcgcgccgttcttgatgtcgcccttttcgtcgaaggcgatcgggccggtcacgcccttgtattgcaccttgccgacttccggcaggtacttttcggggtcggaggaaccggccttgaccatggcttcagccagaacgttgaccgcgtcgtagacgtacggtgcatagatctggacttccacgccgttcttggccttgaacttggccttgaagtcttccagcggctgcttgaagtcgccatcgacaccgccggcttcggcgcaaaccaccatctcttcgccgatggcatcgccagccagcttgggcagctcgccggtgcacaggccgtcgccgcccatgaacttgacgttcaggccgagttgcttgacctgcttgagcatcgggccgccaacggcgtccatgccgccgaagaacagcacgtcgggcttggcagccttgagcttggtcaggatggcgttgaagtcggtcgacttgtcggtcgtgaactcgtggccgacgatggtgccgccagcagccttggccgccttttcgaactcttcggcaacgccctggccgtaggccgtgcggtcgtcgatcacggcaatgttcttgcccttgagcgtttcgacggcgtacttgcccagcgtgccgccgagttgcgtgtcgtcggccaccacgcggaacgcggtcttgaagccttggcgcgtgtacttgggattggttgccgaaggcgaaacctgcggaatgccggcgtcgctgtagagcttggaggcgggaatcgtggtgcccgagttcaggtggccgacgatgccgttgaccttgctgtcgaccagcttctgggccactgccgtgccttgcttcggatcgccggcgtcgtcttctgcgagcagttcgaacttggcaaccttgtcaccgatcttgaggcccttggcgttcaggtcttcgatggccatcttggcgccgaactcgttgtccttgccaaggtgggcaatggcgccgctggtgggaccgacgtggccgatcttgacgaccagcgtgcttgccggaggcgctgcaggtgcgggggccgctgccgtgggcgccggagcggcgggtgcagcagcttcttcttttttgccgcaagccacaagcgtgagagcagccagtgcgaccgcagtccatttcaattgcatgagaacctccagaacattgataaataaactaagaaccggtcgtgtgatccgggcgcgcagacctcgcaagtttcgcgccgcagaccagcggcaccctcccgccccaccgacctggcgcgcagtttagctgaagctttacgctccggaagttggcacagaccctgtgttttcggagagctcggcggccattgcttcgatcaccaaagcccgcaatacggcctcgatttcttcgcgcagccgaggcaccatggcatcgagttgctgctgcacggccgccgagaccgtgtcgctcaaacgctcttccaaagacaggtcgacgcgctgcagcacgcgatgcaggagctgctcttcgaggcggacgatttcggcctcggagcgctgctcggccggaggcagcgcaacggcttccgcggggtcgatggacggggccggcgcggccgcagggctcgccggctcggtgcccacaggctcggccggcaggtcgagcaccgtggtcagggtgggaacgaaccggggcggtgtacgcagcgtgctggccatcaggaagcgctccttgcaaagtcgtgcggctggatggtgtagccccggtcggcatagtggcgccaccgcgatcggccgatctgccggtctgtggcctcgtcgctcacgatgtcgatcaggcgctcgaagcgctcgaaccccgccgggacctcggcccccaaattcacgagcatttcgcggtgcggcagcgatgcggcctccgcgccctcggccgaaagaatgaccggcgagcgggccaccacatgaggctgcgcgtcggcgcggcaatgggcaatgaagtcggaaggcatgagctgccagagcgcggcatccaccgcctcgagcgtctgcgcctcgcccaccacgaccacgcgcagcccgcgcgcgttcacggcctttcgaaccagccggcaggcgtagttcaccttgtccggcgtattgaaatgaaagccgatttccgtcactgcgcggaccgggcctttcgggccgccgaaccggcgctcttgcgagcggccttcgacggggcggccggcttggcggtgccgctgcgcgcgcgctccatcaggtaggacaccagcagccccacgggccgcccggtcgagcccttggccgccccgctcttccaggccgtgcctgcgatgtccaggtgcgcccaggcgaagtcgccggcaaagcgctgcaggaacttggccgcggtgatggcgccgccggcacggcccgccacgttggccacgtcggcaaagttgctcttcaggccatcggcatattcgtcgtcgagcggcaggcgccagcagcggtcttgcgattcttcgccggccgcctggagcgccgcggccagcgtctcgtcagtcgtgaacaagccgctgcgtacgccgcccagtgccaccacgcaggcgccggtgagcgtggcgatgtcgatcacggcggccggatcgaaccgcttggcgtacgtgagggcgtcgcacaggatgagccgtccctcggcgtcggtgttgagcacttcgatggtctggccgctcatgctggtgaccacgtcgccgggcttgattgcgcggccgtcgttcatgttctcgcacgttggcacgaggcccaccacgttgatggccggctggatttctccgagcgcgcggaaggtacccagcacgctggccgcgccgcacatgtcgaacttcatctcgtccatttcggcggccggcttgagcgagacgccgccggtgtcgaaggtgatgcccttgccgaccagcaccaccggcgcctggtccttggggccgccctggtagcgcagtacgatgaaccgcagcggttcggccgaaccttgtgcgacggcggcgaacgagcccatgccgagcttctgcacctccttggggcccagcacctcgcatttgatgcggggcagcctggacaggcccttggccgcctccgccagcagagtgggcgtgcaatagttgccggggcggttgccccactcttttgcaagctcgatgccggacacggtggcgcgggcttcgtcgaaggccttgcccaccgccgcggcgtcggccacgccgagcgtcaggttgcggatggtgcggccgttctcgccgttcgaggtctttgccttggtcgtggtgtagacgtagctggcgtcggcggcggcggccacggcgcaggccacggcggcaccatcggcctcttgcgcgaaggccatgaccacgcgcctgggcccgtaggccttggccgcgttgaccgccgcgatgacgccgccgcgcaccgacgcgggcttgccgtcgccaatggccgccagcacgacgcgcgaggccaccacctcgtcggggtggtagagcgcgagcagcttgccggccttgtcgggcaggtcgccggccttgcgggcgctggcaatcagtgcggaaagcgggtccttggcggtgaggggtgcgctgccgacgagcacgatcagcacgtcggatttttcggctgccgcgcgggcaacggtgagggtcttgagctgaaagtccataatcctttttttcctcgaacgatgttattccattcttccttacgcaaggagctgtcgcgcagcttcggagcgaccctcgtcgtcctggtcaccatcgtgatgaccatgatgctcatccgcacgctcgggctcgcctccaagggcagcgtgaacccgtccgaagtgttcctggtgatgacatacacggtgctcggctacatgccgaccatcctgagcctgagcctcttcatcgccattgtcggcaccttgtcgcgcatgtaccgcgacagcgaaatggtgatctggttctccagcggacgcggcctggccgatttcgtcgagccgctgttccgctttgcctggcccgtgctcgcgttgatcgcggtcatggcgctggtgggctggccctgggccaactcgcagaccatcggcatgcgtgcgcagtacgaaaggcgcagcgacatcgaacgcgtcacgccgggcgagttccgggaatcctccgggcgcatgcgcgtcttcttcatcgacaaggacacgcctgacggcgccacggcgaccaacgtgttcatctgggccgtcgagcgcgggctgcagatcacgacctcggcgcgcagcggccgcatcgagaacatcggcgagaaccgctacctgatgctgagcaacggccagcggctcgaacgcccgatgctgcccaccgagggcctcaagatcagcgaattcgaaacctacggcacccgggccggcggcaatgcggacctggcgggcgacagcaccccggcgcgcgccaagccgacgctgcagctcctgcgggagcccggcaacacaagccgcggagaactagcctggcgcatcggcatgctgctggccggcatcaacttcgtgctgctcgcgttgaccgtgtcgagcgtcaacccgcgcgtggggcgcagcggcaacctgctctttgcactgttcgccttcgtcgtctactacaacatgctcaacctgggccagagctggatcagctccggccgcttcggcatgggttccttcatgctgctgctgcacggcggcgtcctgctcatcggcgtcgcgtggctggtcctgcgcaacaacaactggggccggcggcgcaagaccgagcgcgtcatcgccggcggcctgccctcccagaccgcgaaaatcgacccgacctcgtgaaaacaatccgacgcctgatctatgtcgaggcactgaaagccgtggctttcgtgacgctcggcttcctgagcctgtttttcttcttcgacttcgtcgacgaactgcagtccatcggcaagcccgaaagcctggcttacggccccgcgcaggcactgatctacgtgaccctgctgattccgagccatttgtacgaactgctcccgatcacggtgctgatcggatgcatcttcgtgatggcacgccttgcgcaaagctccgaatacaccattcttcgcaccagcggcctcggcccctggcgcgccctgcgcaccctgctgctgctcggcgtcggctttgtcgtgttgacctttgccatcggcgactacatcgcgccggtctccgaacgcaccgggcaacttctcaagtcgcgctaccagggcgcgtattcgctggtgggcaatacgggggcctggctcaaggaaaagcgcgagaacgtgtcctatgcggtcaacgtgctgtccatcgcgcgcgatggctcgctgaagaacgcgcgcatcttcgagttcgacgccaacggctacgtgcgcaaacagctcgtcgcatcttcggcgcgcatccacgacgaccgctgggtgctgtcggatgtcgaactgcaggactacgacacgcgcaccaccgcggacaaggcccacatcgtcaccaccaaggtgccgcagctcgactggccgaccacgctcacggccgaaatggtgtcggtggcactgctgcggcccgaccgcatgggcaccatcgacctgttcgactacatcagccatctcgaagccaacggacaaacggcgcagcgctacgagatccagttctggcgcaaggtcttctatccgctctcgtgcctcgtgatggtggtgctcgccctgcccttcgcgtacctgcacttccgccaggccggcatcaccacctacgtgtttggcggcgtgatgatcggcatcagcttcttcctgctgaacaacgtgttcggctaccttggcaacctgagcaactggtcgccctggctgacggccgcggcgccggggctcatctattcggtcatgtcgcttgccgcgttcagctggctggttctccgaagataaaaagagaagaaaaaccaccgatggcggctgaaaaagcaaggggcatcatcctcttggcccatggatcgcgcgacgagcgctggcgcgcgccgatcgaggccgtggccgcgcgcgtcacggcgctcgacccgcaggcccgcgtggtttgcgcctacatggaactggccgcgcccgatctgcgcaccgcggcggcggccttgattgccagcggcgcccgctcgctcagggtggttccgctcttccttggcatgggaaagcatgcccgcgaagacctgccgctgcagctcgacgcattgcgcggcacctggccgcaggtcgatttccagctggccagcatcgtcggcgaggagcccgagctggtcgaactgctggccagaattgcaagcaaatcttgaattcgcagctatttccatagactccgaaggcataatgaattccgcaataagacggaatttgatatgaatctgcaccagttcaagtttgttcaggaagccgtgcggcgcaacctgaacctcacggaagcggccaaggcgctccacacttcgcagccgggggtgtcgaaagccatcatcgagctggaggaagaactcggcgtcgagatcttcgcccgccacggcaagcggctcaagcgggtcacggagccgggccagcatgtcatcgccagcatcgaactgatcatgcgcgaggtgggcaacctcaagcgcatcggcgagcagttcagcgcgcaggacagcggcaccctctccatcgccaccacgcacacccaggcgcgctatgtgctgccggtgcccgtggccaagttgcgcgaggcctacccgaaggtcaacgtgagcctgcaccagggctcgcccgaccaggtggcacgcatggtgatcgacgagatcgccgaggtgggcattgccaccgaatcgctggccgactacgccgagctggtgacgctgccctgctacgaatggcagcacgtgctggtgctccccaaggaccacccgctggccgccaaggaccgcatctcgctcgaagacctggcgcacgaacccatcatcacctaccacccgtctttcaccggccgcacgcgcatcgaccacgcctttgcgcagaagaagctcacgccgcgcatcgcgctcgaagccatcgattccgacgtgatcaagacctatgtgcgccttggcctgggcgttggcatcgtggccgaaatggcggtgcgcgacgagtcgaacgccgacctcgtggtgcggcccatgggccatgtgttcggccagaacatcgcacgcgtggcgttcaagcgcagcgcgtacctgcgcaatttcgtgttcaagttcgccgagctgctgtccgaccggctcgaccgcaacctgatcgccaaggccctgagcggccatcagcaagactacgaactctgagatccagtccccagcttcctccgaccacgaccatgagcaccgctacttcttctccccgcacaccggccatcggcaccaagctgcccgccgtcggcaccaccatcttcaccgtgatgtccgccttggcggcggagaagaacgcggtgaacctcggccagggcttccccgatttcaactgcgacccgaagctgctcgaagacgtgacagccgccatggccgcgggccacaaccagtacccgccgatgcccggcattccggcgctgcgccaggcgattgccggcaagatcaccgcgctctacggccacagctacagcgccgccgacgagatcacggtgaccgcgggcgccacgcaggcgatcatcacggccatccttgccgtggtgcgcgcgggcgacgaggtgatcgttctcgagccctgctacgacagctacgtgcccaacatcgagcttgccggcggcagcgtggtgcgggtgccgctcgtgcccggcaccttccggcccgacttcgacaagattgcggcggcgctctcgccgcgcacgcgcgcgatcatcgtcaacacgccgcacaacccgagcgccacggtgtggaccgcggccgagatgcgcaagctcgaagaattgctcgccccgaccgaggtgctggtgattgccgacgaggtctacgagcacatggtctacgacagcgcacagcacgaaagcgtggcgcgcttcccgggcctggccgcgcgcagcttcatcgtgagcagcttcggcaagacctaccacgtcaccggctggaaggtcggctacgtggcggcaccggcaccgctcatggccgaattccgaaaggtgcaccagttcaacgtgttcaccgtcaacacgcccatgcagcatgccctcgcgcagtacatggccgaaccggggccctacctggaactgccggccttctaccagcgcaagcgcgacctgtttgccgccggtctggccgaaaagacccgcttcaagctgttgcgcagcgagggcagctactttcagtgtgtcgacatctccgaggtcagcgagctttcggaggccgacttctgcctgtggctgacccgcgagatcggcgtggcggccattccgctgtcggctttctatggcaacggcttcgaccagcgggtggtgcgtttctgcttcgccaagaaggacgagacgctgctggcggctctggaccggctggcacggctataaagccgacgctgccggtaggatagtcctgaccgccgaaggagcggctttccggcgtgtttttcgcccctggacggcgagcatgaatgctcgtaacaacaacgtccaggagataagcatgtccctctcgttcattctgctgatcgttctgatcctgctgctgataggcgccttgccgagctggggctacagccgaggctggggctactggcccagcggcggcctcggcctggtcttgctgatcgtcatcatcctggtgctcatgggacggatatgaagcttccggacatttcgcgcacctgaaaggagcccgcggcaagcgggctttttttcgcctgcctgccggggtcaggcctgcagctgggcccaggccttgtccagccgcttgatgctgaccggctgcggcgtgcgcagttcctgcgcgaagaagctcacgcgaagctcctccagcagccagcggaattcgagcatgcgctcgtccacggcacccttgcgctccgccaccagccgccaatagcgctgctcttgcggccgaagctccgccagcttggcggcatcgcgcgcgggatcggcgcgcagcttgtccaggcgcagcacgatggccttgagatagcgcgcgaaatgctgcagctgcgtccagggcgcatccgagatgaagcgcttgccgaccagtcgctgcaattgctgcgcggcatcctgcacggcttcgggctggatcttggtgtccttgatcttgcgcgccgcagcggcgtactcggccaggatggccgaggccagccgcgccacctcgttggcaatcagggtgagccggccgcggccctcttcgaggcggcgcttgaaggcgaattcatctgtgggcagcggctcctgcagaaaggccctgtcgatcgcgacgtcgatgatctgcgcgcgcagctcttccgacgtgccgagcggcatgtaggccaccgccatcttctgcagatcggggatgttcttttcgaggtacttcagcgcatctttcagctgcagcgcaaacaagcggcgcagaccggcgcggtgcttcgcggcggccacggcgggctcgtcgaacacctcgatggtgacggcatcgccttcgtcccgcagggccgggaatccgatgagcgactgcgcgccacggcgcacttccatcagctcgggcagctcgccgaagctccagctcgtgtagcgctggcccgcgggcaggctcggcgcagcgggggctggcgcagtggcatggcccttggcctgtgcctgtccttcggcggcttcggccggcttgcggtcggcggaagccttgacgttgagcccggccagcgcctggaaggcgcctcgcgcctgcgcgcccagttccgccttgagcgcgcccaggttgcgtcccatgccgagctggcgtccatgctcgtccacgatgcgcaggttcatgaacaggtgcggcggcagcatgtcgagcttgaagtccgcgcgcttcacgtcgatgctcgtcgcatcgcgcacgcgcttgagaagcacgtcggtcaacgaaccatggccgaacacctcgggcgccgagagttcttccgcgagctttgccgccgaatcgggcagcggcaccagccgcgagcgcgggcgctgcggcaggctcttgagcagtgcctggatcttgtccttgagcatgcccgtcaccagccattcgcagcgctcttcgctcacctggttgagcacgaagagcggcgcgctgaccgtgaggccgtccttcgcatcgccgggttcatgcaggtagcttgccgcgcagtcgacaccgccgagccgcagcgtcgacgggaacgactgcgtggtgataccggccgcctggtggcgcatcagctcttcgcgtgtcaggaagagcaggcgcggctgctccctcgaggcgtggcggtaccagttctcgaaggtgatgccgctcgccacgtcggcgggcagctgcgcgtcgtagaaggcgaagatcagctcgtcgtcgaccagcacgtcttggcggcgcgacttgtgctccagcccttcgacctcgcgcaccagctttcggttggccacgagaaacggaaacttgctctcccattgcccaccgaccagcgcttcgcgaatgaagatctcgcgcgccgccaccggatcgaccttggtgaagtcgacccggcgtccgctgtagaccacgaggccgtagagcgttgcacgctccagcgccgaaacctgcgcgcccttcttctcccaatgcggatcgagcagctgcttcttcagcagatggccggccacctgttcgagccactgcggctcgacgttggcaatgccgcggccgaagagccgcgtggtctcgaccagctcggccgccacgatccagcggccgggcttcttcttcaggtgcgcaccggggtgcttgtagaacttgatgccgcgcgcaccgaggtacgcctcgtcgtcctcgagcttccagccgacgttcccgagcaggcccgcgagcatagagaggtgcagcggctcgtagccggcaggctcggcgttgatgcgccatttgtgctcggtcaccacggtgagcagctgcgaatggatgtctcgccactcacgcacgcgccggatgttgatgaagttctggcgcagcagctgctcgtactgccggttgctgagcttgtgagtgtcgccatggccgccgcgcgcatcggcgatccatttccacaggcgcaggtagccgctgaactcgctcttctcgtcgtcgaatttcgaatgcgcctggtcggcctgctgctgcgcctccatcggccggtcgcgcacgtcctgcacgctcagcgccgacgcgatgacgagcacttcttcgagcgcgccgcgtgtgcgcgcctccaggatcatgcggcccacgcgcgggtcgagcggcagcttggcgagctcgccgcccgtggcggtgagctcgttggcatcgtcgaccgcgccgagttcgttgagcagctggtagccgtctgcaatggcgcgcggcgaaggtgcctctagaaacgggaaccgcgccacgtcgcccaggcgcagcgacttcatccgcaggatcacgccggccagcgaggaacgcaggatttccggatcggtgaaacgcggtcggccttcgaagtccttctcgtcgtaaaggcggatgcagatgccgttggccacccggccgcagcggcccgcgcgctggttggccgcggcctggctgatcggttcgaccagcagctgctcgaccttgctgcggaagctgtagcgcttgacgcgcgcggtgccggtgtcgatcacgtagcggatgcccggcacggtgagcgaggtttccgccacgttggtggccagcacgatgcgccggcccgtgtggctgtcgaagatgcggtcctgctcgggccccgacagccgcgcgaacagcggcagcacctcggcattgcgcagcagcggctggtggctcaggtggcggcgcagatgatcggccgcctcgcggatttcgcgctcgccgggcaagaacaccaggatgtcgcccgcgttgtgcggatcgcgccagagttcgtcgacgccgtcggcgatcgcatcgttcaggtcgtgttcgcgcgattcttcgaagggccggtagcgctgctccaccggaaacgtgcggcccgacacatagatgatcggtgcgggccctttggccgaggcgaaatgctgggcgaaccggtcggcgtcgatggtcgccgaggtcacgatcaccttcaggtcgggccggcgcggaagaatctcgcgcaggtagcccagcaaaaagtcgatgttcagcgagcgctcgtgcgcctcgtcgatgatcagcgtgtcgtaggccttgagcagcggatcggtctgcgtctcggccagcaggatgccatcggtcatgagcttgaccgaggcgtcgcggctcagccggtcctggaagcgcaccttgaagccgaccacgtcgcccagcggcgtcttcaactcttcggcaatgcgcttggccaccgagcttgcggcaatgcgccgcggctgcgtgtggccgatgagccggcccttgcctggcggcgcatggagcttgccgcggccgagcgccagggcgatcttcggcaactgcgtggtcttgcccgagccggtttcgccgcagacgatcaccacctggtgcgcctcgatggcggccatgatttcgtcgcgccggccggagaccggaagcgattcgggaaagtcgatgcgcaagggagcggaaggtgtcgtggtcgtcaagggaaaagctgattcgcgaaggcgcggcgggcaaaccgtcgattatcggtgcgcgccgcccctgttgcacgccttgcgatgccacccggctgctgcgggcgatggcccaccccgcgcgaaccgccctccaagaatgcacaatcacgctccatgtccaccgttttcaacttcaccttcgtgccctggttccgctcggtcgcgccctacatccacacgcaccgcggcaagactttcgtggtcgccctggcgggtgaggcgatcgcggcgggcaagctgcagaacattgcgcaagacctggcgctgatccagagcatgggcgtcaagatcgtgctggtgcacggcttccgcccgcaggtcaacgagcagctcgcggccaaggggcacgaggcgcgctactcgcacggcatccgcatcaccgacgaggtggcgctcgattccgctcaggaagccgccggccagctgcgctacgagatcgaggccgcattcagccagggcctgccgaacacgccgatggccggctccacggtccgcatgatttcgggcaacttcatcacagcccgccccgtgggcgtggtcgatggcgtggacttcaagcattcgggcctggtgcgcaaggtcgacgccgcgggcatccgccgcacgctcgatttcggtgccatggtgctgatgtcgcccttcggcttctcgcccaccggcgaggccttcaacctgacgatggaagaagtggccaccagcgtggccatttcgatccaggccgacaagctgatcttcctgaccgagattccgggcatccgcatcgacagcgaattgcccgagagcgaagacaaccccatcgacaccgagctgccgctcgccgcggccgaaaagctgctggcgtcgctgccgccaccgcagaagccgaccgacaccgccttctacctgcagcactgcgtcaaggcctgcaagggcggcgtggagcgcaaccacatcctgccttttgccctggacggcgcgctgctgctcgaggtgtatgtgcacgacggcgtcggcaccatggtgatcgacgagaagctcgaaagcctgcgcgaagccacggtcgacgacatcggcggcatcctgcagctgatcgagcccttcgagcgcgacggcacgctggtcaagcgcgaccgcaccgagatcgagcgcgacgtgggccactacacggtcatcgagcacgacggcgtgatcttcggctgcgcagcgctctacccctaccccgaggcaaagaccgccgagatggccgcgctgaccgtctcgccccagtcgcagtcgcagggcgacggcgaacgcatcctcaagcgcatcgagcaccgcgccaaggccatgggcctggaaagcatcttcgtgctcaccacccgcaccatgcactggttcctgaagcgcggcttccagcaggtcaaccccgactggctccccgaagcccgcaagcgcaagtacaactgggaccgcaaaagccaggtgctggtcaagaaaatctgaacctttgaacctttgaagggaagcccgccgccatgacgttcgccaccgccttgctgttctccatcgtcgcgctggccgccatcgcaacgcccgggccgaccgtgctgctggcgctgagcaacggatcgcggcgcggcgtgcgcggcgcgctgccgggcatcctgggcgccgtgctgtccgacttcgttctggtcggcgcggtggcgctgggcctgggcgcgctgctggcagcctcggagttctggttctccatgctcaagtgggtgggcgccgtgtaccttgcctggctgggcgttcgcatgctgcgctccaaaggcggcagcttcgacacgccgcgtgccgacgcaggcgagccggccacgggcatgaacggagacggccgcaaggtctttttcaagtcattcctggtggcggtcaccaacccgaagggctatctgttctgctcggcgctgatgccgcagttcatcgaccccgcagccgcgcagggcatgcagtacgccatcatcgccgtgctgtttgcctcgctggacgcattggtgatgggggtctacgccttcgtgggcgcacgggcaatgcggctgctgacggccgccgcaggccgctggatcgaccgcacctgcggcgcgatgctgctggcgctggccggctcgctggcgttctaccggcgcagcggtacctgagcggcgcgggagggctgagcggccggcgacccgtcgccgataatcgctctccatgaatcccctgctttccaagctccagccctatcctttcgagcggctgcggcgcctgttcgagggcgtcacgcccaatgccgatttcgcgcccatcagcctgggcatcggcgaacccaagcacgccacgccggccttcatcaaggaagcgctggccgccagcatggccacgctcgcggcctacccggccacggccggcaccctggcgctgcgcaccgcctttaccgactggctgcagcgccgctacgccctgcagctggacccggccacgcaggtgctgccggtcaacggctcgcgcgaggcgctgttctcgcttgcgcaaacggtggtcgacggcagcaagacccccgcgccggtggtggtttcgcccaacccgttctatcaaatctacgaaggcgcagccctgctctcgggcacagagccctactacgtgccgagcgtaccggcgcgcaacttcgcggtggactgggacagcgtgcccgaggccgtctgggagcgcacgcaactggtgttcgtctgctcgcccggcaacccgaccggcgccgtgatgccgctggacgaatggcgcaagctctttgcgctctccgaccgctacggcttcgtgattgcagccgacgagtgttacagcgagatctacttccgcgacgagccaccgctcagcgggctggaagccgcctccaagcttggccgcgccgacttcaagaacctgatcgcactcacctcgctgtccaagcgcagcaatgtgcccggcctgcgcagcggcttcgtggcgggcgacgcggccatcatcaagagctttctgctctaccgcacctaccacggcagcgccatgagcggcaccgtggccgcggccagcattgcagcctggggcgacgaaacccacgtggccgagaaccgggccaagtaccgggccaagttcgctgccgtgacgccgctgctcgaaccggtgctcgacgtgcggctgccggacgccagcttctacctctgggcgggggtgcccgaagtgtgggctggcgacgacgaatccttcgcccgcgcgctctacgctcaatacaatgttacggttctgccggggagctatctggcgcgcgacacggcacacagcgccaaccccggccgtggccgcatccgcatggccctggtggccgaaacggccgaatgcgtggaagccgccgagcgcatcgtccgcttcgtgcaatccggccaaccaggccggggctgaaccgctgctttcccggctcccatttttcacacgagactttctccatgacccagcaactgcaacaaatcatcgacgccgcgtgggaagaccgcgccaatatctcgcccagcgccgcctcggccgaagtgcgcgacgccgtcgagcacgtgatttccgagctcaacaacggcaagctgcgcgttgccacgcgcgagagcgtgggcaagtggaccgtgcaccagtggatcaagaaggccgtgctgctgtcgttccgcctgaaggacaacgagcagatgcaggccggttcgctcggcttctatgacaaggtgccgaccaagttctcgcacctgtcggccggcgagctgaaggaatcgggcgtgcgcatcgtgccgcccgccgtggcccgccgcggcagctacatcgccaagggcgcgattctgatgccctcatacgtgaacatcggcgcctacgtgggtgaaggcaccatggtcgacacctgggccaccgtgggttcgtgcgcgcagatcggcgccaatgtgcacctgtcgggcggcgtcggcatcggcggcgtgctcgagccgctgcaggccggccccaccatcatcgaggacaactgcttcatcggcgcccgttccgaagtggtcgaaggcgtggtgatcgaagaaaactcggtgctcggcatgggtgtgtacatcggccagagcaccccgatcttcaaccgcgacaccggagaaactctcttcggccgtgtgccgtccggcagcgtcgtcatcagcggcaacctgcccaagaagaccaaatcgggccaggactacagcacctacgcggcgatcatcgtcaagacggtcgatgcgcaaacgcgctccaagaccagcctgaacgacctgctgcgcgattgatcccgcctttgtccctttagaaaacaacagcacccgaggagagtgagagcgatgaacatgatggagcgaatccttcgtctgatggccgagcgcaaggcgtccgacatctacctctcggcgcactccccggtgctgatccgcatcaacggcacttgcgtgccgatcaacgcccaggtgctgccggccaccgcgccgctcgcgctgctggccgaagtggtgcccgaagcccgcatccaggagctggagagcaagggcgagctcaacatggccgtgatgctcgagggcgccggcaactaccgcatcagcgccatgcgccagcgcggcagctatgcggtggtggtgcggcacattgcctcgaccattcccagctttgccgacctgaacctgcccgacattctcaagacgctgatcatggagaagcggggcctgatcctgatggtcggcgccacgggcgcgggcaagaccaccacgctggcctcgatgctcgactaccgcaacgagcacgccacgggccacatcctcacggtggaagagcccatcgagttcacctacaccaacaagaagtcgctggtgaaccagcgcgacgtgggcagcgacaccgagtcgctgcatgtcgcgctcaagaacgcgctgcggcaggcgcccgacgtgatccagatcggcgaaatccgcgaccgcgaaaccatgaccgcggccattgcgtatgcgcagtcgggccacctgtgcgtggccacgctgcacgccaacaacagctaccgcgcgctgaaccgcatcctgagcttcttcccggtcgaggtgcgtcccacgctgctgggcgacctgggctcggcgctgcgcgccatcgtctcgcagcggctgctgcgcacgcccacgggcggccgcgtgccggcgctcgaggtcatgctcaacacggccctggtggccgagctgatcgaaaaaggcgatttttccgccgtcaaggaagccatggagcaatcgatggccgaaggctcccagaccttcgaggaagacattgcccgcctcatcaccgaagagcgcgtgacgcgcgaggaaggcctggcccagtccgactcgcccaccaacctgatgtggcggctgcagaaccgcgccgcgcccaagcagaaggccgaagagcgcaacctgatggaccaggtcgacgaacccacctttaccgacatcacgctcgacgtgaagttctgacccagcctctccggctttttttccgatgtcccgtacgctccagctcgccgaacaactcatctcgcgcccctcggtcactcctgacgatgcgggctgccaacagatcctcagcgaacggctggcgccactgggcttcacgctggagaccatcgagagcggtcctgcggatttccgcgtgaccaacctctgggcggtgcgccgcccggcggctgccgcggcaacaaagacgctggtgttcgccggtcacaccgacgtggtgcccaccggcccggtcgagcaatggaccagccaccccttcacgcccacgcaccgggacggcaagctttatggtcgcggcgcctgcgacatgaagacctcggtcgcggctttcgttgtctccatcgaggagttcctgcgggccacgcccgatccgaagctcacgctggcgctgctgctcaccagcgatgaggaaggcccggcggtcgacggcaccgtcgtcgtctgcaacacgctggcggcgcgcggcgaggtgctcgactactgcatcgtcggcgagcccaccgccgtcgagcgctgcggcgacatgatcaagaacggccgccgcggcaccatgagcggcaagctcacggtcaagggcgtgcaggggcacatcgcctacccgcacctcgcaagcaaccccgtgcactcggtggcgcctgcgctggccgaactcgtggccatcaacgcggccggcggctgggatgcgggcaacgactacttccagccgaccagttggcagatcagcaactttcatgcgggcaccggcgcgagcaacgtgattccgggcaacgcggtggtcgatttcaatttccgcttttcgaccgagtcgacgcccgagtcgttgcagaagcgcgtgcatgcggtgctcgatgcccatggcgtcgactacacgctggcctggaccgtcggcggcctgcccttcctgaccacgcccggcgaactcgtctcgtcggtgcaggcagccattgccgatgaaaccggcatcgcgaccgagctctcgaccagcggcggcaccagcgacgcgcgcttcatcgccaagatctgcaagcaggtggtcgagctcggcccggtcaatgccagcatccacaagatcgacgagcacatcgacgtggccgagatcgagacgctgaagaacatctacaggcgcacgatggagcggctcgaagcgtcgctggtcggatgagcgccgcgccgggccgccccaagcaagctcgcaccgcagcgcgaagcgcggaggtaattcagtgagcacggtcatcgagctgatcgaggccggcgccaagcggctcgaagccgccggcgtggccttcggccatggcaccgccaacgcctttgacgaggccgcctggctggttctgtggcgcctgaagctgccgctcgatgaaatcgatgccgtggccgacacgcccgtttcgccggccgatgcgagcaaggttgccgcgttgctcgacgaacgcatcgccacgcgcaagcccgccgcctatctgacgaaagaggcctggctgcagggtgtgcccttctacgtggacgagcgcgccatcgtgcctcgcagcttcattgccgagttgattgccgacggcagcatcgactactggctcggcgaacacacgcagcgcgtgctcgacctgtgcacgggcaacggcagcctggccgtcctggcggccatgacttatccggagaccaccgtggacgcggccgacctgtcggtcgaagcgctcgaggtggccgccatcaacgtcacgcggcaccagctcgacagccgcatcaggctgatcgaatccgacggcctggccaacctgcccggcccgtacgaccttgtgctgtgcaatccgccctacgtgaacagcgcgagcatggccgccctgcccgccgaatatcaagccgagcccgaactggcactggccggcggaaccgacggcatggacttcgtacgccggctgtttgccgatgctccctcgcgcatgagcgaagaggccgtgctggtgctggaaatcggcaacgagcgggactacttcgaagcggcgtttccgcaactcgaggtcgtctggctcgaaacctccgcgggtgaagaccaggtcctgctcgtgacccgggccgcgctgctggccggcgccggcgcgcgttagctgccccagccctcgccttttcttcccctctgccgagtttccgcagcgacggctgcaagcccttcttttaccgggcggcgtcctcatttgcccctttgcgccgagccgccacggccgggcgggataatcgcccctacggttcctatttcatgattactctcaaaaacgtcattcttcgccgcagcgccaaggtcctgctcgacggcgccaccgtcaccatcaaccccggtgaaaaggtcggcctcgtcgggcgcaacggcgccggcaagtcgaccctgttcgcgctcttcaacggttcgctgcacgaggacggcggcgacttctacgtgcccaagcagtggcgcatggcacaggtggcccaggacatgcccgaaaccgaggagtcggccaccgacttcgtggtgggcggcgacacccgcctggccgagctgcgcgccacgctggcggccatcgaggccgcctacgaagccaaccccgacgacgccgacatcggcatggaactggcgcacgcctacaccgacctggccgacgccggcgagcacgacgccgtgccgcgcgcccaggccctgatcctcgggctgggcttcaagtcgcacgagctggatggccccgtcaacagcttttcaggcggctggcgcatgcgcctgcaactggcccgcgcgctgatgtgcccgagcgacctgctgctgctcgacgaacccaccaaccacctggacctggacgccctggtgtggctcgaagcctggttgcaaaagtacgccggcaccatgatcgtcatcagccatgaccgcgagtttctcgacgccgtgaccgacgtgaccttgcacatcgccaacgcccagctcacgcgctacggcggcaactacagcaagttcgaggacatgcgcgcgctgcagatggagcagcagcaggtggccttctccaagcagcaggacaagatcgcgcacctgcagaagttcatcgaccgcttcaaggccaaggccagcaaggccaagcaagcgcaaagccgggtcaaggcgctggaacgcatggaaagggttgcgccgctcctggccgaggccgacttcaccttcgagttcaaggagccgggcaacatccccaacccgatgctgtcgatcagcaatgcgagcttcggctacgaaatcgaagatgccgagcccaagaccatcctgcgcggcgtgagccgctcggtgctggcgggccagcgcatcggcatcctgggcgccaacggccagggcaagtcgacgctggtgaagaccatcgcgcgcgagatgggcgcgttggccggccaggtcaccgaaggcaagggcctgaacatcggctacttcgcgcagcaggaactcgacgtgctgcgtccgcaggacaacccgctcgagcacatggtgcgcatggcccgggaactgggcagcgccgtcaaggaaagcaccggcgagcaggccctgcgcggcttcctcggcagcttcaacttcagcggcgacatggtgaagcagcccgtcggcaccatgagcggcggcgaaaaggcgcgcctggtgctcgcaatgatggtgtggcagcgtcccaacctgctgctgctggacgagcccaccaaccacctggacctggccacgcgcgaggccctggccgtggcgctgaacgagttcgaaggcacgctgatgctggtaagccacgaccgcgcgctgctgcgctcggtgtgcgacgagttctggctcgtggggcgcggcgtggtggccgatttcgacggcgacctcgacgactaccagcgctacctgctcgacgaagccaagcggctgcgcgaggaggccaagatcgccgtgcgcgacgcggccgccgcaaccgctgccgagcccgtggccgttgccgctgctcctgcacccgccgccagcgaacccgcggccgcggcgaacaagaacccgcagcagcgcaagcaggacgcccaggggcgccagcaacgcagcgaccaggccaagccgatcaagcgcgagatcgcgcagatcgacgagcgactggccgcggcgggcaccgagcgcgccacgctcgaggcgcgcctggcacagccgctaccgtccgccgagattgccgaagcgggcaagcgcctgaaggctctcaacgacgaaatcggccgactcgaagagcgctggctggccctgtcggaccagctcgagacgctggcggcctgaccctgcaaaggaggcacatcgcatgccgtctgccatcgaactggcccggggcgacgaaaaactgatcgcggccattcaccgcagccgccgcctgatcggccgcaaggccttgatggccgcggccgccagcgccgttccgttgccgggcatcgactgggccgccgacgcggccctgctcgcacgcctcgtgccgcagatcagcgccgagttcggcctttccgtcacccaggtcgaaaagctcgcgccacatcagcgcgaacgcatccagaaggccgccaccacggtcggcgccttgctggtcggccgactcgtcacccgcgaactgctgatcaagctcgcccggtatgcgggcgtgaagctcaccgtcaagcaggccaccaagtacgtgccgttggccgggcagatcgtttccgccgccctcggctatgcggccttgcgcgccctcggcgagcagcacatcaaggattgcgtccgcgtgagtacgacgctcgccctttcgccgcccgaaccgcacgcgcccgcctgaacgcgcaatcgtcgaacaagacaatcctctctggtcaggttgcgtgcaggttcagcgaacatagtggaggctctcccgtggcctgcactccctcctgatcctccctcctccagcaggtcaccttccagcccgcccttgtgcgggctgtttttttggcgcgcagcgagaaaagattcaaccgatgcaggcataaaaaaagccgctcgatggagcggcttcttgaggggtggtaggacgtactggattcgaaccagtgaccaacggattaaaagtccgctgctctaccaactgagctaacgtcccggaaccatttttctttttcacgctttgccggggttgatccggcaaagccaaagattataacgtggcgttgctcgcaattttgtcgagaacccaacctgccgcacattgaccgaaagtagccgtgacgctaaccaccgagccgtagccgtggcagttgagcgagccgtcgctttcgatggcgcaggaggcatcgggcggcgcgacgctctcgcggctgaagacgcaggtcacgccgatcttgcggccctcgcgcggagcaccatgctccttgcgaaggcgctgccgcagctgggccagcagcgggtcgtgcgtgacgagcgagagatcgtcgatgtcgaccttgtgcgcctgccgcttgccgccggccgcacccacggtaacgaaggccgtgcccgatgcgcgcgcccatgcggccatcgtgagcttggcctttacctggtcgcaggcatcgatgacggcggttgcagggccgttggctcgctgcgccgcttcgagcagcatcgtccagttgccgggctcgacgaactcgtcgatcgcaagcaccttgcactccgggttgatctgcgcgatgcgatcgcgcatggcctcgaccttggcctgtcccaccgtcgcatcgagcgcatggatctgccgattgatgttcgactcggacacatggtcgagatcgaccagcgtcagccgccccactccgctgcgcgccaacgcttcgacagcccacgagccgacaccgccgatgccggcaatgaggacatgggcgccgcggatgcgcgcggcaccggccactccgtagaggcgttcgaggccgccgaagcggcgcgcaaagtcaggcgccgccgcggtgtcggtgatgacgacatccacggcggcgttcgatgcttgcggaagcgttgctgcgctcaagcggaggctccgctggcgctagcgcagtcgcgagagacgctcgcggcccgcctgtgcggcttcggattggggataggccttggtcaggtcttccagcgtgcggcgcgcggcgcgcgtgtccttcagctcgatctggcagttggcaatcgacagcacggcctcgggagccttggcgtggtcgggtgcaagcgacagcatggagcggaagttcgcaatggcctcgttgtagttgcgcgtagcgtattgcgcattgccgagccagaacaacgcagaggcgttgtagccgctttgcgggtagcgcttgacgaactcggcgaacgcggtttgcgcctgcgcgaactggcccgcgcggaagatgccgagcgccgcatcgaagtcggctttttccttgggatcggcagtgaactcgcggccgtccaccgacaccttggccggctcgttctgcttgagccggtcgtcgatggtggtctggcgcgactgcatttcgctcagcgtgcgctgcagctgctcgttctgcccggtcatgcgtgcaagatcgccccgcatctgctcgatctggttttgcagttcgagcaggctgcggcgcagctggccgttttcgtcggtcagccgctggtcggtctgctggcgcatcgcctcgacccgctgccgcaggtcgaggatggcgcggcgcgcttcatcatcctcgaacaatgcagcttgcgagccgatcgaaacgcaaagcaaggcggcagccagggccgcgcctcgcaacaaggcgcgttgcatcaccgggtgtatcggatttcagcgcggcggttctgcgcccaggcttcttcgcccgagccctggaccgcgggcttttccttgccgaagctcacggcttcgatctgggcgtcgttcacgcccagaagcgtcagcgcacggcggacggcttcggagcgcttctggcccagggccaggttgtactcgcggccgccgcgatcgtcggtgtggccttcgatggaaacgcggcgctgctggttggccttgaggaaacgggcatggccgtcgatcagggcttggaactcgggcttgaccgtgtagctgtcgtagtcgaaatagacgatccgttcgatcccgaccggaccttgcgcggtggatgcattggggtcgatggtgacgggcgcgactgccgtcgagctgccctgctggccgccggcggtgccggagcggtcggtcaccggggcgtcgttgagcttggtgcccgacgagcaaccggcaatcagagccacgatggccagcgaataaatcgtacgtttcaacattgggtactcctcaaataaaccttgatcattgcttttgaaacggaccccagtccggttctcttatgtctcccgcctgcccggcgagccgcgcttttatttttccgtccagcgtggtcgtcatgagcgcttcgcggccttgcagctgcgttgcgtagacgatcagcttgctgttgggggcgaaactgggactctcgtctgccgaggtgtcggtgatggccgagacgttgccggtggccaactccatcacatggagtttgaacgcaccgcccacgcgagagatgtaggccaaccaccggccatcgccgctgacagatggagaaatgttgtaggtgccactgaaggtaacacgggtcggcgcgccgccgctggcgcccatcttgtagatctgcggagccccgccgcggtcgctcacgaagtagatcgtgccgccgtcggccgagtacacgggttcggtgtcgatgctggcgctctgggtcaggcggcgtggctcgccgccgcctgccggaatggtgtacagctgcgaaccgccgtcgcggctcagcgtgacggccagcgagccgccatcgggcgcccacgccggggcgctgttggagccgcggaagttcgcgagcaaccggcgctgtccgctggccacgttgtgcacgtacaccacgggcttgcgcgattcgaaggacacgtaagccagctgctggccgttggaagaccagaccggcgagatgatgggttccgggctcgcgagcgcggcctgcgagttctcgccgtcggcgtccgccacccacagcgaataccggctgccgcccttggtgacgtaggcgatgcgcgtcgagaagatgcccttgtcgccggtcagcttctcgtagacgtagtcggcaatgcggtgcgatgcgaggcgcaggtcgccttgcggaacggtgtagctctggccgccgaggtcttgtccgcgcaccacgtcccagaggcgaaagcgcacgtcgaagcggccgtcggccaagcgcgtgacgctgccgaccacgagcgaatccgccgtgcgctggcgccagagcgaaagatcagggcgcgaggcttcgtcgagcgcctggccagaggcatcgacgccgcggaactggccgctgcgttcgaggtcggcctgcacgatctcggagatcttctgcggcgatgcgtcttgccccttgaacggaaccagcgcgatgggccgttgcgtcagtccgacgcccgacacctcgacccggaactgggcgagcgcgggcagcatgggagttgcagcaagagccgcaatcagtgcgcggcgtgcaaaaagcgatgaagaaggagttggaatggaaacgggcaacggcttgatcatgcggttcggagatgtttcggggtaaaaagttctccccaagtgcgacgggccacatgttacacactggtttggccgcgcaatcacaaaaggtgtatcggtcggtgccgtcctacagcgcggccttcaaggcgcctgccggggcccccgtagaatccgccgccatgcaagcatcccccggcagcgagaccgcgcgccctcccctgttgcgccgactggcgcgactcatgacctggttcggcggctcgcgccactggtgggcggtcgcgctcatcggcgccttgatggcggccatcaccgagccgctgatggccgccctgctgaagccgctgctggaccgcggcttcaaccgcgggcagctggcgctgtggatggtgccggccgccgtgctgctgctgttcgcggtgcgcggcattgcccagttcatttcgcaatatgcactctcgcgcattgccaacgaaggcatgcagcgtctgcgccgcgtgctgttcgagcgcttgctgggcgcggagctggccctgttctcgcggcaatcggccagcgcactctccaacacggtggtgtacgaggtgcaaaccggctccatgctgctggtgcaggccctgctcgggctctcgcgcgacggcttcacgctgattgcgctgcttgcctacctcgtctacctgaactggaagctcacgctcatcgtcgccttcctggtgccgagcatctcgtggatcatgaaggtgttctccaagcgcctttatcgcctgacgcagcagggccagcaggccaccgacgagctggcctacgtggtggaagaaaacgtgctcgcgcaccgcatggtgcggctgcacggggccgaggcggcgcaaggcgagcgcttcgagcagttgagccagcgcctgaaccggctggccgtgaaatcgaccatcgcgcaggcggccaccacgccgctcacgcagatgatggcatcgctcgcgctgtcgatcgtggtgatgatcgcgctgtggcagagcggcgaacagggactgacggtgggcggattcgtcgcctacatcacggccatgctgatgctgatcgcaccgatccgccgcctggcggacatggcagcgccgatcacccgcggccttgcggcgctcgaacgcggcctggtgctcatcgacgacgtggcccccgagccgcagggcagtttccgcatcgagcatgcgcagggtcgcatcgagcttcgcgaggtgaaggtcagctaccgcggcgaggacgaagcccgagcgctcgacggcgtgaacctggccatcgagccgggccaggtggtggccttcgtcggcccctcgggttcgggcaagaccacgctggtcaatctgctgccgcgcttcgtgctgcccagcggcgggcaggtgctgctcgacggccacgacaccagcgaatgggagctcaagagcctgcgcgcgcagttcgccatggtgagccaggacgtggtgatgctcaacgacacgctggccgccaacgtggcgctgggctccgaaatcgatcgcgcgcgggtgcagcaatgcatagaggccgcgaacctcgcgagccacgtcgagagcctgccggagggcgtcgacacggtgctcggccacaatgccacgcagctttcgggcggccagcgccagcgcctggccatcgcgcgcgctctctacaagaacgcgcccatcctgctgctcgacgaagcaacctcggccctcgacacggaatcggaacggctggtgcaggatgccctgcagcgcctgatgcagaaccgcaccacgctgatcgtcgcgcaccggctctcgaccatccagcatgccgaccgcatcatcgtgatggaacaaggccgcgtcgccgagcaaggcagccacgcgcaattgatggcgcttgacggactctatgcccgcctgcagacgctggccgtgcgcagcgcgaccccgggccaggacccgacgctctgagggctcagagcagcacgatgtcgtactggccttgcccgatggccggctcggactgcaaggagatgggcttgccgatgaaatcgctcagccccgccaggtgctggctttcctcgtcgagaaacagctcgatcacctgcggcgacgacacgatgcggaattcgcgcggcgtgaattgccgcgcctcgcgcaatatctcgcgcatggcgtcgtaggccacgctgcgcgcggtcttcacgatgccctgcccgccgcacgcgacgcagggctcgcacagcatgtgggccagcgattcgcgcgtgcgctttcgtgtcatctcgaccagcccgagctgtgagaagccgccggcggtggtcttgacgcggtcgcgcgcaagctgcttgcgaaactcggccagcacctgttcgcggtggtcgtcgcgccccatgtcgatgaagtcgacgatgatgatgccgcccaggttgcgcaagcgcaattgccgcgcaatggcttgcgccgcttccaggttggtcttgaagatggtgtcgtcgaaattgcgcgcaccgacgaagccgccggtgttcacgtccaccgtggtgagggcctcggtctggtccaccacgaggtagccgcccgacttgagttcgacccggcggcccagcgccttggcgatttcctcatcgaccgaatacaggtcgaagatcggccgctcgcccttgtaatgctgcagcttgccggccgcctgcggcatgtattcgagcccgaacttgagcagcacctcgaactgttcgcgcgaatcgatgcggatggtctgcgtgtcttcactggtcatgtcgcgcagcacgcgctgcagcaggctcaggtcctggtgcagcaacgacatcggcggcatcttgctcgatgcttctcggatgcgcgaccaggtcttgcgcagatacgcaatgtcttcggccagctcggcatcggacgagtcttcgccattggtacgcaggatgaagccgcccgtgttggcaggcaccacgccaccgctgtcggccgccgcggccgcctcgatcagcgcgagcatgcgcgtgcgcaacgattcacgctggtccgaaggaatcttctgcgaaacgccgatgtggttgtcctgcggcagaaacaccagcagccggccggcaatgctgatctgcgtcgacagccgcgcccccttggtgccgatggggtccttgatcacctgcaccagcagcgactggccttcgaacacctgcttctcgatgggcacgatcggcccgccgttgcggtggtcgcgctcgggcgccggtgcgctggggcgcgagcccggcgtgaacggcgccacgatgtctgccacgtgcaaaaaggccgtgcgttccaggccgacgtcgatgaaggccgactgcatgcccggcagcacgcgcgacaccttgccaaggtagatgttgccgaccagcccgcgctccaacgtgcgttcgacgtgcagctcttgcacggcgccgtgctcgaccagcgccacacgggtctcctggggggaccagttgatcaggatgtcttgcatgggattggaattctcaggtattgaaaccggcgctgcgaagaagctgcgcggtctcgaacatcgggagtcccatgatgcccgaataggacccgctgatgtgctcgatgaacgcggccgccgcgccctgaatcgcataggcgccagccttgccgatcggctcgccgctttccgcgtagcgcgcgacctgcttcctggtcatggtggcgaagcgcacgcgcgaaacactgagtgccgcatggcggcggcggccatgctgcagcgccacggcggtcagcacgcgatgcgtggcgccggacagcagcgccagcatgcgttcggcatcgcgcgcgtcttcgggcttgccgaggatggtgcggccgagggccaccgtggtgtcggcgcagagcaccggcgcatcggcgagtccgaggcgcttgcgccgcgcaactgcggcatcgagcttgagcgcggtgacgcgctgtacgtaggcggtgggcgattcgttggccagcaccgcctcgagcgattcggcatcttcttcagggccggcaaggagaagctcgtggcgaatgccgaattggccgagcaactgggcgcggcgcgggctttgcgacgcaaggtagatgaagtcggccaagttcaaggctccgtgaggttccagaccaatccatgcggcaagcgctcgggtccgaacaggaaatgaaggacgcgccggcgggcaggaacccgggcgcgcgaagaagcgtgcagcagcaacggccgcatggcgagggcatcgccccgcgcggcgggacaggtcacctcgccgtgcgcatcgcgcatcgcccgcgccgccggctcgtccagtcggcccgcgcgatggctacccgtcaccacccgcagcgggcctgcgtcgacgccgcaatcgtccaggtgcacacgcacggcgagcagcgactccagcacgcccacgggcggctggacatagtgcgcaccttccttgatggcgatgggcattgccgcatcgggcgggttcaccgatgccggaatcgatgtgtcctggtgcagcgcgaccggccagttcctgtcggccgtcttgtcgaacagggtgcactgcacggctgtggcgttgtcgccgagcaggccgattgcagccaactgcgtctggagttgtaccgccatgtcgcggcaccccggttgcgtcagcagattgcggctgccaaccgcgctttgcagccacggctccagcgactccgcgatttcgttcatgtgcccggccggcagcagcgcaggcaaaagcgcgtagcccgcctcatcgagcaaggcgaccggcccgatcattcccggtggtacggatggcccgcgttgaccgaccaggcccggtacaactgctccacgagcagcacccgcgccatcgcatgcggcagggtcaggtcggagaggcggatgcgttcgtgggctgcggccttgaaggcgggatcgagcccgtcggggccgccgatgacgagggcgacgtcgtcgccctcgccctgccaggcctgcaggcgcgaggccagcgccttggtggtgagcgaggtgccgcgctcatccagcgccacgatgcgcatgcccctggcaatggcgccttcgatgcgctcgcgttcggcagcgtagatggtttcgagcgacttggaaccgcggggttcggtcttcacggcccgcagctcgagcttgagctcgggcgggaagcgcttggcgtagtcgtcccaggcagtctgagcccagtcgggcatgcgctgcccgacggcgaccaccaggagcttcatgcgcggcgggctggcgccttcttggcaggcgccttctttgccgcgggcttctttgccgcgggtttcttcgcggccggcttgccgaccaccttgaccggcacgcgcgcggtcgtggtcttctttgccggcgccttcctggcggcggttttctttgccgggctgcggctggctttctcggccttggcttcctgctcggccgcgcggatggcggtcttggccgcgctggtacggcgcaggttgggcatcttggccgcaaccggcttcttctcgtcgatcaccttggcggcggttgcaagggccggtttggtgccgccgagcttggcgcgcacgggcttgtcgccccagatctcttcgaggtggtagtactggcggatggccggctgcatgatgtgcgcaacagccgcgccgcagtccacgatgatccactcgccgttgtcctcgccctcgatgcgcggcttgccgaagccggcctcgcgcaccgcatcgcgaacgctggcggccagcgccttggtctgccggttggaggtgcccgaggcaacgatcacgcgttcgaacagcggtgaaagatgctcggtatcgaaaacctggatgtcctgcgccttgacgtcttcgagtccatcgatgatggctcgctggagtttttgggtgtctttcttggcggcggcttcagtggtcatcaggcagagcggtaaaggtggtgtcggtcaatatagcgtgcaacggctggcggaaccagcgaggaaatgttctcgccaagcgccgcgcgccgccgtatatcggtggcgctggtgtccatggccggcagttcgagcgcttcgaaacgcgcgccagccggaaggccgggcagcatcttcggatcaaaacgagcagtgccgcccgtcgataatgcgcgatacgctacagaaacaatagcaatgccgagtatagcctgccagccatgccacttcggcaaggcgctggcttggtcggcccccatgatcaggaccagctgggcgccgggctgctcccgctgcaattcatgcagggtgtcgagcgtgtaggtgggaccgtcgcgcagcacttcgcggctgtcgaccaccaccgttcccttcagccccgagaaagccagccgcgtcattgcgagacggtcttgcgccggcgtcagcgcccggctcttgtgccaggcctgccccgtgggtatgacgtgcagctcggccaggccaagctgcgaaagcgccgcctcggccaatgccacgtgggcgttgtgcggcggatcgaaggcgccgccgaaaatgccgatgcgcgggggcgacttgctggcgggagggttcacaaccagtcgcgccgcacgatgaaatcgctgtagagcgcggcttcggggctgcccggttccggctgctggcggtaggcccagcttgcgagcggcggcatcgacagcagaatcgattcggtgcgcccgcccgattgcagcccgaagtgcgtgccgcggtcccacacgaggttgaactccacgtagcgtccgcgccggtagagctggaacgcccgctcgcgctcgccccagggcatggcgcggcggcgctcgatgatgggcaggtaggccggcaggaaggcattgcccacggagcgcagcattgcaaaggcattctcgaatccgccctcggcgaagtcgtcgaagaagatgccgccgatgccgcgctgctcattgcggtgcttgagaaagaaatactcgtcgcaccaggtcttgaaacgcgggtatttgtcgtcgccgaaggcggcgagcgcatcgcggcacgtggtgtgaaagtgcaccgcgtcttcttcaaaaccgtagcagggcgtcaggtccatgccgccgccgaaccagcacacggggtctttgccttcaggcagcgcagccagcatgcgcacgttcatgtgaacgatgggcacataggggttgcgcggatggaacaccagcgaaacacccatggcctcgaacggcgcgcccgcgagttcgggccggttctgcgtggccgagggcggcagcttcgcaccgcgtacctgcgagaagccacagcccgcgcgctcgaacagttctccgccctcgaggatgcaggtgaggccgctgccctgcagcgcctcgccgggttccttctgccaggcgtctcgcgtgcaggcgccaccatctgccgcttcaaccgccgcgacgatctcctgctgcaacttgcgcaggtagtcgccgaccgccgccggatgggtctgttgcatcaggcgtgcggggtgccgcgcgcgtggaccgcgcggtgcccgatgtccttgcggtattgcacgccgtcgaaattgatgcgcgcggcgacttcgtaggcccgctgctgcgcctgcttcacgctgtcggccagcgcagtcacgcacagcacgcggccgccgctggtcttgagctcgccgtcctgctgcgtggtaccggcgtggaacaccacggcatcgggcgcttctggcggaatgccggtgatgcggtcacccttgcgcggcgaaagcggatagccgtgcgccgccatgaccacgccaagcgccacgcgccggtcccactgcagctcgacctggtcgagcgtgccgtcggtagcgtgccagaacacttcgaacaggtcggacttgagccgcatcatgatcggctgcgtttcgggatcgcccatgcggcagttgaattcgagcgtcttcgggtgcccggccgcgtcgatcatgagaccggcgtacaggaagcccgtgtacgggatgccgtctttttccatgccgcggatggtcggcaggatgatttcgcgcatggcgcgcgcatgcacttcggccgtgacgaccggtgcgggcgaatacgcgcccatgccgcccgtgttcggcccttcgtcgttgtcgagcaggcgcttgtggtcctggctggtggccagcgcggtcacgttcctgccatcgcacagcacgatgaagctggcttcctcgccctgcaggaattcctcgatcacgacgcgcgcgccgccatcgttgtgcgacacgccgaacttgttgtcgaccagcatgaaatcgaccgcctcgtgcgcctcttgcgcggtcatggccaccaccacgcccttgccggcggccaggccgtcggccttgacgacgatgggagcgcccttggcgtcgatgtaggcatgggccgcggccgcatcggtgaaggcctcgtactcggccgtcggaatcttgtggcgcttcatgaacgccttggagaacgccttggagctctcgagctgcgcggccgcccgcgtggggccgaagatgcgcaagccgtgggcgcggaattcatccaccacgccggccgccaggggcgcctcgggcccgacgacggtgagcgagatcttttccttggcggcccattcgcgcagcgcggcgggctcgctgatgtcgatgcagtcgtagcgctcgtcgctcacggtgccgccgttgcccggcgccacgtacacgcggctgacccggccggcctgcgccagccgccacgccaatgcgtgttcccggccccctcccccaattaccagtaccttcattcgtgggccttcttcattcgctgtggatcaatagtcattcattcggaaagcgcggcgttgtgatagacctcttggacatcgtccaggtcttcgagcacatcgagcagcttctgcatcctggcggcgtcttcgccggtcagttcgatcgtgttttcggcccgcatggtgacttcggccacctcgggcttgaggccggcggcctcgagtgcgttcttgacggtttcgaaatcggcgacggccgtgatcacctcgatggcgccgtcgtcatcggtgacgacgtcctcggcgccggcttcgagcgcggcttccatgaccttgtcttcatcggtgccgggcgcgaagatgatttggccgcagtgcttgaactggaaggccaccgagttttccgttcccatgttgccgccgtgcttggagaaggcgtggcgtacttcggccacggtgcgcacgcggttgtcggtcatggtgtcgacgatgatcgccgcgccgccgattccgtacccttcgtaacgaatttcttcgtaattgacgccttcgaggttgcccgtggccttgtcgatgttgcgcttgacggtgtcgatcggcaggttgaccgccttggctttttcgaccgccagccgcagccggggattggcgctcaggtcacccccgccggcgcgcgcggccaccgtgatttcgcgaatggcgcgcgtccagagcttgccgcgcttctcgtcctggcggcccttccggtgctgaatgtttgcccatttgctatgtccggccatggctttctatctcgcagtcttgtgttttcaaagcaggctccgagtttactgtccggcgcacacaacggctcgcgagtcggcgccgaggcggcgctcccttttggtgataatcccccgatgacgccatcgccttccgtcgggcccgggaatccgaccaccctgccgccgcacacccccttgccgctgtactacaagaacgaggcagagcaccaggcgttcctgcgtcgcatcttcgacagcaccgccgccgactacgaccgcatcgagagcgtgctcgccttcggcaccggtccgtcctaccggcgggccgcgctgtcgcaggccgggcttgcccagggcgcgcaggtgctcgacgtcggcatcggcaccgggctggtcgcccgcgaggcgctcaagatcatcggcccgaccggcaaattgacaggtgtcgatcccagcgtgggcatgatggaacagatcgacctgccgggcgtggagctggttcccggcgtggccgaggcgctgccccggcccgacgccagctgcgacttcgtgagcatgggctatgccatgcgccacatcagcgacgtagcggccgccttcggcgagttccaccgcgtgctgcgccccggcggacgcctggtggtgctcgagatcaccaagccgaacggccgcatcgccaccgcgctgctcaagggctacatgcgcgcggtggtgccgctcatcgcccgcgtggtcgggcgccgttccaatacctcggagctgtggcgctattactgggacaccatcgaggcctgcatcccgcccgaacgcgtgctggaggcgctgcgcgccgccggtttcaccgacgtgcgccggcacgccagcctgggtgtcttctccgagtacatggcccgcaaaccggaaaccgctgtcgaggccggctgaccgtgcaagtccagggcgaaacctcacatctgcgcgtcgagcgcctttcactgcccgcctgcctcgcgctggccgcgaacggcgccgcgccttttgcggcgctcggctacggcacgccgcacgagctggcgtggatgccgacagtcaacgcgcgcgttctttcggcgcagggtgccatggccgacgtatggcacgtgaccggcgcgcacgtcgagtcgggcaccaccggcatcgcccgctggcgcaccgatggccattggctgctcggcgccatcgatatcgacgaatccacggaagaacagaacctcgccgaaatcgcccaccgcgcctatcgcgacctgttcaagacgctggaccaggccgccacaccgcacctgcttcgcatctggaactacctgccgcagatcaatgccgacggcggcgggctggagcgctaccgccagttcaacctcgggcgccaggaagcctttttcgaggccggccgcgccgccttcgagggcgccccggcggcttgcgcgctgggcatccaccagggtgcgttgtcgatccgcttcctggccggccggaccgcgccattgccggtcgaaaacccgcgccaggtctcggcctaccgctacccggaaacctacgggcctcgctcgcccaccttctcgcgcgccgcgctggccgacatcggcaatggcgaggtggcgctgttcatctcgggcaccgcgagcatcgtgggccacgaaaccgttcatcacggcgacgtgctggagcaaacccgcgaaacgctgcgcaatctcgaagccgtgatcacggccgccaacgggcaggtgacccacgtctcgggagcgttttcgctcgccacgctcgactgcgtggtctacgtgcggcatccggcggacaccgacaaggtgcgcggcgtgatcgagagcgcgctcggcgccggcgcgccgatgatccgccatgccgtctacctggaagcggacatctgccgcagcgacctgctggtcgagatcgaagcccatgcggtcgctccgggtcgcctgcgggcctgacccgctgcgatcgatcggaccgacgaccccatgtcgatgactcgcgtgctgcgcattctcacggccattcccctcgcgttgatgctctacgcgctgctgcttttcctcggactcatttcgctggcctggaatttcgtcgccatgctgctttatccggtgatgccggaggcgccggcccgcacgctggggcggctgaccatcgcctttgcgtaccgcatgttctggggcctggcctccgtgaccgggatgatgcgcatcgacgccagctgcctggacccgatgcgcaacgagcccggcgtgatcttcgtcgccaaccatcccacgatgctcgacgccctgctgctggtggcgcggctgccgcgcagcgcctgcatcatgaaggccgacctgctgcacaacatcttccttggcgcgggtgcgcggctcgcgcgctacatcagcaacgaatccgcgcgcaccatggtgcggctggccgtggccgacctgcgcaacggcggccagctggtgatctttcccgaaggcacgcgcacggtcacaccgccggtcaaccccttcggccacggcgtgacgctgatcgccaagctcgcgcacgcgccgatccagacagttttcatcgagaccgactcgccctatctcagcaagggctggccgctgtggcgcgtgccgccgctgcccatcgtcttcaagctgcggctgggcgagcggttcgcaccgcttccggacagccacgtgctgcaagcggagctggaacaatactttcgccaaaacatggaacagcgcgccaccgacgcgtcccccgcatgccagacgcctcgcgcacacaccttgtcctgatccccagctacaacacgggcgaacgcctgttctcgacggtcgaagcggcgcgcgcgcagtggaatccggtctgggtggtggtggacggcagcaccgacggcacgggcgagcgcctgcagcaaatggccgccagcgacccgggtctgcgggtgtggctgctgccgcagaaccagggcaagggcgcggccgtgctgcacggccttggcgaagcgctcaaggccggtttcacgcatgcattgaccatggattccgacggccagcatccagccgatctgattcccgccttcatgcgcgcatcgcaggcccggccggaaaccatggtgctgggccgcccggtgttcgatgcctccgccccgctgctgcgcgtgcgcggtaggcgcgtgtccaacggctggacccagctcgagaccctgtttgccggcgtgggcgattcgctctacggatttcgcgtgtacccggtggccgacctcatcggcgtgatggcgcggcagccatggatgcgccgattcgacttcgacaccgaagccgtcgtgcggctcgcctggcgcggcgtcaagccagtgaacatcgatgcaccggtgaagtacctgacggccgaggaaggcggggtgtcgcactttcgctatgggcgcgacaacgtgctgctgacgtggatgcacacgcggctgatgatcgagttcgtcttgcgcctgccgggcctgctgtggcgcaaggcgcggcgcatgccgccctttcaggcttgatctgaactcggcggctagatcattccgccgttgatcgagatcacctgccccgtgatgtaggccgcctcgtcactcaccagaaaagaagccagcgccgccacttcctgcggcgttccggcacgcttcatcggcaccatctggttgaccatggcggggtcgaacgccgcatcggccatgggcgaggcgatgatgcccggcgcaatggcgttgacggtcacgccgcgcgacgccacttcgagcgagagcgccttggtcgcgctgttgagcgcgcccttggccgcggcatagttgacctgcccgcggttgccggtcagcgccgacaccgaagaaatgttgacgacgcgcccccagcgcgtgcgcatcatcggcagcagcaacggctgcgtcacgcggaagaatccgttgagcgaaatgtcgatgaccttgtgccactgctcggcgcgcatgccgggcagcacggcgtcgtcgtgcacgcccgcgttgttgacgacgatctgcaccggcccgctttcgagcatgcgttcgcacgccacccggcaggcgtcgtcgctgcgcaggtcgaacacgtggcgctcggccttgccgcccgcggccgcgatggcagccgccagttgctccaccgcttcggggcgcgagttggcatgcagcagcaccgtggcgccgtcgcgcgctaggcgctcggccatcgctgcgcccaaggcgccgctggcgccggtgatgagtgcgcgttttccttccagagtcatgggtaaacctcccccctgcgggctgtggtgcgagtcccttcgggcggccgggcgggactcatggcgtggctccggttgcgagcggcgtgttcagcaccaccacggcgcggccttcggccagcacacgcccggcgctgtcgttcaccgcaaattcatagaggatctggttcgtatcgcccgagaggcgcttcgcctgcacctgcagcgcaccggcaacgtcgtcgagccgcgcgaccgacaggcgcacattgcgcgcactcgcaaggaacccggccgacggcgtgcttccctcggcagccagcaggccgccgtgcagcgccatggcctgggctgcgtactcgatggcggtgggcgcgagcaggccgcccgccgtccgcagcggattgtcgggctgcaggtgcgtgcgggtgctgcagtggatggactcggcgtcccagcgttcgagccgctcgagcaggcacatgctgccgctgtgcggaatgcgctcggcaatgccggcacggtcgagcgtctccggggccatggtcacgcggtgggctccaggtcggccaccagcagcacgttggcaaagggcgtgccttcgctcattggaatgctctgcacgcgaaactccagccgctgcagcaccgccacccaatcggccagcgggcggccccaggtgggcgacaccttgtggccgcggatgcgcgtcacggtgcgatcgacccattggctgatggcgaagccgcgcttgctcgacgcgtcgccgatgcgcagcagcagccgggcattcgcattgctgccgcgccgcaatgcgtcgcgcacgcgctgcagcacgccgtcttgcgcctcgatgtcgacatagtgcagcacgtcgagaatcacgaccaggtcgcactcgggcagcggtgccgtgcacatgtcggcgcaaagcagccgtggcgccggctgcagatgcccgatggacgccgcagcgcgcgccacgtccttgggcatcagttcgatgccggtgtagtcggccgccgtcggcgtgggcttccaggacgagggccagcggccgtgcgcctgcatgcggctcatcgacgccagcaagctcgcaaaaagcccctgcccgcagccgatatcgaccacgcggcgatgcgccgagtcgatcagcccgcgttcgagcagcccgcgaaacaccgggtcgcggcccagcttgccgcgcgcgaaatgccaggcgaagctgccgcccttcttgtagggaacggtggcggcttcgtgaagctcgcgccaggcggtgtcggtggaaaaaggcggcacagcgctcatggttcaaggccttccggcaaggtgacggcgcgcagtccgccggcgcgcaaacgttcgagaagcaagggcaacacctccagcaacacgggggttccctcaggagtgcgcgcggcattgccgtcgtgcagaagcaggatgtcgcgcgcctgcagattgcggccgaggcgcgccatgaccttggcggggtcgccttcccgcgtgtcgaagccgcggcgcgtccagctcaccagcgacaggccgagccggtgcagcaccggctccaggaacggattgcgcaacccggccggcgcgcggaaacaggtaggcctttggccggtggtttcggccaggatgtcttgcgcccgcgcaatctcgctggcaaagccgcgggggccgagaaaagaaaaattgtgccgatgccgcgcggtgtggttctggatgctgtggccccgcgccacgatctcgcgcgccaatgccgggtgggcaagcacgcgctcggcaatgcagaagaaggtggcgcgctggccgtgtgcgtccagcaggtcgagcacccggggcgtgacctcggggtccgggccatcgtcgatggtgatcgccacctggccccgggcgccggccgcttcaggcagccgcgtgacgttggggcccagcaggctgctgcgcggcgtgagccccgcgccggtgatcagcgcatggttcagcacgatggcaccgatggcccagggcatggcgcccggcaccagggcgcccgcgccgatggcggccacgtgccaggccgcgctggcgcggatggctgtcggccaaggccaggattcggacggtgcagcagatgcggaagacatggcgcgggattgtcccatcagccgtgcgcggcaggcggcgccaatcgccgcgcgaatgcggccgacagcaaaagcgccagcagtgcacccggcgcaaccacgcggccgatcgatgacagcgccggaatgtccgagatcgcaatcaacccgaaagacaccaccgtggtcaggttggccagcatcagcgaggccagcgtgtcctcgtcggcccgcccggccacgcgcagttggtcgaagaacagcgcgtagttggagcccaccgccacgatcagcaacagccccaccaggtgcaggatgcccagcgggacctgaagcacggccatgccgccgagcgtgagcacgaccgcgaccaccaacggctggcacaccgccagcaggcgccggcccgaacgcaggtagatgccgagcagcaccaccactgccagcgcaccgagcagcacctgcacgaaggcctcgtgcagatagcgctggtagagccccgcgagctcgcggccgacgtcgaccacctgcacttcgggcacgcccgcgagcgccttttcgagcccctccgcacggaagttcgggccgggatgcagaaccaccagcgtcgaccagccgccgcccgggcgctggtacatgagcgtattgaccaccgacccgagcggcccgccggtcaggtcggtgcgccgcaccggtgccagcttgcgcgctgcttcgacgtcggccaagaaaggcccgagccgcgtggccggaagcggcgagccttgcgtggcctcggccagccgggtgcgcagcgcttcgctctcgggcaggctggccagacgcgccgcttgcgtcgccacgctcggcagcacgcgggtgacggcctcgaaaccgccgagctcgcccttgtcgaccagtgtctcgagccgtgccgtggcggcttcggtgttgcgcagcgccgtttcttcatcggcgccgtagaccaccaccagcgtgccgccgtcgccagtgccgatgtcggcacgcagcatttcgtcgagttgctgtgccgacttgggcaccgggctcatcgcaccgaggtcggcgcgccagagatggccgccctgccagaccaccaccaccagcgcggcggcgccaagcccggccaacacccagcgcaggcgcgggaggccgcgcacgagcatgccggcagcctgcgccatgtacctgcgcatgcccatgccggtggcgccatcgggcgcgagcacgggcagcgcgtagcgcgtggccagcgcggcagccacgagccccgcgatggaaaacacacccagctgcgccaggcccggaaatcccgagaacaccagcgccgcgaaaccgcacaccgaggtcagcagcccgagccgcacggtgggccaatgcacctcgcgccagcgggcccagccggtgccggccacggcggcgccgcgggcctggatcaggtaatagatggcgtagtcgaccgtctccccgatcagcgtgctgccgaagcccagcgtcatgccgtgcaccgagccgaacaccacgctcaccgcggcggtccccaccaccacgccggtggccaccggcaggaacgcgatgaccagcgcgcgcggcgaggcgaacgccagcagcagcaggccgcccatcacgatgccgccgacgatggccaggtgaatggcctcggtcttgatcttgtcgcggctcagcacggagaaaacgggcgggccgctcagcagcagcttcggcctgccggcctcggccatgccctgcgttgcggcgtcgaaggccgcctgcacccgcgcaatggccacggcctgcgcatcgagatcgctgcccgccgcgcgcgtggtggcgatcatgagcgcgcgcggcgcggtgcgcgacatccacacgccgttttcgctgcgcggcgcgctggccggcgtcagctccaccgcgatgcgctgcgtttcgccggtcggatcgcggtcgagcaatggcttgatggcattgccggccggcgtgcccagcatcgacagcgtttcgtagatcgcgtcgcgcaggccggcgaccgtgaactgctcgggccgcacgccgggcgagagctggtagcggtgctcgaagacccaggtgccggcttcgctccaatcgccggtatcgccgttctggatcaggtcgaacagctggctttcgcgcatggccttggcgacagcgcgagacaccgcggcacgctgcggcgcgttggcaccgccctcgatgccgagcatcagcgtgcgcgacgccacgccgctttgcagctgctcgatgagcacctgttgccgcacgtcggggctcttgggcagaaaggccgagagatcggcgctgaagtgcgtgcgcgcaatctgcagtgcgccgccgagcaggaccaaggcccataccagcagcaccaccgcccggcgccgccagctcggcgggccttccccggcctcgcgtgccttcacggcgtggtgcgtccggcagcgcccgggcgttcgggcgtgatgctcatcaccgagcggtccccgccgacgaattccatttctaggccaatcacctcgctggcgcgcccgctgatgcggatgcttcgcacctgggcggcaagccggctgtcggccggcagcaggtcgagcgtccagttcgcggccgagccgctcaccgtgctccggaagtaccgctgcaaggtcgtgccgtcgccgctcagggtgccgcgcatggcttcgaccagtccgagcagctcgggcatgctgtcgagcgtcagggtgcggttgcggccgccgcgcgacagcgtgagtgtgttgccttcgaccgccatcgtctcgtcacgcggcgacagggtgcgccgcaccagcttgtcgggggcgctgaagctcagcgtgccgcgcgaatcgagcgggccttcgaggccgtgtacgaagcgctgttcggtgaagcgggcttcgccgctcttctgcttggaaagcagccccatcagctcgggcaggtcgaaagcccaggccggcgcggcgcagcaggccagcgccagcagcaggctcctgcacagccagtcaaaccgaatcttcgagccagaaatcatgaaaattgaaccagttgtacggataggcgcggcacagcgcttccaggcgcgtcacgtaggcttcgaccgccgcgcggatgcggcgttcccgctcggcgggatcgattggccgctcgctgaagtcggccaggaggtcgaattgaacatcgtagcgcgcgccgccgccatagaggccggccatgaagaacaccttgcgccgcagcagcgccgccaggcggaacgggccgtcgttgaagcttgccgggtggccgaggaacggcagcacgatggtgttgccgcgctgttgcgccggctggtcttcgctgcccggcagggtgcggtcggccagcatgccgccgaggccgccgccatcgagccagtcgcgcagcgcgagcatcgaatgcgggcggcccagcgcgatcacgtggggccgcagttcgggcaggctgatggcgttgaggatggccgtgatgcgctgcgcattgtcgggatacatcagcatcgcgagccgaagctcttgcttgtgctcgcttttttgcttgcaggcgcccatcgcctcgaagctgccgacgtgcgcacccagcaaaaaggcgccgcgcccgtccagcgcctcggtttcgagcgcggggttgcctttgacctgcacgtcgaacaggtccatgcgcccgcgcaggaagtacacccggtcgagtaccgtcgaggcaaaggcgtgcagcaggcggtagccgtcgatccagccggcgtgcggaccgatggccctgaacaggtagcgcttgatgtggcggcgcggcgcgggcgcgaacaagagaaagtacaggctgatcggcggcagcagcaggcgcgtgacatggcgcccgcagaccagcgccatcaggcagatgaaccgcagcgccagcatgttgctgcgctcgggcgtgtgcgcccagtcgccgcggtggtccgcctgcgccgcatcgctcacggcgcgcgtctcggcatcggtgtgcttcatcacgcagactcttgcacggcggcccagcggccggtgacagccaccacgccgtcgcagcgcacgtcgaagcgcacgccgcgcgccgcgccgggctcgggttgcagatcgatggagagcatgctccccggccgcacgggcgcgaggaacttggcggacgcaagggtgggatggctgccgagccgcgcgaccagcgcgggcacgcgctgcacggcttccatgacctcggccaatatcagcgcgcccggaagcagcggctggcccggaaagtgcccggcgaacgccggatggtcggcgggcaccgcatgggccagttgcaccggcgtgttgtcgtccgcgagttgtgcgagcgcgaattcgcgcagtgcccgcaccgtgagcttgccggtgccttcgcgcggaaaagccttcacctgcaccacgcggcgcggcacgaacaccggctccagccgctgtcgcagggcggcaatgatttcgccggccgagagcgtgggcgccaccacgaaggccacggggcgcaccacgccgtcggccacttcgtcgggcagccagaacgcgccgtcctccacgccaggaatgctgttgaggtgatagttcaggtgtgcgagcgaactgcgccggcccgccacgtggatcaggtcgttggcgcggccgaacagccggaagcggcgcgcgtcgagcagttcgagcacgtcggccatgggcgtgggttcgggcaggaagtcaccgctgaagataaagcgctcgggaccgtcgccctcgcccggctcggcatgcacgcggatgctgccgaagttctcccagatttcgctctgggtggtgcggcgggtggcgacctgtcccgattcggtgctgccgtagatttcgatcagcacgccgccgagcgcctgctcggcctgggcggcgagttgcggcgacagcggcgcggtggcggaaagaatcaggtcgaccgccggcagttcgatgcccgacagcagcagcgtcttcagatggaagggcgtggtgaccagcgcgcgcggacgcggcaccgattccagggtttttgcgacatcggccggaaagaacggccgcccgctttcgaacgcggcgccgccgagcatggccagcagtgccgacgattccagcccatagctgtgctgcaccggcacggttgccaccagcgtcaggccggcgagcgtcggcagcccgagcaagctggagagccgctccaccgccaccgcaacgtcgccgaccagcgtgtcccaccgcttggcgtgcggctggggcacgccggtggagccggaagtcagcaggctcaccgcgtgcatggcaccgtcgatgagcggtacctccaggccgtcgccgccttcggggctggagcggtcttcgatcagcacacgctgcatgccgggcgtggcgagatcggcatcgtcggtcagcgcaaaaaggctcgatccgccggattcgagcaggcgcgcgagcgtgtcgggccgcgcgtcgggcggtagaaggctcgcatggccgcgcaccagcgcagccgccaggctgacggcaaaggcgtagcggtcgacgcacaggttgacggctttcccctccgccggcagcaccggcgcgaagcgggccacgtcggccagaaactgccgcgtgctgatcggcacgccggcccgccaggccaggggcgcatcgaggccccggttggcgatcagcggcagcaggcgggtgtcggcggtcacgcgggtggcccctctttcatcggccgccggtgccgtggtcgatggtcgatgtgccttgaaaggcgcgcaccgcatcgatgagccgcgtgcgctcgaattcgggatgcagccgatagcgcaccaggtgctcgcccacgaaaagaagcgtcaccgagagcggggtcagcacgttcgcgagcagcgaccaggctgaaaaaggcagggtcaggtacaccacgatggacgacaccaccaccagagcgaaatagacggtccagatgcgggtgagctgcgtggtgtaggccagcatgtggcccttgagcggatgcacgcgctgggcgaactgggtgatcagcggaagccccgggccgcgcagcgaagcaccgaaccagccgcacagcaagccgttgatggcgacgtgctggaacacatagagccggttggtgtcgcccgcttcacccaggaacacgagcgcgaagccagcaatgccgagcagcgttgcggcggcaaagccccagcggccgaacttgctggctgcaaaaccgatggcggcaagccagagcgggccgagcaagaccaccaccgcccacggctctgtggggtggaacagcatcatccagtgagagaggccggcataggccacccccaccagcagcaggagcgccagtcgccatcgtgacatggatcaggaagcgctgcgatgctgggcgacgtgggtcgcgagcgtgcgcagcgactggaagatctgttggttgcgctcgtcgtccgagcgcagctgaaagccgtagcgccgggacacctcgagcgcaacttcgaggatgtcgatcgagtcgaggccgaggccttcgccgtacaacggatcggtcggcacgatgtcttcgggcgcgacttcgaggttgagcgcgttcaccagcaggacggccaattctttttcaatcggcgactgttcaggtgaatcgccaacggcgggaatggggggctgagcagtcgatgacaagaaaacctcctgaaactttttcggttactacctcgggggtcgtggattataggagggaggcttgattagactgcccgcttcgatacgacccggagcccctcatggccgacccccttctgatcgcgcgccacgacaccatcgagtgcgccctgctgcccagcctggccaaccgccacggcctgatcaccggcgccaccggcaccggaaagacggtcaccctgcagaccatggccgagaggctctcgagcattggcgttccggtgttcatggccgacgtgaagggcgacctgaccggcatgagccagaaaggcgccatcggcgaaaagatggcggccacgctgaaggaacgcggcatcgacctgcccgaatcggccgcctgccccgtcaccctgtgggacgtgttcggcgagcagggccacccggtgcgcgccacggtatccgacatgggccccctgctgctgggccgcatgctcgacgtgaacgaaacccaggccggcgtgctgaacctggtgttcaagatcgccgacgacaacggcctgctgctgctcgacctgaaggacctgcgcgccatgctgcagtacgtgggcgagaacgggagccagttcaccaccgaatacggcaacatcagcgccgccagcgtgggcgccatccagcgcggcctgctgcagatcgaaacccagggcggcgacaagttcttcggcgagccgatgctcaacatcgccgacttcatgcagaccgtgggcggcaagggcgtgatcaacatcctggcggccgacaagctcatgaactcgccgcggctctacgccaccttcctgctctggatgctgtcggaactgttcgaacagctgcccgagatcggcgaccccgaccagcccaagctggccttcttcttcgatgaggcccacctgctcttcaacgaagcgcccaaggcgctggtcgaacgcatcgaactcgtggtgcgactggtgcgctccaagggtgtgggcgtctatttcgtgacgcagaacccgctcgacattccggattcggtgctggcccagctcggcaaccgcgtccagcacgcgctgcgcgccttcaccccgcgcgaccagaaggctgtgaaagccacggccaccaccatgcgccagaagccgggcctggacatcgaaaccgccatcaccgagcttgcagtgggcgaggcgctggtgagctttctcgacgccaagggccgcccgagcgtgaccgagcgcgtgtacgtggtgccacccggcagccagatcggccccatcacaccggcgcagcgccaggcggtgatagccggttcgctcgtggccggcgtgtacgagaagacggtggaccgcgaatcggcctacgaaaagctcaagggccgcgccgaaaccgcgcccgatgcaccaccggtcaagccgggcgccaagggcgcggccgaatcgtccgaaggcagcagcatgctgaacgacctgctcttcggcagcaccggcccgcgcggcggcaagcgcgacggcttggtgcagaccatggccaagtcggcggtgcggaccatgggcacctcggtgggcaaggagatcttgcgcggcgtgctgggcggcatcttcggcgccaagaagcgctagccgaggtggaccggcccgctccgggccgggcaaatcggcttaccagcgcagcaggcgcggcccgagcacggcgcccgccagcaccggcagcgcgatgccgctgacgtaccagaccgccaggaagggcgccgtcagttccatgcagtgcagcgcatagacggcggcgcccaccccgcccgccagtccgccggcggccgcaccggccaatgccggccgcgtgggcgccaggcctttcaacgccagcagcgcggccgcaaagacgggcagcgccatcagcccgatgctgagtgcgcaaacgcgccacgactcgcccatgagcaagggcatgcggtcctgcggcggcgcattgaaccaggccatggctgccagcacccacaccacgagcaccggcacggcggtgccgagccaggcgcgccgcacctgcaccccaggccgcgcgaggcgctgcaccatcacgaaggccgccgccgcaatgcacagcggaaacagcaccttgacccagaacatcggccagaacatggcctgcaccagatcgcggcgcaggccgtattcagtgaacaggatgacgaaggacaagggcagcgccgtgaacaatgcaaaggccaggcggcgccccgcggcacggcgcggcgcggccgtggggccggtggccagcatggcgacgagatcgtcggtcttcatgatgccttgcctcccatccttgccgcgagcgccttgagcccgcgatggatgccgaccttcacggccgactcggacatgccggtcaggctggcggtctcggccaccgaaaggccttcgagcttcacgtgcacgatcggcaggcgctggcgctcgggcagcgtctgcagcagaccgcccaggtcgcggcgcgcgtcgctggcatcggtggccgattcggcgaacaccgccaggtcgtcgtccagcgggtcatgcagcgcttcgcgtgcggacttggcgcgcagcagatcgatcatcttgtagcgcgcaatcgcatgcacccaggccgtcaacggctggtcgctttggtaggtgtggcgctggttgtgcatggcgagcaggcattcctggacaaggtcttccacttcatcgggccagccgaacaggcgcttgcccagaaaggcgcgcaagtgcgcgctgagtttttgcaggaactcgcgataagccgctgcgtcgccgtccaggccgcgcaggaacaggctccgcagcgccgcctcggcttcgctcattcgcgtcctgctgtccactgtgtttcgtaccatcggaccggctggttacagccctttcgaaaaaagattccgccggattgtgccgtgccccggcggcggcgccgggatcgatgctcggctaagctcgcccgaacccacggaaggagcgcccatgcaagctgccacctcatgccgtccggtccgcgcacagcgcccgggctggaactgaagccgatgctggccgcgctgacttcgcacccctgggcctatccggcgctggaagtggtgcacatcgtcggcattgcgctgctgttcggcggcctgctggtcttcgaattgcgcgtgctcggcctcggacgcgagctttcggcgccgcaactggcccgcctgacgctgctgccggcactggtgggcttcgggctgtgcgccgccaccggcctcaccatgttctccacgcagccgggcgaactgctggccaacaacgcgttccgggtcaagctggtcctgatcggcctggcgggcgccaacgccatctggtttcacgttcgcggcggccccgccgccactggcaaggtggccaaggcgcaatgcctcatgtcgttggggttttggctcgctgtcatcatctgcgggcgctggattgcctacatctaagcgaaggatctaagccaaggagaacgagatgattcagagaagacgcttgttggttgccggttcgctgggcgtggccctgccggcctgggcgcaccatgggtggagcagcttcgatcaggaccggccgctttacctggaggggcgtgcgaccaaggtcatgtggcgcaatccgcatggcgagctggaactcgagctgcccgagaacccgaccctgccggccgacctgaagcagcgtgcgttgcccagccaaagcgcgaccgtcgatggccccggtctgctggccaaggcgcagctgccgacgcggcgcgaccgcaagtggaccatcgaactggcgccactcacgcgcctgcaggcctgggggctcgacgagatcaagcccggcacccaggtggccgcgctgggtttcaccttcaccggcgaaaaaggcgagccggtgctgcgcgccgaatacgtgttcgtcggcggcaaggcctacggcttgcgctcctcgccggcctgagcggcactccggccgcggcaaatgccgcggccatcggcggctttgaccacgctcgcgccctgcttgccagccgcgcgagtgatcggtacattgcattttttgagggcctccaatgtccgcagatagcacagcgaccccttcggcgaccccggcgactccggcaactcctgtcgtctccccccttcccccgctccacccttcgtcgtcgaccggccacatccggctgacctcgcatgccggaggctttggcgccctgcccatccgatggggcgcggccaccgccaccgagcgcgggcccgtggtgggcaccaccacgaagcgggcgcatcgcaacgtcatcggcacgcacagcggctcctacagcgtgtaccgcgcactggccgtggcggccggcgccctcaagcgcgagcacaaggccgacctgaccaataccgcgcccaccgacgtgatcggcccgtacccgcagtggagcgagccgggccgcatcgtttcgctcgacccctggggcgcattggtggccgatgtgttttccgccgaactggcagcgggctacgacattcgcccgaccatcgcgatcaccaaggcgcacgtgatcctgcccgaggtgatcgaggcgctgcagagcggccgcctcaaggccgacggccactttctcaccgccggcggcgccgccatggtgaccaaggccgccatcgaacccgtgtggtacctgcccgaggtggcgcggcgcttcggctgctccgaaaccgacctgcgccgcacgctcttcgaagagaccggcggcatgtaccccgagctcgtcacgcgctccgacctggaagtgttcctgccgcccatcggcgggcagacgctctacatcttcggcaacccgcgcgacctggccaacccggaggtggagctcaccgcgcgcatccacgacgaatgcaacggctccgacgtgttcggctccgacatctgcacctgccggccctacctcacgcacgctatcgaagagtgcatccagggtgcgcagcgcgggggcgtcggcctcatcgcctattcgcgcaaggaaggccgcgcgctcggcgaggtgaccaagttcctggtctacaacgcccgcaagcgccaggtcggcggcgacacggccgaccagtatttcgcgcgcaccgagtgcgtggccggcgtgcaggacatgcgcttccaggagctgatgcccgacgtcttccactggctcggcatcaagaagatccatcggctcgtgtcgatgagcaacatgaagttcgacgccatcacgggctcgggcatcgagatcggcgagcgcgtgaacattcccgacgaactgattccggccgacgcccgcgtcgagatggacgccaagatggccgccggctatttcacgcccggcccggtgccggacgccgacgaactcaagaaggccaagggccggggattgagcgaatgagcgacaagaaggaaaaaagcagcaactacctgcccgccgacggttcgggcagcctgccgccgggcagcgcgggcgacatcgatccggcgatcgaattcgcgccggacaccgcccaccccgcgggcgccgccaccgtgctgcgcaccacggccgccatccgcgagcgcgccgccgccctgctggcgcgcgcgcgccggggcgagtcgcagtggttccgcatcggcgacgacagtgcgatagacgacgcggcgcgcacggtggccgaggtcacgcgcgagcgctatccctgggacaccattccgtaccacagccgctggcgccacttcgaggccggcggcgtcgaccggttgaagcagctcgaccagctgctcggcaagcgcatcgacgcccggcagcgcgcccgcgcgcacatcgacctcgtgctggtgagcgtgctgctcgatgccggcgcggggcccgactggcactacaccgagccagcctcgagcgggcgcttcacgcgctccgaagggctggccgtcgcgagcttccatgccttcaccagcggcctgttctcgtccaaccccgaccatccgctgcaggtggatgcggccgggctgcgcggtctcgtgaccgaccggctcggcgacgccttccaggtcagcgacgtcaatccgctggtcggcctggccggccgcgcggtgctgctgcgccggctcggtgaagccatgagcgaacaacccgagactttcggcgacgacggccggcccgccggcatgttcgatgcgctggtcgcgccgcttggcgctgccgcgccgcccacagcggagatcacggcgcaccagatcctgtcgctgctgctcgagacgctgtcgggcatctggccctccgccaatgccatcgacagcatcgcggccgatggcagcgacgccacgggtggcgtcggctggagcgacccggccctcgcgctcggcgactgctggcgccacagcgcggtgcgcgggcccggcctcaccaacggctggatgccgttccacaagctgtcgcaatggctcacctattcgctgctcgaacctttcgaatgggcgggcgtgaaggtgcgccatctcgatgcgctcaccgccctgcccgaataccgcaacggtggcctcctgctcgacagcggcgtgatcgtgccgaaagacccggcctttctttcgcgcacctggaaggcaggcgacgagttcatcgtcgagtggcgcgcgctcaccgtggcgctgctcgacgagctggcgccgcacgtgcgcaagatgctcgaccgaacagagcaggaactgccgctggcctgcgtgctcgagggcggcacctgggccgccggccgcgtcttggcacagcgcttgcgtgacggagcgccaccgctcctgatcgaaagcgacggcaccgtcttttagactcccggcttcagcaacggtagaaaaaatccaatgagcaacgtccacctcgtcgaccatcccctcgtccagcacaagctcacgctgatgcgccgcaaggacgcctccaccaacagctttcgccggctcctgaacgaaatcagcatgctcatggcctacgaggtcacgcgcgacatgccgatgcaggacatcgaagtcgagaccccgctcgaaaccatgcaggccaaggtcatcgacggcaagaagctggtgctggtgtccatcctgcgcgcgggcaccggcatcctcgacggcatgctgaccgtggtgccgggcgcgcgcgtcggccacatcggcctgtaccgcgaccccaagacgctcacggccgtcgagtactacttcaagatgcccggcgaaatggagaaccgcgacgtgatcgtggtcgacccgatgctggccaccggcaactcggccgtggccgcggtcgagcgcctgaaggagctcaaccccaagtcgatcaagttcgtctgcctgctcacctgccccgaaggcatcgcgaccatgcagaaggcgcaccccgacgtgccgatctacaccgccgcgatcgaccgcgagctgaacagccacgggtacatccttcccggattgggcgacgccggcgaccgcatcttcggcacgaaatgaacccacccccgtccctcgctcacttcgtgtagctcgactcccccctcaagggggcaacaccagcggcccggcaaagccggttccgcggtgtttctggaagaggcacggggagcgccgtcgagaatttttaaaccgaggagaagcaccgtgacagcacgccgtcagttgatcattcgttcggtcgccatcgcagccgcagcgcttgcggcgggcacgcccggccttgcgctggcacaggccaagctcaaggtggcggcggtgtacaccgtgcccttcgagcagcaatgggtgggccgcatccacaaggcgctcaaggcggccgaggcgcgcggcgagatcgaatacaaggccaccgagaacgtcagcaatgccgactacgagcgcgtgatgcgcgagtacgccacgggcggcaaccagctgatcttcggcgaagtgttcggcgtggaagcagcggcgcgcaaggtcgcgaaagactttccgaaagtggccttcctgatgggctcgtcgctcaagccgcaggcgcccaacttcagcgtgttcgacaactacatccaggagccggcgtatctctccggcatgattgcgggcggcatgaccaagagcaaccgcatcggcatggtcggcggcttccccattcctgaagtgaaccggctcatgaatgccttcatggccggcgcgaaggaaaccaatcccaaggtcgaattcagcgtgagcttcatcaacagctggttcgacccgcccaaggccaaggaagcggccttcgcgatgatcgacaagggcgccgacgtgatgtatgccgaacgcttcggcgtctccgatgcggccaaggaaaaaggcaagctcgcgatcggcaacgtgatcgacacgcaggcccagtaccccgacacggtggtggcctcggccctgtggaacttcgaaccctcggccgaccgcgcgatcaagctcgtgaaggaaggcaagttcacggccgaggactacggcgtctactcgaccatgaagcacaagggctcggagctcgcgccgctcggcactttcgagaagaaggtgcccgccgacatcgtcgccaaggtgaaggcgaagcaggccgacatcctggccggcaagttcacagtgaaggtcgacgactcccaacccaagtccaccgcaaaatgaaggggccgacgacgatgcgctggcgctcttttctcgcggccggcgtgttggccctcggcctcgcgggttgcgccggcgtctacaacaagaccggcggtgccggcaccggcggcacccgcctggacgacacgccgcgcatcgccgtgatctcggctttccagcccgagctcacgctgctgctgaaccgcctgcagggagcggcgaagcacagcgtcaacggtgtcgagttcaccaccggcacgctcgagggcaagccggtcgtgctgttcctctcgggcatcagcatgaccaacgcgacgatgaacacgcaggtggtgctcgaccgctttcgcatcaccagcatcgtcttcagcggcatcgcgggcggcgtgaatccgcagctgcacgtgggcgacgtcacggtgccggcccagtggggccagtacctcgaagtgctgatggcgcgcgaaaccgcgccgggcaaatacgccgcgccgcccttcatcaaggatgccacgctgcccaacttcggcatgatgcatccgcgaccggtcgaggtgcgctcggcggcgcatccgcagatcgtgcgcaagttctggttcgaggccgatccgaagatgctcgaggtggcgcgcagcatccgcaatgtcgacctggcgaattgcagcgccggcaagtgcctggcgcgcaagccccagctggtggtgggcggcaacggcgtctccggccaggccttcatggacaacaaggcgtatcgcgaatacaccttcaagaccttccaggccaacgtgctcgacatggagaccgcggccgtgggcatggtggcctacagcaacggcgtgccctacatcgccttccgctctctcagcgaccttgcgggcggcggagacggcgagaacgagatgggcaccttcatgggcattgcggccgacaactcggccaaggtcatgctggcgttcctggccgcatggaagtgacggtggcgcccgtgcgcctcgtgctgctgccgggcatggacggaaccggcgatctcttcgagccgctgaagaaggccatggggccgcatgccgcgatcgacgtcgtgcgctacccgggccggcgggtgctgggctatgacgagctggagccgctggtccgtgcgcagcttcccctgcaagagcccttcgtgctgctcggcgaatccttttccggcccgctggcgatctccatcgcggcctctcgtcccgctggcttgcgcgggctgatcctatgctgcagctttgcgcgcaggcctacgcccgcaatggcgatgctgcgtgcaggactgctcgagctggcgatgggcctgctgcattcaaaggccatgcggctgccgatgcgccacctgctgctgggcggcaacgcgcccgcggagctggcgagccagctgcaggatgcgctggcgcaggtgtcggccgctgtcatgatccgccgcatgcaagaggtgcagcgcgtggacgtgctcgacaagctctcgctggtgcaggtgccggcgatgtacttgcaagccctccaagatcgcatggtgccagggcacgcggcggcactcatccgcaagcgcttgccgtcgctgcgcgtcatcaagctcgacgggccgcacggcctgctgcaggcatcgagcgccgcgtccgcacgggccatccaggacttctgccgcggcctgcggcccgtttccccatgacgcccgccaccgtgctgcgccttcgtggcatcaccaagcgcttcggctcgctcgtcgccaacgacgccatctccctcgacctgcaggcaggcgaagtgctcgcactgctgggcgaaaacggcgcgggcaagtcgaccttgatgtcgatcctgttcggccactacgtcgccgacgaaggcagcatcgaggtcttcggcgcgcccttgccgccgggcaaccccaaggcggcactggccgcgggcgtgggcatggtgcaccagcacttcacgctggccgacaacttgagcgtgctcgacaacgtgatgatgggcaccgagccgctgtggcgcctggtctcgcgccgtgcggccgcgcgtgcccggctgctcgacgtggcgcagcgttttggcctgcccgtgcagcccgacgcgatgatcggcaacctctcggtcggcgagcggcagcgcgtcgaaatactgaaggcgctgtaccgcggcgcacgcatcctgatcctcgacgagccgaccgccgtgctgacgccgcaggagagcgaagcgctatttgccacgctcgcgcagatggtggcgcagggcctgtcggtgatcttcatcagccacaagctcggcgaggtgctgcgcgtgtcgcaccgcattgccgtgttgcgcggcggcaagctcgtggccgaggcgcgcacggccgagaccacgcaggctcagttggcgctctggatggttgggcatgcggtcgacgccccgcagcgccggccggccaggtcggtgggcgatgccgtctgcgtgctcgaccacgtgagcactgcatcggccaaggacggcgggcaggaccattcgagcgcccttcgcgaggtgtcgctgacgctgcgcgcaggcgagatcaccgccatcgcgggcgtttcgggcaacggccaggtggcactggccgagctgctgtgcggcacgcgccgcgccacttcgggcaccgcccagctgatgggccgcgcgctaccgccctcgcctgcccggctggttcagcgcggcgtcgcgcgcattcccgaagaccgccatgccgtcggcgtggtcggtgacctgccggtgtgggagaacgcggtgtcggagcggctgcgtagcccggtgttctcgcgctggtcgtggttcgtgcggcgcacggtcgcgcggcttcatgcccggcgcatcgaaaaagcattcgacgtgcgcggcgccggcctgatggcaccggcccgttcgctctccggcgggaacatgcagaagctgatcctggggcgggcgctgctggcgcccgagcaggcagaagatggcgacaacaagaaatacccgacacgcgcaccgcgcctgatcgtcgcgcaccagcccacgtggggcctcgacatcggcgccgtggcctatgtgcagcagcaactcatcgccgcgcgcgatgcgggcgcggcggtgctggtgatttccgacgacctcgacgaagtgctcgcgctcggcgaccgcgtggccgtgatgcatggcggccaattgggcgaagcgcgcccggccgccgcctggacgcgcgaagccatcgggttggcgatggccggtgcgacagcaccgcagcagcagtcgcgcgcgggaaccttgccatgatgcggctcgaacggcgccacgaaacctcgcgcgccgcgctgatgctggcgcccatcggcgcggtcgcgttcaccatggtggtgagcgcgctgctcgtgctctgggccggcgcgccggtcggccgcacctatgcgctgcttttgcagggcggcttcggctcggtgtttgcatggagcgaaacgctgacgcgtgcggtaccgttgatcctcaccgggctggccgcgacggtcgccttcaaggcgcggcttttcaacatcggcgccgaggggcagctgttcgccggcgcccttgccgccgtggccgtgggcggcatgcacggcggcaccggcttcgagctcgcgccctggctgctgttcccgctgatgatgctggctgcggctctcgctggcgccctgctgctgctgggcccggcactcatgaagaacaagctcggcgtcgacgaggtggtgaccacgctgttgatcaacttcatcgtgctgctgggcgtctcggccctgctcgacgggccgatgaaagacccgaccgccatgggctggccgcagagcgtgtcgctgcagcccgatctggagcttggcaagctcatcgcccagacccgcgtgcacaccgggctcctctgggctgtgtcgctggcggtgacggtgtgggcgatcttcaagtacacggtgctgggtttcgacattcgcgccatgggcgccaatgcgcgcgccgcggcctttgcgggcgtgccggtcacgcgcacggtggtgttggtggcgctgctctcgggcgcgctggccgggctcgcgggtgccatcgaagtggcaggccgcacgagttacgtcacgctcgacatgtcgcctggctatggctacacaggcatcgtgatcgcgatgctcgcaggcctgcatccgctgggcgtgatcgccgcgggcgtgttcgtggcgggcgtgctggtcggcgccgacaccatgagccgcgccgtgggcgtgccgacctacatcgccgacgtgatcgtggcggcctcgctgatcgcggtgctggtggcgaccttgctgacgcaataccgggtgcggatgaaatgactccgctctcctcgtcggtcttgctccttcccccgctgggggaacgctgggatgggggcgtcagcgtccatatcgagtgccgcctgcccccaccccaaccctcccccgggaggggagggagaaatacgcgatgaccgatctgctcgacatcctcgccaacccggccttctgggttgccgttctgcgcatcgccacgccgctcatcctcggcacgctcggcgtgctgctgtgcgagcgcgcgggcgtgctcaacctgggcatcgaggggatcatggtggcgggcgccttcacgggctggctcgcggtgtatgccggcgcgtcgctgtgggtcggcgtcggcgtggccgcgctcacgggcatggtgttcggcctgctgcatgcctttctcaccgtgggccttgcgctgtcgcagcatgtgtcggggctgggcatcacgctgctggccaccgcgctcagctacttcggctaccgcgtgagttttccgaaggtgaacacgccaccgaccatcgcgcccttcgcgccgatggagtggctgccggtgccgatcttgaacgcgcagacgtcgctcaccctgttcgcgctgctgctggtgccggccatcgcctgggtgctctaccgcacgccgctcggcttggcgctgcgcatggtcggcgagaacccgcaggcggccgagagccagggcgtatcggtcgcggccacgcgcaccggcgccatcgtggcgggctcggcgctgatgggcgtggcgggctcgttcctcacgctctccgccttcaatgccttcttcttcaacatggtgaacggccgaggctggatctgcgtggcgctggtggtgttcgcctcgtggcggccaggcaaggccctgctcggcgcgctgctgttcgcgtttttcgacgcgctgcagctgcggctgcaacaatcgggcgatgcggtgctgccctaccagatctacctgatgctgccctatctgctgtcgatcctcgcgctggtgctggtggcacgcaaggccagctatccgcaggcgctgatgaagccgtatcgcaagggagaacgctgatgccgaagccggccgcggcacgtggaacgctgctcatggcgctgctggcggtgtgcagcgtgggcgtgcacgcgctgggcagcgaccagccctacgagcgcttcaagacccccgacgcggtcaactgggtgcagctgtgcggcatctggggcaaggatcacaagggcacctaccgcgtgatccatgcggaccaggacgcgcagtccttcctctacgtgcaatggatgcgccgcgacgccaatggcagcctgcatgccgagcacacgaccgccatcgccgaactcgacaacgaccatgccgagatcgcgctcagcgacctgacctgccgcgccacgccgcgcggcatcgtgctgacggcgcgggccgcctccgggcacgacgacaagctgcgccgcgtgaccatcgaggtcgggccggcggcgggccaataccgctatcgcgcgcagcgcacgcgctgaacaaccgccacccacagccacaagatccgacgccgatgctcgacctcctcatcaccaacgccaccctccccgacggccgcaccggcatgtcgattgccgtgcaggccggccgcatcgcggaagtcacggccggcctcgacgcaccggcgcacgagaggctcgatgcggagggcctactgctcgcaccgcatttcgtcgatccgcactttcacatggacgccacgctgagctatggcctgccgcgcgtcaaccagagcggcacgctgctcgagggcattgcgctgtggggcgagctcaagccgctgctcacggccgacgcgctgatcgagcgcgcgctggcgtactgcgactgggcggtggccaaggggctgctggccattcgatcgcatgtggacacgagcgaccccagcttgctcgcggtcgatgcgctgctcgaggtccagcgccaggtcgcgccttacatcgacctgcaactggtcgcctttccgcaggacggcgtgctgcgctcgccgggcggggtcgacaacctgaagcgcgcgctcgacaagggcgtggacgtcgtcggaggcattccgcatttcgaacgcaccatggccgacggtgccgccagcgtgaagctgctgatggagcttgcggccgagcgcggcaagctggtcgacatgcactgcgacgaatcggacgatccgctctcgcgccatatcgaaacgctggccttcgaggctcagcgcctgggcatgcagggccgcgtgacgggctcgcactgcacgtcgatgcattcgatggacaactactacgtgagcaagctgctgccgctcattgccgagagcggcgtcggcgtggtgtcgaacccgctcatcaacatcacgctgcagggccgccacgacacctaccccaagcgccgcggcatgacgcgcgtgcccgagctgatggccgccggcgtgaacgtcgccttcggccacgactgcgtgatggacccgtggtacggcatgggctcgggcgacatgctcgaagtggcgcacatgggcctgcacgtggcgcagatgacgagccaggccggcatccgccagtgcttcgaggccgtgaccacgaatgccgcgcgcgtgatgcacctggagggctacggcctggaggccggctgcaacgcgagcttcgtgctgttgcaggcgcgcgatgcggtcgaggcgatccgcctgcgcgccacgcggctcaaggtgttccgcaagggccggttgctggcggaaacgcctgcggccacagccgcgcttcatcttcccggccgtggcggccagacgaactggatgattccgaaggcctgagccttggcgccccacgatccctgctcgccagattcagcggccgagatccaggtcgcaccacatatggaccttggccagcagttcgttgccgaccgcaatggcgagcggctcgacgccgaagacctgaaaaccgcagcgctcgtacagcgcctgcgcggtgcggttgccttcggtcacggtgagttgcaccagccgcagccgttcgacctcgcgggcatgcgccagaaccgcaaacaccagccggcgcccgaaaccggcgcggcgcgctgaagcagccactgtcatgccgaaaagcgtggccttgtggcgtgcgcgctgccgcgtttcgaggctcaagcccgccgcgcccaccagcgcgcccgtgtcgtcgaaagccccatagaccacgctggcttcgctcgtgtcagcgcccagccgttcctcccaccagcgaagcggcaggcccgcgcgctcctccacggtggtagtgaaagcgctcgggtgcgtggcgtacgcgtcgagcatcaaggcgcggtaggccgcggcatcggctgccgccaggcggcgaacggcgttgaggtcgttttcttcagaagcggacacagacggattgcctttcctgcagcacggcctcctggccgaaacgctgcctgtaggtgccgatgatgccggcgatggtggcgtcgtccctggagctgcccggatgcagcagcaccacgagcttcgagggctcgcgcaccacgctgcccgaggcgccgcgccactgccccgcggcatcgatcaccgtgaggcccttcggaaaggcgggcgtcacgaccccatcgaggaacgcagcccactgcgcatcggacacctgtccgccagcggggatggcacggccgaaatacagcgtgtcgcgctcgaaggcttcgaagcccgcggcacaggccctcgagggctcgggcgcaggtggcaatgcgccgcacccggcgaggatggcaaccgttgccacagcgaccgccaggcgcgaacgggtgacgacctggggcacggcgcggctcattggggtgcgtgggtttcaggcctcgggcgcgatggcttcggcgtactcgtagagcgcacccaggatttcctcgccccgctcgtccgcggtttcggacagcgcatcgacctcgctgaacagcatttcgatggtgcgaaccccgccttcgcccttgaagagccgtgcaacgcgcaacgcctcccagcgttcggcctcttccgggctgagcatctcgggccaattgcgcgcacggtagcggaagagaatttcctcgaggcgcccgtcgtcgaacccggtgcggtccttggcaagctcttcgggcgacagcgcgcgcagctggttcaggcgccgccggtcggcgttgccgacgaacccgccgtagaggtcttcatcgacgtcgggcgtggcttccttgggtcgggcgtacacctgcgaccagatggcgctcatgtcgggcaggtcgcgcgcgatggccgcgtgacgcatggccgcgtcgagatcgacgttccagcgctcggccatggccggcgcgagcgtgcgcaggttgccgaccaccatcggcgacttgttcaggtgaatgcccttcaccggcaggcggaccacgccttcgggcaggtcggcggtgcgcgtgaacaggcgcaggcgcaaggtctctacgtcgatgtcgcgcagctcgctggggtcgtgcgccaggtcccaggcgatcagttcgttcttgttggtcggatggctcgcgagcggccacatcacgccgaggcagccgcgctcgacaggaaacatgcccgacacatgcaggaaaggccgggccgtttcacgcatggccggcaagccgagctcgctggcgacgcggtctttcttgtgcaagccgaaggcgaactcgaacagcttgggctgccgatcgcgaatcagccgcgccagcgcgatggtggcgcgcacgtcggacagcgcatcgtgcgccgactcgtgcagcaggccgttggcgcgcgccaggtcttcgagtttgaagctgggcttgccatcttccttcttgggccactcgatgccgtcgggccgcagcgcataggtgaggcgcaccacgtcgagcaggtcccagcgtccgcagtcgttctgccactcgcgcgcgtacgggtcgatgaggttgcgccagaacaggaagcgcgtcacctcgtcgtcgaagcgaatggtgttgtagcccacgccgatggtgccgggctgcgaaaaggccttctcgatctgcgcggcgaaggcgtgctcggggatgccgcgctcgaggcacacctggggcgtgatgccggtgatcaggcaagcctcggggctcggcaggtagtcgggcgccggcttgcaatagatcatcagcggctcgccgatttcgttcagccctgcgtcggtgcggatggctgcaaactgcgaaggccggtcgcggcgcggcacggcgccgaaggtttcgtagtcgtgccagagaaaggtgtggttcattcagagcaagggggaaaacaatcgtgcaatcgcgtcgccgaggcggcgccagaaactctgcggccggtgggcgcgcaccgcgccggagctgtggagatcggtttcgaactgcgcggccagcggacgcgccagctcggggccgtagaccacggcgctcacctcgaagttgagcctgaaactgcggttgtcgaaattcgcggtaccgatcatcgcgcaatggtcgtcgaccaccaaggtcttggagtgcagcatgcgcgccttgtactcccacaccttgacgccggccgcgatcagctcgtcgaaataggagcgcgcggccgcgctcacgatggccgaatcgctgcggcgtggtaccagaaggcgcacgtccacgccgcgcagcgcggcgctggtgagcgccatcagggcgggctcgccgggcacgaagtacggcgtggtgagccaggcgcgttcgctcgccgaatgaatggcctccacgtgcatgcgatggatgggctccagaacgttgtccggaccgctggtcacgatctgcactggaatgttgccggcctccacctgcggcagcatggcgtccatcagggggtccatgttgcgcaggtcttcgccggtggcatagacccagtcttcgagaaaggtcgtctgcagccagcgcaccgcgctgccttcgatccgcaggtgtacgtcgtggtacgcatcgggccgcgtgcgcttgtcttcctcgtcggtgatgttgacgccgccggtgaagccgacgcgcccgtcgcacaccacgatctttcggtgggtgcggtagttggtcaccggccgcaggcggcggccgatgcgcgtgtcgtggaagagcgcgacctgcacgccggcggcatgcagcggcgccatgaacttgcggccgatgcgcttggaaccgagcgcatcgagcaggaggcgcacggccacgccctgccccgcacgctccaccagcaggtcgcgcagcgcggtgccgatcttgtcgggctcgaagatgtagtactcgaggtggatgtggtcgcgcgccccgcgcaccgcatcgaagatggcgtcgaaggtgcgcgcgccgcccgaaagcagttccacgcccgtcgcgctggaaaccggcagtccgcacgcggcggtgccgagccgcgccatctgctgcagcgccggcggcgcgttctgcgccgcgtcccgcagccgcgccagttcggcctgggtgtgggctttggcgcggctgcgcaggcgcttgacccgctgcttgcgcaagcgctgcggcccgaggaagtaatagacgacgaagcccgcaaacggcagcagcgccagcgacaggatccagctcatggtggacaccggcgcgcgcttctgcatcacgatccagaccgacagcacggcgatatagccgctccaggccaaagagaggccggttttccattcctggctgagctcgggaaaaatcaaggtagggcttgcggtacgggtaaattccggccccaagaaaaaaggccggcagcgaatgctaccggccttttcagtgttgccagaaatacagcggcaccggctccgccgggccgcttaccctgcggcagcctcttcggcttcgggcttggacttgccttccttcttcggcagcggctggatgtccagctgcacttcgcccttgtcgtcgatgtcgaccgacaggcggcccccgtcgatcaggcgaccgaacagcagctcgtcggccagcgcacgacggatcgtgtcctggatcaggcgctgcatcgggcgggcgcccatcagcgggtcgaagcccttcttggccaggtgcttgcgcaagccgtcgctgaacgtgacgtcgaccttcttctcggccagctgcgtttcgagctggagcaggaacttgtcgaccacgcgcaggatgatctgctcgtccagcgccttgaagctcacggtcgcgtccaggcggttgcggaactccggcgtgaacaggcgcttgatatcggccatttcatcacccgcctggcgcgggttggtgaagccgatggtcgccttgttcatggtctcggcacccgcattggtggtcatcacgatgatcacgttgcggaagtcggccttgcgtccgttgttgtccgtcagggtgccgtggtccatgacctgcagcagcacgttgaagatgtccgggtgcgccttctcgatttcgtcgagcagcagcaccgcgtgcggcttcttcgtgatggcttcggtcaggagaccgccctggtcgaacccgacgtagcccggaggcgcgccgatcaaccggctcaccgcatggcgctccatgtattcggacatgtcgaagcggatcagctcgatgcccatgatgtaggcgagctgcttggccgcttcggtcttgccgacgccggtggggccgctgaacaggaacgagccgatcggcttgtcttcgcggccgaggcccgagcgcgccatcttgaccgcggacgccagcacctcgagtgccttgtcctggccgaacacgacgctcttcaggtcgcgttcgatcgtctgcagcttgccgcggtcgtcgttgctgacgttggccgggggaatgcgtgcgatcttcgcgacgatgtcctcgacctcggtcttgctgatggtcttcttgcgcttgttcgcaggcaggatgcgctgggcggcaccggcctcgtcgatcacgtcgatggccttgtcgggcagatggcggtcgttgatgtacttggcgctcagctcggccgcggcctgcagggcggccaccgcgtacttgacgccgtggtgctcttcgaagcgcgacttcaggcccttcaggatgtcgacggtttcctgcaccgtcggctcgaccacgtcgaccttctggaagcgacgcgacagggccgcatccttctcgaagatgccgcggtactccgtgaaggtggtcgcaccgatgcacttgagctggccgctggaaagcgccggcttgagcaggttcgacgcatcgagcgtgccgcccgacgcggcgcccgcaccgatcagggtgtggatttcgtcgatgaacaggatggcgttcggcttgtccttgagcgacttgagcacgcccttcaggcgctgctcgaaatcgccgcggtacttggtgccggccaggagcgcgcccatgtcgagcgagtagacctgcgcctcggccaggatctcgggcacgtcgctctgcgtgatgcgccatgccaggccttcggcgatggcggtcttgccgacgcctgcctcgcccaccagcagcgggttgttcttgcgccggcggcacaggatctggatgacgcgctcgacctcgtattcgcggccgatcagcggatcgatcttgccgtccttggcgagctggttgaggttttgcgtgaactgctcgagaggcgaagccttctcgttcttctcgccgccgccctcttcgccctcgcccgaagacgattcgctgctgcccttgacggcttcaggcggatcgctcttcttgatgccgtgggcaatgaagttcaccacgtcgaggcgggtcacgccttgctggtggaggtagtacaccgcgtgcgagtccttctcgccgaagatcgcgaccagcacgttggcgccggtgacttccttcttgccgttgccggtggactgcacgtgcatgatggcgcgctggatcacgcgctggaaacccagcgtcggctgggtgtctacatcatcggtacccgccacctggggcgtgttgtccttgatgaagttggtgagcgacgcccgcaggtcgtcgacgttggccgagcaggcgcgcagaacttccgcggcgctcgggttgtccagcaaagcgagcaacagatgctccacggtgatgaactcgtggcgctgctgcctggcctcgacgaaggccatgtgcaagctgacttccagttcctgggcaatcatgtgatttccttttgccttgctgtaaataacttctcagatgggttggagcttgcgcaattcaactggttcacgcaacaggctcgctcacgcactgcaacggatgcccggcctggtgtgccgcctccatcacctgattgactttggtggccgccaggtcgcgagaataaaccccgcaaacaccgcgcccgtcgagatgaatctttaacatgatctgggtcgcggtttcgcgatccttgttgaaatattcttgcagcacgacgatcacgaactccatgggcgtgtagtcgtcgttcagcatgaccacctggtacatctggggaggcgcggttttttgcggccgccgctccataacgaccgaatctccgtcatccccggccggtttctgggccggcggagtgctgggagtctttggaattctcgttgccataaaaaagattctatagagcgtgcaagcaacgtgccggcgcaagaagacttggtggcgcatattcgacaaatcaagggccttgcgccgtgtgcgccagcacgtagggcttaaaaaattcaagcgtccgcgggatgcctcgggaatattgcacggctgcggcttgggagacccgtccgcccggatccggggaattgatgtcctcgtcgatcaagaggtttcggaccccacggcaggccacctccggagcaagctgtaccagcctgtccggactctgtgaacggtcacggaccggcttggtctggcgaggggaaaaccaagaaaaagccctcgagaccggaacgatctcgagggcccatggcttctcggcgcccggagcgccaaacgctattgctcgcgcaattacatgtggtcgatcatgacctggccgaagcccgagcagctcacttgcgtggcgccgtccatcaggcgggcgaagtcataggtgaccttcttgctggcaatcgacttttccatcgagctgatgatcaggtcggctgcttcggtccagcccatatggcgcagcatcatttcggccgagaggatttcggaacccgggttcacatagtccttgccggcgtacttgggagccgtgccgtgggtggcttcgaacatggcgacggtgtcgctcaggttcgcgcccggggcaatgccgatgccgccgacctgggccgccagcgcgtcggacacgtagtcgccgttgaggttgagcgtggcaatgacgctgtattcggcggggcgcagaagaatctgttgcaggaacgcgtcggcgatgctgtccttgacggtgatttccttgccggtctttgggctcttgaacttcatccaggggccgccgtcgatcagctcggcgccgaactccttggctgccagggcgtaggcccagtcgcggaagccaccttcggtgaacttcatgatgttgcccttgtgcacgatggtgacgctgggcttgtcgttgtccacggcgtattgcagcgccttgcgaacgaggcgctccgtgccttccttcgagacgggtttgacgccgatgccggaggtgttggggaagcggatcttcttgacgcccagttcgtcctgcaggaacttgatgagcttcttggccttgtcgctttcggcttcgaattcgatgccggcgtagatgtcttccgagttctcgcggaagatgaccatgttggtcttgtgcggctcgcgcaccgggcttggcacgccttcgaagtactggatggggcgcaggcagacgtacaggtcgagttcctggcgcagcgcgacgttcagcgaacggatgccgccgcccacgggcgtggtcagcgggcccttgatggaaaccacgtagtcgcgcacggcgtgcagcgtttcttcgggcagccagacatcggggccgtagaccttggtcgacttttcgccggcatagacttccatccagtggatcttcttcttgccgccgtaggcctttgcaaccgctgcgtccaccaccttgagcatcaccggggtaatgtccagacccgtgccgtcgccttcgatgaagggaatgatcggctgatcaggcacattgagcgagttgtcggcgttgaccgtgatcttctggccgtcggcggggactttgatgtgctggtagctggacatgaggggaagtgactccgggaatgacgtaattcgggcgactgtctgcgaattcagacagcgacggggaatcgctgtacagcccgcgaacaaatcgctgtacattttagacgcaacccatcagctggcgtttgtcaacccgcgaggcaacgacctcgttagtggctgaccttctgctcgccgggaggcgtttccaaccaattctcgatagaggaatcatcaatgagcaaaattctcgcagtcatgatcgctggcctgttcgccgctggcgcctacgcccagaaccccaccggcaccacgcctgagcaagggaacgccaccaacagcaagccccaagcacgcgctgaagccaagaaggacgccaagcccgctggcaaggtggctgctcccgctggcgacatcgccaagacccccgaaggcggtgctatcggcaccgacaaggctgcagcatccggcgaaaagcgcgccgaaacgcgcgaccagcgtcgccgcaacaaggacggcagcgtcaagcgcaagtcgacccaaggcggcacgccccagtaagtcggccttggccgtacaagaaagcgctctccggggcgcttttttttcgcctgcgatggcacaactgctgtcaaccagggcaagcggctgatgcgttgaatgttgaccttccgccgggaggtgatccatatcaacaatctcaaaggatgtctcaatgaacaagctgctcgcagccctcgtcgccggtctcttcgctgccggtgcatttgcgcagaccccgcccgctccggcgccggccgcacctgccgtggtccacaaggctgcgccctcgacgaagcacacggtcaagaagcacaaggctcgccaccacgtggccaaggcgcacgtcgccaagaaggtgtaagctgccacgctcaccggcaatgcccgccaatgcccgcatcagcgggcatttttattggccccgcgcccttgaacccgccctgaaagaagccttccgatgtttcagcgttttgttgccgccctgctcctgcttgccgcctccctgatgggcgccgcacaagcccagcagcaaccccagaccgacctgcaacgcaccaagttgtccgttggcctgtacaagatcgatgcgcaagtcgcgcagaccccccagcaacgggaaatcggcctcatgttccgcaaggaaatgccgcaggccgagggcatgatcttcgtcttcgatcagccggccacccagtgcttctggatgcgcaatacgctgctgccgctgacggccgccttcgtggcggacgacggccgcatcgtcaaccttgtcgacatgcagccgatgaccgagaactcgcactgctccgaagagccggttcgcttcgtgctcgaaatgaaccagggctggtttgccaagaagaacatcaagaagggtgccaagctgggaggcgagctgttcgctgcttccaaacgctgagctccgcccgcctgtttggcccacgaaaaagccgacccgcaggtcggctttttcaatgaggaatccggttcaaccgaagttcttggcagcgaagtcccagttggccagcttggccaggaaggtctccacgaacttggggcgcaggttgcggtagtcgatgtagtaggcgtgctcccagacgtccaccgtcagcaccggggtgtcgccggtggtcagcggcgtgcccgcggcacccatgttcacgatgtccagcgaaccgtcggccttcttcaccagccaggtccagcccgagccgaagttgcccacggccgacttcacgaacgcttccttgaaggcgtcgtagctgccccacttggcatcgatggccttggccagcgcgccgccgggagcgccgccgccctggggcttcatgcagttccagaagaaggtgtggttccagatctgggcggcgttgttgtagatgccgccgctggacttcttgacgatttcttccagcgtcatcgactcgaattcggtgcccttttgcaggttgttgaggttcaccacgtaggcgttgtggtgcttgccgtagtggtactcgagggtctccttcgagtactcgggtgccagcgcgtcgagggcgtaaggcaggggtgggagcacatgttccatggtttcttctcgtgggttggttgcggggaattaacgattctagaaaggaatcaggagcccggcgtcggacgcgttcccgttttgccgggcgtcacggtcaggtcgaccgagccgtcggcgagccgtgcgaccacggcatcgcccggattcagttttcttgcactgacgatcgcacgaccgtcggcgccggtgagccaggcatagccgcgctgcagcaccagcgcggggtcgagcagcttgagccgcagcgccacgcgttcgagccgatcgcgccgctctgccagcgcgcgctcgagcttgcgagggaaatcggccgcgatcgaccgcggcgcatgggccaggcgctcggttctcgatagcaccgcatagcgcaggcgctgcgattggtgcgcgagccgaagctgctggcgcgccaccagcgtggagggccgccccaggcgtgacgccgcctggtcgaggcgctggcccagcacgtcgagccgggtgtccagcgcgccttgcaaccgttcgcccagaagatcgatcgcgccgagccacattgcctgcggcgcgctgacgagttccgccgcggcggtgggcgtgggcgcccgcaggtcggcgcaaaaatcggcaatggtgaagtcggtctcatggcccacgccgcaaatcagcggcaccgggctttgaacgatggtgcgggcgagggtttcgtcgttgaaggcccagaggtcttcgatggagccgccgccgcgcaccagcaggatgacatcgaccgcgggcttgagggcatacaaggattgcagcgcgcgcacgagctcccccggcgcgctggcgccctgcaccgccgcgggcgccaggaccaccgggatgtgcggcacgcggcgtcgcagcgcggtcaccacatcgtgcagcgccgcggcgcccagcgaggtcaccaggcccaccgcgcgcggcatgaccggcagcgcccgcttgcgctcggcatcgaagagcccttcggcttcgagccgcgccttgcgttgcaggaactgctcgaacagcgcgccttgtccggcacgttgcaggctttcgaccaccaactgcagatcgccacgcggttcgtacaccgccaggcggccgcgcacctcgacctggtcgccgtcgcgcggagaaaaatcgagcaggccggccgcacgccggaacatcgcgcagcgcagttggccggaatcatccttgagcgcgaagtaacaatgcccgctcgacgcgcgcgaaaaaccggaaatctcgccgcgcaccgcgaccggattgaagcgcgcatccagcgcatcggcgaccgcccggcacagcgcgccgacaggccagatgcgcggacccggtgtggtgttggaatcacgcaatgtcacaactcggccggatagcgggtgaccactcttccacagtgaggcggcaagcccccttgcccggatccgggtgcggaacaagtgcacggtttgtcgtgcaagctcttgatttcattcagaaaactgctgctcaaaattcagtcgatctaatggaaagcccacgccatgcgggtcggggcacgttgcccatcaggttaatcacaaagttatccacagaatctgtgcgtccttgcttacaaacaaacaaggcgcgtggcgatggtgggctcggtggataatcgccgcgcatttgcagtctattcggggccggaggattccttgttttccatcatagttgccgcgggctggccaatctggccattgctcgcttgttcgatcatcgcgctcgcgctggttatagaacgtttcacaagtcttaaaaccgtcaaggtcctgccgcccaagctgctcgatgaagcgatgacggtgtcgcacggttccgtgccggggcccgacgtggtgaccaagctcgagcgcaattcgatgctcgggcaggtgctggccgcgggccttcgcgccctcaacgccaatccgcgctgcaccgaggacgacctgcgtgcagccatggaagcctcgggccgcaccgtggcgcacaagctggagcgctacctgcccgcgctggccaccatcgcctcggctgcgccgctgctcggcctgctggggacggtgatcggcatgatcgagatcttcggctcgcaatcgcccggaagcggcgcggtgggatcggggaacccggcgcaactggcgcacggcatttccatcgcgctgtacaacacggcgtttggcctgatcgtggccattccgaccctgatcttctggcgctatttccgcagccgggtcgatgaatacctgctgaacctcgaactctccggcgagcgctttgcccgccacctgaacgcattgcggaaatgatggccttaacgcttgccactgcgagcgcagcgctgtccagcggaggctcgccatgacccgcggccgcatgcagtttcgccatggcgcccgcgatgagccggagatcaatctgatcccgttcatcgacgtgctgctggtcgtcctcatcttcctgatgctgtcgaccacctacagcaagttcaccgagatgcagttgcgcctgccgacggcggacgtcgactcgcagcgcgactatcccaaggaagtgatcgtggcggtgtccgccgacggtcgctattcgatcaacaagacgcctctgccagaccgcaacgtggcgacggtggccgccgcgctgggtgcggcagccacgggcggcaaggacagcgtggtgatcatcagcgccgacgcgagcagcccgcaccagtccgtgatcacggtgatggaagccgcacgccgcgcgggcctggtgcagatcacgttcgcagcccaatcgacggcccaagcagggcactgagtgccgttgcagggccgcagcactcccggcaacagccgcgcggccagtgcgcccgcttcgcggctgcagcgtgcctggctgcaccgcggtgcgttggcctgcatgctgtggccgctgtcgctgctctatgcggcgctgttcgcgctgcggcgctggctctatcgacaaggttggctgcaaacggaccgcgtgtccgtcccggtgatcgtggtcggcaacgtcattgcgggcggcgccggcaagacgccggtggtgatggccgtggttcggcatctgcaggctcgcggcctgcgcaccggcgtggtgtcgcgcggctacggccgccgcaccgacgactgccgtgaagtggaggacgaaagcgatccgcaagatgttggcgacgagcccgcgctgatccgccgtgccaccggcgcgcccgtgttcgtggcgcggcgccgcgtcgaggccgcgcgcgccctgcttgcccggcacccggccacgcaggtcatcgtgagcgacgacgggctgcagcacctggcgctcgctcgcgacgtcgaaatctgcgtgttcgacgaccgcggcgtgggcaacggctggcggctgcccgcgggccccttgcgcgagcgctggccgcgtccgtgcgacctggtgctccatagcggcgagcacccggcattcgaggacggctacaccgccactcgcgccctggcacaagacgcggttgcgagcgacggaaaacgcacaccgctcgatgccctggccggcaaaccggtgatcgcgcttgcggccattgcgcggcccgaggccttcttcgagatgctgcgcgcgcgcggcctcgccctggcggagacgatcgcgctgcccgaccacttcgacttcgagggctggcaacgcccttccgaccgtgatctccctctggtctgcaccgagaaagatgccgtcaagctctggcggcaagccccggatgcgctggccgtgccattgcacttcgtacccgagccgcaattcttcgcggcgctcgatgcgaagctatcatcgctcgatggatcccaagctgcttgaactgctcgtctgccccgtcaccaagggcccgctgacctggaaccccgaaaagcaggagctctgctcgcgcagcgcacgcctggcctatccggtgcgcgacggcattcccgtgctgctggagaacgaggcgcgcacgctgtccgacgaagagctggggctgtgagcgcggcgccaagggagaaccaatgagcttcaccgtcctggtgccggcacggctggcttcgacgcggctgcccaacaaaccgctggcggacattgccggcctgcccatggtggtgcgcgtcgcccggcgcgcgagccaatccggcgcggcgcgcgtggtggttgccggggacgatccttccatcgtcgcggcctgcacggcacacggcgtgcaggccatcctgacgcggcaggaccatcccagcggcaccgaccggctggccgaagcctgcgagcaactgggcctggacggcgacgatatcgtcgtcaacgtgcagggcgacgaaccactgatcgacccggccctgatcgacgcggtggcctctgagctggcagctcacccggaagccgccatgagcacggcggcccacgagatcgattcgctcgacgactttctgaacccgaacgtggtgaaggccgtgctcgatgcaaagggcaatgcgctctacttcagccgcgcccccattccatggtggcgcgacggctccaccggcggtgcgccaccgggcgtgctcccttcgcctcggccgctgcgccatatcggcatctacggataccgcgccggcttcgtgcgcaagtttccttcgctggcgtccgcccccatcgaggccaccgaagcactcgaacaattgcgcgcgctctggcatgggcatcgcatcgcggtgcatgtcagccaggtggctcccggtccgggcatcgacacgcccgaagaccttgctcgcgtgcgcgcggtctttgcagcccagttggccccctgagttgcatcaatatccgtggcgattgacggaaattcttcacgcttacgcatgctatcctcgacgcaattccgccttgcacggctctagggccggcgctgggtgcgacacaagatccaagaaccctccgaggacaccatgagactaattttgctgggcgcgcccggggcgggcaaaggcacgcaagcggctttcatctgccagaagtacggcattcctcagatctcgaccggcgacatgctgcgcgccgccgtcaaggccggtacgccgcttggccagcaggccaaggcggtgatggaatcgggtggcctggtgagtgatgacctgatcatcaacctcgtgaaagaacgcatcgcgcaacccgattgcgccgatggcttcctgttcgacggctttccgcgcaccattccgcaggccgacgccatgaaggcggccggcgtcaagctcgactacgtgctcgaaatcgacgtgccgttcagcgacatcatcgaacgcatgagcggccggcgctcgcaccccgcgtcgggccgcacctaccacctgaagttcaacccgccgaaggtcgagggcaaggatgacgtcaccggcgaagacctgattcagcgcaaggacgacgaggaagaaaccgtgcgcaagcggctcgatgtctacagccagcagacgcgtccgctggtcgagtactactcggcctgggccaaggccgatccggccgcggcgccgaagtaccgcgccatcagcggcgtcggcacggtcgacgaaatcacccagcgcgccctcgctgccctgagcagctgaacgcgagccgccgtcaggcggcagtggcttcgagcagctccagcatcagcgcaatgcgagccttgacgggcgtcagggcaccggcgtcccgcaagcgatcatcagctcttggcaggatgcgcccgctcgcacagcgtgtggcgcgcagcacggccactcccgcatcctgggctcgcagcgcggcagcctccagcgcatggtgcaccgtgccattgccggtcgcggccaggaccaatccccgaatcggctcggccacgccggctgcacgctcctgcagcagcagatcgacgatggcgccagttgcgccggcatggctggtgacgatctcgaccctcggccagtgcgttgccgcgcctgccttcgttgcgggaatcttcgaagccgcactcaccggcaatcgcggccagtcgcgaagaagccgcaccgccccctcttccacgtagccgatcgggcctgcatcgcccgatgaaaacgcatccggtcgataggggtgcaccttctgcacatccagcgaaccgtggaccgtgcccgcgcagaccaccgtcacgccctgcgctcccggcgtggccgcaacggcgatggcatcgcgcacattctgtgggccgtcgggcgaaagagaactcgcgggacgcatggcgcaggccaggaccacgggcttgccaggtgcaagcaccgcctggagaaagtaggccgtctcttcgatggtgtcggtgccatgcgtgatcaccacgcccgccacgtcggcctcggacagccagaacgcgcagcgctgcgcaagttgcagccagacatcgaagcccatgtccttgctgtcgagctgcgccacctgctcggcttcgagcgccacgccatcgggcgcatcgacgccgccgagcaggtccgccacgcccacctgccctgcggtgtagccgatgttgtcgccgccgctggcggcgcgacccgcaatggtgccgccggtgcccagcaccacgacgcgccgcaggccggacgaaagggaattgaccatgcttgccaacttttaaaaactggttaaaaatacaggtactggatattcagccagtgccgcaaggaaccacatatgcagttcgccgtgaagcttaccgcccgccagcagcaaatcctggacttgatccagagcgccatcgcccgtaccggcgctccgcccacgcgggccgaaatcgccagcgagctgggtttcaagtcggccaatgcggccgaagagcacctgcaggcgctggcccgcaagggcgtgatcgaactcgtcagcggcacttcgcgcggcattcgcctcaagggcgatgcgctgcgttcgctcaacgagtcgcgcaacaaccagttttccctctcgctgcccggcatggcgcagcttgcgctgccactcatcggccgcgtcgcggcgggctcgcccatcctcgcgcaagagcacgtcgaccagacctactacgtcgagaacacgctgttccagcgccagcccgattacctgctgaaggtgcgcggcatgtccatgcgcgacgccggcatcatggacggcgacctgctggcggtgcaagccaccaaggaagcgcgcaacggccagatcgtggtggcccgcctcggcgacgaggtcacggtcaagcgcctcaagcgcaacaagcaggtcatcgagctgcacgcagagaaccccgactacccgaccatcgtggtccagcccggcgaacccttcgaaatcgaaggcctggcggtcggcctcatccgcaacaccatgctgatgtaggccctgcggcctgccgaaagcagcacctcattcggccgcaacaggtggcgggcgtatggcgcaaagtcgccatcaccctgttgcgtcccttcaaagaaatcctgcctgtgttcaacctcagacttttttggagttcacatgggaatcgccctcctcaccatcgttgatttgtggatgccgctgcaatcgctggcaagccgcctgctgccggcacgccggccccgccaccgcgacaatagcggcagcgcctccgccggactgcgctacgtcgcggttcggccggcctgcacggcgcgcccccacggcgccgcggcacccaatgcagcaccagcacccagccggccgcttcgcgtcattcgcgtggtcgacgggccccagggcgaaaagcgcagcaccaaccgcatggtgatctcggggcgcatggccgacgtctgcgccgaactcgatcggctggcggcgctcgaagccatggaggcggtcagcaccgcaccacgctccacgcgcctgcactgaacccgtgcaagccccggtgaccatggccgggggtgggtatccaaacgttcacacgcgcgtcatgtcaatgctgcgaggcacaatggcacgccatgaacattgtgatcctcgacgattaccaggacgccgtgcgcaagctgcgctgcgccgccaagctggacgcgtacgcggccaaggtctataccaacacggtcaagggcatcggtcaactttcggttcgcctgaaggatgccgacgtgatcgtgctgatacgggagcgcacccacatctcgcgccagctgatcgaaaagctgcccaagctcaagctcatttcgcagaccgggcgcgtgggtggccacatcgacgtcacggcctgcaccgagcggggcgtggcagtggccgagggcaccggctctccccaggcgccggccgagctgacctgggcactcatcatggcggccatgcgccgcctgccgcagtacatcagcaacctcaagcacggggcgtggcagcagtcggggctcaaatcggcctcgatgccgcccaatttcgggctgggttcggtgctcaagggcaagacgctctgcatctggggctatggccgcatcggccagctggtggcgcgctacgggcaggccttcggcatgcaggtggtcatctggggccgcgaggccagctgcgccaaggcccggtccgacggcttccaggtagcgcagaaccgccacgagttctttgccgccgccgacgtgctgtcggtgcacctgcggctcaacgaagaaaccagcggcctggtcaagctcgaggatctttcgcgcatgaagccgaccgcgctcttcgtcaacacctcgcgcgccgaactggtcgaggccgatgcgctgctggccgcgctcaaccgcggccggccggggctggccgccgtcgacgtgttcgagagcgagccgccgctgcagggccatgcgctgctgcggctcgaaaactgcatctgcacgccgcacatcggctatgtggagcaggacagctacgaaagctatttcggccaggctttcgacaatgtcgtgagcttcatcaagggcaaccccaccaacatcgtgaatcccggcgcgctgcaggttcgccggtgatctcatgagccgccgggccgccccaaggcggataccgcagacgaaggcgaaggtccttcagtgagccggccggcgccccggggcgcgctctgggcgctgctggccggcaatttcgtgatcggcacgggcgtgatggtggtgcccggcacgctcaatgagatcagcacgtcgcttgccgtcaccgttgcagctgccggccagctgatcacggccgccgcgatcgtgatgtgcctcggtgcgccgctgctggcggccgtggtcgcgggctgggatcgccgccagttgctcgccctcaccctcgtctggtacgccgccgggcatgtggtcgcggccttgatgccgagcttcggcgccctgctgccggtgcgcatgctcacggtggtggcaccggccatcttcacgccccaggccgcggcctgcgccggcatgctggtgccgccggagcagcgcggacgcgccgtgactttcgtttttctcggctggtcgatggcctcggtgctgggcctcccccttggcgcgctgattggcggccacctgggctggcgcacggctttcctggccgttgcgctgctcagcatcgcgagcgcggcgtcgatctggctgaccctgccgcgaggcatccggcccgcggcactgacggcggcagcctggtcgcgcgtgctccgcagcccggtgctgatgggcatcgtttcggtcaccgccctgcagggtgccggccagttcgttctgttcagctatttcggcccgctgctgaagcgaaacttcggcgcggatcccaccacgctgagcctgatgtgggccctgttcggcgccttcggcctggttggcaacatgctggtgagccggttcatcgaccgtgcgggcgccggccgcatggtgctcgtgaccagttcattgattgcactcagcctctttctctggccctgggccggcacactcccatggctggcggcggtactcgtgccctggggcctgggctgcttcgcgaccaattcggcgcagcaggcgcggctggtgggcctggcccccgctctcgcgccgggctccgtggcgctcaacagctcgggcatctacatcggccaggccgtcggtgccggactgggcggatggctgcttgccaacgatgcggtggcttggatgaactgggtcggtttcgccttgctgctgctggccatcggcctgagcgtggccatcgagcgcagccgccgcgcggcctgaagcgcggacccgcgtaaaacccggcacgcccccgaggcccgtggctgcaaaatcgaaggctgcgcaactccgggcccggcgcctgcaagcaggcccggacccatcaaccagcgaaaatctttttcaatgacagtgaactacacccggatcggcgtcgtcggcgccggcgccatgggtcgaggcatcgcccagatcgctgcccaggcgggcagcgaagtgctgctgctcgacagttttgcaggcgcggccgaacgcgggcgtgaagccctcgcggcccaatggaacaagctgcacgagaagggcaagatcgacgccgcggcgcgcgatgcccagatcgcccgcgtcaaggcggtcgattcggttgcggccctggcccagtgcgacctcgtgatcgaagcggtggtcgaagacctcgaggtcaagcgctcgctgttccgcgaactcgaatcggtggtcgcgcccacggccacgctcgccaccaacacctcgtcgctgtcggtcaccgccattgcggccgggctcaggcagccggagcgcgtggcgggctttcacttcttcaaccccgtgccgctgatgaaggtggtcgaggtggtggccggcttcaagacctccaccgaagtctgcaaacagcttgccggctatgcggtgcagatgggccatagcgccgtgcaggcgcaggacacgccgggcttcatcgtcaaccacgccgggcgcggctacggcaccgaggcactgcgcatcgtgggagaaggcgtggccgacttcgccaccgtcgaccgcatcctcaaggagcaggccggctttcgcctgggcccgttcgagctgctggacctgacggcgctcgacgtgtcgcacccggtgatggagtcgatctatcaccagtactacgaggagccgcgcttccgacccagcgtgatcacggcccagcgccttgcggcgggcgtgctgggccgcaagaccaacgaaggcttctacagctacaacgacggcgtgatgcagcaggttcccgaagccgcaccgcccacgctctccgagctgccttccgtctgggtctcgccccgcgccgcgcgccgggccgagttgctgcggctggtcaacgccttgggcgcccagatcgacagcggtgccacggccgcgcccacgtcgctcatcctggtggcgccgctgggcttcgacgtgaccacggtggccgctgtcgagcgcctggatgccacgcgcaccgtcggcatcgacatgctgatcgacgatgccgccaccaagcgccgcgtgctcgccaccaacccggccacgcggcgcgacatccgcgatgtggcgcacgccctcttcgcacgcgacggcaaggccgtgagcgtgatccgcgacagcggcggcttcgtcacgcagcgcgtgatcggcaacatcgtgaacattgccgccgacatgtgccagcagcgcgtctgctcaccggctgatctcgaaaccgcggttcagctggggctgggttacccgcgcggcccgctggccatgggcaacctgtatggccccaccaacatgctcgaggtgctgttcaacctgcagaccgtctacggcgatccgcgctatcgcccgagcccgtggctgcgccgccgcggcgcgctgggcctgagcctgctgcacgaagaagaataaacaagccaaccccaacgaaagcatcacagcgatgaccgccgaactgaagagcaccagcgagggacgcaccatggtgctcaccatcgccaacccgacccagcgcaatgcgctgggccccgagatctacgccgcgggcatcgaggcgctcaacggcgccgagagcagcgaggagatccgcagcgtcgtcatcgtgggcgaaggcgcatggttctgcgccggaggctcgctgcagcggctatccgacaaccgccagcgcgacccttcggtgcaggccgaaagcatcgagggcctgcacaactggatcgattccatccgtgccttccccaagccgatcatcgcggcagtcgagggcgcggcggcaggcgcaggtttctcgctcgcattggcctgcgatttcgtcgtggccgcacgcgatgcggtttttgcggcgtcctacagcaacgtcgcactgtcgcccgacggcggcctgagctggcacctgggccaggccttgccgcgccagctggcgagcgaatggctgatgtgcggcgaacgcatcggcgcgccacggctgcatgcgctggggctcgtcaatgaactgagcgaaaacggccaggcgctcgccagcgcgttggcgctggcaacccggctcaacgctcgcgcgccaaactcgcttgccagcatcaaggagctgctgagcgaggcgcgcggcaccacgttcgcatcgcagctatcgcaggagcgcgaccacttcgtgcgcaacctgcatcatccgaacgccggcatcggcattgccgcgtttctcgagaagaagcctccgcagtacgagtaacggcattacgtcgctctcgtgacaccctccagcatttcagtcgccgacaggacagaccaatggacgaccccattcttaccatcgaagaacgtgaagcgatcaacagtggtcgctggttttcttctctatctccctcgctgcggcacgacattctccgatgcgctttcgtcaaacgctacaaggacggcgacctgatcgccgcccgcggcgatcctcccgaccactggattgcctgcgccaagggcgcggtgcgcgtcagttccacggccgtatcgggcaagcaggtgacgctgacctacgtggagccgggcatctggttcggcgacgtggcgatgttcgacggggaccggcgcacccacgacgcctatgcgcatggggaaaccaccatcctctgtgtggcgcgggccgatttccagaagatcctggccacgcacgtggagctgtacgaagcgctcatgcgtctgcaggcgcgccgcatccgcacactcttcgggctggtggaagacctcaacaccctgcccttgcgcgcgcggctggccaagcagctcattcacctggtgcgcagctacggcgtgcccaatctggaagacggcagccagatgcgcatcgggctgcagcttgcgcaggaagaactggcgcagctgcttggcgcatcgcgccagcgcgtcaaccaggaactcaagaccatggaacgcgagggcaccatccgcatcgagccgggtggcctcgtggtcctcgaccgcgtggcactgatgcgcgtctccgaagcggatatctgacatgagccaggacttctccaacttcatcggcacccgggcagtttcgcagcagcacgccttcgacgtcgacgcgctcgcggcctggctcgagaagaacctcgacggtttcaagggtccgcttgaggtcgagatgttcaagggtggccagtcgaatccgacctacaagctcgtcacgcccacacagagctacgtgatgcgcgccaagcctgggccggtcgccaagctgctgccctcggcccatgcggtggagcgcgaattcaaggtcatgagcggccttgccggcaccgacgtgcccgtgccgcgcatgcactgcctgtgcgaggacgaatccgtcatcggccgcgccttctacgtgatggagttcatgcagggccgcgtgctctgggaccagtcgctgcccggcatggacaatgccgagcgcgcggccatctacgacgaaatgaaccgcgtcattgcggcgctgcacaccgtgaagttcgccgagcgcggcctggccgactacggcaagcccggcaactacttcgagcgccagatcggccgctggagcaagcagtacaaggcttcgaccgatggcgccggcgaactgtcgcagccgatcgaggccatggagcgcctgatcgactggctccccgcccacatgccggcgagcgcgcgcgacgaaagcaaagtctcgatcgtccatggcgactatcgcctggacaacgtgatgttccacgccaccgagccgcggatcatcgcggtgctcgactgggagctctccacgttgggccatcccctggcggacttcagctaccactgcatgtcctggcacatgccccccaccaccggccgcggcatcggcggcgtggatgtcgcggcgctgggcattcccaccgagagcgaatacatccgccgctactgcgagcgcacgcgcatcaccacgcccgaggcgctggcgcccgactggaatttctaccaggcctacaacctgttccgcatggccgcgatcctgcaaggcattgccaagcgggtcgaagccggtaccgcttcaagcgagcaagccgtggcctccgcccgcggcgcgcgaccgatggccgaaatggcctggcagtttgcccaaaaggcgtagctgcctcacacccccaccaggagacaaacgatggacttcgaatactcggcaaaaaccaaggaactccagaagcgcgtgagcgcgttcatggacgcgcacatctatccggccgaagccgagtattcggccgaactggccgccaacacggccgccggcaagcgctggaccgcgctcaagacggttgagaaggtgaaggaaaaagccaaggcccaggggctgtggaacctgttcctgccggtcgacagtgcctccgcctcgggctacgaaggcgccggcctcacgaaccaggaatacgcaccgctggccgaaatcatgggccgtgtgccatgggcctcggaagccttcaactgctcggcgccggacaccggcaacatggagaccattgcccgctacggctccgaagccatcaaggcgcgctggctcaagccgctgctcgaaggccagatccgctcggccttcgcgatgaccgagccggacgtcgcatcgagcgacgccaccaacatctcgacccgcatcgaacgccagggcgacgagtacgtgatcaacggccacaagtggtggatttcgggcgctgccgacccgcgttgcgccgtgttcatcaccatgggcaagagcgaccctgacgcgcccaggcattcgcagcagagcatgatcatcgtgccggctgacgccaaaggcatccgcatcgtgcgcccgctcaacgtgatgggctacgacgatgcgccgcacggccacgtcgagatgtacttcgagaacgtgcgcgtgcctgccgacaacatgctgctcggcgaaggccgcggcttcgaaattgctcagggccgcctcggcccgggacgcattcaccactgcatgcgcctcatcggcctggccgagcgcgcgctcgaactcatgtgcaggcgcgcctcctcgcgcgtggctttcggcaagacggttgcgtcccagaccgtgacgcaggaacgcatcgccgaagcgcgctgcaagatcgacatggcgcgcctgctcacgctcaaggccgcatggctgatggacgtggccggcaacaaggttgcgaagaacgagatcgcaatgatcaaggtggtcgcgccgagcatggcctgccaggtgatcgactgggccatgcaggtgcatggcggcggcggcatgagcgacgactttccgctcgcctacgcctacgccggtgcgcgcacgctccgttttgcggacggcccggacgaagtgcaccgcaacgcgattgccaagtgggaactgggcaagtattcgccgaacaaggccgatgccgaaatgccggtcacgcgtttctgatttgtcttgttccctctccctccgggagaggattagggtgagggccgacggcgccaaacgcgcctcggccctttttacgttcagagcttcttctgcagaaacaccgcgtgtccaaacgccggatcaagctgatagccgatgaatccttcacgctcgtagctgcgcagcgcaggctcattgcctgagagcacttcgagcgtcagcttgcaggcgccacgcgccctcgcctcctgctccactcgcgcgaacatgcgctgcgccacgcgctggccgcgatggctgggcaggacgaccacgtcgtgcacgttgaccagtgggcggcaggcaaaagtcgagaagccttcgatgcagttgacgagaccgacgggctgtgcgccgtcgtacgccagcacgctgaaggcttgcggccgcgcggccagtgccgcgggcaggccggcgcgcacgctggcttcgagtggcgtgccgccgccggcgggatcgcgcgcataggcgtcgagcagatcgaccagcgcggccgcgtgcgcggcattgcggtaatccgccaagacgacttcgatggccgtcaacgcgcgggctcgagggttgccgcaaggcgtttcgcgcacgcttcggcctgcttcgcgtcgcgcgcttcgaccatcacgcgcaccagcggctcggtgccgcttgcgcgaatcagcacgcggccgccatcgccgagttcggcttcggtacgctgggtttcgcttgccagggcgtcgttgttcttccagtcctggccgggcgccagtcggacattgatcaggacctgggggaacagtgtgagatccgaaagcaattgcgccacggtcttgccgctgcgcacgcaagcctgcagcacctgcagcgcactcacgatcccgtcgccggtggtgtggcggtcgagcaccagcagatggcccgagccctcgccgcccagcagccagccgcgcttgtcgagctcttcgagcacgtagcggtcgcccaccttggcgcgcacgaactcgatgccctggccgcgcagcgccacctcgacggccttgttggtcatcagcgtgccgaccacgcccacgggcttttcgccgcgcgcgatgcgctcggtcaccatcaggtagagcagttcgtcgccgttgaagagacgcccgctcgcgtcgacgagctgcaggcggtcggcgtcgccgtcgagggcgatgccgtagtcggccttctgctcggtcacggccgccaccagcgctgccggatgggtggcgccaaagccgttgttgatgttgagcccgtcgggcgtacagccgatgctggtgacctcggcgcccagttcgtggaaaacgttaggcgccacctggtaggccgcgccatgcgccgcgtcgatcaccagcttcatgtcgcgcagcgtcaggtcgttggcgaaagtgctcttgcagaactcgatgtagcggcctggcgcgtcgttcagccggcgggccttgccgagttcggcagaggttgcccacacaggagcctcctcgagcgcggcctctaccgcaagctcccactcgtcgtcgagcttggttccctgtgcgctgaaaaacttgatgccgttgtccgggtaggcgttgtggctggcgctgatcaccacgcccaggctcgcacgctgcgcgcgcgtcaggtacgccacgccgggggtcggcagcgggcccagcagcaccacgtcgacgcccgcggaattgaagcccgactcgagcgcgctttcgagcatgtagcccgagatgcgggtgtccttgccgatcagcaccgtggggcgcgactggctcctcttgagcacgcggcccacggcatgcgcgaggcgcagaacgaagtcgggtgtgatgggcgactggccgaccgtaccgcggatgccgtcggtgccaaagtattttcgggtcacgggatctcctcttgttgttgatcttgtgaaacttgcaaatcgggatgcggctcttcggccttcatggcgcgccatacggcgagtgccgacaccgtttcgcgcacatcgtgcacccgcacgacggccgcgccccgctctactgcgagcaccgctgccaccacgctgggcaccatgcgtccgctggcaatctcgatgccgctcacggcgccgatcgacgacttgcgggaccagcccagcagcagcggatagccggctccgagcaactcgcgctggcgtgccagcaggacaaaattctgcgccacggtcttgccgaagccgatgcctgggtcgagcgtgatccgcgaaggatcgatcttcagcgcctgcaattgcgccagctgctccgcccagaacgacagcaccgcgggcaccacgtcaccctgcatcggcgcggcctgcatggtttgcggatcccggtgcatgtgcatcaggcagacgccgcacgaaggatgcgcagccacggcttcgcgcgcaccgggctgccgcagcgcccagacgtcgttgacgatgtcggcgcccagttcgagtaccgcgcgcatgacttccggcttgtaggtatcgacggagacgggcacgttcaacttgaccgcctcccggaccacgggcagcacgcgcgccagctcggcgtcgagcggcacggccgggctgcccgggcgggtcgattcgccgccgacgtcgaggatgtcggcgccctctttcagcagctgctcgcaatggcgcagcgcggcctcggtggaggcatgcgctccgccgtcggagaaggaatcgggggtgacattgacgatgcccatcacgcgcggctgcgcgagatcgattgcgaaacgcgcggtctgccagaccggtgcgtgaggcgtcgtcatgctgcggcaccttcatcgaaaacggggcccagggccccgttgctgtttgacgccggatgcacttcaggcaactgtgggcgccggatccggattgacggctggcgtgccgccgctgccgccactgcccgacggcgggatgcgcggcgtccagtccttgggcggacgcggggcgcggccggccatgatgtcgtcgagctgctcggtgtcgatggtttcccattcgagcagggccttggccatggcgtgcatcttctcgctgttttcctcgatgaggcggcgcgcctgggcgtactgctcgtcgatgatgcggcgcacctcggcgtcgaccttttccatggtctgttcgctcatgttcgtggtcttggtgaccgagcggccgaggaacacttcgccttcgttctcggcgtagaccatcgggcccagcgcgtcggtcatgccgtagcgcgtgaccatgtcgcgagcgatggaggtcgcgcgctcgaagtcgttgctggcgccggtggtcatctggtgcatgaacacttcttcggcaatgcggccgccgaacagcatgctgatctggttcagcatgtactcgcggtcgtagctgtagcggtcttgcgccggcaggctcatggtcacgcccagggcgcggccgcgaggaatgatggtgaccttgtggaccgggtcgcacttgggcagcagcttgccgataagggcgtggccggactcatggtaggccgtgttgcggcgctcttcctcgggcatgaccatgctcttgcgctcggggcccatgaagatcttgtccttggccttctcgaagtcctgcatttcgaccacgcgcgcattgcggcgtgcagccatcagggcggcttcattacaaaggttggccaggtcggcgccagacatgccgggcgtgccgcgcgcgatgacgctcgggttcacgtcttggcccagtggcaccttgcgcatgtgcacgccgaggatctgctcgcggccgcgaatgtcgggcagcgtgacatacacctggcggtcgaaacggcccggtcgcagcaaggcggcgtccaggatgtccgggcggttggtggcagccaccacgatcacgccgaggttggtttcgaaaccgtccatctcgaccagcatctggttcaaggtctgttcgcgttcgtcgttgccgccacccaggccggcaccgcgctggcgacccaccgcatcgatttcgtcgatgaagatgatgcagggagcgttcttcttggcgttctcgaacatgtcgcgcacgcgggcagcgcccacgccgacgaacatttcaacgaagtcggaacccgagatcgagaagaacggaaccttggcttcgccggcaatcgacttggccagcaaggtcttgccggtacccggagggccgaccagcagcaggccacgcggaatgcggccgcccagtttctggaagcgctgcgggtccttgaggaagtcgacgacttcacggacttcttccttggcctcgtcgcagcccgcgacgtcggcaaaggtaaccgtgttgttgttttcgtccatcatgcgggccttgctcttgccgaagctgaacgccccgcctttgccgccgccctgcatctggcgcatgaagtagatccagacgccgatcaagagcagcatcgggccccagctcaccaggagcgtcatgaggagcgagccctcttcgcgcggcttgacgtcgaacttgacgttatggtcgatcaggtcgcccaccagaccgcggtcgagcacggttgcggttgtgcggatcttgcgatcgtcattggtgacggccacgatttcaccgccgccggcaccttcagggatgacggcactcttgatctggttgttccggacctggtccaggaactccgaatagctcaccgcccctgagccgaccccgccacgggtgtcgaactgcttgaacacagtgaacaacaccatggcaatgacgagccatacggcaactttggaaaaccactgattgttcaaacgaagctccagtcgaaagcgcgtgacaagattgtgaaagaacgcgctatggatacgcaattgcgccccattttaggcttttcaagctacgaaaagcgggcatttccctaaagcagccatagcttgacaagggtttgcgccccattggcgccctgccggggcctccggcgtcaaggtatcaaggcgtttcctgggctttcagacccatgccgacgagaaaggtttcggacgatttgtcgcgcgaagccttgggtttgaaaggcttcaccgtgcggaaattcgccttgaacagcttcaccagctcgtcatagccgctgccatggaaaagcttggcgaccagcgccccttcgggcttcagatgatgccgggcgaagtcgattgcaagctcgatcaggtgggccacgcgtgcggcgtcggccgaatggatgcccgacaggttgggagccatgtcggacaccaccaggtcggccttgcggcccgccaggacgcccagcacctgttcgagcaactccgcctcgcggaagtcgccctgcaggaaggtcacgccctcgatcggttccatcggcagcatgtcgagcgcgatgatggtgccgttcagctcgccggccgcagcgccgtcaggggacatccgccgccgcaggtactggctccaggcaccgggcgtggagcccaggtcgaccacgagctggcccggcctgacgaggcccagcgattcgtcgatttccttgagcttgtaggcggcgcgtgcgcggtacccctcccgcgtggccagtttgacgtacgggtcgttgatgtggtcgtgcagccacgccttgttgacttttttgcttttcgccttggtgctcatggggaccctctcgtgcttcgcgctgcggtattcgccttggaagcggcccggcgtttcgagaggttgctttctaccctcgataatacggggatgcccgccattcaacttacccctgccgagcgcaaggtgcaccgcgccgaagctcaccacctggatccgatcgtcatggtcggtggagacgggctcacccctgccgtgaaaaaggaagccgacgcggcgctcaaggcccatggcctgatcaaggtccgcgtcttttccgacgaccgcctggcccgcgacgccatgctgcgcgaactggccgaggagctcgacgcagcgcccatccagcacatcggcaagctgctggtgctgtggcgccccaagcccgaaaaggagcgtgtggtcgatgaagaccgcatgcccggcccgcgcgacatcaaggtgctgaagtacagcaagcgcggaggccagcgccccgaaatcaagaccctgcgcgtgctcggcaaccagcgcctcacccccggcggcaccatcaagcgcgccaaggcgaagcgcccgctctcggccaagaaacgcaatcaggcagactgaacttggtggcagcgcaaggcgtccagcgccacattctctgcatgaagtggggcaccaaatacggccccgaatacgtcaaccgcctctacgcgatggtgcgccgcaatctcagcggcgacttcaagttcgtgtgcctgacggacgacggcaacggcatccgccccgaagtgacgtgcctgccgatcccgccgctgaacctccagctggcgccgggccagcgcgacggcgcatggaagaagctcacgaccttcgaaaaggacctgcacggcctgcgcggcaccgccctgttcctggacgtcgacgtggttgtcgtgggcagcctcgacgccttcttcgagcagtccggcgaattcctgatcattcacgactacgcacgcccctggcgccgcgagcggatcacgggaaattcatcggtgtaccgtttcgagctgggcgcccatgccgacgtgctggcgtattttcgcgacaacatggacaaggtgcaggccgaataccgcaacgaacaggcctacctgtccgacatgctgcacaagcagggcaagctctcctactggcccgcggcctggtgcccgagcttcaagtaccacggcattcccatgtggccgaccaactactgggaagagcccttcgtgcccgagggcgcacgcatcatggtgttccatggcgaatgcaaccctccggatgcactcgcgggccggcgcaaccgggctttccgcttcatccggcctgcgaactgggtcgcgaagttctggaaagaatgaaatgaacggttgacggacgggacaggcaggcggtcctgccgccccgcttcagtctgccgtgggcgccctggcagcgcccatgcgccagagcagcgcaccagcacagagccattgaaccaggtacatcccgcttcccacggcgtgccacagcttgaggttgtcgcgcgccagaatgcgcggcgccacggcatattgctggagcagcgccagcagcaacgcacccagtatcaggaagatggcggtcatcgaggcgctgtcgatgcggtcgtccatcctggtcctgaaatgaaccaggaggagcaggccgcagccaatggcgatccagctctgcgcctcgaacagctggccggcaaaattgccggccaccgcgggattgccgagcttcgcgaagagcatcggcaccaccaggaaaccgattgtcgtgagactgccccaccagaaggcggccagcagcagcgcgaggcggtctttcatccagcgcggatcagaggtagcggaccgccacgatctcgtagcgcttgaggccgcccggggcctgcacttctgccacatcgccctcttccttgccgatgagcgcacgcgcgatcgggctggagatgttgatgaggcccagcttcaggtcggcttcgtcctcgccgacgatctggtatttgacgccttcgcccgactcttcttcctcgagctcgaccgtggagccgaacaccaccttgccgcccgcgtccagctcggtcgggtcgatgatctgcgctgccgaaagcttgccttcgacttcctggatgcggccttcgatgaagccctggcggtctttcgcgacttcgtattcggcgttctcgctcaggtcgccctgtgcacgggcctcggaaatcgcgttgatgacccaggggcggtccacggtcttgagctgatgcaattcagcgcgcagtttctcggcaccgcgcttggtaattggaatggttgccatgtttggttctccataaagcgaaaccgccgaacgctgccgttcggcggtcgattgggggaaaggatcagacgagggtgcgcctggtcagccggctcaggatggcgagcgggctcgaatccggattgtattgcttcgccgcgggcagatgaagggtctgctcgagcatgtactgccccgccatgacggcgtgcgaggtctggtcggagaagcacacccacaccgaacctggcgggaactccgccttctcctgcggtgaattctcctggtaggccatgtctgacttcatgccgtcgtgcagctgcagcatcaggtggtcgtattcgctgcggaacgacttggtcacatgcaacgcctgcagcagcttggcctgccatcgcacataagtcttggcacgcggcagaaagcgcttggcaatgtcttcgaagggctcgcccacgcgccacacgcgcggcgcgccgtcggggttgacgttggtgaacacgcgcaggatgcgctcgccatagttgggccgcgacggaaacgcatcgacgtgcaagcgccggtcatcggcgcgccacgactgcacgcgcgtctcgacctgggccggccggtagctggtcggcgccagtcgcaaggcaggcgtgtagtgcggcagcaggccatggatgagttgctgtgcctgagtgcgaaagcgcccgaccatcgccgcagttgcgcgctgcacctgctcgtcgcccgccacccccttgaggtggccgttggcatcgaggctgatgttgcgcacgtcgggcgacagcaggctgggcgtcagcaggctgcgctcttccggcagcagctcgaagcccagacgcggaaagtacagcaccttgccggcctcgagcgccgcgatccacgcctcgttgggcgtggccgcgttccagtcggccaggtccagttcgaccagctgggtttccatggcgctcaggcggcggccagctgcgcgtgcatctcctgcaccgagatcacgccgagctcgtccatgaagcccatgccttcgaccgcggcttcagcgccgaagatcgtggtgaacgtggtcacgcgcgccagcagcgccgaggtgcggatctgccgagaatcggtgattgcgttgcggcgctcttccaccgtgttgatgaccagcgcaatctcgttgttcttgatcatgtccacgatgtgcgggcgaccttcggtcaccttgttcaccgtcgcgcattcgatgcccgcggcgctgatggcggctgcggtgcccttggtggcgatgacttcgaagcccagcttgacgaggccacgcgccacttccacggcgcgggccttgtcgttgttcttcaccgaaatgaagaccttgcccgatttcggcaggtgcgtgccggcgcccagctgcgacttcacgaaggcttcgccaaaggtcttgcccacgcccatcacttcgccggtggacttcatctcggggccgaggatggtgtccacgcccgggaacttgacgaacgggaacacggcctccttcacgctgaagtacggcggcgtgacttccttcgtcacaccctgcgacgcgagcgactggccggccatgcaacgtgccgccaccttggcgagctggatgcccgtggccttgctcacgtaaggcacggtgcgggaagctcgcgggttcacttcgagcacgtagatgacgtccttgccgtccttctgctggatggcgaactgcacattcatcaggccgaccacgttgagcgccttcgccatcgcggcgctctggcgcttcagctcggcgatggtctcggcggtcaggctgtaaggcggcagcgagcaggcggagtcgcccgagtgcacgccggcctgttcgatgtgttccatcacgccgccgatcagcgtgccgccttcggcatcgcggatgcagtcgacgtcgcactcgacagcgtcgttcaggaagcggtcgagcagcaccggcgagtcgttgctcaccttgacagcttcgcgcatatagcgctcgaggtcgcgctgctcgtgcacgatttccatcgcgcgtccgccaagcacgtagctcgggcggaccaccagcggataaccgagggccgcagccttttcgagcgcttcgggctcggtgcgggcggtggcattcggcggctggcgcaggcccagctcatgcagcagcttctggaaacgctcgcggtcttcggccgcgtcgatcatgtcgggcgaggtgccgatgatcggcacgccgttggcttcgaggtcgagcgcgagcttgagcggcgtctggccgccgtactgcacgatcacgcccagcggcttttccttgtcgacgatctcgagcacgtcttcgagcgtgagcggctcgaagtacaggcggtccgaggtgtcgtagtcggtcgacacggtttcgggattgcagttgaccatgatggtctcgtagccgtcttcgcgcatggcgagcgcggcatgcacgcagcagtagtcgaactcgatgccctggccgatgcggttggggccgccgccgagcaccatgatcttcttcttgtcggtcgggtcggcttcgcactcgtcctcgtaggtcgagtacatgtaggccgtgttggtcgcgaactcggccgcgcaggtgtccacgcgcttgtagaccgggcgcacgccgagggcacggcgcttctcgcgaatcgcggtatcggtggtcttcagctggcgcgccaaacggcggtcggagaagcccttcttcttcagcgcgagcagcgtgtccttgtcgatatcgtcgagcgacttggtttcgagttcgagttcgatcttcacgatctcttcgatctgcaccaggaaccacggatcgatcttggtcagcgcgaacacttcatccacgctcaggcccatggcaaaggcatcgcccacgtaccagatgcgctcggggccgggctcgccgagttccttctcgagcacttcgcggtcctgcgtcttctcgttgaggccatcgacgcccacttcaaggccgcgcagcgccttctggaacgattcctggaaggtgcggcccatggccatcacctcgcccaccgacttcatctgcgtggtgaggcgcgaatcggcctgcgggaatttttcgaatgcgaaacgcggaatcttggtgaccacgtagtcgatcgacggctcgaacgacgcgggcgtggcgccgcccgtgatctcgttgcgcagctcgtcgagcgtgtagcccacggccagcttggccgcgaccttggcgatcgggaagcccgtcgccttggaggccagcgccgacgaacgcgagacgcgtgggttcatctcgatgacgaccatgcggccgtccttcgggttgatggagaactgcacgttcgagccaccggtgtccacgccgatctcgcgcagcacggccagcgaggcgttgcggagaatctggtattccttgtcggacagcgtctgcgcgggggccacggtgatcgagtcgccggtgtgcacgcccatcgggtcgaggttttcgatcgagcagacgatgatgcagttgtcggccttgtcgcgcacgacttccatctcgtactctttccagccgagcagcgactcttcgatcaagagctcgttggtgggcgaggcctcgatgccgcgcttgcagatggtctcgaactcttccgggttgtaggcgatgccgccgccggtgccgccgagcgtgaagctggggcggatcacggtcgggaagccgaccgacttctgcacggcccatgcttcgtccatcgagtgggcgatgccggagcgcgccgagccgaggccgatcttggtcatcgcgtccttgaacttcaggcggtcttcggccttgtcgatggcttcgggcgtggcgccgatgagttcgaccggcttgttggtggccgcgcccgtgtacttgtcgagcacgccgttgcgccagaggtcgagcgcgcagttgagcgcagtctgtccgcccatggtcggcaggatcgcgtcggggcgctccttggcgatgatcttctcgaccgtctgccaggtgatcggctcgatgtaggtgacgtcggcggtggccgggtcggtcatgatcgtcgcgggattgctgttgatcaggatgaccttgtagccctcctcgcgcaatgccttgcaggcctgcacgccggagtagtcgaactcgcaggcctggccgatgatgatcgggccggcgccgatgatgagaatggatttgaggtctgagcgcttgggcatcttatttgtccttggtgaaaccgatgccgcggccgctgtaggcgcccggcttcggctcatccatcagttgatggatcgcgttgaatacatcgcgaaagttctggtcgtaccgctgttccagcgcgttcagcttgcgcttgagatcggcgtgctccgacagcatgctgcgcagcttgacgaaggaacgcatgatctcgatgttgacggccacggcgcgttcgctgcgcagcacgctcgacaacatggccacgccctgttcggtgaacgccacgcttcggtagcgcgcgccaccggagcccggcttctcgggttttgagatcacaagttgtgatttcaaattctcgaggtcctggttctccagggtgaaggcgaaatccgccggaaaacgatcgaggttgcggcgcatggcctgcaacagcacccgggtctcgacgccatagagcgcggcaaggtcctgcgccagcatgaccttgaggccgcgcagcgcgtagatcttgccctcggcatcgcgcaaggcggcgatgaccgaagcgtcgagcaccgcgggtgcatcagccacgtgcctgctccatgagcgcggtgaagcggtcgaacaggtagccgatgtcgtgcgggccgggcgaggcttcagggtggccctggaagcagaacgcgggcttgtcggtgcgggcgaggccctgcagcgtgttgtcgaacaggctgatgtgggtggcgcgcaggttggccggcagcgacttttcgtcgaccgcgaagccgtggttctggctggtgatgctcacgcggccgttgtccaggtctttcaccggatggttcgcgccgtggtggccgaacttcatcttgaaggtcttcgcacccgaggccagcgccatgatctggtgccccaggcagatgccgaaggtgggaatgccggtctcgatgagttccttgaccgcgctgatggcgtagtcgcaaggctccgggtcgcccgggccgttggccaggaagatgccatcgggcttgagcttgagcacatcggcggcgggcgtttgcgccggcaccacggtgatgcgggcgccgcgctgcgcgatcatgcgcaggatgttcttcttgacgccgtagtcgaaagccaccacgtggaacctgggtgtgatctgcacgccataaccagcgccgagcttccactcggtttcggtccactcgtaggtctgcttcaccgacacgaccttggccagatcgagcccggccatgttgggcgcgcccttggccgctgcaatggccttgtcgatcagcgcctgcgtgaccgcctcacccgcggccaggcccaggatgcagccgttctgcgcgccgtgggtgcgcaggtggcgggtcagcttgcgggtgtcgatgttcgcgatggccaccgtcttgccggccacgaggtattcgctcagcgtggccgtcttgcggaaattggatgcgacgagcggcaggtctttgatgatcaggccagcggcatggatcttgtcggcttcgatgtcttccccgttgacgccgtagttgccgatgtgcggatacgtgagcgtcacgatctgctggcaataactcgggtcggtgaggatttcctggtaaccggtcatggaggtgttgaacaccacctcaccggtcgtggagccggcggctccgatcgaattgccttgaaagaccgtgccgtctgcgagcgccaggatggcgggcgggaaacttcccttgagagacaaaagcactgggttctccggatggttacggtcgcccggagccccaggcgcgttgcctgcggactgctgcttaaggggattttggcgttaaaggcggccgggcgacgctattgcgagtaagcccccgattgtagctcggcggcatcgctctcccgcctcgcggggccgtaaaacatacgcgcctcatgcctttatggcattggcaaatcaggaaacggcctgcgcaaacccggccgcaccgctcgcgtgcaggcagatggccgccgcggcagccacgttcagcgactcctcgccgcccggttgcgcaatgcggatgtgatgcgtggcccgcgcttcgagcgcgggcgaaacgccctgcccctcgtggcccatcagccaggcgcaggggtttggcaggcgcgcctcgtgcagccactcgccccggtgcgaactggtggccagcagcggtaccttcagctcgtcgagcgcgtcggcttccacgccttcgatcagccggaggccaaagtgcgcgcccatgcccgcgcgcagcaccttcggcgcccacagcgccgccgtgcccttgagcgcgatcacctgcttgaagccgaaagccgctgcgctgcgcaggatggagccggcattgccggcatcctgcagccggtcgagcacgacgctcggcgcgtcgggcagcagcgcgggccgggaaggcagctcgagcacgaatcccatcggcgccggcgattccagcccgctgacggcgcgcaggaggtcatcgtcaaccactaccgttttagtagcagcattcgcccactcggcgggggccagcggccaaaaagattcagaaaaaacggcgatggcgggcttgaccccccgcgcgagtgccgcgcggcagagatggtcgccttcgagccagagtcggccgagtttgcggtaggcgcccgggtcctgggccagcttgcgcaagtccttgagcagcgggttgtcgcgcgagctgatgtggctcgcgccggtcggggtggtcatgtggcggctcagcgctcggcgcgcaggtcgaggtgcacggtctcgaccgttgcaatggccatcggcagcggcatggcggcttcggccaacgcagctgcatcggccatcgtgcgcgccagcgccgcggccaccggactgaacgacctgcggtgatgcacgcatgcaccgtggcgctgcagcgcctccaggtgctccggcgtgccgtaacccttgtggccggcaaacccgtaatggggaaactcgacgtgcaactgctcgcacaggcggtcgcggtggaccttggccaggatcgacgcagcggaaatcgccttgatccgggcgtcgcccttgacgatggcttcagccagcacgtcgagcgtcggcaggcggttgccatcgaccagcaccttggcgggcttgagccgcaggccctcgaccgcgcggcgcatcgcgagcatcgtggcctgcaggatgttgtgggtgtcgatttcttccacgctggcttgcgccaccgagcagcacagcgccttggccaggatctggtcgtgcaggcgctcgcgttgcagcgccgtgagggtcttggaatcggccaggccgcggatcgggcgctggtcgtccaggatgacggcggccgccaccaccggaccggccagcgggccacggcccgcctcgtccacgcctgcaacgaggcccggggcgtcccacacgagggcagcctgctcagccttcaagaactttctggatcgcatcggcgcaaagtgtcggcgtatcgcgctgcagttgcacgtgcagctctgaaaatttttgttgcagcgcctgcgtcttttggggcgcatcgagccaggcgagcgtggcctgggccagcgcctgcggcgtggccgcgtcctgcaggagctcgggcaccacgaactcgcgcgacaggatgttgggcagaccgacccacggctggagctgcttgcgctgcatgaggcgccacgacagcgagttcatgttgtaggcaatgaccatcgggcgcttgaacaacgccgcctcgagcgtggcggtcccgctggcgatcagcgtgacgtcgcaggcggccagcgcggcatgcgactggccgttgagcaaggtcacgcgcccggcgatgccgctggcctgcagcagggcctcgacctcgacgcgcaggctcggcaggatgggcgcaacgaactggagcgcgggccttgccttcagcatctgcgcggcggcagcaaagaaccgggcggccaggtagcgcacttccgaacggcggctgccgggcagcaaggcgacgacctccgcgtcgggtgcgaggcccagcgcggcacgggccgcgccacgatcgggcgccatgggaatcacgttggccagcggatggccgacgtagctgccctgcacgccatgttcggccagcagcgcgggctcgaacgggaagatgcacagcacgtggtcggctgcggcgcggatcttttcgatgcggtcagggcgccaggcccagatcgagggacagacgaaatgcaccgtcttcatgccgcggccgcgcaacccggcctcgagatcgaggttgaagtcgggggcgtccacgccgatgaagagttcgggccattcgcgcagcagccgcgccttgagctggcggcggatgccggcaatctcagcatagtggcgcagcacttcgatgtagccgcgcacggccagtttttcttgcggccaccagctctgcaggccatgcgcaagcatgcgcggcccgccgatgcccaccgtctggagcgacggccagcgcgcctgcaggccatcgagaagaaggcccgcgagcaggtcgccggaagcttcgcccgcgaccagcgcgaaccgccgctgttcgtccttgcccatgccgagagttacttcaacgcgcgatgccgcgcgtcgaattggccaggaagcgctccatcagcgccacgtcctcggccgcctcgggcgtgtcggccgccaaggcggtgatgccggcgcgcgcttcttcgagcgtcttgccctgccggtacaacagacgatgcatctgcttcaccgcggcgagccggggtgccgaaaaatcgcggcggcgcaggccgacgagattgaagccgcgcaccgccaacggattgccgtcgaccagcatgaagggaggcacgtcctgcgacaccgcactggcaaagccgaccatcgcgtgggagcccaccgagacgaactggtgaatgccggtcagcccgccgatggtgacccagtcggccaggtgcacgtggccggccagcgtggtgttgttggccagcgtggtgtggtcatcgacgcggcaatcgtgcgcgatgtgcgtgtacgccatgatccagttgtcgttgcccacgcgcgtaatgccgcccgcccccggtacgccgaggttgaaggtgcagaactcgcgaatgacgttgcggtcgccgatgaccagctcggtcggctcgccggcgtatttcttgtcctgcggcacggcgccgatcgacgaaaactggaagatccggttgtcgcggccgatggtggtgcggccctcgatcacgcaatgcgcgccgatgctcgtgccggcaccgacccgcacgtgcggaccgatgatggtgtagggccccaccgaaaccgaggcgtcgagctctgccttcgggtcgacgagcgctgtcgaatgaacctgcgtcatgccttgtcgtaaccgccgcaggatcagttgatctggcgcatggcgcacatcagcgtggcctcgcaggcgagctcgctgcccaccagggcgcggcccttgaacttcgagatcccggctttcatgcgctcgatctcgacttcgagcgtgagctggtcgccgggctccaccgggcgcttgaagcgcgcgccgtcgatggccgcaaagtagtagaccgtgttgtcgtcgggcacgatgtccagcgaatggaacgacagcagtgccgccgcctgcgccatggcttcgagcatcagcacgcccggcatgaccgggcggtgaggaaaatggccgttgaagaacggctcgttcatcgtcacgttcttgagcgccgtgatgcgcttgcccttttccatgcccagcacgcgatccaccagcaggaacggatagcggtggggcagcagcttgaggatttgatggatatcgagcgtcgtcgtcatgattttctgttcctgcatcgtcttcactttttctggggggccttttcgagcgctttgagtcgttcgcgcaggctgtgcaactgcttgagcgttgcagcatttttttcccagctcgcattgtcgtcgatggggaacatgccggtgtactggccggccttgtggatcgagcgcgtgaccaccgttgcggccgaaacatgaacgccgtcggccaccgtgagatggcccagcacgatggcgccgccgccgaaggtgcagtgcgctccgatggtggcgctgcccgccacgcccacgcagcccgccatggccgtgtgcttgccgacccgcacgttgtggccgatctggatcaggttgtcgagcttgacgccatcttcgatgacggtgtcgtcgagcgcgccgcggtcgatgcaggtgttggcgccgatctcgacgtcgttgccgatgcgcaccgcccccagctgctcgatcttgacccacgtgccctggtgcggcgccaggccgaagccgtcggcgccgatcaccacgccgggatgcagcaggcatcgctcgccgatcacgcagtcttcgctgatcgtcacgcgcgacttcaggaccgtgccggcgccgatgcgtgcaccccgctccaccacgcacaacgcgccgatgcgcgccgttgcgtccacatgggcttcgggatggatcaccgcggagggatggatgcggtcggcttcgggacgcgcatggtgcgccttccacagctgcgtgaggcgcgcgaaataaagatagggatcaggagcgacgatgtacgcgccgcgtgccgccgcggcttcgcgcatggcgggcgaaacgatcacgcaagcggccttggaggctgccagttcctgctggtatttgggatggctcaggaagctgagcgcatcgggctgtgcattctggagcggcgcaagccgctcgatggacagcgccgcgtccccgtggagctcgccccccagggcgctgacaatggctccgagctgcaatgacacgccgatttcgcggcgttacttgccgcccgttggcgaagaagcggtcgaggcgttcagcgccttgatcaccttgtccgtgatgtcgtgcttcggattgatgtagatcgcttcctgcaggatggcgtcgtacttttcagcctcggccacctgcttcaccacgcggttggcacgctcatagacctgctggagctcttcgttcttgcgcgcattgaggtcctcctggaactcgcggcggcggcgctggaaatcgcggtcctggtcgaccagcgcgcgctggcgcgaagcacgctggctttcggacaaggtgggcgcctcgcgctcgaacttttcagaggccgtcttcagtgcctcgccctgcgtcgtgaggtctttctcgcgcttgaggaactcggcctcgagcttggcttgcgcggccttggccggctgggcttcacgcagcacacggtctggattcacgaatccgatgcgaaaggtttcctgcgcctgggccgcggtcgcggcaaccagtgcaaaaacaggaatcaacaacgcgccggctgcagcgcgaatcaaatgcttcatttagaaagacgttccaatctggaattgcaagcgctggattctatccttcgggatcacgatcaacccggtattcggatccaccacttccttttgggatttgatggggaaagcgtaggcaagacgcagcggacccagcggcgaaatccagctaatccccaagccgaccgaggcgcgcagcttcttctgggccttgtactgctcgtcggtcaggccttcggcgcgcgagccgaacacgttgccgacgtcgaagaagccgtaaaggcgaagggtgcggtcattgccggcgccggggaacggcgtgctgagctcggcattgaagaccgccttcttggtgccgcccagagcggcgccttcggtctggccaatcagtggcacgtcgcgcgggcccagcgaattctgctcgaagccgcggatcgaacccaggccaccggcgtagaagttcttgaagatcgggtagaccttgccgcccagcggcttggcataacccacgtccgcgttgattgcgaaggtgtattgcttgttgatcgcgaagaactgctggtactggtagttcgtcttgatgtactgcatgtcgccgccaacgcccagctcgaggttggcacgctgcatgcggccggtggtcggaaccagggcgctgtcgcgattgtcacggccccagccgacggtcagcgggacgccccacacgctcttctgggcgcactcggtcacgaacaagccgctcgcatccttggcgcactggaagtagcgcaggtaggacgctggcgtgaagagccccgagaacgaggtcgaggtgttcggatcgaacgcgtagcgctcgaggccggcgccgaagaagaccgtgtcgacttcgctgaacggcacgccaaagcggatcgaagcgccctggttgaccagcttgtagtcgccgtcgacgttggtcgagtatggacgcgtggtggtgtggtagaggctgatcgtgcgcgagatgccgtccttcgtgaagtacggatccgtggtggtcaccgacagcgtgcggttgtacttgctggtgttgacctggacgcccaggaagttgcccgaaccgaagacattctcttgcgagataccgaaggtgagagccaccttttcggcgctggagtagccggcaccgagctgcaggctgccggtgggcttttccgccacgttgacgaccaggtcgacctggtcgggcgaacccgggatttcctgggtctcgacgttcacttcggtgaagaagccaaggcggtccacgcggtcgcgcgagagcttgatcttgtcgccgtcgtaccaggaggcctcgaactggcggaactcgcgccggatcacttcgtcgcgggtcttggcgttgccgcccacggcgacacggcgcacgtagacgcggcgcgaaggctcggcttgcagcgtcaaggtgacgcggttgttgacgcgatcgatttcggggcgtgcctgcacgcgcgcgaacgcgtagccgaaggtgccgaaatagtcggtgaaggccttggtggtttcggtgacctgctcgccgttgtagggctcgccgggcttgatggtcacgagcgacttgaattcctcgtcacggccgagatagttgccgtcgagcttgacgccggccaccacgaacttttcgccttcggtgatgttgacggtcaccgacagatcctggcggtcgggcgagatggcaacctgggtcgaatcgatgcggaattcgaggtagccgcgcgtgatgtagtacgagcgaagcgtttccaggtcggcgttgagcttggaacgcgagtactggttggacttggtgtaccagctcatgaagccgccgctgtcctggtcgaacaggctcagcagggtcgattcgctgaatgccttgttgccgatgacgcgcacttcgcggatgcgggcggaatcgccctcggtcacggtgaacgtgaggttgacgcggttgcgctcgatgggcgtgaccgtggtcacgatctgcgcgttgtagaggttgcggctcacgtactggcgcttgagctcctgctcggcgcggtcggccagtgccttgtcgtagggccggccatcggccaggccgacttcgcgcagcgccttctgtagggcagccttttcgaattccttggcgccgacaaaatcgacgtcggcaatggtgggccgctcttcgacgatcaccaccagcacgttgccgttgacgtcgatgcgcacgtccttgaacaaacccaggtcgaacagcgcgcgaatggcggcggagccgcgttcgtcgctgtaggtgtcgccgacacgcagaggcagcgatgcgaagatcgtgccgggctcgacccgctgcaagccctcgacgcgaatgtcgcgcaccgtgaaaggctcgacggcccaagctgccgtggccgccagcgcgctggccaccaccgcggcaacgctacgcaggcgaaagcgactgaagtttgtgttcatctgtgaattgggccggcgcggaaagggccggcagaaagttaaccaaagagccgcgtgacgtcgttgaatagtgcgaccgacatcatgaccagcagcaaggcgacaccgccgcgctgcagccgttccatccaggcgtcagagacgctcttgccggtcaggccctcccaaagataatacatcaggtgccccccatcgaggaccggcagcggcatgagattcagcacgccaaggctcacgctgatcagcgcaaggaacaccaggtactgagtgaagccaaggctcgcggacttgcccgcatagtcggcgatcgtgagcggtccgctcaaattcttgagcgaagcctcgccgatcaccatcttgcccatcatgcggacagtgagggccgagacctcccaggtgcgcacgatgccgcgccagactccgtcgatgggcccctgccgaaccatgaccatctcgggcggcgcaccgacatacgcaccgatgcggccgaccttcacggcgccctcttcgcgcagctcgggcttgacttcaagctcgatcgactgcccgccacgccgcacttgccaggtttgcgcacgcggctggtcgccgtcgatcgacgtgcggatcacttcgcgcaattgctgtccgtcgacgatggccgtgttccccacggcgcgaaccacgtcgccattgcgaaggcccgcgcggtccgcggcgctgccggccatcacctggccgatctcgggccgggtcagcggcgcgatcacgccgatcttgcggaacatctgcgggtcggcgtccttggcctcgatgcggctgaggggcaggacgatctgccgcgcagcctgcccgccctcgcccgccacctcgagcgtgaggtcccggccgtcgagggcgccgcgcgtcatccgccaacgcaggtcttcgaacgattgcaccggctccaggtcgccctcgaagccggcgcgcgtgacgtgctcgccgccgcgcaagcccgcggcctcggccagcgaggccgcgaccggccgggccagcttggcgacgggctcgtccacgccgatccagttgacggccgtgtagagcaccaccgcgagcaacaggttggcaatggggcccgcggcaacaatggcggcgcgcgaacgcagcggctgcgtgttgaaggcacggtggcgttcttccggcgctaccggcccctcgcgctcatcgagcatcttgacgtagccgcccagagggaacgcagcgatgacgaattcggtttcctggcccgggtgctgccgcttgggctgccagcgatagagggtcttgccgaagccgaccgagaaccgcagaaccttgacgccgcacgccaccgcgacgcggtagtgcccatactcgtgcacggcaatgaggatgccgagtgcaaccacgaaagcgatgacggtaagcatccggatcctctatcggctagggggtgtcaggccgcgaagcgcagtgccgcggcattggcggccgcccgcgcactggcgtcgagcgccagcaggtcggccagcgatgcgggcttggagggggcaacggcctccaaagtttccatgttgaccgcatgaatgcggtcgaagcgcaggcgcctgtcaagaaaggcctcgaccgcgacttcgttggcagcattgagcaccgccgtggttccaggtgccgcgcgcagcgcatgccaggccaggcccaggcccggaaacagcgccgcatcgggggcatagaagctcagcgccgccatctggcggaagtcgaggcgccccgcgccactctcgatacgctcgggccaagccaggccgacggcgatgggcacgcgcatgtcgggggttccgagctgggcgatcaccgacgcatcggtgaactgcaccatcgaatgcaccacgctctgggggtggatgaccacctcgatctgttcgggcagcacaccgaacaggtggcgcgcctcgatcacctcgagcgccttgttcatcatggtggcggaatcgaccgaaatcttgcggcccatgacccagttcggatgggcgcaggcctgctcgggcgtgaccgaaccgagggtctcgggcgcgcgcgtgcggaacgggccacccgacgcggtcaagatgatcttgtcgatgcggcgcgaccaggtcgacggatcttccggcagcgactggaagatggccgagtgttcgctgtcgatgggcagcagcgtggcgccaccctcgcgcacggtgcgcatgaacagctcgccgccgaccaccagcgcttccttgttggccagcagcaggcgcttgccggcgcgcgccgcggccaggcaggggccgaggcccgcggcccccacgatggcggccatgaccgcatcgacctcttcatgcgatgctatcttttcaatagcatcgatgccactcagtacccgcgtgggaagattgttttgctggagcttttccgccagctgcgccgcatgtgccgggctggccataacggcgaaccggggcgaaaagcgcgcgcactgcgccagcagctcgtcgaccttggtcgaagcggacagcgcaaagacctcgaagcggtcggggtgccgcgaaatgacatcgagcgtgctgaccccgaccgaaccggtcgaacccagcaccgtgatgcgttgtttgggtgtgttcacaaggaagccagcatcattgcaatgggaagtaccggcaagagggcatccacgcggtcgagcacgccgccgtggcccggcagcaggctgctgctgtccttggcgccggcactgcgcttgatcagcgattcgacgaggtcgccgacgacgctcatcgccgcgagaaacaccacgcccacgagcagcagccaccagccgcgctcatgcagccgggtatagaggcttgccaccgtggcgccggcggccttgtcggcccagacccaggcgaaggccagcaccaccacgccggccatgccgccccacacgccttcccagctcttgccgggactgatggcgggcgcgagcttgccgcgcgtgaacttgagaccgaatgcgcggcccgcgaaatacgcgaaaacgtccgccacccagaccagcacgagaatcgagagcaggaagttgatgccgaccacgcgggcctgcactgccgcgagccatgccacccacagcgccagcaagccacccaccaggcgcaggccgcgcggaatgcgaggccagcccggaaccgccacccgcagcagcgcggccccgccaagcacccaggcggcgctggccagcagccacatgagcatcagcggctgcgcaagcagaccgagccaccacgaaagcgcgcacagcgcgactgtttcgaggccgaggaacaccgacagccgctgcccgtatccgttgaggcggccccactcccatgccgcagcgccgatcagtaccagcatgacgcaggcaaagggaacgtgggacggatagaagagcgccggcagcaggatcgccagcaggacgatggccgtgaggatgcgttgtttgagcatgcggctgaggagtcgggccgtgaaggccctcaggccatctggcgatctgaagaggaatcgctgccggccgtgacctgcgcggatgttttgccgaaccggcgctcgcgggcctggaacgcggcaattcccgcgtccaattcggcctcgtcgaactcgggccagagtttgctgctgaagaaaagctccgcgtatgcgctctgccagagcaggaagttggacagccgctgttcgccgccggtgcggatgagcaggtcggggtcgggcacgtgcgccagggccatggcgcggtcgagattggcctcggtgagggcctcgccctgctccaccagcttggcggcggcgcgcgcaatgtcccaccgcccgccgtagttgaagcagacgttgaggatcagtttggtatttggcgccgtggcttcctcggcattgaccagtccctgcaccattttcttggagagcccggcgcgttcgccgacgaagtgcagccgcacgccgtcgcggctcagctttggcacctcgcgtgcgagggcaccgaccatgatttccatcaggcccgagacctcttcggccggacggttccagttttccgacgagaacgcgaagaccgtgagaatgcccacgccgcggtcgacgcaggccttgacgcagcgccgcagcgactcgacgccctgcttgtgtcccgccacacggggcaggaaccgccgcgtggcccagcgtccgttgccatccatgacgacggcaatgtggcgcggaatctgcggcaaggagggggccatgcgcagcctcaaacggccatgatctccgcttccttggccgcgaccagacgatcgatttccgcgatgtggcggtcggtgaccttctggatctcggcttcggcgcgcttctggtcgtcctcggaggcgagcttgtccttgaccagcttcttgacggcttcgttcgcgtcgcggcgcaggttgcgcgtggcgatcttggcggtttcgccttcgttgcggaccagcttggtcatttccttgcggcgctcttcgctcatggcaggaagcggcacgcggatcaggtcgcccatcgaggccgggttcaggcccaggtcgctttcgcgaatggctttctcgatcttggcgcccatgcctttttcccagggctggacgctgatggtgcgcgagtcgagcaccgacacgttggccacctggctcagcgggacttgcgagccgtagtactcgacatggatcgaatcgagcagcgcggagttggcgcggccggtacggatcttggtgaggttgttctggaacgcagcgagcgactggttcatcttcgcatcggtcgtgctgcgaatttctgcaatggtgggggtcgtcatctcaatttactcctcaggcatgcaccagcgtgccttcgtcctcgcccatgacgacacgcttgagcgcgccgttcttgaagatcgagaacaccttgatcggcagcttctggtcgcggcacagcgcgaaagccgtggcgtccatgatgccgagattcttcgcgatcgcctcatcgaaagtgagcgacgtatagcgcgttgcatcggggttggtcttcggatcggcggaatacacgccgtcgaccttggtggccttgagcaccagctcggcaccgatctcggcaccgcgcagcgcggcggccgtgtcggtggtgaagaacggattgccggtgcccgcggcaaacaccacgaccttgccctcttcgagatactgcaatgccttgggccgcacataaggctcgaccacctgctcgatggcgattgccgacatgacgcgcgccaccagcccctgcttgttcatggcgtcggccagtgccaacgaattcatgaccgtggccagcatgcccatgtagtcggccgtggcgcggtccatgccgacggagcctcccgcgacgccgcggaagatattgccgccgccgatcacgactgcaagctccacacccatgttcaccacctcggccacctcttcgaccatgcgaacgatggtggcgcgattaataccaaaggcatcgtctcccattaatgcctcgcccgacagcttcaacaagattcgcttgtgggctgggcggggatcagacatgggcaatttccttacttggggttggcggggcgagtgtagaacgaggcggtgaaaaagcggcggcacacacacgtgcgccgtcgctttggggcgtaacagtttttacgcggcggccttggcggcagcaacttgagctgcaacttcggctgcgaagtcgtcgaccttcttttcgatgccttcgccgaccacatacagggtgaagcccttgatgctggtgtcggcggccttgagcatttgctcgacggtctgcttgtcgttcttcacgaacggctggttgtgcagcgagacttccttgaggtacttctgcacgccgccttcgatgcgcttggcaacgatgtctgcaggctgcggcttcttgccttcggcttcggccgtcttgcggtcttcctcggccttgccggcggcaacagcacgctctttttcgatcaggtcggcaggcacgtcggcggccgagatggcaaccggcttcatggcggcgatgtgcatcgcaacgtccttggccgaggtgtcgtcgccttcgaactcgaccatcacgccgatgcgcgtgccgtgcaggtacgaagccagcttgccgttgccggcaaagtgcttgaagcggcggaagctcatgttctcgccgatcttgccgatgaggcccttgcgcacgtcttcgagcgtggggccgaagccgtcttgctcatagggcagcgcgcccagcgcggcgatgtccgcggggttgtgcttggcgaccagcatcgcggcagcgttggccatggccaggaagctgtcgttcttggtgacgaagtcggtttcgcagttgatctcgatcatgccgccggcagcgccgtcgacaaaagccgtgaccacgccttcggcggtgatgcggcccgatgccttgccagccttgttgccgagcttgatgcgcagcagctcttcggctttttccatgttgccgtcggcctcggtcagggccttcttgcattccatcatcggcgcgtcggtctttgcgcgcagttcgccgaccatgcttgcagtgattgcagccattgttctatctccgtgtccaaaaaatcaggttaaaaaaaaggggcaccaaagccccttcttcaggctcgcgagagcaccaatcaggccgaagcgccttcttcgacttcgacgaattcgtcgctgctgccttcggcgatggccttgaccacgtcaccaccggcgctgttgcggccttcgatgatcgcgtcggcgatgccgcgagcgtagagcgtgacggccttcgacgagtcgtcgttgcccggaatgacgtagtcgatgccttcgggcgagtggttggagtccaccacgccgatcagcggaatgccgagcttcttggcttctgccacggcgatcttgtggaagcccacgtcgatcacgaagatggcatcgggcagcgcggtcatgtcctggatgccgccgatgtccttctcgagcttctcgatttcacgcgagaaggtgagctgctctttcttgctcaggctgtcgaggccggcttcttgctgggccttcatgtccttcaggcgcttgatcgaggtcttgaccgtcttgaagtttgtcagcatgccgccgagccagcgggtgtccacgaaaggcacgccggcacggcgggcttcggcagccacgatttcgcgggcttggcgcttcgtgccgaccatgaggatcgtgccgcggttggcggtgagctgcttggcgtacttcatcgcatcctggaacatcggaagcgacttttccaggttgatgatgtgaatcttgttgcgatggccgaagatgtacggggccatcttggggttccagaagcgggtttggtgaccgaagtggacaccggcttccagcatttcgcgcatggtggtagacattgaaaattcctccaaaggttgggtctaaaatccagcccgttttgcgcctccttcgaatggagtcgcaacaccttgattgggccggtttgcggatgtgtcttgctgtgtgtggcggtagccgtcacacggtcagcgaaacccaaagagtatagcacggccctccctggcttttgtccttgccccgccccgtaaccaagccgtccgcgccccccaaccgcccatgaacgaccttcacgccacccgtctgaatctgttggcaggtggcaccgatgcacgcaccgaattggagcatgccatcggtatcgcccagtctccggcctgcagccacgtcttcacccgcacgctgttcgacgaagcccaccggcaggtcgcgctgccggcgccgcaaagcaggctcgcggggctcgccttcaccgccaaggacctgttcgacatcgaggggcagccaacccccgccggctccgtcgtgctttcgcatgccccggcagccagggccgatgcagtggcggtcgcacggctgcgcgccgcgggcggcgtgctgaccggccgcaccaacatgagcgagttcgctttctcgggcgtgggagtcaacccgcaccatggcacgccggccaacgtgagcgacgccaccacgccgcgcattccggggggttcgtcgtcaggagccgccatttcggtcgcgaccggggcggctttcatcgggctcggctcggacacaggcggctcgatccgcattccggcggcactgaacggcatcgtgggattcaagagcaccgcccgcctcgtgccggccgatggcgcgctgccgctgtcgaccacgctcgacaccgtctgcgccatgacgcgctcggtccgggatgccatcgccgcgcacgagatccttgcggcccgacgtgtgaccgccggcgccgcctcgctgggggcctaccggctcgccgtggtgaaaaacgtgttcttcgacgacatcgagcccgcggtggccagcgccttcgagaacgcgctgcaagcgctgcgcagcgcgggcgcccaggtcgaggaaatcctgctgccggaactggcggagctgcaggccatcaacgccacaggcgggttttcggcggcagagtcctatgcttggcaccggctgctgctggaacgcagcggcgccggctacgacccccgcgtcgctcagcgcatcatccggggcgccgtcatgaaggcgcacgaatacatcgacctcgtgaatgcccggcgcgcatggatcgcccgcgttgaagcggcgctgtcgtctttcgacgccgtgctgtcgccgacggtgccgatcaccgccccctccatcgccagcgtggcgccgggtgccgagcgcgacgacgagttctttcgcgtcaacgcgctgctgctgcgcaatccgtcgatcgtcaacatgctcgacggctgcgccatctcgctgccctgccatgccgccggcgaactgccggtcggcctgatgctgtggcacgccgcgctgcacgacgacgcggttcttgcgattgccctgcaagccgagcacgcactgcgaagacaatagctccacgcccatcgaagggcgtgagccatctcttcttactcaaagattcaatgaaaatcgcgatcgtgggcgccggcatcatcggcgtcaccaccgcctgggaactggtttcggatggccatgaagtctccgtgttcgagcgccgcggcgccgctgccgaggaggccagttttgcgaatgcaggcgtggtcgcgccgggctatgtgacgccttgggcggcgcccggcatgcgggccaaggtgctgcgctccctgctctccccgcacggtgccatcaagctgcgctggccactgagtacgcgcgatctgggctggatgtcgcgctggcagaaggcgtgcaagctcgaaacctaccttgccaaccgcgcccgcatgcaacgcctggcgttctacagccgcacccggctgcacgaggtgaccgaggcacgcgagctgagctacgagcgcagcgacggctacctcgtgctgctgcgctccaagcgcgagaagaaactggtccagcccgggctcgaggtgctgcgcgcggccggcagcgtcttcaaggaagtcgatgccgacgaagcccggcgcatcgaacccgccctcaacaccgacaccgcgctcgcaggcgccatccacctgcccgaagacgaagtagccaactgccgccagttcgcgctgctgctcaagtgggaggccgaggcactcggtgcccaatttcatttcaattgcgacattgcgccgctgagccgcgccgagcccacctccgtctcgctcgcaagcgggtcgccgccgctgcgcttcgatgcggtggtggtgtgcgccgggctcgcctcggcccagctgctgcgcccgctcggcctcaagattccgctggcgccggtgtatggccattccatcagcgcgccgattcgagaatcgctcaacgccccccgcagcgccgtgatggacgaacgctacaaggtcgccatctcgcgcctgggccagcgcgtgcgcgtggccggaagcgccgagatcggcggctcgctgagcaccatgaacccgtccgcggtgcaaacgctctacaaggtgcttcacgactggtttcccggcgcggtcacgctgcagtcgggcgtgcagcaatggaagggtgcgcggccgatgctgcccgatggccctccggtgctcggtgccagtggcgtgccgggcgtgtggctcaacctgggccacggttcgagcggttgggcgctgtcgtgcggcagcgcacgcgtggtggccgacctggtcggtggccgcgatgccggtgtcgacctcgaaggcctgggcgtcgagcggctcagcctctagggttcgccccacccaagcattcggggctcctggtcaagcgcttcatccatcggccgccgagcggcaaaatggcccgatgcaacgcatcacgtccgccaccgccgccgatctgttcgacattgcggcgacgcggcgcatcgagcacgcagccgcggccagcctgccctcccacacgctgatgcagcgcgcgggcttggccgtggcacggctggccatggcgctcgcgccgcacgcacgcacgatctggatcgcctgcgggccgggcaacaacggtggcgatggcttcgaggcggcagcgcagatgcagcaccggggcttccagccggtcgtcacattcacgggcgatgaaaaccgcctgccgccggatgcaaaggcctcgctgcaacacgcgcggaacgccggggtgatcttcgccccgcagccgcctgccacgtatgaactggccatcgatgcgctgctcggcatcggatcgacccggccgcccgaaggcgtcatggccgagtggctgcggcagatgcatgccggggggcaaccggtgctcagcgtcgacctgccctccggtttgaatgccgacacaggggtctggaacgccgcccatccggcggccgacatctcggcttgcgtgaccttcctgaccctgaagccaggcctcttcacggcccaaggccgcgacgcggcaggtacggtctggttcgacgacctgggttgcagcagcatggccgagccgcctgtcgctcgcctggctggcacaccaacgaaccggccgcgcagccacgcatcgcacaagggcagctatggcgatgttgcggtgatcggcggcgcacctggcatggcgggcgccgcactgctcgctggatcggccgcgctgcatgcgggtgccggacgcgtgtttgtcggactgctcgacccgagcgcagcccccgtcgacctgtcacaacccgagctgatgctgcgagacgccaacgcactcgatctttcgggcatgaccgcggtctgcggatgcggcggcggcacagccgtgcgcgcggtgctgccgcgcgtgctggcgacagcggctgcattggtgctcgacgccgatgcgttgaacgcgattgctgccgacagcgggttgcgaatgcagttggcgtcgcgcgcccggcgcggaaagcccaccgtgatcaccccgcacccgctcgaagcggcgcgccttctgaattgctcggccgccgacattcaggcagacaggctcgcagcggcccgcgagttggcgtcgcgctacggcgtggtcgccgtgctcaagggctcgggaacggcgattgccgacggcagcggcgcaccaccggtgctcaatgcgaccggcaacgccaggctcgcgaccgccggcacgggcgacgtactggccggaatgatcggcgccgcgctggcgatgcaaaaaccggccttcgaggcagcgcgcgaagccgtctggcgccacggccgcatcgccgacacgtggccggccaatgcgccgccgctgacggccggcgccttggcgcgccaggcgccgcgctgacgaggttctgtctgctctagccgcgcccgacgaagggcatcttcgttgccatgacggtatggaacagcacgttggcctccagcggcaggttcgccatgtagagcaccgactgacccacgatcttgacgtccatcagcggctcgatggcgagttcgccgttggcttgcggcacccccttggccatgcgcgccgccagttcggtcatggcattgcccacgtcgatctgacccacggcgatgtcgtacttgcgcccgtcgagcgaagcggtcttggtgaggccctccacgccgtgcttggttgcggtgtacgcggccgaattcggccgcggagcggtggccgagatggagccgttgttgatgatgcggccgccgcgcggggtctgcgccttcatcgtgcggaaggcctgctggatgcagaagaacatgccggtcaggttgatgtcgaccaccccgcgccattgctcaggcgtccagtcttcgaacgggcccggcgggttgcccacgccggcgttgttgaacagcaggtccacgcggccgaagcgttccaccgcggcggcgaacagagcctctaccgattcggcgttggccacgtcggtgggcaccgcgaaagcccgtgcgccggcgcccgactcttccgccacctgttccagcggctccaggcggcgcccggccagggtcacgttccagccgtcggccagcaatgccagcgccgcggcgcgtccgatgcccgtgccggcgcccgtgacgatcgcgatgcggcccttgttgttttccacgctcatgttcagtgtctccttctcggtgtgtctgtaggggatgggtgcagtgcgttgcccgtcatgcacggcgaggcttgcgccccttcatcttgttggcagccttcttgaccgccgatttgaaggcctgcatggccgactggggccccaccgcaacggcgctcgcgccgcgttcgctgcgcggctcgggaacggcctcggccttgtggcgcgaactgcgcttggccgatgccttgaccggcacgccggtcgagcccacgcccttgtccttcatggcacgcgcggtgagctcttcgccctcgcgcaccaggcggaaatcgatcttgcgcccgtccaggtcgacacggctcacctgcacccgcacgcgcgtgccgatggcatagcgaatgccggtgcgctcgccgcgcagctcctggcgcatttcgtcgaacttgaaatattcgccgccgagttcggtgatgtgcaccaggccttcgacatacatggcgtcgagcgtgacgaagatgccgaaggtggtggccgccgtgaccacgccgccgtattcctcacccaggtgctcccgcatgtacttgcacttgagccatgcctcgacgtcgcggctggcttcgtcggcgcggcgttcgttggcgctgcaatgcaggccggcagcttcccaggccaggacttccttggttggcgcgacggtggctttctgcggcttggtggttggcgccttgacgcgcgaggccagccgcttggccagcttggcatgcgcctcgcccggcgtcggcagcatcggcagctgatagcgcgtcttgccgagaatggccttgatgacacggtgcaccagcaagtccggataacgccggatcgggctcgtgaagtgggtgtaggcctcgtacgccagaccaaagtggccgctgttgatgggcgtgtagatcgcctgctgcatcgagcgcagcagcatggtgtggatctgctgcgcgtcgggacgctccttggtggcctcggcaatcgcctggaactcaccgggccgcgggtcgtcggtgatgctcaaccccacgcccatggccttcaggtagccgcgcaggatttccttcttctcgggcgtcgggccttcgtgcacgcggaacaggcccgggtgcttgccttcggcgatgaagtcggcgctgcacacgttggcggcgagcatggcttcttcgatgaggcggtgcgcctcgttgcgcgtacgcggcacgatcttctcgatgcggcccgcgtcgtcgcagatgatctgcgtctcggtggtttcgaagtcgaccgcaccacgcttgccgcgctgcttgagcagtgccttgtagacgtcggcgaggttcagcagatccttcacgcggtccttgcgcttggccgcctcggggccgcgcgtgttgccaagaatggcagccacttcggtgtaggtgaagcgggcgtggctgaacatcaccgccggatagaactggtaggcgtagatttcgccgtcggcggccacgagcatgtcgcacaccatgcacaggcgctcgacctcggggttcaacgagcacaagccgttcgaaagcttttccggcagcatcggaataacgcggcgcgggaagtagacactggtggcgcggtcgtacgcgtcgatatcgatcgccgagccggtctgcacataggcgctgacatcggcaatggcaaccagcaggcgccagcccttgccgcggccaaccttcgcgggctcgcagtacacggcgtcgtcgaagtcgcgcgcgtcttcgccgtcgatggtgaccagcggcacgtcggtcaggtcgatgcggcccttcttgtcggcgggccgtaccttctcgggcaacgccttggcctcgaccaggcattccgcggagaactcatgcggcacgccgtacttgcgcacggcaatctcgatctccatgccggggtcgtcgatctcgcccagcacttccttcacgcggcccacgggctggccgaacaaggccggcggctcggtgagctgcacgaccacgacctgccctaccttcgcgggaccggtcgcgcccttggggatcagtacgtcctgtccgtagcgcttgtcctcgggcgcgacgagccagatgccgccttcatgcaacaggcgaccgatgatcggctgctcggggcgttcgacgatttcaaccacccgtccttcgggacgaccgcgccggtcttggcgcaccacgcgcgccttgacgcggtccttgtgcagcaccgcgcgcatctcgttcgggggcagataaatgtcggcctcgccgtcgtcgcgctgcacgaaaccgtgtccatcgcgatgcccttgaacagttccttcaaattcatccagcagaccgctggaatggccattatttttgatatgattctctctttcctgaaattcaaaacataactgcttcggcagctatgtgggcccagatggcggaattggtagacgcactagtttcaggtactagcgagtaacatcgtggaggttcgagtcctcttctgggcaccacccctaccaagctgaaacccctgtgaatcatcgatttacaggggttttttctttgccctgggaacatgatcgagggatgctctccctcgcaaaagccggtcgtgaccaaacaaggcccgaccgacagcaagccgccgctttcgcacacaccttcgcggtccccgttcgagacctcttgcgggattgtttcgggcggcacggattcgaacagatgcaacgggcttcgtcttctcatgaaatgctgcggcagccgctcagggagagcggctttctcgccattctgacgcagtacatcgacgaatgatcgcgcacagtctcaagaagcggggcaaccaatcaatacaccgtgttgccagtaaaggtgaaccgcaaacccaacctgatgggcgcggcgttcaactcgccgaagtgaccacggttggatctgcgggttgcgacggcctgtgaagccgacatgcaccttaccacgccgcagcgtcgcggctccgacgatctggccgccagggctcggcctgccaaactgcgccatagttcgcgccggcacgtcgcgctctccgaatccccactgttcatggccctttttcaaagcatcaggcaatgggcgtcgcgcatcaagcgcgacgccgtcacgctgtggtttgcctaccgccatcccggcacgccctggttcgccaaggcgcttgccgcatttgtcgtcgcctacgcgctgagcccgatcgatctgataccggatttcatccccgtgcttggctatgtcgacgacgtattgctgctgcccgccctcatcgcgctgaacatccggctcattccagccgatgtgctccaggaatgccgcgcgcaggccgacaggtggatgaaagaacaaggctccaagccccgaagcattgcgggcgctgtgatcgtcgttgccatctggatcggcttggccgctggccttttggcgtggttcaacaggcaccgctgagtctgctcgccagggcctcgacaggcattgaatttactgtatatttatacagtcttttcacaaaggataactgcccatgtccgcccctgaagaaaccgctcccgcacgcaaccacgccttggcagaagccttggcatggatttcaaaatttgcccacgcgtggaaggcgatcgaacccgcgcctcgttcgctgagcatcgatggattcatcatctgggggcccgtactctatgaaaagcacggcaaggaggaccccgtggcactcgccgcccagttgtacggcaaatcgggtgactacttcaaatacctctatccgggccgcacgcaggacgcaggcgaagcgcttccgttctagcggttccagccgttacagaaatcgccaggcggcaagtcgcaggacagtcggcccatggattcagacggggaagtcgtggcaaaaatcacactttgccgccaaacatgcgtctaaaagtaaccgaaacgcgcgcacaatgttacctttggtttgtgtaattcaaatttaaggagtcaactgtgatcgcagcatttactttgatcgccggcatgtttcttggcgcgttgttcatgagccttctggtcatctcacgttcggatgactgagagcaaccgggccctgcccgtcccgatcgagcctttttggaaagcccgcttcaagcgggctttccttttggcgggtcagatcggcagcgcaatcaggtcgtggccctcggcacccacgatgcgggccttggtgaattcacccaccttgagcgtcttgctgattttctcgggcggcagcaggcgaacggtgccgtcgatctcgggcgcgtcggcgtaggtacggcccacgccaccttttcggcccatgcccggcgcggaatcgacgagcacctgcatggttgcaccgatgcgctggcgcagcttggcgatcgacaccgcctccgccacttccatgaagcgggcacggcgcgcttcgcgctcggccggcggcagcatgccgggaatgtcgttggccgtggcaccttcgacggggctgtaggcaaagcaaccggcccggtcgatctgcgcctcgcggatgaagtcgagcagatgctcgaactcttgctcggtttcgcccggaaagcccgcaatgaaggtgctgcggatcacgagttcgggacagacctcgcgccaacgcgcgaggcgctccaggttcttctcgccgctggccggccgcttcatgcgcttgagcacgtcggggtggctgtgctgcagcggcacgtccaggtaaggcagcacctgcccgctcgccatcagcggaatgatttcgtccacgctcggatacgggtacacgtagtgcagccgaacccaggcgccgtagggctccgcgatttcgcccagcgtgcgcaccagttcgagcatgcgcgtcttgaccggcttgccgtcccagaaaccggtacggtacttcacgtcgacgccataggccgaggtgtcctggctgatgaccagcagttctctcacgccgccttcgaacagtgccttggcctcgccgagcacgtcgccgacaggacgcgacaccagatcgccacgcatcgacgggatgatgcagaaggtgcagcggtgattgcagccttcgctgatcttcaggtacgcatagtgccgcggcgtgagcttgaggcctgcgatgccgaaagtgttgggcaccaggtcgatgaagggatcgtgcggcttgggcaggttggcgtggaccgcatccatgacctcctgcgtggcgtgcggaccggtcacggccagcacgctgggatgcatctgccgcaccaggttgccgccctggtcgccggtcttggcgcccaggcagcccgtgacgatcacgcggccgttttccgccaatgcctcgccgatggtgtcgaggctttccttcacggcatcgtcgatgaagccgcaggtgttgacgatcaccaggtcggcgccttcgaaggtctttgccgtctggtagccctcggcgctcaactgggtcaggatcagttcggaatcggtcagggccttgggacagcccaggctcacgaagccgactttgggggcagccggcgtggccgtacgttcaggggaggcaacttcgctcatatgcctctattgtcccagctatcggacgggaccgggatttcaggggcgtttgatgccgaatgcacccagaacctgctcggtattcttctgcatctgttcctgcatttgcaggaacacgttcttggactgctcgacgtagttgcccatcagtccctggagcatcggcgactgcagggtcatgaagcgcgaccacatttcgggcgtgaggccttcggccttttcggtgagctgggcctgcacttcggtcatggcctggatgttcttctcgagatacgggcccatgtagccctgcatcgcctgtccgtagaaacggatgatgttggacaacacctgctcggtgaacatcggcgcgccacccgcttcttcttcgaggatgatctgcagcaggatgcttcgcgtgaggtcgtcgcccgttttggcatcgcgcaccacgaactgggcgttctgtatgaccagctgcttcacctcggtcagggtgatgtaggtggatgtctcggtgtcgtagagccttcggttggggtacttcttgattacacgttgcaccggcttgaccccggacttcttgctctgcactgcggactccttcacatggatgcccatgtcatccgatcaattctaggtagcggttttgctgcatcgcgacaaggtttaccctgaccgcccttcggccagcgaatccgcgtccttcttcagtcgagcgttgtggcgtattcggcgccgcatgcggcgcaggtcgccgtctcggggcgatcttccgtggcctctcgaaaacgcaagggactcttgtggccgtagacgacccagcagcgcggacagtgctcctggccggaggtcggcagataggcgcgagcacgctgttcggcgcgctcttgcgtcacgggcatgccctgccgctgggcgcgcgccacctcgcgcgcagccatggtgtcggtgcggccgcctgcgtggtcgttgatgccatagaccgcgcgcgcaaattcaatgggggcttgcctgagcaatgcggccaagcgcttggcggcatgagcccgatcaaccagcgttgatcgcgtattcatcagatcgcttgtcaagaaaattggaaaaggtttgcagtgtggccaaggtagcacaacaatgtggccatggtctttgtctgcttcaccgcagggacgattgagacaccggggaacccggtgaaagctctgttcaacagacccggtggttggccggatgttggaacagaaattggtaggcgcgattggactcgaaccaacgacccccaccatgtcaaggtggtgctctaaccagctgagctacgcgcctaaggatgtgtccgagaagcagctattgtagcaggagaaaacgcgctttttagcgccgacgtgcagatcgcacaccagccactgccgtcacgatgcccagcacctgcgtcagccgcgctgcgtctgtgatctctacagtgaacgtcatccatgccgtgcccttgaccgattgcgtctgcacgccgatcacattcatcttctcgcgtgcgaagacatcggagatgtcgcgcaagaggccctggcggtccgccgcttccacggccacgtcgaccgcatagaccggcgcctcgccacccttcttggccgctccccattcgacatcgatgacgcgctcgccgtcgcgcgcggccatcgtgcgaaagttgctgcaatcggtgcgatgcacgctcacgccatgaccgcgggtcacgaagccgctgatgggatcgggcggtgccggcttgcagcacttggcaagctgcgtcatcaatgaagacacgcccaccaccagcacaccgcccttgccggatttttcgctcgcgcgcggcttcttgatctgcacgccgtcgtccggattgggcgcgggctccggcgggcgcagcagcacctcgatgttgcgcagcgagaactcgtccttgccgaccacttcgaacaaatggtccgccgacttgaagcccagctgcgaagccaggtcctcgagccgcgtggaagtcttgccttcgcgctgcagcagcttctcgacggcttcgcgtccgcgcgccacggtctcgtgcgtgatctgcgcgttgaaccacgcgcgcaccttggctcgcgcgcggtggctggcaaggtagcccagctcggcattgagccagtcgcgcgacgggccgccctccttggccgcgatgatctccaccgtctgtccgttggacagcggcgtgttgagcggcaccatcgcgccatcgacgcgcgcgccgcggcacctgtggccgagcgtcgtgtgcacggtgtaggcaaagtcgaccggcgtcgcgccctgcggcagctcgacaatggccgcgtccggcgtcagcacgtagatgcggtcgtcgaacagcccctgcccctgcgagccgcccgaaagatcgcgctcccatgccaggagctgccgcagcacggcgatcttcgcgtcgtactctccgctcgcccacacgcccgcatagcccttgtgcccggcttccttgtaggcccagtgcgccgccacgccgtgctcggcatggtcatgcatttcttccgtgcgaatctggatctcgatcggcttgccgggcttgccgtcgaccatctcgcgcaccacggtgtgcagcgactgatagccgttgggcttgggccgcgcaatgtagtcgtcgaactcctcgtcgatcggcaggaaatgcgaatgcacccaggccagcgccgcgtagcaatccttcacgtcgggcaccaccacgcgcagcgcgaggatgtcgaacacctgcgcgaagtcgagcgacttgccgcgcatcttcttgacgatgctgtagatgttcttcggccgcccctgcacgatggcgcgcacgccctcggcctgcagctcgctttcgagctgcgagcgcagctgctcgacatggccttcgcgctcgacccgcttctcgtcgagcaggcgtgcaatcagcttgtaggtttcgggttccaggaagcggaacgagagatcctcgatctcccacttcacctgccagatgccgagccggttggccagcggcgcaaacacctgcagcgactcgcgcgccacgctctcgggcgccggccgcttgctggccgcggcatgccgcaaggtctgcagccgcgacgccaggcgcagcatgaccacgcgcaggtcgcgcgaaaacgcgagcagcatcttgcgcacgttttcagtttgcgcgcccgcgccttccgacaggtgatggccctgcgaagccgagcgggcctgctcctgcacgcggaccagcttggtggtttcgaccgccagcgccgcaaagttgtcgccgaacaccttggcaatcacttcctgcgggcggttcaggtgctggcaggcatagaccagatagctcgcggcctgcatggcctcggagccgcccatctttgcgacgatggccgccacggcatcggcgtgcgccagcgtgttctcgccggtgtcgagcttttcgtcggcaatcaacggctcggcaaatgcgcgcgcacgggcgagcatgttctccatcaccggagtgcgatccgccgtggcggcggacagcggatagtccgccactgccgaatcgggagagtgtgccgtttgaaggctcgaagaatcgcgcttcacgctgccctcaatcgaacaggaaggatgtgacagccaggacctgcgcagggtcgacgaaggtgggcgcatggcccacgccttcgaattcgatcagcgccgcgcgaggcccgcgctgcgtcatggccagcgccgtttcgtgcgacagcagatccgactgggcgccacgcgtcaccagggttttcgcctcgatggcgtcgtacaggctccacatcaccgcgccgccctgggccgcggcctcgggcgtgacggcgcgcagcgacacggcaatggccgggtcgtagtggagcaggcagggaccggcttcgccgccgccggcttcgtcggcctccagcttgcacgcaccatcggccgtgcgccgggatgccggcaccaccatgtgcctggacagtgaaagccattgctcaggcgtatgggggccgaagctggtcgaaattgcccacatggcgtccgccgcttccttcaggctcgcatagcggccgccctgccccacgtagccgccaatgcgctggatggccacggcctcgatcgtcgggccgacgtcgttcacgatgaaacggcgtatgggttggggcagcggcaattgcttgtggccggccagcacgaaaccgatgagtccgcccatgctggtacccagatagtcgagcgtctcgatcggctgttcgcgatgcagttgcgccaggagggccaccatgtcggccgcatagaccggcacctggtagagcgccggatcgcgcagccagtcgcttcggccacgccctgcgacatcgggacagaccacacgcacgtcgccgccggcacgcgccacgatggcctgggccagcacgtcgaaatcgcgcccctggcgggtcaggccgtgcacgcacatcaccacacgcgcactgcgcgcgctgccccattgccaataggccatgcgatgcccgccttgggggtcgtcgcacgccacgtaatgaagcgtcggttctgtcatgaaaacgaagtcgtcctggtgcggataatgtctcgtcgcatcctaattcatccggagattgaacttcatgctcaaaggcaaaaccgcgcttgtcacggggtccaccagcggcattggccttgccattgccgaggcacttgcacaacaaggcgcgcacatcgtgctcaacggcttcggcgatgccgaggcgcccaaggcccgcatcgaagcgctcggcgtgcgtgccgaataccacggcgccgacatgagcaagcccgaccagatcgaggacatgatgaagttcgccgcgtccaggttcggccgagtcgacatcctcgtcaacaacgccggcatccagcacgtggcaaaggtcgaggactttccgccagagcgctgggacgccatcatcgcaatcaacctcacgagcgcgttccacacgacgcggctcgcgattccggccatgcgcgaagccaattggggacgcatcgtcaatgttgcgtcggcccacgggctggtcgcctcggcgcagaagtccgcctacgtggcggccaagcacggcatcgtcggcttcaccaagtcggtagcgctcgaaaccgcgaccaccggcatcaccagcaatgcaatctgcccgggctgggtgctgacccaactggtgcaaaagcagatcgacgaccgcgcggcacgcgaaggcatctcggccacgcaggcgcaaaacgaactgctcggagaaaaacagccttcgctgcagttcaccacggtagagcagctcggcgggctggcggtgttcttgtgctcgccggcggccgaccaggtccgcggcgtggcctggcaaatggacggcggctggaccgcgcagtgatcgaaggggagcggcccgcgccctcccccacgcctgcctggccctctacttgagctgcacagaacccgacacgttcaccaccacgctggtcttcccggcttccaccggcaccggcgcatcgggagaaaaagacttggccgatgccgccatgacgcgcggccggatcgggccgctgtcgttcgcgttcaccgagacctcgcgcagcgtgtagcccgcaaagccgaagcccttggccagctccgtggccttctgcttgaagttctcgatggcgatggtctgggcctcggtctcgcttttggcgcgctgctcgcggctcagtgcaaagccgacgtttccgacgttgagcgtggtgatgcggcccgcggtctgcgtgatgcgcgggaagtcgcggccctcgagcaccatttcagcggagccctgccagccgttgatctttccttcgcgggtgtagcgcggcgacaggctgaagttgccggtgcgcacgtcgagctgaccgggttgggcattctttttggcttcggccagcgcggcgtccaccgcagccttgagctgcgactggaccgtggcggcatcggtcgcgtcgcgggtggtggtgagcgtcatgctcagcagatcctgctgcacttcgaccgtgccggaggcagtgagctgcagcacgttctgcggcggcggggccatgttctgggctgtggcgctgcctgcggccgctgccgcggccaacgcggcgcaggccgcgatccaactgattttcttcaagacgagttaccccctggattggtattcaatgaacgcaaaaaaagcgcgccgcgccgcttcagcggcgctggctgcggggcaaggtcaacgcgcgggccgccgacatcggcggcggcgcgattcgctcggccggctgcgattctgccgaattcattgccctggggggtgtgccgggcggcgcccactggccgcgcacctgctggcgcaactcgaagagttcggccgccgtcaggcgcctgccggccgccgcctcctccctgcggatctcggcgcgctgcgacgcgcggtgagccgccaccgcctcgcgaacctcgctgcggcgcgaatccccgaccttgaggaattcgccagccgtggccagggtggagccgcagctgcaggcaacgaggatcggcaacgcggaaaagagggttctcattgaacagaagtcataggacaagtggactttgccaccgcgggacgaaggtcggatggctagacagctagcgaccgcaagttttgtaacttagtgtcaaaccataagtaaaactggctcagcggcggctcaacgccttcagaatcgacgctgttacaaattcaacgttgtagaaatgactcaagttcccgctcgcactgacaagatcgtgatcgtcgacgacgacgcccgcatccgcgacctgcttcgccgctacctgacccaggaaggtttcgaagtgatcgtggccgaggacggcaaggcgctcaaccgcatcctgttgcgcgacacggtcgatttgatcgtgctcgacctgatgatgcccggcgaggacggcctctcggtctgccgccgcctgcgcgccgccaacgaccgcacgccgatcatcatgctcaccgccaagggcgaagacgtcgaccgcatcgtcggtctcgaggtcggcgccgacgactaccttggcaagcccttcaacccccgcgaactgctggcgcgcgtgcacgccgtgctgcgccgccgtccgccgctcgaggcgcccggtgcgccttccaccgagaacgaaaccgtcactttcggcccgttcgccttcgacctcgggtcgcgcacgctcaagaaggacggcgaagagctctccctgaccaccggcgagttcgcgatgctgaaagcgctggtgcgccatccgcgccagccgctctcgcgcgaaaaactggcccagctggcacgcggccgcgaattcgagcccttcgaccgcagcctcgacgtgcagatctcgcgcctgcgcaagctggtcgaggccgacgccgcggcgccccgctacatccagacggtgtggggcgtgggctatgtcttcgtgccggacggcacggcctgacgacatcccgaggtggccatcggcctgaattcagccagacccagcccagcccaggaggacggcgcccaggtcacgatgccgagccctctggagggcgccggccagcgtgaccggcaaccgggcctcaagctcggcttcagccttttctggcgcacatttttcctgctcgcgctgttgctggtcggttgcacggtcgcgtggctgcagacctttcgctcgctcgaatacgagccccgcgccatccagacggcgcaccagatcgcctcgctcgtgaacctcacgcgcgccgcgctggtgtattcggacgcgatcacgcgggtgtcgctgatcaagacgctggccgatcaggaaggcgtgcgcatcctgccgcgcgaacccaacgaccgcttccagccctacaccagcggcgcgctcgaccagcgcgtcaccgaggagctgatcgaccagctcggcgaaggcaccaccgtggccagccgcgtcaacgacgagcccggcctgtggatcggcttcaccatcgaaagcgacgcctactggctgctgctcgacccgacccgcttcagccgcgtggggggccgcacgtggctggtctggctcagcaccgccatggccttgtccctggccggcgcagcgctgatcacccggctcatcaacctgccgctcaaacagctgtcgcgcgccaccatgcaggtgcgcgaaggcgagtacgaggcgcaccggctcgacgaaagcgcgcgcaccaacgagatccgcgcagtcaacatcggcttcaaccgcatggccgaccagctcgccaagatcgagcaggaccgcgccatcatgctggccggcatctcgcacgacctgcgcaccccgctggcgcgcttgcgactggaaaccgagatgagcgtggccgacgaagacgcacgcgaccacatggcggccgacatcgcccagctcgacgcgatcatcgacaagttcctcgactacgcacggcccgatcacgtcgatcccaagcccgtgctgctgcgcgacgtggtcgatgcctgcacctatgccgtgcaggactacgaagaaatgaagatccgggtcgacgtgccgtccgacctccgtgtgctgggcgacgaggtcgaactcacccgcgtgatctccaacctggtggagaacgcgcggcgctacggcaagacgccttccaccggcgtggccgacgtggtgatccaggcccaggccaacaacgacgcggtgctgatcaaggtacgcgaccacggcgcgggcgtcgagcccgccctgctctcgcaactgaccaagccattcttccgcggcgacgtggcacgcacatccgccgccggcgccggcctcggcctgtcgatcgtggccaagaacatcgagcgcatgggcggcacctttgcgctcaccagcacgccggggcgtggcctggcggcgcacatccgcatgccgcgcgccatgcccgaacccaggcccgtcgaagccccggtccggcgcgcctgactcagcggtgcagcagcaccaccgcgcgagcttccatcgcgcggccctcaccgaccggcccgagcttttcggccgtcttggccttcacgttgacctggtcgggcgcaaggcccagcgccgttgcaatgcgctggcgcatggccgggatgtgcggcgccagcttgggcgcctgcgcgatcaccgtgctgtcgacgttgccgatctcccagcccgcggcacgcacgcggcgcgccgcctcgccaagcagcacggccgagtcggcgccgcgaaactgcgcatcggtgtcgggaaaatgccgtccgatgtcgcccaggcccgccgcgcccagcaatgcgtcggtgatggcatgcagcagcacgtcggcatcagaatggcccaggaggccggtggtgtgcggcacctcgacaccgcccaggatcagcttgcgccccgccaccagttggtgaacgtcccagccctcgccgacgcggatgttgaacgacgcgctcatgccctgcctttcttgcggcccagcaataccgcttcggccagcgcaaagtcttcaggaaaagtcaccttgaaattctgcgcgctgcccggcaccagcagcggcgcaaggccgatggcctcgatggcaccggcttcgtccgtcaccgaatcgcccacgcgctccagcgcatcgagcagcatgccgatgcggaacatctgcggcgtctgggccagccacttgtcggcgcgcggcagcgtctgcgacacccggctttcggccgatgacaccttgagcgtgtcagccaggcgctgggccagcagaccaccgatggcatcgtgctcgcaggcggcgatcagcgcctcgatctggctcgacgtgaccaggcagcgcgcggcgtcgtgcaccagcacccagtcgtgcgcgccggccccttttttccgcagcgcggccaagccgttgcgcaccgtggccgcgcgcgtgacgccgcccacctgcagcaggaactcgcccgtggccggaaagcgcggcagcgccgcctgcacgtccctgtcgtccggcgccacaaccaccgccaggcctgcaaagcggcccgccagcgcacggaacgcctccaccgtgtgagccaccaaggacgcgcccgcaaggcgctggtattgcttgggcagcgcaccgcccgcgcggtgccccgagccggcgcaaggaatcagaacgaaaagacgggaggaagacatgggctccggcaccgggcgacggccggcaagcgaacaaggggccgccattctagaatcgaccatctcacacccctcgccagcggcgcggggtgttctgcattttcataagggtctgctcacgctatgcaaggggtcgcgaagctcgccacagcccgcccatcaaggcgcgtgacgccgtgcgtgcgtctgcacgcacaaggaacgcaacgccgaagggcgggctgtggcgagcttccctccgggttgcttcgcaaaggggccgtctgcggcgttgcccgcgcttgcaaggcgcgagccttgctgcgcgcgggcgccttgcagccagcccctttgtgaagcaacgcgaccccttgcatagtgtgaacagaccctaggcgttccatggacctcccccacctcacggcgggcaagcgattcacgctgccgcgtcctcccttgtcggccgatgcgctgctgctggcgcagctgggcatgcgcgaaaaggccgcgggccgcgccaccgcggtgttcacggcggacgccaacgacgcccagcgcctgatcgacgagatcgcgttcttcgcgcccgacttgcgctgcgccctgttccctgactgggaaacgctgccctacgacagcttttccccgcaccaggacctgatcagcgagcggctcgccacgctctggcgcatcagccagaaggaggccgacgtggtgctggtgcccgccaccaccgcgctctaccggctggcgccgccggccttcctggccggctacacctttcacttcaaggccaagcagaagctcgaggaatcgaagctcaaggcccagctcacgctggccggctacagccatgtgacgcaggtggtgagcccgggcgaatacgcggtgcgcggcggcctcatcgacctgtttcccatgggctcgccggtgccctttcgcgtcgacctgttcgacgacgagatcgactccatccgcaccttcgaccccgacacccagcgcagcctctaccccgttcccgaggtgcgcctgctgccgggccgcgagttcccgatggacgacgacgcccgcgcgcgctttcgcagccgctggcgcgagctgctcgagggcgatccgaccaagagccgcatctacaaggacatgggcaacggcgtggccaccgccggcatcgagtactacctgccgctgttcttcgacgagacggccacggtgttcgactacttcggtcccgacgccaccgtggtgctgcatggcgatctcgaacccgcgttccagcatttctggcaagacaccaatgagcgcttccgcctggtgcgcggcgacccagagcgcccggcgctgccgcccgaggcgctgttcctcaatgccgagcagttctaccaacgcgccaagccgcatgcgcagctcgccattcgaggcgacatcgccaccgaaacgccttacgccgagttcgacaggctcccgtcgttcgcggtggtgcgcggcgccgaagacccgctggtcggcctcaaggcccacatcaaggcaaccccgcaccgggtgctgctgattgccgaaagcgaaggccggcgcgaaagcctgctcgacttcctgcgcgccagcggcgtgagcccgccggctttcgactcgctggccgagttcgaggcatcgaccgacgaaaaaatcggcatcgccaccgccgcgctggcctcgggcttcgcatggcgcgaacagggcatcgacctcgtcaccgagaccgagctcttcgccaccgcgcccaccacccgccgccgcaacaagaagcaggaacaggtcagcgacgtcgaggcgctgatcaaggacctttccgagctgaacgtgggcgacccggtggtccacaccgcccacggcatcggccgctaccgcggcctgatccacatggacctgggccagggcaccgacgccgaaggcaagccgctgctgcaggaaatgctgcacctggagtacgccgacaaggccacactctacgtgcccgtttcgcagttgcaccagatcagccgctacaccggcgtcagcgccgacgaggctccgctgcacaggctgggctccggccaatgggaaaaggccaagcgcaaggccgccgaacaggtgcgcgactccgccgccgaactgctcaacatctacgcgcgccgcgccgcgcgccagggccatgcgttccgctattcggccgccgactacgaggtgttcgccaacgacttcggcttccaggaaacggccgaccagaaggccgcgatccacgccgtggtgcaggacatgatctcgccgcagccgatggaccggctggtctgcggcgacgtgggtttcggcaagaccgaagtcgccctgcgcgcggcgttcatcgccatcaccggcggcaagcaggtggcgtttctcgcgcccaccacgctgctggccgagcagcactaccagacgctggtcgaccgcttcgccaagtggccggtcaaggtggcggaaatgagccgcttccgttcggccaaggaaattaccgcggcggccaagggcctggccgaaggcacggtcgacatcgtggtcggcacgcacaagttgctgtcgccgtcgatcaagttcaagaacctgggcctgctcatcatcgacgaggagcaccgcttcggcgtgcgccacaaggaggcgatgaaggccatgcgggccgaggtcgacgtgctcacgctcacggccacgcccattccgcgcacgctgggcatggcgctcgaaggcctgcgcgacctgagcgtgattgccaccgcgccgcagcggcgcctggccatcaagaccttcgtgcgcaacgagggcaccggcgtgatccgcgaagccgtgctgcgcgaattgaagcgcggcgggcaggtctacttcctgcacaacgaggtcgagaccatcgagaaccggcgccagaagctcgaagagattcttcccgaggcccgcattgccgtggcccatggccagatgcccgaacgcgagctggaacgcgtgatgcgcgacttcgtggcgcagcgctacaacctcttgctgtgctcgaccatcatcgagaccggcatcgacgtgccgaccgccaacaccatcgtgatgagccgcgccgacaagttcggcctggcgcagctgcaccagctgcgcggccgcgtcggacgatcgcaccaccaggcctatgcgtacctgatggtgccggacaccgagggcctcaccaagcaggcggcgcagcggctggacgccatccagcagatggaagaactgggctcgggcttctaccttgcgatgcacgacctggagatgcgcggcactggcgaagtgctgggcgagaaccagagcggcaacatgatggagatcggcttccagctctacaacgagatgctgagcgaagccgtgcgcgcgctcaaggccggacaggagcccgacctgctcgcgccgctgtcggtcacgaccgagatcaacctgcatgcccccgccctgctgcccgacgactactgcggcgacgtgcatctgcgcctgtcgttctacaagaagctggccaccgccaagacacccgaccagatcgacacgctgctggaagaaatcgtcgaccgcttcggcaagctgccgccgcaggcgcagacgctgatcgacacgcaccggctgcgcgtgctggcgcggccttacggcgtggtcaaggtcgatgcggcgccgggcgtgatccacatcaccttcaagaaagacccgccggtcgattcgatggccatcattcacctgatccagaagaacaagcacatcaagctcgcgggcaacgaaaagctgcgcatcgagcgcgaactcaaggaaccgaaggagcgtgcgcaaatggtgcgcgacgtattgcgcagcctcggccaacccatcgtcaaggaaactgttcccgcatgaacgccatcgaaatttctcccggcctcgtcgtccagcgcgtgaagccgccgctggcgctggccgatttcaagctgatcgcgttcgacatggactcgacgctgatcaacatcgaatgcatcgacgagatcgccgatgccgtcggcaagaaggccgaggtggccgccatcaccgaagccacgatgcgcggcgagatcaaggacttcaaggaaagcctgcgccgccgcgtggcactgctgaagggcgtgccggtcgaggcgctgcagcaggtgtacgacgagcgcctgaagctcaatccgggcgcggccgaactggtggcagcgtgcaaggcggcgggcctcaaggtgctgctggtctcgggcggcttcaccttctttgccaaccgcgtgaaagaccgcctgggcatcgacttcgcgcgttccaacctgctggacgaagccgacggccgccttaccggccaggtggtgcagcaaagctggggcgacatctgcgacggtgccgaaaagcgccgaacgctgctcgaagtcgcatcgctcatgggcatttcgccgcaagaggccatcgccgtgggcgacggcgccaacgacctgccgatgatgggtgaagccggcctctcggtggcgtatcacgccaagccgaaggtgcgtgagcaggccatggtggcgatcaacgaaggcggcctcgacagagtgctggagatcctgaaatgaacgacgacaccaccccgctctacagcgctgacgcactcagagactacggcagcgcattgctgcagaaggccggcctcgctgcatcgatggccgacagcgtcgcccgcacgctggtcgaaggcgacctgctgggccacgacacgcacggcctcgccctgctggccggctatgtgaaggaaatcgaatcgggcggcatgacgcgcgacggttcgcccgaggtgctgtcggaccgcccggcggccgtgctgtgggacggcaagcgcctgcccggcccctggctcatggaccagggcctggacctgctgctgccgcgtgcgcgcgagctcggcaccgcctcgctcgtgatccgccgcagccaccacatcgcctgtctcgcggtctacatgctgcgtgcactgcaggaagacatgctgatgctgctggcgtgctccgaccccaatgcggccagcgtcgcgcccttcggcggcacgcaggccgtgttcacgccgaatccgctggccatgggctttccgctgtcgcagggcggcgtgatggtcgacatctcggcctccatcaccaccaacggaatgagcaaccgcaagcgcgcggctggcgagacctttgccgaggaatggctgatcgatgcggccggcaagccgaccaacaacccgcaggtgctgttcgaccagccgcccggcacgctgctgcccgtcggaggcctgagccacggccacaagggttacggcatggcgctgctggtcgagacgctgacggccggcctcgcgggccacggacgggccgatccgcccgaaggctggggcgcgacggtccacgtcacgctgcacgatctgcatgcgttcggcggcaaggaagcttttctgcgccagatggaccacgtggcggcgcagtgccgcaccaacacgcccatcgatcctgcgaagccggtgcggctgcccggagaaggcggcttgaagcgccgcgaagcgcaatcgaagaacggagtgcgcctgcatccgtcgatcgcgcgttcgctgcaggacgcggagcagcgccacggccttcaactggcccaggcgctgatctgaagggctagatttcctcgggtggttcttccgcccgctccccggccgggcgcggtgcgcgcttgccgggcttggccaggatctcgacatggaactgcttgccggcgtccttgacgacgccgtcgatcaggcccgtgatggccgaaagatgtacggtttcggcggtttccgccgagttgccgaacttgcaatcgaagtcccagaagtcgctgccttcgggcaggacgcggcgccgctcgcgcttgatgtacttgcggatctcgtgcttgatggcttcgaggagacggtcggggtgcttgccctcgacctgaagctgaaaggtttttctcatgggtgatggtaaccaatgccacccggctgtcctgtgtacagtcggcggctcaacggaaaacaggtgaacgacatggcgcgcgcaaacgactgggcaagcaaggtaatggcattggtcaacggtggcaatgcatcggcggccatcgcgcagatcaaggtcgcgccctcggtcaaggacctgaaggcgcttcagacgatcatgacgctatcgaaaatgaaaggccgtcatccgaacgtggatgcggccattgcggagaacctggcgctgctggcggcgccgcggctgcaccgctcgccctgagcgaagactacgaagactacagggcttggccgaggcgcttcacgccctcttcgatcttcgccacatccgccgtcgcaaagctcaaccgcagcgtcgccatgtcgggcttctcggcatagaacggcgctccgggcacgaaggccacgagctgctcgatggcgcgctttgccagttcgcccgcatcggccagcttgccgttggcgcccgtgaggcgggcccagaagaacaggccgccctgcggctgcgtgaagctcacggcgtcgcccagctcgcgcttgagcgccgcgcccatggcctgcgcgcgctggccgtacacctcgcgcacatgcgccagcgtgccgggcatgcggccgctcttgaggtattgcgcggccgtggcctgggcaaaggtgctggtgtgcgcatcgctgaactgcttgcacatggtcgccttggccagcagttcggcgggcgcgatcatccagccgatgcgcagccccgggctcagcaccttgctcaggctgccgcagtgcgccagcaattcgcggctgcccggcacgtccttgctcagagccaggatcgaaggcggcggggcctcgccgaagtaaaggtcgccgtaggggtcgtcctcgacgatcagcgtctggtacttgaccgccagctcgagcaccttcttgcggcgctccagcgtcagcatggcgccgctcgggttgccgaaggtgggaatcaggtagacgaacttgggcttgtgctcggcaatgagtttttcgagctcgtcggtcttcacgccgttggcgtcgatgggcgcgctgatgagctgcgcgccatacaggcgaaagcactggatcgtggccaggaaggtcgggccttcgacgatcaccttgtcgccgggcgagatcatggtcttgcccagcaggtcgagcgcctgctggctaccggtggtgacgatcaggccgctggggtccacgtcgacgcccttggtcttcatgaaggcgctgagctgggtgcgcagcggctcgtagccttcggtggcgccgtattgcagcgcgccgccgggttcttcggtcagtgccttgttgctcgcctccttcaagccctcgacgtcgaacatggcgctgtcggggaacccgcctgcaaagctgatgatcccgggcttgcccaggagtttgaagagttcgcggatggcggaggtttcgacgttgtcgaggcgggaagcgaattgcatggaggttctcactttctggacgccattgtcgcgaaagccgcgggcaataaagctgcgtaaggctatcgcctttcaacgatatattgcgtctatcgcgcccctgcccggcatggccgacgagcgctgcgtttcccggaccccatgaaaaaagacaacattcccctcttcttcgccaccctgcaggcggccaatcccacccccgaaaccgagctcgaatacgccacgccgttcgaactgctggccgccgtgctgctctcggcgcaagccaccgacgtgggcgtgaacaaggcgacgcgcaagctttttccggtggcgaacacgccgcaggcgatcctccggctgggggtggaaggcctggaggaatacatcaagaccatcgggctttaccgcagcaaggccaagcacctgatcgagacctgccgcatgctggtggaactgcatggcggcgaagtgccgcgcacgcgcgccgaactcgaggcactgccgggggtcggccgcaagaccgccaacgtggtgctcaacgtcgcgttcggcgaggccaccatcgcggtcgacacgcacatcttccgcgtcggcaaccgcaccgggctcgcgccgggcaagacgccgctcgaagtggagctcaagctcgagaagcgggtgcctttcgagtttcgcctgcatgcgcaccactggctcatcctgcatgggcgctacatctgcgtggcacgcacgccgaaatgctgggaatgcgcggtggcgccctactgcgactacaaaccgaagacgccgcggcccaagtcggcctgaacccggcccgagcctcgcctgttctccggctacatctcgaacgcctcgacctgccggccgtcgatgtcggtaaagccgtactcgcgcgccaggtcggccacgcgatgcacgccgccgctcttctccagcacccgcgaatcgcccgccagcgcagcgacggcgcggccgagatagcgcggcgactcggtccgcgccagcgccgggcgctcgtgccaatgtgcctcgtcggtcttgtggccggccagcacgaactcggttcgcatccagcccggcgacaccgcaagcgaagcgacgccgtgcggacgcagctcctgcgccatgccgaaggccagccgcgtcatggcggacttggcgaggtcatagaacaggttgccacgcaggtagttgccgcggtcccagaaggtggtggtcacgacgagcccgctcttctgcgacaccatgatcggcgcggcgcacctgctggccagcaggtggttgcgcacgccgcggtcgaacatcgagtcccagttggaaagcggatgctcccagaacggcgcctcgaacacgccggtgaaagtctcgtggccgccccacgcgttgttgacgagcagatcgacacggccctgctcgcgctgcacctgcgcaaagagctgcttcacctcgtcttcgtgcgtgtgatcgcagcgcaccgcaatgccgcgtccgccgaggcgggtgacttcgtcggcggtttcgtcgatgctgcccggcagggcttcgagctccgagagggcgagcaactggccgtaggtggtcgccggctgctcccgcgtgcttcgccccgtgacatacacggtggcgcccgcggcgccgagttccaccgcgatgccgcggccggcaccgcggctggcgccggtcaccacggccacatggcctttcaacggctggtcattgttttcggcatgcattggttttttcctttcgttccgagttcgaagcgacagtaaggccgcctcaacccgccgtcttggaagaacccgaaatcgcgcggcccagaaactccgtcggcgtgagaccgcagagcgcctggaactcgttgaccaggtgcgattggtcatagaaaccaccgtccagcgcaaggctcgcccaggcgggcgcgcgctgcaggcgcaaggcgcgcaggcaggcatgcaaccgcgcgagccggctccaggcacggggcggcaaccccacctgctgctgaaagacctgctgcagccgccgctcgccgagcccgacggccgccgccacctcgcgcagcggacgccgtccccccgacgccgcaatgagttgcgccgcgcgcatcgcggccgggtgaacggtggcatcgccatcggccagttgccgctgcagtgcggcgcagagcaccgacacgcgcgaggcgtcgtccggctgcccagccatgcgctccagcagttcggcaccacggccgtgccacagttcgtccaggtgcacggcggtgccggcgatctcgctggccggcattcccaacagggccgcggccgcgccggggcgcagggttaccgacagtccttccatctttcggcggaggcgcaccaggaccggggctgcggaagcgcccagggcctcgacagcttgcccggcgctttcgtccgccgacggcgcatcgcccagattgaagacaaggcgcaccgccccatcgggcagcacgcgctcgacaacctcatggccttcgggcagcgcttccctgtagagaagaatgtgcgcgacatgcgccgcgagcggtgccgcaaccggaaaggcgcacaacgttcccgcgggcatgtcggcctccggcccgtgcaaggggtcgccgtcgaggcgtatgtacaggcgttcgttcgtggaggggttcggcatcgcggtgacggcggcagaccgccttgtcgctttccatcagccgcattcgatcagctggcatgccccgtagtcaatgggcgccgacggccattgcgtggcgtcgtcgacgcgccgcacgccgcggtgcagcagttgcacggcgcgcatcacgcctgcatgcgtgacccacaccgcgtcttgccccgacacgcgccaatcgtcgaaggcagcgcccgtgcgttgcagaaagcgcgccgtgctttcgccgtggccgcccggaagcccctcggcgaaattgcaggtccacgcgtcgaactcggtgcgagcgatggacgaccagggccggccttcccaggcgccgaaatccatttcgaccaagcgcgcatcggcccgcatcacgagatcggggcgcagcgtgccgatggcctgtgccaactcggcacaacgccgcaagggcgagtggaccagcgcgatgccttccggtatgccggacaccaccgcgtgcgccaccgccagcgatgctccggccggcacgcccacgtccgccctgccgtagcaaaggcccggcgcggcgtcggtctcagcatggcgcaccagccacagcttcatgcctgccacgccagcgcaagatagatcgcaagctcgcacacctgctgcgtcgcaccgagcccgtcgccggtgaacccctgcagccggcgccggaacatgcgcgccatcaccagcgccgcaagagcgcatgccaccgccacggcgagcgttctcgcggggccctgcgtcagcagcaccagcccggcagcaggcaccgaccagagcacgccaaccagcaaggcaccaccgccgattgcatcggccagcggcttggccttgctcgcgccggcatcgcccacgtagggcaaccagcgaatcaggaacagcggcgccagccgcgaaagcacgtgcgcgctggcgatggcagctgccagcgccagcgcgccctgccccgccatcgacgcgagcagcgcggccttgagcccgagtgccagcaccagcgcaatggcgccgaaggcaccgatgcgcgaatccttcatgatctccagcgcgcggctccggtcggacgctccgcccagcccgtcggccacgtcggcgagcccgtcttcatgaaacgcgccggtgagcagcaccgtcgcggccatgctcagcagcgccgcggccagcgcaccggccgtgcccggcaagccctgcagtgcgagcacgaaaacggccgcgccaacgccacccaccagccagccgacgccgggaaaatgcgccgcgctcgcacgcagcatcgtcggactgaacccgacccattcggcaagccggccggttaccggcacgcgcgtgaagaactgcagggccagcaggtagtggcgaacaccgttcatcgagttcaggcgtccttgcgcgacacgcccgccgcctcgaagctcgccatttcgcgcaggatgcggcaggccgattcgagcagcggccaggccagcgccccacccgagccttcgccaaggcgcaggtccaggttcagcaagggctccagtccgaggtgcttcagcagcagcgcgtgcccgggttccgccgagctgtgcgccgccacgcagcgctgcaccacatgcggctgcagtgcctgtgcaacgagcaccgcggcactcgcaatgaagccgtcgaccacgatcacccggcgttcctgcgccgcctgcagcaccgcgccgaccagggtggcgatttcgaagccgccgaatgcagccaaagcatccagcggcgaaaccgccgatgcatgcagcgccagcacttcgcgcagcaccgtgcgcttgcgcgcgagtcccgcggcgtcgagcccggtgccggagccggtgcaggcatcgatatcgagccccgacagccgcgcgagcagcatcgccgccgccgagctgttgccgatgcccatctcgcccagcagcaaagcattgccgggcagcacctgcaccacgtcgcggccgttggcaatggcctcggcgcattgcgcggccgtcatggccggcaccgctgatgcatcggcggtgccggcggcgattcgccgcgacaccaggcccgggcgcgcctgaaagtcgcgccgcacaccgcaatcaaccaccgttaatgcgagtccgtgctggcgtgccagcacgctcacggccgccccgcccgcgaggaagttctcgaccatctgccaggtcacgtcgctcggaaacgccgagacaccgcgcgccgcgaggccatggtcgcccgcgcacaccagcatctgcggtgcttcgagcagaggcgtttcgctgcccaggatcaggccgatacgcagggccaggttttcgaggcggccgagcgcgccgagcggcttggtcttgttgtccagcgcgctttgcaggcgtgccgcaagcgtgtcgtcgtgaatgtcggagatggagggaatggtgtcgttgtcggtcatgcgatcaggccttgcagtacgccggcctcgaagtgggtgtcaatgaaatcggccaggccgtcgaaggtggaatcgagcgtgggggccgcggcgccgaagagcgcgtgcagcgcggccgcatcttcgaacaagccgtgcaggtagaggcccagcacattgccgcgcgcgttctgccatgccagcccctcgggcatcacggcacggccctcctgcgccatctgcgggtgaatcgcggtctggccgtgatgaatttcgtagcctgcgaccgacacgttcgaaagcgcagcccattcgccgcccagttcgccaaagacggcggcccggtggcgcacggttttctcgcgctcgaacacggtcaccagcggcagcaggcccaggccgggcgcattgccgtcgatgccgtgcggatcgaccagcgcctcgcccagcatctgcaagccgccgcagacgcccagcacggcgccgccggcggccgcgtgcgcggcaatggcgctgtccagcccctgcgcgcgcagccatgccaagtcgccgctggtgtgcttggagcctggcagcacgatccagtcggcgccagccgcgtccgccggcgtgcgcgcccagaccaggcgcacgccgggcacgttcttgagcggctggaactcgtcgagattgctgatgcgcgggtacgccaccacagccaccgtgcgcgtgacgatgccgctcgagcggcttcgatcgtcgaacacgccgtcttcctccggcaggccgtgctgccaccacatcggcagcgtcgcgacggtggcgatgccggtcagtgcctgcagttgctgcggggccggggccagcaacgaggcatcaccgcgaaacttgttgagcacgaacccgcgcagcaatgcacggtcggtctcgggcatcaatgcccaggtgccgtagagatgtgcgaaggcgccgccgcggtcgatgtctgtcaccagcaggcagcgggcatccgcatggcgggccacgcgcaggttgacgatatcgctcgccatcaggttgatctcggccggcgagcccgcgccctcgatcaccaccacgtcgttctcggcgcgcagcgcatcgaacgcctctgcaatttgcggccagacgcgctcgctgcgcccgcgccagggcatggccgtgagttccgcgctcacctgacccatcagcaccacctggctgtgggtgtcgcgctcgggcttgagcagcagcgggttcatgcgcacgtcgggcacggcgcgcgccgccagcgcctggaaatattgcgcgctgccgatttcgccgccgtcgaccacgcgcgcgttattgctcatgttctgcgccttgaaaggcgccaccttcaggccctgccgcgcataccagcggcacagcgctgtcaccagccagctcttgccagcgccactggtcgtgccgagaaccatcacgcatcgggttgtcatgcggctattgtcgttgccgccgcatgccgtttccgcagcgcggagcggcaaagaaaaaggggcttgcgcccctttggtgttcagcgtgccgcggtctgcagcgtggcagcccctacgggctgagcctgtgccgtggcgggcggcacttcccagccgccgccgatggcgcggatcagccccacggccgcctggtactgcgccgacttcacctgcagcgcctggcgccggttgcgtaattcgctgcggcgtgcatcgagcaggtcgagctggctgatgtagccattgcggtagcgcgtgtcggacaaactggtcgcgcgctgggccgacgtgacggcctgcgcctgcacggtcgactggtcttgcaggatgcggatggcggacagctggtcttcgacctcctggaacgccaccagcacctggttgcgatagttcgcgagcgcgccgtcgagctgcgcattggcgccctgcacacctgcttcgcggcggccgccgtcgaagatcggcagcgagagcagcgcacccacgccccatgaacgggccgaccacttgaacaggtcgccgatctccggcgacgcatagccggccgcgccggtcagcgaaatgtccggaaaccacgccgcctgtgccacgcccacccgggcctgcgccgcaagcaccgcgttctgcgcggacgagacgtccgggcgtcgcgagagcaccgtggccggcacgccaggcggaacggacggcagcgcggtggcccagtcgtcggtacgcaggccgaagctggaggccgaatcgcccaccagcaccgcgagcgcatgctcgacctgggcgcgctgccggtcgagcgcgagcgcgtctgactcggtggacgacacctcggtctgcacgcgcgccacgtcgagctcggcgatgtcgccggcctgctgcctgcgctgcgtcaggcgcagcgtgtcgcggtaggcctcgacctgctcgcgcaccagggcgcgctcggcgtcgagcgcacgcagttgcagataggtctgggccacctcggcctgcactgcgaggcgcgtgctttgcagcagcccttcgcggcccgccgcatcgagcttggccgcattgctcgcgcccgagaggcggccgaacaggtcgagctcgtacgagaacgtggcgccgatgttggtcatggtggccggcctggtgctggccgtggccttgtcgagccccgcgccgcgattggcacctgcgctcaggccgatctgcggcatgcggttggcgttggtgctgcgcgccagggcgcgggcttccgccagccgggccgcggcggcctggatgttgttgttgttgacgtcggccttctcgaccagcgcattgagcaccgggtcgttgaacgccagccaccaggcgccgcgggcctgtgcctcggaaggcacggcacgcgtccagcccgcgggcggcgcggcgccctgctccttgaactgggcggtggtctggatctccggcacgccggaaggcactgtcgcgcagccggccagcgccagggctgccaccagcggcagcaaggcggtacgggcccagggttgaaatgcgaatttcatgatgatgaactttcttcttgatcgaccgtgcgatcagtcatgcgactcgtgcgaaggacgcggcgaggccggcaccggatgcagcccgccaccgccggaaccaccgtgggacggcgcagccggatgggccgccgagacgaagtcttccccgtgcggcacatcgccgtgcagcttgagtgcgcggttgcccgcgagacggcgcatcagcacatagaacaccggcgtcaggaacaggccgaaggccgtcacgccgatcatcccggcgaacaccgccacgcccatggccttgcgcatctccgagcccgcaccggtcgacagcacgaggggcagcacacccatcacgaaagccagcgaggtcatcaggatggggcgcaggcgcaggcggctggcttcgatcgcggcctggatgggcgtgcgtccggcgaactcgagctcccgtgcgaactccacgatcaggatcgcgttcttcgcactcagccccaccagcacgatcaacccgatctgcgtgaagacgttgttgtcaccccccgatatccatacgcccgtcatcgcggccaggatgcccatgggcacgatcaggatgatggcgatcggcagcgtcaggctttcatactgcgcggcaagcaccaggaacaccagcaggatggccagcgggaacaccaggaaggcggagttgccggccaggatttcctggtaggtcagctcggtccactcgaagctcacgcccttgggcagcgtctcggccgcaatcttggtgatcgcgtcctgcgcctggcccgacgaatagcccggggccgggccgccgttgatgtcggctgcaaggtagccgttgtagcgcatggcgcgttccgggccgaaggtcgagttgaccttcatcagcgcggccagcggcaccatctcgcccgaggtcgagcgcaccttcagcatgcccacgtcttcggcacgggcgcggtaaggcgcatcggcctggacgcgcacgctgtacgtgcggccgaacttgttgaagtcgttcgcatacaggctgccgaggtagatctgcatggtgtcgaagatgtccgtcaccggcacgccgagctggcgcgccttggtgcggtcgatgtccgcatacagctgcggcacgttgacctgccagctcgtgaacatgcccgtgagctcgggggcggcatatgccttggccatgaaggctttcaccgccgcgtccatctggtcgtagccgaccgaggcgcggtcttcgatctgcagcttgaagccgcccgtggtgcccaggcccgccaccggtggtggcgggaacatcacgatgaacgcatcctggatgctggcgaacgcgccgttgagctgcccggccaccgcaccgccgctctggtcggcgcgcttgcgctggtcgaagggcttgagcgtggcaaacacgatgcccgagttcgagctgttggtgaagccgttgatcgacaggcccgggaaggcgatggcgtcttccacgttcgggttcttcttcatgatctcgcccatgcgctggatcacgttgtcggtgcggtcgagcgtggcgccgtcgggcagttgggcaaaaccgatcaggtattgcttgtcctgcgccggcacgaagccgctgggcaccgccttgaagagaccgaaggtcacgccgatcagcgcgaggtagatcaccagcatcagcgtcttgcgcgagatcacgctcttgacgccgccgctgtaggcttcagagccgcggctgaagagcttgttgaagccgcggaacagccagccgaaggccttgtccatgccgcgcgtcagcgcgtccttgggagcatcgtggctgcgcaggagcaaggcggcgagcgcgggcgacagcgtgagcgagttgatggccgagatcaccgtcgagatcgcgatagtcaccgcgaactgcttgtagaactggcccgtgagaccactgatgaaagccagcggaacgaacacggccaccagcaccagcgcgatcgcgatgatgggcccggacacttcgcgcatcgcgcggtaagtggcttcacgtggcgtcaatccggcttcgatgttccgctcgacgttctccaccaccacgatggcgtcgtccaccacgatgccgatggccagcaccagcccgaacaggctcagcgcattgatcgagaaaccgaggacgtgcagcaccgcgaaggtaccgatcaccgacaccggcacggccagcaaaggaatgatcgacgcgcgccacgtctgcaggaacaggatcacgaccagcaccaccagcgcaatggcttcgagcagcgtgtggatcaccgattcgatggacgcacgcacgaactgcgtcgggtcgtaggcgatgcggtattccagcccttcaggcatgttcttgttgagctcggccatcgtcttgcgaacgttggacgagatgtcgagcgcgttggagcccggcgcctggaacacgcccatgccgacggccgggtcgttgttcaagagcgaacgcagcgaatagtcggcggcgcccatttccaggcggccgatgtcgcgcaggcgggtcacggcgccgtcggtgccgctcttgacgatgatgtcgccgaactcttcttcactctgcaggcgcccttgcgcattgatcgagagctgcatgtccacgcccgagaggcccggcgaagcgccgaccacgccggcggcggcctgcacgttctggccgcggatcgcagccaccacgtcgctggccgagaggccgcgctgcgcaaccttctgcgggtcgagccagacgcgcatcgagtagtcgccgccgccgaagatctgcacctggcccacgccttcgatgcgcgcaagcgggtccttcacgttcagcaccgcgtagttgcgcaggtagttgatgtcgtagcggtcgttcggcgaaacgaggtggaccaccatcgtcaggtcaggcgcgctcttgacggtcgtgatgccgaggcggcgcacttcttccggcaggcgcggctcggcttgcgagacgcggttctgcacaagctgctgtgccttgtcgggatcggtgccgaggcggaaggtcaccgtcagcgtcatcacgccgtcggtggtcgcctggctgcccatgtagagcatgccttcgacgccgttgatctgctcttcgagcggcgtggcaacggtttcggcaatcaccttcgggttggcgcccggatactgggcgcgcaccaccacggagggcggtgccacttccgggtattcggagatcggcagcccgcgcagcgcgatcaggccggctatcaatatcaatagcgacagcacgccggcaaagatcggccggtcgatgaagaatttagagagattcatgttgtttctccggcgagcgcaaacgcgctcccctccgagttcaggacttcgcggcttccgcgacgcgttccggttgttgttgcttggtatcggccttggcgtccatcgtcacggtctgcggcaccaccagcgcgccggggcggatgtgctgcaggccgttgaccaccacgcgatcgccggccttcaggcctttgctcacgacccgcaggccgttgatcgatgcgccgagcgtcacttcgcggtacatcgccttgttgtcctcgcccaccaccagcacgaacttcttgttctgatcggtgccgatggcgcgttcgctcaccagcaacgcggagtcgctgcgtgcctggcccatgcggatgcgggcgaactggccggggatgagcgcgccgtccttgttgtcgaaggaggcacgcacgcgcaccgtgccgctgcgggcgtcgacctggttgtcgatcagctgcagcttgccgatgaagggcgttccgtcgaagcccgaggtgcccatctgcaccggaatgctctcgatctggccgcgggcgctggcgccgctcggcaagtctttcagcgcccgcgtgatcacctgctcgtcagcatcgaagctcgcgtagatcgggctcaccgacaccagcgtggtcagcaccggcgcgccggggccggcagccaccaggttgcccacggtcacctcgagcttgccgatgcggccgggcacgggcgcacgcacctgcgtatagccgaggttcaggcgcgccgactgcagcgacgcttgcgcggcacggaggttggcatcggcttcgcggctggcgttcacgcgctcgtcatattcgcgctgggcgatggcttgctggtcccacaggcgcttggcacgttcctgctcgctgcggctgaacgcctggcgggcctgggccgatgccacctgcgcttcggctcgctccgcttcggcggcgtacggtgcggggtcgatggtgatcagcaggtcgccctgcttcaccagcgcgccttcgcgaaagtgcaccgcctgcacggcgcccgccacgcgggaacgcacgtccacccgctgcaccgcctccagccggcccgagaactcgtcccaggcgttgatctcgctcgacgccacggccgccaccgacaccggcgtgccctgcggcgccgcggcgggcgccgtggcctcggccttgaagctgtgcatgcccagcaccccggcggccacggccagcactgcggtgaggccggtcacggcgggccacaggcccttgcgggcgacggaagacagtttttgattgttgttcgacatgatgattcgtccttctcgatgactttttgggatgcaacaggccaccccggtgcttgtggcaccaggaggcggaattcgaaaacgaccggggttaccggtgggccgaggggtggcgtcgcgcgtcagccaggctgctgcgactggcccacctagctgggcttgagtgctaccggaggcggcgtggtggcactgaaaaattcgcggaaatgctgctgcacgctggcctcgcatgccttgcagcccgagggctcggggtcgtacagggccttgggccagttcgcggcaccgggcagcacgctgctcgtgacgtcgatgccggccgcgcgcagccgcccggcaaaagtcatcgcctcgtcgcgcatcgcatcgtcggcgcccaccagcaccagggcgggtgccagggaagacagccggagcgatccgctcggcaccgcgtaggggtgcatcgcgttggacgggcagctcaggtacttttcccagcccttggcccagcggcattcggcctcgtcgttggtggcattgcgcagagatgccgtgcccgcgcacgggtcgagcatgggcgacagcaggatctgtcccgccagcggtggatgcgcccggtcacgggcgatcagcgccacgccggccgccaggttgccgccggcttcctcgccggccaggtacacctgcgcgcctttgccgccgatcttcacgcgctgcttgtagagccactcgagcgcggcatagcccacttcgatgggttcggggaacggcgattcgggcgccagcggataagccaccgacaccaccaccgcgcccgcgccggccaaaagccgggccacgttgcgcccgttgtccaggttgccgcaaatgaaggtgccgccatggaaatgcagcaccagcggcacggtttcgccccgggggcgttgtccgtacacccgggcgcccacggggtcgcggccgggcagctcgatcgaaagatcggcttccacgccttctgccgcggcgagagcagcggcttcggcagagcgggacgacggacggggtgacatggaggcaacctcaggaggattggcgatagtcgaaatataaggcggccagtgtggggttaaacaggcaacctgcccctactctgtttccaaaccgctaacaatccgggaaacgctgtgggattgtcaccttgtgtgagaatccgcgtcctcccggcatggccgggctcccaggaacagtcatcaatggatcaaatccaggcaatgcggatctttgtccgcgtcgtggaagcaggcacgttcacccgggcggcggactcgctcgccctgcccaagggaacggtcaccaagcagatccaggcgctggaatcgcgcctgcgtgtgaagctgctcaaccgcaccacccggcgcgtgaccgtgacgccggacggtgcggcctactatgagcgcgcggcgcgcctcttgaacgacttcgacgacatcgaagcgagcatgaccaatgcgcaggcgaacccgacgggacggctgcgtatcgacgtgggcacctcggtggcgcggctcatcatcctgcccgcgctggccacgttttgcgaccgctatcccgagatccaggtcgacctgggcgtgagcgaccgcacggtcgacctcatcaccgacaacgtggactgcgtgatccgggccggcgaactcagcgaccagtctctggtggcccgccgcatcggcaccctgcacttcgtgaccgtggcgtccccggcgtacatcaagcgctatggccatccgcagcatcccaacgacattgaaaagcgccaccacgtggtgagctacttttcgggcagcacgcggcgcgtttacccacacgagttcaagaagggcgacgagtccatcgagctcaacgggccctaccgcgtgtcggtgaatgagagcaacgcccacatggcggccgtgcttggcggcttcggaatctcgcagtgcatcaccttcatggccgagccgcttctggaaagcggcgaactgatcgaagtgctgcccgaatggcaccgcgacccgttgccgattcacgtggtctacccgcccaaccggcatctgagcgcgaaggtgcgggcgttcgtggactgggcggccgaactgtttgcgaagagcccgaggctgcagcggcgatgagttcgttcgctgcccgccgcttcagtcggcggcggggaacaccggctcgcaacgcacctcggtcttcactgagttggcaatgaagcactcttcgtgcgcccggtggtgcatgtgttcgatctgctcgcgcgtcggcaggttgtcgcccgagaacgtgacctcgggccggagcgtgaccaccgtcatcgcgagcctgccttcggcgttcttttccatgatgccgctcgccgcatcgaagtagcggtcgacgttgaacttgcgcttcattgccatggtgagaaaccacagcatgtggcagctcgacagcgaagcgacgaaagcttcttcgggatcgaccgccgccgcatcggaaaacggcagcggcaccacgtgcggcgacgaagagccgggcacttccgcgccgccgtcgaagcgcatcgaatgccttctgctgtaggtgttgccgaggaagtcctgctcgcctcgctgccagaggatttctgcggtgtactgggccatgccttgctctccagcgcaaatagtggccgccattttgcgtcagggggccatcggccgcgaacgccctcaaacgcccatcagcctgaccagcaacggcaccagcagcgccgtcgcgatgccgttgagccccagggccagcgcggagaatgcacccgccgtttcgttcacctggatggcgcgcgcagtgccgatgccgtgcgccgccaagcccaccgagaagccgcgcaccgcgggctcttcgatgcgcagcaggttcaggaggccggtggccatgatggcgccagagatgcccgccacggcggccgccaccgcggcaagcgacggcagcccgccgatcttctcggcgacgcccattgcgatcggcatggtggccgacttgggcgcgagcgacatcatcagttcgtgcgatccgcccagcgcccaggcaatgccgatggccgacacgatggcagccaccgagcccaccagcagcgccacgccgatcggcagccacaggcgccgcagccgcgcgagctggccgtaaagcggcaccgcgagcgccacggtggccggcccgatcaggaagtgcacgaacttggcgccttcgaaatacgtgtcgtaaggcgtgtgcgtgacgagcagcacgctcacgatcgcaatcaccgacaccagcaccggattgactgccgggttggcgccgctacgtctgtgcagccacagcgcgcccaggtaggccagcagcgtgatggacagccacagcagcggcgactgcgccaggaagacccagatttcggaaagcttcggggatgggctcattccgcgtccttgcccgtgatgcggatcatccagcgcaaggtgagcgcggtcaccgtcatggtgaaggccgcccccacgatgccggccgcgaagaacggaagccattcgcgccctacccgctcgaaatgcagcatgaccccggtcacggcggggatgaacagcagcatgaggttgcgcagcagatggcccgaggtctcgctcaacgcatcgggcacgccgccacgaacgagcagcacgatgaagagcagcagcatgccgatcagcggacccgggatcggcaggcccagccactgcacgagcagttcaccggccagttggcaaagaaagagcgtggtgatggcgtagagcatgcggatgtcctgcggatcgtgttgaccttcagtgttcggccgaggcaacggcgcgtgtccaggcttctttcagtgcctgctggctctgcggcggcagcacgcccagccgcacgaaccccgtcaggccaaaggaagcgcagtcgcgcagtttgatgccttcggcgcgcagggccgcggcgaaccgcgggtaaggcgcatcggtgcgcgcgcagaagaagttggcatcgctgggcaggcattgccaacccagcgattcgcagagggtgcgctgctgcgccttccatgcccgcaaggtgtgcaggctctgcgcgagccaggcctgggcttcggtgccgatccaggtttcgagcaaggccacgccgtgggcacccaccggccatgacggggccaggcgttcgaggcgctgcaacatcggcacggccgcagcgtcgtcgggcgcgatggcgtaggccgcgcgaacgccggtgaggcccatcgccttgttgggcgtccacagctgccacacgcggtttcgctcggcggcatcgagcgatgccgcgccttcgagacgcagcggttcataggccaggtcgagcacgcagaggccgccggccctggtgtgccgcgtgagatcggactctgcctggccgagcgggctcgatggttcgcagcaccatcgcagcgccgcagcgccgtgcggctccggaaagcgcagcacgtgcaggccccaggccaaggccgcacgctcgtagtcgccatagctgtgcgcgggcagccacgcctcgcggccaccgccctgcgcaaaggcggcgctgatgcggtggatgaattcgcttgcgctggccgcgatcgcgatgcgctccgttgccacgccatgaaaccgcgccagcgcaccgcgcaaccgcgcatagccagggtccggatagtgggccgcgtcggccgcgcgcagcgcggccaggacgacggggcacgaccctgtcgcattgccattggtcgaaaaatcgtgccaaggcgtgccggctccgtcggggccgccatgcaccgcagcttcgaaggtttcgtcttcctgggtcatgccggcctcgtgatcgcgaagatggccaatgatgcacacacagccagcgtcagcgccgccctgccgcccaattgcgcagcgcgatgcgtatcggccgcttccgcctgccggccttcggcattcaaggcatagacgcccggcttggcgagccgcacaccgagcagcagcgccatggccgccatgggccagccgctgttgggcgacggggtgcggcgcgcctcgcgtgccacgcctgcgggccattgccacgccgcgagcgcgagcagccctaccgtgagccgcgccggtagccacgagagcacgtcgtcggcgcgcgcggcccatttgccgaaccacgtccagtcgcggccattgcgttcgccgcgatagccccacatggcgtcggccgtgttggcgaagcgatagaccgccgcgcccggcaagcccagcagcacgaaccagaacaacggcgccacgagcgaatcgttgaggttctcggccagcgattcgatggcgctttcgcgcacctcgcgttcgctgagcgcgcagacatcgcggctgacgagccgggccagctgcgcgcgccccgcatcgagcgaaacgcccagcgccgcctcgaccgcgagcacttcgtcgtgcagcatgcgccacgcgaaaagcggtttcagcgcaaaggccatcgccatcgccagcgcccatgcgggcagccattgcaccatcgcagcctgcacgccggcggcgaccatccccacgcacatcgcgcccacgcaccacgtcagcgccccgatcaagaagagcgacaggtcgcgcggcttcgccttggccgccggcggtgcgatgcgcgagccgatccagccgaggtactgccccatccacaccaccggatgccagcgcgcggcgggctcgcccagccagcagtcgatggcaagcgtaagccacagcgcggcggcgacgaccagggcgtgttcgaggggaaaggcgggcatgggacgcgaatcaggcagcggtgacgaacaggacggcatcgacggccagcatcaggcaggctccacggaagacggggttgaaaacaggtccgacggctggccccagcgttcatcgaacaccagcgccgacaagggctcgcgccgggcccagcgttcgcgttgcagcatcggctcttcgtaaaaatcgtgcaccgggcccaggcacagcagcgcgatcggttccgcaccctcgggcaggcccagcagggccgacacctcggcgggatcgaatagcgagacccagcccatgcccagcccttcggcacgcgccgcaagccagaggttctggatggcgcaggacgccgaggccaggtccatttgcggcaaggtgcgtcgtccgaacacatgctgctcacggccgtcggccagcgacacggccagcagttcggccgcatcgagcacgccctgcaccttgagccgcatgaacgcgtcttcgcgctcgccgagggcgcgggccgtcagcacgcgttcgcgctcgatcacatcgtgcagacgctggcgcaaggcaccgtcgcgaacgcgaatgaaccgccacggctgcatgaatccgacactgggcgcgtggtgcgccgcttcgagcagccggcgcagcaactcgggcgctacctgcccccctgcgaagtgacgcatgtcgcgccgctcatggatggcgcggtacaccgctctcacctcgtgagccgcgaaggcttgcgacatcgaactcaatcctcgataccgcgctgcgccggaataccggccttgaaggcgtgtttgaccagggccatctctgtcacggtgtcggccagctcgatgatctctggcgggcagcggcggccggtgagcaccacgtgcacgtgcttgggccgcccgcgcaacgtttcgagcacgccctcgagcggcagccagccgtagatcagcggataagtgatctcgtcgagcaccaccaggaagaactcgccggacaaaatcgccgccctggctttttcccagccgtcgcgcgccagctcggccgagtgctcgaggtcctggctcttccagctgaagccgtcgcccaggccttggatcggaatgccgagctgctcgaacatgcggtgctcgccgaaacgagccgagggcactttcatgaactggaagatcttcacggccttgccgcggccgtgtgctcgcaatgcaaggccgaaggctgcggtgctcttgcccttgccgtcgccggtgttgacgatgacgatgccgcggcgctcgccttcgggcttgtcgtacggcttctcggtggggggagtttcgatttgcataatgtatttaggccttgtgttgatgctcgtcagttcggcagtgcgatccactggtcggccacgcggtgcacgcggatgcgatggtcgaacacctcttcgagcgcggcgtgggtggccggatcgctgctgccgccatggtgcaccacgcggccgtggttcatcaccaccagttcgtccgcggccagtgccatcgggagttcgtgcagcacgctgaccacggtgcggccctcggccaccagggcgcgcgtggtctgcatccagtcggcctggtgcggcggatcgaggttggcgagcggctcgtccatcaacagcagctcggcctccacggccagcgcacgggccagcagtacgcgctggcgctcgccgcccgaaagctggccgagcggccgctcgcgccactcccaggcctgggtgctgcgcagcgcgcgctccaccgcctcgcggtccgccttgctcggcgcggcaagccaacgctggtgcggcaggcggccgagcatggcaatgtcgtagaccatcaggtcgtcggcactgccctcgcctgccgcgccgctctggcccagccatgaaaggcgctgcgcgcgaatgcgccccggcaccttggccgccgcttcaccgaaaagaaagacgtcgccgcggtgcgggagcagcccggcaagcgccttgagcaaggtcgacttgccggcgccgttcggcccgaccacgctggtccaacgtgcggcgccgagcttcaggtcgatgccgtgcagcacctcggcggtgccgagcgtggcgctcacgctgcgcgcttcaagagcggggatgtgagtgctcattgggtaacctccgtgctgcgcactgcggtgcgagcccccttcggagcggccgggcgggggctcatgccacgccccctcgcgcgccgcgccggtgcatgagccacagaagatagctgccaccgagcacggccgtgagcacgcccacgggcagttcctggggcgcaatgagccagcgcgccagcaggtcggccgccatcagcagcaagccgcccatcgcggccgacagcacgatcaatcccgcgtgcgtggtcttgaccacggaacgcacgaggtgcggcgcggccaggcccacgaaggcgatcaggccggtctgcgccacggccgcgccggtggccagcgcgagcaccaccaccagcgcggcgcgcatcgcacccagcgggagccccaggctgcgggccgtcgcttctccgagcgcaagtccgtcgagcaccggcgcgagcgcccaggccagcagcaggcacgccgcaccgaccgcggccatcaccgcgcacgcgctccagccgaccaggccggtgctgcccaggatgaagccctgcagcgcctgcaggatgtcggccgaggcgatggtgatcaggtccttggcggcgccgagcaccacgccgacgatcacgccggcgagcagcagccgcagcgtctgctgcacgccacgcgccagcatcagcgtgagcatcaccgcgcacaccgcccccacgaaggccgcgccggtgagccccaggcgcatcgcccattgcatgctggcggccgagccgccgaacagcatgagcgccacggccacacccagcgaggcccccgatgcgctgccgagcaggtaaggatcggccagcggattgcggaacagcccctgggccaccgcacccgcgaggccgagcaatgcacccgccagccacgcgccgagcgtgcgcggcaggcggatgtcccagacgatctgcagcgccaccgcatcgtgccgcgccgccagcaggctttggaagccggtgctgccgatgcccaggccgaacaccgccaatgcgctacccacgccaagcagggctataccgaagagccagacgcggcgccgatgacgcgtgtgcatgagatccgcgcggctcaaccggccttctccgcgatgcaccgggccatgagcctcgcggcctcgtccatgcgcgggccgggccgcacgagcacgtcggcctctgcggcatcgaagcggcagatgcgcccctcgcgcaccgcgcggatgccgctccagcccggtcgctgctccatgcccgccgcgctgcgcacgctgaccatgatgaggtcgggattggcgcgcaccacgtattctgggttgagcttgggaaagggtccgagcgaagccggcacgatgttcttcatgcccaggcgcgtgagcgtctcgccgatgaacgacgactcgccggccgcatagggcgcgctgttgacctcgaagtagacgcgctggcccttcgcactggcgggcagcgactgggcggcagccgacacgctggcatcgatcgcgcgccagatgttcgcggcctcgtgggtgccgagcacctggtcgagcttgtcgagcacgcgccgcacgtcggcatggctcttgggttcgagcaccaccaccttgaggccgagcgcctcgagccgctgggtcacgcgcgacgacttggcaagcagcaccgcatcgggccgcagcgcgacgatggcttcgacgttgggatcgattccgccgcccagtcgaggcaagccaagcaccgcgttcggcgagttggaatagttgtcgacgcccaccagccgcgaacacgcgcccagtgcgcagaccccttcagtcaatgacggcagcagtgtgacgatgcgctgcggcggctgcggcaacgtcaccgtcacgccgcgctcgtcgaccacgtcgagagcattcgccgccaatgcgaaaacgcccaggccgacggcgagggagaaagaaaggatccagtgtcttgtcatgcggcaggcgccttcaaggtcagcggcaatccggccaccatcagcgtgacccggccgcacgcggccgccacgtcctggttgagtcggccgagcgcatcgacgaaggcccgcgtttcgccgccaagcggaatcacgcccaggccgatctcgttgccgaccagcaccaccggtccgcgtgcttcgcgcagcgcgacgagcagcatggcgatatgcgtcgccggcgtgcgcgtcatcggccgcgccgattcggaacgcagcggcatcaggaggttggtcagccagagcgtgaggcagtcgatcaccaccagcgtgtcgggcgcactctgggtgacgatttcgcgcgcgagttcgatgggctcttccaccgtgcgcatggcgggcacgcgctgcgcgcggtcggcctggtgacgtgcgatgcgctcgcgcatttcgtcgtcgtaggcctggcccgtggcaatgagcacggcgcggtgcgttgctggcgcttcggccagccagtcaatagcgcgctgttctgcgcgccgggacttgccgctcttctgaccgccaaggatgagttcgtgctcaggcatgggcatgggcatgggcatcagcgctaagttcgccgtttgcgtcgggttggcttattgcggtgtccacttcaggccgaggtaagcgttgcggccgccggtggcgtagccgcgcgccagcgtgtagtccttgtcgcccacattgtccacgcgcgccaccaggccaaggtcgcgcgtgatctgcgtgctggccaccaggttcagcaccgtgtagccgctcagggtgcgggtgttggcggcatcgtcgaagcgcttgctcgacgactggatctcggcacccagcgtccagccggccacgcgccagtcggcgcccagcgtgccgtggcggcgggcgcggcgcgccagcaggttgtcggtgtccaaatcgcgcggatcctggaagtcggccgacgcacgcaaggtgacgttgccgatgcgatggccgcccgacagcgtcacgccctggtagcgggcacgcgcggtgctggcatagcagccgaagccggagcggcagttggtgtcgaacacgatcaggttgttaacgcggttctggtagaccacgatgcccgcatgcgtgccgccgtcggtgtaccgcaggcccagttcgacgttgcggcccgactcgggcttgaggctgggcgtgccgtattcgctgaagcgctggtacagcgtgggggcgcggaaagacgttccagacgacacggtggcgcgcagcttgggcgtgatcgagaagccgtaggccgcactgccggtggtcttgccgccgaactcgctgtcgtcgtcgcggcgcacgtgcagctgaagcgaatgcgcgccctgcacgaagccgtagccgagcgaaaccgcatcttgcgagcgcttgctggagagcaggccggtgaagagggtcggcgcgttttccagcgcgtcttcgcggcgttcgagggtggccgtcaccaggtgcgggccgaagcggaattcgttctggaacaggtagccgcgaaggttcgtctcggtgcgatagaacgaaggctgcgtcttgtagaccgcttgcgaatcggtgacctgcacgcgcgtgctgtagatgtcgttccagttcgccgaccacgaaagcccggccgtgcgcagcgtgttgttgccgatgtcgttcctgaactggatcggtgggcgggccctggagctgacctgtgcgtcgtagcccgcttccatgtcgctgtagagcagcgtggcgtcgagccgctggtcgggggtgagctggtagcccaggcgcaggttgccggcgttgctgcggtagccgtcgcgatcggggctggtgtagccgtctctcgagggcgtgcgcttgtccagaggctgcacgttgaagcccctgctctcctcatgcgcgacacccagcgaatagtccagcgcgccggactttccgctcacgccagcttcggccttgcgcaggccatggctgccgaagccgacgcccgcataaggagacacgccttcttcgccgcgcttggtgaagagctggatcacgccgcccacggcgtcggaaccgtacacggctgcagccgggccgcgcagcacttcgatgcggtcgatctgcgagaggggaatgctctcccagccggcgccgccggtcgattgcgaatcgacacgcacgccgtcgacgtacacggccgtgaagcgcgtctccgcgccgcgaatgtagaggctggtggtgttgcccacgccgccgttgcgcgtgatctcgatgccgggcaggcgcgccagcacgtcggcgacgccgaccgcgccgctgcgctcgatggtctgccggtcgatgaccgacacgtcgcccaccaggtccgacagcggttgcggcgtgcggttggccgtgaccacggtttcgctgagtgcggcagcggccacgacttgctgcgcatgcgccgcgaggggcagctgaaacagggccatgccgccgaaagcggaggccagcgcaagcggcaggcaggcaaggcggcgacggcgcgcgggaacacggccgagggaaaggggaccacaggaagtcatgaatggagcgaacgaacgtctatgcccgtcgccggcctccccgccaacttttgggcgcaatggctgcctcatgcatcgaaatcgatcgcgcatgcggcagccgcctcgttggccggtatccgggctggcagtgcaaccccaccgccttcccaggtgcctgtttcagggcacccagtggctgaatggatgaggttgacgcttgcggcgtcgactgcttgaccgttgcgggggcagcgcaggcggcttcggcccggttccgtttccggggagcgttcactcctgcttcccgttgaaccgcggcgtgtgaaccacgccgcaggcaccaacgggcaggattttagggcctctgccggcgcagtaagccaaaagttgcgccgttcgttgttcggcgggaaactacaatcgccaaccatgcccgcctccagccccatcgaccagatcgccgagcgtgtggaacgcctgctcgtgcgtcatgaagaggtgcagcgcaccaatgcgctgctgcaggagcaggtcgaagcgctcacgcgcgagcgcgacgcgctcaagtcgcggcttgccgcggcccgcacgcgcctcgatgcactgctcgagcggctgccggccgaaccaccttccgaagattcccccgcatgaagcagatcgaagtacaaatcatgggccagagctatctgctcggctgtcccgacggcggcgaggcgcagctgcgcgaagccgtcgatcgcgtggacgcggccatgtgcaagatccgcgatgcgggcaaggtaaaagcacgcgaccgcatcgcggtgctggcctcgttgaacctggctttcgacctggccgcgcaacagaccgccgccgcggctgcagcggcatccgcacctgctgccgcggctcccgtgggcgaaatcggcgaggccggcgaagccgatgccaaggccgcgcaactcatccagaaactcgatcaagccctcgcgggcgatgatcatttgctctgagcggccgcgtccggtccgccagaggcgtaaaatccgaactgtctgcggtgcgcgtcgggcttaatatttccttgttccaatgctctccggagccgggcttggtacatcgcttgacgggcgtgatcatctcgcgttagatgaacccgaagtcttgctgccctcgcccacctgaaccctggttcaggatgcgggttcggcgcccacttgcagacacctttttctgttgacacggcccctgcatgcactgcacggggccgttgctttttttcaaggccccgctgcgtgacttccctgctcgaccccctcctgatcgccgaattggccgcgctcggcctgggcaccggttttctggcgggcctgctcggcatcggcggcggcatgctcatggtgcctttcatcacgatcatcatgggccatcgcggggttgcttccgatcttgcggtgaagatggccattgccacctcgatggccacgatcatcttcacctcggtgtccagcgtgcgcgcccatcacaagcgcggcgcggtgcgctgggacatcgtgcggcgccttgcgcccggcatcgtcatcggcagcctgctgggcagcctcggcgtgttcgcgctgctcaagggcacggtactggccatcgtcttcgcgctgttcgttggcttctcggccacgcagatgttcctcgaccgcaagcccaagcccacgcgccagatgccgggcaccgcggggcagctgtcggcgggcggcgccatcggtttcatctcgggcctggtcggtgcgggcggcggcttcgtcagcgtgccgttcatgacctggtgcaacatctccatccacaacgccgtggccaccagcgcggcgctcggctttccgatcgcggtggccaacgtgctgggctacgtgatcagcgggcagtcggtgcagggcctgccgggcggctcgttcgggtacatctggctgccggcgctggcggtcattgcggtatgcagcgtgctcaccgcaccgctgggcgcaaaggcggcgcacaacctgccggtgaagaagctcaagcgcgtgttcgcgagcatcctgtacctgctggcggcctacatgctctggaagggcctgcaaggctaggcccaccacccgaaaacccctcgggtcccgggtgacacccgttgcgacgccggcgccccggccgtataacggtcgcatgaaaatcctcatcgccgtcgacggcagcgcctatacgcaaaaggcgctcagctacatcctcgccaaccgcgccatgttcgtggatggtcacgagctgaccatcgtgcatgtctgcaccggcatctcgggccacgtcgcgcgccacctcagcaaagaggtggtcgacgactactacgccgaagaaaacgccaaggtcatcgagcccgtgaaggcgcggttcgcggagaacggcgtgaccaactacacggtcgacaagcgccacggccacgcggccgaagagattctcaagtcggcagcggcggcacacgccgaactgatcgtgctcggcacccacggccacggcatcttcggccgtgcgttgatgggctcggtggccaccaaggtgatttcagagaccgacaccaccgtgctgctcgtgcagtaagtaggtaggcaggcaggcgccaagccttcttttttctttctattgaacgcgctgctgccgccactcgcgcggcgagcagccgaagcgttctcggaatgcgcggctgaagtgcgccgcgtcattgaagccgcggccgtaggcaatgtcggccaccggccgcccggccaggcgcggctcgagcaggtcgcggctgcaggcttcgagccgccgctcccagatgtattgcgaaggcgtgagcggctcgctcttgaagacgcggtggatgtggcttgccgacacgccgagctccgccgcgaggcttcccaccgaaagagacggatcggccagttgctcgtcgatgcggcgcttcacgcgcgcaaggtggtacgccgtgagactgctcagccccggcgagcgcgccgcgggcaacgtctgcaggcccgcaaccagaatgctttgcacaccgttggccaccgcgagcgcggaggccggttgcagcgtgtcgatgtcttcgcgcagcgtgcggatcatgccaagcaacaggtgccccgcgccctcgcgtcccgataccgtggtggccgtcagggcttcggtatcgtgcagttcgctgcgcaggcgttcgccggggagcttgagcacgatctgctcgaaggtatcgtcgaacagcagctcatacggccgggtgctgtcgtacagcgcgaagtcgcccgtcgccagcacggcatcgcgcccatcctgccgcaccacgccttgcccgcgcgcctggatgctgaccaggaagtaatcgtcgcccgagcgcgagatgtgccccggcgtgcgcatgaccttctgcggccctgacttgaccaccgacacgtccaggctcggcagcgtgtgctggcggatgctgccttcgaagttgcccgcgccccgttcgcgcaccggatcgcacccgagctgcacgtagacgttgcagatcatgtcggtccagtaggcgagccgctggtcgcgcgggacggcgtcggtgctgagcaactggttcatcgggggtccttgggggagtcggcatgcaacgctggaacaagaacgccgcaagttcggatcaaggcgtttcgcggcggcgaatctacgcttgaagcaacccgcatgccaccgcgcaaacccggtgccaggtgtgcgaagttgtttcatcaccccgtttctggagacccgccatgcccaccaccgttcatcccaagctccgcgtcgccgccgtgcaggccgcgcccgtgtttctcgacctcgacggcaccatcgacaagaccatcgacctcatggcccaggcggccggccagggcgtgaagctcatcgcctttcccgaaacctgggtgcccggctacccctggtggatatggctcgactcgccggcctggggcatgcagttcgtgcagcgctaccacgacaatgcgctggtcgtcggctccgccgagttcgaccgcatcagggaagccgcgcgcaagcacaagatctgggtttcgctgggctacagcgaaaaggccgccggcagcctctacattgcgcaggcgctgttcgacgacgagggcagcacggtgcagacgcgccgcaagctcaagcccacgcacgtggagcgcaccgtgttcggcgaaggcgacggctctgacctggccgtggtcgagacgcccatcggcaacgtcggatcgctctcgtgctgggagcatcttcagccgctcagcaagtatgcgatgtatgcgcagaacgagcagatccactgcggcgcctggcccagcttttcgctctaccgcggcgcggcctatgcgctcggccccgagctcaacaacgccgcgagccaggtgtacgcggccgagggccagtgcttcgtcgtggcgccgtgcgccaccgtgtcgcaggcgatgagcgagctgatgtgcaccgacgcgggcaagcagcagatgctgcgcgtcggcggcggctttgcgcgcatctacgcgcccgacggctcgccgctcggcacgccgctggccgaagaccaggaagggctggtgatcgccgacatcgacctgggaatgatcgcgctcgccaaggcggcagccgacccgagcggccactattcgcgccccgacgtcacgcaactgctgctgaacaagacacgccgcgagcccgtggtgctgcagcgcgcgcccgaggtcgaaggcggtgccttcgaagccatcgtcgccacgcccgagccggcagcggcgccgcgccagcagccgctggccgcctgaaacaccggagccacgccatggaatccgccattgccgagcacctgaagtgtccccgcacgcgccaccgccgcgtggaggacgactacgcgccgccctaccccgtctggtcggcacgcgcgccggccgaggtcaagcaggtcgtgatgggctatttcggggtgcagtcgcgcggggccgaaatgcgcggccgcgcgtgcgcggcgctgatgaagatcacggccggcttcgccctgcccgacggccccggccatcacgacttcgcgcatcatgtcgatgccgacggctacgacaacatgatcgccatcgcctactgggacgaccctgccgcgcacgctcgctggtgcggggcacccggcatcgatgcctggtggcgctccgacgagcggctggcggatggcctcggctatttccgcgaaatcgtttcgccgcgcgccgagcacttcgagaccatgttcaacacgccggaccgcctcgaaggcgtgggcgtggtgatgggtggcgtgagcggcgaactgcaggagcatggctactggggttcgatgcgcgaccgcatcccgttgtcgcagaccgatgccatggcgccttcgggcacgcgcgccatcatcgccggcgctcccgcaccggggcagcgcgtgcgcgtggcaggccacgagaacatcgcgatgatccgctccggccaggagtgggctgacaccacgggccaggaacgctcgctctatctcggcgaaatggaacccgtgctgcgcgagggcatgaacttcctgcgcgaccagggcctgggcatcggctgctacagcaaccgctacatgcatcacctcgacggcaagggtgctccgctggaaaaatcgttcggcctgagcttctggcgctcgctcgccgacatggaacgctgggccgaatcgcatcccacgcacgtcgcgatcttcggcagcttcatgcgctacgtgcaggcgctgaacttccagctgcagctgcgcgtgtaccacgaggtgtcggtgctgaaggccgacgagcagagctacgaatacatcaactgccatgcgcgcagcgggctcatgaacggggtgggcgtgggctgacccattgcccagcgccgcacgccggaatccgcggacgccgccaaggaaaagccctaggcgaacagccgcttgtgctgctcccgcagcagcgccttctgcaccttgcccatggcgttgcgcggcagttcgccgacgacaaagcagcgcttcggaatcttgaagttcgcgagtttcgacttgagttccgcaacgatggcatcggcgtcgagcactccgcccgccttgggaatgacgatggcgacgccgacttcgccgaagtcggggtgcggcacgccgaccacggcgctctcggccacgccggggagctcattgatgtagccctcgatctcagccgggtagacgttgtagccgccgctgatgatcaggtccttgctgcgcccgacgatggtgatgtagccgctgccgtcgatcttgccgacgtcgccggtcttgaagaaaccgtcgacggtgaattcttccttcgttttttcgggcatgcgccagtagcccgcgaacacgttcggcccgctgacctcgatgttgccgatctcgtcggtggtgcagttgcggccgctgtcgtcacgcacgcgcagctgcacgcccggcagggcgaagccgaccgtgccgccgcggcgctcgccctgcgcggggctgtaggggttggaggtgagcatgatcgtctcgctcatgccgtagcgctcgagaatggtgtggccggtgcgctcgcgccactcgtcgaaggtttcgatgagcagcggcgcggagcccgcgacgaagaggcgcatgttgcgcaccgcttcgcgcgtgagaccgggctcggccagcagccgcacgtagagcgtgggcacgcccatgaacaccgtggcctcgggcagcttctccaccacgcgcttcgggtcgaacttcgagaaccagatcatcttgctgccgttcagcagcgcaccgtgcaacgccacgaagaggccatgcacatgaaagatcggcagtgcgtggatcagcacgtcgccttgggtccagccccagtattccttgagcacctcggcgttcgacagcaggttgccatgcgtgagcatcgcgcccttgctgcggccggtggtgccgctggtgtagaggatggcggccaggtcgtcggctttcctcttcgcaatcacatgctggtcgctgcactgcgcggccgcttccagcagcgtgccggtgcggttgtcgtcgagcgtgaacacgtgccgtgtgcccgccgcgttggcgatgggtttgacccacgaggcattgcggctggtgcacaccaccacggccggttcggcgttgccgatgaagtattcgatctcggcgctttgataggcggtgttgagcggcaggaacacatagcccgcgcgcagcgtggcgagatagagaatcatcgcctcgaccgacttctcgacctgcaccgcgacgcgggcgccatcttccaggcccaaaccgccgagcaggttggccatcatggcgctggcacggtcgaggtcgcgccacgaatagaacaggccgtcgtccgtttccacggcaatgcggtcgagattggcgggaaaggacgcgcgcagggcggcgaacaggttgtagttggctttcgtcttcatcgggcaagtcttcagaaattcggtgtgcgcttggcaagaaaggcgtcgatgccttcgcggtgttcggcggagtcggcgtaatcgtaggcggttgcgagcaggttctcggtcgaatgcgcgcctgccttcagcatggcgaaggtgcgcttgtgcagtcgcgcggcctgcggcgccagggcggcgatgcgcgcggcatgggcctctgcggcgggagccacctcgttgtcgggcagcacctgcagcagaaaacccgcgtcgtacaggcgctgtgcgccatgcacgccggcggccagcagcatgtcgcgcgccagcacatcgccaatggcgccatggaccagcgcggcctctcgcggcgccatcggaaagccgagctttgcgatgggtgcgccaaactttgcggaggcgcccgcaaggcggatgtcgcagcagctcgccatctcgatgccggcgcccatgcacgcgccttcgatctgcgcgaccacgggcagcgggcaatcgagcatggcctggagcgcgccccagacctcgttctcgtggaactcgcgcaggctggcttcgtcgaaacggaacgacgggtactcggagatgtcgccgccggcgcagaaggcgccgccctcgccgcgaaccacgacacagcgcaactccggatcaaccgcctggcggatgccgtcgaacaccgcacgcagttcgcgccacatgccgcgcgtcatggcattgaggcgacccgcgttcgacagggtgacaaacgcaacggcgccctcgcggcgcagtgaaacgtggcgttcgcccatcactcgagcttggcgcccgaggccttcaccaccttggcccagcgcttgatctcggagttgacgaagccgccgtacgaagccatggtgagattcggaatctcggagccgttctgggtccagatggctttgagctcgtcgctcgccagcgccttcttcatgtcgtcgacgatgcgcgcctgcaggtcggccggcgtgcccttgggggcccacaggccgtaccaggtggtgacggtgtagtcgggcagccccacctcggcggcgcagggcacgtcggggaacgcggggttgcgcttgctgcccgcgaccatcagcgccttgatgcgcccgcccttgatgtgctgggccgaagaaccgaggccgtcgaacatcaggtcgacgttgccggcaatcaggtcggacagcgccgggcccgcgccgcggtagggaatgtgcgtgatgaaggtgttggtctgcagcttgaacagctcgcccgccaggtgatgcgaagtgcccgcgccggccgaaccgtagttgagcttgcccggattgcgcttggcggcggcaacgaactcctgcaaggtgttggccgtgacgcggcgcgggttgaccaccaccacctgcggcacgttggccagcagcatcagcggcacgaagtctttctcgaggtcgtagtcgagcttggggtagatcgacggcgcgatggcgtggtgcaccgcgcccatgaagagcgtgtagccgtcgggctgggccttggatgcgatgctggcacccaccgtgccgcccgcgccgccgcggttgtcgatgaccagcgtctggccgctgatcttggcaaactgcgccgagagcgggcgtgcgaaggcatcggtgccgccgccggccggaaacggaacgatcatgttcaccggccgggtcggccagttagccccctgcgcacgcgcaccgccaccgcacagaacggcggcaccggccgcagccaggcgcagcacgtcgcgtcgttgaaaactctgggtcatctgtcatctcctgtcgttgtggatttgccgcgccatgcggccgccggcacctcgcgcgccggactttttctttcagaactcagcccttcttgaaaaaaaggctttcaacatctcccgataccgccacctttccctcggcgagccacgcgcgatgcttgtcgagccgcttcagatcgtagaggtaattcaccatcaggccgtaagactgcttctgccccttgggcgagggatcgccggcccagttgagccgctccacgcgagcgccgttgcccaggtgaaagcgcgccaccgggtcggcgggcgtgccgtcgatcagcgtatggccaaggtattcggcggccgcctgcagcagccattggcgcagcggcgacttggcgtcgagggtggccgcggcgtccaccgctgccagcaggcggtcggcggtgggcggcagcgagccgacgaggcggccgagttcggcctctcgtttttcgtccaggcgcggcagcaggtccgcggcgttcttggcgagccagctgcgaaagccgggaaccggcgacagcgtggcaaagaccttgaggcgcggcagctcgtcctgcagcgtctcgaccacgcgcttgatgagcgagtcgccgaagctcacgccgcgcaggccgttctgggtgttgctgatcgaatagaagatggccgtcgtcgccttggccggcaggatcggcacggcggtctcgtcgagcagcggcgtgatgccctcgctgatgcggtcgaccagcgccacctcgacgaagatcagcggctcgttgggcagccgcggatggaagaagccgtagcagcggcggtcgctgtcgtcgagccggttcttcacgtcggtccagctcttgatgtcgtgcacggcctcgtagcggatcagcttctcgatcagcgacgccggcgagttccagtcgatccggcgcagttcgagaaacgcgacatcgaaccaggtagagaacaggtgctccagttcggcgtccagcgcgatcagccgcttgtcggacttgagaaaaggcagcagttcggcgcgcaggtcgaccaggaaacgcatgccttcgggctcgaccgcgaagcgctgcagcaggcgcatgcggggcgagaccagcgcgcgccgcagccgcaactcggcctggccttcgtcgggcgttccgaccgcggcctggtgctggtcgcgtgcggacttgagcttgtgcggatcggccgcgaaatgctcgctcatcagcgcccaatagtcgcgccgctcctcaggcgcggcgctggcgtacgcggttgcaatggcatgcgcgcggcgcccaccctcgacctcgctcacgcgcggatcgatcacggcctgcaaggcggccagcacgcggcgcagcgcgcgcggcgacaaggcttcgtcggccttgcgcagggtggcttgcatgcgctcggcggtcgagcgcaggctcggcttggcggcggccttgggcgcgccgcgggtggcaccctcgggcgccaccggcaccttgttgccggacttctcgccagagcgcagtcgcgcctggaaccattcggtcgcactcatcgacaaactccaatgctgtgaggtgcggggaggtcttttttcatgtcgttcatgacatcaccctggatttctgttgccgcgccacctcgcgcagtgcttcgcgctggcgcgtcaggtgcgtgcgcatggccgcgtccgcgccgtcgctgtcgcgcgccttgagcgcggcgaacaccgccagatgctccgacaggctctgctcgagccggcccggcgcatgcagctgctggagccgcgcgagcttgagtatcttgcgcagatcgccgatcacctgcgccagccatctgttgtcggccagctggatgatcgcctcgtgaatgaggtggttggtggcgtagtagtcgttgatgcgcttggacttggcatggcgcaccagccgttcgtgcagcgcatcgagctcgtgcagctcggaatcgcttgcgttgcgcgcggcctcgtaggcgcaacggccttcgagcagcgcaatgactggaaatatctcatcgagatcgcgctccgtcacctcgcgcacgaagcagccgcgccgcggttcatgccgcagcaggccttcggccgtgagcaccttgagcgcctcgcgcaagggggtgcgggaaatcgacagcctctcgcacagtgcggcctcgtccagaaagctgcccggtgccagcgcgcccgcgaagatctgctcgcgcagcgtggcggccacttcgtcgtgcagggagtttgggacgaggcgcatgaggatgtgaaacgcgggggcaggcgtaatttcctgtaattacacataattgtgagtccgcgatgaacgcggcacaaggccgcgcggcacgcccgcggcccgtgcttaccctgagtgccggagcctcaggccgtcgccggctggcggcgctgcgccgcccagatccacaggccgatgccgaagatcaccatcggcacgctgagccactgcccctggctcaggttgagcgcgcgcaggccgagaaaatcatccggctcgcggaaatactcggcaatgaagcgcagcacgccatagccgatcatgaacaccgcggccacctgtccttgcttgcgctccttgcgggcgtacagccacatgatgacgaacagcagaagcccttcgagcaggaactggtagacctgcgagggatggcgcggcagcatcgagccgctctgcggaaacaccatgccccagggcaggtcggggctgctgaagcggccccagagctcaccgttgatgaagttgcccacgcggcctgccgccagccccgtaggcacgcagggcgagacgaaatccatcacctgccagaacggccgggcacgcgaacgtgcgaaccagagcatcgccccgatcacgcccagcaggccgccgtgaaagctcatgccgccctgccacacgtaaagaatctgcagcggattcgcgagatagaactcgggcttgtagaacaggcagtagccgagccggccgcccacgatgacgcccatcaccccgagaaagagaatgtcctcgatgtccttgcgctgccacgcacccgcgccgaccagggagcggtacggctcgtgccgcaggcggcgcgtgccgagaaaatagaacagcgcgaacgcggccaggtatgtcaggccgtaccagtgaatggcaacgggcccgagctgcagggcgatgggattgatctgcggatacatgagcatccgcggattgtgcccggagcaaatgactcgcctcccaggcttcgcgcacttcgtgtcgcttcgccctccccctaccgggggaacacttgcggcccggcaagccttgcgcggccgaaccagaaccacagcgcgaggccgacggtcaccatcggcacgctgagccactgcccctggctcaggctcagggagcgcaggccgaggaagtcgtcgggctcgcggaagtactcggcaaagaagcgtagcgcgccgtagccgatcaggaagaccgcagccacctgcccctgcttgcgctccttgcgcgcatagagccacatgatcacgaacagcagcaggccttcgagcagaaactggtagacctgcgacggatggcgcggcagcatcgagccgctttgcgggaacaccatgccccagggcaggtcggggctgctgaagcggccccagagttcgccattgatgaagttgcccacgcggcccgcagcaaggccggtgggcacgcagggcgcgacgaaatccatcacctgccagaacggccgcgcacgcgaacgcgcgaaccagaccatcgcgccgatcacgcccagcatgccgccatgaaagctcatgccgcgcttccacacgtacaggatctcgagcgggtgcgtgaggtagaactccggcttgtagaagaggcaatagcccagccgccccccgacgatcacgcccatcacgccgagaaaaagaatgtcctcgatgtccttgcgctgccaggcgccggcgcgggccagcgaacggtacggctcgtggtgcagccggcgcgtaccgagaaagtagaacagcgcgaacgcggccaggtaggtcagcccgtaccagtgaatggcgacgggtccgagctgcaaggcgatgggatcgatctgcggatgcacgagcatccgcggattgtgcccggagcaagtgacacgccccccaggcttcgcgcacctcgtgtcgcttctcccccctgtcggaggcagcacctgcggcccggcaaagccggttccgcggtgtgacgcgatttagctgctcactacttcgcccgcaccgtacgctcccgcacgaattccacgaaacgggccagcgccgggtgcgccgcctgcgcagaccacaccagactggtctcgcaagccggcagcgccacgcggcgccgccccacgcccttgaactcgtcggcctgccggtagaccacgcccgcgcgccggaactgcatcacgctgtgcggcacccaggccacgccgatgccgcccgagacgagattgacgatggtctgcatctggatcgcctcctgtgcgacctgcggcgtgcggccggcggcgtgatagaggtcgaagacagcgtcatgcagcgaaggcacgatgcggcgcggaaagatcaccagcggctcggccagcacctctgccagcggcacgggccgcgcgcgtgcgagccggtgctgcgccggcagggccagcaccagcgcctcctcctccaccggcagccgcgcgagccccggcggcgcggcgcccggcgaatgcagcatcagcccggcatcgatctcgccgcgcgcaaaggcttcgagctggacgtcgcccgtggcctcgaccagttcgagcgccacctcggggcaaagcacgcggaactcgcgcacccaggccggcaactgctcgaaaccgacggtggagacgaaggcgatgcgcacgcgccccacctgccccgccgccgcggcccgcgcccgcgccggaagcgcctgggcgcgcgccagcagttcgcgcacatcgggcagcagcgcctcgccggcgggcgtgagcgccacgcgccttcgggtgcggtcgaacagcagcacgcccaatgtcttttcgagctgggcaatggcctgggtcaccggcggctgggtcatgtgcagccgcagggcggcgcggccgaagtgcaattcttcggccaccgcgacgaactggcgccaggcccgcagatcgatcaggctttctttcatatgcctagcatatcaatccgcactgaaaaatggattggaatgaatcaatgagaagtccgatacttgggcttccccccgatctccccacgacacaagagacaccatggacaccaagccaatccagatcaatcgccgcagcgccaacatcgtcgaaggcaagagccgcgcgcccaaccgctccatgttctacgccatgggctacgaggaaagcgacttcaagaagccgatggtcggcgtcgccaacggccacagcaccatcacgccctgcaactcgggcttgcagaagctggccgacgcggccatcgcgggcatcgaggaagccggcggcaacgcacaggtgttcggcacccccaccatctccgacggcatggccatgggcaccgagggcatgaagtactcgctggtgagccgcgaggtcatttcggactgcatcgagacctgcgtgggcggccagtggatggacggcgtgctggtggtcggcggctgcgacaagaacatgccgggcggcctgatgggcatgctgcgcgccaacgtgccggccatctacgtctacggcggcaccatcctgccgggccgctacaaggggcaagacctgaacatcgtgagcgtgttcgaagccgtgggccagaacgccgccggcaacatgagcgacgaagacctgcgcgagatcgagatgcgcgccattcccggcagcggctcgtgcggcggcatgtacacggccaacaccatgtccagcgcattcgaggcgctcggcatctcgctgccctactcgtccaccatggccaacccgcacgacgaaaaggccaactcggccaaggagtcggccaaggtgctgatcgaggcgatcaagaaagacctgaagccgcgcgacatcgtgaccaagaaggccatcgagaacgccgtggccgtcatcatggccacgggcggctcgaccaatgcggtgctgcacttcctggcgattgcgcatgccgccgaggtcgagtggtccatcgacgacttcgagcgcatccgcaagaaggtgccggtgctgtgcgacctgaagccctcgggcaagtacctggcagtcgacctgcacaaggccggcggcattccgcaagtgatgaaggtgctgctgaacgcgggcctgctgcatggcgactgcatcaccatcaccggccagacgattgccgaagtgctgaaggacgtgcccgacgtgccgcgcgccgaccaggacgtgatccgcccgatcgacaagcccatgtacaaccaaggccacctggccatcctcaagggcaacctgtcgcccgaaggcgcggtcgccaagatcaccggcctgaagaaccccgtcattaccggcccggcgcgcgtgttcgacgacgagcaatcggcgctcaaggccatcctggacggcaagatcaaggccggcgatgtgatggtgctgcgctacctgggccccaagggcggccccggcatgcccgaaatgctggcccccacgggcgcgctgatcggcgcgggcctgggcgaaagcgtgggccttattaccgacggccgcttctcgggcggcacctggggcatggtggtcggccacgtcgcgccagaggcagcagcgggcggcaccattgcgttcgtgaacgaaggcgactcgatcaccatcgacgcgcacaagctggtgctcgaactcaacgtgcccgaagccgaactcgccaagcgccgcgaaggctggaagccgccggcgccgcgctacacccgcggcgtgcaggccaagttcgcgttcaacgcctcgagcgccagctcgggcgcggtgctcgacaagttctgaaacctggtcaggccatcatccacgcgccgtagccaaaggccaggaagccaaggcccacgatcgcgaggatgctgcggaattcgaattccatcgacggcggcaggctctgcacgacgaagtgcagcaatgcgccggcgccgatggtcatgaagccggcaccgagcgccctccccagccgctcgtccggatacagaaagcagacggcaaagccggccacgaagaccaggttggccagcacggtgccgcgcgtgcgccagcgctgctgcgcggacgtggccttgcgctcaaccggcgcgccggcctggggccgcccctccttgatcgccatgccggtgaagaagaggccgaacatcgtcgggaacagcccgaagaggccaaatccccagacggcgccccacatgttctggaagtccgccaccagggcttgcgccgggtcggccacgctgtagcgcacctcgaccgggtcgccccattccttgtccgacagtccgccgccgagtcccttgacgcggcgcttctggccgtcaggcgcgatgtattcgacgatgggggcgcgcgagaccgtggtgcggccgttgctgtccttgctgcgctcgtcgacgaactcgaccaggctgccctgcacgctggccgtgccctcaatcgactggtagcgatgccagccgatcgtcgcggcggcgtagaggcccgcgcagccgatcagcagcgccccgatccccacgccccagaacaagcccttgagccatcccgccaaaccgccgatggccggcccggccagcagcgagagtccgaagaccagcatcgcttgccgggtcgcttcttcgtccatggcgggtgccggtgcatgcagtggacagggccgcccggcgtgtgcgtgccgctcagcgcttcggtcgctggcccttgctgcccggcaggcccatgttgctgcgctggcggtcgatgcgggcctgcttgcgccgctcttcgcgctcaatgaccttgcgcttggtgtagcccgacgaatcggcccatgcccaccacgccacggccagcgcgaacggcgagagcacgatccaccagctccagccggcaaccatgcccacttcgaagtatttgaggcctatgcccagcaagcccagcagcagaaaaagcatcgcgaatccctcgggttttgttcgaaacgcttccggacgccggtgcacggcgctacctacaatcgcgttagatcgaatgtaacccagccattacgaaatacatccccatgaagagactcctgtcatccgcgattctgggcttgggccttgggttggcggcgcccgctttcgcagacctggccctggccacgtcgaaaaactgcatgagctgccacgcggtcgaccgcaaggtgctcggcccttctttcaaggacgtggcggccaagtacaaaggcaacgccggcgccgcggacatgctcgcgacaaagatcatcaagggtggttcgggcgtatggggcccggtgccgatgccggcgaacaaccaggtgagcgaagccgacgccaagaagctcgccgcctgggtgctgatggcgcgctgagcctgggcgcccaggcccgcgtcgtcaaacccgtggatcgatgtccgtgggcagcggccggcgctcgatgcggtcttcgagctggccgatgtgcgcggccacggtgttgtcggactgctccgaacgctggcgcaccacgctctcgacctgccccagccgggtcagcaacgcggcatgccgctcggcgttttgcgccatgtgcttgttctcctgcgtttccaggaaattgcgcagctcggtgaagcgcgaagcctcggccttgtcggcaagatcgcgctgcacctgcatttccttgttgtggcgcttggcgtcgagcaacaccgagctgtgcaggtacagcacatagaccaggaagaacacgcccagggcgaccgtcagcgcaagcatcatcaagccgagcggcgcggaaatcgtcatgaagcccagcgagaccggcacgggcgccgaaagcgttccccagttgagcgcggcaaggaccgcgatcaacagcagaatgacgaacagaaaagcggatctcacgcccatggggggcctccttcgtacagatcgaacacagctgaacgcgccctgcgcatcgaagcgcacggcggctctgctggttttacctcaggccgaaggccgctatggccgccgctctccagtaacggccgtgtcctacagaaccaatcaattggtctgtgacaactgctccagaatggccggattctccagcgtcgacgtgtcctgcgtgatcgcctcccccttggcgatgctgcgcagcaggcgccgcatgatcttgccgctgcgcgtcttgggcaggttgtccccgaagcggatgtccttgggcttggcaatcggcccgatctccttggccacccaggcgcgcagctcgttggcgatctgcttggcctcctcgccggtcgggcggctgcgcttgagcacgacaaaggcgcacaccgcctcgcccgtcacgtcgtcgggccggcccaccacggccgcctcggccaccaggtcggtcttggacaccagcgccgattcgatctccatcgtgcccagccggtggcccgagacgttcagcacgtcgtcgatgcgcccggtgatgcggaagtagccgcggtcggcactgcgtacggccccatcgccggccaggtagatggtgccgcccatctcctcggggaagtagctcttcctgaagcgctcggggtcgttccagatggtgcggatcatcgagggccagggccgcttgatgaccagcatgccgcccgcgccgtggggcaggtccttgccggtctcgtccacgatggcggccatgatgcccggcagcggcagggtgcaggagccgggcaccagcggcgtggccccgggcagcggcgtgatcacgtggccgccggtctcggtctgccagaaggtgtccacgatcggacattgctcgcggccgatatggcggtggtaccacatccaggcctcggggttgatgggctcgcccaccgagccgaggatgcgcaggctcgaaaggtcccagttcttcggatgcactttctcgtcgccttcggcggccttgatgagcgagcggatggcggtgggggcggtgtagaagacgctgaccttgtgcttctcgatcatctgccagaagcgcccggcgtgcgggaaggtggggatgccttcgaacaccacctgggtggcgccggcggccagcgggccgtaggccacgtaggtgtggccggtgatccagccgatgtcggcggtgcaccagaacacgtcttcgggccggatgtcgaaggtccagtccatggtgagccgggcccacagcaggtagccgccggtggcgtgctgcacgcccttgggcttgccggtggagccggaggtgtagaggatgaagagggggtgctcggcgttcacgggcacgggcgggcagtcggtgctctggccctggagggcctcggcgaagctctggtcgcggccttcgacgcgattccaggcggtgggggtgcgctcgtagacgaacacggcccggatcgactcgcagccgcccatggcgatgccgtcgtccacgatggctttgaggggcagctccttgccgccgcgcagctggtagttggcggtgatgacggccacggcgccggcgtcgatgatgcgctcttgcagggccttggccgagaagccgccgaacacgacgctgtgggtggcgccgatgcgcgcgcaggcctgcatggcgacgacgccttcgacggtcatgggcatgtagacgatgacgcggtcgcccttttggatgccggcggccttcagggcgttggcgaactggctcacgcgggcgagcagttccttgtagctgacgcgggtgacggcgccgtcgtcggcctcgaagacgatggcggtcttgtgttcgacgggggtgccgatgtgccggtccaggcagttggcgctggcgttgagttcgccgtcgccgaaccattggtagaagggggcgttggattcgtccagggtcttggtgaagggcttggtccaggtgaggttgtccttcgccaggcgggtccagaagccttcgaagtcctgctcggcttcctggcacagggcttcgtaggcggccatgcccgagatgcgcgcgccggcgctggcgcgggcgtcgggtgggaatacgcggttctctacgaggacggattcgatgttcttggatgcgctgctgctcattttcttgtctcctgggtaggtgcggccgtaatgtcggcgggcccacttacgggtcactgacgggttcgtccaggtccgatgttagttcgcagggttatcacgagtcggacacaagggcacctctagaatcgccggtcgttcccaacctcccgtccaatgtccgctcccgaccctttcgaccgcccccacacgcccgccgccgcctcgcccctgcggccactccccaagctgatcttcgcgagccgctggctgcagctgccgctgtacctgggcctgatcgtggcgcaggcggtgtacgtggtgcacttcctggtcgagctgctgcatctggtcgaggcggccttcggcagcaaggacgcgctgcaggccctgatcaccagcatcggctacaagacgaccgcgccggtgggcacactcaatgaaacggtgatcatgctggtggtgctggcgctgatcgacgtggtgatgatctcgaacctgctcatcatggtgatcgtgggcggctacgaaaccttcgtgagccgcatggacctcgaaggccatcgcgaccagcccgagtggctgagccatgtgaacgcctcggtgctcaaggtgaagctggccaccgccatcatcggcatcagctcgatccatctgctgaagaccttcatcaacgcggacaactacaccgaccgcgttctgattgcgcagaccgtgatccacatcgcattcctgttctcggccatggccattgcctacaccgacaagctcatgacgtcgaacgcgccgcaaggcggcggctcgcactgagccctgcccgcttctagcctgcgtgcggcagatcccacgcgggcacgtcggtgaattgctcggccagaaagtcgagcatcgtgcgcagcgcggccggcatgtgcttgcgcgaggcatacaccgcgtacatgcccaccacctgcggttcgcaatcagggaagagcggcaccagttcgccggccttcacgaggccggccgtcaggtaggtcggcagcatcgcaatgcccgccccggaccgcgccagctgcatcaggctcgcagcatcgttggtcgacaggttgccgcccacggccaccgagaccggctccccgttgtccttgcgcgtgaaattccagaggctgcgcccgaagtacgagtgcgtgaggcaattgcgctgggccagctcctccacgcgcacaggcttgccgtgttccttcaggtagccgggtgacgcgcaaaccaccgaccggcagtcggtgagccgccgcgcgatcaggttgggatcgatctccaccgccacccgaatggcgagatcgatgcgctcgtccaccaggttcaccgcgcggtcgagcagcaccaggtcgaccgccaccccggggtacagccgcacgtaatcggccacggcgccggccagttgcgcctgcgcgaaggaagtgctggccgtgatgcgcaattggccccgcggcgcctcggccgggtgccgcacggcggcctgcatgtcgcccgcgagttcgagcacttggcggcagcgcggcagcagttcctcgccggccgccgtgaggctcagccggcgcgtcgtgcggtgcagcaggcgcgcgccggtccattgctcgagttcggccacgtagcgcgtgaccaccggccgggaaagatcgagcttgtcggccgcggccgaaaggctgcccgagtcgaccaccgtgacgaacacgcgcattgcattcaatcgatccattcgaacgattttaggaataaacaagcgcgaaattcgaggtatttctttcgaaagcagaaacctaagatgcgcttcatcgcatcaacttttcaggagcattcatgagccacatcgccatcatcggcgccaccggacgcgctggcggccgccttctcgaggaggccctgcgccgcggccacaccgtgaccgccattgcgcgcaaggccagcgaaaagctgtcgggccgcgccgatgtgaagcccatcgacgtcgacgtgctcgacgcacccgcgctcgaaaaggcgctggccgggcatgacgccgtgttcagcgccgcgcacttctccacggtaccgcccgccgccatcatcgagcccgccaagcgcgccggcgtgaagcgcctgctggtggtcggcggcgccggcagcctgttcgcagcgccgggcctgaaggtgatcgacacgccgaatttccccgaggcgtacaaggccgaggcttcggcgggcgccgcgttcctggaggtgctgcgaagcgagaaggaactcgactggacctttctttcgccttccgccgaattcgtcgaaggcgagcgcacgggcaagttccgcctgggcaaggacgacctgctcgtgagcgccgagggccgcagctggatcagcttcgaggactacgcgatcgcgttcatcgacgaactcgaaaagcaggcccattcgcgccagcgctacacggtcggctattgatcggctcgatcggcctgatcggccggccgcaaaaaaaggacccgcacgggtcctttttttcgccttccggattcaccggccggtcatgttctcaggcaccacccactggtcgaactgctcggccgtgaggtggcccgaggcaatcgccgcctcgcgcaggctcgtgccctccttgtgtgccttcttcgcgatgtaggccgacttgtcgtagccgatgtgcgtgttgagcgcagtcaccagcatcagcgagcgctggaccagctcggtgatgcgctcgcggttcggctcgatgcccacggcgcagtggtcgttgaagctcaccatgccatcggccaggaggcgcacgctctgcaggaagttgtgctccaccatcgggcggaacacgttcagttcgaagttgcccgaggcgccgccgatgttgatggccacgtcgttgccgaacacctgcgcagccagcatcgtgacggcttcgctctgagtcggattgaccttgcccggcatgatcgacgagccgggctcgttctcgggaatgctgagttcgccaatgccgctgcgcggcccgctcgcaagccagcgcacgtcgttggcaatcttggtcatgctggccgcgagcgtcttgagcgcgccgtgggcatgcaccagcgcatcgacgctggccatggattcgaacttgttcggtgcggtcacgaaaggcaggcccgtgagcgtcgccaactcggccgccacctgctccgcgtagcctttgggcgcattgagtccggtgccgacggccgtgccgcccagcgccagttcgcacaggtgcggcagcgccgcgcgcacatgcgcctcgccgtgcgccaattgcgccacgtagcccgagaactcctggcccagcgtgagcggcgtggcgtcctgcagatgggtgcggccgatcttcacgatgtcggcgaagtccttcgactttttctccagcgtgccgcgcagcttggcaatggcgggcaacagcttgtgcgtgatggcctcgacggcggccacgtgcatggccgtggggaacacgtcgttgctcgactggctgcggttcacgtcgtcgttcgggtgcacgaggcgcccttccccacgctcgccgccgagcagctcgctcgcgcggttggccagcacctcgttgacgttcatgttggtctgcgtgcccgagccggtttgccagaccacgagcggaaactcgcccgggtgcttgcccgcgatgacttcgtcggccgcggccacgatggcctgggtcttcttgtcgtcctgcagcccgagcgcatggttgaccaccgccgaggcacgcttgacctgcgccagcgccttgatgatctcgcgcggctgctgctcgccggaaatgtcgaagttctgcagcgagcgctgcgtttgcgcaccccacagcttgtccgccggcacgtcgatcgggccgaacgtgtcgcgctcggcacgggtcttgggggaagtcgtcatgatgaaaaaagctccgcggtcttgaatggttgcgcccgctcaccgggcgcggtgccgagtatggcctcgataagaatggctcgcatttgcctaggcttattcgccccggacgcccggcccacgatacgccccgggcttgactcacgtaatgtcaaaaagttataattgcgggcttcagacgaccaacaagtcatgttggttgcccttgcgctactcgcggatcaccgaatcccgtcgcggtgcaaggctctccccgccgggccctgcccggcaacccggccggatctttccggccccattgccacgtcacgctcatccaggcggcgcccctcgaccaggcccgccgctctgcgaatgaagcatccggcgggcactggcttcgtcgccatgtcgtcttcagtgcctgtcggcagccttcgaggctcgccgggccattgcacgcgcgtttttcacgcgctctgttcgggcagccccatcggctgatggcgtggccgttgccgccctccggggcggcgctgtgtccaaccatcacacaaggagccccggcgtatggccaaaggaattctcatcgaccatgttttcaaggtgttcggcgactcgcccgaacaggcgctcgaacgggtccggcaaggtttttcgaaaaaggaaatcctcgcgcagacgggccagtcgatcggcgtgttcgatgccaccttcgaaatccaggccggcgagatcttcgtcatcatgggcctctcggggtcgggcaaatcgacgctggtgcgcctgttgaaccggctgatcgagccgaccgcgggccgcatcgtgatcgatggcgccgacatcaacgaacattccgacgccaagctgcgcgcactgcgccgcaaggacatcagcatggtgttccagtccttcgcgttgatgccgcacatgacggtgcgcgagaacacggccttcggcctcgaactgtcgggcaccagcaagaaggaacgcctcgcgcaggccgacctggcgctcgcgcaggtgggtcttgcgggctggggcgacagttatcccgacgagctctcgggcggcatgcagcagcgcgtgggcctggcgcgggcgctggcttccgatccgtcgatcctgctgatggacgaggccttctcggccctcgacccgatcatccgcaccgagatgcagtcggagctgttgcggctgcagaaggaacagcgccgcaccatcgtcttcatctcgcacgacctggacgaggccatgcgcatcggcgaccgcatcgcgatcatgaaggacggccaggtgatccaggtcggcacgccagacgagatcttgcgcagcccggccgacgactacgtgcgcagcttcgtgcgcggggtggacgcggcggccgtgttcaaggcggcggacatcgcgcgcaagtcgctcaccgtggtctgcgagcaccccgagcgcggtgcgcatgcggcactcaaggtgctggaagaccaggaccgcgacttcgcctacgtgacgagcccgaccaggcgctacctgggcaccgtgtcggccgatacgctgcgcgcggcgctcgacgggcattcgggcccgctggggctgcgccacgcgttcctgaacgacctgggcgtgatcgaggccgacgcccccgtggccggcctgatcggccaggtgggccaggcgccgtgtgccatgcccgtggtggccggcgacggccgcttctgcggtgcgatcagcaagacgacgctgctgaagtttctcgaccgcgacacgccgccgatcgacccggcgcaccagcgccagcaacccgtccctgctgcggccgccatggccgttgcctgatcgacttcgaaggaccccttgatgaacgacaccgcactgccctccgaactcgcgcccttgaacgacgcttccaccgccgtggccccgcaagcagcggcaccggccgatccctgggccgccctgtccgccgcccccgacgcctccgcgaccagcgcctggctcgacgcccccgtcgacacggctcgtcagctggccggatcggccgacgccgccaccggcggcttccaattgcaccgcctctgggacggctcgctgcccgtcgaatcctggatcaaccagggcctcggctgggtggtcgagcacttccgcccgttcttccagaccgtgcgcctgcccatcgacagcacgctgaactgggtgcagagcctgctgaccggcctgccgacgctcgcgatgatcgcgttgatcggcctcttcgcctggcagttcgcgggccgcgcgctcgccttcggcaccacggcggcgctgctgctcgtggccatgctgggcatctggcccgaagccatggtgacgctgtcgctggtgctgacctcgttggtcttctgcatggtcatcggcctgccgctcggcgtgctgctggccagcagcgaccgcgcccagcgcctcacgcgcccggtgctcgacgcgatgcagaccacgcccgccttcgtctacctggtgccggtggtgatgctgttcggcatcggcaacgtgccgggcgtgatcgtgaccatcatctttgcgctggcgccgctggtgcgcctgaccaacctgggcctgcgccaggtgcggcccgacctgatcgaggccgcgcgcgcctacggcgcctcgccgtggcagatgctggtgaaggtgcaactgccgctggccatgccctcgatcatggcgggcatcaaccaggcactgatgctgtcgctgtcgatggtggtgatcgcctcgatgatcgcggtcggcggcctgggccagatggtgctgcgcggcatcggccggctcgacatgggcctggcgaccgtgggcggcctgggcatcgtgctgctggcgatctcgctcgaccgcctcacgcaagccatgggcaagtcgcgccgcagcgccgggcgccgctggtggcacaccgggccggccggctttgcgctgcatctgctgcagcgcctggcgagcacgccgccgcgtggtgcgaacgaacctgttcccgccctgtccacgcaagcgcaatgagcgcccacgaaggaatccaacgcatgaagaaaacccgtctccatcacatcgcccgcggcctgctggcgctcggcttcgtcgctttcggcatggctgcgcaggccgccaacgacctgcccggcaagggcattaccgtgcaaccgctcaagagctcgctcgccgaagaggcgttccagaccctgctcgtgatgcgcgcgctcgaaaagctcggctacaccgccctgcccatgaaagacctcgaacccgccaccgaacacctggccatcgccaacggcgacgccactttcatggccaaccactggagcctgctgcacgccgacttctacaagaacagcggcggcgacgccaagctgtggcgcaagggcgtgtactcggacggcgcggtgcagggctacctcatcgaccgcaagacggccgagcaacacaacatcaccaacatcgcccagctgaaggacccggccatcgcgaagctgttcgacgccgacggcgacggcaaggccgacctgacgggctgcaaccccggctggggctgcgaactggcgatcgagaaccacctgacggcctaccagctgcgcgacaccgtcacgcacaagcaaggcagctacgccgcgctgatggccgacaccattgcccgcttcaagcaggacaagccggtgctgtactacacctggacgccctactgggtcagcgccgtgctgcggcccggcgcggacgtggtgtggctgcaggtgccgttttcttcctcgcagggtgggaacgcggacacgcggcttccgaacggcaagaactacggcttccaggccaaccaggagcagatcgtcgccaacaaggccttcgtcgagaagaatcccgcggccggcaagctgttcgaggtgatgaaactgccgatcggcgacatcaacgcccagaacctgcgcatgagccagggcgccaacacccagcaagacctggagcgccaaaccgacgcctggatccgggtccaccggccgctgttcgacggctggatcgaggaagcccgggccgccgcaaggtagcgcgacggggccgggcgcggcggctgagataatcggggggcgtttccacactccaaaaaacaccccccaccatgacgaccacgatccagcaggccgacctgatcgaatcgatcagcgccgcgctgcagtacatcagctactaccaccccgccgactacatcgcccacctggccaaggcctacgagcgcgagcagagccccgccgccaaggacgccattgcgcagatcctgaccaacagcaagatgagcgccacgggccaccgcccgatctgccaggacaccggcatcgtcaacgtgttcctcaaggtgggcatggacgtgcgctggggcggcttcaccggttcgctggacgacgccgtcaacgaaggcgtgcgccgcggctacaaccaccccgacaacacgctgcgcgcctcggtcgtggccgacccgcagttcgatcgcaagaacaccaaggacaacacgcccgcggtgatcttcaccgagatcgttccgggcaataccgtcgaagtgaccgtggcggccaagggcggcggcagcgagaacaagagcaagctcgtgatgctgaaccccggcgacagcgtggtcgactgggtgctcaagacggtgccgaccatgggcgccggctggtgcccgccaggcatgctgggcatcggcatcggcggcacggccgagaaggccgcgctgatggccaaggaaagcctgatggacgacctcgacatgcacgagctgcaggccaagaaggcctcgggcgccgagctcagcaaggtcgaggcgctgcgcatcgagctgtacgagaaggtcaacgcgctgggcatcggcgcgcagggcctgggcggcctggccaccgtgctcgacatcaagatcaagatgtacccgacccacgcagccagcaagcccgtggcaatgatccccaattgcgcggccacccgccacgcgcacttcgtgatggacggcagcggcgcggtctacctcgacccgccgtcgctcgacctgtggcccgacgtcaactgggcgcccgacgagaagaagagcaagcgcgtcgacctggacaagctcacgcccgccgaagtggcgagctggaagcccggcgacaccctgctgctcaacggcaagatgctcaccggccgagacgccgcgcacaagcgcatccaggacatgctggccaagggcgagaagctgccggtggacttcaccaaccgcgtcatctactacgtcggcccggtcgacccggtgggcgacgaggccgtgggccccgccggcccgaccaccgcgacgcgcatggacggcttcaccgagatgatgctggccgaaaccggcctgatcgcgatgatcggcaaggccgagcgcggcccggtcgccatcgaggccatcaagaagcacaagagcgcctatctcatggccgtgggcggcgccgcctacctcgtgagcaaggccatcaagaccgccaaggtggtgggcttcgaggacctgggcatggaagccatctatgaattcgacgtggtcgacatgcccgtgacggtagcggtcgatgccggcggcaccagcgcgcacatcaccggcccggccgagtggcagaagcgcattgcgagcggcgagttcaagaccatcatgatggaagaagcttgaaacccatcggagtgttcgacagcggcgtcggcgggctcagcgtgcttgccgcgctgcgcgccgagctgccgcacgagcgcttcgtctacttcgccgacacggcctatgcgccgtatggcgaacgcggcgacgactacgtgatcgagcgctcgcgcaaggtggccgaacagctgatcggcgagcacggcatcaaggcgttggtcgtggcctgcaacacggccaccacggcggcgatccacctgctgcgtgccgagtatccggccttgcccatcgtgggcctggagcctgcactcaagcccgccgtggcgacgagccgcaccggccacatctcggtgatggcgacgcgcggaacgctggccagcgccaagtacgcggcgctgcgcgactctttcgctgggtctgcgaatgtccgcgccgtgccatgcgacggcctcgtgaaagccatcgaaggcttcgacaccgcggccatcgaggcgctctgcgcgcgctacatggccgaggcgggccccttcggcgatgggccgggccaagtcgataccgtcgtgctcggctgcacgcactacccgctcgtgaaaagcgaactgcagcgccatgcgccaaccgcgctgcgcttcatcgataccggcgcgccggtcgcgctgcagacccggcgcgtgctggcgtcgattggccgcctggcggacagcggcgaaggcggcttggtcctgcaaggcagcggcgatctggccgtgctcgaagccgcagccgcgcactggctgcaacggcggccgcaagctgcgacggcagctgccgcaaccgccacctgaaccccgacccgcatgcgtccccttttgcgtcacggcttgctcctgctgtgcctttcggccgcgggcctcggccatgccgcctgcgagagcggcctggccgaacgcatgcacgccaagctgcatccgaaccgcacgctcgacgagcgcctggccgcctgcaagccatggcccgccttcccggggcgcagcatcgtggtgctgcccgtgccgcgcgagaccagcagcacgggcgccaaggtcttcgatctcgagctgctgctgatccagcggcccgacaacggcaacaccgaacgcgacacggtgatcggccgcatcttccagcccgaggcgctcgacgaagacagtgcgaccgcgatccaggacatccggatcgacaccgcgcgctatgttctgtcggccgacacgcgcgccttcgggctgcgcgtgcgctaccgtggcacagcgccgggcagttcggttgcgagcgaatccattcgcctctacgtgcaccacggcagcaagcttcggcaggtgctgcaggaggtcgagctcgaccacgacagcggcggatgggacagcacctgcaccggccgactcgagaaactgcgcaccatgctttcggtgggcaaatcgtcgagcaacggctacgccgacctgcaactcgcgcgcacgctggtccagagccacgcacagctgcaggaagaccagggctgcgccgagaaaaccctgcccgcgcgattcaacaccgtgacgctgcgctacgacggcgagcgctaccgggtgcccaagtccctgcagcagcaggtgccctgagccacaggccctatcggctgcctactaccggctgcgcaaagcggcttcgcggccgcgcgccatgtcgatgggcagcaacagcagcagacccgccacgaagagcgccgcggtcgagagaatggcgatgcgctggttgccgcccgcggcccacgtgatggcgccgaacatcagcgggccgatgatgcttgccaggcgcgtggcgaaggtccagagcccgaagaattcggccagctgccgcggcggcgcaaggtagccggtcatggcccggccggccgactggctcgagcccatggcaagccctgcaatggcggcggcccaccagaaggtgcccttggtggtcgccagcgcggcaatcacgcagaccgcgatccacgccaccagcgtgccggccagcgagaccttgtggccgacgcggtcctgcacatagccgaaggcaaaggcgccgaccgcggccgcgatgttgagcacgaagatcagcaccatggtctcgctcgccacgaagccgatgacctgttcggcatagatggccgccagcgtgatggccaccgccacgccgccctggtagcacacggtgcagaccagcagccacatgaagtcgcggtaggcgcgcgcctcgcggaacgtggcacgcaactgccgccaggcgctcggcgcgccgccggccgttcggggccgcgcgcgctcgggcagcagcgcaaaagtggcgcaggccgccgtgccgtagatggcggccgtgatcagcatcgtgaccggtacgaagtgcgatgccggcaaccccttggcttgcgaggacagcacgtaggccaggcacaagccaagtgcgagcatgccgccgacgtagccgaaggcccaaccccatccgctgaccttgcccatgccctcggccgttgcgagctcgggcaggaaggcaccggtcagcgactcgccgtacgaatagaaggtgttggagacaatcaccagtcccatggccaccgcgacgcctgcggcgcccgaaaagcttggcgtgagcgcaagcgcggcggtgccaagcacgcagcccgctgtcgcaacggccagcacacgcttcttggctgcgtgccggtcggcccaggccccgatggcgggcatggagagcatcacgatggcataggagacgctgagcgccgcggtccatgcaaacgcggcccatggcgcgcccttggcgatgccgcccacgaagtaagcggcaaacacggccgtgatgacgaccgtggtgtagcccgaattcgcgaagtcgtacatcgcccagccgaacacctcgcgcttgcgcacgccggcgttcagggcggaagacgggaacagcgccatgcggcggtgaatggcggcgccaggagagcgggctggcctgcgcgtcagtgcaggtggcgcggacggcgaccaccgccatgcccaccaccgccgctgccactgccgccggtgccgcgcgggcgcttgccgatctcgagcgaattcacgagcgcatcgaagcggtcgctgaagaggcgatcgatttcggacaccacgccgccgagttcggcgccatcgaagtggcgctccatcaggttgacgacgtcttccaccagcaggtcgcgctgcacctgcatgatcgcggccggattggggccgacgaacagcatcaggaaatcgtcgcgcgattcttcgtcggggtcgccctcttcctcgtcgaagtcggtgtcgtagaaggtgacctcgatggcggcaccgcgttccgacagttcgttcagcgccatgcacatctcgtcgagcgcctggcgaaagtcgtcgtcgccgggcacggtccagcacatctggagcatgtggtccttctgctcgaaacggatgccgggctcttcttcgtaggtgctcgtggcgccgtcggccagcgacttggcgcccgaataggcccacagcggcttgagtgcttcttggatctggtcgaaggtgacgtcagaccgcagcggcacgtcgccgtgcacatgaatttcaaatggagcgttgtaacgaggcatggagtgctcccttgtctaagtatggtgcccggaacgggggtcgaacccgtatgccccgattaaggaagcggcggattttaagtccgatgtgtctaccaatttcaccatccgggcctcgggtttgaacatcgacgataacccaaacgcaacgagccccggcaacgcaggttggcggggctattttcgatggaggttggatcgaactgatcaggagaggtggaggcgcgacccggagtcgaaccgggctagacggatttgcaatccgttgcataaccgctttgctatcgcgccacgctgctgaaaacgaaatcgaactcgcgaaaaaaagggaagcagtgcttccctttttcaaaactggagcgggaaaagagtctcgaactctcgacctcaaccttggcaaggttgcgctctaccaactgagctattcccgcgtttcgagcctcgaattatagaacactttttcggggctcggcaagttccgccaatcaatgtttgacggagccctcagaggcctgcgttccgcgctgcttggccagctcggccacggcagcggcggaggccgcgacttcctcgtcggacaacggctcgggcatcttctcgagcgcgatctccaggaccttgtcgatccacttcaccggcacgatctcgaggccgttcttcacgttctcgggaatgtcctgcaagtctttcgcgttctcttcgggaatcagcacggtcttgatgccgccgcgcagcgctgcgagcagcttttccttcaggccgccgatggccgtgacctcgccgcgcagcgtgatctcgccggtcatggcgacgtcggcacgcacggggatgcccgtcagcgccgacacgaaggcggtggtcatcgcggcgcccgcgctcgggccgtccttgggcgttgcgccatcgggcacgtggatgtggatgtcgcgcttctcgaacacctcgtccttgatgcccaggcgtcgcgagcggctgcgcacaaccgtgcgcgcggcctcgaccgattccttcatcacgtcgccgagcgaacccgtgcggctgatcacacccttgccgggcatggtgacggcctcgatggtgagcaggtcgccgcccacttcggtccacgccagaccgaccacctggccgacctggttctgcttctcggccaggccgaagctgtacttgcgaacgcccaggaactcgttgaggttggcgccgtccaccgtaaccttcggcgtcatctgcttgagcagcaggcccttcactaccttgcggcagatcttggagagctcgcgctccagcgaacgcacgccggcctcacgcgtgtagtagcgcacgatgtcgcgcacggcttcttcggagacgagcaactcgtcttccttcacgccgttgttcttcatctgcttgggcagcaggtacttgatcgcgatgttggtcttctcgtcctcggtgtagcccgagaggcggatgacttccatccggtcgagcagcgccggcgggatgttcatcgagttggaggtggcgacgaacatcacgtcggagaggtcgaagtcgacctcgacgtagtggtcgccgaaggtgtggttctgctccgggtcgagcacctcgagcagcgcgctcgacggatcgccgcggaagtcggtgcccagcttgtcgatctcgtcgagcaggaacagcggattgcgcgtgccgatcttgttcagcccctgcagcaccttgcccggcagcgcgccgatgtaggtgcggcgatggccgcgaatctcggcctcgtcgcgcatgccgccgagcgccatgcgggtgtacttgcggccggtcgccttggcgatcgactgcccgagcgaggtcttgcccacgcccggtgggcccacgaggcacaggatgggcgccttgaccttgtcgacgcgttgctgcaccgcgagatattccaggatgcggtccttgaccttctccaggccgtagtggtcggcattgagcaccgcctcggcgttggccaggtcgtgcttgatcttggtcttcttgctccagggcaggcccaccagcacgtcgatgtagttgcgcaccacggtggcttcggccgacatcggcgacatcagcttgagcttcttgagctcgccctcggccttcttgagcgcttccttcggcatcttggcgagcttgatcttcttctcgatctcctcgatgtccgcgccctcttcgccttcgccgagctccttctggatcgccttgacctgctcgttgagatagaagtcgcgctggttcttttccatctggcgcttcacgcggccacggatcttcttgtcgacgttgaggatgtcgacttcgcgttcgagctggccgaacaggttctccaggcgcgacttgacgtcggccaggtcgagcacggcctgcttgttgtcgagcttcagcggcagatgggccgcgatggtgtcggccaggcggcccggatcgtcgatgctcgagatcgaggtgaggatctctggcgggatcttcttgttgagcttgacgtactgatcgaactgctgcatcaccgcacggcgcaacgcctcgacctcggtgcccttctcgccgccttcgggcgcctcgaccggcgtcacgttggccgtgaaatgggtttcaccgtcgtcgatgcggttcacgcgggcgcgctgctggccctcgaccagcaccttcacggtaccgtcgggcagcttcagcatctgcaggatggtggagacgcagccgacttcgaacatgtcctcgaccgagggctcgtccttggcggcggctttctgcgccaccagcatgatgcggcgctcggcctccatggccagctcgagtgccttgatgctcttggggcgccccacgaaaagcggaatcaccatgtggggaaacacgacaacgtcgcgcagcggcagcagcggcaggtcgatcgcgtcggcaggcaggggggtatgaccggacatgaatatcctttgattgatcaggcaaagatggatgggcctgcgggcatttcaagcccgtgcacccgttctttgtcgaaggcgccggaagcctcggtgagaagagccggcgccgcgttcactcaggccttcttggccgcttcgcggtacacgagcagcggcggcttgttttcatcgattgtggattcttcgaccacaaccttgtcgacgttggtggcattcggcagctcgaacatggtgtcgatcagcgactgttcgaggatggagcgcaacccgcgcgcgccggtcttgcgtgccagcgccttgcgcgcaatcgccttgagcgccgcggggcggatctccaggtcgacgccttccatctgcagcagcttggtgaactgcttgaccacggcgttcttgggctcggtcaggatctgcaccagcgcgtcttcgctgagctcggccagcgaggccaccacgggcatgcggcccacgagctcgggaatcaggccgaacttgatcaggtcttcgggttcgacttcgcggaacacctcggtgatgctgcgctgcgccttgctcttgaccgaggcgccgaagccgatgcccgaggcctcggtgcggttttcgatgactttctcgaggccggcaaaggcgccgccgcagatgaacaggatgttggtcgtgtcgatctgcaggaagtcctggttcgggtgcttgcgcccgccctggggcggcacgctggccatggtgccttcgatgagcttcaggagcgcctgctgcacgccctcgcccgacacgtcgcgggtgatggaggggttgtccgacttgcgcgagatcttgtcgatttcatcgatgtagacaatgccgcgctgggcgcgctcgacttcgtagttgcagctttgcagcagcttctggatgatgttctcgacgtcctcgcccacgtagccggcttcggtcagcgtggtggcgtcggccatgacgaagggcacgtcgagcatgcgcgcgagggtttgcgcgagcagcgtcttgcccgagcccgtgggcccgatcaggagaatgttgctcttgctgagctcgacgtcgtcgcccttggccttttccttgtggcgcaggcgcttgtagtggttgtagaccgccaccgacagcatgcgcttggccggctcctggccgatcacgtagttgtcgaggttggtcttgatctccagcggcgtgggcaggtcgctgcgcgcctcgcgcgcctcttcaccggccgggagctcgtcgcggatgatttcgttgcaaaggtcgatgcactcgtcgcaaatgaagaccgaagggcccgcgatcagcttcttgacctcatgctggctcttgccgcagaacgagcaataaagcgttttttcgctggaggagccttttttttcggccatggacaggtgcctcgtaaaggggtagggacaatgataacgaaacaaaaacggcgtttcccttgtggaaaacgccgtttttgtctttttggcgccaccggcgccgtggcgcaggttttaccgatcaaccgcgcttggcaatgacctggtcgaccaggccgtagtccttggcttcgtcagcggtcaggaaatagtcgcgttcggtgtccgacttgactttttcgagcggctggcccgtgcgttcggccaggatgcggttcatctggtccttggtgcgcaggatgtcgcgggcatgaatctcgatgtccgtggcctggccgcgcgcgccgccgagcacctggtggatcatgatcttcgaattgggcagcgagaagcgcttgcccttttcaccggccgccagcaggaaggcgcccatgctggccgcaaaaccgatgcacatcgtcgacacgtcgggcttgatgaactgcatggtgtcgtagatggccatgccggcgctcacgctgccgcccggggagttgatgtagaacgaaatgtccttgtccgggttctcgctctccaggaacagcagctgcgccaccacgagattggcggtctggtcgttgacctcgcccaccaggaagatgatgcgttccttgagaagacgcgaatagatgtcgtaggaccgctcgccgcggcccgactgctcgatgaccatcgggatcatgccgaggcctttgatttcctgtgcgctcattgatttgctctccggaaggggttcgttcgctgttcgtatttgactgtacgcctgagtgaaatggggctcgtgccgcaaagcacaagccccattggcgtcgcgggcggaggcgcggggcggacccccggcgcggcgctcagccctgctgctgcgccatcagctcgtcgaacgtcaccgacttttcgttgaccttggccttggcgagcacgaattcggtcacgttgttctcgatcaccacagcctcgacttcggccaggcgattgttgtcgctgaaataccagcgcaccacgtcggccggcttttcgtagctggcggccagctcgtcgatgtgggccttgatctgctcgggcttggcctgcaggttgttggcgcgcaccagctcggccaccaccaggcccaggcgcacgcggcgctcggcttgcggacggaacacttcgtcgggaatcggtgccttgtcggcgtccttgatgccgcgctgcttgagctcggcgcgggcgccttcgaccatgcggttcacttcggactgcacgctggcgttcggcaggtcgagctcagcattggccaccagggtgtccatcacggcattcttgttgcgggccagcaggcggaacttcacttcgcgctcgaggttcttcttgatgtcggcgcgcaggccttcgaccgtggcttcggcaatgccgagcgacttggcgagctgttcgttgacttcgggcaggtgcgaggcctcgatcttcttcacggtgaccatgaagtcggcttgcttgccggccacgtccttgccgtggtagtcggccgggaacgacagcgggaaggtgcggctgtcgccggccttcatgccgcgcacggcgtcttcgaattccttcagcatctggccttcgccgaccacgaactggaagtcttcggccttgccgccctggaagggctcgccgtcgatcttgccttcgaagtcgaccgtcacgcgatcgtcgtcctgggccacggcgtcttgcgcgcgctgggcgaaggtgcggcgctggcggcgcaggatgtcgagcgtcttgtcgatcgcgtcgtcgcccacttcggccgagagcttctcgacttcggcgcccgacaggtcgttgatcttgacctcggggaacacctcgaacaccgcgtcgaaggcgagctggccttcgggcgactcttccttctcggtgatgcggggctggccggccacgcgcagcttggcttcgttggcggcttgcgagaaggcttcaccgaccttgtcgttcatgacttcgtagtgcaccgagtagccatagcgctgggccacgacgttcatcggcaccttgcccggacggaagccgtccatcttgacggtgcgcgcgagcttcttgaggcgcgaatcgacttcggactggatggtgccgaccggcagggtcagcgtgatcttgcgttcgagcttctcgagagtttcaacggtcacggtcatggtgtcttccttgtgaggggtgtggctggtgcgcggggccggactcgaaccggcacgttcttgcgaacgtcaggacctaaacctggtgcgtctaccaatttcgccacccgcgcttgccaaatttttcaggtgaatgcaaaggcggacggccctggtgcagcgaacctccgataccggatatccgccgcccaaagaccgtccgcctgaaatcggtcaacctgctattttaagcgctaatcggaagctctttcggctcccgcttgacgcggaacgccgcggcgtacattgccggcagtgccagcagggtcaataccgtcgccacgatcaggccgcccatgatggccacggccatcggcccccagaaaacgctgcgcgacagcgggatcatcgccagcacggccgccgcagccgtgagcacgatcggccggaggcgccgcacggccgattcgacgatggcgtcccaggccggcacgcccgcctcgcggtcgctttcgatctggtcgatcaggatcaccgcgttgcgctggatcatgcccatcagcgcgatcacgcccaggagagccacgaagccgaacggccggttcagcaacagcagcgcaccggccacgccggcaatgcccatggggccggtgatgaacaccagtagcgagcggctgaagctgtgcagctggagcatcagcagggtgaacaccacgaacagcatgatcggcacgcccgcgacgatggaggtcgagcccttgctgctttcctcgaccgcgccggccacttcgatgcggtatccgccctgcccggccgcgtgccagccggcttcgagctgacgcagcttcggcagcagctgctcggtcaccgtggcgccctgcaggccttcgaccacgtcgccctgcaccgtgatggcgtagtcccggttctcgcgccacatcacgccgggttcccagctgaacaccggccgcgcgatctgggtcagcggaatcgaacggcccgacgtggtgggcagataggcattgccgatgtccgagatggcctcgcgctcgtccgccgactggcgcagcacgatgtcgatcagcaggtcgttctcgcgatactggcccaccgtggtgccggagaacatcgtcttggaggcctgtgcgatcgcctggctggtgacgccgagcgcgcgcgccttggcctggtcgacctcgagacggatcaccttgaccgattcgttccagttgtcgttcacgccgcgcatgttggcgttctcgcgcagcacggccttgacttcgtcggcatgggcgcgcagttgcgcgggctcggtgccgatgacgcggaactgcaccgggtacggcaccggcggcccgttgggcagcaatttcacacggccgcgcacttcaggaaactcctgcgccagcagggccggtagcttgatgcgcaggctctcccgaaccttcaggtccttggccagcacgatgagctgagacacgttggtctgcggaaacacctggtcgagcggcaggtagaagcgcggcacgccggagccgatccaggtgctgaccgtcttcacgccctcttccttcatgatgcgctgctcgacccgcttggcaacctcttcgttcgcgaggaacgaggtgccttcggggaaccagatgtcgaccatgatctcgggccggctcgaatccgggaagaactgctgctgcaccttgcccatgccgaagatgcccagcgcaaagatcagcaccgtggcgccgatggtcagccagcgatgctgcacgcaccagttcaccgtgcggcggaaggtgttgtagaacggtgtgtcgaacagctcgtgcggcggcgcatcggggtcgtgcggcttcaccttgagcagcagcgtgccgaggtaaggcacgaagtacaccgagacgatccacgacagcaccagcgcaatcaccgtcactgcaaagatcgcgaaggtgtattcgcccgtcaccgacttggcgaggccgatgggcaggaagcccgcggcggtgatgagcgtgccggtgagcatgggcttggccgtcacgtcgtacgcgaaggtggcggcgcggaccttgtcatagccctcttccatcttccgcaccatcatttcgaccgcgatgatcgcgtcgtcgaccagaaggccgagcgcgatgatcagcgaccccagcgatatcttgtgcagcccgatgttgaagtagttcatggccaggaaggtcacggccagcaccaggggaatggtgatggccaccaccagccccgggcgcatgtcgatgtaccagccgaagcgcccgcccttgtgcaggcccagcgagatgatgctcacggccagcacgatggccaccgcctcgatcagcacgccgacgaattcattcaccgagctggccaccgacaccggttggtcctgcacctgcgccagcttgacgccggccggcaggcgctggtcgatcgtcgccgtggtggcgcgcagcgcctcgcccagcgcaatgatgtcgccgcccttggccatggaaacgcccagcgcgatgacctccttgccctggtggtgcaccttgaccgccggcggatcgacgtagccgcggcgaagttcggcaatgtcgccgagcttcagctggttgcccgaactgccgcggatcggcatctcgcgcagctgctcgacactggtgaactgcccggccacgcgcacctgcaccacgtcggcgggcgactggatcgtgccggcgctttccactgcgttctgggagccgagctgggccagcaccgcattgaagtccagacccagttgcgccaggcgcttctgcgagatctcgatgtagaccttttcgtcctgcacgccgaactggtcgaccttggcaacgtccttcacgcgcagcaattgctggcgcacttcgtcggccagggtcttgagctcggcgtagctgaagccttcgctctccagcgcgtagatcacgccatagacatcgccgaaatcgtcattgaagaacgggccctggatgccagccggcaacgtgttgcggatgtcgccgatcttcttgcgcaccgtgtaccagacgttggcaacgtcgccgggcttggaggagtccttgatctggaaaatgatctgcgactcgccgggcttcgaatagctgcggatcttgtcggcatagggcgcctcctgcagcgtgcgctcgagcctgtcggtcacctgctcggccacctgctgcgccgtggcgccgggccagtaggtgcgcaccaccatggcgcggaaggtgaacggggggtcttcgtcctggccgagctggaagtaggcaaaggctcccagcaccatcagcaccaccatcaggtagcgcgtgaggggcgcgtggtccagcgcccatttggagagattgaagcctgcgggcttgtcggtggtcgcagcgccctgcgtcatttggcggcacctgctgcgatctccttcttcgtggccgaaacggcctcggcggacggcgcgggttccttcgcgttggcggctgccgcggccgcctccttgctctggtagatggtgaccttctgtcccggcgagagcacgtgcacgcccgcggccacgaccatcatgccgggcgcgagcccgccgccgatcacggcctcgttgccgtcggccgtggccacctgcacggcctgcgaacgcacggtcatggtcgccttgtccagcacccagaccgaggtgcccttgccttcctggcgcagcgcgctggtcggcagcttcatgaccacgccgccggcgcgcgccagtgcctgcggacgggcatagacggtggcgccgagcgccggcgaagtggccgcgtcgatcgccaccttgaccgaataggtgcgcgtaaccgcgtcggcgctggccgccacttcgcgcacctggccttgcagttcggtgccgcccgaccagccgcgcaccgtgaccggcgaaccgggcttgatcagcgcggctcggtcttcgggcaccgcaaacaccacgtcgcgcgcgccgtcctgcgcgatgcgaacgaccggcgtgccggcctgcaccacctgacccggctcggcctcgatggcggtgatgatgccggccacgtcggcgaccagcgtggtgtagctggcctggttgccctgcgacgaaagctgggcctgcgcctgctcgagctgggcctgggccgccttccaggtggactcgcggcgttccagctccgcgccgctgatgaagttctgctcgcgcagttcgcggtagcgcttgaggtccgccgccgcgagatcgcggttggtctgcgccgcggcgagttgggcgcgcgccgcttcagccgccagccggtagtcctgcggatcgagctgggccagcacctggccggcctgcacgtgctggccgagttcggcctggcgtttggtgatcttgccggccacgcgaaagcccaggcgcgattcgacacgggcccgaacctcgcccgagaactcgggctgggcatcgaagtcgctggtgcccaccgtcaccagcttgaccgcgcgcacgggttcctcggctggtttcgactgggaacagccggccaggaacaaggcgggaagcagcagccatgcaatggcgccgcgggcaggagaaaagccggaggaggcggtcatgagacaccctggaaaggtcgaacctggtcattactgacccactggttagtaatctagggtaaacctccaggactgtcaatcgcggagttcgaagattcgctaggttctctggcccatctcgaccagacggttgtccggaagctcgaaatagtcggacgccctgcccgcgttgcgttgcagccagccgaagagcgcgcggcgcacggggttcatgcccggaaggttttcttccccgaccgacgcgcgcgaaacgaagtacgaggtcttcatggaatcgatagccagccccttctggtaggcgaatatccgcatgaactcgggcacgtcgggccgctccatgaagccgtgccgcgccgtgaccacccagatgccatccatcaggtgctcggcctcgatgcggatgcccgcatcgacacgcggggtgtcgcaagccagtacccgcagcacgaccacctgctcgtgcaggacctggttgtgcttgaggttgtgaagcaaggcgtggggcaccgccgtggcgtcggcattcaggaacaccgccgtgcccctgacgcggtgcggcatgtcgagcgccagcgattcgaagaaaggcttgagcggcaggctttcggccgcggcggcctccagccccagtcggcgtcccttggcccaggtcgtgaaaagcaccatcaccccggccgccacggccagcgtgagccacccgccttcagccaccttgaggctgttggccgccacgaaagtcaggtcgaccacggcaaatgccaccactccgagcaccaccgccaccctgttccagcgccagagcccccaggccacgacgccggccaacagcgtggtggtcaccatcgtgaccgacaccgcaatgccgtacgccgccgacaacgcccccgaactgcgaaagcccagcaccagcagcagcaccccggtcatcagcagccagttgaccaccggcacgtagatctggccgatggccgagcccgaggtctgcaccacccgcatgcgcggcaggtagcccatgcgcatggcgtgggccgtcaaggaaaaggcgcccgagatcacggcctgcgaggcaatcacggtggccatggcggccagcaccaccatcggcaaaacgccccaggcgggaaagagccggaagaacgggttgtcgacggccgcggggtcggccagcaccagcgcaccctggccgaaatagttcagcaccagccccggcagcgcaatgaagagccaggcgagccggatcgcccgcgtgccgaagtgccccatgtcggcgtacagcgcttcgccgccggtaaaggcaagaaataccgcgcccagcaccgccagcgactgcagccggtgctcgaccaggaagccgatggcgcggcgcgggtcgagccccgccagcacctgcggatgctgcagtacttgccagccgcctgcgagggccagcaccccgaaccacaacaacatgactggcccgaacaccttgcccaccgcgccggtccccttgcgctgcacggcaaaaagcccaagcaggatgaggatggtgatcgggatcaccgcgcgctgcagcacgggtgcctgcacctccagcccctcgaccgccgacagcacggaaatggccggtgtgatcaggctgtcgccgtagaacatggccgcgcccaccaggccgagcgccccgatggcattccacagccacggccgggtctgcgagcctccagccgcgctgcgggcaagcgcctgcagcgcaagaatgccgccctcgccgtcgtggtcggcgcgcagcacgaacaccacgtacttgagcgtgaccacgaacatcaagccccagaagatgagcgagagcaggcccagcaccgtatcgggcgtgaaccccacgccgtgctcggggttcagcgtttccttgaaggcatagagcggcgatgtgccgatgtcgccaaacaccacgcccagcgccgcgatcatcaggcccggccccgccgcagaagacgcctcgccgtgcgttggactctgggcagcgggaacctgtgcctgtgcgttcatgaaatcgtgagcttcgattggagggtgacgccgcgagcatagtgcgcggcaggtgtcgcggacaatcgccgcgtgcctgaaccatcccacattgccgcgccgccggcgcattacgagaattttcccgtggcctcctggctgtgcccgcctcatctgcgaccgcccattgccgcgatctaccatttcgcgcgcaccgcggacgacatcgcggacgaaggcgacgcctcgcccgaccagcggctggccgacctccgtgcctatcgcgaggagctgcgcgccgccgcgcgcggcaacgtgccggccgcctcgcgctggccgtacgtgttcggcccgctggcgcacagcatcgcgcagttcgcactgcccgaggaattgctcgccgacctgctgagcgccttcatgcaggacatcgagaagacgcagggcagaggaacttacgccgaccgcgccgagctgctcgactactgccgccgctccgccaacccggtcggccgcctgctgctgcacctgtacggcgtgaacgatgccgaggcgctgacgcaaagcgacgccatctgcagcgccctgcaactcatcaatttctggcaggacccgagcgtggacctgccccgcggccgcttctatccgccgctggccgactgcgcccggcgcggcctgacgcgcgagagcttcaaggccttcatgccgctggccgatgcgccgcctccgcaggaagccatcaacctgatcgcggtcgcaagcgcctgggcgcgcgaactcatggcccagggcgccccgctggtccaccgcctgccgggccgcgccggctgggagctgcgcttcgtcgtccagggcggcctgcgcattctcgacaagatcgaagacctgggcttcgacaccttctcgcaacgccccacgatcggcaagaccgatgcgcccttgctggcctggcgcgccctgcggatgcggagacaattgccgcccatgaaagcgcccctccgatgactcccgagcaatacgtacaagacaaggccgccgcctcgggcagcagtttctattacgcgttcctgtttcttcccaagccgcggcgtgccgcgatcacggcgttctatgccttctgccgcgagatcgacgacgtggtcgacgaggtcagcgaccccggcgtggcggccaccaagctcgcctggtggcgcaccgaggtggcgcagtcgttctccggcccgccgcgccaccccgtgatgcaggcgctggtgcctcatgccgccgcctacggcatcgagcccaggcagctcaacgaggtgatcgacggctgccagatggatctcgaccagacccgctacctggactttccgggccttgcgcgctactgccacctggtggccggcgtggtcggcgaagtcgcggcgcgcatcttcggccagaccgatccgcagaccaccgcctacgcgcacaagctggggctcgcgctgcagctcaccaacatcattcgcgacgtgggcgaggacgcgctgcgcggccgcatctacctgcccgtgaacgaactgcagaagttcgacgtcaaggcgcacgagattctcaaccgcgtgcattcggaacgcttcgtggcactcatgaagttccaggcccaacgcgcgcacgcggcgtacgacgaagccctcgccctgctgcccgccgcggaccgccgcgcgcaaaaacccggcctcatgatggccagcatctaccgcaccctgctgcgcgagatcgagcgcgacgacttccaggtgctgaaccagcgcgtgagcctgacgcccgtgcgcaagttctggctggcgtggaaagtccaggcgctggggagcatttgaaaaccgccgtcgtcggcgccggctgggctggccttgcctgcgccgtcgaagccacgcggctcggccatgccgtgacgctgttcgaaaccgcgcacatggcgggcggtcgcgcgcgccgcgtcgaccacatgcatgggctgacgctggacaacgggcagcacatcctcatcggcgcctacaccgccaccttgaagctgatgcgcgagttgggcgtcgatgtggaacaggccctgctccggctgccgctgtcgctgcgctttgccgacggcggcgggctgaagctgccgcgactgccggcgccgctcgatctgctggccggcattttcacggcacgcggctggacgtggcgggacaagtccaccctgctgcgcaccgccgtgcaatggcgcctgcgcgggtttcgctgcgacccgggcaccagtgtggccacgctctgcaccggcctcacgccgcgcgtgatggaagagctgatcgagcccctgtgcgtctcggcgctcaacacgccggtcgatcagtcgagcggcgaagtgttcctgcgggtgctgcacgacgcgctcttcagcggcagcggcggcgccgacctgttgctgccgcgcgtcgacctcggcgggctttttcccgatgcggccctggcgtggctcgcgaagcacgacgccacgctgcgcatcggcatccgcgtgcacgcgatctggcccgagggtggggcatggcgagtcgacggcgagcgcttcgaccgcgtcgtcctggcctgtgcgccgtgggacgccgcgcggctcgttcgcgcgtccggcctgtccggcccgccggcgcaccgctggtgcgagaccaccgaggcgctgcgcttcgaagccattgccacggtctatgtgcgaggcgccacgccgcttgcggaaccgatgctggcgctgcgcagccgtcccgacaccgcaccggcgcagtttgtgttcgaccgcggccagcttggcggccccgagggcgtgcttgccatggtcgtcagcgcgaacgaaactccgcgcgaggcgttggaacaccaggccatggcacaggccgcgacccagttgggccagaccgcgctgcaacccgtgcagaccgtggtcgagaagcgcgccacctttgcctgcacgcccggactcgcgcggccgcccgcggccatcgcccccggcctgcaggcctgcggcgactacaccgaaggcccctaccccgcaacgctcgaaggcgcggtcctgagcggactggccgccgccaaggcactgacatcaccatgaccgaattgcgctacctggatttcgactacagcgaagacaccgaaggccacggcaccttcgacgcgatggcctcgaccgtgcccgaaaaaacgcgcgaagcgctggccgagattgcacgggtcctggcctgggccgactcggcctttccagatgcgcgcggcgcgctggacgacggcgcgatgtgggacttcgacctgcagcaggcccgcgaagagccgaacctcgatatcgtgaccttctcgctcagcggcacggccgacttctgcgctgcgtttcgcgagcagttcgcagtggattgaaaagtccgacaagcccgccgccgcggaggctgcgccccacaaccatccggtcccggaaagaaacatggtcacctgctacctgcgctacatcgtcgatccgtacaagctcaaggaattcgagcactacggcaagctctggatcccgctggtcgagaaattcggcggccagcaccacggctacttcctgccctcggagggcgcgaacaacgtggcgctcgcgatgttcagttttccgagcttcgccgcctacgagcagtaccgcgccgattcgatgcaggaccccgagtgccaggctgccttcaagtacgccgaggacacccgctgcatcctgagctacgagcgcagcttcttccggcccgtgttctcgtaaggcgggaactcaagcgccgagcgccacgcacagcgcgtgcaggttcggcacgatcagttgcggacgcgcgccgtgcacccacggccgctcgtcgcgtaccagccaggccgcctgcatgccggcgttgagcgcgccgaccacgtccagttcagcgtcgtcgcccacgtgcagcacgtccttcggcagcaggccgaccgacgcggccgcggcgcggaagatcggcgcatgcggcttgccgctgccgaaggcgcgcgcattgaacgcggtgcgaaaccaacggcccacgccggtcaggtggatgtccgcattgccattcgaaatggccaccagcggatagcgttcgctgagccacttgagggccggcagcgcatcgtcgtacaaggtcacgcgctggcgttcggcaaagaaggcatcgaaggccggatcggccaacgccgggtcttcgcccgcgtgcttcagtgccgtgcggatcgattcgcggcgcagcgcgctcaggtcgtgcgccagatccgaccgttccttggcggtggcttcgcgcagctcgcgcaggacgcccgggttcagcagcagcgacgcggtcttgggtgcttcgcgcagcagccattcctgcagcacggtctcggcacgctcgatggtcggccagatcggccagagggtgtcgtccagatcgagcgagatcgccgagatgcgcttgatgtcgagtggctcggcgcctgccggcgccgtgaaaacggaagtcatgcccgagaatatcgcatgcctcaagacaacgggaacaacagttccatcgcctcgcgtaccgccgtactctggtgcaacctgggctcacccgatgcccccaccacggccgccgtccggtcctatcttgcggagtttcttggcgatccgcgcgtggtcgagattccgaagctgctctgggccttgatcctgcacggcatcatcctgcgcgtgcggcccgccaagtcggccgccaaatacgcgagcatctggatggccgagggctcgccgctgaaagtgtggacgcagaagcaagccaccctgctcgccggctggctcggtgaacgtgggcatcgcgtggcggtgcgcgatgcgatgcgctatgccagcccctcgatcgcttcgcggctcgatgcgctgcaggccgaaggcgcagcgcgcgtgctggtgctgcaggcctatccgcaatactcggccaccaccacggccagcgtgatcgatgcggtgaacgactggagccgccgccagcgccgcattccggagttccgtttcgtcaaccagtaccacgacgatccggcctacatcgaggcgcttgcgcaaagcatcgagcgccactggaagaccgaaggccgcggtgaggtgctgctgatgagcttccacggcattccggcgcgcaacatcgcgctcggcgatccctaccaggcgcagtgcctcgaaaccgcgcgcctgctcgcggcgcggctcggcctttcagcggcacggcatcgcgtcacctttcaatcgcgcttcggccgcgccaagtggctcgagccctataccgaacccaccctgcgcgaactcggcgcaagcggcgtcaagcgggtcgacgtggtgtgccccggctttccggccgactgcctcgagacgctggaagaaattgcgatggaaggccgcgaggccttcatgcatgccggtggcgaagccttcagctacatcccctgcctcaacgacagcccggcctggatcaccgcgctggcggggattgccgaacgcaacctcgcgggctggcccacgcagcgccccaccggtacttagaacttgcccaggtagtccatcttgccgatgggcatgcccttgtggcgcagcacgtcgtaggctgtggtcacatggaagaagaaattgggcaacgcgaattgcaaaaggtagcgctgcgcggtgaagtgcgcctcgccttcgcgcgccttgatggtgacggggcgttcctcctggccgtcgatcagcgtgcggtccacggtagcgagaaaatcctgtgtcttcgcgatgcgggccagcagttcgtcgtacgtcttttcctcgtcgggaaagctcggtgccgtgatgcccgagatgcgcgccacgccgagcttcgacgcatcgctggcgcgctggatctgcccggccagcgtgatcatgtcgggtgcgagcctcgcgtccacgagcgtcgccgggtcgatgtcgttggccttggcgtgcgccaggctcttctcgagcacatgggtgagttggccgagcccgcgggagaagaccggcacggacaggtcgtacatcgaaagcgccatgggtaaatccttgtggttggaatcggcggcgattgtctcgccgactcgcgcctagcggccggcggcccggataaacccttcaaccagatccagttgttccggcacgttgagcgcgggcgcgtggccgcacccctggatttcgatcaccttcagcaacccggcagtgcccgggccccgctgctgcatctgctgcgtgacctcgggcagcaccaggtccgattccgcgccgcgcaggcacagtaccggcacttcgatgacgtcgtagtgcggccagatcaggtagtcgttgtcgtgcgcgctgaactgccggaccatggccgggtcgtaatgcggcgtcacgcggccgtcgggcaggcggcgggtggagctctcggtcaaacggcgccattgcgcatcgctgagccagccgtagggcttgtagacggtgcgaaagaaaagctcgagctcggccacggtgtcgaatgcgggcggctcgccggcataggcgcggatgcgctcgatggccgcctgcgcgagctgcggcgcgttgtcgttgagcgtgaggctcgcaatgcgcgccctcatgcgcggctcgaacaggcccgacgcgcagaccgtgccgatggccccgcccatcgaggtgccgacccagtgcacgcggcccaggcgcagctcgtcgcacagcgcggcggccatgcgggcgtagaacgagagctggtattcctcgtcgggcagcggactccactggctcagcccgcggccgatggtgtcggggcagatcacgcggaagccgcgcgcggcaaagtgctgggccagctcgtccatgtcgcggcaggtgcgcgcgaggccatgccacgcgatgatcaccggcgcgtcgggcgcgccccaatcgagccagtggacttcgcggcccgcgagctgggcgtagcgggaaaccggaacgggaagatcgttgctcatcgtgcagccctcgccctcagcttgccgacgatgccggtcggaaagtaatagaccgagagcacgaacagcacccccagccacagcagccagcggtcgggcgacagcagcgccgcgagccatggcagcccgctcgcggcctcgctgcccacgcgcagcaggtcttgcaagtagctttgcgccaccacgaacagcaccgcgccgatggccgcgccgtagatcgtgcccatgccgccgatcaccacgatcagcagcacgtcgatcatgatctcgaagctcagcgaggtgtcgggcccgttgtagcgcagccagatcgcgagcatggcgccggccagcgtggcaaacagcgccgacagcacggctgccgtggtgcggtacaccaccacgcggtagccgatggcctcggcgcggaactcgttctcgcggatggcctgcagcacgcggccgaagggcgaattgacaatgcgcagcagcgcgagcaccagcaccaccgccgccacgaacagcaggtagtagcacagcagccggccgtcgagcgagacgccgaggaaaggctcttcggagaactcgaagctcggcgaaatcagctcgggcagcttgaaggtaagcccgtcttcgccgcccgtgaaatccgacagctgcgaagccagcgtctggaaggccgaggccaccgccagcgtgatcattgcgaagaagatcgcgcgcaccctgagcgagaacagcccgatggcgaacgagagcaccagcgagattgcgagcgacgcgccgagcccgagcagcaccgcgccccagctgggcccgagacgcgtggcggagatggcgatgccgtaggcgccgatgccgaagaacatggtgtgcgcaaagctcacgatgccggtgtagcccagcagcaggtcgaagcttgcgaccagcaccacgaacaccaggatcttggccgcaacgctgagcgccttcacgcccgggaagatgaaaggcgcgaaggccagcgcgatgaacagcgccaccagcagcagcgccagcaggcggctcttgggcgtgtcattggagagaagtcgtttcaggaacatggcggcttcttccttctcagcggttggcaaccgggtacacgccctgcggacgccacagcagcaccgccaccatcagcaggatgctcgcgaattgcgtgagcgtgggcagcaggaagccgatgtagttggtcatgagccccaccagcagcgcgccgatcagcgccccgcccgtcgagcccagcccgccgatgatgatcacgatgaagatcagcacgttgacctgcgcgcccatctgcggcaccaggttctgctggaacagcccccacatcacaccgcccagcccggccaatgcgctgcccaccacgaacacaccgacgaacagccggccgatgcggtagccgagcgactcgaccatctcgcggtcttgcacgccggcgcggatcaggaggccgatcttggtgcgactcagcgtccatgcgagcaggccgaacaccacgatgcccaccgccaccgcgagcaggcggtacttgctgatggccgcatcgccgatcagcagcgagccgcgcaaggcttcgggcagcggcagcggcacctgggccggtccccagatcaccttgatgagctcttcgccgatgatcatgccgcccatcgtgatgaggatctgcttcaggtgctggccgtacacgggcctaacgatgaagcgctcgaaggccagccccaccgcgccagctaccaccatcgcgaccagcatggccggaaacacggcgacgaggttgcgccacagttcgcccgaaccggtccagtcgcccatcaggccgagcacgctgctggccacgaacgcgccgagcgcaatgaacacgccgtggccgaagttgagcacgtccatcaacccgaacaccagcgtgaggcccgaggcgatgatgaagatgatcatgcccatcgccaagcccgcgaccgtgagcgtgagccaggtcgagaacgagcccgtgagcggcagcgcggccagcgcgaggatgggcgcgagaagcagcggcttccagtcgaagtcgagtgccttcattgctgcgctcccttttcttgctccctctccctttgggagagggttggggtgagggccagcggcgccaacatgagggcacggccattgcacaggccgcctgccctcaccctagccctctcccagagggagaggggacaagtcatcgaatacttcatagggcgagtcccagcagcgattgctgcaattgcgcatccgcggagaacgccgccatgccgccgctgtgcaccacgcggccgttgtccatcaccgcgacgttgtcgcccaggcgttgggcgaagttgatgttctgttccaccagcaggatcgtcacgccgctgcgcttgagctcgccaaacgcatcgatcatgttgttgatcatcacgggcgcgaggcccttgctgggctcgtcgatcagcagcagctcgcgcggctcgacgatggcgcgcgacacggcgagcatctgcttctgaccgcccgagagcttgccggcgggatggttccagaacttctcgacggcgggaaacagcttgaaaatccacttcagccgcgtgtcgtcgatctgcgcggcgttcttggcgccgcgcgcggcgagcagcatgttctccttcaccgtcaggtcggaaaagatgcccatgttctccggcacgtaggcgatgccaagctcggcgatctgcggcgtgtgcatggcggcgatgtccttgtcgccaaagcgcacccggccctgcgacgcatgccacaggcccatgatggtccgcagcgtggtcgtcttgcctgcgccgttgcggcccagcagcatggtgagctggcccttgggcaccgcaaggtcgacgccatggaggatgtggtacgccccgatgtgcgtgtgcacgccttcgagtgtcaggaggttctgcgttgtcatcggtcttgctccttccccttccgggggaaggttgggatgggggcatgcggcgcttgaagggccgcggcggtgtgaaggccgcttgcccccacccctgccctcccccagcgggggagggagaaattcatcaacgccttcatgcagccgcctccttcgcgatgccgaggtacgcctcctgcaccaccggcgaggcaatcacctcggccggctcgccatcggccacgagcgtgccgttgtgcagcacgatgatgcggtccgcgagttcgcgcaccacgtccatcttgtgttcgaccaggaggatggtcttggtcttgtcctgcttgagcttgcggatcaggtcgaggatgacgggtgcctcggcggcattcatgccggccgtgggttcgtcgaacatgaagaccttgggctcgagcgccatcaggagcgccacctccagcttgcgctggtcgccgtgcggcaggctggccacggtcgcgagctcgcgcgacttcagcgccacatcggccaggatctgatcggcgcgctcggtcagcgccttgtggtcgctccagatgctccacaggttgagcccacggcggtgcggaccctcgcgcgtggcctgcaccgccaggcgcacgttctccagcactgtgaggttcgggaacagattcgtgagctggaaggcccgtcccagccccgcgtgcgtgcgcgccgacggcgacaggcccgacagcagatgcccgtcgagcgacaccgtgcccgcactcgccttgagctggcccgagatcaggttgaagtacgtggtcttgcccgcgccgttggggcccacgatggccgtcagcgtgcccggcgcgaaggcgcagctcacgctgttgacggccacgtgcccgccgaagcgaatggtcaggtctttcgtctcaagcatcgttggtcattgcaaatgaaagtggtgcagatcggctcaacagctgccgatcacgtagtagttcgggccggtctgcttcagcgtggtcgtgacgtagatgttccacagccccatcgattgcccggaaccgtaggcataggtgaggccccacagcgcgtaggcacgcccggccacggtgtgcgcgtagttgctggcggtgtagcaggtgccgccgccaccgctgccggcaagcgtggtgcccgtggccgcggccgacatcgcaccttgcgcattgctggcgtccaatgccgccacggtccagctgtaggtggtcgacgcggccagtccgctgtcggtgtagttggtgccggccaccggcgcggcgttgaccttgctgccgccgcgatagacgttgtagccgctggcgccggagacgccattccatccgatcaccatgctgctgctggtcgcgccggatgtgcccacgccggtgggcgccggcagtgccgagccgccgccggagccggtcacgcgatcgaccatggccttgagcgccgccatctgcgggcccgacttcttcgcatagttcgcgttgtcgtagccccaccagtcccagcagctgttggtggccgcggtgctggtctgcggatagatcagcacgatgttgttggtgtcggcccagcggttgtagccggtcttgcgcacatattggtcgcctacgtcggtgtagttctgcttgcagccgtgcagcaccatgtgcacgcggcacgacgcggtggtgcaggcctgcggcacgtagatccagccggtagctgccacgccgtggccggagatgaactccgactggttgaactcggtgaacgtgccacccagcgcgccgttgttgcgcgggttgagcggcccatacagatgctgcaggatctcgcccgcgaggtcgaagccgcagttgttgatgtagggtgcggcggtggtgctgcaggcggcgccgaagtcgtcggtgaccatcgcgtggccggcgccgatgttgttcttgtagaccgtgttggccgcgggcacgaagctctggtagtaggtcttcaggtcacccatgaccgcgggcttgaccgtgttgtccgacgtgccggagaacaggtacaccttcgacgcggtcatgttcgacaccgggtcgatcgcgccgctggcggcccagctgttggtggtgctcacgagcgtcgacaccgggatgctggtgctgtgcgccatgcagcgccctgtggcattgaccaccgagccctctgcgcagtagtacggcccgccggccaccacgccggcaccgcgtttgaaggtggccgaataggccacgtgcaattgcacggccatgaagccgcccgccgagaggccggacacgctcacctccgccgggtttgcgcccagcgacgggagcggcaccgccgcagtggccgtgcaggcatacacgccaaacgccattgccgcagccgcggccaatcccttccagttccctcgcatcgctgccatcgctgtctccttgcgttgcaggcgtgtcgaacgcttgcttgattgctgacgaacaggccattggttgcgccgccacgtccgccacgaaggcgcaggctggcgcttcgcccggcggccatgccggggcgaaagggatgcggcctcaggaccgcggaatcggggtgccgatcagcgcttgttcttgatcgggatgtccatctcttcgggcttgatctcgcgcaccagttcaggcacgccccatgcaaaggcggggtcgttcttgatcttgaagtggtacattgactgcatcgcctggtggtcttccttgcggaaggtcatcttgcccttgggcgtgtcgaagctcatgccttccatggcgctgatgagcttgttggtgttggtgtcgccgccggtcttcttgagcgcggaaaccaccgccattgcggccgagaagccgccggccgtgaagaagtccggcggcgtcttgaattccttgtagtgcgccgcgacgagagcttcgttcaccggattcttcggaatgccgaagtagtaatacgccgcgccttccatacccggcaggcccttgtaagcggccatggccggcaggatgttgccgcccgtcgcgatctcgatgttgtagcgcttcaggtccaggtcgacgatcttgaacggattgcccgcgccggcccagacgatccagatgatcttgcggcccggctggtccttgagcttgtcgatcaggcgctgggcaccggccgtgaagtcggtggtggcgggcggcaggtattcctcgtgcaccagcttcgccttcttgagcgcggcgccgaaggccttcacgccgtcacggccgaaggcgttgtcctgcgcgagagtcgccacggtcacgccggccttgtcgatggccaccgcgttgctgatcgcatcctgactcgaattgcggccggtgcggaagacatacttgttccacttgtcgccggtgatcgaatcggccaccgcgggctcgacgatcaggatcttcttgtactcctcggccaccggcagcatggccagcgcgacgcccgaagccgtgggacccaccgccagcgcggccttgtcgtcggaatacgcggcggccagcagcgacttgccgaggtcgggcttgccctggtcgtccttctcgatgaccaccagcttcttgccattgaccgtcatcgtgccgccggtggcgtaatccaggcccatcgtgaagccggtctgcgtctgcttgccataggcctcgagcggaccggtcttgctgtatatgtgcgcaatgcggatttcgttggactgggcccaggcgggggctgcggcggcgcaggtggcgagtgcggccagggcgacgaggtggcgacggttcattctttgtctcctgaaataggtgactgaatattgcacagttcgtgccacacgcccaagccattgataacaatggtttcttcattggagaagacgcgctttcgcctgatttaggaacaattttgatgcctgatattcaggcatttgtatttttatcagtcagggttttcgagaaggttcgctcgcagatcgccgccactgttcagccacttttcgaattgcgagcgacaggacacaggaagacggtgctgcgcccatatttttcccagattcatgcctacattggcacttggcacccctggctacctccccctccccctcctccctccgacgcgggggctgcccctgacccgcttcggcgggtcttttttttgctgctgccattgcgccgagggcgcctctcgcgccatggttcaggcgcttcagcgaaccggattcgtcatccgttcatacagcgtcgcgcgtgaaatgccgagcagccgcgaggttgcgagcttgttgccgcccgtgctcgcgagcgcagcggctatggctttctgctccagctccgcaacctgttgcgccagcggccgcagcagcgccgcctcttcgtcgcctgacgagtgcaggacatcgggcggcgcgatctggtccagccccgcttcgcgcaggatgcgttcgagctgcgcggcatcgatgcgctgcgaatcgctgcgcatggtcacctgctccagcacgttgcgcagctcgcggatgttgccgcgccagtgctggccggccaggagcgccagcgcatcgggcgtgagttcgggcggcgcctcgccgctgcgcagcgccatgtcttcgcccaatgcctccaccaacgccggaatgtcgctgcggcgctcgcgcagcggcggcacgcgcagcggcagcacgttgaggcggtagtacaggtcttcgcggaactggccgcggcgcaccagctcgggcaggtcgcgcgaggtagcggcgatcacgcgcgcatcgaatggcaccagcttgttggagccgagcggctcgatctcgccctcctgcagcgcgcgcagcaacttggcctgcaggccgagcggcatgtcgccgatctcgtcgagaaacaggctgccgccatcggccagcttgaacttgccttcgcggccgcggcggtcggcgccggtgaaggcgcccggtgcgaagccgaagaactcggcctccagcagcgtgtcgggcacggccgcgatgttgacgctgacgaactgccccttggcacgcgccgacgatgcgtggatcgcatgcgcgagcaactccttgcccgtacccgtttcgccgagcagcaacaccgggctcgtggactgcgcggcccggcgcgcatggcgcttcacctccaccgccgcggggctgctgccgatgaagctggcaaaggtgtatttggagcggcgctgcccgtcggccgcgtgctggtacagcgggttgttgcgctggctcgccagttcgcgccgtgcgtcgtcgaggtcgcgctgcagcagcgcaaatttgctgatgagcggctgcagcgtggtctcgggctggtcgaacagaacgatgccgatggcgccgatgacctctcccgccctaccttcgcgcccatcgctttcggcgcgcagcggaatgcggctgacaacgaaagtacccgccttgttggtgagaaggtccacgagaatcggctcgccggtttcgagcacgcgccgcatctgcgtgttgggaatgacgtcctcgaccatgtgccccatgaactggtcgatcgacgagaagcccagggccggcagaaaacgccggtacccttcgttcacccacacgatgcgcccgctgcggtcgaccagaaacatgccctggctgatgctcgagaacagatggaacatcgagcgagcggccaatgcgaggatgccttcggcatcgagcggcagggtgggcggtgcggcaacaggcggagcggcggacatgcgcggatcgtagcgcgcatcaatcggcgccgaatcaagcatcaacgcgcggccggaacatacacagaatagatatccgccgacccatacgaagaaagccctcatgcggccataagtaaatcaatcgtttgattgcctccgtggtctaatgccggcatgagcgcccctgccctccaagccctttccgcgcgcgcgccacgcagcgacggcgtcgaagcgcgccagcgccttctctatgccgcgctcgccctctttgccgccaacggctacgccaagacctcgacccgcgagattgcccgcgcggcggacgtgaacatttcggccatcagctattacttcggcgacaaggccgggctgtatgccgccaccttcggcgagccgatgggcggcaatgccggagacttcgtttcgctgtacgacgcgcccgatctgccgatggaagaagcgctgcgcatcttcttcacccacatgatcgagccgctcaagcaaggcgagatcgtgcggcagtgcatccagctgcacatgcgcgagatgctcgagccgacaagccagtgggccaaggaattcgagcgcgacatcaagacaccgcacatcgccgtcgcgggcgtgctgtgtcgccacctcggtcttgcgcggccggacgacgacgtgcatcgcctcaccttcgccatcaccggactcgcggtgcagcttttcgtgagccaggatctcgtcgacgccatacgcccctcgttgctgaacacacccaaaaacgtggacacctgggcgcagcgcctcacgggctatgccgttgcgctggtcgaggcggaagcactgcgccgcaaagccgccaccaagcccgcggcggtatctgccgtccgttccgggagaaagaaaacatgagacgactccgatggattgctgccgcctgcctgggcctcggccttgccggctgcggcctgacgcgcccgccggccacggtggaggcgccgttccccgcgcagtggcatgcgccgctgccccacggcggctcggtggcttcgctggctgaatggtggagccagctcgacgacccgctgctggtcgaactgattgccgcggccgaagccgcaagccccaatctcgcgagcgctgcggcgcgcgtggccgaggcgcgctccacgcgcgtgcaggccggcgcggcgctgctgcccaacctggacggcacggcgtcggccagccgcggcgtctcgggctcctctttcggctcgggcggcacgacttcctcttccagcagcagcgcggccatcgcgccggtgaccacgctgcaggccggcctgcagtccaagtgggagatcgacctgttcggccgcctgcgcgccgatcgcgattcagccgagcagaagctcagcagcgccaccgccaaatggcacgacgcgcgcgtggccgtcgcggccgaaacggccaacgcgtacttcgccgaacgcgcctgccagcagcaactgcgcgtggccgagtcggacgccaaatcacgcggcgaaaccgcgcgcctcaccgacctgtccgcgcgcgccggcttcaccgcgccggccgacgctgcgctggcgcgcgccagcgcctcggacgcctcgggccgcctcacgcagcaacgcgcccaatgcgcggtgcagcgcaaggcactggtggcgctcagcggcatcgacgagcccgcgctcgaacagaagctcgccgcctcgcccacgcagcgcgcgctgccagtggtcggcagcattgccagcgtgccggccgacgccatctcgcagcggcccgacgtgtacgcggccgaactcggcgtggcctcggccagcgccgacgtgggctccgccgaagccgagcgctatcccaagctcagcatctcgggctccatcggccgcatgcagatccgcaccagcggctttcgggaatcgctcgacacctggtcgattggcccggtgtcgctcacggtgccgctgctggacttcggcgctcgcgccgccaacagcgatgcggccaaggcgcgctacaccgaggccgtgtcgctctaccgcgcgaacgtgcggcaggcggtgcgcgaggtcgaagaagcgctggtcaacctcgacgccaccgatgcgcgcgccaccgacgccgactccgcggtgaagaactaccaggcctctttcgacgccacccaggcccgctatggcagcggcctggccagcctgttcgagctcgaggattcgcgccgcacgctctttgccgcacagaccgcgcgcgtctcgctgcaacgcgaacgcgcccaggcctgggttgcgctctaccgctcgatgggcggcggctgggcccgccccggatcgccctcaatgacctccaacccggccgccaaggtcgcgacgtcgccatgaaaagtatcaaacgctccaccctcgccatcgcgctgctggcgctcgtcatcgtcattgcggcggccgtgtggctgacgcgcaagccagcgagcgagcccggcactccggcggcggccgccaaggacaaggcgggtgctccggctgcccggccgacgttgacagtcacggtcgccaagcccgagctcaccgagctcacgctgacgctcgcagccaacggcaacgtggccgcctggcaggaggccatcgtgggctccgaatccgccgggctccggctcgccgaagtgcgcgtgaacgtgggcgacgtggtgaagaagggccaagtgctcgccgtcttctcgcccgagacggtgcaggcggacatcgcgcaatcgcgtgcctcgctcgccgaggccaaggcgaccgccgccgacgcagccggcaatgccgcgcgtgcccgcacgctgcaggccaccggcgcgctgagccagcagcagatcaaccagtaccagaccgccgagcagaccgccaaggcgcgcgttgaggccgccgaagccgtgctagccgcgcaacaggttcgcgggcgcaacacgcaggtgctggcccccgacgacggcgtgatctcatcgcgcaccgccacggtcggcagcgtggtggcctccggcaccgagctgttccggctgatccgccagggccggctcgaatggcgcgccgaggtcacgtcggccgaactcagccgcatcgcggtgggcaccacggccttcgtggtcagcgccagcggcgcgcaggtgcgcggcaaggtgcgaagcatcgcgcccacggtcgatccgcaaacgcgcgcggcgctggtctacgtcgacctgccgaacgtgcagcagaacaccggcatcaaggccggcatgttcgcgcgcggcgacttcgagctcggccggagctccgcgcccaccgtgccgcaaacctccatcgttccgcgcgacggcttcaacaacgtcttcatgctgttgcccgacaaccgcgttgcgcagctcaaggtgcagagcggccgccgcgtgggtgagcgcgtggagatcaccagcgcgctgcccgaaggcgcgcagatcgtggtgcagggcgccggcttcctgaacgacggcgacctggtgcgcgtcgtcgcggcgcccgcaccggcggccgcgggtgcgcaaccggccgccccgactgaaacgaaggcacgcccatgaacgtttccgcatggtccatccgcaacccgattccggcggtgatgctgttcgtgctgctcaccttcggtgggctgctgtcgttcaacgcgatgaaggtgcagaattttccggacatcgacctgccgaccgtgacggtctcggcggcgctgcccggtgccgcgccttcgcagctcgagaccgacgtcgcgcgcaagctcgagaactccattgccacggtgcaaggcctgaagcacatcaccaccaaggtgcaggatggcgccgccacgctgatcgtcgagttccgtctcgagaagccggtgcaggaagccgtggacgacgtgcgctccgcggtgcagcgcgtgcgcgccgacctcccggccgacgtgcgtgacccggtggtcaccaagctcgacttcgcggcccagccggtgctggccttcaccatcgcctcggcgcgcatggacatcgaggcgctgagctggttcgtggacaacgacatcaccaagaagctgctcgcgcttccgggcgtgggtgcggtgaaccgcgtgggcggcgtcacgcgccaggtgcatgtcgacctcgatccggccaagctgcaggcgctgggcgcctcggcggccgacatctcgcgccagctgcgacaggtgcagaccgaaagcgccggtggccgcatcgacctgggcggcagcgagcagccggtgcgcaccatggccaccgtgcagtcggccgaccagctcgccgacatgcagattgcgctctccgacggccgccgcgtccggctcgaccaggtggcgcgcatcagcgacaccatcgccgagccgcgcgccgccgcactgctcaacggcaagccggtggtcggcttcgaagtggcccgcagccgcggcgccagcgaggtggaggtgggccgcgccatccagaaggcgctggccgacctgcgcgtgcagcgccccgatatcgaactgacggaagccttcaacttcgtcgacccggtggaagaagagtacgacggctcgctgcacctcttgtatgaaggcgccatcctggcggtgatcgtggtgtggctgttcctgcgcgactggcgcgccactttcgtctcggccgtggcgctgcccatgtccgtcatcccggccttcatcggcatgcacctgctgggcttctcggtcaacgtgatctcgctgcttgcgctttcactggtggtcggcatattggtggacgacgccatcgtggaggtggaaaacatcgtgcgccatctgcgcatgggcaagtcgccttacgaggcggccatggaggcagccgacgaaatcggcctggcggtgatcgccaccaccttcacgctgattgcggtgttcctgcccacggccttcatgagcggcatagccggcaagttcttcaagcagttcggctggacggcctcgctggcagtgttcgcgtcgctggtggtggcgcgggtgctcacgcccatgatggcggcctatatcctgaagccggtggtcggtgcccaaaaagagccgcgctggctcacggcctacatgcgcgccgtggaatggagcacgcaccatcgcttcaagacgatggtgctcgccaccctcttcttcttcggttcgctggcgatgatcccgctgctgaagaccggcttcattccgccggacgacaactcgcagacgcagatctacctctcgctcgcgcccggctccacgcttgcgcagaccaccgcggccgcggaagaaacgcggcgccgcgtgatgcagatcaagcacgtgaaaagcgtctacaccaccgtggcgggcggcagcgcgggcggcgatcccttcgccaacttcggaacgcccgaaacccgcaaggccacgctcaccatcaagctcgacgagcgcggcgaccgcccgcgcaagcaggtgatcgagaaccagatccgcacggcgcttgaaaccctgcccggcgtgcgcagcaccgtgggccttggcggctcgggcgaaaaatacatcctcgctctcaccggtgaagacccggctgcgctggccagtgcggccagcgcggtcgagaaggacctgcgcacggttcccggcctcggcaacatcacctccacggcaagcctcgtgcgccccgagatcgccgtgcgccccgacttcgcgcgcgcggccgacctgggcgtgaccagttcagccatcgccgagacgctgcgcgtggccacgctgggcgactacgaccaggcgttggccaagctcaacctcgcgcagcggcaggtgcccatcgtggtgaagctcgaagactcggcacggcagaatctcgacctgctcggccgcctctcggtgcccggcgcgcgcggccccgtcatgctgagccaggtggcttcgttgacgatggaaggcggcccggccgtcatcgaccgctatgaccgctcgcgcaacgtcaacttcgagatcgagctttcgggcgtgggcctcggcgatgccaagaccgcggtcacggcgctgccctcgatccagaagctgccgcccggcgtgcgcgtgaccgaggtgggcgacgcagaagtgatgaccgagctgttcgcgagcttcggccttgcgatgctcacgggcgtgctgtgcatctacatcgtgctggtgctgctgttcaaggacttcctgcatccggtgacgattctttgcgcactgcccctggcgctcggcggcgccttcgtgggcctgctcatcgggcagaaggcgctttcgatgccgtcgctgatcgggctgatcatgctgatgggcgttgccaccaagaactcgatcctgctggtggagtacgcgatcgtggcgcgccgcgaccacggcatgacccgctgggaggccctgcgcgatgcctgccacaagcgcgcccggcccatcatcatgaccacgctggccatgggtgcgggcatgctgccgattgcagtgggcctcggtgccgccgattcgagcttccggtcgccgatggcgatggcggtgatcggcgggctgatcacgtcgaccgtgctgagtctgctggtggtgccggctgtgttcacttatgtggatgacatcgagcactggattcggcggactgtgcgcagggtgcgggggcagccggctgatccgcatattgatgatgatctggtggagcggactgctggttgacgctgttcgttcagactttttgacgcttcgcgggatttgttttccgaggccgggatatccgcccggcggcggactcactttcttttgcttcgccaaaagaaagtgagtcgcccgccggggcgagtcccggcctcgggaagcaaccgccgcgcagcggtaaaaaaacaactacccctcgccccccaaaaatgagggcaagaagacagaaaagtcagaccgccaaccgagccaacttccgctcactcatgcgcttcgccacgcgcggcaacacaagcacagccacgatgatgaccaccagcgtgatcgacatcggccgctggaagaacaccgcagcactgccctccccgatcgacatcgcattgcgcaattgcgcctcggcgagtggccccagaatcatgcccaccaccacaggagcggtcggaaagtcgaagcgccgcatcaccacgccgagcaggccgatgccgtagagcaggaacaggtcgaacgcgctctggcgcatgccgtaggcacccaccgtcgcgaagatcaggatgccggcgtagagctgcggcttgggaatcttcagcagcttgacccacaagccgaccatcggcaggttcagcaccagcagcatcacgttgccgatgtagagcgacgcgatcagcgcccacaccaacgcggccgaggtggtgaacaactgcggccccggctggatgccgtagttctggaacgcgccaagcagaatggctgtggtgttcgacgtcggaatgccgagcgtcagcagcggaatcagcgcggcagtcacggtggcgttgttggcggcttcggggccggccacgccttcgatggcgccggcgttgccgaactcggccttgtcttccggattcttggccagcttcttttccatcgcatagctcaggaaagtcggaatctccgtgccgcccgcgggaatgcagccgaacggcgtgccaatggcggtgccgcgcaaccatgcaggaatcgagcgcttccagtcgcgcttggtcatgtggacgcggctcagcttgttctggccttcgaccaccttgccctcgtagagcaccgcgtacagcacttcggccaccgcaaacaggccgaccgccaccagcacgatctcgatgccgtcgagcatttcgggaatgccgccggtgtagcggccctggcccgagatctggtcgaggccgacgcagccggccgcgaggccgatgaacagcgccgtcatgccgcgcagcgtgctcttgcccagcaccgcgctcaccgtggtgaaggccagcagcatcagcaggaaatactcgggcggcccgagcttcacggcgaactcggccacgaagggcgcgaacatcgtgacgatgaccgtggcgatggtgccggccacgaaggaaccaatggcggcggtggcgagcgcggcgcccgcccgtccgctcttggccatcttgttgccttccatcgccgtgaccatgctggccgtttcacccggcgtgttcagcaggatcgacgtggtcgaaccgccgtacatggcgccgtagtagatgcccgagaagaagatcatcgaggccgtgatttcgaccttgcccgtgatcggcagcagcatggccaccgccacagcgggcccgatgcccggcagcacgccgacggccgtgccgagggcgcagcccaccaggcaccagagcagattgacaggggtgatcgccgcggcgaaacccgtcatgagtgcgttgaagatttccatgtcaggcctcccgccgggccgccccaaggcaggcctgcgccccctcggggggcagcgaatacacgaagtgatgagcgtgggggttcatgtcagatccagccggtggtcgtgaggcccggcaggttgatggccaggaacttggtgaacatccagaacacgggcgccgagatgagggcaccggtcaggaggtcgatggcccaggtgcgcggctggttcgccgaaggctggccgcccgcgcggcgcaggccctgcacggccagcacgtagcacagcgtgcagctcaggatgaagccgagctgggtgatgagcgccgcattgagcagcaggcccgccgacacccagacgaaacccggccagtaggcgcgctcggcgcccgtcggtgcgtcaagctcgcgaaagccgccggtgcgtgcctcccacacgatccaaccgccgcacagcgtgagcgcgctcgacaccagccagggcaggaagttggggccgacgccgccatagccagcctcggaagaaatgccgatggcgccgaaagccagcgccaagccggtcagcagcacgccggcgccgaccagggtttgcggccagatggccgcggcttgcggcgagaccgaggattctggagttgtcatttttttctcccacagtcagggaaaagaagagggcctactgaaaggcccacgattcaaaagaactccccacccgtccccgctcccttccaggaacaccgcggaaccggctttgccgggccgctgatgttgcccccgtagagggttggcgttggcgtagcgacgcgaagtgcgcgaagactgggggcgagccaaattcagaccattccggacttgaccatgatggcgcgcaggctggcgaagtcgtcgtcgacgaacttggcaaaagcctcgcccgagagcacggccggcgtccagtcgttcttcttgagcgtttcggcccacgacgggctcttgagggcagccagcaccatgtcggtcagcgccttgcgctgttcggcggtgatgccgggcgcgccgtacacgccccgccagttgccgatctcgacgtcgatgccctgctccttgagcgtgggcacgttgatgcccggcaggcgctgggcggacgtgacggcaatggctttcatcttgccggcggcaatgtactcggcgaactcgctgtagccgctgccgccgatggtgacgttgccgcccagaatggccgccgtggcctcgccgccgccccggaaggccacatagttgatcttggacggatcggcgccgaccttctgcgcgatcatggccgcggcaatgtgctcggtggagccgcgcgaaccgccgccccatttgacgctgccggggtctttcttgagctgatcgaccacgtccttcatggtcttgaggggcgagttggccggcagcacgaagacgttgtattcggtggtcatgcgcgcgatgggcgtggcctgcgaaagattgaccggcggcttgccggtgatgatgccgccgagcatgacggagcccatcaccatgagcgcgttcggatcgcccttggagccgttcacgaactgggccaggcccagtgcgccggcggcgccgcccttgttgtcataggtgaccgtgtcggccagcttggattcggtcagagccttgcccagcgcgcggcccgtggtgtcccagccaccgcccgggttggctggaatcatcatcttgacgttggctgcggcgcgtgccgacaacggcagcgctccggcggcggccagcgcggccaatgacttcaaaaaggtgtcgcgacgcatcgatgtctcctggtaactaaagaaaacctgacttggacctgagccgctatcatgcgccgccccgctgtcagttggctgtccaccggactggggaaaacaccaaagtaccattctcccctccacgccccatgaagctgctgctggtcgaagacgatccctcgatgcaggttaccctgcagcgcgccctcgcccgcagcaagatcgacgtgcggatctgcggcgacggcgccttggccgtcgagcaatggcgcgcgctggagcccgacgtggtggcgctcgacctgagcctgccgaacctggacggcctccaggtgctggccgaggcacgcgccgcggggctgcgcacgcccgtgctgctgctgacggcccgcggcacggtgggcgaccgcatcatgggcctgaatgccggcgccgacgactacctgcccaagcccttcgacctcgatgagctggaggcgcgcatccgcgccctgcgccggcgtcaccagaacgccggcgccgacgtgatcctgaacccgcaggaagtcggcggcctgcgcttcgagcccgaaagcggcgccatctaccaccgcggcggcatcctggaactcacgccgcgcgagctggcgctgctcaaggcgctgatgatgaagccgggccacgcagtcagcaaggaacggcttttcgagctggtgtttccaggcgaagccgacgtgcagtacgaggctgtcgaggtggtggtgtatcgcctgcgcaagaagctcgtgggcaccggcgccgcgctgatgacgctgcgcgggctgggctatctcttgcgcgcggagccatgagggcggccctgtcgctgcgcgcgaggctgctgttcggcattctcgcgccggtggcgcttttcatcgtgatcaacagcgtgagcctgtaccggcagagcctggccgcggccaccaccgcctacgaccggaccctgctcgcgtcggccaagaccatcggcgagcagctcgacgtggaaggctacgacgacggggcacggctgcgcgccatcgtgccctattccgcgctcgaggctttcgaggccgacaaccgcagccggcttttctatcgtgtttcggccctcgacggcgaaatggtctcgggctttgccgaactgccgttctggcgcggccgcattcccgatcgcggagcctattcggcgctggtcgatttctacgacgcgcgctttcgcggccagcccgtccggatggctgtattgctgcaacccgtgtccagtggccgcggccgcggcatggccgtggtgcaggtggccgaaaccctcgagctgcgcgaaacgctggtgcgcaagctgctcgtcgacatgctgtggcggcagctgctgctgatgggcgtcatcgcgctggtcacggtgctggtggtgcagcgcgccacgcggccggtgcgggagcttggcgaagccatcgagaagcgcgcggccgatgacttttcgcccatcgatgcccccgatgccccgcgcgaactgcggccgctggtcgacgccaccaccgaggtcatgggccggctgcagcgcctgctcgaccaccagaagcgcttcgtgcgcgacagtgcccatcagttgcgcacgccgctggccgtgctcaaggcccaggtgcagtcggcaaggcgcggcgatgtggcgcccgaacaggcgctgcgcgaaatcagccagacggtggagcgcgcgactacgctcgccaaccagatgctgtcgctcgccaaggtcgagcagctgcggcagcagccggaatcggttccgctggagcttggcgaggtggtgcggcagatagcgctggacctgtcgccgctgatcgccgacaagtcgctcgatttcgagctggacatcgaccaccccgtgacggtgcgcgcgcaccagtggatgctgcaggaactcacgcgaaacctgctgcacaacgccatcaagcagagcccgcggggcggcgcgctttccgtcatggtgcgctccgacgaggacgaagccgtgctgacggtgcgcgacgagggacctggcatttcggccgaactgcgccagcgcctgttcgcgcccttctccgccggcgacacggccagcggctccgggctgggcctcgcgatctgccgcgaaatcgtgctggcgctgggcggacgcatcagcctggacaaccgcagcgtgcaggaaaattccgcacaggtggtcgggctcgacgctgtcgtgcggctcccggtctaccgccacaattcttgaatatggatcgcttgcgcatcgacaaatggctctgggccgcccgcttcttcaagacgcgatccctggctgcggatgaaatcggcaagaaccgggtgcaggtcaacggggacattgccaaggcctcccgggaggtcaaggcgggggacaccgtggccatccgcctgggcgccgtgacgcgcacggtcacggtgcgcggcttgagcggccagcgcgggccggcacccgtggcgcagcagctttatgaagaaacgccggagagcatcgcggcgcaggccgagatgcgcgagcaacgccgcatgggcagcgagccagccttggccatcgtgcagggccggccgaccaagcgcgaccggcgcgaactcgacggcgcggcacggcatgccgactgggacaaccgctggagcgcgtccatcgatccgaacgacaccgatcgctgatcgcccgctgccgatcgcgtacgctgcgtgtctttgcacggagcccgggttcatggccaacctcaagaaataccgcgtcgacagcaccttcaaactctcgcaggtaagccccggcgaaacaccctttctcgagggaaacacggccgcgcaggtcgccgagatcgacgccctcgcggtcgaactcgacgagatgcaggatctgctgcatgccgaaggccgccgcaaggtcctcttggtgctgcaaggcatggacaccagcggcaaggacggcaccgtgcgctgggttttttcgcgcacttctccgctgggtgtccgggtcacggccttcaaggtgcccaacgacgacgaacgcgcccacgactatctctggcgctgccatgcggtggtgccgcgcgcgggcgaaatcgcggtgtggaaccgcagccactacgaagacgtgctggtgcccgtggtcgaaggctggatcgacagggccgaggccaggcggcgctatgcgcagatcaacgatttcgagcgactgctggtcgagaccggtacggtcatcgtcaagtgcatgctgcacatcgacaaggacgaacagcgcgaacgcctgcaggcgcgcatcgacacgcccggcaagcaatggaagttcagcatgggcgacctcgaagtgcgcaccaagtggaacgcctaccaggaggcctacgacagggcactgcgcgccacctcgaccgagcacgcgccctggtacgtgatacccgccaaccacaagcggcatcgcaatctcatgatcgcgcaactgctcatgaagaccttgcggcagatgaagctcaaggcgccgcccgtggatcccgcgctcaagggcctggtcatcaagtgagcgagcggctggttgccgccggcgcgcaccgtgccggcatgctcccgcgtcaggagcggcgaacggccggctgccccagcacgcggcacttgccgaattcgcagcgcaccgcccaggtggcgccgttcgaacacggcacgctgtacgactcgtagcccgggcccttggccatcagttcagcccgcggctgaatgctgcattggccggccttggcaagagtttcggcgttgtaggtgtccacgcccgtcctgcgcggcgccagaacgacctcggggttgaaggtatggccgtagaacgtgtcgcgcacgttggggtcgagattgcggtagccgcgcttggccatgcagtgcaccagcgcgatctgctgatgctcggcaatcaggctcgcatcgggccggtaggacatgtcgatcgccgccgccgaaatgcccgtgtacgaagccgcggcaacgatgccctggccatgcaccgtgatcaggcccaggcccaatgcgagccacatggcgtcgccagactcgctacgcgcggtgatccgcatcgccgcagcgcggcaaccggccacgtcgctgtcatagcgggccttgtcgacaccctccatggccaccatgggcacataagtaagccccgatcctgttccgggctgcgtcggagtcggtggcggcgtgctgacgcacccggccaatgcaacaacggcgcacacgatgctcagcagcagcttcatggaatttccctcgtcctctttcgcgatatttccgccgatttaaccatacagatggttacttttgcgccaattttgtcgcaacctcgcgacggccagcggcttgaatgctttcggctacaggcttcggaggacgaggcgttgtacgcggcactgcacgtgcgctggatcagagcgtctcgtgttccttgagcacgcccgccttgcgcagggaagccaccagccacttggccgtcgtgtcgcccctcgcaatggcctcgattcgcgctgcttcttcctcgaccttcagttttgccgcgcgaatgaacgcttcgactttttcccgctcgaccaccaccacgccgtcggcatcgcccacgatcaggtcacccgaacggacggccacgccgcccacggacaccgtgtgcccgatccgccccggggccagcttggtcggaccgttgggattggtgccgaccgagaagacgggaaagtccatctcgtcgatttcggcgctgtcgcgcaccgcgccatcgatcaccacgccggcaatgccgagctgccggcaggcggtcatcatgatggtgcccatcagggctgcgctctggtcgcccttgccatcgatcaccagcacgtcgccgggctttgccagcgcaatggcggcgtggatcatcaggttgtcgcccggccgcacttccaccgtgagcgcactgccggccagcttcatccggtggcgcaaggcccggatacggccatgcagcgcgccccggcggcccgcaacgtcggcaaggatggcgggctggaaagccgaagcctgccggaccagatcgggggaaacgcgttcgaagtcgcgcacgatatcgggaagctggttcatcgtctctctcgttctcgttcttactcggccttgacgtcggcgtctttcaccacgcggccccatttgcgcttgtccgcagccaggaaggcgcggaactgctcgggcgtgctccccacaggctccaggccgtcggcggcgagccgcttggagatctcgggcatcgcgagcaccttggcgacttcgcgctggatacgctcgacgacggccggcggtgtgttcttcgccgcgcaaatgcctgcccatgtcacgggttcgaagtcgggaacgccggcttccatcaccgtcggaatgtcgggaaaggcggccagccgacgcgagctggccacggccagcgcgcggagcttgccagcgcgcgcgtactgcatcgagctgacgggctggtcgaagatcatcgagacctggcctgcaatgaggtcggtcatggcttggccggtgcccttgtaggccacgtgaacgatgtcgatgccggcgcggctcttcagcatctcgcccgcaagatgcccgcccgtggccgtgcccgatgaagcgaagttgatctcgcccggcttctgtttggcgtaagcgaccagttccttgacgcttttcaccggaagcgtcgcgttgaccatcagcatgtagggcgcgtagatgacctgcgtgaccggcacgatgtccttctcggaatcgaacggcatgctcttcaggacatgcggctggatcgacagggttccggtggtgcacatcagcagcgtgtgcccgtccgcgggcgcgccgagcatggccgacgcagcgatgttgccgccggcaccggggcggttttcgaccagcacctgctggccgaggccttccgccagtttcggagcgatcaggcgtgccacgacgtcgttggatccaccgggcgagaagccgacgaggatcttcaccggtttcgacggaaaagcatctgtaccctgcgcctgggcggcgccgagccagacggtgcttgcggcaagagccggcagcagcttcaggagtggtcggagtttcattgcagttcctggttgatggcttggcccgaaagttcatcgcgcgcctgcgcaatgcgacggcaaccctccagcagctgttgggtgctggcggcaaaagaaatgcggaaatgcgtcggcacgccataggcgctgccctgcagcgccgccaggtcctgcgaatcgagcaggtgcatcacccagtcgtcgctgctctcgattgcgacgcccttgcgtgtgcgaaggccgaacaatgcgctgcatgaggcgaagatgtagaacgctccgtcgggcacttcgcaccggatgccgtcgatggcattgagcgaggcaaccaccgtgtcgcgccgcttctcgtattcgcgccggttcgcggcaatggtgtcctgcggccccgtgagcgctgcaacggccgcagcctgggcgatggagttcggcccggacgtgctttgcgactggagcttgaccatcgccttgacgagtgccgaaggccctgccccgtagccgatgcgccagcctgtcatcgcgtaggccttggaaacgccgttcaccgtcagggtgcggtccttgaggtcgggcgcagcctgggccatggtggcgaacgctacatcgccatagatcaggtgctcgtagatgtcgtcggtcaagatccagacgtgagggtggcgccggagcacctcggccagtgccagaagctcggcacgcgtataggtcgccccgctcgggttgttcggcgagttcagcatcaaccagcgcgtcttgccggtgatggcgcgctccagatccgcaggctgcagcttgaagcccatggctgccggacagtcgacgaagaccggaacgccgccggccagcagcgcgatgtcggggtacgacacccagtaaggcgccggcacgatgacttcgtcgcctgctgcaaccgtgcacatcagcgcgttgaagattacctgcttggcgcccgtgccgacgatgatctcgctcggcgcgtaggccagtccgttctcgttcaggaacttgccggcaatggcctccttcagcgacggcgtgccgcccacatccgtgtaccgggtctggcccgccgccatggctcggattgccgcctccttgatgtgatcgggcgtctcgaaatcgggctcgccggcggtaaggccgaggatgtcccgacccatcgcgcgcagctcgcgcgctcgctgtccggccatggaactgggagacggcttgattcgattcaggcgtggagcaatgtgaagcatgcaagcagtatcgaagtccggttgccgcaggacaaacgagaaatcggagcagtgagctattcctttttttcgtgcggcaagccttgggcgtacattccactggaatgaacttcaccttcaagcagctggaggcctttctcttcagcgccaggctccagagcttcagcgccgcggcggtgaagctgcacaccacgcagtcggccatctccaagcgcctggcggagctcgagcagtcgcttggcggccccttgctgcatcgcacgtcccacggcctggaactggcgcaggccggcagagagctgctgccgctcgcggaagaagcccaacggctctggcagcgcatccagcacgacatcagcgtcgacaagacgctgcgcggcaccttccgggtgggtgtgacggaactgatcgcgatgacctggctcacgagcctgatccagctgctccagaagctgcacccccaggtgacgctcgagcccgtggtggacgccgggcttacgctcttcgagcgcctggaagccaacaagctcgacctgaccatcatgcccggcaccttctggggccaggctttcgaatcgatcaaggtggggcaagtcgaccaggcctggatcgcgagcccgcggctcgacattcccgcccgggccctgaagccgcatgagtttgccgattaccccgtgatcgagcagcccgccggcgcctcgaagaacaggttctacgaagcctggcgcgcagagcacgggtttcgcttcggcaaggtcatgctgacgaacagcacgaccatcctgcgcgaactgacgatcagcggcttcggcatcagccagcaggcgctcgactacgtgcgcccggacatcaagagcggcctgctgcgggtggtgaagagcgaccccatgccaccgcccctggtctacagcgcggtctaccggcgcgacaatttcagtcccgcgctgacgcgcatcgtcgagctggccgtcaagacctgcgacttcaccctacgggcaagccagcacgacgtggccccggcccgcccgccgcggggctcgggcgggcccctgcggcaacgcgcgctccgccagggtgcgaaggcaccggtcaggaagaccagaaaatagttgattcatcgagcgcgcagacctcgccgtccaccacgcactgccggcacttcaacttggccagggctctgcgcaatctcggcaaaccatttcgttgcatcggtgccgttgcagcttgcctcgaaatcagcgcaccccgggtgcaaagagcaagccgctcgtcgcagtggtttaccgattaccggtaaacactataaaatgcaacatggcgatccaatccttctcctgccccgataccgaagagcttttcaccaagggcaagaacgctcggttcgccaacatcaaggatgtggccacgcgcaagctgacgcaactggatgcagcgacttccgtggcattcatgaagatgcctccgggcaatgatttgaagttttacgacgatgcgtggcacgtcaggatcaaccaacaatggcgcctgaccttcaagtgggcagagtcaggcccctacgaaatacgaattgaagacccacactgaccggccagcctgccggataccgcacctagatagggcacttttatgatgaaaaatggaatgcgtccggtccaccccggcgaagtcctccgcgaggattacttgaagccgctcgggatgaccgcgaacgcgctggccaaggcactgcgtgtgcccgcctcgcgcatcaatgacatcgttctcgaacgccgcggcatcacaccagacaccgcgctgcgcctgacccgctatttcggcggcgaagaggcggacgcgcagggctggatcaacatgcaagcgacgtacgatttcaaggtcgctcagaaggccgttgccaaggtcatcgcgaaggaagtgaagccgcgcgacgccaaggaagctgcggcaccaaacgacgagcgattcgcattgggcgcttgagggcgggaatgggctggaaagcctcagaacgcccaagaggtcagaccaatgaaaaagcccagtaaatcaatgatctactgggctttttgggggcttctggaaggcaccagaagccgtattggcggaaccggagggattcgaaccctcgatgaggctctacaccccatactcccttagcaggggagcaccttcggccactcggtcacagttcctgaaagaagccgagattatgccaccgtcaggcggccggttgatccagatcgaaggctttgtgcagcgcgcgcacggccaattccatatatttttcgtcgatcacgaccgaggtcttgatctcgctggtcgaaatcatctggatgttgatgccctcttcgctcagcacgcggaacatcttgctggccacgccgacgtggctgcgcatgccgatgccgacgatgctgaccttgcaaatcttggtgtcgcccacgatttcggtcgcgcccagcgagggcatgaccttcgactgcagcaggtcgacggtcctggcgtactcgttgcggtgcaccgtgaagctgaagtcggtgcggccgtccttgctgaggttctggatgatcacgtcgacctcgatgttggcatccgccacggcgccgaggatgtgatacgcgatgcccggcttgtcgggcacgccgagcaccgagatcttggcctcgtcgcggttgaaagcgatgccggatacgacggcttgttccatgttttcgtcttcctcgaaagtgatcagcgtgccggacttggcctcttcattgatgtcgatgtcccacggcgtgaagctggagagcacacgcagcggcaccttgtacttgccggcgaattcgaccgagcggatttgcagcaccttggagcccaggctcgccatttcgagcatctcttcaaagctcacggtcgagaggcggcgcgcatcgggctccacgcgcgggtcggtggtgtagacgccatccacgtcggtgtagatcaggcactcgtgcgccttcatggcggctgcaatggccacggcggaggtgtcgctgccgccacggcccagcgtggtgatgttgccgtcttcgtccacgccctggaagccggtgatgacaaccaccttgccggcgtcgaggtcggcgcgcacgcgctcgtcgtcgatgctctcgatgcgggccttggtgtaggagttgtcggtgcgcaccgacacctgccagcccgcgtagctcacggcttccatgccttcggcctggagggcaatggccagcagcgccgacgacgcctgctcgccggtcgaggcgagcatgtcgagttcgcggccatgcgcctcgctgggtttgctcggcgcaagctccttggccaggccaagcaggcgattggtttcgccgctcatggcactcgggaccacgatcatctggtggccggcgcgtgcccatttggcgacgcgcttggcaacattcttgatgcgctcagtcgagcccatcgacgtaccgccgtatttgtgaacgatcaatgccatgggtgaattcagagaaaaagaaagggccgctccactccggagtgcaagcgcggcgccctgcaagccgtcagcgcgaagccttgggcgagggcccggaattgtaccaatgcagaaaatcgcccctgcgctcgatgaaaccactggccaccttcaggtggatgcgatggccgcgggtggtgcaggcacgaacctggtccagcagctggtccagctgcgccgcgctgggcgcgcagccgtgcgcctgcatgagccagtggcgcagcacattggcctgccgcgcgcgcgaaagcgcctgcagctctgcgatgcggggcggatcgcccaccacggccaagtcttgcgcggcgagttcgctcagcaattcctgcgcctgcgcggcgtggccgatgctgcgcgcgaaggtggcgcggaattgcggaaaaatccgagccagcgcgggtagcagcactgcgcgaatccggttgcgcgtatagcgctcgttctggttggtcgggtcctcgatccaaggcaaatcgaggccttcgagccaagcccggatatcggcaccagcgaccgccagcaacggccgatggatgtcgagtccgtggcgctgcgcatgcgcgggcatcgcggccaggcccggaagacccgcgccccgggaaagggccagcaacagggtttcgacctgatcgtccgcatggtgccccagagctatggatttgatagcgccagcgggttcgccctcgcgcgccattgctgcaaaagcttcgtatcgggcgcgccgggccgcatcttcggggctgtcgccttgggcatgccgggcatcgacgcggtgcaccaccagcggcacgccgaggcgctcacacaccgcggcgcagtgccgttcgaaatcgtcagccgcggcctgcaggccatggtgcacgtggaaggccaccacctgccccggccaggcggacgcgcacgcggccagcaaggcggtggaatccgcgccgccgctgaagcccaccgccagcggcagatgcgccggctcgaacgcggccatcgcgcgttcgaaggcttcgttcatggggcgcttgcttatctgccggtgtcggccttggtgtcgttgaagcggccgtagctctgcaggcgctcatagcggcgatcgagcagttccttcggcttcaggtcgctgacctggcggaatgcgtcgttgagcgcgcgcttgaggaaagcggccatctggcgatggtcgcggtgcgcgccgccaaccggctcattgacgatcttgtcgaccaggcccagggccttcaggcggtgcgccgtgatgccgagggcatcggccgcttcctgcgccttgtcgctggtcttccagagaatggaagcgcagccttcggggctgatcaccgagtagatggagtactgcagcatcacgagctggtcgcccaccgagatggccagcgcgccgccggagccgccctcgccgatgatggtgacgatgatcggcacctcgagctgcgccatctcgaagatgttgcggccgatggcttcggactggccgcgctcctcggcatcgatgcccgggtaggcgcccggcgtatcgacgaacgtgaagaccggcagcttgaatttttcggccgtcttcatgaggcgcaaggccttgcggtagccctcgggcttgctcatgccgaagttgcgcgcagtgcgctccctcgtgtcgcggcccttctggtggccgagcaccatgcagggcgtgccgttgaagcgcgcgaggccacccacgatcgagaggtcgtcggcgaagtgccggtcgccgtgcagttcgacgaagtcggtgaagatctcgttgacgtagtcgagcgtgtaggggcgctccggatgccgggcgatcttggtgatctgccagggcgtcaggtcgctgtaaatgtccttggtgagctgctggcttttcttgccgagctggtcgatttcctccgagatgtcgaccgccgattcggtctgtacatagcgcagttcttcgatcttggattcgagttcagcaatgggctgctcgaagtcgaggaaggttcgtttcgccaacgtcttctcctgttgttcagtatgcgaccggtaccgggtcgagcgagcgccaaatataccaagtcgccacgctgcagtacggcgcccaggccacggcgacgtcgcgggcatcgcttcggctcaccggatcgcccgaaaaataattgacgctgatgccgttgagcaggccgaggtcgtcgaccggcagcacattagggcgcatcagatgaaagatgaggaacatttcggccgtccaccggccgatgccgcggatggcaaccagttcatcgatgatgagctcgtcggccatgtccttccaggcgtcgacgtgcaccgcgccggaatcgaaatggatggccaggtcgaccaggtactcgaccttgcgggccgacagccctgccccgcgcatgtcgtcgaccttgagcttgagcacgttggccggcgtcagtttgcgcggcagcaccgcgaacttgtcccagaccgtttgcgcggccttcaccgaaatctgctggcccacgatgcttcgcgcgagcgtggtgaacgcgtcgccgcgcgactccaggcaggcatctccgaacttcggaatcagccgcttcatcacccggtccttcttggccaggtgcttgcaggcctcttcccaatagtccggcgtgtagatcttgaccgccggattcctggaagcgggcatggggttggtcgttccgttcactgggcggccgcccaggtcgtgccggtgggcgaatccttgagcacgatgccctgcgcaagaaggtcgttgcggatgcggtcggcctcggcgaagttcttcgcggccttggcggccgcgcgcgcgtcgatctgcgcctggatggtggcttcgtccagcgtcgcgcccgcgcgcaggaagctcgtcggatcgctctgcagaatgttcaggcagccgcccaacgccttcagcagcccggcctgtgcgggcgatcgcgtgcggttcacctcgcccgccaggtcgaacagcaccgcaaccgcctcgggcgttgcaaagtcttcgtccatggcggccttgaagcgcgccgcataggggtcgttccagtcgatggctacagcttcaggcgcgaccaggtcgagtgccgtgtaaaggcgcttgagcgaattgcgggcgtcgtccaggtgcacgtcgctgtagttgagcggacggcgatagtgcgcccgcaccacgaaaaagcgaatggtctcggcgtcgtacttcttgagcacatcgcggatcaagaagaagttgcccaggctcttggacatcttctcgttgtcggtcacgatgaagccgttgtgcatccagtagttggcgagcggcttgccggtggcaccttcgctctgtgcaatttcgttctcgtgatgcgggaactgcaggtcttcaccgccgccgtggatgtcgagcgtttcgccgagcagttcgcaagccatggccgagcactcgatgtgccagcccggacggcccggcccaaactcgctggcccacttcacttcatcgggctcgctcgccttggcgctcttccagagcacggggtcgagcgggtcgtccttgccgtcgagcacggccacgcgttcgcccgcgtgcagctcgtcgatggacttgccgctgagcttgccgtagcccggaaactttcgaatcgcgtagttcacgtcgccgttgtccgagcgataggccaggcccttcttctcgagcgtgccgatcatcgacagcatctgcgggatgtagtcggtggcgcggggttcgtgcgtgggacgctcgatgccgagcgcatcggcgtcttcgtgcagcgcgtcgatcatgcggtcggtgagcgagcggatcgtctcgccgttctcgacggcgcggcggatgatcttgtcgtcgatgtcggtgatgttgcgcacgtaggtcacgccgtacccgttggccttgagccagcgctgtacgaggtcgaacgcgatcatggagcgggcgtggcccagatggcagaggtcgtagaccgtcatgccgcaaacgtacatgcgcaccttgccggcttgcaatggggagaattcctccagttcacgcgagagcgtgttgtagatgcgcagactcatgaggctcggaaagcgtcgcttcgcgcacgtgcggcacgggcgaacgacggtgtatttcaggggtgacggggcagtggctgcgaggggttggacatggcccctcggctacaatgcagcgcagtataaacggctactgccgtgtccttccgggtgttttcgaggcccgcatttcccaatcctgccgaggcttcatgaagcacgtcgcattcaccaaattctccctcgcctttgcactgctcttcagcctgtggggttccgccgcgtatgccaacgactacgacgacgtgaacaccctgctgcgccagggcaagtcgaacgaggcgctcgccaaggccgacgcctacattgccggcaagccgcgcgacccgcagatgcgctttctgcgcggcgtgatcctcaccgagcagaaaaaacagaacgaggccattgctgcgttcacgcagctgacgcaagacttcccggaactgcccgagccctacaacaacctggccgcgctctatgcatcgcagagcaagttcgaccaggcgcgcgcggcgctggaacaggcactcaagctcaacccgaattacgccaccgcgcatgagaacctgggcgatgtctacgcccgcctcgcggcccaggaatatgtgcgcgcgcagcaatttgccagcaccaatgccagcgttgcgcccaagctctcgctgatccgccagatcttcacccccaagaccgaagccgatgccgcggccctgccggcggcaccgcccgaagctcgcaagccggtcggccgcgcgagcaagtagtagcctgcgagcaaccgccaacgcgttggtgccgcggcagcttgcattggccggcccgagccccacatcattcgcacaccggagccttttcttgacgacccaagtccttatccaatccgctcgattcagccgccgcgccgcgctggtgctggcgtccgccctcgccttcgccggcgctgcacatgcagaagccggcccgcgcgtgaagctcaacacatcggcgggcgacatcctgatcgaactcgaccaggccaaggcgcccaagacggtcgagaactttgttcagtacgtcaaggacaagcactacgacggcaccgtgttccaccgcgtgatcgacggcttcatgatccagggcggcggcttcacgcctgaaatgcaacaaaagccaacccgggcccccattgcactcgaagccagcaacggcctcaagaacgacaggtacacgatcgcgatggcacgcaccggcaatccgaactcggccacctcgcagttcttcatcaacgtgaagaacaacgattcgctcaacgcgcccaacccggatggctacggctacaccgtgttcggccgcgtcgtgtccggcaccgacgtggtcgacaagatccgcgctgttcaaaccggtaacaagggcggcatgcagaacgtgccgctcgagcccatcatcatcaagtccgccacactggcgaagtaatttccgaacatccgaaagaaggactccctcatgagcaaccccaaaatcgaactccacatcaagaactacggcgtgatcacgctcgaactcgacagcgtcaaggcgccgaagtcgtccgagaatttcgtcaactacgtgaagaacggccactacgacaacacggtgttccatcgcgtgatcccgggcttcatggtgcagggcggcggcttcgagcccggcatgaaacaaaagcccaccggcgccgagatcgagaacgaagccaacaacggcctcaagaacgacaactacaccgttgccatggcccgcacgagcgcaccgcactcggccaccgcccagttcttcatcaacgtggccgacaacggcttcctgaaccacaccgctccctcggcccagggctggggctatgcggtgttcggcaaggtcactggcggcaccgacgtcgtcgacaagatcaaggccgtgaagacgggccgcaagggcttccatgacgacgttccgctcgaagacgtcgtgatcgaaaaggccgtggtcgtctcggaataaagactggcgcggcatgggctcggacatcgcggcacccccggctttcaaggagctgctcgccccgcccgcatggcgcaccgtcgacctgatttccgacctgcacctgcaggccggcgagcccgccaccttcgaggcctggcggggctatctggagaccacgccggccgatgcattgatcatcctcggcgacctgttcgaagtatgggtgggcgacgacgcggccgacctcccaggcttcgaggccgagtgcaccgaattgctgcgccgcacggccgagcggctgccggtgtacttcatgcacggcaaccgagacttcctcgtgggcccggcgctggccgcgcgatgcggctttgcgctgctggacgatcccacggtgctggtgctgcaccgtgaacgctggctcctgagccacggcgacattctttgcctggacgacaccgactacctcaagtttcgcggccaggtgcgcacgcccgaatggcaggcggcgtttctggccaggccgctggccgagcgccgcgcactcgcgcgctccatgcgcgtgcaaagcgaagaccgcaagcgcgacccgtcggcgcgctgggccgacgtggatggcggcgccgcccgccaatggcttcatcaggcgcgtgcgcgcacgctggtgcacggccacacgcaccggcccgccaatcacgacctgggcgacggcctgcagcgcatggtgctgagcgactgggacgccgcggcccacccgccgcgtgcgcagttgctctgcctttccaccgccggcgcgcagcgcgtcgacctgcgctagcgcggcccatgttcaagtggctgcgccggttgcgcgccctgcccccgattcccgaagctgcctggcgtgccacgctcgagcgctatgcctttcttggcgcattgcccttcgacgcgcagcagcggcttcgcaccctggccgccgaatttctgcgcgacaaggaattccatggcacccagggcttcgtcatcaccgacgaggttgcgctggccattgccgcgcaggcggtgctgccggtcctgaacctgaagggcgggctgaactggtatgacgatttcgtcggcatcgtggtgcatccgtccgaggtggtcgcgcgccgcaagatcgtcgacgaagcgcaggtggtgcacgaatacgacgaagtggtggccggcgaagccatggaccgcggaccggtgatgctgagctggcaggacgtgcttgcgagcagcatcacggcgggcggcggctacaacgtcgtgatccacgaattcgcccacaagatcgacatgcgtggcggcgacgccgatggctgtccaccgctgccgccaggctttgcgggcaagcacagtgcccgcgaatcccgcgccgcctggatcgcagtgctgcagcccgcctatgaggattttcgcgagaagacgatcctcgccgaccgcttcggcgccgaagcgccctggctcgacgactacggcgcgacatcgatcagcgaattcttcgcggtggcctgcgaggcctacttcgtgaaccgtccgaacttcgcgcgcgacttcccggcggtgctggctctcttcgacgaattctttcgggccgaacaggcctgatcgcgcatcgcaatctgcgtttccttgcttacgcgcacgatacggcccgcctaccccgtccagggtatgagccgcccgcgcggcaccttgtctttgcaggccgcaggcgtagcatcgctgcggccatcgcccaccacagccccgtagcaccgttgcgcgcgtgatgacctgaagcgtcgccatcgggggcggcgttgcttcatgtgatgccccccgtggataacgcaggagcgaaaaatggtgacctatatcggtatgctgaatttcacggacaagggcatccagagcgtcaaggaaaccaccaagcgcgccgctgccgccaaggaaagcgcccaaaagctcggcgtcaaaatgcgcgatatttattggaccatgggcgactgcgacgtggtctgtgtgctggaggccgaggacgagcaggcgatcgccgcattcagtctggcgattgccatgcagggcaatgtgcacacgcgctccctgcgggcctacaccgccggtgaaatggaccagatcctggccaagctgccttgagcggtgtcggctggacgccgggactgcggcgctgccgagtcaggtgaaatgaaaaagcccgcgcgcggcgggctttctcgtgaacttgcgccgaagaagccttacttgcgcagcaaggccttcagtgcgttctgcaaacggcgtgcgctcgccgtgtcgtgcgccgcagccagtaccttgcctgcgtcctggccccaggtctggaccggcggtggatcgccgcgcttcgtcagcagtttgagctgcagtgcgcggcgtgcgtcgagctgctcggcgggcgtcggcacttcggcggccatttccaggcgcaacagtgcttcggctgcttcatcgggagcggccttgggcgccgaaccgacggcctgagaccagccgctgcgcaccgcgggcgtcaccgcacgccccaactcctgcacgctgggcagcttcgaggcatcgcgctgttcccatgcgccaagcacttgcgtgagcgcttcgccatgcgcttgcgctgccagcttgcgcagcgccatgtccgcacgctcgagcgcttcgcgctgggcgcggaaggcggcatcgccgagcctcgggctacggtcctcgaagcgcggcggacgatcgccgaagcgtccggccggcgcgccgcggtcgccgcgggcatcgggacgaggcgctccgcgatcgccgggacggccagggccgcccgggcccgggcgggcgccgtcgcgccgatcgccgaacctgccgccagcgcggccagcaggtgccgcgtccgtcttcttgctgccaggacggtcgtcgccgcgcatggccacgaccggcttggatgcaggcttcggtgccgccgcgggcgccgggctctcgacagcagccgcttcgccggcttcgtgtgccgcatcatcggtgcgcgcagacgcgtcagcgccgtcggccggtgccacgaggtcggaagttgcagcttccgcggcttcgacgcgtgcagccggcaaggcttccgcatcgctcgagcccggggcctgctcggcgctttcgccgaattcagccgcagcctgtccgggcgcggccacttcggttgcgccaaccgaggggccgtcgctggaagcggccggcgcttgctcgggcttcgcggcgggtgccggcgggggcgcttcgccacgcagcgcggcttcgaggcgcgcgatggcggcgcggatcttctgcacgtcgccgccagcgttggccgcgtcgagcgccttggaggcctcgagcacgtggcgatcatgttcgctcatggcggaggcagacttctcgcgctctgccgtcttgcggttgaaggcttcgtcgataggggcgcggaatgcgtcccacagcttctgttcgtggcggcggtcgagcggcacgctctgggcttccgcctgccagcgctgctgcagcgccttgacggcatcgatgcgcagcatgggttgggcgccgagttcggccgcctccgcgatcatggcctggcgccgttcgatgctggccttttgcgcggtctcgaagggagcacgcgcggcaccgaaggcttcgttccactgcggctgcagctccgcgaagaccttctcgcccacgtggccggcatcgcgccagcggtcggcaaactgatgcagcgcgcggttgtgcgccttcaggtccgaagaggcggcatgctctgccgcccaggccttgacctcttcgatgagcgccacgcgatgggcgcggtgctcggccgcatcggcgcgaaccttttcgagccaggcttccaccaccttgtgggcttcgttgcaggcttcgtcgaagcgcttccagagcgcatggttcggcacgccgccctggtcggcctgtttccactggtcgcgcagcgagcgcagcgtttcctgcatcttgcggccgccgagcgcctggccttcggggcgcttgagcaagccttcagccttggcgacgaggtcttcgcgcaccttgtcggcgctccagcgctgccagccttcgagttcgccggcggcaaccagcgccgcatgcacacgggcttcgagcggcgcatcgaccagcttgccgtgttccttcagcactgcgcgcagcgctgcggccgcaccggcgctggccttgccgtggccttcggcggtttcctgttcgagcttggcgagcgcggcctgcacggcgtcttgcgcggcggcgcgcacggacgggtcgaccttgggtgcggcgggcttggcaggcgcggccttgggggccaccacctcgccgcgggcggcacgcagttcgtcggcccacacgggcaccggcggcaggggggccgcggcatcggctgccgcagcctgcgcctgggccagcgcaccgtggaaggcatcggacacgaccagcaattgcgccttcgacgactcgagttgcggggcaaacctggcgtcgaggctgttccagttggcatcggccgtgatgtcgccggcctgctgctgccagtgggtcacgtcggcgcgcagcgattcctcggcggcctgcgcgtcctgccagctcttggtcgacagcacttcgaagcgctgcgcgagcagcacggcggcctcgcggtgcacctgggcacggtgctgcaggtcttcgatgcccttgacgcgctcggagagttgcaccttgaaacctgcgagcggctcgcgcgacagcggcgcgccggccttggcggcgtcgcgctgccaggcaagcgcatcggcaatattgagcttggactgggccagcaaggcctcggccttttgcgcccattcggccgcaatggcttcctggcccttggcgcgcttgagttcgtcgagcttttcgcgcaagaggcgcgccgcgcccttgtcgcggccgctcagttccttgaagacttcctgcatttgctcaggcgcggggttgcccgcgagccagtcgcggatgcgcgcggcgcgctcgcccgaagttggcgcggtgaaggcgccgccggtgagcgtgtcgagggcctggaggtcgtgtggcttggaagaagtagaggtcacttgcgcgaaatcgttgtctgaagagagaaagcgaaggcgccggcaaaggccggcgcacatcgacattttcacccacttgtggcgggcggttgaattacatgccgcaacagcagccaaatggccgccggaatgtcggcggcggctgcctacatatatagcgcggcggtacgaaaaaccaagtgtctgcgggtcatttcatggccagcttgagttcggcgccgggcttccagtcggcaccgcccgccgtggttttcacggcgccaaggaacaggcgttcgctcggcagcttttgcgccagcaggtagtcgcgcaccacggcaccgcgctcgacggccagttgccggatcgactcctcgtcgaccggaacgctcgcgagcagcaggttttccatctccttgacgggcaggtccttggcgagcccgaccatgttgcgcggcttggtgatgtcggcgcgcttgtacacggcggtcagcagttcggggtactcggcatcggtgaccggcggcacgtcggtgcccgcctggccggcgcgcaccaccacgcgccgcttctcggcctgggccagctggcgcaggcgctggcgctggtaggcgtcgcgctcccgctcgaggctggccgtgccgaccacggtcatctgcagggccgggcgctccgtcaatgccttgacgaccttgtccaggctctccttcgcgccggtgctgagctccgagcttccggattcgaaagcgacggtgctcgattcgctgctgccgccgcccagtccgccggtcagaagattgaagggcgcggtcgccgccttcacgatgaggttgaccacggccttgaagatcagcgggccgatgctgaactgcggatcgttgagcgagccgctgagcggcaggtcgacatcgatcacgccgttgcggtcggccagcaaggccaccgcgagccgcaccggcaagctgttgggagcgccctgcacttcttcgccgaactgcaactggttgagaaccagcttgttggtggctgtcagctggccatcgggcgctatcttgtagttgacgtccatgctcatcttgccgcgctcgatgccgtggcccgaatagcgcaccgagtacggcgacagcggcgccaggtcgaggtcgcgcatcttggccgtgatgtcgagctcgatcggcttgaccagcgggttgagcttgcccgtgatttccagcgcggccgtctgctgcgccttgccgcgcagttccaggtcagccagcgcggggcggccgctctcgcccttcggcggattcgacgagaaggaactgagcttgccggtcagttcgctcagatcggcggagtagttgggcttcacgaacaggtcggtgaagtcgatgcggccattgaccaggctcatcgggccgaagttgatgaccggttggggcccggcatcggcttgtgcctgggccgctgcgaccggcgccgaggccggcctggccggctccgagctgccgccgaccatggactcggccgataccggcgcgccgcccgcctgcgacgggggccgggtcgtggtggtcgttccgcccaggctcctgcgggtcttcgcctcggtggtggctgcggcggcggcattggcttccgcttcgcccttcttggtgaggttcacgaggttcaggcggcctgtggggtcgacgatcacgcgcgcgaagaagtcggtcagcgtggtttcgcgcacgtccaccgccggcgccgcattgggcgccatgctcacctgcaggccgcgcaggctcagcgtcttccagctcagcagttggttggtgttgcggtcgaagccgggcgactgcgtgagcgagatgctgttggcgcggaaatcgtcgagcgccgtgtcgccggccagcttgagagtcatgcctgccggtgcgttcgcatagcgcacggtgccgcggtagctcgcgaaggcacggcggatgtcgacgttgagggcatctgcgtagtacgccttgaaggcatgggcgggaaacgacgccacgtcgagccggccctcggccgcgagcggcttgagcaccaggttgcccttgtagtcgaagcggcccggctcggaacgcctcgaaccgatgcggcctgaaatctgcaggggcgacaccgtggcggtgtcgggcgcgatcttctgggcgttcacattcagcgccgtgaactcgaccgcgaccggcgtggcgctggccttgtcggcatatgaaagcgtgccgttctcgaccgccagggtgccgatggtcaaggcccagggcttggtgttggcgccgggcggtgccgttgcggtgcccgcgccggcgggcttgggcgcagccaccttggcctgtgctgccgccccgttgccggccgccggcgccttgagccagcgctcgaacatccagcgcttctcgctgtcgcgctcgacgttcaccttcgggttggtggcggtgaacgaagccacgttcagcgtgtgcttcgtcatgtcgacctcggcatcgaccagctcgaagcggcccacgcttgccagcgcggtctttgcctgggtcagcgcaaggccgtcggcggccaggcggcgggccttgaaccggagatcgggctcggcccaggcgatgtcgatctgcccgctgagcttgccgtcgagcgtgggctcgaggctgtgtgccaggtatggcgccgccagggacagcggcagcgcatcgacctcggtctgcacgtcggccttcttgtcggtggcgctgccctggaacttgagcgtcgcgccgccaatggcggtgctgccgctgaactgggccggcttctccatcggccaggtgacgccggtcaggtcgaggccgagtgcgctcgcctggacggccgccgcgggctgtaccgtttcgtcgcgccacccgatgcgcccgccgctgagagcgaccttgtcgacctggaccttcagcttcggcttttcaaccgtctttccggccggggcgctggctgcggatgcgggcggggccaccttttcggcagcccccgtggccggatcggtggcgagcaggttgagccggccttgcgcatcgcgcgcgaccgcaagctgcgggttggacagcgcaacttcgctcagatggaacaccgactccagcgggcgcacgtccgccagcgccagcttgagcgagtcgaagctcagcaggtcgcggccgcgggcgtcgcccaatttggcactctgcgcttcgaccgtgccggtgatcttgaggccggcggtggcggcctgctcgaagtcgattttcaggtcggcatccaggctgcccgcctgcagcttcaccggcaggccgcccggcaggtaacccaggtagggcgcgaggtcgagccccttgaactgcaggtgggcgtcggtcttgcggcttttcgcgaacggcgtggtgagggccgccgaatcgaacttgccgccgttgagcgcgaacgcgagcttgggctcggtgttcacgtcgcgcttggaggcgaggttgctcaggaagggcacgttgagcacgaaatcgcgcagttcatgcttgcgcttgaccgtctggtcgtcgaagtcgaccgcgccgctcttgatcgagatgttgtagatcgcaaaacgtgccggctcggcgttggggtcggacggcggagcggcggccagcttggccaggatgtcgtcgatgtcgtacttgccgtcggcaaggtgcgtgagcaggatggccggcgattcgatggtgaccgcgtcgatcaccggcgccaggcggacgagcgattgcagctcggcgtcggcatagattcgcttgacggccacctggggccggctgccgtcggccgtggcaatgcgcagatcgttcagcgcaagttcgagggtccagggcttgaagtcgatcttgccgaccgtgacctgccggccgagcttctcgctcgcgatcttctggagctggctcttggcgatcggcggtaccgcgagccaggcaacgatccagagcgccagaagagccagcaccgcgacgatcccacgtcgcacccatttgttttgtttgagcgaagctgcatccatcgcgggagtgtgccgtaaagaaagaacaaggcagaaacaagaaagcccggcaatcagacgaatgtctcattaccgggcttgatggcgggcccgagacccatgccatcgattcgcgcgaccggaagtcaatggttcctgccgtgctggcagcaagagattgccgccgtggatcctctgccgttcgagcccttgacttgcacctcgggctatctgacttcggaacacgcctgaataactcaggcgtgtccagattaggcgcctgacccttgcattgcaatcccatccaccaaggggataccctagggtaggcccgctcaatgggaacaatctgtttaaatatgtaattgcataagaacaaggtttcttatgcttgaccgagtatttagccacgctagaatccggcctgcccctggctgcccagacccagcaggggcctcctgaatccgccgccgaactcccccggcttgatcaggtcgccgcgcccttacccctacacctccacgcgcggagcctgattcgtaccaatccaagcgccgtagccttcatccatcgccttcccggcgctgcgaacaggtgccgcacagaaaggaagagcgatgaacaaggcgtttgatgccacggcccgcgggctaaggacctttgcgtccgatgtggcagacggcttttttgaaatcacccacaacgggtttgcactggtcggcctcgccatcgtgttcgcggccctcgccctcgtggcacggccggacctgcgccagaccggtgaggagcaactgatgggctggctgcaatcgcgcaagccggcaccggaagccaccgacctcgagccgaccgccatcgtgcgcaccacggccgcaagccctggcgacctgcccaagcagcaggccgccgtggcatattggctcagcaagaagtaccgcgtggcggccgaaccgctgagcgtgctggtcgccgaggcctatcacctcggcaagcgcaccaagctcgacccgacgctgatcctcgccatcatggccgtcgaatcgagcttcaacccgttcgcccagagccacgtgggcgcccagggcctcatgcaggtcatgacgcgcgtgcatggcgacaagtacgaaagcgcgggcggcacgctcaccgcgttcgacccggtgaccaacatgcgcgttggcgtgaaggtgctgcaggaatgcatcgcccgcgccgggtcgctcgaaggcggcttgcgttactacgtgggtgccgccaacctcgaagacgacggcggctacgcaggcaaggtgctcgccgagcacgaacggttgctgcaggtcgccaatggccgcaatccgcccacggcggcgccggtggtgcgcgcgcagccgatccccgtcgcgacgcccccgaagcggcagcaggcctccgagccggcagccgacccgcagaaagtggccctgctttcggaagtttcctgaggccctgcgctacacttcaccccgtacgcgactggcgataggcgcagcaccccccgcggtgccccgcgctgacgtggaataccactgggaagcgtgccgcctggcatccatacaggcgttcagccgttcgcctgggcagcccttgtttggttgaagaacaaggacctcgtcttcaaaggactgccatgtatcaccgcaatatcctggtcgaacagaccgatcccgaaatctgggctgccatccaggccgaaaacgcgcgccaggaacaccacatcgagctgatcgcgagcgaaaactacgcctcgccagccgtcatggccgcccaaggctcgcagctcaccaacaagtacgccgaaggctaccccggcaagcgctactacggcggctgcgaacacgtcgacgtggccgagcagctggccatcgaccgcatcaagcagatcttcggtgccgacgccgccaacgtgcagccgcattgcggcgcctcggccaacgaagccgtgatgctcgccttcctgaagcccggcgacaccatcatgggcatgagcctggccgaaggcggccacctgacccacggcatgcccctcaacatgagcggcaagtggttcaacgtggtgagctacggcctggacgccaacgaagccatcgactgcgacgcgatggaacgcaaggcgcacgagcacatgcccaagctgatcatcgcgggcgcctcggcctattcgctgcgcatcgacttcgagcgcttcgccaaggtggccaaggacgtcggcgcgatcttcatggtcgacatcgcccactatgcgggcctggtggccgcgggcgtgtaccccaacccggtgccgcacgccgacgtggtgacgtccaccacccacaagagcctgcgcggtccgcgcggcggcatcatcctgatgaagtcgcagcacgagaaggccatcaacagcgccatcttcccgggcctgcaaggcggcccgctgatgcacgtgatcgccgccaaggccgtcgcgttcaaggaagcgatggcgcctgagttcaaggcctatcagcagcaagtggtcaagaacgcccagatcgtggcggacacactgaccgagcgcggcctgcgcatcgtgagcggccgcaccgaaagccacgtcatgctggtcgacctgcgctccaagggcatcaccggcaaggaagccgaagccgtgctgggcagcgcccacatgacgatcaacaagaacgcgattcccaacgaccccgaaaagccgatggtgacgagcggcgtgcgcattggcacccccgccatgaccacccgcggcttcaaggacgaagaggcgcgcatcaccgcgaacctggtggccgacgtactggagaacccgcgcgacgccgccaacatcgatgcggttcgcgccaaggtccacgcgctgacaagccggttcccggtctaccgctgacccaggaagacgtggccgcatgaaatgccctttttgcggtcatctcgaaacgcaggtcgtcgagacccgcgtgtcggaagacgccgacttcgtgcgcaggcgccgccagtgcagcgcctgcgacaagcgctttaccacctatgagcggccggacgtcaactttccagtcgtcgtcaagaaggacggcagccgcgccgacttcgaatcgtccaaggttcgcgcctcgatgatgctggcgctgcgcaagcggccggtgagcatcgagcagatcgacaacgcattgctccgcatcgagcagaagctgcttgccagcggcttgcgtgaaatcgattcgaccaaggtcggcgaactcgtgatgcgcgagctcaagaagctcgacaaggtggcctacgtgcgctttgcctccgtgtaccggagcttcgaagacgtggacgagttcaggcagctgctgcgggacatttgagcggagccggtccgccgttcgcgtgcggcgggttcattggctgtccttgccgcaggcgccgcttccgcaatcgcccttgaggtcgggattgcagactctcgcgcggcccgaggccgacacgacgatggacgccctgcggcccgactccgccttcaaggtcaggcagccggcgccgaagcccgagccccccgcccggcgcgagaagccgttgctgtcgtagtccaggccctgcacaaaaccatctccaagccccgcatcgatgccgacaccggccgggagcttttcgaagttgcgcactatctgcggtgcggcatccgttcccgcccgcaccgcccatccgctcgaccagtcatttgcggtcagcgccacgacgtgaaccctctgcgaacgttgaatggcttcggtgcgggcgagattcagcgcggcgacaaaaccgctggacgcggccgccaggcgctggttgagcagcagatcgcgaaatgccggtacgccgagcgagccgaggatcgccgcgatggcgatgaccaccatcaattccaccagcgtgaagccgctgcgcggcctgcgcaacggcgcgcagcgcttcattgccagcacctgcttggcgcggtgccgtcacagcccttgtcgcccgtgctgtcgagccagagcgccccgacctccggatcggagaggcccggcctgggggttgcggtcagcctgacgcagcgatcgatgctgtcctgcccctcgcaattgccgctttggaccaggtatttgccgcctgcgccgccctcgccggagccgccttcgtagcgcttgtactgcccgctcagggtgtagttgcgctcctgctgctgcatctgctgcaccagggccgaccgcgcctcggtgcgccagcctttgcgcatgaagtccaggtatgacgggtaggagattgcggccaggatggcgacgatcgcaaccacgatcatcgcttcgatcagggtgaagccgtggctgcgcctggcaccgcgttgcacggtcttcatggtttcgcactccggtagtcggcaatctggcgccagttcaggcgtccggacacctgggagacctggccgccctccacggggcgcgccgtggaaatacggaccccgcgcgagccgcccggcacaccgacgttgatgacggacaccttcttcgtttccgttcggcgcccgaacgcatcggtggccgtgtaggcgccctcgcccagttcgaccagaagaggcgacgacagcagcccgacgctcgaaggaacgcaggttccgccttgcgacaggccggtcatcgcgttcaccgaacagcttcggccgccgccgttggcgccgcatgcttcggcattcggtatcagcgtgttgaagaacagatatccgtcgctcagcgccaaccgcgagacctgccgctcgcccagttccagcgcgcccgggaagtcgaagtaccagccgcggcggctcacggcgcggctggtgcctacgccatagacgaagggctcgcccacgatggccggcaacgattggcccgcggcggcaacagcccgccgcgcctgcagttgcgtacgcgtttcgctggcgggaatcgcagtgccgctgtcgtacacgccgtacaggctctgcgcgccgcggctggcccggcccatgtcttcggcgctcacgaacttgccggtaccgaacagcacgatggcgccgccgttcggccccaccccgacttcgggcgccacggtgatgggctggcgcttcgcgtttgcgccgcccgatgtcgcgaccatcaatggaaggctgcccagcccgagtgcgttggcttcgctccacggcgcattgcccgtgaagtcgaacttccagaggttgccttgcgtgtcgccggcgtacagccagcgtgcccagccgtccgccgcggcaaagtcgccgggtgttgccaaggcattcacgagcgtgctgtctgccggtgcgggcagcatgatcttgtgatagttgaggccccgcttccatgcagcaccggccggtttgtcgagcgagagcaggaacagcgcgctccgcttctcaatatttgcgttgttgaacccggagggaacaaccgcgaaccaggcgtacgccgcgggctgggtgcgagtcgctgcggacacacggaacttcatgatgcgcggcgcctggagcacatggcccatgtcgccatcgtccgcgccggtgaactcccacaagaccttgtccgccgaaaaggcggcagggtcggaaatgtcgagcgcaaaaacgccggcagcccctgcccccgtgccggagaccagcaccgtcttccaggcaccgctggccattcgcgcctctaccgccgcggccgagccgtcgacatgggcctggtgcgcatagccgggcgaggtgtagccggccagcttcgaagacaccgagcggggaacataggcgaaaagctcgttgcccgtggcggccgagaatgcatgcagcatgccgtcgttggcgccgacgtacacggcctgcggccttgccttgtgagcatcgagaaactgttggtacccggcgcctcgcacgttcgggctcggagggccgacgaagagcgggttcgaattggcaacgtcgcccatcaccgaatcgcgcacgcggaaggtcccacctggcgcagaaagctccttgcgccggtcgccgcgcaggtaggccagccgctcggcgcccaggccatcggttgctgctggcacggcatagggctcggcgttcaaggcgctttgcagcgccttgtccagtgcgttccactgaaaaggcgcgccgacgccggcagccgagagggtgaagatgcttcggtccgccggctcgcgcgcaggcactgcaggttgggccgatgcatcgccggtcagcaaggctcccgcgtcccagctgggctcctcggcctggcgaacggtgcccgagcctgcgtcgtaggccagtggatacgccagcaacgttcccgaccatctgcgcccgctgaaccgggccacgtaaagactggcgcccgtcgctccgatgcggttcgaagagattgccgcgtccgccgtgcttccgcccgatggcgcggccgccgactggaacaccttgcggattgcggccagtagctggtgcggctcgccggcgaggaagtagttggacggcttcggctggccgtcgtcgtcgaggccttcggcccattcggcattgctgcccacgtccgcccggccaccgccacccgatgcgacgaacggattgccgtcgccgttgctgtccacgaagccaccgtatttggacgcgaggtacagggcgctgccacgctggccctgccgaatggcgccctgcccgctcgcatccagatcgatgccgaaggtctggactcgggcctcggaaaaatcggcgcggatcttctgcgtattggcccagtaggccagacccgccatgccgaacgagcccctttctgtgcctgtttccgcgccggcgatggtgcccgacgtcagttgcgcgccgcccttgtagttgaaggccggaaggcctcggttgccggtggtggcaaggccggtcctctccgaaggatgcgcataggaaaacgcttcgcggttttcgaacgcaccgacgagtcgtgtccagtaggcggtgtccggctcgaacgacgcgctgctgaagccgcggccgccgccgggcatgcctggcaaggaatggtcgtcgtgcgtatcgagatcaccgatcgccaggatgtggttcttgcggcagctggccgccaccgggtcccagctgctcttgcggctttcatcgcgccatgcggccgtgtcgttggagaccggcagcccgtccttgcggggatcgttcgttgcgaccacgcccgccagggcttccggcgtcggagccttggcctgcaggtagcgcagcgactcgtagtagagctcgcccgcagggtcgaacttcttgtaggcgccgccgcgcccgaaccggttcaggtagttgacgatgccgctgtatcggccaccctgcgcagccgcatcgggatcgtcgatgaagacgccagtcgtcgcgttccactcggcccgggggttgtccacgctgtcgaggccggcgtcgagcttccgaggccccgtgtatttcatcggcgcgcgcagcacgccgccgtagcgcgccgggtcgttgtccagcaggtagccgaaaacggcgaagcgcatgcgactcgaatggcgctggatttcgcccacgggcttgaattggccgcccgggtatttgaggcagagatcgatgcgcgtcgcggcctctgccgccgtgcaaacctcgacccgcgcaaagtaaggtgcactcgcagcgcccgggccatattgctggtcggtaccggggcttgcgcaaccgccgctggcgctcggcccgacgaacatgcggtcgagacaatggttgaagtgaacagtgcctgccgcgcgaacgcccgtgcggctgtccgcgacgagcggcgtgagcttgtccaggttgcccgtcacggccttgtcgggaaagtagctgctgcgatagaaatcttcttgcagcaccgcgcgctgcagcacggtgcggccggcttcgtccaccacgcggtctccgcctgtcaaggcgagtcgcagcacgtcgatggtggagatggccgcccagttcagcaaattgccgctccactgattggcgcatgcaatttcgccgtcggcgagcttcaccgcaggtgcaaggcgcctgaaataaccatcggccgccgcatagccgtagcaggccatcggatcccaatagccgcggtagaccttcttccagtcgaagctgccgcgatacgccgcaccggcgttcgagaactccagcgcgagatcgagcaccaggttcggatcggcgcgcgatgccatggaagacagcggttcgcccggaaactcgacctgctccgccgccaaagcgcatggagcgttgcaaagggccaaggccgcaacgaccgcagccgcgatgccgcagctttcaagagaacgcattcgggttccgtttcaagatgaagaactcaggaagggcagcccgggctcgcgcccgacttgtacaaattggtctgcagcaccacttgcgtgtcctcttgcatgccgtagccgatggccgtgacgcgaaagagatgcgaggcattgcgcgcactcgcgctctgcaactggcccgactgccagccgccgagattgcgaaccgcctcgacgatgtagcgcggcgcgcgcgcgggcaatgtcccggcgcgtacgtccgcagccccgtcgccagcggcataggcttgtccggtgaaggtgccgtagacgacggatgtcgtgctgtcggcagcgaagtcggcggtcatccacgctggcttgtcgccggactcggccggcgcgcacagcccttggcgcatgcccgcgccaccgcatccgggaacgaaggccgagatatcgctgccgctgaaaagacagaggcgctgggccgcgctggaattggggccgagcacgtctcgttcggcgtcgacgagcgcggcttccgcggcctggaacgcaacctcggtgtcgcggtcgttgcgcgcgcttcgctcgcccaccagcgaaacctgtgccgcaccgatgcccagcaccatcgcaatgaccagcatcaacagcaccacgatcaacgagaagcctcgttgcgacaagcgatccgtccggctcatggcgccggctccttcatgacgttgcgcagcatgacggtgaaggtcgaggtgcgacgcagcctgccatcggccgggggcttgaaactcgtgcctgaaaactccgcgcccaaggggtagagcgtctcgccctgcagacgcggcccactgttgttgcggccacttcgcgcgaccatgccgatgcgaagaccgacgaccttgcgccattcggcgttgatggcggcaaccgatcttgcctgcgcttccagttgcgcggcgtcgagccagcgctcgggcacgccatcgccgttgacgtcgtaggcatagacgaccttgaacacttcgatgccgcgcgcgagcggctcggacttgaacgtgtccaccgtttcgctgtggtacttgcaatagagctcgggctccttgtcggccgcttcggcgacgtgaaagaagctccacgcacgatcggcaagcgccggcttcccggcagacggcccggcctgcgcgatccccatgcagtcgaccatggtgccgtcgggctcggtgccgtcgcctccagtgcggctgcggccgaagaagcgcacgcgaagcgagtcgcttccgttcacgcccttgctgttgtgggtgccgtggctttcgccggcagcgctgaccttggcattgctcgcgccgacgatgtcgaggtcggacggatcgtccggagatgccgccagattggcgctgctggcaatgaccacggtgccgtccgcggcggcgtgatcgggcgcgtagtcggaatatccggcctggcgcacgatgccccggacgacgaaacctgcgaacctcagcgaatcttccaccgcctgcgcttccgcgttggcaacgaagagctgcttgctgccgaggaaggttgcagtcgccgcaagcacgacgaggagtccgacagccatcgcgaccagcagctcgacgagcgacatgcctcggtggccgcccagccgcgcggtatcaggacccgtcatgaccatcctgtgcccagccggagaccagctgcatcacgaggcgaggtggaagctctcgttgcggttcgcccttttgcttgccgattgattcattcgcgtgcgatgcccagccgagctttgcgatcaggctgcggccgctctggctgcatctccaggcaaattcgccggccgccgcgttccagggtttgtcgtcgaagcacacgcgcacccggacgccaggcaacgccttggcgactcggcgtgtccattcatcgacgtcccacgcggccaggcccgctgcgtcgcaggtcgcgcccggcgccgcacagccgccggtcgcggggctcacggcggcgctatccgccgagtgctcgaccaggtaggtgttggccgcaccgttgcctgccgcgacacccggattcatgcgaaccttctcggacaggtcgcgcacgagcccgaccgccgcgttgaacgtagcggcctccttgcccgcgcgcaccgcagccagcagcatgccgaccgcgccgagcaggccaatgctcagcaccgcgaccgaaacgagcacctccacgagcgagaagcccgcaccggaccgccttggggtcgtcatttgtcgatgtcctcccgtcttgcaacttgtgttgcttctttattcgcgccatcgaatccgcagcgtaggcgtcgccttcggcagtgcatttgccgttcgtccgcttttgactgccgctcgtatgatccggcggctccggtgttaattaattcctcctctcgcagcccatgccctcccccgaacaagaagcacaagacgcgcagcacatggccaccgctttgcggctggcttccgccgcgctgttgctgaccgaccccaacccgcgcgtcggctgcgtgctgtgcgacgcagcgggccgcgtgctgggccagggccatacgcagcaggccggtgggccgcatgccgaagtgatggcgctgcgcgatgcggcggccaagggaaatgaggtcaagggcgccaccgcgtacgtcacgctcgagccctgctcgcaccacgggcgcaccggcccctgctgcgacgccctcgtcgcggccggcatcggccgggtcgtggcatcgctggccgatccgaatccgctggtggcgggccaaggcttcgcccgcctgcgtgcggccggcgtccaggtggaaaccggccccggcgccgccgagtcgcgcgagctcaacatcggtttcttcagccgcatggtccgcaagctgccctgggtgcgcctcaaggtggcggcctcgctcgacggcaagaccggcctggccaatggcgtgagccaatggatcaccgccgaagccgcccgcgccgacggccacgcctggcgcgcccgtgccagcgcggtactgacgggcgtgggcaccgtgctcgaagacaacccccgcctcgacgtgcgcctggtcgacacgccgcgtcagccgcaccttgtggtggtcgacagccatctgcagacgccgccagatgctcatgttttcatagcaggccggccggtctggatctatgccgcagtgcgcgacgaagcccgcgccaaggcgctggaagcacggggcgccacgatcacctgcctgcccaacgcaagcggaaaggtcgacctggccgccatgctgcacgacctggctcagcgcggggtcaacgagcttcacgtcgaagccggccacaagctcaatggctcgctgattcgcgaaggctgcgtcgacgaactgctggtgtatctggcacccaagctgatcggcagcggcctcgacatggcgagccacctgcatgccgagggtccgctcacctcgctggcgggcgcgctgccgctcgaattcaagtcggtggagatgcttggaccggatctccggatcgtgtcgcgggtgagcggacgcgacaacttctaagcgccttgcactttcaggggcggatcacatcggctcaaagcaccgcgaaaagccggggggctcacgcatctgcgaaaatgtgcgaatgttcaccggaatcattaccggcgtggggcgcatcgccgccatccacgacctcggcccctcctcctcctcctacggcaaaagactcggcatttcggtgcccgacgggtatctcgacgatgtcgggctcggcgacagcatcgcgctcaacggcgcctgcatgaccgtcaccaccctcgatccggcgcagcagcagttcaccatcgacatttccgccgaatccctcgacaagaccgcgggcctcaccgaagacggcgcccgcatcaacctcgagaaggcgctgcgcgccagcgaccggctgggcggccacatcgtctcgggccatgtggacggcatcggcacggtgagccactttgcgcccgtcggcgaaagctgggagctgcgcgtgctggcgccgcccgctctggcgcgctttctggcgtacaagggctccatcacgatcaacggcgtgagcctgaccgtcaacagcgtgtccgacaacacaggcggcagcgagatcagcatcaacctgattccgcacaccgtcgagaacacttcgctgggcgacctgaaggcgggctcccaggtcaacctcgaaatcgataccgtggcgcgctacgtggagcgcatgcttcaggccggcgttcttgcgcccgcatccatggcctccacgcaatctgcgcaatccacgtattccaaggacactgccgaatgaacgcttccgtcacgcccatcggcgcgccccgcagctcgcgggccccggcgccgatttcctccgtcgaggagatcgtggccgagctcgccgccggccgcatggtgatcctggtcgatgaagaagaccgcgagaacgaaggcgacatcgtcatcgcggccgaccacatcacgcccgacgccatcaacttcatggcgcgccatgcgcgcggactgatctgcctcacgctctcgcgcgaaatgtgcgagcggctgcagctgccgcccatggtgtcccgcaacggcgccaagcactcgaccgccttcaccgtttcgatcgaagcggccgagggcgtgaccaccggcatctcggccgccgaccgcgcgcgcaccgtgcaggcggccgtggcgcgcaacgccgtggccagcgacctggtgcagcccggccacatctttccgctgcaggcggtggacggcggcgtgctcatgcgcgccggccataccgaagccggctgcgacctcgcggccatggccggctgctcgcccgcctcggtgatctgcgaggtgatgaacgaagacggcaccatggcgcgcctgcccgacctgcagatctttgcggccgagcacgggctcaagatcggcaccattgccgcgctcatcgagcaccgcagtcgcaccgaatcgctggtcgagaaggtcggctgccgcgaaatccagaccgcttggggcaccttcaccgcccacgccttcacagacaagccgagccgcggcgtgcaccttgcactggtgcgcggcaagtgggcgcccgaagacacggtgtcggtgcgcgtgcacgagccgctctcggtgctcgacgcgctggagatcaaccgctcgctgcactcgtggagcctggatgccagcctggcgcacatcgcgaacgaaggcaagggcgtggccgtgctgctcaattgcggcgaaacggccggcgagctgcttgcgcagttcgacggcaccgcgcgccccgcgcaagcccccgagcgcggccgcatggacctgcgcagctacggcatcggcgcgcaaattctgcgcgaatgcggcgtgcacaagatgaacctgctcggcacgccccgccgcatgccgagcatggccgcaggctacggcctcgaaattgccggctacctcacgaaagactgacacgacatgcaaggtgcaaacaagggcgcggatgcaaagccgctcgacggaaaagggctgcgcatcggcatcgtgcaagcgcgcttcaacgccgacatcaccgatgcgctggccgcggcctgcctctccgagctcgagaagctgggcgtggccgcggacgacatccatcatgtgcaggttcccggcgcgctcgaagtgcccgtggccctgcaggcgatggccgtgcgcggcggctaccacgcgctggtggcgctgggctgcatcatccgcggcgaaacctaccacttcgaactggtggccaacgaatcgggcgcaagcgtgagccgcgttgcactcgaccaccgccttcccatcgccaacgcgatcctcacgaccgaaaacatggagcaagccattgcccggcagaccgacaagggccgcgatgcggcccaggtggctgtcgagatggcgcaattgctggcctccctcaaatgaccgaagacaacaacaagacaacaggcgccaagccgcgccaggcgcgcaccggactcaccagcaccggcgcgcgcaaggcttcggccaagtccaaccgcagccgcgcgcgcgagttcgcgctgcaggcgctctaccagcacctggtgggccgcaacgacccgaccgagatcgatcacttcacgcgcgacctcgcgggctttcacaaggccgacgccgcgcactacgacgcgctgctgcatggctccatcgaaggcgccgagcagctcgacgcgctgatccggccgctgctcgaccgcaagttcgaagagatctcgcccatcgagcatgcggtgatgtggatcggcgtgtatgagttccagcactgcctggacgtgccgtggcgcgtggtgctcaacgagtgcatcgagcttgccaaggaattcggcggcaccgacggccacaagtacgtgaacgccgtgctcaatggcctggcgcctcaactgcgcgctgccgaggtcgaggccgaccgggcctcgggcaaggccagaacgtgaagatttcggcgcgcgcacagcgcatcgaacccttctacgtgatggaggtcgccaaggccgccggcgtgctcgcgcgcgaggtggcccacaccgaccggccgatgatcttcctcaacatcggcgagcccgacttcaccgcgccgccgctggtgcaggaagccgccgcgcgcgccgtgcgtgccggcgccacgcagtacacccaggccaccggcctcgacctgctgcgcgagcgcatcagcggctggtatgcgcagcgcttcggcgtcgacgtgccggcccaccgcatcgtggtgaccgcgggggcttcggctgcattgcaactggcctgcctcgcactgatcgaatctggcgacgagatcctgctgcccgaccctagctacccttgcaaccgccacttcgtgagcgccgcggatggcaaggccgtgctgataccgaccacggccgaagagcgctttcagctcaccgccgccaaggtcgaggccgcctggaccgacaagacgcgtggcgtgctgctcgcctcgccctccaacccgaccggcacctcgatcgcgcccgatgagctgcgccgcatccacgaagtggtctcgcagcgcggcggcatcacgctgatcgacgagatctacctgggcctgtcgtacgacgaaaccttcggccagaccgcgctggccatcgacgacaacgtcatcagcatcaacagcttcagcaagtacttcaacatgaccggctggcggcttggctggctggtggtgcccgaagtgctggtgcccgtggtcgaacggctcgcgcagaacctcttcatctgcgcaagcaccgtgtcgcagtacgcggctctcgcctgcttcgaggccgagagcattgccgagtacgaacgccgccgcgccgagttcaaggcgcgccgcgactggttcattccgcagctcaacgcattgggcctcaacgtgcccgtggtgcccgacggtgccttctacgcctgggccgactgcaccggcgtggccgagaagctgggcatttcgggcagctgggatttcgccttcgaaaccatgaagcgggcccatgtggccgtcacgcccggccgcgatttcggcaccgccgagacagccaagttcgtgcgcttctccaccgccagttcgatggcgcacctgcaggaatccgtcgaacgcctgcgggccatgatcgcgaaccccgcccgatgagctacgcgtttccgatccgcgtctactgggaagacaccgacgccggcggcatcgtgttctacgccaactacctcaagttcatggaacgcggccgcaccgagtggctgcgctcgctgggcgtggagcagcgaaagctgcgcgaggaaaccggcggccagttcgtggtgagcgaaacgcagctcaaatatcatcgcccttcccgcctggacgacgaactgctggttacagccgaccttcaacaactgggcaccgcgtcgttgataatcggtcaacgcgtgctatcaaaaacagagcaagagcgaacaggagcctcagcgcctgtcctgctgtgcgaaggcacgatccgcatcggctgggtggatgcatccacgttgcgccccgcgcgcataccgagccaagtttcgggaaccctcgagcgctgcggcggctccatgactcaacctttcaagccatgaaccaagatctctccatcgtcaatctcctgctccatgcgagcttcgtggtgcaactggtcgtgctgctgctcgtgatcgtctcgatcgccagctgggccgcgatcatccgcaaatactttgccctgcgtcgcatgcgcgcgctcaacgacgacttcgagcgcgagttctggtcgggcaccagcctgaacgaactgtttgcctcggccgcgcagaacgccaagttcgcaggccccatggagcgcatcttcgcttcgggcatgcgcgagtatcaaaagctgcgcgagcgccacgtgagcgacgcccccaccttgctcgacggcgcccgccgcgccatgcgcgcgagcttccagcgcgaactcgacgctgcggagcagaacctctcgttcctcgccacggtcggctcggtgtcgccctacgtcggcctcttcggcacggtctgggggatcatgcatgccttcaccggcctggccgccctcgcgcaagtgacgctggccaccgtggcgcccggcattgccgaagcgctggtggccacagccatcggcctgttcgccgccattccagccgtggtgggctacaaccgctttgcgcgcgagatcgacaagatcgccattgccctggagacctacatcgaggagttctccaacatcctgcagcgcaacctctcggccaacccggccgcggtggcgtcggcaacttcgacggctccggccaaccgctgaacggaggtccagcgcatgcccgccgtttcatcccggggccgaggccgccgcacgatcaacgagatcaacatggtcccgttcatcgacgtgatgctggtgctgctgatcatcttcatggtcacggcgccgctcatcacgccgagcgtgatcaacctgccctcggtcgaccgcgccaacaagcagcccgacaagccgatcgagatcgtcatcaagagcgacgatgaagtgcagatcaagaaggacccgtccaccggcagcggcggcgcgtcgattcccatgacccagatcggctccgcagccaagaccgcccaggggggcgacgaccagcgccccgtggtcatcagcgccgacaagtccgtcaagtatgaaaccgtcgtgaaggcgatgaaccagctcaagcgcagcggcatcgagcgcgtgggcctgtccgtcaccaccacgggcggcaaataaggcatgtcgctcgccctggatcgtcccgagttcgcacccccaccgcagcgcggcacgccgcgcgcggtgatgctcgcactggtcgcgcatgcgctcctgatcgcggcgctgacgtggggagtgcgctggcgcagcgaggccgacgacggcgcggtggatgccgaactgtggtcttccacggtgcagcaggccgcgccgcgcctgtccgcaccggaggcgcccacgcccgcccccgcaccgccgccgcctgcgcccccaccaccgcccccgccgccgcaagtgaaggccccggagcccgcgccaccgccgcgcgcgcccgacatcgccctggagcgcgagaaaaagctcaaggaagaaaaagagcagaaggagcgcgagctcgagcgccagcaacagcagcgcaagaaagagctcgaggccaagcagcgcgccgaagacgaagccgagcgcaagaaggaacagcagaagaagctggccgagcagcagaagaagcagcaagaagccgaggccaagcaggccgaagcgaagaagcagcaggaagctgccgccaagcaggctgccgccgaccgcgccgccacgctcaagcgcatgcagggcctggcgggcgcgagcggcagcgacgattccaagggcacggccctgcgttcgtcggggccgtcgagcggctatgcgggccgcattgccgcagcggtgcggccgaacatcaccttccccgatgcggagacggtgaacggcaacccagccgccgagttcgaggtgaatctcgcgccggacggcaccatcgtcggcgtcaagctcaccaagtcgagtggattgccaagctgggacgaagccgccgaacgcggcctgcacaagaccgacaagctgccacgcgacaccgacgggcgcatctttccgtcgctgatcgtctctctgcggcccaagcgctgatacagcatgacggttccgggtggccttttcacgaggccgcccggaactccgttgctgtcgcgctggatggcgttcggaccgcagccgctcgtttaggatcgtcggcaactcattgcctggcgctcctgacatggtcgaaaccactcccgccgttcgcctcgaagacctgaccccgctgccctaccagcaagcacttgccgcccatctgcaagcgaacgagcccgaggtctggcactgggctgcctcggctgaagcgcgcgaggagcatgccggggcagtgcgcgccgacctgctgcgcaattcgtaccggctcgatgccgacgcccatcccgatctgcacgcgcattgcaccgcggccgcgctgcgcttgggcatcacggcgcgcgtcacgctctaccaggcgggcgacggcacgatgaacgccacgctctacttcgtgcccggcgaggcgcacatcgtgctctcgggcccgctgctggaacgcctccaaggccccgaactgcaggccgtgctcggccatgaactcgcgcactacctgctgtgggagcgcgacggcggcaagtaccacgtggtcgaccgcatcctgcaggccgcggcggccgactcccgcgccgacgcgagccatctgcatgcggcgcgccgctacgggctctacaccgaggcttttgccgaccgcggtgcctgcatcgcctgcgaagcgctcgaacccgcggtcaccgcgctcgtcaaggtgcagaccggcctcgcgcaggtcaatgcggcaagctacctgcggcaggccgacgagatctgcgccgagcccgaactccagacgcgcggtaccagtcaccccgaggtgttcgtgcgggcgcgggcgctgcgcctgtggaccgagcgccagcccgaagccgacgaatggctggcgggcgcgctcgaaggcccgctggacatcgccacgctcgacctgctcggccagcagcgcgccaatgcactgacgcgcgagaccatcgcccagttgctgcaacgcccgttcctgcactccgaatcgctgctggcccacgcgcgccgcttcttcccgaacttcgcgccgccctcggcgaccatgccgccgcccgcgccggtgccggctggcgtgcacgactacctggccagcgtgctggtcgatttcgtcgcggccgaccccgacctcgacgacatcacgctcgccgccgcgctcggtcttgccgaagccatgggctgcgccgaccagctcgaacagcgcgtcgtgaaagacatacgctttcccaagcgcagcctgacccgcgtgaagcgcgatgccgccaccctgcttgaaaaggcagcggcccaacatcttcagggcgcatccgcatgacgacacccgccacctctcccattcagcagctgctggacaccggcgaggcccacggtggcctgcagaccgacgacgtgctgagcctcgtgctgccgctgctgcgcgaggtgtccgccttgcacgagcaaggcaaggtcgccgcgctcggaagcgtattcgcctaccgtgtcgacgacacgcccgctctcgcgctcgcacagcccacaggcacagagccgcgccagaaccgcggagccatcgctcctctggaacagcccgccgcctccgtgctgcgcgtggtcggcgagcaccgcgtgacgctcgatgccgacgaaggcttgtcggtcgagaacctcgcggtcatgaccgacgccgcgcccgacgccctgccgacgcgccccgtgtacctgcccggctacaccgcatgggagttgcgcttcgggcaccatgacgcgctgaccgacatcctctgcctcggccaggtgctggccagcctctcgtgcgggctcgacttcaccgacaccgaagaactgggccgcttcgtcgcggaccgcggcaacctgttcgcactcaaccgccgtctgcacccggtggtggccgcggtgatcggcgagatgaccgcgctcgaccgccacgaacgcgcacgcgacctgccctcggtgatccgccggctagaaacctaccgcgaccagccgctggacctcggcctcgaccgcattgcgcccgcgagggacggcgcgggccagcgccgccaggcgatccgcctgcatctgcgcgaccgcctcttcgacctctcgcgacgcaaccgcctgctgcatttcaaacccagccagacgcacgtgaacctcacggtggcgagcgtgccgctggtggtcgacatcaagaacatccgcgtcgaccagctctgcgtgtgggacggccggtttgcgagcgacatcgccacctgcgaccccgtgccgctcgcgcgctggctgcgcttcgaagaccagccctacctaccgggcgcgctcgaccgcatcctgcaggaggcacggcgcgaccgctccgaatacggcttctcgcagctgtcgctggtgatcgccttcctgcgctggcacaacctgaaagaaggagagaccgagcgggccgagcgcatcgcctcgcccctcctgatgctgtcggtcgaactcacgcgcaagaagggagtgaaagaccagtacctgcttgaagccgcctcgagcgaagcccaggtcaacccgacgctgcggcaccacctgcgccagctctacggcatcgtgctgcccgagaccgtggatctgcgcgaaaccaccatcgagcagttccatgctcagctcgccgcacagatcgcggcgagcgagcccggcgtgcagctgcggctcgtgaagcagcccgagatcgaactgattcatcagcgtgcccgccagcggctcgaacagttcaagcgccgtgcccgcgtgcgcaaccccggtgcgcaacccgtcgcggcgcaggacttcagctacgcgcgcgacgacttccgcccgctcggccttcagctctttcacgcgaaggtgcggccggttccgctgccgttgcgcgatgcggtcggcgcgcggcccgtgccgcgcgcaccgcagatggggtccaccgccgcccagaccgagcgcgagacctttacgctgcgcgaaagcgctggcaacccctaccaatgggacgtcgacctcacctcggtgacgctcggcaacttcaaccatcgcaagatgtccctggtgcgcgactattcggcgctgagcgaaaccgaaatcgcgagcgaggccttcgaccgcgtgttctcgctgcagccgcgccaggtcgatgccgaaccgccggccgcgctgccgctggccgaccaatggcccgtggtgcaggccgacgccacgcagaccgccgccgtcgcgctggcgcgcaccggcaccagctacatcatccaggggccgcccggcacggggaagtcgcagaccatcaccaacctcatcgccgactacgtgggccgcggccagcgcgtgctcttcgtctgcgagaagcgcgccgccatcgacgtagtgttccaccggctgcggcagcaggggctggacgagctctgctgcatgatccacgactcgcagggcgacaagaaggccttcgtgcagaacctcaagaagacctacgagcactggctcgcagcgcccgaggagctggaggctgagacccgcgagcgcacgcaactcgtcgacaccatggacgccgacctgaaggcgctggagcggttcgacgccacgatgcgcgaagcacccgaacacctggccgtgacggtgcgtacgctgatggcacggctgatcgcgctcaagccgcacgacccggcgctcacgccgttgcaggccgaggccctgcccaccttcgcggcctggcgccgccatgccgacctgatcgcccgcctgcacctcgccgtgaccgaaagcctgggcgtgccgtatcttgcgcagcatgccttcgcgcagctcgcgccggcgctgctgcggcaggagcggccgcttgcgcgattggtcgaactcagcgaccgtgcggccgagcagatcggcccgcaccgcgatgcactcatcgaagcctggccgccgctcgccgacgcccgcgtcctctggggcgacgcactggccgtggtggccgacgcacgccgcgtggccgcactcgctgcgcgcgggcatctctcactgctcgacaccgcacaccccaccagcctcgctttcggcgaggcaatggcgcagcgccgtgcgttgcagcaggtgctcaaggaagccctcgaacgcacgatccactggcacgacaagttctcgccgggcgacaccgaagccggcctcgctcaggccgaggcgcaacaaggctccttgctgcgctggctccagccctcgtggtggcggctgtcgggcgagctcaagcgccgctatgacttcgccaagcacgcagtccgcccgcagcccagccaggtgctcgaggaactgctggccgagcacacggcccgcgcggccgtcggcaagcaggcggcgcagatcgaagccacctacggctgcaccgaccctgacgatttcctgcagcagctcgacgcgttgcgccgcggcgacggcaccggcaacggcgtgcgcgcagccttccatgcgcacctgcgcaccgaacccggcgcgagccgcaacgtcgaacgactggccgccctcgggcagcgcacggacgcgctcgatgccctgtggcacgaactgctggccgaccctgccgcccagccgctggcgtcgctcgaagcgctggcccgcacgatgcgcgagcaggccgacaccctgcccaccgtgctgccccacctgcaggaactggccgatgccgaccccgccctggccaaggccctgcgcacgctgccgctcttgccagacgccatcgaatacgccgtggcccgcgaaggcctggaacgcgtctaccgcaccgagcgctggctgccgcgcttcgacagcgccgcgctcgcccgccatgcccagcgcctcgccgaaggagagcgcaagctgctcgaccgcaacgcccgcacccttgccgccgcggtgcgccagcgctttcgcgaccatttgcaaaagagcgccctgcccgcaagccagctcgacgctggcggcaagctcttcaagaaaagctacaacgcgggccggcgcgaactcgaacacgagttcggcaagaccatgcgctacaaggccatccgcgaactcgcctccggcgacaccgggcaggtggtgcgcgacatgaaaccgatctggctcatgagcccgctctcggtgtcggacacgctgccgctcgccgccgatctgttcgacgtggtgatcttcgacgaggcgagccagattccggtggaagaagccgtgcccgcgctctaccgcgcgccgcagatcatcgtggtgggcgacgagatgcagctcccgccgacgagcttcttctcctcaggccgcgatccggaggacgacacggtgtcggtcgaggatgagggcgaccgcatcgccgtggtgctcgatgccgacagcctgttgaaccagggcgcgcgcaacctgccggccaccctgctcgcctggcactatcgcagccgctacgagtcgctgatcggcttttcgaacgcagccttctacgcgggcaacctgttcaccattccggaccgcagcctgcccgcggccgcgcgcgacgagatcctcgtgcagtcgcgcaacccgacggacgaatcggtggccgcacaggtcgatgccctgctctctcgcgccatcagcttccaccgcgtgaccgatgcggtctatgaaaaccgcatcaacgacggcgaggcacgccacattgcgcaactggtgcgcgaactgctgaagcgcgagaccgggcgcagcctcggcatcgtcgcgttctcggaagcgcagcagaccgaaatcgaggccgagctcgacgcgctgggcgccaccgatagcgacttcgccgcgcggctcgaggccgagtacgtgcgcgaggaagacgaccagttctacggtctcttcatcaagaacctggagaacgtgcagggcgacgagcgcgacatcatcatcctgagcatctgctacggcccgaaccccgagggccgcatgctgatgaatttcggtccaatcaaccagcgcggcggagaaaagcggctgaacgtgatcttcagccgcgcacggcatcacatggcggtcgtctcgaccattcgccacgaggcgatcaccaacgatcacaacgaaggcgccgcggctctcaagcagttcctgcgctatgcggagtgcctgtcgcgtggcgactcgtccaccgcgcggcgcgtgctcgaaggcatgaacccactcacgcgggccggcagcgcgccgcatgcgcgtgccgacgaggtgacagcgcagctcgcggccgcgctgcgtgcgcgtggccacgaaatcgatgaacaggtgggccagtcgcgcttccgctgcgaccttgcgctacgcgcgcccgaggccggccactatgcactgggcatcctcgtggacaccgccacgcattacgagaaccgcgacgtgctcgaacgctacgtctcgcgtccgcgcgtgctcgatgcgttcggctggcaggtggtgcaggtgctcgccaaggattggctgcatgcgccggagaccgtgctcgaacaaatcgaactggctctgcgcaagaagggagacaaggcgggcgaactcgccgccgccactgcggccagcgcaccaggcacagccgcttgaggtcgagttcggcctgcgagcgcgcgcgagtgctacgcaaccgcgcgccttgcttgcctcttactcgtaaaccaccgaagcttttccagcttccgcctgcgccgtccagctcgcgagcgctgcgtcggtcgggaagaacttggcgcgctcgccaagttgcagttcgacctgcgcaccaccacgcgccatcgagagacgcaccggtagcccctgcaccaggtcgccatgctcgctctgctcggtgcgcggcggaaagtctttcaccaggcgggcgatgtcgggcgccttgccgttcacggccacgcgcaggaacttgccgaagcggcagcgcgcggtggccaggtcccacacctgctgcacctgaaagcgtgcctcgaaaccgccgcgccccggctgcagccggccgctcacgatcaccagttcgtcgtccttcaaggtgttgcggttcgcgttgatcagcgcctcgtcagcggtcgcgtcgatcgagtccgacttgtcgtcgagcttgaagatcgcgaggcgcccgcgctggccgttgatcacgcggaagtcgctcacgatgcccgcaatcacctgctgctcgcgggtgtccatcaggtcgccgatctcgcgcttgcagaagcgccgcacctcgtgcgagacctcgtcgaacaagtggcccgagagatagaagcccacggccgttttctcgtaggtgagccgctccttcacgccccagggcgtcgcatccaccagttcgggctcctgcgtggccgagccgtgctcgctgtcgccgaagatgtcgacctgcgcggcattggcctcggtggccgacgcgaactcgaaggcgcggtcgaccgaagcgatcagcgacgcgcggttctgctggatcgcgtcgaaggcgccggccttgatgagcgcttcgaccgttcgcttgttgatgcgctggcgatcgatgcgcacgcaaaaatcgaacagactcttgaacgggccgccttcttcgcgcgcccgcacgatggcctcgaccgccagctggcccgtgcccttgacggcgcccaggccgtagcggatcaccttgtcggtgacgggctcgaagcggtagttgccgcggttcacgtccggcggctcgaaggtgatgccgaagtttttctgcgcatcctcgaacaacaccttgagcttgtcggtgtcgtccatttccacggtcatgttggcgcagaagaactcggccgtgtaatggactttgagccaacccgtgtggtacgccagcagcgaatacgcggcggcatgcgacttgttgaagccatagcccgcgaacttctccatcaagtcgaagatctcgtcggccttgtcttgcggaatgccgtgcgtcgacagtgcgcccgcgcggaatttctcgcggtgctcggccatctcctcgagcttcttcttgcccattgcgcggcgcagcaggtcggcgccgccaagcgagtagccgcccaggatctgcgcggtctgcatcacctgctcctggtagaccatgatcccgtaggtctcggacagcatttcggccacggccgggtgcggatactccacctcttcgcggccgtgcttgcgcgccacgaagctcggaatcaggtccatcgggcccggacggtacagcgcgttgagcgcaatcaggtcttccaggcgcgtgggccgcgcgtccttcagcatgccctgcatgccgcggctttcaaactggaacaccgcttccgtcttgccctcggaaaacagcttgtaggtttcgcggtcgtccagcttgatgttctcgtacgcgaagttctcctggcccttatggcgcttgacgatgaactctttcgcgatctcgaggatggtgagcgtggcgaggcccagaaagtcgaacttcacgaggccgatggcctccacgtcgtccttgtcgtactggctcacggccgagtcgctgccgggttgctggtagagcgggcaaaaatcggtgagcttgccgggcgcgatcagcaccccgcccgcgtgcatgccgatgttgcgggtcatgccttcgagcttttgcgccagctcgaccagcatgcgcacttcttcttccttctcgatgcgcgccgcaagctgcggctccatctcgatggcgtagttgttcttgtcgccctccaccttcgggtccggcggatactggatcgtgacgggctggcccggcttgttcggaatgagcttgctgatgccgtcgcagaacatgtagctcatgtccagcacgcgccccacgtcgcggatggcggcgcgcgcggccatcgttccgaaggtggcaatctggctcaccgcgtcgcggccgtacttgtccttcacgtagtcgatcacgcggtcgcggttgccctggcaaaagtcgatgtcgaagtcgggcatcgagacgcgctcgggattcaggaaacgttcgaacagcagcttgtattcgagcggatcgaggtcggtgatcttcagcgcataggccaccagcgagcccgcgcccgaaccgcggcccgggcccaccgggcagccgttgttcttggcccacttgatgaagtcgcccacgatcaggaagtagccggggaagcccatgttcaggatcgtgttgatctcgaactcgaggcgctccacgtagcgtgggcgctcggcatcacgcttggcgacgtcggggtaaagatgcgcaagacgcgcttccaggccttcaaacgactcctggcggaaaaactcgtcgatcggcatgcgaacgccttcgctgacgaaaggcgtcgggaagtcgggcagctgcggcttgccgagcaccagcgtcaggttgcagcgcttggcgatctcgaccgtgttggccagcgcgctcggcacgtcggcaaagagcgcttccatctcggcgctcgacttgaaatactgctcttcggtgaacttgcgcacgcggcgcgggttgccgaggatttcgccttccgagatgcagacgcgcgcctcgtgcgcctcatagtcctggcgctcggcaaactgcaccggatgcgtggcgaccaccggcaggcgcagccgggccgcgagcttcacggcggcaatcacatgcggctcgtcctcggggcggcccgcgcgctgcagctcgatgtagaagcggtgcgggaacatgcctgccagctgcagcgccagttcggcggcgcgctcctcctgcccctgcaacagcggcgcgcccagcgggccggcctgcgcgcccgaaagcgcgatgagcccgccctgcagttcctcgagccattcgagcttgcaggccgcctgcgactggccccggcccacgttctgcgtccaggcacgggccagcagctccgacaggtgaagatagccctcggtgttctgcaccagcagcacgatgcgcgtgagcacgccgggctccttgcccagtccctcgatgaaaatctcggcaccgatgactggcttgacgcccttgccccgcccctctttgtagaacttgaccgcgccgaacaggttgttcaggtcggtgatggcgagcgcgggctgcttgtcggcagcggccgccttgaccacttcgtcgattcggttggtgccgtcgacgacggaaaactcggtgtgcaggcgcaggtgaacaaacatcctctcattgtagaaagccgcactccacgatgtgggttgacgatccctacaattgcgccccgtgcaagagattttgaatattgcggcttacaaattcgtagccatcgacgacagccccgtgctgcgtgaagacctgcgcgagcgcgcccaggccctgggcctcatgggaaccatcctgctcgccccggaggggatcaacctgttcctggcgggcctgcccgacgccatccgcagctttgtagcgagcctgcgcgccgatgcgcgcttcgccgaccttgaaaccaaggaaagctggtccgccgcgcagcctttccgtcgcatgctggtgaagctcaagcgcgagatcatccgcatggaccacccggctatccagccgtccgctgggcgagcgccgggcgtggacgcccccaccctcaagcgctggctcgaccaggggcacgacgacgaaggccgcgaaatcgcgctgctcgacacgcgcaatgccttcgaggtcgacgaaggcaccttcgacggtgcgatcgactggcgcatcaataaattcaccgaattcccgcccgcgctgaaggcgcatcgcgccgactttgaaggcaagacggtcgtgagcttctgcaccggcggcatccgctgcgagaaggcggccatcctgatgcgcgaagaaggcgtcgagaacgtgctgcagctcgaaggcggcatcctgaaatatttcgaagaggtcggcggtgcgcactaccacggcgactgcttcgtgttcgacggccggcgcgcgctggcgcccgacctgagcgcacgcgcggccgatgccagcgcacgcgcctcggaagacatcgacctcagtagcggcctgaagaaatagccggcgggttgcccgccacgcgctctggagatcagaccggcgtggtgcccacgtcaggctcgcgcatcccaaatggcttgcccggcagcggaatgaattcggtctctcccggcacatggcccatgcgctgtgcggcccagtcggagccggcttcgaggatgcgatcgcgtcggctcgaaacaaaattccaggtgatgtagcgcgggccatcgagcggctcgccgccgatcaccatcaggcgtaccgcggtggtcgagctgagcaccgcgccctggccgtccggcagcaccgccattgtgtgcacgggaatcggctcgccgttgacgctcgcatcggcatcgacggcatagaccgcgagctcgggcgccagcgcgggcaattcgaaacgcccacccgcgggcagcgcgatgtcgagatagatcgtctgcgacagcgtcttgaccggcgagcgctttccgaaagcctcgcccaccagcacccgcaccgccacgccctgctccaccagttcgggaatgtcactggccggcgtgtgctcgaagctgggatcggtttcttcgtgcgcctgcggcaaggcagcccagagctgcaggccgtgattgacgtaggtgtcggccttgaggcgttcgggcttgcgctcggagtgcacgatgccgcggcccgccgtcatccagttgatggcgccgggcaggatctcctgcacgctgccaaggctgtcgcgatgcatcatcgcgccttcgaaaaggtaggtgacggtggaaaggccgatgtgcggatgcggccgcacgtcgtgctgggcgccgggctgctctgtggccgggccgaagtggtcgaagaagacgaagggcccgaccgaacggcggttcgcggccggcagcaggcgccgtaccttgaagccaccgcccaggtccttgtcgtgcggttgaagcagttgggtctgtgcggtggtgtcggtcatcgtgcgctccgtgaatggctgggttctatccgcgcgatcttgccaccgccgcaatgcgctcgccgaaagcgcgtgcggtgtcgaggtcgcccttgaacatctcggcggggctcgcgtccgaaggcgattgcgtcagcaggccgccgtagccgcccacgtagttcatcgaatcgcgcgaggccgccttgttgttggtcggcaggatgcccatgctgacccagaggccgctgtgctgcatcgcaagcgtccacaggtaggcgatggtcgccaccttgtcgccgttcatcgtggcgctgttggtgaagcccgcgaagagcttgtccttccagccctgcgtgtaccagaccttggacgaggcatcggcaaatttcttgaactgccagctcacgccgcccatgtaggtcggcgagccgaagatgatcgcgtcggccgcggccagcgtctcccagccgccttcgggcaggttgccatcggcatcgatagcgagcagctgcgcgtccgcgctatcggccacggcttgcgccacgcgctgggtgtggccgtaaccggaatggaagacgacgacgatgtttgccattgggtgattctcctgggtggacgcgatggtcattgatgcgaagccttggggatcagcttacttcttgtcgatgctgaagcggccggcaccaaaggccacgaaagcgagcaggccaccggtaacggcaatgttcttgaagaacatcagctggttcacgaaggccttgtcggcgggcatgctccagtagttgtggaacagcaccgacgccaccacggtgaagattgccagcaccacggccgcgaagcgcgtcttgaagccgacgagcagcatcaggccaaggccgagttccacgatgatggcaatgaccgccgcaacctgcggcagcggtgcgccaacggacgagatatacccgaccgtcccggcaaagcccatgagcttgctgaagcctgccggcacgaacaagagtgccagcaggacgcggccgacgagggacagagtgtcctgtgccacattgggggtggtggctgcggctgcgttgaatgtggtggttgccatgatgaagtaactccttggttgtcgattgattgaaagaaaagaacgggaaagcaagacagatgccgggcggcgcgcgcccggcgcgggaatcaggcggccagatcgaacaccagcacttcggcgtccttgccggcgcccagcgtgagttgcgattcgccttcgagcattgcggcatcgccgcccgcgagcttctggccattgacttcgagctcgccgcgcaccaggtgcacgtagctcttgcgcttcgggtcgagcgccaggctggccttttcgtcgccgtcgataaggcccgcgaacaggcgcgcatcggcatgcaccgtcaccgaaccgtcggcgccgtcgggcgaggccaccaggcgcagcttgccgcgcttctcgtcggtgccgaacttcttctgctcgtagccgggcgcaatgccgcgcacgttcggctcgatccagatctgcaggaagtgcgtggtctcgtcggccttgtggttgaactcgctgtgcatcacgccgcggcccgcgctcatgcgctgcacgtcgcccggcggaatcgcttccacgttgcccatgctgtccttgtgcgccagttcgcccgacagcacgtagctgatgatttccatgtccttgtggccatgggtgccgaagccggcgcccgcggccacgcggtcttcgttgattacccgcagattgccgaaacccatgtgggccgggtcgtagtaaccggcgaaagaaaagctgtggaacgagcgcagccagccatggtcggcataaccgcgttcctgtgatttacggacttgcaacatcgtcgaactccttcggcccattccccgagggggatgctcgggccttcttcgtatgccgcgccggatgcgcagcggatgtgaagaactttaggcccgcacccctgctttgaaagcgccggggtttgatggcatcattcaaattttttgatcaatcgatcgacccatcatggagccacgatgcccagcgccagagacgtactgacccccgacgcgctcgccatgctgcagaccgtggccagcacgggcagctttgcgggcgcggcccgcgccctcaacctggtgcccagcgcgctcagctaccgcgtgcgccagatcgaggacgcgctcgacgttctgctgttcgaccgcagcgcgcgccaggcccgcatcaccgaggcgggtgccgaactgctgcgcgaggcggcccggctgctgggcgagattgacgcggtggccaaccgcgtgaagcgcgtggccaccggctgggagccgatgctcaccatcgcggtcgacagcgtgatcgcgcgcgatcccctgctcgacctggccaccgccttcttcgcgctcgatccgcccacgcggctcaagctgcgcgatgaaaccctgctcggcaccatcgaggctttgaccagcggcgaagccgacctggccatcggcgcggtgctggatgcggcgagcctcgccttcacggccacgggcatccgcagccggccgatcggcgagctgtgcttcgtctatgcggtggcgccgcatcatccgctggcgcggctgcccgagccattgaccgatgaagtgctgcgccaacaccgcgcggttgcggccgcagactcggtgcgcagcgggccgagcatgacggtcaacctcgtcggcgggcaggacgtgctcacggtgccgagcatgcatgccaagctgagtgcgcagctgcacggcctgggcggcggttttctgcccgagccgatggcacggccgtatatcgaggccggccacctggtcgaacgcaagaccgaacgccgccccccgctcgcgaccatgcactgcgcatggcgcgtgcgcagcgcgggcgggccgggccgcgcgctcgaatggtggctcgcgcaattcgaccacgaggccacgcggcgggcgctgctggagcggcaccgggggcgctgagcaccagccgcccgaaagcgcccttcgcagaccgttgtagagtccgaatacatccatcgtctcccctacacaagaaaagagtccctcatgaccactcgcgcaactgcaaaggcgaccgaccgccaccgaacacccaccgccccacgccactacgccgtcgtcggcgcgggcattgccggcgtggcctgcgcccgaaccctggtgcaggccggccacaaggtcacggtgttcgagcgcgaagccgcgcccggcgggcgcatggcaagcgtcgaaactgcctttggccgcttcgacagcggggcgcagtatttcaccgtgcgcgaccctcgttttgcgctggcactggaagccacgcccaatctctgccgcccatggagcgccaacctcgtacgtgtgctcgatgcgcatggccgcgtggccgaggcagccctgcccggccgcgaatcgcactgggtggcccagcccggcatggatgcactggtgagccactgggccgcaccgctcggcggcagcctggtgcccaacacgcaggtgacgcagatcgaacccgatgcgctcgatgccaagcgctggcagctgcgcaccgcgggccaggacgattcgcagcacgtgtactcgggcttcgacggcgtactgctggccgtgccgccttcgcgcacgcgcgtgctgctgggcgacggcaagctctccgcctccgtcagccagaagatcgagccggtgcgcatcgcgccgtgctggacgctgatgatcgccttcccccaggccaaccagcccaccatgtcgcacctgggcccgcaatggaatgccgcgcgcagcacccaccaccgcgtggcgtggctcgcgcgcgagtcgtccaagcccggccgcgaacgcatcgagcgctggacgctgcaggccagcgccgcgtggtcgcaggaacacctgcgcgacgatgccgcacgcgtccaggccaagctgctgcgtgccttcgccgagatcaccggtatccatgccgcgcccacgcatgccgaggcgcgctgctggaccgaagcccagacccaggttcccgtcggcaaaagccacctctgggacgccaaggcccgcatcggcgtggccggcgactggtgcaccgggcaccgcgtggaagacgcgttcctctcgggcctttcactggcgctggcagtgatctgattcaaggatgcgtgagaccggccgtttcgcgccctcgcccaccggcccgctgcatgccggctcgctggtggccgcgcttgcgagctggctcgacgtgcgcgcccgcggcccgcaggcgcgctggctgatccgcatcgaagacgccgacaccgaacgctgcctgcccggcatgggcgaacacgtgctccggcagttggccgactgcagcctgctgcccgacgaaacgccggtgtggcagacagagcgcaccgcccgctatgaagcggcgcttgccaggctgcaggctctcggcctcgcctacccctgcggctgctcgcgcaaggacatcgacgaggcgctggcgcgccttggccggccgcacacgcgccatggggagcgcgtctatcccggcacctgccgcaacggcctgcacggcaagcccgcgcgtgcctggcgctttgccaccgagaagttcgaatccgcccagccggcgctgccggacggtgaactctgctggaccgaccgccgcctcggccgccagtgccagcacgtcagccgcgaggtcggcgacttcgtgctgcgccgtgccgatggcccctgggcctaccagctcgcggtggtggtcgacgacgcggaacaggacgtgaccgacgtcgtgcgcggcgaagacctggccgacaacaccgcacgccagatcctgctgcagcgcgcactcggcctgcccacgcccagctacctgcacacgccgctggtccgcggcgccgacggcgacaagctctccaagcagaacggcgccacctccatcgataccggggcgcccgaggccgcgctggcctcgctcgacgccgcggcacgcgtgctcggcctgggcgccgcgcaaggcggctcatgcgccgcggcattggccggctgggtgcccgaatggcgcgatctctacaattcgcggccgtaatgacctcttccgacaccgtgccccacgaccttccacccggcgacgacgacgcgggcgacgacgacaacaaaccccacccgctgcaccgccgcctcaagagcttcgtgaagcgtgccggccgcaccaccgacggccaggcgcgcgcctttgccgagctcggcccgctgttcctcattccctacaagcccgaaccgctggacctcaccgccgcttttggcggccgggccgcgccgaccgtgctcgaaatcggtttcggcatgggcgaggccaccgcgcacatcgccacggtgatgcccgagaccaactttctctgctgcgaagtgcacgagcccggcgtaggcgcgctgctcaagcgcatcggcgagcagtcgatcaccaacatccgcatctgcgcgcacgatgcggtcgacgtgctcgaccacatgctgcagcccgattcgctggccggcgtgcacgtgttctttcccgatccgtggcacaagaagcgccacaacaaacggcggctgatccagcccgggttcgtgaaaaaactcgccgagcacctgcgcccgggcggctacatccattgcgccaccgactggcaaccctacgccgagcagatgctcgaggtgctgtcggctgaaccgctgctgcgcaactcggccgaaggctacgcgcccaagccggcctaccggccgctgaccaagttcgagaaccgcggcctcaagctgggccacggcgtctgggacctggtgtttcagcgcgcctgagcggcacccgctttttttcaggcagagacttcagggctttcggcccaaggcggcccgcagccttgtcgcgagctgctgcgcatgcgcggcggagccgatgttggtgaagcccatcagcagcccctcgtcgcgaaaagccgccgtgcctcgccgcgacagcggctggcagttcaggccggcaagctgcgcgcggtgggccagttcctcgtcgttttcgcaccaccggtcgaagcgtgcgatcaggtgcatgccgccgctctgcagatcgatgcgcacgtcctcgccaaaggccttctgcaaggcggccgcaaacacgctgcggcggcgcgcatagagcagccgcatcttcttgaggtgacgggagaagtggccttcgcgcatgaagtcggccaccaccgcctgcgtgagctgcgggcatccgttggaccacgtctgtgcggccacgccgaaggcgctcagcagcgagtcgggcgcgaccacgtagcccagcgccagccccgggtagagcaccttcgagaagctgcccgcatacagcacgcgatcatggccgtccaggctcttgagcgcgggcaacggcgggccggcgtagcggtactcgccgtcatagtcgtcctcgacgatccaggccttggcctcggaggcccagtcgagcagttgcagccggcgcgcgagcgacatcgacacacccagcggtgcctggtgcgaaggcgtgaccacggccatcttcgcttttgctgccttgcgcatgccatgcgcaacgtccatgccttcctggtccaccggcacggacaccgggcgctggccggcaccgcgcagcacctcgtgcgtgggcgtgtagcccgggtcttccacccacacacggtcgtccttcgcgagcagcgtgtgcgagatgagcgcgagagacgcgcggtagccgccggtcacgaagacctgcgacggatggcacgagacgccgcgcgacacccgcagataggcggcaatggcggtgcgcagcaccgggtggcccgaagggtcgccatagaacatgtcggccgcggtcgtcgccctcgcgcggcgcgcagccaggcgcgcccagagcttgcgcggaaacgcatcgagcgccggaatgcccagctgcaaaggcggcggcggagcaggctcggcaagcgcctggccggaggcttccgccccggttcttcgaggcccgcggcgcaccggccggcgggcggggagcgatggggaaaccaccgtgcccgcctggccctgcggcgagaaataaccttcacccgcaagctggctgtaggccgtctcgatggtgccccgcgccacgcccagttcgctcgccaggctgcgtgcagatgccacgcgatcgcccgggcgaagcacgcccagttcgatggccgccctgaagcgctcgtagacctgccggtacagcggcgcaggcgccgcgcggtcgattgccaggtgggcggtggaaaaggtcttctcttgaatcatggcccattcatttttgcgaatcttggctctttcgagtgtggcatcgaaaacctaagctcgaccggtcgaacagccagcaggacaaaggacatgcgatgagcgagaagatattcgtggcgggtgcggccggcgccatcggcagtgcgctggtcccgctgttgatcgaggccggctacaccgtgtacggcagcacccgccgccccgaacgcgcgtatgcgctggaggcgcgcggcgcacgtccggtcatcgtcgacgtgttcgacgctgaagctctgcgcgtggcactgaagcgcatggcgccaatggcggtgatccaccagctcaccgacctgccgcccgacctcgatcccaagctgatggccgatgccgcccatcgcaacgcacgcgtgcgcagcgaaggcacgcgcaacctcgtggccgcggcgctggcggccggcagccgccggctggtggcccagagcattgcctgggtctacgcaccggggcccctgccccacctcgaagagcatccgctcgatctcgaggccgaaggcagccgccgcgtcagcgtggacggcgtggctgcactcgagcgcagcgtgctcggcacgccgggcatcacgggcacggtgctgcgctatggcctgttctacggtccgggcacctcgaacgccgggcccaagggcgcatgcccggtccacgtggaggccgcggcctgggcggcggtgctggcgctgcggcaggcgcaaggcggcgtcttcaacatcgccgaggacaaccccgaggtcagcagcgaaaaggcgaaacgcgatctcggctggcatgcatcgctgcggctgcgtccgcggcaaggagttgaatcgtgaaggcggcccggcttcatcgcgggccgctgggggctggcatcgccgcgctctcgctggtgctggccgccggctgggcgctgatgccgaacggcaaccggcaggaggcggtggagtggttcgccgaggtgtgcagcagcgtcgcgcgaccgatgttctcgtccgccccggcgcccgcgggctcgggcgccgacgccaggcccgccacttcggtcaaggttctctcgtgcgaagcgctgccgaacgtgccgggcaagtcggtcaccacggttctggtcgactttccgccactcgcgtattcgccggcccatcggcacccgggctcggtgaccgcgatcattctcgagggcacgatccgctctcagcttggcggcgggccggtgggcacctacaagagcggcgaaaccttcttcgagccgccgcgcacgctccacctctttgcggaaaaccccgatccggtgcgcccagccaagctggtggccgtgttcgttaccgacgagaactgcggaccgctgttgctgccacccgacgccgactgaagaggtgcctagggtgcgggagcattccgcacaggcatcgaacttgctacacttttttactaatttgtacgaaaggtggcgcatggacggctctcgaagaaaactggtgcaggcgtgcggggcgatgctgctgggcggcagccttcctcttcccgtgctctcgcaatccaccaaggcagcagcagcgggctcgcgggtcgtcctgctggggcagtcggtgcccttgaccggtgcggccggcgagatcgggctggccttcgcagccggcagccggctggccgtgagcgacttcaacgagcgcaatgccgccggcggcctccagctcaagctgctgcagctggacgacggctatgacgccggccgggccgccgccaacgcccgcacgctgctgggcccggacaaggccgacatgctgttcggcttcgtgggcaccgccagcagcgacgccggggcgagcgtcgccgcgcagcagggcaacctgctgttcgcgccttttgccgcagccgattcgctgcgcgaggcgagccatccgaacgtgttccacgtccgccccggcatgatcgacgaagccctgaagatcgtgcgccagtgcgccaccgtggggcagacgcgcatcgcgctggtgggcgacgacgacgccatgggccgcgccggcctggccgccgtgcagcaggccatcaccgaactcaagctccccgcgctggttgccacggccatggttcctgcgggcggcgacaagctcgacgcggcgctgaagacagtgcagcagcagacgccgcaggccatcgtgctggtatcgctctcgggcaccaccgccaatgcgatccgcaagctgcgcaagagcggctacaccggcagcttcatggcgttctcgatcgtgggcatcgacccgctctacgccgagctgggcaaggacatcggcggcatcgtgatctcgcaggtggtgccgtcgccgcggccttcggccattcccatcgtcaaggagtatcgcgccgcggtcgacaactccgaccagacgccatcgtacgaaggcctggagggcttcattgcggccaaggtggtgggcgaagcggttcgccgcgcggggcgcggcttcacgacggccagcctgcagcgcgtgatgaccgccatgacggactacgacgtgggcggcttccgcgtcaacctgcgcccgggcctgcgcgatccgtcgagaaacatcgacctgatcagcatctcggccgacggccgcgtgctgcgctgagtcatccgctcctgaccagcgcctgcagcgcatcgaccgacaacaggtcgatgcgcccgtagcccagcgaaatcacctcgtcgcgcgcgagtgcgttgagttctttggagagcgtctgccgcgagacgccgagcatcatggccagcgcctcctgcggcagcatcagcgtacggcgcaagtgcaccgactgcgtggcatcgcctcgcgccagcaccaggagccggtgcgccacgcgcgcacgcaggctgcgcagcgtggcatcttcggtcaggccgtagagcatgcgcacgcgcgcggccagcatcgcggcaatcgcgttcgcaaagaccacgtcgcgcatctggtgggcaaaggcctccggcggcaccacgagcaggtcgagcgattccagcgcagtggcgtcgtgcgtgcgcggcgagccgtcgatcagcgtgatttcgccgaaccagttgccgggctcgagcaccgcgaggatggcctcgcgcccatcctggcgcagcgacgagatcttgatggtgcctgccgccagcccatagaagccaccgcccgccgcatgcaccggatcgccctggcgaaacaccatggctcctcgccgcacgtgaatcagttcggccgcgcccaccagcgcctcgcgctgtgcgcgcggcatgctggtgaaccacgggttgcgctccattgcggcgcggtgcagagcggaaagacgcagcttgggagcggccatgcgggagaaattgcctcgaagacgcctcggggcggggtttaccagagccttgcattgtcaaattcaagacagttgaacgtcaagcacaggtctacagtggccggcattccccgagaacatggagacgacacgatgagcgaacgggcaagtttcaagagcatgcaggagagcacgcgcgaggactggcaactgatcggcggcgagttcaggcagtttgcgggcggcctgcccgcacgcgtgatcaagcacctgcagatcctcgaaggcgactacggcggctttccggtcgaccgctacacccattcgctgcagaccgcgacgcgcgcactgcgcgacggccgcgacgaggagtacgtggtgtgcgcgctcttgcacgacatcggcgacacgctcggcagcttcaaccaccccgacattgccgcggcgattctcaagcccttcgtgagcgaagccaaccactggatggtgcagcaccacggcatcttccagggccactatttctttcatcacattggcttggaccgcgacatgcgcgacaacttcaagagccatccgcactacgagcgcacggccgagttctgcgcgctgtacgacaacccggccttcgaccccaaggccgagacgctgcccatcagcgagttcgaacccatgctgcaacgcctgatggccgagcccaagcagagcatctacaaggccgcgatgaaagaacccgcggccgcctgaaaccgaccaggaacccgagaaggaaacaccccccatgaacgcagcctcccaacccgaaatccagaagctcgtgtccgccgaagaatggcagctgcgcgtcgaccttgccgcctgctatcgcctggtggcgctctacggctggagcgacctggtgttcacccacatcagcgcgcgcatccccgggcccgagcaccacttcctcatcaacccctatgggctcatgttcgacgagatcactgcgtcgagcctggtcaaggtcgaccagcagtgcaacaagatcatcgagtcgccctacccggtgaacccggcgggcttcgtgatccacagcgcggtgcacgccgcgcgcgaagacatccagtgcgtgctgcacacccacaccaaggccggcattgccgtgagcgcgcagaagaacggcgtgctgcccatcagccagcaatcgaccttcgtgctggcttcgctcgcctaccacgactatgaaggcgtggccttccgcgacgacgaaaagccgcgcctgcaggccgacatgggcagcgccaatttcctcatgctgcgcaaccacggcctgctcacctgcggcaagaccattgcggacgccttcctttcgatgtacaccttcgagaacacctgccagatccagattgcggcccaatcgggcggtggcgaactcacgcacgtgaacccgaagatcgtcgaaggcgtgggccaggccatgaaggtgcagaccggcggcctgggcggacagttcgtctggccatcgctgatccgcaagctcgaccgcatcgacgacagctacaagcaataagcgccgatcccggtttacacggctgccagcgcctgcgcgacaggtgccggcagccatttttttagaagaaccagaaagaggagacaacaaggcatggacgctacgctcatcgtgacccgcttcctgttcggcgcgctcgcgctggtgatgttcgggctcgggctttcgctttcgctggacgacttccggcgtctcttcaggcaccccaaggcggtgaccatcgcgctcgcgctgcaggtcgtcgggctgccgctggcctgctacgcgatcatcgtcggcttcgggctgtcgccggtgttcgccatcgggctgatgctgctcgcggcttcgccgggcggcatctcggccaacctgttctcgcacttgttcggcggcaacgtggccatgaacatctcgctcacggccgtcaacacgctgctgtcgatcgtcacgctgccgctcattgccaactgggccatcggccactttgcgcagagcggccaggtggtgccgctgcagacgcgcaagctggtggaggtgatcgccatcgtgctggtgccggtggccatcgggatgatcgtggcctcgcgccggcccggcttcgcggcgcgcatggaaaagccgaccaagatcttcagcgccgtggtgctcgcggtggtcacggtgctggccatcgcgaacgagtggaagaacatcaccgcgaccttcgccgagatcgggttgccggtgctgctgttcaacctcgtgagcctgctcgcgggctactacctgagccgcgccgcgggcctcgacaagccgctggccacggccatcagctacgagatcggcattcacaactccacgctggccatcttcatcgccgtgagcgtcctggggagctttcagctcgcgctgccggcggccatctactcggtggtgatgtacatcaccgccccgctgttcggctggctggtgttgcgccggcggcaaccggtggccgtgcctgcgcgatgatgcgggcatggaacttcggcaactgcgctacttcgtcaaggtctgcgagcttcgcagcatgggccgcgcggccatcgaactgggcgtggtcacttcggcactgagccagcagatcagccggctcgagggcgaactctccacccggctgctgcagcgcagctcgaccggcgtgacgcccaccgacgccggcctcgccttcttgcagcaggcgcagctcacgctgcggcatgccgacgatgcggtgcgcgcggcgcagcaggcgcgcctctcgggccatgtgagcgtgggcctcgcgcccaccacggccacggtgctcggcgtgccgctgatgcgcgccatgcaggagcgctaccccgaggtgcggctgcacatggtcgaggcactgtcaggccacctcaccaccatgctgcaggcgcgccagctcgacctggcggtgctgttccagaccgacacgccgcggcgctggagcgtgctgccgctgctggcggaaaagctgttcgtgatcgcatcgccccatcttgcgcagcgcccgtccggcgccaaggtgcggctgtcgcaactggccgagctgccgctcatcctgcccagcggaagccacggcttgcgcgccacgctgatggccgctttcgcgcgggcgcgcatccagccgcgcatcgtcgccgaggtggatggcctggcgttgctgatggacgcggtgcgcgcgggctacggcgccaccatccagcccggtgcggccaccgcgcgccatgacagcgacgaccttcagctcactcagatcagcggtgcgcacgtgggccgccacaaccttctggtgagcctgtccgacgacgaactttcgccggccgcgctggcggcgcgcgtggtgcttgccgacacggcccgcgccctggtgcgcgagggccgctggaccggcgcaagtcttctcgatcactgaacacccgttgcctcgatcggcctttcgcgtgaaggccgcgctccctaaagtctcctgcattccaaggagacccacgagtgatcgatgtattggttgtcggtggcggcaatgccgcgctgtgcgccgcgctgatggcgcgcgaggccggtgcctcggtgctgctgctcgaagcctcgccgaaggagtggcgcggcggcaattcgcagcacacccgcaacctgcgctgcatgcacgacgcgccgcaggacgtgctggtcgaggcctaccctgaagaggaatactggcaagacctgctgaaggtgaccggcggcctgaccgacgagcacctggcgcggctggtgatccgcgcctcttccgactgccgcgactggatgcgcagccatggcgtgcactttcagccgccgctctcgggtgcgctgcacgtcgcgcgcaccaatgccttcttcatgggtggcggcaaggcgctggtgaacgcctatttccgcagcgcggaacggctgggcgtgcagatccgctacgacacgcccgtggcctcggtggagctcgacggcgagcgcttcgtggccgtgcgcaccgaggccggcgagcgcatcgaggcgaagagctgcgtgctggccgcaggcggcttcgaatcgaaccgcgaatggctgcgcgaagcctggggccggaacgagcgcggcgagtggccggccgacaacttcctcgtccgcggcacgcgtttcaaccagggcgtgctgctgaagtacatgatcggcgccggcgccgacagcatcggcgatccgtcgcagggccacatggtggcgatcgatgcgcgcgcgccgctctacgacggcggcatctgcacccgcatcgattgcgtgtcgctcggcgtggtggtcaaccgcgaggcaaaacgcttctacgacgagggcgaagacttctggcccaagcgctatgcgatctggggccgtctggtggcgcagcagccggggcagatcgcctggtcggtgatcgaccagaaggcggtcggccgcttcatgccgccggtcttcgccggtacagaggcgaacacgctcggcgaactggcgcagaagatcggcctcgacgaagccaccttcgtgcgcaccgtgcaggactacaacgccgcctgccgcgtcggcagtttcgaccacgccgcgctcgacgactgccataccgaaggcctcgcgcccgccaagacgcactgggcccgcccgctcgacaccgcgcccttctacgcctaccccgtgcggcccggcatcaccttcacctacctgggcctgaaggtggaccagaccgcggcggtgcgctttggcggccggccgagtcccaacctgttcgtggccggcgaaatgatggccggcaacgtgctgggcaagggctacacggccggtgtcggcatgagcatcggcacggccttcggccacatcgcaggcacgcaggccgcgcgggccgccaagaacctttcgaagaaatccccggagaccgcccttgcagcagctcactgatctcgtcgcacgcgcccgtgcggatgccgacggcatcggcagcgccccggtgcgcgtgatccccatccgccccgcgctgccactgaccgccagcgaagacgaagttgcgcgcatcctgcagatctgcaacgcctgccgctattgcgaaggcttctgcgcggtgttccccgcgatgacgcggcggctggagttcggcaaggccgacacgcactatctcgccaacctgtgccacagctgtggctcctgcctgcatgcctgccagtacgcgccgccgcacgaatttgcggtcaacgtgccgcaggcgatggcgcaggtgcgcatgcagacctaccacgactacgcctggccccctgcgatgggtgcgctctacaggaaggccggcctcaccgtcgcgctggccctggccggtgggctcgcactgttcctggtgctggccgtggcgatgacaggcacgctgctgcacgaaccgctcgcgggcaatttctacgcgatctttccgcacaactttctcgcgctggtgttcggcgcggtgttcgccttcgtgctgttcgcattggcaatgggcgtgcggcgcttctggcgcgaggtgtcgccggcgcaggagaacccgcccacccaagtggccggcgtgcgcgccgctgcgagcgccgaggccgctcacgatgcgctgcgcctcacctacctgggcggcggccatggcgagggctgcaacaacgaagacgaccgcttcacgctctggcgccggcgctttcaccacttcaccttctacggcttcatgctgtgcttcgcctccacctgcgtggcgacgctctaccactatctgctcggcctgcatgcgccctatgcgctcacgagcctgccggtgctgctgggcaccgcgggcggcatcgggctggtggtcgggccggtcggcctgctttggatgaacctgcggcgccatgcggcgcagggcgacgtggcgcagcgaccgatggaccgcggcttcatcgcgctgctgctgctcaccagcgtcacgggcctggccctgctcgcctggcgcgacaccggcttcatggcgctgctgctggcggtgcacctgggcgtggtgatggcgctttttctcacgctgccctacggcaagttcgcgcatggcatcttccgctcggcggcgctgctcaagtttgcgatcgaaaaacgcctgcccagccgcttgcagctgggcgccgactgaagcgcccggatccgacgcagggcgagcctctgcgaaccggatgtaacagcgccaaagcccgaccggacaagtctgccccgctttggcgtgagaatggcgggccatgcacgttcgaatccccgccatggcggtcctgctgggcctggcctgttttctctcccccgcttccgatgcagcccctcccaccaccagggagacccagggcgcggacgcccgtatcgattcgctcatcgcccgcatgacagtcgaggagaaagtgggccagctcagcctctacggccccgccgacaccaacattcccggcaacccccaagccggccagcgcaacgcacaacaagagatcgacgatgtgcgcgccgggcggctcaccggcctgttcaacaaccagggactggaacgcaagcgcgtgctgcaagaggtggccgtgcgcgaatcgcgcctgggcattccgctgctctacggcgccgacgtgatccacggctttcgcaccatcttccccatgccgctggcggaagccgctagctgggagcccgcgcttgccgagcgcaccgcgcgcgcggcggcggtggaagccagcgccgacggctttcgctggaccttcgcgccgatggtggacattgcacgcgatgcgcgctggggccgcggcatcgaaggtgcgggcgaagacgtgtacctggccaacctgttcgcggcggcgcgcgtgcgcggcttccagggcagcgacctctcgcgcggcgatgccctgctggccacgcccaagcactttgcggcctatggcgccgcggagggcggactcgactacgcggccaccgacatctccgagcgcacgctgcgccaggtgtacctgccgccgttccgcgccgcgctggacgcgggcgcgctgtcgatcatgagcgccttcaacgagatttcaggcattccgtcgattgccaacccggcgctgctgacgggcgtgctgcgcgaggaatggaagttcaagggcttcgtggtctccgactacaccgccgacgaggaactgattgcgcacggctacgcggccaacgggcgggaggcggccaggcagtcgttcctggctggcaccgatgtcagcatgcagagcggcctgtacatgcgctacctgcccgaactcgtggcctcgggcgaagtgcccatggcgcgcctggacgatgcggtgcgccgcgtgctgtgggtcaagcagaagctcggcctgttcgatcagcctcttcgagggctcgatgccgcaccggcccgggcacgcgccgagaaccccgagcacatcgccctcgcgcgcgaggatgcccgccgcgccatcgtgatgctgaagaatgagcgcgcggtgctgccgctgcccaggtccggcaagaagatcgcgctgatcgggcctttcgcctcgggaacgcaggacctgctcggcgcctggagccttttcccgggccagtcggctcccgtcggcatcgaagacggcttgcgcgccgcgctgcgcgaccccgcggcgctggcggtggtacgcggctcgggcatcgatgcgccgttggccggcggcatcgaggccgcggtggcggccgcgcgcgacgccgacgtggtggtgctcgccatcggcgagggccagctcatgtccggcgaggcccgttcgcgcaccgacatcggtattccccaggcccagcaggatttggctgaagccgtggcggccaccggcaagcccgtggtcgtgctgctgagcaacggccgcgccatggcgctcaggggcgcggtgcgcaacgccgacgccatcctcgtgacctggtttctcggcgtgcagaccggcaccgccattgccgacgtggtgttcggcgacttcaatccttcgggccggctgccggtgagctttccacaggcctccggccaggtgcccttctactacggccagaaacgcaccgggcggccgctgcccgacaacgaccaggccatggcattcaagacacgctacgtggacaccaccaatcaggcgctctaccccttcggccacggcatcggctatgcaccggtgcgctacgacagcgtggagatgagccaggaccggctgccgctcggcggcacgctgcgcgtgcgtgccaccctcaccaacaccggccagcgcgaggccgaggaagtggtgcagctctatgtcgcagaacgcgccgcgagcgtgacgcggccggtgcgcgagctcaagaacttccgcaaggtgcgcatcgagtccggcgcatcgaaggtggtcgagttcacgctcggtgccgacgacctgcagttcatcggccgcgacatgaagccgaccgtggagcccggtgagttcgacctgtgggtcgcgccttcggccacgggcggcctgcgaaagagttttgcgctgacgcgggagtgaggccccatgaccacctcccccgtacccatcgaacagcgcctggacctcgtctccgagacggacatcgagacctactggtttcagccgaccggcaccgtctcggcaacgctgggcgaacggaacgggcctgtgtgcgcgccggtgtttcagtacagcgtactgtccgacgacagcatcgagattgccgacagcgagcgcgtgattgccacctggacgcgcatcgaagtcgacggcgatgtgttgcgtgccgagtgcaacggaaagttcaagactttccgcatcggctgacgggacgaccgcctcaatgaaaacgggcccgagggcccgcttcatcgtcagagaacgatcggcttacaggccagcttggcgcgtgaacgacacgctgggcttcttgtaggcttgcggcacttcgtcgcggtagaaagcgcggcggtcgaggctggcgagcgggtcgtgcgccttggcaacggcttcggcctggatcaccgagcggtcggcggtcgagctgaaggcttgtgcgccggcgctggcgccttcgctgtattcgttgccggcgcgggcggctgcaacggcttgcggggcgacttcggcgcgcgagacgccggagttcacgctcaccacgccttcataggtttcagcgtgcgcaccggcagcagccaggagcgagagagcagcggcagcgaggatcttcgaggcattcatttcaatctcctaatgggttggttggtgagatgaagtttgagcccgaagccccatgaaaaaacgccgcaaaatgaatcacggcgttcacgggattgaaacaatcgagcgccacgaatccatcgtgccgccccgattgattagcgcagcattagtgcgaaatcatccatggccgcttcgacggcgcagacttcgcgccgttcgccgcggtcaccgtcgcaccgctgcgcctggacgatcccgagcaacagccgcagcccgccggatgcttgaagcgcgcgtagtcccgcgaactgcccggttcatgccgcgcacgctcattggtctccatcgcacggcgcgtgcccgaggccatcagcgcgagccgtggcgcggccgaaagtacacgcggcgatgcgcctccgcagtcggggcacgcggccggctcgtcgcgttggcccgaaggccgcagcgcatcgaatccgccgcattggccgcaggcgtagtcgtaggtcggcatgggcgcctcaggccaggtcgtgcgacagcggcatctcgatgctgccgtcgatcatcttcaccggccccgatgcattcggattgatgtcgaagtcgaagatctgcgtgggcagccagagcgtggcgcaggagttgggcacatcgaccacgccactgatgtggccctgcacgggtgctgtgcccaaaatcgaatacgcctgtgcgccggagtagccgaacttcttcagatactcgatggcgttgaggcaggcctggcggtaggccacgttcacgtcgaggtagtactgcttgccgctctcgtcgaccgagatgccttcgaagatcaggtagtcgttgtactgcggcgtgatcacgctcggcttgaagatcggattcttgatgccgtacttggccatgccgcccttgatgagcgtgaccttcatgtgcacccagccggccatctcgatggcgccgcagaaggtgatttcgccatcgccctggctgaagtgcaggtcgcccaccgaaaggcccgcgccgtcgacatacaccggaaagaacaccttcgagccgcgcgacagatccttgatgtcgcagttgccgccgtgttcgcgcggcggcacggtgcgggcgccctcggccgccgccttggcgcgtgcttcgccgctcatcttgcccatgtgggcggtgccggccgagggcgggttggccaggccgggcacgcgggtcgggtcggtgtcgatgagcttctgctcgcgctcgttccacatgtcgagcatcggcttgtcgggcaggcagccgatgaggcccggatggatcaggcccgcaaagttgacgcccggcacgtggcgcgagctggtgaacatgcccttgaagtcccagatggatttttgcgcttcgggaaaatggtcggtcaagaagccgccgccgttcttcttcgagaagaagccgttgaaaccccagaggctgtcctgcttggcgccgatgtcgagcaggtcgaccaccagcaggtcgccgggctcggcgcctttcacgcccacggggcccgagaggtagtgcaccgtgctcaggtcgatgtcgcgcacgtcgtcggcgctgtcattgttcttgatgaagccgccggtccagtcgaaggtctcgaggatgaagtcgtcgcccgggttcacccagcaggccatcggaatgtccggatgccagcggttgtggatcatctcgttctcggtgggcgacttggtcaaatcgaccttgatcagcgtgtccgtcatttgcagtggctcctggttgggttgtgggtaacggaagaagaggtcatacggagagataggccttgatgtggttcacatcggtcttgtcgcgcgcggtctcgtgcaccaggcggccgccctcgatcacgaaaagccggtcggccacgtccatggcaaaactcagcacctgctcggacacgacgatggtgatgccgcgcagcttgcggatctcgttgagcgccttggcgatgtccttgatgatcgaaggctggataccctcggtgggctcgtcgagcaacagcaccttggggtcggtgacgagggcgcgtgcaatggccagttgttgttgctggccgccggagaggttgccgcccttgcggcgcttcatgtcccaaagcacggggaacagcgcatagatttcttcgggaatgcgttttgtcttcgagttctccaggccggtctggatgttctcttcgacggtcagcgtcgggaagatcatgcggccctgcggcacataggcaatgcccttagccacgcgcctgaagctttcgtcgcgcgacacgtcctgccccgccacttcgatgcggccgctcttgatgggaagcacgcccatcaagcttttgaacagcgtggtcttgcccatgccgttacgtcccatgatggctacggtttcgttggcgtggccctcgaaggagattccgtgcagggcttcgctctggccgtaggctacgtgcaggtcatcgaccttcagcatgatgttgctcatgtcacttcctgggttgttcgttctggacgctgctgttcagggcgggtgcaaagggcaccgggtactcccctccgcgaatgtcccccgggcttcgccctcctcctttatttcgctgcggggagcacccgatgccctgtgcacttgggcacgcggctggtgtgcggctgatcagcaaccgccctttccaacgctcacgtcgatggggtgccttgcgcagcgaaataaaggaggaggccgcaggccgggggacattcgcggagaaaggtaccccgtcggcgggagcgcgccctgaacaacgcacaacgtgacgaatagaacaaccagtcatctagtgccccagataaacatcgatcaccctcggatccgcctgcaccttctccatcggcccttcggcgaggatctttccctggtgcatcacggtgaccttgtgcgcgatctgcttcacgaaggccatgtcgtgctcgatgacgatcaccgcgcggttctggcagatgcgcttgagcagctcggccgtgagctcgcgttcgcgcgcgctcatgcctgcaatgggctcgtcgagcatcagcagctcgggctcctgcatcaacagcatgccgatctccagccactgcttctgtccgtggctcagcaggcccgcctcggtgcgcagcttgtcggccaagccgatgtcttcggccaccgcctgcaccttggccttgacctcgtcgtcgcacttgaacgccagcgcaccgagcaccgagcggcccttggggaacgacacctcgaggttctggaacacgctgaggttctcgtagatcgatggtgtctggaacttgcggccgatgcccagccgcacgcgcttgtgctcggccattttcgtgagctcggtgttcttgaacttgatgctgccgccgctggcgcgtgtcttgccgcagatcaggtcgagcagcgtggtctttccggcgccgttggggccgatgatcacgcgcagttcgttcttgtcgatgtagagcgtgaggtcgtcaatggccttgaagccgtcgaaggagaccgtgaggtcttccacggcgagcgcgaagtcggtgttgctcatgaagtggtgactccgggttcaggcgtgctggctgccgacgccttcgggcaactgcgggtcgggcgaagacggcgacgaggaaagagaggccggtgcgggcggcatcggtgtggatgcgggcggctgcaccgccgcctcgcgcagcgccttgcggcgatccttccaccagggcttgatcttttcgtcccaaaggcccgcgagccccatcgggaaagccatggtcacgccgatgaagaggccggccatcaggaacagccacaggtccggaaaactctccgagaaaagcgtcttgcccgcattcaccagcagtgcgccgtacaccgcgcctaccaggctcatgcggccgcccacggcgcagaagatcaccatctcgatggacggcacgatgcccacgaagctcggcgacatgaagcccacctgcagcgcgaacatggcgccaccgatgcccgagagcccggccgcaaggcagaagatgaagaccttgaagttcgacacgtcgtagcccgagaagcgcacacggtcttccttgtcgcgcatggcgagcagcagcgtgccgagcttgctggtctggatccagcggcatagcacgatgctgcagaccagcaggccgacgcagacgtagtagaggatgtacttggcgctatcggtgcgcgtgtcccagcccagcatcgtcttcaagtcggtcatgccgttcacgccgccggtgtagccctgctggccgatgatgagtacggtgcaaatgagcgccaccgcctgcgtgatgatcgcaaagtagacaccgcccacgcggcgcttgaacatcgcaaagctcacgagccaggccagcgccatcggtgccagtaccaccagcatgaggctcagcggcaggctcttgaacggcagccacagcatgggcagctcggtgatctggttccagtccatgaagtccggaatgccgggcgtcgactggatcttggtcgtgatggggtcggaggcttcgagcttgaggaacatcgccattgcatagccgccgatgccgaagaacacgccctgccccaggctcagcaccccgccgtagccccacaccatcaccagccctaccgcgacgaaagcgtaggtgaggtacttgcccacgaggttcaggcgaaagatgtcgagcgacagcggcagcgcgactgccagcagcaagaccagcagcaagaggctgccgagctggtagcgcaggatcgaggccttgatgaagttcatcatcgaaacgttctccagaaaggaatcgggttcatcagcgccggactttcacggcgaaaagcccttgcggtcgcatcatcagaatcagcacgatcagcgagagcgtcagcaccttggccatcgagccggtcatgaagaattccgagatcgattgggtctgcgcaatgccgaaggccgagaccaccgtgcccagcaggctggccgcgccgccgaaggtgacgacgagaaaggcatccacgatgtagagcgagcccgaggtcggcccggtcgagccgatggtggtgaaggccgcgcccgccatgccggcaatgccgcagccgatggcaaaggtcagccggtcggtcttcatggtgtcgatgccggtggcgttggccatggtgcggttggccacggtggcgcgcacgcgcaggccccagcggctcttgtgcagcgcgaccagcacgctgccggtaaccagtgccgtgagcgcaagcacgaacaacccgttgatcggaatgtcgaggccttcatgcggcgtccacgagcccatgagccactcgggcaatgtcgggctcacttcctttgggccgatgaaggtgcggaagagttgctgcagccccaggctcacgccccaggtggcgagcagcgtgtcgagcggccgcttgtagaggtgccggatcagcacccactccacgatccagccgacgatgaaagcgaacacgaaagccagcccgatggcaatcggaaagtagtacggcatgaacgcgggcgccaggctttcggtaacgcgcgcggccaggtagatcgaataggcgccgatggtcatgaactcgccatgcgccatgttgatcacgcccatctggccgaagatgatcgcgagcccgaggcccatgagcagcagcaccgcaaagaggctcagccccgcgaagccctgcatcaggccgatgttcatcatgtccgacagagtcatggagagttcccgtattggctgttggctccttccccctctgtgggaaggctgggatgggggcaggcagagcgtgtccactggcaacgccgcttgcccccacccttgccctcccccagagggggagggagaaagtcatcaggggtttattgatagcccttcggaaacggatccggcttgatcaactcagccgattccgccaccaccttgaacgtcccgtccagctgcccctgcccgatgcgcgccttgctccacaggtggtggttcgcgtccagcttcacgtagccttccggcgcggtcttcagttcgatgcccggcgagccggccaccaccttgtcgacgtcgaagctgccggccttctccactgccgccttccacagccacgggccgaggtagcccgcctgcgtaacgtcgccgatcaccgcgtccttgccgtacttggccttgaaggcggccacgaacttcttgttgttctcgttgtcgagcgactggaagtacttcatcgacgaatagaagcccgcgaagttttcgccgcccacgccggtcatttcgtcttcggtgacggcaagcgtcagcaggaactgcttgtcgcccgtgatgcccgcggccttgagctgcttgtagaaggccacgttcgagccgcccaccaccgccgcgaagatgcagtcgggcttggcgaccttgatcttgttgatcagcgagttgaagttggtgtggcccagcgggtagtactcctcgcccttgaccgaacccttctggaagttctcgatgtgcttgcgcgcgatcttcatcgaggtgcgcggccagatgtagtcggagccgacgaggaagaaggtcttggccttcttctccttcgcgccccagtccaggccccagatgatctgctgcgtggcttcctggcccgtgtagatcacgttcttgctctgctccaggccttcgtagaaggtcgggtagtacaagaggccgttctccttctcgaacaccggcagcacggccttgcgcgaggcgctggtccagcagccgaacaccgcggcgcagtggtcgttgaccagcagcttcttcgacttctcggcgaaggtcggccagtcggaagcgccgtcttccttgatcaccttgatcttgcggccaaggatgccgcccatcgcgttgatctggtcgatggcgagctgctcggcctggatggagccagtttccgagatggccatggtgccggaggacgagtgcagctggcccaccgtcacttcggtatcggtcaccgcgagcttggtggtgttgaccttggccgtggggaactgcgactggccgaagctcaggccactcaggcccatcacgggcagcgcggcagcgccctgcagcagtcgtcggcggcgcaatgccagggcatcgagggagggatcggaagcacgcgacatcaggaactccaggcaggttgaggaaaaagaaacccgggttggccgcgcaccatcgctgtgcatcggacggtgccccgagcaccatggctggtactttagaaatcactcgcgccgccgcgaatacgtcattcaacgtagcggccggaggcgcggctgcagccagactcgcaggccgtgcactggcggcggcaggtggcaaaacggcagggagcgcttcttgctgtgtcttccgccatgccactgccgccgccctcgccgcaagagcccaccatgcaatccgtcaccggccagaagatctttcgcatccgccgcgactacaacacgtgggtcgcgaacgaaacgctggaggactacgcgctgcgctacacgccgcgcagctttcgcaagtggtcggagttccgcgtcgccaacgcggccttcggcgccacctcgttcctggcgctggaggccatcggcggggccattgcgctgaactacggcttctcgaacgcgctgtgggccatcctggtggtgggactcatcacgttcctcacgggcctgccgatttcctactacgcggccaagcacggcgtggacatggacctgctcacgcgcggcgcgggcttcggctacctgggctccaccctcacctcgctcatctacgcgagctttaccttcatcttctttgcgctggaggcggccatcctcgcgctggcgctgcagctgtacctcgactggccgctgccgctgctctacctgctctcgtcgatcgtgatcgtgccgctggtcatgcgcggcatcacgctcatctcgggcctgcagctgtggacgcagccgatctggatcgtgctgttcgtctgccccttcatcgcggtgctggtgaagaagcccgagctctatgccgacttcaccggcctggtgggccgcacctcggacagcagcggcttcgatccgctgatgttcggcgccgcagccacggtggccttttcgctcgtggtgcagatcggcgagcaggtcgactacctgcgattcctgcccgagaagacggccgccaaccggggccgctggtgggccgcggtgctggtggcggggccgggctggatcgtgccgggcatgctcaagatgatgggcggcgccttcctggcctttcttgcgctgcagcacgagattccgggcaagcacgccatcgagcccacgctgatgtacctcacgggcttttcgtacgtgttgcgcgacccggcctgggtgctggcaatcaccaccctcttcgtggtggtgtcgcagatgaagatcaacctcaccaacgcctatgcgggctcgctggcgtggtccaacttcttcgcgcggctcacgcacagccacccggggcgcgtggtgtggctggtgttcaacgtggtcatcgccattctgctgatgacgctgggcgtgttcgcggcgctcgagcacgtgctgggcttctacagcaatatcgccatcgcatgggtcggcgcgctggttgccgacctggtcatcaacaagccgctgggctggagcccgcgcaccatcgagttcaagcgcgcgcacctgtacgacatcaatccggtcggcctgggagcgatgctggtggcggccgcgctcgccatgctggcgtattccggtgtgctgggccaatgggcgcgcgcgttctcgcccttcatcgcgctggcaacggcgctggtggtttcgccgctgctggcctggcgcacgcgcgggcgctactacctggcgcgcaccgacatccaacgctggacgccggggcaattggtcaagtgctcggtgtgcgacaacagtttcgagtcggaagacatggcgcactgcccggcctacagcgcgccgatctgctcgctgtgctgcacgctggaatcgcgctgccacgaccgctgcaagaccgactcgcgcgcggccgagcagatgagcaactggctcaaggcgctgctgccgcccgcgctgtcggggcggctcaactttcgcgtggcgcactacctgatggtggccacgtcgctcgtggcgctggtggccacggtgatgggcgtcgtgtatgcgcaagagaccatcgtgggctcggacctcctggacccggcccttcgcagcgcctttctcaaggtgtttgcgctgctctcgctggtggcggcggtggctgcgtggtggatcgtgctgggcagcgagagccggcagatggcgcaggaagaatccaaccgccacaaccacctgctcaccgtcgaggtggaggcgcacaagcgcaccgacgcggcgctgcagacggccaaggaagcggccgaggccgccaaccaggccaagacccgctacgtggccggcatgacgcatgagttgcgcacgccgctcaacagcatcctgggctactcgcagatcctgctcaagggcgaggcggtggcggcgccgccgcgcgacgcggtgcagaccatccagcgcagcggcgagcacatgctcggcctgatcgacgggctgctcgacctggcccgcatcgaggctggccgcctgcagctggaacccgccccgctcgcgctgcccgcctttctcgacgagctcgtgcacatggtgcggccgcaggcggagagcaagggcctggcgttcgtgtacacgcacagcgggcggctcccgccctgggtgcatgccgatgccaagcggctgcgccagattctcatcaacctgctggccaatgcggtgcgcttcaccgacagcggcacggtcacgctgcatgtcgacgcgcgccgcgaagtgctgcgcttcgacgtggtcgacaccggcatcggcgtggcgccgcaggaccaccaacgcatctttcttccgttcgagcgcggcgccgcgggacgccggcgcggcgagcccggcaccggcctcggcctcaccatcaccggccttctcacgtcgctgatgggcggcgagctgcgcctggccgacacctcgcccgcgggcagcaccttcggggtgcgggtgtacctgcgcgaagtggccgagccggggccggaggcgcaggccggcgcattgcgtcggccggtgtcgggctacatcggcgcgcgccgaacgctgctggtggtggacgaccagccggtgcagcgccagatgctggccggcatgctcgcgccgctgggcttcgaggtgcgcgaggccgcgagcggcaccgagtgcctcgacagcctgcgcgaaaacctgccctccgcgatcctgctggacctcaccatggacgacatggacggctggcagaccgcggcgctggtgcgcgcctcgggcttcgaccgcattccgatcatcatcgtctcggccaacatgttcgagaaccagggcgagttgctgcgcgccgcgggctgccaggccttcgtgggcaagccggtcatcgagtcgcagctgatcaccacgctggagcgccacctcgggctcgaatggctggccctgaacgatcccatgccgcccccggtcgacatcgccccgcggccgcagcaacttgcgctttccgaggacgaccgggccgaactgatgcggctggtgcagatgggccatgtgcgcggcctgcaccaggtgctcgaccggctcgccgccgcttcgccaccggcggccgtgacctgcacctggctgcgcggcatggtcaaccgcttcgatctcgacaatctccgcaaggcactcgcagaagaagatgcagacactctctccccctgaagccgaacgccacgtggtgctggtggtggacgacgcccccagcagcctgggcatgctgtgcgacacgctcgaagccagcggctacaccgtgctggtggccgccgacggcgaggccgcgctgcagcgcctcgaactggtggtgcccgacgccatcctgctggacggcatgatgcccggcctctcggggttcgagacctgccggcgcatcaaggccgatgcggcgctcgcgcacattccggtgctgttcatgaccgggctttcggaaaccgcgcacgtggtcgagggcttcgagtgcggcggcgtcgactacgtcgtgaagccgatccgcgcgcaagaggtgctggcgcggctgcacacgcacacgcgcaacgcgcgcatcacgcggatggcgcgcgatgccgtcgacgtcgcaggcatgggcgtggtcttcgtcgattcgcacgggcgcatcgcctggcgttcaccgcaagccgcgctgtggctccatgccctcgacgcaccaccggcccctgggctgttgcccgcctcgctcgaagccgcgctggtacccggcgcggccattgcgctggccactgcggcgggcacgcggctgtcggtgcgcaacctgggcgcagccgcgctcggggagaccatgctgctccttgctacccagcgcgacggcgtgacggccggttcttcttctgccgcacgccttgccgatgcggcgctcacgccgcgcgagaccgaagtgctttcatggcttgccaagggcaagaccaaccgcgacatcggcgagattctcggcaccagcccgcgcacggtgaacaagcacctcgaacacatcttcgaaaaactgggcgtggaaacgcgcgccgccgcggcggcgctggcgagcggccagctggcctgaccgcagaagcaggagccggcggcatcacgccgcccggcccctgtttccgacttcttacctcttgggcgccggtgttgcaggcaccgcgggcgtcgtcgtgttggtgtccgacttggacgccggcactgcgggcgtcgccggcgttgcagacgtcgtggacgtcgtggacgatgaagattgcgcggacggcgtggccggtgtcgctggcgtggccggcgttgcaggcgatgtcgccgtggctggcgttgcaggcgttgcaggcgtggcgggtgtcgccggcgttgcggcattggccgatgcgttggatccgctggtcgcgcccgcgccactgccattggcgcctgcggcggcgcctacgccggcactgccgcccccgctaccgccaccaccgcccgaacctccaccgccaccgctaccgctaccgccgcctcccccgccgccacccgcggccaaggcaaggggtgcaacgcaggcgcccatgaggaccgccaccagggtcggcgcaatacgtcgtttcagcttcatcggattctccttgttgatgtttcgacaaggccaagctagacgacgcagcaagccgcccttgtagtcaaaagtcagcatggcaggccggcctgatcggtcgggcgtctgcatcgctatgcaatcgatagctgcacggttcggctcgacggtgtccgccacaaggatgcggccagagagcagcgcgcgagggggccccggctatcccgtcgtgccgcgaggcagatggacggtgaatgccgtgccttctgccgaggacgacgtcaccgtgatggtgccgccgtggcccgtcacgatctcccgcgcaatgtagaggccgagtcccaggctcgtggcgggccgctcgtgcggcgccgattcgcgggtcgcaacctgcaccagcgggttgaagatcacctgcatcgcgtcgggaggaatcggcctgccccggttcttgacgaccagggtcgcatgcgccacttcgtccctgatcagcagcaccacgggataggtggggtcgccgtgctgcacggcattgctcagcaggttcgtcaggacctggcgcatgcgggccgggtcgaacatcaggatcacgtcgcctggcagatcggcaaccaatgcccgctggggatacgccgcgcacacctcgtcgaaggcctcctggcacagggcgcccaggttgccttcctgcggaaccacctcgatgccgcggccgagccgggtgcgcgtgtactcgagcaggtcggtcaccatgtcgttgatcgacgcaatgcttcgcctggcgacctggagcgtgcgctccttgggcttggcatcacctgacaggccgaggagatgaatgcaggaactgagcgcgctcagggggtttcgcaggtcgtgccccagcacggccaggaaggtgtccctggaattggcgacatggtcggaatacgtggccatggcctccgcaaggccctggtcaatgccctcgttgaagcgcaccacttcttcgagcaccgcggcgtcgaccgcgcccaccttccccatccacaagcgaagcaccgtggcccgcagcgcgcgatattccgcgcccagctgagacaaatcgaagcccacccgctggcgcaagcctccatgttcggcggcaaaggtctcttttgcgaacggtacggcaaaacccttggacttggcttcgcgctccttttcggattgcgtggactccatttcgcttgcaatggccagcaggatttcatgcgcatggtcccggagctcgacgacggacatggtctccgccggcgggatcatcgttcgtgcaaaggattcccactcgacaagaatgggttcgatgttgtctttgatgaattggctaaggcgcatgctggacggagtatgcgctcgtgtaggacaacaggcggttcggcgaacagcgcctgcctgccggagcgacggaagaaggggtactcgacgaagcgtatcctgaggcccctcgtcccccggaatacatcccatgaccgaacagccgctttccgggacgaaccccgtcgccccgcccttcttccacgaggcctccggcacggtccgcttctgggtgctgatcgatggccacgccatgggcgccagcattggccgggagatcctgcactaccgctaccactccggcgcccagggcgacgatccgctcgaaacctacacgcagcacgccgatcagatggaagcggccgtgcgccgccgggtcgcgcaaggctccatcgagcccgtgatgctgcgcgagtacgacttaccccgcgtttgatttcgtccatggctccagcgggctcgcattgctggcgccacccgagtcggtagtttccccagcagtggtgaaggctgattgacagcctcgctgcctacgatggatgcaaaccactcaggagacgccatgaaatcccagcttttctcgttgaatcgcctgacccgccgcaccgccctgctggccgccgcggccgtgcttgccggatgcggcatcctcagcagcccgccgcgcgccggcggcgacatccacgtgatgacctcgggcggtttcaccgcagcctacaacgacctgcgaccaggcttcgagcgcagcagcggccgcacggtcaagaccgcctacggcgcttcgatgggcaatgccgaggattcgattccgagccggttgtcgcgcaacgaaccggccgacgtggtgatcctcgcgcggccggccctcgacgcgctggtggcagcgggcaaggtggtgccgggaagccaggtcgacctggtcaagtcgtcgatcggctttgcggtgcgcaagggcgcgcccaagcccgacatcggtacggtcgatgcgctcaagcgcacgctgctggccgcaccttccattgcctattcagccagcgccagcggcacgtactacgagaccgagctgctcaagaaactcggcatcgaagatcaggtcaagcccaagagcaagcgcatcctgagcgagcgcgtgggcacggtggtggcgcgcggcgacgcggcgctggggctgcaacaggtgagcgaactgctgccgatcgaaggcatcgactacatcggcccgctgccggccgaggtccagcgcgtgacggtgttctcggccggcattgccacggcctcgaagcagcccgaggcggcacgccagctgatccgttatctcaactcccccgaggccgcgccgaccattgcaaagacgggcctcgagccgctgacggcacgttgatgcgctgatacggctggtcagtaaactggcgctcatcctccttttgaacgatggacgccatgacccagccacagccacagcccattgcccccgctcttgtttccaccttcgcgcccagcggcacgttgcgcgcgtcgatcaacctcggcaacccgatcctcgcgaacaaggacgcggccacgggcgagccggtgggcgtgtcgatcgacctcgcgcgcgagttcgcacgccggctcggcgtaggcatcgagctggtggtgttcgagaaggcggcggcatcggtcgacgcggtcaagaacgagaaggccgacatcggcttcttcgccatcgacccggcacgcagcgaagggctgcgcttcaccgcgccctacgtgctgatcgaaggcagctatctcgtacgcgacgcatccgagctcaccgacaacgcgcaggtggaccgcgcgggccaacggatctcggttggcgcgggcagcgcctacgacctgttcctcacgcgcgaaatcaggcaggccgagatcgtgcggctccagggcgcggccgcggctttggccgcactccgttcgggccaggtcgaggtggccgccggcattcggcagctgctcgaaggcgaggcactgcgcgaaccgggcgtgcgtgtgctgcccggccgcttcatggtgatccagcaggccatgggcacgccggccagccgtggcgccgaggcacaggcactgctcgcggccttcgtcgaggagatgaaggccagcggcttcgtggccgatgcgctcgaacgccacggcatcgaaggcgcgatcgtcgcgcccgcggcctaagcggcgcgttggccgcgtcgcaagcggctcacagcttgtggacctcgacgggtccttgcgaatagaacaggaagtagccggttccagtgctgaagtcgttcttcttccagcccggcggcaccttgaacacgccgagctgtccgctcgccacgccgacgaaggctgtgttcccggtgtcggtggtgatgcggcgccaggcttcgcgcgtgacgggctccatctgcatcttgggttcgctccactcggcggtgcgcaccttgtcacgcatgatgtagcggccgtcctgccgctcgatcttgaccagctctttcaggatgccgttcttcttcacggcatacacgccgaccagctctgcttcgggcccgccacccggtccgcatgcggtcaacaacagcagcgcagatgcgctggccaccagatggttgaatgcttttttcatgaggctgcccttcagcgcttctggttctcgcgcagcttcaggctgccctggtagcgcagtgcgtgcggatagtcttccttgccggccgtgtcctgcgccatcgtcatcatcttctgctggctggcctcggtcttggcaagaagcgtggacggcaggttgacgatgttcttgatctggtcgtactgcgcctgcgtgatccggcctaccgacagcaggcggaacgcgtcccgctcgatgttgagcagcagcggcttgttgtcggcaaagttctgcgccttggccagcaggtcgctccacgactgggcgctgtagttgctcacgtagtagtcctgcccggtcggcccggccagcaccgcggtgcagcccggaagatccagctgcgtggtgctgctcgccatcacgaaggtcttgcgctgctccatcgcgtcaccgtaggccagcgtcacgggaatggtccatgaagacgccggatagacgttctggttgggaaacggctcctggctgatcgacacgtaggtgcggtcgcccgcgcattgcgcgtccaccgtgagcagcggcacgccggtctgccggatgaagctgtcgccgatgtcggtcactttcttgccgccgctcgccttctcgagcgaactccacagccgcgacggcgtgacgttgccgaaggcatagtctttcaggtagatctgcaggcccttctgcatcgcctcctcgccgatgtagttctggatcatctccagcacgtggctgcccttgttgtagacgaagatcgaagggctgatgaagccgaaagagcccgcatcgttcaggttgcgctgcaccggcaccgccgtgttgcgcaggtccgccaccaccacggtgtgcttgtccagcacgtagtcggagaagctgtagtagtcagggtggaatttgatggtggtgcggcggtcgaaccagcgcgcgaacgattcgttgagccacacgttgtcccaccagtcgagcgtgaccaggtcgccgaaccactggtgcgcaatttcgtgcgtgaccaccgtcaccgaatagagcgtgggcgtgtcgcccggcttggtcagcacgcggtcggcaaactcgaagatggagccccagttctccatgccgccaaagccggtgttgggcttgttgtcgtagctgtcgttggcggccacggtgtcgaacttcttgaacggcagcgcaatgccggtgtagttgtagtagtagtccatggccaccttggtccactccatcgcgaaggtggcccaggtggagcggcccggcggcgtgaaccagcgcagcggcatttcgctgccgtcgagcgggctcttgaaggtgtccgagagaatgtcgaacttgccgccgccaaagaaggcgagatacatcggcatcgaaggcgtcttctcgaacgacacctgctggtagccgtccggcagcttgacggcggacttctgcgcggcgttcgacaccgtctgccagtcgcccggcacctcggccgagatttcgaaggtgtggcggaaggccggctcgtcccagcccggaaaccattgccgcgcatagttggtttcgccctgcgtcacgatggcgtcgctcgtcacgccctcgggcgtggaaaggccgaccttgaagacgccggtcgcggcagagcagaacgggttgcgcgccatctcctcgggcgggcagtactccgcatcggagaactggatcttgccatcccactccatgtgcagcaggtacttgcccttggcgatctgcccgtcgctgagccgcagctgaacgaagtcgcccagcgtctgcggcgtgggtatcaacgcaatcgcctcggagggattcgacagcttgcgcaaggtggttctgccattggcaaacttcaggttgtgcgcggcaacgacgatcgcatcgaccggcttgagcacttcgatctccacgtcccctcgccccacgaaggtcttgagctccgcatcgggccggaaccacagcttgtagttgatgggccagacggtgtcaggcagctccatcggcttcgcggatcggtcgatctgcgccacggccgcgtcgggtgcgagcgccggtccgtcgtcgggtgtcttgggcgacgccgaaccgtccgccgtgagcgtgggcgcattcaatgcgctggctcccagcgaagaatcgcctccgccgcctcctccaccgcaggccgccaaggtggcaagtgtcacggcggtgatggcaagatgattgacggctggcttgacaagtttcttcatgatgatgaacgcctcttggtacagacaggcgccgccgcgcatgcaccggcggatagccggcaatgcgcgaacgcgcgcgatgatggaatgaacgacacatcgacaggcaacgccgcgccctcccggcgaacgagacgttcgtcaggaaagacacgagctgtccagcgatttttttcagccggcgcggcgcgaacgcgccacgcctaaccacgccgcgagcgatgcgggcggtcccaggatgcggggagtgatgggttccattcccgtcgatgtgcgagggcgatggaatgcggctgagcctaaatgcctggatggttggcttagcgcaatcgcgtcaactctgcgggttcaggcagagagataacggttgaagaagcgattgaataaacgattgaaatggcggtcgcaacggcaagttctcttgtagctgttctgaatagcttcacgtgcgttctccctccttggaagtgggcacatttttagctgagcacagatgacagcgtcaacgaggcgcggaacttttctctctcaaaatgttcgcgcgccatacgacgaatggagtcatcgattccacgcgtgcaatgcactacgaagatggttctttcttcatgccgcgcgcggcgtgcggggcgagaacgccacgcgcatccggtgtgaccgtgcagccacactgaatgcgcgaacaggccctggaagatgtggcgcagcgctgcccgatcagcgcgcgccgtagcgcgccaccgtcaggccttccatgtcgatcgcgggctgcctgccgtcgatcaaatcggccatcacgcggcccgtgccggccgccatggtccagccgagcgtgccgtggccggtgctcagcatcaggttgggaatgcgcgtggcgccgatcaccggcgtgccgtcgggggtcatggggcgaaggccggtccagaaggacgcctcgcgcacatcgccgcccttgggaaagagatcggtcacgacatgctcgagcgtgtcgcgccgcccggcatcgagcgccaggtcgaagcccgagagctgcgcggtgccgcccacgcggatgcggtcgccgagccgggtgacggccaccttgaaggtctcgtccatcacggtggattcgggcgcgccgctggcatcggaaatgggcacggtgatggaaaagcccttgaccggatacaccggcaggtcgatgcccagcggcttgaccatggccggcgagtagctgcccagcgccaccacgtagcggtccgcggtgaagctgccggcatcggttctcacggcggtgacgccgccggcgccgtgctcgatggcctggatgcccacgccgaagcggaacttggcgccggccgcctcggccagcgtggccagtgcctgcgtgaacttgaagcagtcgcctgtctcgtcgcccggcaggcgcaggccgccgacgaacttgctcttcacccccgcgagcgcgggctcgtactgcacgcagccttcacggtcgagcacctggtagggcacgccggaggcctggagcacttccacgtccttggcaatgccgtcgagctgcttctgggttcgaaagagctgcagcgtgcccagcgcgcgttcgtcataccggatgccggtgtcggcgcgcagcgccttcaggcaatcgcggctgtattcggcgagccgcaccatgcggcccttgttgagctcatagcgcgcctgcgtgcaattgcacagcatcgacaggccccagcgccacatggccggatcgagcatgggcttgatcaccagcgggctgtgctgcatgagcatccacttgatggccttgagcggcacgccgggcccggcccatggcgcagagtagccgggcgacacctcgcccgcattgccgaagctcgtttcgagcgcgggcgccggctggcgctccagcaccgtcacgtcgtggcccgcacgcgccaggtagtacgccaccgaggtgccgatgacaccgctgccgaggatcagaacctgcatgagaacaaccccttgaaagccgcacgcgacaatgcccccgagggtacaggctcccccgcgctacaggccgagtgcttcttgcaattgccgtgccgtccagcgcctgggctcgcgcggccagtcttcgagcagcgcgaacattcttgcgttgcgcggcgcggccaggtcatggtcttgcgcaagccgcacgacttcgccgctgagcgcatcgatctcggtgcgccgtccgagcgccaggtcgtccgccatgctggagcgggccttggcgtcgatgcgcagcatgcgcgccgcgacgatgcgaaacagccagtcgggcagccgcagcaccgcggacagccgctgcgccggcaccgcggccacctgtgccggcgcgatgccggcacggccgagcacgcccagcgcctcgtcgatcagcgcggcaaagcagcgccggtagccgcgctgcagcagctcatcgcgcagcggcaggccagacagcgcgttgacgggattgttgaggttgagcagcagcttgccccattgcaccggcagcaggtcggcgtacaggtcgagcggcacgcccgcacgctcgaagaccggcagccaaggccgcagtgcggcatcgtccttggcggccagccgtccggccgtgccccggtgaaaggcacccgggccgatctcggccacgttgtacggcaccatgccgggcagcaggctgagcgtgggccccgcttgcgaggccgcggcgcagttggaaatgccgttctggaacgagacgaccgtggtgcccgcgggcaatgcaaaggccagctcggcggccgcctcggccgtggcgccgctcttcacgcacaggagcaccaatgccggcgcggcccctacgggcacctgctcgctgaaccgaaggctggcggccggcaggcgatgcgtaccgccttcgaggtcgctcagcacgaggccatgttccgcaaggccccgcagcacgcgtggccggccgacgaaggtgacgggaacacccgccgccgccaggctgccgccgatgaagcaaccgatggtgcccgcccccatcaccagcacttcgccgggaggggggccgagcacctcggtggcggccatcaggtgcgttccgcgacccaggcttgcaccgattggagcgcggcaggcaggcccgcggcatcggtgccgccggccatggccatgtcggccttgccgccgcccttgccgcccacttgctgggccacgaagttgaccagctcgccggccttgaccttgcccaccgtgtcgctcgtgacgcccgcggccacctgcaccttggcgccgtcggccgcggccagcacgatcactgccgtcttgagcttgtccttcagcttgtccatggtgtcgcgcagcgtcttcgcgtcggcgccgtcgagcttggcggccagcaccttgatgccgttgacgtcgatggcctgcgccaggagttcgtcgcctttcgacgacgcgagcttgcccttgagcgagcccacttcgcgctccagcgccctcacctgctccagcacctgcgtgagccggccctgcagctcggcggccggcgacttgagcgtggcggccacgctttgcaccgtggcttcgaggtcttgcaggtagctgagcgcgttggcgcccgtgacggcttcgatgcggcgcacgccggcggccacgccgccttcgctcacgatcttgaacaggccgatgtcgccggtgcggcccacgtgggtgccgccgcagagttcgcggctggtgccgatgtcgagcacgcgcacgctctcgccgtatttttcgccgaacagcatcatggcgccggtcttctgggccgactccatgtccatcacgcgcgcatgcgtctcggtgttggcaaggatctcggcgttcacgcgcttctcgatctcgaggatctggtcgtgcgtgacgggcgcgttgtgcgcgaagtcgaagcgcgtcttgtcggcatcgaccagcgagcccttctgctgcacgtggccgcccagcacttcgcgcagggccttgtgcatcaggtgggtgaccgagtggttgcgcatggtggcgtcgcggcgcgcggtgtcgactgcggccttgaccgtgtcgcccaccttcagcgtgccttgcgtctgcgtgccgtggtggccgaacacgtcggccttgatcttctgcgtgtcttccacgccaaactgcacgccttcggccaccagcacgccctggtcgcccacctggccgccgctctccgaatagaagggcgtggtgtcgagcaccacgatgccaggctggccttctttcagctcttgcacggctgcgccttcgaagtacagcgccacgaccttggcgctttcttcgaggtggtcatagccggtgaagacgttgcccgcgccgccgtattcgacgttgcggtccatcttgaacttgccggcggcgcggcccgcggccttctgcttttccatggcggcggtgaagccggcctcgtcgacgctcacgccgcgctcgcggcagacgtcggccgacaggtcgagcggaaagccgtaggtgtcgtgcagcttgaaggcgacttcgcccggcagcgtcttggcatcgccggccagggcggcatcgagaatttccatgccgttggccagcgtttcgaagaagcgctcttcctcggccttcagcgtatcgatgatgcgtttttcatcggccacgagcttggggtacgcgtcgcccatcagcttcacgaggtcgggcacaagcttgtggaagaacggcttcttctggcccagcttgtagccatggcgaatggcgcggcgcacgatgcggcgctgcacgtagccgcggccttcgttcgacggaatgacgccgtcggccaccaggaacgaggtggcgcggatgtggtcggcaatcacgcgcagcgagttgttgcccaggtctttctcgccggtttcgcgcgccgcggccttgatgagcgcgtcgaagatgtcgatctcgtaattgctgtgcacgtgctgcaggatggcggccaggcgctccaggcccatgccggtgtcgacgcagggcgccggcagcttcttgaccgagccgtcgggctgcatgtcgaactgcatgaacacgttgttccagatctcgatgtagcggtcgccgtcttcgtcggggctgccgggcgggccgcccgggatctcggggccgtggtcgtaaaaaatctcggagcacgggccgcaggggcccgtgtcggccatcatccagaagttgtccgacatgtagcggccgcccttgttgtcgccgatgcgcaccacgcgctccggcggcaggccgatttccttggtccagatgtcgtaggcctcgtcgtcctcgatgtagaccgtggcccagagtttttcggccggcagcttgtagacctcggtcagcagctcgaaggcccacttgagcgattcgcgcttgaagtagtcgccaaagctccagttgcccagcatctcgaagaaggtgtggtggcgcgcggtgtagcccacgttctccaggtcgttgtgcttgccgccggcgcgcaggcaggcctggaccgaggcggcgcgaacgtacgggcgcttgtcttcgcccaggaacacgtccttgaactgcaccatgcccgaattggtgaacatgagcgtgggatcgttgcccggtaccagcgagctggaggccaccaccgtgtggcccttggaagcgaagaaatcgagaaaggtcttgcgaatgtccgcgaccgtgaatgtgggctggctcatctttggatttcgtctgctgtcgagggcggcctggcgatggcgaccctctcgtcgaaaccacggcgtcgaaccgacctgactgcttgatttgcttgaacaaacgattataggtttggccaccgggccgcagcccccgcagccgggagcggcaccgcccggcgcccggaatcccgaaactgatatgagcattagcacgcagaaccaaatgcgccgggcttcgtcctattcgtttcaaaggtgaatcaaggagcacgcatggcaggccaagaggcggcacactggaagatcgaggatctggacttttcgcgcattgcgcgagcggaggtccgccaggacgagaaccttttctacctggttgcttccgcctcgttcatcgaaagcgggtcggacctctacacacagaacctggtcgactttttccgcggcgacgacgaagtcacggcctggctcacccaccactgggaagccgaggaactgcagcacggccgggccctgcgcgcctatgtgtcccatgtctggcccgaattcgactgggaaaccgcctaccgcggctttctggaggaatacgccacctactgcaaggtcgaactcctctccccgacgcgcggactcgaactggccgcgcgctgcgtggtcgagaccggcaccgccagctactaccgggccctggcccgcgccaccagcgagccggtgctgcgcgacctggcgggccgcatcgcagccgacgaggtcagccactacaagcacttctaccgattctttcggcgctatcggcaagaagaaaaattgggccggatccgcgtgctgcgcatcattggccggcgcacgctggagctcaaaagcgaggatgccgagtgcgccgttcgccacgcggtgcgcgtccgatcacccgagcgggcctgcgattcggcttacatccggcaactgggcgcgcgcatcaacggcacggtgcgcaccaacctcagccccggggccacgctcaagatgctgatgcgcccgctggaactgccggccagggtggaaaccgtgatccagtacccgatcaggcagttcatggaacacgtgtttctgcgctgacggaccggcttcgaaaactgggtacgcaggggatggcggcgcggcctacatgggcgatcgactttccccgacgcaggggtttgggtaaatgcgaaaaattcacattaaaaccaaccaacccccatggccggcagtagaagcgtctacgcaagccggatcggagaatcaaatgcccctatttcttctgttgaggctgcaacgggtgcagctgcctgtccgtgtcaccgacccggaggaagtccgccaggtctcggtgcttctggccaccggcctgatcgaggctgagttcgcaaccatcaagtcgcgggtgcggcatgccgtggagagggtagcaaccgtgacccgcatcaccgaagaaggcctggctgagatcgcggcggtgggccagtcgccagcgttcgcgcagccctttgttcgattcgcagggggattgcgattgatgtgagagtagttatttccgatatgtactaccaaatgtgtacaactttgctccgtgccccatccactgcatccatcacagagggcgagttctccaccattgcggtggataagacggtggaaaagcatgtgcgcatcgccggagaaccttgctacgcctgccccgcgacacggcgcctgtaaaagcggcatcgcagcccttgggcgatttcctcgaagctgcggctgcttgatggcgcggacatcgaagagcatggacctatactcccagctgtcgtcgttggcgcaggcatgcccctcgacggtgggtgcagcgtagtttcctcaaaaagctatgtcgaaacccaggctgaagtgccaagcctatcggggtgagatcgggtaaaccaatcgatgccgagaagttgatcgtcctatgccgatcaagcacttggggccgaaagctcgttgtgcatcagcgagttgcaaaatgcgggtgtagttcaatggtagaacggcagcttcccaagcttcatacgagggttcgattcccttcacccgctccaatcaaaggtccaaaccggtcctagcgctccctaaaagtcattaatagtcaaagacttagagaggaccgcgattcctaagtcttccgattgtttccgaacgaatccaacgcgattccggggcacacgccggggaacattggcatactcactccgaaatgcctcactccgaaatgcctctcctgttcccctagactcacagaactcagctgcaagaacgcgacgtgccgcccgagaagagacgagcacggtttaacgatggaggaaatctctatctcggaactgcaccaaacggctcgcagtgttggttttggaagtactcgttcgatggaaaggaaaagcgcctcgcaatcggcagctacccaaccgtcaggctcaaagatgcgagagccagccgcgatgaggctcgcaaggtccttcagaccggagttgatccgactcagcgccgtcgactcgacaaggccgccgttcgcgtcaacgcggtcacaacctacggaaaggtggctcgcgagttccacgccgtcaaaatcaagggctggagcgaagcgcacagcaccaagtggctgcggattacaggaaagcaatctctttccctggataggcggacttccgcttcgggacatcacagccagcgttttgcttgatcccttacgccgagtggaaagcaaactgaacggaatgggcatggggtgacgtcgaaaattgccaagtcatcattctggccgcttcaatgaagcgaacaaagcaagcgaagctcaacggcgagccccacatggtcccgcttgccccacaggctgttgcatcgctgaagcgcatgcaggtgctgacgggacatggccgctatgtattccccagcttgctcacggccgagcgaccaatgtccgacaacacggttaacactgcattgcggcgcatgggcttcgacaacacagagatgacagctcacgggtttcgcgccatggcgagaacgatcatggtcgaggaactattttgaccagctccgagcggcaagcccaccgcgacctgatgcgatgctttcaaacggtccgggacttcactcggctcattgccaagtccatctgcccgagtctgcgagagaccgaggactacgcctagctccaaaagaagctcataaagctgccgacttcgggtcttgaaattcaatccaacatttcagaggcagaaaaagcggcgctgcttcgaatcttgccaggcctgccaccgcacgccggtatgtccgcgcaagatcgagcggtgttaagcatggtccgctcaacaacctcaacatgcccggcatgacgatggtgttcggagtcaaggacgacgccatgctcgacaagctcgagaccggcgccaaggtccgctttcaggcggaaaagatcgacggtaagatcgtcgtcacgaagatcgaaacggcccgctgatcgcatacaaagcaggcgtcgatatcgaaaggacggagggaaacatggcttactccagcgcgtcgcaagtcgttcgtcaaatcctggaggggccggtcacgcgaccagccttgcagcgctggcgacgccagcgatttttttcagaggccgggttcggcagctacttcggtgtgttcaacagtttcgaggaagcgcgagactggctgcctaccgggccggaattcgaccatgccgctttggcggaggagtacgtgaacgtccgtacaaagaaggtgtttgcatacgactacccagtaatgtggtggctcgaacgcgccttcagagtcggcgccaccaaggtagtcgacattggtggttcggtcggagttcactttcacgcctatcgccggtacttcgagatgcctgcggcgctgtcctggcgcgtcgtcgaagtccccgcgatcgcgtccatcggacgagaactggccagccagtccgaggccaatggactgagctttaccgacgatttggcaccggcgctggacggcaatgacatctggatcgctgcaggctccctgcaatatttcgaggattcgcatcccggcgatctgcttcaacaatgcgagaggcggccacggcatgtcctgctgaacaaactgcccctctacgacggcgaggactacgtcacggcacagaacatcggtgccggctgctttgcgccattgcatgtctacaaccgccaaagcttcatccagaagatcgaagcgctgggctacaccctgcgcgaccagtggcaggttcaggagcgttcgttgtacctgccggggtttcccgagcgctgcgctccgacgttcagtggtctttactttgccagttgagcggcgcaggccaagcatcgatgcgcgctggccagtcctgacggaccgggacgcgcgttgttcgcagtcgagagggagaagatgaggcatcgcatcatcgtgccggcgcattctgttgtgagtggcgatctccgccggtctatcgggctgcgctgatttctaccggcagtttcgcgatttccaggatggctggcgtaccggcgagattgtcgagcgtgcccatgagcagcgttgtagcgaagctcaaagacaaagatcgctgctgattggtgttgcaatcaccgctgccctactcagccgttggctgcatctccggccctccgcatctgcatctatagacgacccgaccgaccgccgcccggacgactttaggcgtaagcaccctcgccgcacctcgggtgcgcctcgcatctctcagcatgttgatgtcggcagattcctccccgcaagcggggaaaggagttacggtcttctagagctgatacctacatcaagccaaatcgaagcagcagcccacgtagtatggcttgtcgccaccctcgacgaatggcacttcgattggcttgccctcgttgcgccaggcatcgcggcgcttgtagccagcctccctgagctcggcccacagttcctcgacgtgctggatgcgataggggcagaacgcaatgccgatgctgttgatcgtgtagagcgtgcgttcggggtgcgcggccgtcgcgttcagcacgatgcgtttcggctttaccaagagatgggacagaatctcggagatgcgctgcggcaaatactgcaggctgcccgagacatacagcacgtcgcagccgcttgcatcgctgtaattggtggtgaagtccatctgggcgggcgcgtcgcgctgaacggccagctctttccctgtttgcaccacgccggggacgtcgcagactgtccagcgcaggtcatcgggataaggcagaacacggcgaaacgcgtaatactttattcccacgtttccacccagatcaaacacgcgcctcataccatcgtcgaacgatcttccgagccagaaaaggcccggatagtcgtagaaataaatttgatggctgtagagctcaccagccgccttggcgttgctgtagccgacagccttcgaatttggcgcaccagcctctgcggccgcaaagctctcgaacgaacccatgaagaggttctcggtttcattgatcaggaacttgcgccgataggcttggatgcggtaacgcaagggcagcaggtcgggaagcatgaactggtttcctctctggctaaaagaacacactactccgcaacgcttttgaaggcgtgcagcgccgagcacggcgacctccaaatcctagcgattccttcctaggtggagagcaggcgttttcccgggcacatcggggtttcggtaggaggatcacccacggccctgtcagatgcacaagttcgaactgtgctgcgcgcaaggcgaagaaattgttgactttggcgcctgtctagatgtgaagcgtcaagaggttgtttcttgacgagttgagtctggacatgggcgcgacgtcgccgatgccgctgtgagggcgatgccagttgtagtggtgctgccggcttgccagggcatcggttcgatgggctgagttctggtaggtccagccgtaggcccactctcgcaacgcggactggatgaacctctcggccttgccgttggtctgcggccggtagggccgcgtgaagctgtgctcgatgcccagttcgatccacgcccggcacaagcagccggtgacgaatcgccccgccgcctagtcacgcacatcaatgacagcgcgctggtcggcatcgatggccggcgcccggacagcatgttgccgagcggtatttccatttcacggccccaccacgccagacagtgcctcggcgccaatttgcaacttcggctttccgcccagcttggcaaaggtgttgcccggcccgcagccgagatcgatgaccaccttgcggtccagtcgccgccagcggccagccacctgctcttgaagtgcgcgtcacgatggcagtaatccagatacccctctgcccattgcgcgttgccgaaataggtggcattggcaatgatcgcgtcggaggtccgttcgagtttcgaatatagatagcttccagaacgttcgaggacggtcacattgggcaataaaatatcacctaacatttctcgtccttcaacaaaaaccccagcctatcaatcgagttgttgcagagaatcacacgacgcccggatttcttgccgaattttttaaaactcttacagagtttgggtaattcattacaaatccactaccgcccaattgccgaacttcataggccataggtagtaggcctcaagacccggattcgtcgcgtgccccagcggaaacggcgcttatccaatagccgtcagggacgcctcgcctgcttccgatacccgaaatcggatctagccatcccccgcctcctctaccgaatttgagtcaccgcccgggtggggcgcacgcctgcgcgccggcaaatcccgccgagccggacgcgcgcagcagcagcaggcgctttgtcatggttgtggaccgcggaaagggggcgattgtctcctcccaaagggggcgcatcgctcatgcgggcggggggcgcaatttctacagtgagtcccatggctaaaagcctttccgtgaaaaagcgatgccgcgcagataggaaagcccggacccgccgggcctgcgctcggctcgcaactccgcggtaaaggcgttagctaccctattcaagcgatctgaggtagtacggttatgtaacgagcgtttccggaatgcaacttgacaagttttcacctacaccgccccaagcaaagtctctaggattgccagcgaaatacaaacctacgtactacatccattcttcttaataatttgtaaatcgctgtcgatccaattgcatgcatttcttattacatctcccctatgaaatccccatccgcattgccggcaaaattcgcgcccctccatcttccattggaagatgtattggtaccgggcttgaattcaaaaaaaacggacgagcggatcggcagtgcatgggagatcgaaccagaaagtgcactgcgctgggccgagtggatcggtgcctcggcgcagctgcccgatgccccttttgcagcagcctggctcctgttgcaggcccgctggctcggcacgccggagcccgtccttcacgagatttgcagcaccggatcggaaccggcggcgagccgaacggcgattgccgccgtctttgatcccgcccagacggccggcaactggctggccacgctcgacgagcgccgccgtacagcagctgcgaacccgtccgaggcgacaccgaactctctctggctgagcggcaacgccagcaccgccggtccccaggcccccctccgtctttggctgtccaccacttcgggcacgccgcgtcttcatgccgacgcggcggcgacccttctggacccggcaatggcagcgcaattgctcgcggccatcgccgacaccgccgccgacctgatggaccgcgccggcgctcccctcggcgacattcgcaccctctctgccgccgaccgcgagcagcagctgtcaacctggaacgccgcgctgtctccgctggaccgcagcctcaccgtggtcgagatgttcgcccgccgggccgctgccgcgcccgatgccgtcgccctcgcggagggcgatgcgcagatgagctatggcgagctcgaccagcagtcggaccggctcgcccaccgcctccagcacctgggcgtgggtgcgggcgacagcgtaggcctggtgctcgagcggtcgatggaggccgtggtcgcgcagctcggcatcctgaaggcgggcgccgcctatgtgccggtgccgacggattttccgccggagcgcatcgcgtacatgctcgacgaagcgaacgcgcgccaggtgatcgccacgtcggcgcaccgccacctcgtgcccgagtcccgggccgtactgctgctgctcgatgaagccgcgcctcccgaactcgccccatggcgcgcaccggccatcgacggcgaatcggtggcgtacgtgatgtacacctcgggctccacgggcacgccgaagggcatcgagatctgccaccgcgcgatccttcgcctggtcgtggatgtcgactacgccgacctggcaccgggatgcgccgtgctgcacgccgcaccgctcggcttcgatgccgccacgttcgaaatctggggccctttgctcaatggcggctgctgcgtcatccacggcgagcgcgtgcccacgggcgcgggccttgccgccaccatcgctcgccacgacgtgcacaccgcatggctgacggccgcgctgttcaacgccgtgatcgacgacgacccggggcatctctcgggccttcggcatctcatcaccggcggcgaagcgctctcggtgccgcacgtgcggcgcgcactggctgcactcccgggcctcacgctccgcaacggctacgggcccaccgaatgcacgaccttcgcggccacctaccgcatcccgcacgcgctgccggccgacctgcgttcggtgccgctcggccggccgatcaaggacaccgtgctgcgcgtgctgagcccttcgatggcgctgctgccgacgggcttgatcggcgagctctgcatcggcgggcacggcctcgcacgcggctatctgcggcagccgcagctgacggaagagcgcttcgtgcccgatccgttcggcgaagcgggcgagcacctctaccgcaccggcgacctggcgcgctggctgccggacggcacgatcgaattcatcgggcgccgcgacgggcaggtcaagatccacggccaccgcatcgagaccggcgaggtcgagacggccattctggcccatccagccgtgcaggcctgcgccgtggtggcacggcccgatgccgacgggcaactgcgcctggtggcctacctcgtcgcgcgctcgcacaagatctcgtgggacgggctgcgcacgcacctggccgcacggctgccggcggcgctgctgccctccgcccaggtgtggctcgaccagcttccggtcacgcccaacggcaagctcgaccgcagggccctgcccgaaccggtgggcgaccgccccgaactcgcgcagccgttcgaggaggcgcgcaacgccaccgagcagcgggtgtgcgaagcctttgcgcgcgcgttgcacatcggcaaggtcgggcgccacgacaacttcttcgatctcggcggcgattcgctgcgggtgcttcaggtgctggccgaattgcagcagggcagcgcgcaaccgctgtcgaccaccctcttcttccggcatccgacgccgagcgccatggcggcagagctggagccggcctcgggcgaagccgcatcgcccatgcccaccgccgccgcgccgcgcgcgtcgctgcctcgcaccgccgacaccggcgacctttcggatgcgatcgcactgatcgccaccgcgggccgcttccctggcgcggcggacgtcgagcagttctgggacaacctcgtcgccggccgcgacaccatcagcttcttcgacgacgagacgctcgatgccggcgtcagcgaagccttgcgcacggaccctgcctacgtgagggcccgcggcgtgatcgagggcatcgagaacttcgacgccgccttcttcggcatcggcccgaaggaagccgcgctgatggacccgcagcagcgcgtgtttctcgagatctgctgggaatgcctcgagcgcgcgggctatgtgcccgacgccgcgccgggccccgtgggcgtgtatgccggcatgtacaacgccagctacttccagcgccacgtcagcacgcggcccgacctcatcgaagcggtgggcgagttccaggtgatgctggccaacgagaaggactacatcaccacgcgggtggccaaccggctcaacctcacggggcccgcggtgagcgtgcacacggcctgctcgacctcgctggtggccgtggcccacgccttccatgcattgcgcacgggccagtgctacatggcgctggccggcggcgcatcggtcacctgcccgacgcgcagcggctatctctaccaggagggctcgatgctctcgcccgacggccgcacgcgcagcttcgatgcgcaggcccggggcacggtgttcagcgacggcgccgcggtggtcctgctgaagcgcctgtccgacgcacaggccgacggcgacaccatctatgccgtgctgcgcagcgcctgcgtcaacaacgacggcggcagcaaggccagcttcaccgcgcccagcgtggacgggcaggcggcggtgattcgtgcggcactggcggccgccaacgtggacgcgcgcagcatctcgtacgtggaggcgcacggcaccgccacgccgatgggcgacccggtcgaagtcgaggcgctgacctgcgcctacgccgagcacaccgacgcactgggctactgcacgctcggctcgctcaagagcaacgtgggccacatggtgacggccgcgggcgccgccgggctcatcaagaccgccctctcgctgcaccatgaagtgatcccgccgaccgcgcacttcagcgcgcccaacccggccatcgacttcgcgcgcacgcccttctacgtgtcgcccagcctgcagccgtggccgcgcgccggcgcgccgcgccgtgcgggcgtcagttccttcggtgtcggcggaaccaacgcgcatatcgtcgtcgaagaagcaccggtgcgccccgcatccacgtgcgcgaagggcccgcaggtcctgccgctctcggcccgctcggaggccgcgctggcggtggcgacggagcagctcgcggcgcacctcgatgcaacgcccggggtgccgctggccgacgtcgcctacacgctgggcgtcggccgcaaggcgcacgccttccgccgcgcggtggtggccagcgatgcggccgaagccgtggccgcgctgcgcggcaacgacgggccgtggcgcgtcagcggccgcatcgatgcgcgcgcgccgcagccggtgctgatgttcccgggccagggcgcccagtaccccggcatgggcaagaacctgcatgcgaacgacccggtgtttgccgctgcgttcgacacctgcatcaaggccttcggcggcgcgctggacttcgacctgcgcgagcggatgttcggcgccgacgcccaggcgctggtgcccacggccgtcacgcagcccgccatcttcacgctcgaatacgcgctggcacgccggctcctgtcgctcggtgcaaggccgcatgcgctcatcggccacagcgtgggcgagttcgtcgccgccgtgctggcgggcgtgatgcgcctggaagacgccgcccggctggtggcccgccgcggcgcgctcatgcaggcccagcccgcgggcgcgatgctgtcggtgcgcatgggcgcgaccgaacttgcggcccggctcggcccgtcgctgtcgcttgccgcggacaacggccccaaggcctgcgtggtcgcgggtcccttcgacgccatcgaagcactgcaggccgagctgcagaaggacgacatcgcagcccgcccgctgcagacctcgcacgcatttcactcgtccatgatggacgccgccgttgcgcccttcgaagcgctggtcggcgaagtggcgctgcatgcgcccacgatcccgatcttctcgacgctcacgggccggctgctcgaagactcggaagccaccagcgccgcctactgggcccgccacctgcgcagcaccgtgcagttttcgccggcagtgcgcggcgccatggcacatgcggcgcggccgctcttcgtggaggtcggcccgcgcaacacgctcgccacgctggtgcgccagcacggcgcgggcgaagtgatgtcgcttctgcacggcgaaccgcccgacgaggcccgcacgctgcggctggccctggcccgcctctggacctgcggcgcagacgtcgagctgtcccgccttgccgttcgggccggcgcgcagcgtgtgcgcctgcccacctatcccttcgagcgcaagcgtttctgggtcgacatcgcggccccctcagcgagcctggcttccgcgccgctcgccctgccaatcgatgcgccggctgcccctcagcctgcgcttgcgcccttcgttccacccctcatcctggagccgaccgtgacagctgctgcgcccgcgccacttctctctcccgcgtccactccagccgccgaacccatgggggcgcggctgcggtccttgttcgaggacatctccggcaccgacatggcacaggcggacggacacgccgccttcggcgaactcggcctggattcgctcacgctgacccaggttgccacgcagatcaagaagcgcttcaaggtcaacctcagctttcggcagctgatggagaactaccgctgcttcgacacgctcgccgcattcctgcaggagagcctgccgcccgaacccgtggccgcagcacccgcgccggtggcatcacccgccttcgttcccgcatcggtcccggctgcggcgcaagccggcatcgccgtgcagcccaccgcgtacctgtcgccgatcaatgcaaccgctgccgccaacggcatcggagccgcgccgcttgcgcaactggtcgcgcagcagatggaactgatgcggcagcagcttgcgctgctctcgagcatgggagcggacgcggcccctgccaggtccaccgtgctcctgcagccggcgccggccgcggccgcaccggcccaggccgcgccggcccctgccgcgcagccctccgccgacgaaggcagcgcgcccaaggagccggtgcgctacgacgtcaccaaggcgttcggcgccatcgcccgcattcacacccagcgcaccgcggagccgagcggccggcagaaggcccggctggccaccttcatgcggcgctatgtggagcgcacccgcaagagcaaggaattcaccgcggcaaaccgcccccacatggccgacccgcgcgtggtcaacggcttccggccgctgaccaaggagatcacctaccagatcgtcatcgagcgttcgaagggctcgaagctctgggacctggacggcaacgaatacgtcgatgcgctcaacggcttcggcatgaatatgttcggctggcagcccgacttcgtgcaggaagcggtgcgcaagcagctcgatgccggctacgagatcgggccgcagcatccgctggccgccgacgtgaccggcctgatctgcgaactcacgggctgcgaccgcgccgccctgtgcaacaccggctccgaagcggtgatggccgcgctgcgcattgcgcgcacggtcaccgggcgcagcaccgtggttgcgttcaccggctcctaccatggcactttcgatgaagtgctggtgcgcgcgggcaagggcggcaagggcctctcggccgcaccgggcgtgatgagcggcatgttcggcgacatccgcgtgctggactacggcacggccgaagcgctggccttcatccgcgagaacgccgacgaccttgccgcggtgctggtcgagccggtgcagagccgccgccccgacttccagccgcgcgagttcctgcaagaagtgcgcgccatcaccgcgcagcaaggtgcctgcctcatcttcgacgaggtcatcaccggctttcgcaccgccctgggcggcgcccaggaactgttcggcgtgcgcgcggacctcgccacctacggcaaggtgatcggcggcggctttccggtcggcgtgatcgccggcaagcgcgccttcatggacgcgctcgacggcggtgcctggcagtacggcgacgattcgatcccgggtgtcggcgtgacctatttcgccggcaccttcgtgcggcacccgctcgcgctggccgcggccaaggcctcgctcgaacatctgaaggaagccggtccggcgctgcaggcgggcctcacgacgagcaccgccgaattggccggcgaactcacggcctggtgcgtcgaggtgggcgcgcccgtcgccgtgcgccacttcgcctcgctgtggcgcgtgagctggctcgaagaccatccgctgcaggacctgctgttcgccatgatgcgcagccgcggcgtccacatcctggacaacttcccctgcttcctgaccagcgcgcacagcgcggaagacatcgcgaccatcagccgcgtgttcaaggaatccgtggccgagatgcaggagtccggcttcctgccgcgcagggccaccgtcgtcacggggttcgactatcgcaaggcccaggaagaagacggctcggtgctggcccgcgacatcgacggccagcccttctggtacgtgccggacgcctcctcacccaatcaactcatcaacggaaaggccgcagcatgaacgccgttcttcgccctcccgccgccagcggtttcatcgaatgcgtgattcccacgacggaatcgcaacgcgagatctggctcggcgccacgctgagctccgaagcctcgatggcctacaacgaatcggtgctgctgcgccttcgcggcccgctggaccgggatgccatggcgcgtgccgtggcccggctggtcgcacgccatcagtcgctgcgcgccaccatctcgcccgacggcagctgcatgctggtgagccagcccggcgaagatccgatggagcagaaggacctgagcggcctcgcgcccgaagcgcgcgagcaggcgctcgaggcagcgcacgccgaagcggtgtgcacgcctttctcgctggaacacggcccgctgttccgggccgtgctgtgccggctcaccggtgacgagcatgagctcgtcatgtcggcccatcacgtggtctgcgacggctggtcatgggtggtcatcaccgaacagctcggccaactgtatgccgagcagacgggcggcggacacccgctccagcccgccgcctcctattccgactttgccgcggtagaggcggccgaagccctgcatccggacatgcagccgcacgtggactactggctcgaacgcttctccggcggcgccctgcccgtgctcgaactcccgctggaccatccgcgcccggccacccgcaccttcggctcgcggcgtgccgagcgcctgctcgaccgccgcctcgtcaacgccctgcgcacggtgagcgccaaggccggcgccagcctcttcgcgggcctgctcggcggcttcgtcgccacgctgcaccgcctcacggggcaggacgacatcgtggtcggaattccggcctcgggccagctcgcacgcgacatgcccggcctcgtcggccactgcgtgaacctgctgccgctgcgcatcgccgcacccgcccaactgcggttcgatgccctgatgagcgaatgcagcaccgccgtgctcgacgccttcgaacaccaggcgctcacctacggcgcgctgctgggcaagctttctctccagcgggacccgagccggctgccgctggtgagcgtgatgttcaacgtcgaccccgacgtcgccaccagcgcgcagtctttcccgggtctcgaggttgtgcaggacacgatcccgcgccagtatgaaaactccgagatgttcctgaacctgcggccgctcgatggcgggttgcagatcgaggcgcagtacaacaccagcctgttcgacgacgccaccgtgcagcgctggctcgacatattcgagtgcgtgctgcgctccggcgcgcgcacgccggatgaagcgatcggccgcctcgaggtgctgtcggccgaaggcgcgcaggcgctgattgcgctgcagccgccacccatcgcattggtgggagcgccgctggcgcacgccggcttcctggcgcgcgtgccgctgcaacccgaccgccccgcggtgcgcgacggcggacggatctgcagctatgcggaactcgatgcaaagtccaaccgcctggcccgtgcactgcgcgcacgcggcgtgcgccgcggccaatgcgtggggctgtgcctggagcgcagcctcgagatggtcgcctcgctgctggccgtgctgaaggcgggtggcgcctatgttcctctcgatcccgcgttcccgcaggcccggctcgagcactacgccaaggacgcctcgatcagcctgctgctgacctcgtcggacgtcgtgggtgcgccgcgcaactggcgcgccgacccgggcgaccgcctgttcgagatcgaccgcgacaccgcatggcagcaggagtccgccgacgcgttgccgccgagcgatgacgacgcgggccccgaagacggggcctacgtgatctatacctccggctcgaccggcctgcccaagggggtgtacgcgccgcatcgcgccgtggccaacctgctccagtggatgcaccgggtgtcgggcctgcacgcggaggaccggatcggcgcggtcacgaccctgtcgttcgacatggcggtgcccgacctgctgctgccgctggccacaggggcccagatcgtgatggtgcagcgcgaaacggccatggacggcaaccgcctgtccaagctgctggagcaggaacagatcaccctgctgcaggccacgcccggcatgtggcagctgctgctcgacgcccaatggcccggcgcaccgggcttcaggggctggaccggcggcgaaccgctgcggcccagccttgcgtttgcgctgtgcgagcggctcacggaactctggaacggctacgggccgaccgagaccacggtgtactccacggcctggtgcgtcgaccccgacttgatcgtgtcgcgcggcgtgtccatcggccagcccgtcgacaacacggaaatctggatcctcgacgccgacctgcagccttgcccgatcggcgtgccgggtgaaatctgcattgcgggcgccggcctcgcgctgggctacctcgatcgcccggaactcaccgccgagcgcttcgtcacggcccgcatcttcggcgtcaacaaggcgatgtaccgctccggcgaccgcggacgctggcgcaacgacgggctgatcgagcatctcggccggctcgacttccaggtcaaggtgcgcggctaccgcatcgagcccggcgagatcgaggcccgctgctgcgaagtcgccggcgtctcgcgcagcgtggtggtggcgcgcgaagaccatcccggcgatgtccggctggtggcctatcttgcgctgacccctggcgccagtttcgatctcgatgcgctgatggcgcacctgcgggagttcctgccggccttcatgctgccccagcacgtggtcacgctcaaggagctgcccaccctggcgaacggcaaggtcgaccgtgtctcgctgccgccgccgcaggcggtctcgcgcgacgaggtgaagcgcggtgccggccctcgcaacgaacgcgaagccaaggtgctcgcggccatggagaaggtactgagcctgccgggcctcgacatgcgcgacgacttcttcatgatgggcggccactcgctgctggctgcgcgcctcaccacgatgctgagccgcgagttccagatcacgctgccgctgcgtgcgctgttcgaagcgcccacggccgagcggctggccacggtggtcgaagggctgcagggtgcgggcgtgggcgcgcaggcgccgcttgcgtgcaacttcaaccgcaggaccgcgccgctcacgccgtcgcaggaacgcatccgcctgatggaagagctgtatcccggccgctccgtctacaacgcgccctcggtgcgccggctgatcggcgatttcgacgccgcccgcttcgaggccacggtgaaggaaatcatccgccgccagccttcgctgcgcaccagcatgggcatcgacccggccacgggcaagccggcccaggtcgttgcggagcaggtggagttttcgttgcccgtgatcgacctgagtggcctgccggcggaccagcgcgaggccgagctcatggagcgcgtccaggagctggccgacgagcccttcgacatccatcgcgcgccgatggcgcacatggcgctctaccagctggccgagaaggaccacgccttcatcttcgtgccgcaccacctggtctgggacggctggtccttcgacctgctgcagcgcgagctcgcggccatctacgaagcggcggagcgcgggcggccgcacggcctgcctcccattgccaccacccacggcgactacgccgagtggctcgagaaatggatggaggagccggcttgcaagcagcagctggagttctggcgccagcgctttgccagcgcgccgctgccccgcctgcccaacacggacatgccgcggcgcgcgggcaagagcggtcagggcggcgcgcactggatccacatcacgcctgccatgacgcagcagttgcgcgaagtggcgcgcggcatggacgtgacgctcagcatgctgacgttcggcgtctatgcgctcaccatgagccaggtcatcggctccaggtccatcgtgatcgcgaacccgatccggggccggcagcagccggaaaccgaagacgtgatgggctgcttcaacaacgtgctgccggtttcgctcgaggtcgatttcaacctctccctgccggctttcatgcgctacgtgaagcaggagctgctcacgatgatgaacttccagcaggttccgttcgaacgcctgatggcacagtccgggctggagagccacatccgcgcggtcggcccctaccaggcgatgttctcgttccaggatgcgcgcgaacgtccgcgttcgatcggcaccctgcagaacaagcagatgcacgtgatgcagcgcggcgcgaccgacgacatcggcgtctggctgctcgacaagccccaggggatggaaggcgcgctgatctacaacgccgacatctacctgcgcgagaccggagcgcagctgcgcgaccgctatctcgaggtgctgtacagggtggtcgatcactccaaggaaacgctggcggagctcgccaccaccgaaggctcgcccaccgcgggctacctgcgcaagctcgccgccatcgaccccatcaagactttggcaccgggcaacggagcggccactgcgcagaagaacaacgacgctctgctgaaccccgagcacgccaagctcgcgcagatctgggcctcggtgatcgggatcgacgtcaacgagatccgcgccaccgacaacttcttcgaccttggcggagattcgctgctcgtgctgcgggcgatccagcagaccgaacagacgctgggctaccgcgtgaactcgcgccgctacctgttcgagaacctcggccagatcgcgacgtccgggcaccaggggccagacggctccgatctctcggatctcgagaagttgccgctcggcaacctgaaaggcgcagcgcggagcgaagggttgctgagcacccttggcaactggctgcgcaaggagtaatccatcatgggacacgctggtttctttggcctttgttccgtcgatgcgccggtatgccggtacctcgacctggacgaagacgccggccccgaggccgagagcatcctctccgacgaggagcgcgaacgcgccgcgcggctgcagttcgatgcagaccgccggcactacgtggctgcgcatgcggcgctgcgccacgcgctggccgcgcaaacgggcgagcacgccgaggcgctgcgcttcaaccacagcgccttcggcaagccctcgctcgcggggcggtcgcgtgtgcggttctcgctgagccacagccgcgcgctgggcctgatcgccatcggcggccgcggaccgctgggcgtcgacgtcgagcaactgcgtgagatccccgatgcattcgagctcgccgagcggcatttcacgcgctccgaacgcgaagcgcttgcggccctgcctgccgtggagcagaaccgcgccttcctgacctgctggacgcgcaaggaagcgtgcctcaaggccatcggcctcgggctgatcgtgccgccggaatgcttcgaggtcgggctggagtccgactgccgcagcgtcgaagtgccggtcgcgggccgcatcctgtggctcgcattgcagccggcgcccttccgttcggacagcgtgggcgcgctcgccgaatggcgccagacgcacgttcacgccagcgagcctcacgcggggacggaggcgtacctgtgactgcacaccccttcatgttcggaccggcctcgcgccagctcttcggcatcttccatgccgcggaggatgcgcagcccggcgataccgcggtgctcgtctgcccgccgttcggacaggaaggcctgcggacccatcgcctgttcaaggtgctggccgagcgtctctcacgagcgggtgtcgcgagcttgcgtttcgactttcacggctcgggcgattcgccgggcgacgagaccgacggcgagctcgacggctggcggcgcgacctgtgctgcgcgcacgaagagctgcgccgccgtgcgccggcaagccgcattgtctgggtcggtgcgcggcttggcgcgaccattgccgtgctggcggcccgcaacgggcgctgcgacccggcccggctggtgctgtgggagccggtgatcgacgggcggcgctacgcgcgttccttgcgcgaggagcacgtggccgccatcgacacgaccttctgcattcccgatcttgcctggcgccgcagcctggcacgcgagcccgacgccatgcccgaagaggttctcggcaccctgctctcgcccacgctgcgttcgcagctcggtgcgctggtggccgaatcgctcccgctcacggcgctgcacgacaccctggtcttgacgccgcccggcgacgagcacacggcgcaatgggccgcagagcagcagtcgcgccacatgcccgtgcggctcgcctacttccagcaccggctcgactggacgtcggacccctatcccaacagcgccatggtgccggccggtgcgctcaatcgcttgcagggtgcgctctatgaatgacgcgacgcaaagcccggtccggttcggagccggcaacgcactgatgggcatggtcaccacgcccacgcagcaggtgcccgccactgtcgcctgcctgatgttcaacatgggtgccaaccatcgcgtggggccgcgccgcatcaacgtcaagctcgcgcatgcgctcgcggcgaacggcatggcgagcctgcgattcgacctgggcggcgtcggcgacagcgaggccttcgattcggcgcacgacctgcagacccgctcggtgcacgacctgcaggccgccatggacctgctcgaaagcatgctgggcatccggcagttcgtgatcgtcggcatgtgttccggcgtggagcacgccgtgtcggcggccgccgcagacacccgcgtggtggcgctctcgctgttcgacggctttgcgtttccggaacgccgcgcccgctgggagcgcacgctgcggcgtgccctggcggcgcccgcccacccgtctttccccggcaaggccaagcgctggctgctgcgccacctgacgggcaatccgtcggcaaagccgctgcccggtttcctcaccgaaaggcagccgcccgaaatcagggccgcatggttcggcgccaccttgaatcgcctggtcgagcggaaggtcgccttgcagctgctgtattcgggctcgctgcacgtgtgcgaccgcgaccgcgaccagctcggcgcgctcggccgcgagccgttcgccaaagccctgcaataccagttcatgcgaaacgtggaccacacgttctgcacggcggaagggcaggtgcgctacatgcaaaccgttggcgactgggcgatggcatgcgcccgcagcgccagcgcggagcgccccagcccgagcccctgcacgagcccaagccccgcaacggcggccgccgaacgcccgctgcgcggtgcctacgcatcccagtaagccaagtttttccccaagagcaaaggacacaccatggcacacctcgatcaagccggttccttgcgcgttgcacgcgtcccgaccgacacggctgcaccgttcgcacgcgttcgcaaccgaacccggttggccgtcgccgccgtgctgctgccgctgtgtctggtgggctgcgggataccgggtttcagcgatcccggcaacgggggctggaccggctccgaggggagcgggcaacccaagatcgtggccatcacgcccgagctgatccgcaccatggccgcgcagagcccgcaggccttgccggccgagatgcggcagctcttcggcaaggccccggcctacaccatcgggccgggggacgtggtgggcatcgtggtctaccgccatccggagctgatgcccaacgcgggcgcggtcatctcgcagcagtcggatccgacgggtgtgagcgtggcgcccggcttcatcgtcgacagccagggcgagatcagctttccctacatcggccgcacgaaggtcgagggcctgaccgaaagcgccgcctccgacctcatctcgcgacggatctcacccttcgtgaaagacccgctggtgagcgtcagggtgcagtcgtaccgcagccggcgcgtgtacgtggagggcgaggtccgcaccccgggcctgcagatcttcaccgacgtgccgatgacgctggccgaggcgatcaatcgcgcaggcagcttcaacgcgggaggtgaccgctcgcgggtgaccttgacacgcggtgagcgcactcatgtgctcgacctgccgatgctccagcgcttcggcttcgacgcgagccgcatcccgatgcagagcggcgacatcgtgcacgtgggcacccgcgaagacagccgcgtgtatgtgatgggcgagatccgcaatccatcggccctcttgatgcgcaacggccggctgagcctgaacgaggcgctgggcgatgccggcggccccgagctgaacacctcgcaacccggccagatctacgtcatacgcaattcgcgcggcgacgtgcccgaggtgttccatctcaacgcgaagaaccccgtggcgctggccctggccgaccgcttcgagctgcagccacgcgacgtggtctacatcgaccccgtgccgctggtgcgatggaaccgggtgatcagcctgattcttcccgccgcgcaggtcgtgaacctcggaggcaccgccagccgtcgctgagcgagccccgcgccatcccacttcgccccatccgtccaggcaacccacaaaaggtgatcctatgaatgcgcactggcaacccctgattcccgctccttccgaaccggcggccgcggaccgtcccccgtccaggctcagggaacatatcgacctgctgatcgacaaccgatggaacatcgcgaagatcaccgcggtcgcgttgctgatcggtgcggcctacacgatgttcggcccgcgcgtgtacgaatccaacgtgctgatccaggtcgaggattccgatcgctcgggcggcacgctggtcggcgactccgccagcagcgccctgaacgccaagacgccgaccgcgggcgaggcggagatcctgaaatcgcgcctggtgctcgagcaggcgatcgaggacaccaagctgtacatcgaggcagagccacactacatcccggtggtcggcgcctggctggcgcgccattcgaagacgctgtccgagcccggcttcgtgggcatgtcgggctacgtcagcggcaccgagaagatcgtggtggcgcagatggacgtgccggccgatctcgaaggcacgcgcttcctcttgaccgtgaaggcggacggcgcctacaccctcacccaccccaagctcgacgcggcactggagggaaaggtcggcacgccgctcgatgcgaagacgccgcgcggcgcgatccacctcctggtgggctccatcgagggccggccgggcgcggccttcgagctggtgcgccaatcgaagcagctcaccctgctcgaactgcagaaggaccttcgcgtggtcgagaaaggcaagcagtcctcgatcatggacgtgagctggcgcgacggcaaccggctgcagctggcgaacctgctcaacgaggtcgcgcggctctacgtacggaccaacatcgaccagaagaccgcgcaggcgcagcgcgcgctcagtttcctcggttcggaattgcccaagctcaagcaacagctggagcagtccgaggaaacctacaacgagtaccgcaaccagaacggcacgatcagcctggacgacgaggcgcgcaatgcgctgtcgcagaacgtcgagctgcaggcgaagctcttcgacgcgacccagaagcggcttgagctcaccgagcgcttcaccgcccgcgacccgagcgtgcagacgatcgacgcccagatcgcctcgctcaagaaggcgctgggctcggtggagcaacgcatccgccgcatgccgcagctgcagcagaacgccctgcgcatgcagcgcgacatcaaggtgaacaccgacctgtacgtgtcgctcttgaacagctcgcttcagatgcgtctcgcgaaggaaggaaagatcggcaacgtccgcgtgctcgaccacgcagtcgtgcccgagaagcagatccgtccaaaggccgtgatcacgatggcgctcgcactgcttgcgggcctgttcgccggcgcggcctcgaccttcatgcgcaggtcgtggcgcaacaccatcgccagctcggccgagatcgaggcctacaccggcctgaccgtctacagcaccgttccgctcagctcccggcagaaggtgctggacgatgccgtgcgcagcggcgaccccggcgtgcatctgctggcagcgatccaacccgacgacccggccctggaaggactgcggcggctgcgcacagcgctgaagttcgccgtacccgtagcgccgaacaaccggatcatgatctccagcgccacgcctggcgccggcaagaccttcgtgtcggccaacctcgcggccgtgctcgcctccagcggccggcgcgtgctgctcgtcgacgccgacctgcggcgcagcagcctggcaccccatttcggcctcaggcgccgcggcggactgtcggaactgatccagggctcgctcgagctcgacgaagccatccaccggagcgtcctgcccaacctggacgtcatcaccaccggcgcgctgcacctggacccgacggccctgcttacgtgcaacgccttcgtgaagttgctcgagcggatttcggggcgctatgacacggtgatcatcgacacgccgcccatgctgctcgcgtcggaaaccgccgagatggcgacgtacatgggcacgctgctgatggtggcgcgcgccggcgagaacgagctgggcgacctgtccgaaagcgcgaaggtgctgcggaacgtaggcgcgcgtttccagggcgtggtgctgaatgcgcttgacacgcgccggcgctactacggcagcctgggctaccggttcggcggctatcggctgcggatgcatgactacccgggcgcgccggccgagcttcccgcgcccgtgcgtgcgggagcgccatcatgaccacgatccgaacgaacgcccacgtgcagccgcgcggcaactcgccgctgctgacgggcaccaagcgcctcgcggacatcgcgatggcgagcgcgttcttcctgttcttcgggtggctgtacgcgctgatatggatcggcgtgatgctgacctccggcagcccggcgatctacaagcagccgcgctacgggcggcacggacgcgtcttcagcttctacaagttccgctcgatggtgccggatgccgacatggtcctggagcgctacctgcgcgagaacgaagcggcccggcagcaatgggagatgtaccagaagctcgaccacgacccgcgcatcacgccctttggcgcattcctgcgcaagtacagcctggatgagctgccgcagttctggaacgtgctcaagggcgacatgagcatggtcggcccgcgcccctgcatgttcgcgcagaaggagctgtacggcgtctactgggaccactactgctccgtgcggcccggcatcaccggcctgtggcagatcagcggccgcaacgaggtcagctaccgccgccgggtggccatggacgtggactacgtcaccacgctttccatccaccaggacatcgtgatcctgctgaagacctttcgcgtggtggccggggggcacggctccagctaggcaccgcgccgcccactgcatttctcttttttcgacatctcaaccctcaaccgaaagaacagtatgcgtatctacgtagcaggtcatcgcggcatggtgggccagtcgttgatgaagcgcttgcggggcctcgggcacgaggtcgtcacgcgcagccacgaggaactcgatctgctggaccaggaggcggtccgccggttcttcgccaccgaacagatcgatcaggtctacctggctgcggccaaggtgggcggcatccatgccaacatgacttatcccgcggagttcatctaccagaacttactgatctccgccaatgtcacgcaccaggcgttcctcgcgaacgtcaggcgtctcctgttcctcggctcgagctgcatctacccgcggcttaccgagcagcccatccacgaacatgcgctgctaagtggcaagctcgagccgacgaacgaaccttatgcgatcgccaagatcgctggcatcaagctgtgcgaaagctacaaccggcagtacggcgcctcccacggcatcgactaccgcagcgtgatgccgtgcaacctgtacggcccgggcgacaactaccacatcgagaacagccatgtggtgccggcgctgatccggcgctttcacaccgccaagatggaagacgcgcccgaggtgctcatctggggcaccggccgggcccagcgcgagttcctctatgtggacgacatgaccgacggctgtctcatggtgatggacctgacgcgggccgagtacgagcagcacaccacgccgatgtgcgcccacatcaacctgggcgcgggccaggaccagtcgatcgccgagctggcggaactgatccgcgaggtcgtcggctaccgcggccggatccggttcgacacctcgcagccggacggcgcgcccagaaagctgctcgacgtgtcgtgcgccgccagcctgggatggcacgccacggtgccgctggccgaaggccttcgccgcacctatgccgactaccaggaggcgctgcggcccgtccaggagattgcgcacgcctgagccgcgcgctcttcccttccacacaaccgatttgcaaggcacgccatgagaacactctgcttctggttcggcattgcggctgcgttcctgtgcggctgggccgacccggcctggggctacgcggtcctgtgcgtgctgtcggtcgtgcagctggcgatgctccgcgcgccgggcgccagcgtgttcctgctgttgcactacgccaccgtgctcacgtacttctcgctggcaccggcgatgcagatcgccgacgacgtcttcttctgggacgcgggcgtgatcagcccgccggcgcacacgcaggcgctgacgctgctgctgctgtacatggcgggtgtggaactcgctcggctcggcacgcccgagccgctggtgcagtccttccctgcgcggacgccactatccgaaccgcagatggccggcgtggcgcacccgctgctgctgctcttgagcggcatcctcgcggccttcgcgacgctgttcatccggcccgacctgaacttcatcgcgcgcggcgacgtgggtgggaacgaacaaagcgttccgatcgatttcattttctattccacgctgcccaaactcatcgtgctgatgtgcttcgtggcgctggcgatccatgccctgcgccaccgcacgatctggtcctggtgctccgcgggcttcgcgctggtgctgtctgccattgcagcgaacccggtcaacacggccaggcagatcctgctgatcggcctgctgccgcttctcattcatctctttggccgcggccgtcgatggacgctggcactgctgctcttcggcgccatcgcggggctgggcccggtgctgaacctggtgtcgcgcggcagcttctggggagaatcgctcaccacctttccctacagccaggacttcgacgcgatgttcatcgttgccggcatcctggagcgcggaccggaccccgagctcggatgggggcgctacctgctgtcggccttctcgttcttcctgccgcgtgacctgaagctgtatccggatttcgatccgctcggatggccctccatcctgggcaacttctcgcaggccaacctgtcgctgccgccgttcaccactgcgttcttcgacttcggcctggcgggtccggtgctgctcggccttctgatctcggcctgcgcccgctacctggacaagctggtcgatccgcgcggcgtggtgtcgggcagctatctctgcgcgctggtgctgctggccgcgtacgtgcctttcatgcgcggccccatcctgggttggggacccttcgcggcctcgggggtcatagcggcagcgttcgccggggtcttgagttcgggcttccgccggccacgccccgccgcagcgccgtacgtccctcacacgacctgaggttcgccatgtacaaatacctgttctacgacacgatccggctcaacagcgacgcgggcggcgtgctgaacgtggccgatctcctgttgaaaagaatgcagctttgcaagggcacccggatccagccggtcagcgagctgcatccgcgcatctttgccgccgcacggcgcctccggatcagccggttcctcgtcgagatactgctctacaactatcaccgcctgcgggcgctggttgccggggagcaggtgttctcgctgttcccgaactacttcctgccgttcacgccgttcggacgccaccgcgactcgatcgtgatcgtccacgacctccagtacaaggtgtaccccgagtatttcagccgcaccaagcgcctgtggctcgactggtgcctgtggcgcgccgcgcacagccaggccgacgtggtcttcatcagccgcagcagccagcacgatttcgaacgccacttcaagcgctgccaacacgcgacggtcatcttcaatccggtggatgccacgagggcaaccactccaacagctccggccgcacccgcacccgcaaccgcaaccaccgccccgaccggcacggcgcctatcggcgagcgctacctgatcgcgtcctaccactactacccgcacaagaacttcatcggcacgctcaagctcttcgagcgcatgaagcgcgagggcctggtcgactggctggacatcaccggcaacggcgcggccgaagtgaaaagaatgaccgccaccatggcgcccgaaatcagccgctgcatccggcaccgggggctggtctcacgcaagaaactgacccagctctactgcggcgcggcggccttcatttcgctttccgcgttcgagggcttcaatctctcggccgccgaggccgccacgctcggcgtgccgctcctgctctcggacattccggtgcaccgggagctgttcaacggctacgctttcttcgtcggcagcgaggcctgcgatctcggcgagctgtcgcagtatctcgccaaccaccgcgagacccagccggcctggctgcatgccgaagcctgcgcgccgggcaccgtggccaggcgctatctcacgctgaagcgggaagcggtctcgctcgccagggccgtgcaatgacgaggcacgcgcacgttcttcgccggctgctcgcggcatggctgctgccgtgtgcggccctggcggcctccgaggcatcggccgccacggccgccacggccggtttcggcgtgatggtgcactacctgcccgacaagcattcgattgccgatgtcgcccgcttcgacgtcgacgcctttgcggaatcgctcggccagatgcgggcgtcccatctcattttgacgctcgggcagaacaacggccagtacatcgcgcccaatgccacgctggagaagctgtgcccgcaaagcgccgcgaaccggccgccgcgcgacctgccgctcgagatcggccgcgcgctgcgcgcccgcggcattgcgctggtgctgtacctgccgttccgcgcgccgcagtccgacccgtacctgatggagtgcctgggcgacatctcggagcagcagccgccgccggcccccttcatcggccgatgggcggcggtcatccgcgactggtcggagcgctacggcacgctggccagcggctggtggttcgacggtgtctacaacaccaagggcatgtcggcggagggctggaacgcgctgtgcggcgccgcgcacagtgggggcacgaagcggtggctggccttcaatgccggcgaaggccccgagcgcttcagcgtcaaggcggcgccatgccagaacctcatggccggcgagctcatgcagccgccggcgcagcccgccggaacagaggcggggttgaccttccatgtgctgacgccgctcggtgcctcgtggggccgcccgacgccgccgcgcttcacggccgaccaggtgcgcagctggatcgccgttgccaatgcgcgcggcgggctgttcacgctcgacctgccgctggacgccgatttccgctttcttccctcgcacgtggcgctgatccgcaacgcaaccgcgcctcgcccccggaccctcgcatccatcgcccatcaccggccatgaccatgaacaaccccctcgtcttcatcgtggtggaagatcgccagaacaagacactgttgctgtgccgcgagtccgcggcgcaggccgaagaatcgctcgtcgtgctgtccggcaccgacggcggcccgggctacgagcgcctgtgcagcacctatgtgcacctgtcgagcaatacgccggagttcgagaaggtctgcttccggcgctacttcctcctggccgaacacctcaaggcccatcccgattgccaggagttcgtgctgatcgacagcgacgtgctgctgttccgcggcatcggcgcgcacatccggcgcgtggtcggcaaggcggatttctgcggctcgctcatgcaaccgcgcgatggctgggatccgtgccagatatcgccccacgtcagctactggaccgcggcgggcctggagcgcttcatcgccttcgtgctcaacacctatgcaacgcccgccggccaccgaaagttgcgcgccatcgcggcgcggtttgccagccacggcgtgcgcggcggcgtgtcggacatgaccctgctccatctctgggcgcaggccagcggcaatgcggcgcccatcaaccgggtgttcggcgggcgcgtgatcgaccacaacatcaacggcgggcgcaacctgcaatacaacgagttccaggttcgcgggggcgccaagcgcctcgagttcgtcgatggacagccctgcctcgtcacgaccggaggcgagctggtgaccgcgctggcactgcacttccagggcagcgcgaagttggcgatgtcgcacgcgctgcatggccgcgtgcgaatggtcgcgctgctcacgtacgtgctgcgggtggcgcggcgcctcaagaactgggccttcgggcgcggcctgatcgcgcagcgcacgccggacggcggccgcctcgcggacgcctcggcgcccgaatgacatcgggttgaacagcgcaaccgacgcacggccatgaacccgctccaccgcaccttcagcgtcgccggaatgcgcacggtgcagcttcgcggcctgggggcgctggcttcgcggctctacgtctacctgtcgggcttcctggcggtctttctgatggcggcgtatgtctcgcccgcggacttcggccaatactcgatctaccagtcggtgctggaggtggcgctggtggtgggaacgctgggcagcgcgctgctgttctcgcgcaatgcagccaccgtgccgccaggcgtgcgccgcggcgacgtggtccgcacgctggccatcgggcttccgctcgccgtgctgctgattgccaccatcctcacgctccagcgcacggacataggcgacgtgccctttgtactgatcgtggcaacgctcgcggtcttcgcgttcatcagcctgcgtctttcgtacagccgcggccttggccacgcgggcctgctcaacctggaggccggcatccgttcgaccatcctggtgctgggggtcgcggccctcgccacgctgggcttcgagctgcgcgtcacgcacctgctgctcatcaacctgctggccttcctggtggtgggcgcggcctgcatgcacgcgggctgggccgccgggccgccgcgtggaagtgccgcgctcggcctgtcgtcgcagggcagcgccaccgtctattcgctcttgatgttcctgcttcgcaagtcggacctgctggtggtggctttcttcatgccgctcgggtacgtgggcgcattcaagatcgccttcctgttggcggaggcaccatcgcagttcgtgcaggcctttctctacacgaagacgcgcgccatgctgggcagcgatgccagcaattccgatggctcgcagctgcagctggcaaagcactcgttcttgctgggctgcgttctctttgcggcgctcgcggtgctgatcacggttgccgcgccgctgctgaaggtcggtccccaggcactcgagatcttcctgtgcattgcgccctactttctgctgcgcacctacacggttcaccacgagatgctgctcgcgctcaagacgccggtgagcacgctcgggtactgggcgctggccgaggtggcgctgcggctgctgtcgtacggggtcgtcgtcgcgatctttccgggcaagccgcactacgtgttcttcattgccaccgtatccgatctcgtcctctacgaggtgcggatgcgtgcgttgctcggcttctttccgctcgtgcggctgattcgcggttcttccacaaagcagtcatgaaaattcttctctattccatgaacttcacgcccgagctggtcggcatcggaaagtactcgggcgagatggcgcagtggctgcatgccaaggggcacgatgtgcgcgtgatcgcgtcgccgcccttctttccgcactgggcgccgttcgaaggacattcggcgtgggcctaccgcaagacggtgtgcgacggcatcacggtctggcgcgctcccacatgggtgccggcgcggccgcgtgcgctggcccgcatggcccacctcttctcgttcatgttgtccagcatgccgctcctctttgcgcagatccgctggaggccggaccttgtcttcgtggtcgagccgccgctcttctgcgcgccgaccgtgctcttcttctcgcgcatgctgggcatcaagtcgtggctgcacatccaggactacgaggtcgacgccgcctttggcctgggcctggtgcgaggcgcgcgggtgcggcgctttgcgctctcggtggagcgctggttgctgagccgcttcaaccgggtctcgaccatctccgccgccatgatcgagcgggccagggacaagggcatcgacgagacccggctggtgctgcttcccaactgggtagacgtgcgctcgatctacccgcacccggcaggcgcctcggaaacgggcgagccggtgaacggctaccgcaccatgctcggcattccgaccgacgcggtggtggtgctctatgcgggcagcctgggcaacaagcaaggcatcgaactcctggccgatgcggcacggcaactgtccacggccgggcacatccacttcgtgctctgcggcaacgggccgagccgcgagccgctgaagaccgcctgcgccaacctggaccgcgttcattttctcgatcttcaaccggccgagcggctcaacgaattgctcggcatggccgacatccacgtgctgccgcagcgtgccgacgcggccgacctggtgatgccgtcgaagctgggcggcatgctcgcgagcggcaaggccgtgatcgtcacggcccatgagggcaccgagctgagcaacgtggtggccggccgcggactggtggtggcgcccggcgatccggatgcgctctccgatgccattgcccggctcgccgcgtcgcgtccgcaacgcgaagccatgggcgcggccggccgctctttcgccgaaaccgagctggatcgaaacgccatcctgctgcgcctggagaaggagctgctgcgctgtctcgcggactgagagcgcacctcctccacaccacacccaatcgtcacgtcgcgacccatacgcaccccctacaactactacctgggtactccacatgtccgacagcacctcgaatccttccggcgtttcggatttcggccgtgcgcccgagcgccgcacgagctactcgtcgggcgtctgcccgccggccgagccgttgtggccgcactttctgaccgggcaggaagacgcgccggtgcgcgtgctgctcgtcgacgacgacgagttcatgcgacgcgtgatcgcgcaggaactgctgtccgacctgcgcatccagctcgaggggcaagccggcagtgtccgcgacggccgccgactcttggcgacccacgaattcgatgtgctgatggtcgacctgcggctgggcgacgggtcgggtttcgacctgatccgcgaggcccgcaagctgcagcgccattgcgaaatcatcgtgatctcggcgctggaggacgacgcccacgtgattcacgcgctggagctcggcgccaccggctacctgctcaagcacgcctggctccagagctttgcccaggccgtgctgcaagtggtcaacggcggcgccgccatcacgcccaagctggcgcgccggctgctgacgcgaatgaacctgcaaagcggcggcgaaccgccggccatggaaataccggtgcgcgaggcgacgctgacggcgcgggagcgcgaggtgctacgctgcgtggcacgcggctacgtgtccaaggagatcagcttgagactgggcatttcggggcagacggtcaacgcccacatcaagaacatctacaagaagctgcacgtgcattcgcgcgcccaggcggtgagcctggccacgcacaccgggcagctctgaccggtcgcatcgcttgaaaacaagcaacgaagaaggaaggacggacaccgtgaacacccccaccatccatcccgttgtgctctgcggcggcagcggaacgcgcctgtggccgctctcgcgcaagacgcttcccaagcagttcgcgccgctgatcggcgacaagagcctgctgcaactcacgctggagcgcctcgccagcctgaacaggaacatcacctgcattgcgtcggaagaccatcgcttcctggtacgcgaggcggtggacaaggccggcgccacaggccggcagattctcgagccggtggcgcgcaacacggcggccgccatggccgcggccgcgctgctcgccggcaacgatgacctgctgctgttcgcaccggccgaccatcacattcccgatacggatctttttgcagagaccatccgcagcggcgtcgaggccgcgctggccgggcagatcgtcaccttcggcgtgtcgcccacttttgccagcacggcctacggctacatcgaggtgggcgctgtgtcggccgacggccacagccgggccgtggtgcgcttcgtcgagaagccgacggcggacgtggccgaaacgctcatcctgcacggcggctactgctggaacgccggcatcttcctggccaaggccagcgtgttcattgctgcgctgcgcgcgcacgcacccgacatcctgcaggcctgcgaaggcgccaccgccgctctttcgagcgacggaagcttcgaccgcctcgaccgcgaggccttcgaggcctgccgcagcgacagcatcgactatgcggtgctcgaaaagcaccagggcatctcggtcgtgaagttcaacggcaactggagcgacgtcggcagctggaacgcggtggccgcgctgcatccggcggacgacacgggcaaccggttgagcggcagggccagcaccctgcgatcgaaaaataccttcatccatgcgccgtatcggccggtggtggcgttgggcaccgacaacctgatcatcgtggacacgcccgatgccgtgctggtggccagcgccgactgcgcccagcaggtcggcgacgtggtgcgcatgctcacgctgggaggccaggtcgaagcgacggaacacaggcgcgtggtcaggccctggggagcctacgacaggctcgacttcggcgaccgcttccaggtgaagcggctcaccgtcaatcctggcggcaagctgtcgctgcagatgcaccatcaccgcgccgagcactggatcgtggtgaagggcacggccaaggcgacctgcgacgggcaggtcaccctggtgcgggagaacgagtccatctacctgcccctgggcgccatccaccggctggaaaatcccggcaagacgatgctggaagtgatcgaggtgcagaccggcggctacctcggcgaagacgacatcgtgcgcttcgacgacacctacgaccgctgccccggaatcaagacgcgcggcgatgcggagccggtgccgctgccgtccatcgccgctgcagctgccgggatcggagccggggccgaagccaagcagcctgcgataaacggcacgccccatcgccatcacgtagcatccgcgccatgagctacacagtgaacctgatcgattttcccgatgcaccggccgaagtcatttccgcagcagaggcgcgcttccggcgcgaactcgacaaattgctgggcgatggcgtgaggccggcattgaaagccttcgaaaacgccagcgagtcgagcgccaacgaactcaccaaggacgagatcgccctggcggcaagctgggccaaggcctacgaagccgccaagacggccggctttcgcgccttgggcgaagccgacgaagcgtatttcgaagtacggctcgactgacggctggacgtcccgtcctcaccaggcagacctccatgacgaagctctggcctgccttgctgattgccgccctcctggggggctgcgccgcaccgccctccacgaccaccaccgcgccatcggccgcggcggcgccccgcacgggcacggtgtactggcagtacgtgcgctcgacctcgtacgaggcgcggcaaccggggctgggcatcagccatcgctacgaaagccgggtgggctgggtcgacgtgtatgtgtacgacctgaagcaaagcaactggatgccgggcgtggacgacccgcgcttcgatgagcatttcaaggccagcgtcaacgaggtccggctcgccggcacgaacggcgtctatgccaaggtggaagtcggccccgtgagcgacgtgaggatcgaggaccagacccttcgccgcgtgagctttcgcgtgctgcacgccgccaccggcaagcgctacgagtcgttcacgtatctcacggcgcgcaacggccggctgctgaaataccgcatgtcttttgccacgccggcaccggccgacgtcgatgccatcgcgcgcgagttcatcgcgcaaaacctgcgcagcgggcccgacatgccgagggcctcgccgccctttctcaacatctgaccagggcgcaaatagactgtacgttcatacagtgtttcctctagaatgactcgtctccaagagcaacattcgaggcgacaccatgaccaccgccagcccgcccgcgccctccgcgcggatcctgtttttttcgccgttgcggcatccgcaaccgcgccagcatgcgggccgcatttcgacctggccctttcgcgtggtttccgacaaggaccgcgagggcagcgacatccgccttcaggcggcacgcatcatccgaacgacggccgggcaatggtggccgccggccgattgagcgagcgccatgaacgagcagtcctggccgctgcgagagcgcgagttcctgattgcgctgtttcccgatgcggctgtgcaagccgccatcaaggcgcattgcgccgaatggtggtggcccgtgggccattactttccgcccggccatcggctgcacctcacgctgctttgccttgaagatcgcggccgcgccgtcgagcagctgctgcgcgaggcgctggccgaagtgccgaggcggccgctggaactcacgctcgacagttcatgcacctggcgcaacgacgtttcggtcgtgcagcctgccgagaatgaatgcttgcgcgcgctccggaacgacatcgtgcgcacgctgcacagaatgggcctcgcggcatccgccaaggactggacgccgcacgtcaccatcgccaggcagaccgagcgcgccgcgcggccgctgtgccttgcacccatccggtggaaggtgcgggagttcaaactgattcgctcgcaccgcggcaacttttttcaccacgagccgctggcgacctatccgatgctgcgctaagcctggccggcccccagctcgccgagcatgtcctgcgcatcgtcgtcgaagcccgcaatgggttgggccttggcaagcgccagccacacgccgaacggaatgcgctcgaaggcgcggtgcacggcggcgcgcgccaccaccagccgctcgccttcgagcacgagcacaccgcactcggccggaatctcgtcgggtgatgcaatgcatcggccgcgcgcgtcgttgcccagcacgtaccagcactcgccgcccaggtcgaggtaggccgcgcgcttgtcgggcttgcgcagatcgcccagcaggtcggcgcggctcaccttcacctcgtgcacgatcgggtgcgcataggcttcgacgctggtattgcggatcgagaatacgtcgggcctggcaatgcaccagcgcgccttgccgccctcttcgagcggctgcagccgcgcgcgcaggccgaggccgcgccaggcgatgcgcccgccgcgcgtcatctcgcgcgctacgcgttcgaccaacgcttcatgcggcgaaagcgccgcgcggttgagggtgagcgtggtggcgatgcgtgcaatgccggcatcggtcacgcgcaaggtttcgtggccgtgcgaagtgcgcacgcgttcgaggaacccgcccgcgagcagttcgacctcgatggcgtcgcagcagggccagcccgccgaacggtagatttcgcgcagccgccgcgcgtgcagcttgccgaacggcaccgtgccggcgcgctgcatgggcggctctttcacaggcggcggaaatccagggtcggtgaacggcggctcgaccggcggcggatcgccttcgggcggtgggccgaccggcggtggcggcggcatgggaatcggcacgtcgggcgcgggcggcggcggaccgatcggaccggcagcgacgtgatcaacaagggcgagtgcggacatgggagaaacaggttagcgaaaagtcgtggtgcgcgcgagacatggaacgatcggttgcattcattcccgtgtctctcagtggaaatcgcggctggtgttgctctgcgccaggcggcccatgagcggcgtcaggtccttgaagccggtggcgatcaggtgctgcaccttgccgccgctgtcgtcgtcgcgctgccaggtgccctgcaccgccagcaggtgcgacttcaagagcggctcgcgccaggcctcgatgacatggctccagacaatgacgttgacgttgccggtctcgtcctcgagcgtgacgaagatggtgccgttggcggtgccggggcgctgccgccccttgacgatgccgcaggcgcgcaccgtctggccgctgggctgcgcgcgcagctcttcggcgctcatgagcttcatgcgcgcgaggcgcgaacgcagcagcgcgagcggatggcggcgcagcgtgaggccgagcgcggcgtagtcgccgacgatctcctcgccttcgggcgcggccggcagttccagggcctcttcgttgatgggcacgccgcgcagcaaggcgggcgcgcggcgctgcgcggtggcgtcccacacctgctggcgccgatggcccgaaagcgacatcagcgcatcggcggcggccagcgccgccatgtccttgccgtcgagctcggcgcgcagggcgaggtcttcggtgctggtgaacggcgcttgtgcgcgcgcttcgagcaggcgcttggcaccggcttcgccgagactcgaaatccggcgcaggccgagccgcaccgcgggctggttctcgttgcccaggcgctgttcgacatagcgcgcatcggtgccgggcggcacgcgcggcgcatcagggctgcgggcttcgagcgtggtgtccatctcgctgcacgtgacgtcgaccggccgcacctcgacaccatggcggcgcgcgtcctgcacaagctgcgaggggctgtagaaacccatgggctgcgagtcgagcagcgccgccaaaaagcaggcgggctcgtagttcttgagccagctgctcacggtgaccagcagcgcaaagctcgcggcgtggctttcgggaaagccgtagtcgccgaagccgaggatctgcttgaagatggcttcggcgaacgactccttgtagcccttgccgaccatgccttgcacgagcttgccgtggaacttgtcgaggccgcccttgcgcttccatgcggccatggcgcggcgcagctggtcggcctcgtcggcagtgaaatcggccgcgatcatcgcgatctgcatcacctgctcctggaagatcggcacgcccagcgtgcgcgccagtgcgggccgcagttcttctttctcgtagtggatcggcaagcccttgtccacgcgctcgcgctgcttgagataggggtgcaccatgccgccctgaatgggaccgggcctcacgatggcgacctcgatcaccaggtcttcataggtgcgcggcttcaggcgcggcagcatcgacatctgggcgcggctctcgatctggaacacgccgacggtgtcggcgtcgcagatcatgtcgaacaccttctggtcgtcgttgggaatgtggtgcatctgcaccaccgagccgcgccagcggttcatgtggtcgagcccgcggcggatggcgctgagcatgccgagcgcgagcacatcgaccttgagcatgcccatggcttcgagatcgtctttctcccactggatgacggagcggtctttcatggacgccttctcgaccggcaccagccgcgtgagcctggtgtgcgtgagcacgaagccgcccacgtgctggctcaggtggcgcggaaagcccttgagccgctgcgtcatctcgatccattgcaccagcctgagctcgtcttcctccacgcccacgcgcgcggccgccttgaacaactgctcgcccagcacggtgtcgtcgaaccagtaatggtccttggcgaattcgtcgatcaggcgttcgtcgatgcccattgccttgcccacgtcgcgcaatgcgctgcgtgcgcggtagcagatgacgacggccgcgatggccgcgcgctcgcggccgtatttttcgtagatgtactggatgacctcctcgcgccgctggtgctcgaagtcgacgtcgatgtcgggcggctcgtggcggtggcggctcaggaagcgctcgaacagcaggtggcctttttcagggtcgatggcggtgatgcccaggcagaagcagaccgccgaattggccgaggagccgcggccctggcagaggatgtgctgcgaacgcgcgaagcgcacgatgtcttccaccgtgagaaagaacatctcgtacttgagctcgaggatcaggtcgagttctttctgcacctgctcgcgcaccttggcgggcacaccgttggggtagcgctcctgcgcgccttcccatgtcttgcgcaccagcgtctgggccggcgtctcgtggctgcccacggtttcgagcgggtactggtagttctcgcggatgacttccggatcgaaccggcagcgctcggccaccaccagcgtgttcgacagcatgtcgggaagatagagctcggccagccgcacccgctgccgcagatggcgctcggcattcgactgcagcgcaaaaccgcactcggccacggtcttgccttcgcgcacggccgtgagcacgtcgtgcagcggcttgctcgatcgggcatgcatgtgcacgtcgccggccgccaccagcggcacgccggtctgctcgctcgcctgcaagagtgcggcaaaccacaggtcgtcgtcgagctcgttgagcatctcgaccgccagccacaggttttctccgtagaacgccttggcggccagcaggtcttcatgcagcgtggcggcatccatggcgctgcccggcatgcgatgcggcacgaaaagaacctggcagtcctgcagcgaagccacgtcgctgccttcccagctcacgcggtattcgcccttgggcagctcggtgttgcgcgcggcggtgatgaactcgcaaaggttgccccagccttcggtgccgttcgcgatgaccacgagcctgaagcgctcgaagcggaactcgctgccgaacagcagcctgaagccggggttacgcggaatcggcggctcgtcggggtgcttgcgctcgtattcgtcgagcttggccggcaggtcgcgcaggcagacgtgcgcgcgcacgatgcccgccaccgagcattcgtcggtgatggccagggccgtgtagccgagctggtaggcacgctcgaccatttcctcgggcgtcgaggcgccgcgctggaagctgaagttggtgaggcagtgcagctcggcatagtccggcaggcttggcagccccggtttggatagcgcccgctgcggcagcgcatgcacctcggccgagttgcgcccgcgcagttgcttttcgctcaggtcaggcatagagcccctgcaggtaccagcgcacttcgccctgggaaaaccgcgcggagggccgctcgcgaaagatccacaccaggccggcttcggggctttcggcaatgtagtagtcgcgcatcgcgggctggccgccgtcttccttgccgccccaccagccggcctcgatgcgctgcggcccgaccagcttgcctagcggtccgcgatagcaggggcgctcgccgtccatctcgagcagcaggggttcgggcaacagccatgacgggtagatggcatcgggctgcgaggcccgggccttggcttccttgcgggccttgtccggcggcgccttgtccttctgcagcgcgggccgccaggcctgcttgcgctcgggccggtggtcggcctcggccgcgggcaccaccacctgctgcggtccgagccgcacgctgagccgctcgaccatctcgtgcagcttgtcgcccttgcggttgtcctcgggcaggaagctggtgctggcgccggcccacggatcggtttcgagcgtgcgcagccggagccagctggcgggcgcggcgagcgtggcgagggcgagcttttcggacagcaggcggcgcaggtgcgccatgtcctgcgtgggctcggccgtgcgcacggtgacctgctggtgcggcggcaggttgacgccgttgaagcgcttgaggttgagcgtccattgcagctcgagcgcgcgggcgccgcgctgccgcgcgcgcagccagatctgcagcgccgagagcaggcggttggccgaccacatcagctcgggcgcggtctcggccagcgcgggcagttccagcttctgctcgaacacgtcgggcagcgtgagccagctgtggctttctgggcgcaggccccaggcggtgtcgagcgcctcgcgcaacgccgcgccaaagcgccgcgtgaggccgccgcgcggcagggccgccacctcgccccaggtgcggcagccgagccgcgcgagcagatcgaggtgctcgcgcgcggcgctcagcgtgtccaacggcaggccggccggaatgtccttgggccggtcttcgttgcgctcgaacaggcgcagccgggccagcgcgaccaggctcgtggcaccctgcgcgcccagcatgcgcacgtcgggcgcggggttggaggcgaccagctggcgcatcagctgaagccgcccgccccacaggcgctcgcaggccgaaacctcgagcatcagcgcttcgtcctgccaggcgacgtgcggcgtgtattgcagcgcccaccagcccagcgcttcgggcgtgggcagggctggcgcttcaggcgcgtcggattcaggcagccaccgtaatgcgatccagtgcattcccgttccccttctccttccacgcgtcgatgcgcaccaccgtggccgacgacgacgcttcgcccaccggcaccaccgtgccctgctgctgcaggcgcagcttgcggcgcagccgtgcggcggccagcaaggcggccatgcgctcgttgcgcgcgggcagcatcaccggcgcggccagcggcgggccgcggcgcttgaggatgcgcagctcgatctgcgagctgtcggccgcgcagctttccacctgaagccgcagccgcgccggcgaggcgccctgcgcggccgattcgggccggcacacgaaaagcagcacctcgtgctgcgccgccgccagctgcagccgccgcagttcgccgacccgggcctgcggcagccaggccagcacggccgccacgtccgcgcagcgcagcgcctgctcgcaggcccacagccgcgaggccggggcatcgctcctgacccacatcaacgcctctaccggcaggccctgcgccgccagcgacggcccgcaaggctcgtaaggtgcgccgatcagcaccaccggcccgccgcgcgcctggaccgcctgcgccagcgcgggcagcagcagccgccagacatgcgcctcgggcgtgctttgcagcagctccgtcatggcgccgaccggccagccgccgcccggcaactccgcgtccagcgcggcatggccggtggcgacgacctgcgcgtcggccaggccgagttcgtcggcgtgccagacgccacggccggcggcagcggaaaaggagtcgaggaaagggaggcccatgatgtgattgttaactgtatttttatacagtattttcatgggccgcaccagggaaagagagggtaaagatggatttacccaaagagcctcgcctcttaatatggtctgttaacaatttgtgaccatgaaatacacaaagattcatctactggcttcggccctcgccgccttcgtcctcggactctcgcctgccgcgcaggcgcaaaccaagctcctgatcggccagacctacgttcagaccgggccgctggcgtccctgtcgaccgaacccctgatcggcatccgtgccttcttcaccacactgaacgccaccggcggcgtcaacggccggccggtcgaactgcgccaactcgacgacgcctttgaccccgccaagggcgccgagaacgtcaagaccttcgtcaaggagggcgccatcggcatcctcatgcccatcggcacgtcgtcgtcggtcggcgcgctgaaggcggccaacgagctcaagattcccgtggttggcccgtacaccggcgcggcgccggtggtgaagccctccgagtacggctttccgctgcgcatcagctacgacgaggaatacaaccgcatcgtgaaccacctgttcaccatcggcctctctcgcatcggctttgcgcacaacgacaaccccggcgcgcgttcggcgctggaaagcacgcagaagttcgtggccgagcgcggcgagaaactggtcggcagcgtggccatcaagaacgatggctccgacgccgccgaacgcgccgtggaactggccaagctcaagcccaaggcggtggtgctgtcggccaccaacgacgtggcggccaagttcatctcggcctaccgcgccgcgggcggcgagacggccttctactcgttctcgctcctgaacgggcagaagctgttccaggacatcaagaaagacgcggccggcgtggtcatttcgcaggtcgtgccctacccctggaacagcgcgatgccggtgattgccgagtaccaggcagccatgaagaaaatcggcgcgaccgagttcagctatgccagcctggaaggctacgtggcggccaaggtcatggtcgagggactgaagcgcgccggaccgaaccccacgccggactcgctgcacaagggtctcgagtcgttccggacgctcgacatcggcggcattgccgtgtcgtaccggcccggcgaacatcgcggcctgaccttctccgaactgtcgatgctcaaggccgacgggcgctacctgcgctgaggccgctcagcgcccgggcggctgcaccgtgtgcgccaccgcccgcagtgcctgcgagaacgcgcgggccgcgggcgtgagcgaggcgcggtcgcgcatgagcagcgagacatgcgcattgggcagcttgtccgccagccgcaacgcgaccagcccccagcgcgtcgccgaccgcgtgaacagggacgccgaggcgagcgtcagcgcatcggccttgcgcaccagcgtcgcgcccagttgccacgaatggcagatcacgatgtcgcgcggcggcggcatctccagggcagcaaagtttcgtttcagcagctcggcgccgtacggcggcacgacccacatcgccccctgaagcctggccatcgatcgcaaccgtgccagcggatggcccgcacgcgcgatggccgccagcggaaagctgagcagcacttcccggtcgagaccgtcatcggccgcgggctccagctcgccgaggatcgcgaaatcgaaatcgccgcggtcccacagccccttcacgtcggcgccgctgagttcctgcagttcgagcgccacgcccggccactgccgccggaaatccagcagcgccgtcggcagcagctgctcgagcgcgaacgagctgaaggccacgcgcagcaggccgcccgcgcggtcgcgcagctgggcgatctcttcctcggcacggcgcacctcgttggacaggagacgcgcccgccgcaggagcgcatgcccgatctcggtcggcaccacgcccttggcgctgcgcacgagcagctgcgcgcccacgctctgctccagctcgcggatggcgtaggtcatggcgggctgcgtcagcgtggaatcgcgcgccgcggcgcggatgctgccggcctcgacgaccgcttcgaagatcttcagatgccgcaggttcatgaaaaaagcgtggcgagcgagtgatcagatattttgatcgctctggagtttttcggatcttttccttcaccccggctttcgttaaggtgcgccgcggtcctttcacttttccttgcacgagccatcatgaacatccgctccccacttgccctgctggtgctgtccggcagcttgctgaacaccggcgccttcgcccagaccgcagcggacaacggcaatgccctggccacgcgcgcgctcgccctggcggatgcctccgaggcgcaggtgatcgaatggcgccggcacatccaccagcaccccgagctctcctaccaggaggtgcagaccgcggcctacatcgcagccgcactcgcgaagatgcccggcatcgaggtgcagcccggcatcgccaagaccggcatcaaggccgtgctgcgcggcggcaagccggggccggtggtcgccctgcgcgccgacatggacgcactgccggtcgccgagcgcaacgagctgcccttcaggtcgaccgccaaggcgccttggctcaacagcgaggtgccggtgtcgcacgcctgcggccacgacacccatgtcgccatgctgctgggggccgcgcaggcgttctcgaagatgcgtgcggaattgcccggcaccgtcgtgttcctgttccagcccgccgaggaacaaggcccgggccccgtgccgagcggcgcacccgccatggtcaaggccggcgtgctcgacaacccgaaggtcgacgtcgtgatgggccagcacatcaacgcgcgcgccccctcgggcaccatcagctaccgccgcggcggcatcatggccagcggcgacgccttcaagatcacgctcaagggcaagggcggccacggctcgtcgccgtggaccgccaaggagcccatccttgcggctgccgagatcgtgctggcgctgcagaacatcgtgagccaccagatcgacccgctcgacggccccacggtcgtgacggtggggctgctgcaaagcggcaaccgcgtcaacatcctgcccgacaccgcggagatcgccggcaccgtgcgctcgctgtcgcagaagaaccagaaggtcgcgcacgacagcatccgcctgaaggcgcagaagatcgccgagagccacggcctgaccgccgaggtgaccatcgacaccggctacgaggtgctggtgagcgatcccgcggccacgcagtcggtggcgcaggcgctcgaaaccgcggccggggcgggcaaggcgcgcgagtcgcagcccagcatgggctccgaagacttcggctcgttcggcaagaacattcccgtggtgttctggcaactcaacgcctcgccgttcggcgacaagagcggcgcgcccaaccactcgcccgaattcgtgatcgacgagtccacgttgcgggtgggcgttcgcgcgctggtgggcagcacgctcgcctacatgaaccggcccgccgccagcaccggcggcggcaactgagttgctccgtacgccctgaaacggcgaatccggcggcgcggtgatatggtgaacgttccgtgccgccaccccggcggcgcggccgttcgatgacgcccaccggcccgccccctgcgcacctcacccgcgccctgttcctgcggctcctcgcggtgctgccggcgggcgccgttcttccatccttcgcgcaacggcagcccgcccagcccatgcagcagacgaagatgaacactcgccccattccctccacccaggaagccctgcccgtcgtcggctgcggcacctggatcggcttcgaccagcgccccggcaccgacgaatacaagcgcctgcccggcgtgctcgacgctctctttgccgccggtggcaaggtgatcgacagctcgccgatgtacggccgctccgaagaaaccaccggcgagctgctggccgcatcgaagcagcgcgagaacaaggcttttcttgcgaccaaggtttggacctcgggccgcgaagccggcatcgcgcagatggagcagtctttcgcgcggctgcgcaccgagcgcatggacctgatgcaagtgcacaacctgatggactggaaaacccatctcgccacgctgcgcggctggaaggacaaaggccgggtgcgctacatcggcatcacgcactacaccgcgtcggcctacgacgaggtcgaggccgtgctgcgcgccgagaagctggacttcgtgcagatcaactattcactggacgcgcgcgaggccgagcagcgcttgctgccgctcgcggccgagcgcggcgtggcggtgatcgtcaacatgcccttcggcggtggcggcctcctgcgccggctgcgggaccagccgctgcccgcatgggccggcgagatcggctgcgcgagttgggcgcaggtgctgctgaagttcgtgctgagccacccggccgtgacctgcaccatccccggtaccagccgcgccgaacacatggccgacaacgccgcggccggcgcgggctcgtttccggatgcggcgttctggcgcagccatgcgcgctcgatcgggctctgagccgccactgcggcctattcgaacttcacgttgtgttgccgcacggtggcgccgaaggcttcgtactgcgcgcggaagaactcggcgaacttcgcggggctcatgccgtagccctcgaagccctgctgcaccagctgcgcatgcacgtcgggccgcttcagcgtgttctgcagctcctgcgagagcttgtcggtgatggcctgcggcagccccggcggcccgaagaagccggcccacggcgtgatggtgagcttgcccaaccccaactcgctgcccgtgggcacgtcgggcagcaaggcgctgcgctgcggcagcagcgtgaccagcgcgcggatgcgcccttccttcacgaagcccggcgccagcgtgccggtggtgaacatcatgtggatctgcccgcccagcaggtcggtcatggcctgcatgtcgcccttgtagcgcgcgttgaccaccttgcgctcgcccagcagctgcagcatggccagctccgaggcgctgttgctcgatgccgagttgtaggtgccgggcttggccgccaccatggccagcaactcgctcacgctcttcaccggcaggctggccggcactaccaggaacatcgagaactggccggccgagctgatcggcgtgaaggccttgaatgggtcgtagggcggtgtcggccgcagcgtgggcgcggccaccatcgcggtgttggtgcccatcagcagcgtgtagccgtccggctttgcggacgacgtggcctgtgccgccagcacgccatcggcgccgggtcggttctccacgatcacctgctggccgagctgcttcgacagcccctccgcgatgatgcgcgtgagcgcgtcggcgccgccgccggccgcaaagcccacgatcaggcgcagcggcttttccggataggttgcggcactccaggccgccgcgccgggcagcgctgccagcgtgccgccggccgcgagggccgccagggtgatgaggtttctgcgtcgcatgtcgttgctccttctcaaaagagatgccgcacaccaagctcccagcccgacgagcgacgtccgcctgccggtgccacgccgccgctgacgacgtagcgcgcctggccgccgttcatgagccgcgcataggtgccgtagagcgcggtgcgcttcgagaggttgtgcacatagccgatgccgaactggcgcgcatcgtcgcggttgcgcggcatgccgttggcgttgcgcaggctctcgtcgctgcggtcgtccagataggcgtagctcaaccggatgcggccgacctcgaaggccggaatgtgcgcgccgatctcggcggtgttcttgcgcaccgtgccggcggcgagcttcaccgtgaccttgttgtagagcgcgaagaacttcgcaaagcccgcatcccacgagccgccgatgttggcgtgcgtgtagttgccgatggcggcggtggcgttgaagtgcgtgcgcgtgacggccgccgcgatgtcgaatgcgcccgaggcaaagccgaagcgcgcgccggcaaagttgccgtcgtcgcggttcggcgcggtggagtcgttctccccggtgccgatcatcgccatgccgtagaagccgccgagcccggccggcagccagtagctcacggtgttgctgccggtgatggccgtgggcaatggcccggtgcccgcgcccgcgaacgtgaggttgcccgcgcgcgccacgccgttggcgttgaagggatcgaagtagatgctgttgtagtgcgtcgggatgaagtcgcggcccaggcgcagctcgccgaacctctggtgcgacaggctcacgaaggacatgcggtcgaaggtgatcggccccgccgtgcccgcgccgctcgcctggttgttgctgttgctcggccggccggtaccggtgtcggggttcaggctgccctcgagccagaagcccgcgcgcaggccgccgcccaggtcttcggtgccgcggaatccgagccggctggtcgagagcccgccgttggacagcgcttttaccgagccgccgccatcgccgttggtgtactggatgccgaggtccgtcaccccgaacacggtgacgctggactgcgcatgcgccgcgccgctgcttgcaagccccagcgccagcgccggccccatcaaaattttcttcatggtttcttgtctcctgcttcttctcttggttaaaaactcgggaacgcgcgcagggctgcgccaccgggtgcggacgagggtccgcaccggttggcgaaaaccggcgtgaaaaaggtcttagctcgaaggctcgggtcgttcggtgcgcacgagcacggcgcccttcgacagcgggctcacgttgcgccggtactgctgcagccaaccggtgtcgaaggccggcggcggtgcctgccagtcggcgcggcgcgcatggagttcggcatcggtcagcgcaacgtcgaggcggcgctggtcgaggtcgatggtgatcacgtcgccgtcgcgcaccagcccgagcggcccgccgagcgcggcttcgggcgacacctcggccaccaccagccccttgcagaccaggcccgagaggtgtccgtcggtcaggatcgcgacctggtcgcccagacccgcgccgtcgatggcaaacaccacgcgcgaggcgccgccgcccatggccgggccgccgcaggctccggcgccgcgcatcacgaccacctggcccggcacgatctcgcccttcttcagcgccgcgatggccgcgtccgaggtccagaagcacaccgccggtcccgtgaagctgcgcaccttgcgcggggcgatgccggtcttgatcaggcccgattcgggcgcgaggttgccgcgcagcagcacgatggcgggatgcggcgccaccgggcggtcgatggggcggatcacctcggcgtcggcgacttcggcgccgcgcaggttgtcggccaccgcagcgcccgtgacggtgagcgcgccggtgtcgagcaagggtgcaagctgcttcatgagcgcgcggcaaccgcctgccgcctcgaaggcttcgatgctgtgctcgccgatcggccgcacgccggccagcaccggcgtcgtggggccgaggctttcgaagaggccgtacacatcgacaccgcactcgccttcggtcgacaccgcctgcaggtgcttggccgtgttgagcgagccgccgacggacagcaccgcgcgcaccgcgttggcaaaggcgccgggcgtgaggatgtcgcgcggcttcaggtcgtcccacaccatctgcacgatgcgcgtacccgcggcgcgcacatcggccatcatcttcggactcagcgccgccaccggcgcgctgcccggcagggccatgccgagcgcttcgcagacgatgtgcatcgagttggccgtacccaggcccgaacacacgcccggcccgcggatcgcctcgcggctcatgcccacgagctcttccaccggcagcttgccggtgaccgcatgcatcgcgccgatgaacacctcttcgatgtccatgtgccggccgcggtactcgccgctgggctggtagccgcagggcacgagcagagtcggaatgttgagccgcgccgccgccatgagctggcccggcacggtcttgtcgcacgaagtgaggcaaaccatgccgtcgagctgcgcgccttccacggccacctcgatgtcgttggtcaccaggtcgcgcgcacccagcatgtaggcgccgcgcgcacccgcgccggtgatgaagtcgctgggcgctgcggtgcgaatctcgaagggcacgccgccggcggcgcggatcgcggccttcacctccaccgccacgcggtccaggtggctgaagcaggccgcgagttccgaggagctgttgacgatggcgatcttcggcttctcgcagtcttcctcgggaatgccgagcgcgcgccagtgcgcgttgcgcaccgaccagagataggagccgcgcggaaagttgctgcgcagggggcgggtcatggacggtctccggatttcttcttggtgatttcgatcaggccgcggtcggcgtccacgcgcacccagtcgccggtctctatgcattcgagcgggtcgcgttcgaaatcggtcatcgatggcgagtgcgtgaccacggcgccgagcgccatcttggtcgtcatctcgttgaacagaaatgccgccggcgccgagttcatgagccgcgtcatgtggaacatggccgaccatcccgacgagcccttggcccccggaaacaccagcaccttgcccgcgaagctttggccacgcagctcgtgccgcgtctcgatgacggtgccggtacgcggatcgatgccgccccagcccgagatgcggtcgcgcgtgacgagtgcttcgccttcggcaataccgccgaccaccttgcggccgcggatgaccagagtggatgtgtgtgcgatcgcgctcatggtttttctccttcccccgctggggctgagggctgcggctccagttccgcctgcgcggaactggacagcccgaagagcggcagcctctggctgcctgcaccgaggtcgggatgggggcgggcagagcgcgcgatggatgcgccgcatgcccccacccctgccctcccccagagggggagggagaaagacaacgcaagcgtgaagctcattgcatgcctccattccatcgcccggtgcacgccgcatcgacgcattccgccgtgctgccgaaccacgcctgcacaccgagaatcgcgggcaggtagtgcgcctgcttggccgagtcgagcgccacggtcctggtgcccttgggcacggcgcggctcatggcggagcagctgtcggtcatgaggatgccgcccgcgtcctcgatgatcttcgtgtagccgttgcggtcggccagcgacttgatggcgcgcggcgtgaagatccacagctcgcaatccgggtgtaccttgcggccttcgatgagctgcgcggcctcccagatctgctcgatggtgtagtgcgggcagcccagcatcacgtactgcacctcggcgtcttttccggtggcgttgatcttctcgtaggtggcgcggcgctcggcctcgccaaagcgcagcacctcgaccggcgtccttccgccgagcgcctgctccagcgtcagcgcctcgggcgtgatgccggcgatgtggtacatctccacgccgcccgacgacgaggccgccgcgccgaagtgcttgagcctcggcaaattcggcacgcgggcgatgccgcgtcggctgtgcaccaccggcacgcgctcctgcacatgctcgccgatgtagtagccgagcaggccccagtcctgcaccgattccacttcgacgtcgagctcgaccacgtgcgtggcatggcggttctcgtcgaggtgatagccccagtacggaatgcggcccgtgagcatcgccgcgcccgtgctctcgcggccctcggtgttggtgcgcgcgcccagcaccgagttgcaataaacgaccgccgacgattccatccacgcgcagtgctcgccgcgcgtcgggatgttgcccacctggtagggcgtgcaggtgttcatgatctgcgcgccgaggccggccgcatggcgctcgctcttgttgtagaactgcacgatctcctcgctcacgcccatgcgctcgggctggccggggtcgaagcccagctgcaggtggctcgtgaagaccttgaacttcggaatctcgacggtctcctggctgtcgagactgaactcggagaacaccgcgtccatgccgccgcccttggcgagcgcgaagtcgcgctggaaaggcgtggtcgaggtgatggtggcgcagacgttgcgcgtctccaccagccgctcggcgcccagcgcttcgccgtaccgcatcaggaggtccatcgccttctgcacggccggtccgccctggccgtccatcatggctttttcttcatcgctcaggtgcatgacctgtgtctccgttcttgtgctgtcggtggggtcggccgggctagcccggcaagggggtcggcacgtggccgccgatgtcgcgcgcgatggtgagcgcgatgtcgtgcaggcgcggtgcgagttcgttgcgcaggcgctcctcggtgaacacgaaggcggcgccgccgccgttcagcgccatcacttcgccgtcgggcccgatgaggggcacggacaccgagttgatttcacggtggaattcgccgagcgagaggcagtagcccagccgcctggcttcgccgatggcgcgcgtcatgccgggcgcgatgctgtcccactcggggccgcgcaagaggcgcatcgagtcgatcagctggttgcgctgcgcctccggcagtgccgaaaggtacgcgcggcccagggccgaattggccagcggcgcacgcgagcccacgtcgagccgcgccgagagcatcgacgagcgcggccggcaggcttcgatcagcaccatctccatgccgtcgcgtatcgccaggtagaccgaggcacccacctcctccgccatcgcctgcatgctgggccgcgcggcggcccgcacgtcgaggctgccgaggaacacgcgcgagagcgacaccacgccgggcccgagcatgaagcggtcggcaagctgcgcggccttgagcatgcccaacgagagtagcgtggcgacgagccggttgaccgtggggcgcggaatgccggtcatgcgtgcgatgtcggcatggcccagcacgggacgctcttcgctgaagcagcgcaacaccgagatgccgcgctccagcgcgctcacggtgtcggagcggtcgccgcgcgtgtcggcggcttcggaggcgggaaacaaggtgtcgtttttgtcagtggacatggaggaaccctttggaagacgctccaatgtagaggctctcgaaaggaggctggccgggttcatggcaagccgttcaggcactggcttcggccgtggccggcgcatgcgtgccctgcccggcgccggcgcgcaggtacacgccctgagccagcaacgccgactgcagcgcgcccacatcgacgaagcgcggcgcgatgccgccttgcgacgccagcgccgccgccacgcccgcggcctggccggtgatccagcattgtggaatctcgcgcatgaagccgtgcgaattgcggtcgcacgagatgtggcgcccgcaggccaggagcccgtcgagctgctgcggcaccagcgcgccgtagggaatggagatgttcggaaatttcggcgacaccgccggcgtcacgcccacctcgtcggccagcgccacgccgtcgggccactggctgcgcagcaccgcgcccacgccggtgagccgccgcgcatggcgcacgccgatctgcggtgcgctcagcatcaggtaggcgtcctcgaagccgggcgcatgagcccggaagtagtcgaggtgcgcggccatcgcgcggtgcgagcgcacttccacggcggtgaggtcgtccacgtcgagcgccgaatagcccgactggcgcggccccatgaacagcgccacgtcgttgcgccacgagacgaagggccgctcgaacaggccgcattgctcgcggccgcccgccatgaaggcggtgaaggcctcgggctggccggccttgaattcgatccagcggttcatgtccacgccgccgaacagccacgaagtgttcatgcagtggtgcacgtcggcctcctcgatgtcgttcacgtaggccgcaccggcgcgcgcgaacaggtcgccgtcgccggtggcgtcgaccaccacgtcggccatgatggccatgcggccctccttgctctcgaacaccacgcctttcaccgcgccgtcctgcacgatgggaatggccgcccacgagtgatagatgagcttgaccttgcgctccagcacgatctcctgcgacaagagcttgagccgctcggggtcgatggtgggcgaccaggtgaccacgccgtggtacgcggccgtgcgctgcgaccagtgcgcggccttggccgcgtcctgcgaaccccagtcttcgcgcgccgggccggcgatggcgtcggcgggcaggcgatcgaacaactcttgggcaaagccgcggatcacgagcttgccttcccagtcggtcatgcggtcgatccagatcacgaggccgccggtggaaagcccacccaggtggttgtagcgctcgagcagcgccacgtcggcgcccgcgcgggccgcagcggctgcggccgccgtgcccgaaggaccgccgccgaccaccagcacgccgcagcggtggtagaccggaatgctcttgccgggctcggcccaggtgccgtggtcagggcgcttgacgcggctgtcgcggtcgaagatgtcggaggacaggatgcgctcgtcggtgcggacgacagttttcatggatgagtgtcttggatggcttgtttcttcgtattttgatttcaatgttcattttgtcaaacacaaaagtcgcaaagaggcacttcttcggggtattccctagagtgtgtggatttttatgattttctaaatcaatataagaagaacatttccaacggagacatcgatgaagaaaccctgcggcacccgccgtgcgtttggcgcggcgctcggcgcggcggcccttctgggcttggcgcccccggccctggcgcaagactttcccgtgcgcggcggcaagccgatccgcatcgtggtgggcttcacggccggcggcggcaccgacgcgcaggcgcgcatcgtggcgcagaagctcggcgaggtgctgggcaccggcgtgatcgtcgacaacaagcccggtgccagcaccatgctcgcggcaagcgaggtggcgcgcgcgctgcccgacggctacaccctgctctacgcgccctcgtcgaccatggcgcagaacccgcacaccttctcccaggtgccctacgaccccttcaaggacttcaccgccatttcgatgggcgggcgcgggccgctggtgctgtctgtgagcaccaccgtgcccgccagcaacgtgaaggagctcgtcgcctacgtgaaggccaaccccggcaaggtgagctatgcgtcgttcggcgcgggcacttcatcgcacatctacggcgaggccttcgtgaaaaaggccggcatcgacgcggtgcacattccgtacaagggcggctcggacgcggcaaaagatctgatcggcggccgcgtgcagtacatgttcgattcggcctcgtcggccgtcatcacctccgggaccggcaaggtgaagatcctggccatcgcagcgaacgcgcgcattgccgcgctgcccgacgtgccgaccttcgcggaacaaggcgtgacggggctcgacctgccgagctggctcggcttctacgggccggcgcacatgcccgcgccagtggttgccaagctcaacgccgcgctggcgcaggtgctggcgatgccgcaggtgcgcgacttctaccgcagcggcggctatgaagccggggccagcacgcccgaggagtttgccggcatcacgcgttcgagctacgagcgctggggcgccatggtgcagcaggtcggcctggccaggcaatgaaccgtttgccttcctccatcgcccgtcggcgtgctgccgcgtggctcgggctcgggttcgcatttggcgcggccgcatggccgctggccgcgctcgccgccgggcccgcgccgctccccgagaagggacgcagcatccgcatcgtgctcggcctcgcggcgggcggcgcctcggatgcgcaggcgcgcttcgtcgccaacaagctcggcgaggtgctgcagacgccggtgatcgtcgagaaccggccgggcgcgagcttcatccttgccacggaagaagtgattcgcgccgcgcccgacggctacaccttcatgtacgcgccctcttccgtggtggcgcagaacccgcagacgctggcgcaggtgcgatacgacccgttcaaggacctcacgcccatctcgctcggcgcgcgcgggccgctggtactgacggtgcacgccagcgtgccggcgcgcaacgtgcgggagctggtggcccacatcaaggccaaccccggaaagatgagctatgcctccttcggcaccggcacctcgtcgcacatctacggcgaggcctttgcacaacaggcggggctggacgtggtgcatgtgccgtacaagggcggcgccgatgccgcgaaggattttctcgcgggccgcgtgcagtactacttcgatgcggcgcccaacgccatccagaacaccgccaccggcaaggtccgcatgctggcggtggcggcgccgaaacgcagcgcgatgctgcccgacgtgcccacgatgaccgaacaaggcgtgagcggcgtcgacatgccgagctggctgggcttctacgggcccgcgcgcatgcctgcgccggtcgtcgccaggctcaacggcgcgctcgcagaggtgctggcgatgcccgccacgcgcgacttcttccgccagggcgcctatgaggcggagtcgtcgagccccgcgcaactggccgagctcacgcgtgcaacctacgaccagtggggcgacatgatccgaaagctggggctggcgaagcaatagcgaggctcgaggctcgaggctcgaggttcgaggctcaggccaggaagcgcagcagccgccgattgaattcttcggcgcgctcgtactgcgcccaatgccctgccccgtcgatcaccacgccttcgcgctgcggatggccggccgtgagctgtgccaccagcggcctcggatcggcggtgacgtcgtactcgccccacagcagcaattgcggtccgccgagcgtatcgagcgcggcctgcagcccgcccgcctgcgagacgtccttgctgcgaaagcgcgtgccgtggcaggagatgtcgtgaatctcgaaggccagcaggtcgatggcggccttgtcgtgcagcatgagcgcggccaggttgtgcagcagcgcggcgcgttcttcttcgcggctcggcgcggcacgccagttgctcatctccaccgacatgcgccgcattgtgccgtggcctccgctgcccacgagcgccaggcgccggatggcgccgcgccgcaccgcaaagcgcgcggcggtgagtccgccgaaggagaagccgccaagatcgatgggcgtgcccacgccgatcagctgatcgagcgatccgcccagcgcgtcgagcagcggcccgagcggatcgtcgccgggcgctgcgcgcggcggcgcatcggaatcgttgaagcccggcatgtcgggcagccacagcgaatgttcggccgacagcgcctcgacgttgcgcagccagtgcatccagctgccatggccgccgtgcagcagcaccagcggcggctgggcgcttttttcagcaccgaagcggcgccagcaaacgcgaacgccgccgtgcaccacgtcatggcgcgtgccgctcgcggcaatgcgttcgatgagcaggcgggcttcggtatctgaactcgacgttgaatctgaatcgggaatggaaggcatcgcccgattctgccaacccgccgccttttcagctggcggcagcgccgaagcggtagctcgacaccaccagcccgcccatgaaatcgtcttcgtgatagacgcgttcgccgggctcctgctcggccgcgccgacggccaccatcagcggaatgaggtgttcctcgcgcggatgcgccatgcgcgccgaaggggccgaggcccactcctgcagccgctgcgcgcgcgcctgcggtgccgcttgcacggcggtgtcgtcgagccagtcgccgaaggccttcgacacgccatgcgcctgcggcccgaagttgcgcaggttgtgatagctgaggccgctgcccacgatgagcacgttctcgtcccgcagcggcgcgagcgcgcggccgagcgccaggtgctccgccggatcgagaccgcgcttgagcgacagctgcaccaccggcacgctggcgtcggggtacatcgccttcatgggcgagaacatgccgtggtcgaagccgcgttcgggatcgatggccgcgggcagcccggcggcggcaagaagcgactgcacgcgctgcgccagttcgggcgagccgggcgcgtcgtagcgcacttcatacgtgtgggcgggaaagccgccgtagtcgtagatcatgggcgggcgcgggttgccctgcaccgtgaagaccggcgcctcccaatgggccgacaccatgaggatggccttgggcgtgcggccgatctggcgcggcatgtcggccagcgccacggccagccggtcgtagaccccgcccatctccttttgcatccagggccagggaccgccgccatgggagatgaaatacgtgggcaggcgcgaggtgttgtcgtcgtgggtcaagtcgatgctccttgaaagcgttgcatcgactgtagacatttcctggaaagaaatcgacaggctaggatgcatcgattcatttctccacaggaaatcttccatggaccgcctgaccagcctgcgcgtgtttcgagaggtcgtcgaatcgggcagcttcgtggccgcggcggagcgcctgtcgatgtcgccgccaatggccagcaagcacgtggcgcagctcgaaaaatcgctcggcgcgcggctgctgcaccgctcgagccgccacttgagcctgaccgaagcgggcaccgcctggtacgggcagagccggcgcgcgctcgacctgctcgatgccgccgaggcggccatcggccagaagagcgaggcgccgcgcggccagctcaaggtgagcgcgccggtgtggtgtgccacgccgcgcttcgcgcgcgtgctggccgactaccgcgagcgctttcccgaagtgctgatcgacattcacctggagaaccgcaaggtcgacctcgcagccgacggctacgacctcgcgctgcgcgccacgcaggagccctccccggcgctcatcgcgcggccgctgtgccgcgtgccctttcatctggcgggcacgcccgcctacctgcgccgcatgggcagccccacgctgccggccgacgtgggacggctcggcgccatcgtgccgagctacgtgaacctcgacaacctctcgctcaagggaccgggcgggcggatgtttccgctgcggctcacgcccgcgatgcgttcggacgacaccacgctcaccttgcacgcggtgcgcgcggacatgggcattgcgttcttgcccgaatggctgatcgacgacgacctggaagagggccggctggtgcggctcttgcccgaccacgccccgcatccggtcacgctgtttgcggtgtacaccagccgccagtacatggcgcccaagctgcgcagcttcatcgactttctcggcgagcggctgggcggccagccaccggccgccgcgaaacgcaccctttcggggcaaggacatgccagcccgggctaaagtcgccaatccgcctggagatcgcccgccttgttccgcttcttcgaaaaactgcttcacccctaccccgccgccgaaccggcgccgccaccgacgggtttcttcgccttcctgtgggcctgcacccagggcctgcgtctcaagatgggcgtcatggcggcgctcactgccgccatctcgaccttcgaggcgctgctgttcgcggtgctcggccgcatcgtcgactggctcggcggccaggtgccgtcgaaactgtgggcggagcgcggcgacacgctgttgtggctggccgcgctgctggtgatcagcatcggcgtggtggcgctgcagaccatcgtcaagcaccagacgctggcggtgaacctgccgatgcgcctgcgctggaactttcaccgggtgatgctgggccagagcatggccttctaccaggacgagttcgcgggccgcatcaccgccaaggtgatgcagaccgcgctcgcggtgcgcgacaccctcttcgtgctggccgacgtggtggtggccatgggcgtgtacgtggtgaccatcatcgtgctggtgagcgtgctcgatgcgcagctggtgctgccgttcatcgtctggctcgtgctctatgcagtgtcgctgatgtacttcgtgccgcggctgggcaaggtgggcaaggcgcaggccgatgcgcgcgcgctgatgaccggccgcgtgaccgacgcctacaccaacattgccaccgtcaagctgttctcgcacacgcagcgcgaggccggctttgcgcgcgaggcgatgcgcgagttcatgtacacgggctacgggcagatgcggctggtgagcgctttcgagatcgtcaaccacacgctcagcatgggcctgaccgcgggcatggccggcaccgcgctgtggctctggtcgaacggcacggtgggcgtgggcgcggtggccgcggccaccgcgatggcgctgcgtctgcagggcatgtcgcactggatcatgtgggagatgaccagcctgttcgagaacatcggcaccgtgcaggacggcatgaagacgctgtcgcgcccgcgcaccgtgctcgacacgcccgatgccggcgtgctcgaagtgccgcgcggcgaggtgcgcttcgagcacgcgagcttccgctatgcggatgcgggccgccgcgtcatcgacgacctgaacctggtggtgcggcccggcgaaaagatcggcctggtcggccgctcgggcgcgggcaagtcgacgctggtcaacctgctgctgcgctttcatgacctggagagtggccgcatcctgatcgatgggcgcgacatcgcccacgtgacgcaggattcgctgcgcagccacatcggcatggtgacgcaggacacctcgctcatgcaccgctcggtggccgacaacatcgcctatggccggcccgacgccacacaggcgcagatcgaagcggccgccaagcgcgccgaagcgcacgacttcatccagacgctgggcgacgccagcggccggcatggctaccaagcgcatgtgggcgaacgaggcgtcaagctctcgggcggacagcgccagcgcgtggccattgcgcgcgtgatgctcaaggacgcgccgatcctgctgctcgacgaggccaccagcgcgctcgactccgaggtggaggccgccatccagcagagcctctaccggctgatggaaggcaaaaccgtgatcgccatcgcgcaccgcctgtcgaccatcgccgcgatggaccggctcatcgtgctcgacgaaggccgcgtggtggaagaaggcgaccaccgctcgctgatggcgcaaggcgggctctatgcacggctgtgggcacaccagagcggcggctttctgggcgattcgctcgaagaagacgaggcgctgcgggcttgagcgcagcctagggcctgttcacactactaacggagtcgcgaaggcatgccaaagcggacaaatcaaggcgcacgacgatgcgtgtgcgtcggcacacgcaaggagtgcaacgcggagttggccgctttggcatgccttcccttcgggttgttcggcaaaggggccgtctgcggcgttgcccgcgcttgcaaggcgcaagccttgctgcgcacgggcgccttgcagccagcccctttgccgaacaacgcgatctccgttagtagtgtgaacaggccctagttgggcaatgcgccggcctcgtacgacgctgcgaactccgcgctcggcggaatcggcttgacgatgtcgatcagcacaccgttcgggtcgctggtaatgaagtgacgctgaccgaagtcctcgttgcgcagtgcaagaagaatcggcagcccggccgccgcgaggcggtcgtgaatcgcgtcggggtcgtccacctcgaaattgagcagcatgccgcccaccacctgaccgcgcgcggatgcgggaatcgtctcgtgccggccgtccagcacggcgaggttcaccgcggagtcgcccgccagctgcaaatgcacgtaccaatcgctcgtgaacagtggcgtgaatccgaaatgcgcctgatagaagctggctgttgcggccacgtcgttggtcatgatcaccgggtagtagctcgtcactttcatggtgtcggtcctttcaattaacatacagactgcatgtaagtcagatattaatctacagacagcctgtatgtaaatgccaaaatcagtcgccccctctccgtccagaaccaaccgcgaacgcacggaaaccacccgccttgcgctgatcgacgcggcgcgcgccctgttcgtcagcaagggctatggcgaaacctcgacgcccgagattgccgttgccgccggcatcacccgtggcgccctgtatcaccacttcgtggacaagcgcgatctgttcaggcaggcgctggtgcgcgaggccgaagccgtggcggcagacatcgaagcggccgcgccccggcaactcacgccgcgcgaagcgctgctcgagggcagcaaggcttacctgaagaccatgaccgcgccgggccgcacgcggctgctgctcatcgagggccccgccgtgctgggcctcgcggaaatcatggccatcgaccaagccacctcggccaactcgctacgccaggggctggaaaaagccaaggtcggcaaggacgaggtttcgctcgacgcgctcgcccggctactttcggcggccttcgaccgggcggcgctggagatcgatgcgggcgccaatgcggaagaagttggctccgcgatgcgctggctgcttgaaaaggcgctgggcccggcaccgagtcgcaaggccgctccctgaggcgatgccggcacggcgcaggcgctcgcccgggtcttcgcgagtcctacagcacaggccgcccctcgccgacagcaaccggattccctgggcgcgatgctgaagctgtcgtcaacaacgaggagtcctcgcgtgaattccatcatttacatcgtcggtctggtcgtggtggtcgtggccgtgctttcgttcttcggcctgcgctgagcccagccactcccccaggcttcgcgcacttcgtgtcgcttctccttccccctcgccgggggcaacaccagcggcccggcaaagccggttccgcggtgttccacgaaagggatcggtcgcagtcccttttcccgtcgttctcatagagtccttcgcagggcgccgggcataattcgcgcgccccgctcatcgcggagcgccacttgcgaagggaccctgttgaccaacaccgcgttgcgcgaatctgcttttccggacgcggtcatcaccgaggcgatccgatggaccgaggagaaaggtccactcgacgatgcgcaggccatgcgcatcgccgcctcgcgcacacctgacgaacactcacgcatcacggcgcgcgcgcttcagctgggcgaacgcatcgggctgcaatccgaactggcgcgcacgcgccaatggggcccgtgggtgctgcttggcctggtcgcgctcgtcgtcattgccggcctggggctcgcgggcaacgtggtcggcggcggcgaacggcacatcaacgtgatcgtcgcgctcgtgagcctgctgggcattcacctgctcacgctgctgttctggctggtcggcttctggctgccgctcggttccttcaacaccagctcgctcggctggatctggctgtcgctcactgcacgtgtcgccggcggcaagcgcggccaggcaccggtgctggtgcgcgccgccaccgggctcttgacgcgcgccaggctgctgccctgggccttcgggctcgtgagccacggcatctggtcgctctcttttgcggtggtgctggccgcgctgctgttcgcgctggcattccgcagctacacgctgaactgggaaacgacgatcctcgacccgacctttttcgtgcgcgccgtgcaggtgctgggctgggccccggcgcagatgggctttcgggttcccgatgcacaggccgtgctctcggccactcccggcgccgcgggccagcgcgcgtgggcgctgtggctcaccggctgcatcgtcgtgtacggactgctgccgcggcttgcgctcgtgttgctgagcgccgtggtgtggcaccggcgccgggctgcgctccagcccgactggagcgagccctactaccgcaagctgaaggcgcgctttgccgcgctggcgccacccgccatcgtcgatgccgatccgggacgggcaccgggcatcgcgcctgacgggctggcgccttcggacctgcaggacaccctgttcgtcgtcggcttcgaactgcctccggatgcgccatggccgcccgagggcctgcacgccgatgcgaccaccgagatgcagcacatcgacggcagcgcactcgcacgccgcgcccttctcgaccggctggcagaggcccgcccgcgtgccgtgctgctcgtgtgccatgcggcatcgagccccgaccgcggtaccgaacgcttcctgcgcgacctgctggcccattgcggcgaatgccgactgtggctggccacttcggcgggcacttccgcgaacagcacagcggacgccgccgcatcgcaacgctggatcgactggctgcagggcaccggcctgccgcgcgttgcggccacgcaccaactcgaagatgccttgcagggccttggcgccacaccatgacgacacagcacgccatccgcatcgccgttgtcggccacaccaacgcgggcaagacctcattgctgcgcacgctgacgcggcgggccagcttcggcgaagtgtcgcagcgccccggcaccacgcgccacgtggagtcggtcgatctcgaagtgaacggccagccggcggtgcgcttcttcgacacgccggggctcgaagacgcggtggcgcttcgcgagcacctggcgggcctggacccgcaggccacgccgcccgagcgcatccggctgttcctgcagggccccgaagcccacggcgtgttcgagcaggaggccaaggtgctgcgcaccatgctcgacatcgatgcggcgtttctcgtcatcgacgtgcgcgagccggtgctgcccaagttccgcgacgagatcgagctgctcaactcctgcgcccggcccgtgatgccggtgctgaacttcgtgcgcgacgcggccagccgcgagccggcctggaaagaactgctgtcggcctacggcctgcacgtgcaggtgagcttcgatgccgcagcgcctttcgtgggggcggagcgcgagttgtacaacgatctctccaccctgctgcgcgaccggcgcgaactgctgcgcggcgtggtggattcattgaccgccgaggccgccgaacgccgccgcgcggcctgcacgcgcattgccgggctgctgatcgacgccgccgcgttgcgccgcagcatgccggccgaagagttcgccgacacggcgcgccggaaggcgttcgtcgcggcgctgcagaaggaggtattcgacaaggcgcagcgctgcaccgacgacctgctcgcgctctacggcttccgccagaacgatgccggcgaggcgccgctgccgctcatcgaaggccgctggacgctggacttcttcagcccggaagccatgaaggaagcgggcctgcggctcggcaagggcgcggtcatcggcgcggccgtgggcgtagtggcggacctggcggtggccggcatttcgctcggcaccggtgccgcggtgggcggcgccatcggcggcgcggtgtcgcagggctggggtcccttcgggcgcaagctggcgaacaggctgcgcaatgtgcacgagctcacggtggaagacggcgtgctctttgcgctggtggcatggcagctgaaactcgcgcgggcactggagcggcgcgggcatgcggccaccgggcgcatcgcagccgagacgagcgcgacgcaggacgcgccaacgcgcgccacggccgccgccgtgcgcgcggcacggcccgcgcgcagccatccggagtgggagtcggccggggtggcagcgcggaccttctggcgccccgcgccgcagcgcgatgcgctcgcggccgatatcgcgcgcacgctgcaggacgccttcgaggcctgagcaccgcggcgttcggcgttcgcgggtcgcgcacgcaggcccgggctgcggtcaccgcgccgtcatgaggcaaacctagcatccgctggcctttgccctccataaccaagactgcactcccgactcgatgtaccccggcgaacggctcaacggctacacccatctgctcggcctgttgctctctctgttggccacggccctgctgcttgccaagaccgtgcccaccggcgaccccgcccggattgccggcgcgctggtgttctcgctctccgcggtggtgctgtatgcggcgtccacgctgttccacagcacacgcgggcgccggaagcgcttctgggaacgggccgatcactgcgccatctatctgctgatcgggggtacctacactccgttcgcactggtcacgctgcatggcttgtggggctggctgctccttgccgccgtatggagcgccgcgctcttcggcatttgccgcgagttgctgcaggccgacggcgcagcatccaagcctccgctggcgctctacatcggcatgggctggctcggcgtgctggccgcagtgccgctggccgcgcggctggaaagcggcggcctggcctggctgctggccggcagcgtgctctacaccgtgggcacggtgttctaccggaaccggcggggcttcaggcatgcgcatggcacctggcacctgttcgtgcttgcgggcaccgcgagccacttcgtgtccgtgggctgcttcgtgctctgacggcagtcagccggcccgcgctttcaagggatgcaggcacgtgttgccgtatctcccaaggcaatacgtcccaagagatgtgcaaaatgcgcccatgccaaatatcgcctccatcctcaaagccgagatttcccgtgttgcccgcaaggaggtgcgcacagagatcgaaacgctgaaaaaagcatccacgctccatcgtgcttccatcgccgcattgcgccggcaggtcgaaaaactggaaaaggaactgcggcgcgccaccaaggtgtccgcgcgcgtctcccccggcgccgatgccgacgaagcaggcgactcgggaccggcgcgccgcttcagcgccagccgcctggccacgcaccgcgagaagctcggcctttcggctgccgcctatggcaagctggtgggtgttaccggccagaccatctacaaatgggaacagggcaaggcccgtccccgcaaggcgcagctcgaaggcctggcatcggtgcgcggactgcggccgcgtgaagcggcggagcaactgggcgcggactgaaagcgctccaggccccgcattcccccatgtccaacctcatcgtgcacggcggcacgccgcttcgcggccgcatcaccccttccgccaacaagaacgccgtgctgcccgtgctgtgcgccacgctgctcacgaacgagccgctgcgcctctatggcgtgccggacatcaccgacgtacgcaagatcctcgacatctttcgcagcctgggcagcgaggcgcgcatggaccacgccaccggcacgctcgatctgcaccaccgcgaaacggctttcgacgccgcgcgcgaccgcctgccggaggaaatgcgctcgtcgatcatgctggtgcccccgctgctcgcgcgctttggtattgcgcggctcgaggacaacgtcaagggctgcacgctgggggtgcgcgagatcgatccccatgtggacgtgttccgccgcttcggcggccaggtggaacgcgccagcggttcgctcctggttcggtgcgacggaccgctgacacccaccgagcactggctcgactacgcctccgtcacgacgaccgagaacttcgtgctgtgcgctgcggcggccaaaggcacctccacgctcaccaacgcggcgtccgagccgcacgtgcaggagttctgccgcttcatggtcatgctgggcgtgcgcatcgaaggcatcggcacctcgcggctcacggtgcatggcggcaatgccttgcgcggcggggagtttcgcttcgacgaagacttccacgagatcaccaccttcctggcgctgggcgccatcacgggcggcgacgtggtcgtgcgcaacagcgcgcccgagaattttccgctgatcgaccgcaccttcgccaagttcggcgtcaccatcgcgcacgaagacggctggtcgcgcgccagctgcgccggtccgctgaaggtgcagacgcccttcaccagcaacgtgctcaccaaggtggaggccgcgccctggccctactttccggtcgacctgcttcccatcttcattgcgctgggcgtgcgtgccgagggcaatgcgatgttctggaacaaggtctacgacggcgccctgggatggaccggcgaactgtcgaagttcggcgcccacgttttttcctcggatccgcaccggctcatcagcttcggcggcagcccgctcacgccggccgtggtcgagagcccctacatcatccgggtggcgattgcgctcttcatggtggcggccagcatcgaaggccgctccgaaatccgcaacgccacgcccatccgccgggctcacccccgcttcgccgagaacctgcgcagcctgggcgcgcaggtggagtggacgagcgaagagtaggcgccgccgggctcaggcccgcagcgccttcgcgatgatgcgcgccgccgatgcgattacatcgttgcggtattccgcatccttgcgtgtcggaaacgtcaggtacaccgccagcaccagcggcgcgccggccggcggccacagcacgcccgtgtcgttcacggtgccgtacgagcccgcgccggtcttgtcgcccaccttccagtcggccggcacgccggcgcgaatgcgcgtggcgccggtggtgttgcccagcagccaggtttcgagctggctgcgtttcgctgcaccaagcgcgtcgcccagcaccagccgctgcaggcttgcggccatggcctcgggcgtggtggtgtcgcgcggatcgcccggaatggcgctgttgagttcggtctcccagcgatcgagcctgaaggcctggtcgccgatggagcgcgcgtattcagtgaccgccgatggcccgccgagaattttcatcagcaggttggccgccgcgttgtcgctgtattgaatggtggcggcgcacatcgcggagaccgtcatgccctgccccaggaatttttcggtgatgggcgaattgggcaggatgtcgctcttgccgtagctcacgcggcgctccagcaggccgctgtcgcgggcgctgcgctcgaggatggccgcggccagcatcgtcttgaaggtgctgcacagcggaaagcgttcggttgcccggtgctgcacgcgcgcgccggtggcggtatcgaacgcggccacgccgagccggccgcccacggagctttcgagcgccgcgagctctgcctcggccgatgtggcctgcggccctttcgcggaccaggcagtgcaggcgctggccaggggcaatgcggaagcggcaacgaggaaggtgcggcgattggcaaaggatttcatttgtttgtttgtcagcgagtggatggaacgagaggaatcgtaggagcggcatcgcgcaggctccagcgccaggccatgcaaccgcgtctcgcctgtatcgggtgtaaccgcgcaattcattcaactatctggttgaataattgacaggccgcatctatattcaactttatggttgaactagacgacgaacggctggacgccgtgttccacgccctgtccgacagcacgcgccgcacgatgctgcagctgctggcgcagggcgaatgcagcgtgggcgaactcggcgcgccgtttcgcatgtcgttcgcgggcgcatcgaagcacgtcaaggcgctggagcgcgccgggctggtttcccgcaccgtgcaggggcgcgcacatgtctgccggctggagccggcggcactcgcatcggccaacgcatggctgcggtactacgaaggcttctggaacaaccatctggacgcgctggagcgcgagctgcggcgcgaggcatcccgtcagtgaagaccttcctttcttcccttctgccaaggagcaagcaatgaccaagaacggcctcggaaccctgatcgaacccggcacactgcgcatggagcgcaccctgcccgcgcccatcgagcgcgtgtgggcctatttcgtcgaacccgacaagcgcgcggcttggctcgccggcggcaccatggcgcatgagagcggcggcgttttcgagctgcgcttcgaccacacccgtctttccggcgaagtggcacccaaccgcttcagtgcctgccgcagccccatctccgagacatcgcgggtcatccacatcgaaccgctgaagcgcctgaccatcagctggggcagcgagagcgccacggcttccgaagtgagcttcgagttcacgcccgagggcgatgccacgcacctcgtgctcacgcaccgccgcctgcccgaccgcaaggaaacgctcagcgtcgccagtggctggcatgcccacctcgacgtgctcgacgacgtgctgcaccagcgcaagcccagggggttctggacccgccacgcagagctcgaaaaggcttacgaggcccagcttccggcctgagccgccagacccgcctggccgaccgcttgcggagtcggatggcgactacaggcaagcgggccggcttgcgttaaggtgcggagcattcgccgactccgaagcacgcccatgaccacccctccccccgcaccggcccgcaagcatttctcgatgatccggggctttcacctggccgacgtattcacgctcggcaacgcggcttgcggcgtgggggcggtgttccttgccatggcgttcatggccagccagtcgctcggacaattcttctgggcggcggcgctcgcaccggcggccttcgtgttcgacgtgttcgacggccgcatcgcgcgctggcggcaaacgcactccgcgctgggacgcgaactcgattcgctggccgacgtgatttccttcggcgtggcccccgccgcgctggcctttgcagcgggcctggacggcggctgggactgcgtgctgctgatctatttcgtctgctgcggcgtgagccggctcgcgcgctacaacgtcacggccgaggcgctttccgcgggtgccgacaaggtgaagtacttcgaaggtacgcccattccgaccagcgtggtgctggtcggcgtgctggcccttgcagcctggcaaggccgcatcggcgacgcggtgtggggcggcgcctggacgctcggcccctggcagctgcatccactcacgctgctctttgcgttgtcgggcacgctgatgatcagcaagacgctgcgcattcccaagctctgacccggcctcggtgccggtccaatgaaaggagacctcctcatgaagttgtatttcgatccgcacagccgcgcgcagatcgcgaaatggatgctcgacgaagccggcgtggactacgaaatcgtgcccaccctcatccgggagaaggcgcacaagaagcccggttacctgaagatcaatcccgccggcaagctgccggcgctggtcgacggccgcacccgcgtcttcgagaatgcggccatctgcatgtacgtggccgagaagtttccagaggccaggctggcgccgcccgtgggctcgcccgagcgtggccgctacctgtcgctgatggtctattcgacggcgcagctcgagccttcgatgggcgacagcctgctcgggctgcacagcaacaacagcgcgcgcggctggaccgatttcgagcacgccaaggacgcggtggagcgcgaactgggctacggcccctatctcttcggcgcgcagttcaccgcggccgacgtgatgatcggctccatgttcatctggcaccgcgcattcggcggacgctccaaccgggccaagatcgatgcctacatcgaccgcctgcaggcacgccccaagggcatgaagttcggttgaagcacacccccatgtcacaggcaccctttccccacggcgcgaccgccggcctcgaccagctggtccgcatcgccgccgagcagccgctctcgccggcctgcgaccacttctactttctgcgccatggccagaccggccgcaatgcgcagcgcatcttccaggccgtggacgaaccgctgagcgagctcgggctgcagcaggcggcccgcgctgcccagctgctggcgggagagccgatccgcaccatcgtctgcagcgacgcgcggcgcgcgcacgatacggcgcacaccgtggccgcagtccttcgcctcgcgccaacgccccaggcggccctgcgcgaacgcaacttcggtgcgctcattggaacctcgtcggccaacatcgactgggcctgcgaacccgagggcggcgaaacccttgcgcagttcgtggcccgcaagcggcttgcgctcgatgcggcgctggcagagcccgcgccggtgctggtggtggcccatggcggcacgctctatgcgctggccgcgctgctcggtgtgcccatcgacctcgacctgctcggcaatgcgcagccattgcgtttttcgcgcggcggccccacatggaccgtaacaccgctgctgcggcatgccgacggcgattcagccctggcctgacaaagaccgggcgcgtactgttcggcgttcacccccacacagaccgccatggaattcaaggactactacagcgccctgggcatcgaccgcaccgcgtccgacgacgaggtgcgcaaggcctatcgcaagcttgcgcgcaagtaccaccccgacgtcagcaaggaagccgacgccgagaaacgcatgcgcgacatcaacgaagccaacgacgtgctgcgcgacaaggaaaagcgcgccgcctacgacgcactggccgaccgcgtggcgcgcggcggccatcccgagggcgacttccagccgccgccgggctgggacacgggcttcgaatttcaccgcggcccgaaccagggcccggccgaccacgcggatttcagcgagttcttttcatcgctcttcggcgaggccgaacggcgcggcgcggcaaggcacaactaccgcgcacgcggcgaagaccatcacgcggccatcgagatctcgctcgaagacgcactcaacggcgccgagcgcgagatcacgctgcggtcgcaagaaatcgatgcgcacggccggcccgcgttcaagacgcgcacgctcagcgtcaagatcccgcccggcatgcatccggggcagttcatccggctggccggacagggcatgcccggccacggcggcgagcccgccggcgatctgtacctggaggtgcgcatcgcaccgcacaggctctaccgcgtggaagaacgcgacatctacatgacgctgcccgtcacaccgaccgaggccgcgctcggcgcgcaggtgacggtgcccgtgcccaccgggggcgcggtcgaggtgaccgtgccgcccaatgcgcgcagcggcctcaagctcaggctcaagggccgcgggcttggcggcaagcagcccggcgacctgtacctgctgctggaaattgccttgccccccgccaccgcggaggccacgcgcaaggcctacgagcagctcgcacaagcgtcggcttcgttcaacccacgccagcatctgggagtgtgagcatggcgaccgtttccgtcacaacagccatcagcgcgtcgcagccgcttgccgcgagcgagctggcccatgcctgcggcgcagacaccgaatgggtggtgcaactcgtcgaagtcggcatcgtgcaagtcaccgccaccgaggcgccacccgagcggtggcaattctcgagcagcgacctgcaatgcgccctggaggcgcgcaggctcgagcgcgacttcggcgtgggcctcgatgcggccgcgctgattctcgacttgcagcacgaagtgcggcggcttaaagcggtgatccgcgcgcacggcttgcgctgaccggcccggcctcagccggatttgccgcgcgccgtcttcttctggctttcggcgcgcggggtgtttgccgcggccggggcattgctgccgttcaactggtcgacccacaacagcgtgtcgacgtacgacatgaaccggttcagatattcgggcgagagctcatgcatcagcatcagcgaccgatgcacgaggtgatgtgagttgagcgggccggcgttgtccggcaccttcgccaatgactgcgtcagccgccggtctgcgctgagccgcgaccaggtgctcctgaaataccggagcgtcttcagttcggaagcgggcgcggcatcggttgttgcgggctgaccttcggcttgcaacggcgactgccgtgcgatgtgctcgacgagctcggcgagcggcccgcgagcaggcggtgcggcctgcttcgagcccgcatctcgcggcaccgcgggaacaacgcccgcgcgcttttcaagacgctcgcgatacgccgcgagcaggctgtccaccttgtcatcgaggatgcgccgtgcatcgccctggtgctcggccgctcgcctggccatcgcctcgatgaaacgaaagcgcaccgggtccacgcgatgctcgccgcgcgcacgccacgcgtcgagcatcgccatggggtcgtccatgcaactactcacgggccttcgcgccggcgccggtctgctggcggggcgtgggggccatttcgacgcgccggttctttgcccgtccttcggcatcggcattggacgccaccgcctgctcggagccgaaggccgcggcaaacaccgaggacgaaggaatgccttcttcgatcaacgcgcgcgtcaccgtcaaggcgcgctgggccgagagttcccagttgtccgtgaacggccggttgccttccttcgtctgccgcatctgccggtcgtcggtgaagccgctcaccatcagcacctcgtcacgcgcgcggaggtaggcggccacgggcgcggccaggctcttgagcacctggcggccctcgggctgcaggtcggccgagttgaaggcaaacagcacgctgccgctgatgccgatgcgtccgttggtgagcgtgaccctgcccgccgcgagcggccctgccaacgcctgctcgagcgcctcccggcgctgcgtttcggcctggcgctgctgcacctctgcctgcagctttgccgcgaggtccagctgcatgccgagcgctcccaccagaatcagcacgaaggcgccgaccaggcccgacatcaggtcgccgaagactgcccacaccggcacgctcggctccaggccggcgtcgaggtcgtcccgcatcacgcttcgctcgccacggcctgctgccggccggcaatctgctgcaggtcctcgacgatctgcttctgcgacatgatgctgaggtcgatgacttccctcgcctgcgccacgtagtaggccaactgctcgtcgctgcgcgcaatggacttgccgagcgcgccttcgacgcgctgcagatgggccaccagcttgtcgttcgattcgctgaacagctgcacggcaagaccgaaggcttcgccgaggctcgccacttcgacggcgctgccggtgatctgtgcggcaacgccggccatctttccggtttctgcctcgaccttgtcggtgaagcggctgccgactcgctccagcacatccgccgacgcgccgaccagcgcgtcgaccgccgaacgctgctcggtggaggcatggttcacggcgtcgagcagggtgcccagcgtttccatgatgcggctgcgttcttccagcatcgcgttgtcgcgcgccatgctgtcggaaagcttctggcgcagctcggccaccacttcggccgccacgcgcggcgcgtcggacgcggcctgcaggagctgggcgatttcggccaccgtggtcttcgcgtgggcttccgcctgcgccgacatgtcgcgggcggtttgtgcgagggtctggaaaagctgttgctgctggccctccgcgtgcgcgcccgcctgccgccactcttgctgcagcgacgtggccatggccgccagcgcctgcgtccaggccgacaggcgctgctcgtcgcgtgccgcgatctgcgtctgaaggttgacgtgcgcctggtccacggtgcgcagcagcgatgccgcgtgctgctcgaagcctgccgccgccgccgcgaaggactggtgcgcgtcctccgacagtttttcgctcacgcgctgatgctgcgcgagcgcattgccccaggtgtccgacacgctgcccaccgtgctttcgagatgggcggacacgccttccaccagcgatgccgaacgttgttcgaaggtttcggcaaagcggtcgtgcgacgcgcgcaagtctttggccagcgcctcggaagtgcgctcgtgctcggcgagcgcggccttccaggtgtcggccacgctggacgtggcggcctcgaagcggcccgagaggccgtccagctgctgctgcacggtgcgtgcgacggtgtcgtgcaaggaagccgtctcgcgtgcaatgcccgccatggtggcttcgacgaccggctggatggtggcgcccgcgatgcgggcgctttcggtcaggctctgcttcagcgactggtcgaccgacgaggcgagcccggcatacacggcctcggcctgggtgtggaagtgcacctggccggtgacgagccgctcgttcaaggcctgggcctggcgctccatcgtggccatcatcgcctgcagctggtcgaccagccggggcatcatctgcgcctgctgctcgagcaactggaacgacgcctctcgccgatgcgtctcggagtagacacgcagcgcagtcgcgatcttgctgtcgagcatctgtccggcctgcagccgctcgcgccggcacagggccgaggcaaggccgagcatcgccgaggcggccacgccggccacggaggtgccgaacgccagccccaggcccttgacgggagccgacagcgaggcacggatggccggcaggtcggtcgcggtctccagcgccagccctgtgccgttgagcgtcaccaccatgccgaggaatgtgcccagcatgcccagcagcaccagcagtccggccaggtagggcgtgagcgccgggccgggcaagccgacacgctcgccctcgatgcgcaggcgcaccgcgttgcgcagcgacggatgaagctggccgagccatgcgccaaggtccgcgggagcggcggacaggtcggccacggcgcggctcaaggtggacgtcgcctgctggaaccggtgcagctccagcgcacccatgacgtagaacgcgccgacgatcatcgtgacgatgagcgccaatggatgcgacccggcgtagcccgcgccaacccagcacacgacggccaggcccgcggcaaaaacagcgtagtgaagaaatctattcatggcactctggttgcctcatgcgaagggcttcgagcagcccttcgatcggttgaaatcggaaatccagttcggcgagcagcacgttcttcatgtccttgcggaacacatgcagccactcgccggcctggggttcgacgcccaggcgggtgaaatgcttttcgagcagcgcaggcacgcctgccagcaggctgtgctcgcgcgcagccagaacctgctccatgaccacgtccacggcggccagccgggccatggccggcgacctggccgccagcgtcgcccgcaggcgcccgcgcagggggccgatgcccgcctccatggcctgctgcagtgcaaagtagcgacggcggaacggcgcgaagtcggccgctgccgcggcagcgccgtcttctgcgatggcattggcgagcgcggtacgcgcacgggcgcattcccgctcctcggcgttcgcgaaagcccgttgccgggaagaagcagccgccggaactccctccagcgccgcggacagcgaaatggcatcggtccagccgaaccactggctcaatcgatccgcggtggcttgccggggttcgcggacgcccgtatcggccagtcgggaaagcaagcgaacgagcgccgaaccgttgaaaactgtgcgctgtgaaacttgcgccataccgccagaacgaaaaacctggcagtctacactggccacccctcccggaagctctgcccggctgcccctgccccggtgaaacttcaggtaacgcagcggtcggtaaccaggcgttttttgggttcaggctccgcgcttcggcagcagtcttccacgcggcgtggcgtaagtcctaagccctacaagcgcttaccgcgtgcagactcgttacatgccggccccatggccggaaaagctcgaggagcggcatggccatgcaggatcggatcgcttgtcatcgctgcgggcgcgtttgcctgcacgccgacgcgccatgcccggcctgtggcgccgcgccggtggcgagccccgcggtagcgggcgcgaccgagcccttcgtgggacgccgcggcgaactgcaggtggcgcacgatgcgctcggcggtgctctggccgggcgtggccgcgtgatcatggtcagcggagaggccggcatcggcaagacccggctggcgcaagaggtggcaacgctggccgtgcggcgcggcatgctgaccttgtggggccgctgcctcgaggaacccggcgcgccgccattcctgccctggacgcgcgccatgcaggcctgcctgcgggcctgccgcgacgagcgcctgccggcgctgctcggtcgggacgccgccgcggcggtcgagattgcacccgaactcgccgagcgtctgccgccaggcaccgcggtgccggccatcggcgaaggcgaccaggcgcgctttcgcctgtttgccgcggtggcgcatttctggcgtcaggtggcaacgctgcggccgctgctcctgatcctggacaacctgcactgggccgatgcctcgtcgctgcggctcctggccttcattgcgcaagagctcggcgagagccgcatcgtgctgctcggctcctaccgcgaggcggatctgtcgcgccagcacccattggccgcaacgctggccgaactgttgaacacgcggcagttctgccgactgccgctcccgggcctgagcctggaggaaaccgagcggatggtcgcagcggccagcgccgtgacgccgccgcccgcggtgattgcgaccatgcaccgccgcaccgagggcaatccgctgtacctggtggagacgctgcgcttcttgctgcagggcccgtacggaaccgacccgcacgcagccgcggcgctggtcgaaaccgtgcccggcggcattcgcgcggtgatcggccagcggctcaaccggctctcggcgccctgctgtgcgctgctcgcgattgccgcctgcatcggccgcgccttcgacctgccgctcctggccgagctggccggcgccgacagcgaggccgagctgctggccaggctcgacgaagcgctgtcgcaccggatcatcgagatattgccgcccggacctcagtaccagttcagccacgtgctgatccgcgaagtgctttacgacgagctgcccgcggcacggcgcgtcgcgctgcacgggcgcattgccgagtcgctcgaggcgcgccatgccgccgatcccgacgcggtgctggcgcagctggcctaccacgcggccgcggcactgcccgtgggcagcccggcgcgcgcgctggacattgcgcagcgcgccgccgcgcgggccgtcgcggtgatggcgtacgaagaggccttgcgctgctaccggctcgcgctgcagctgcaggagcgctggctgccggccgagcgcgcgcggcacggcgccctgctgctcgctcttggcgcggtgcagacgcatgccggcgaaaacgatgccgccgccgccacctttctggaggccgccacgctggcgcgcgcgctcggcgatgccgggctgtttgcgcaggccgcgctcggcttcgagaacaacggctggcgcatcagcggtccgggcgaacaggcggcggccttgctcgaagaagcgctcgcggcggccgatcgcttcgatgccgcgctgcgcgtcgacctgctcgccgcgctgtgccgcgcctgcatcttctgcggccgacagcctgaggccaatgcggcgcagcgcagcgcggtggcactggcgcgcgaactggcgatgccgcggccgctgttcaaggccctggccgcgatcctgccggcgcgcggcgatccggggcagctcgaggagcgcctgcgctgcgcgcgcgaagccttcgacgtggcggaacacgccggacatctcgaatgggtcgactcgctcaccggctggtactttggcgacctggtcgagaaaggcgcgctcgacgcagcgcgctcgctggcgcaggtgcacgcgcgcgtggcggacgcgatccgccagcccttcatgcaggccatgggcctggccagcctcaccctgcttgctgcgtacgaaggccgcttcgcggattccgaacggctggccggcgagaccttcacgctcgggcagcgctttttgtccggcaatgcgcagggtgcctacagcctgcagatcttcgtgctgcgacgccagcagggccggctcggcgaggtgctgccggtgctgcgcgggctggtcggccgcgtgccgcgcaacagcctgtggcagcccggcctcgcgctgatctgcgccgagctcgaactgcacgagcccgcccgcgaggcttacgaagcgctggcggccgacgactttgcgggcattgcgcgcgacggcatgtggctgaccaacatcgtctttgccgccgaggtctgcgcccgcctgggcgatctgccgcgcgcggcaacgctttaccagctgctcgagccctatgccgggcgcaacgtggtcaccggcaccaacattgcctgctttggcgccgtggaccgttaccgcggcatgctggccgcactggcgggagacgacgagagcgccgcgctccatttcgcggccgcggccgcactcgacgagcaaggcggcagccggccctggctcgcgcacagccgcttcgaatgggcacggtggctggcccggcgcggcggcgatgaggcggccgccaaatcgcatctggaagcggcgctttcgatcggtcgcgagctcggcatggccggcctcgcccgtcgctgcgaggcgctgcagcgcgaactcgaaggcgccgctcgatcacctgcggcgcccgagggcctgagcccgcgcgaagtcgacgtgctgcggctgctcagtgccggccacagcaaccaggcgatcgcgcagcggctgttcatcagcccgcacacggtggcccaccacgtgcgccacatcctctccaagaccgactgccgcagccgcaccgaggccgcggcctgggcgcaccgccatcgcgtggcgtccgaaggctcgacggcgtccgctgccggccgctagccactggccgcgcgcggcccaaatggtcaattcgggcgatgtgcggccgcgccggccgtcctatggtctgtcccaggcccggcgccgccgggtcggcaaaccagaaggagtgtctcgtatgcccgcaaccctttatgaacggctcggcggcgaggagcgcatccagcggctcgtgaccgacgtggtcgagaaccactacaacaacccgctgattcgttcccgcttcgcgaacagcaaccgccccgaggtggagcgccacgtggtcgagttcctctgcgccggcagcggtggcccgcagtgctacaccggcaaggacctggtgacggcgcacaagggcatgaacatcaacgagcaggaactggtcgccgcaatcgacgacatcctggcggcgatgtccaagaacggctacgaccaggccgaaaagaacgaggtggtcgccattctttattcattgaagggcgacgtggtgcggctgtagagaaagccccgcctcccgctcgcgccccggcggcgctcgccggtgaactggaaaggaaagaccatgacacgccaaccatttgctgcctgggcgatcggagccaccctgatagcggccatcgcgacgagttgggcccagaccgctgaccaccggatgatttcggccgccgacttgaaatgggccgacgttccctcgctgccgccgggcgcaaaactcgcggtgctcgaaggaccgatgagcgaggccgtgcccttcacggtgcgcatcaaagtgccggccaactaccggattccgccgcactggcatccggccgtcgagcgggtgaccgtgctctcgggcaccttccacatgggcgtgggcgacaagctcgacatgcaaaagtcgatgcccgtggccacgggcggcatgatgatcctgcaggccaagacgccgcactttgcatggacccaggaggaaaccgtggtgcagcttcacggcaccggcccgtggggcgtcacctacgtcaatccggcggacgacccgcggtcgaaatagccggagagcaaacgagcggcgcagggccgctcgctgccggttcagaccacaacggcctcggcctgcaccgcaggcgggcgcagctcgtcgacctcgatcaccacgtcggccggcaacccgttgcgctgcgccgcctcgcggatcatctctgcgctgggcgcctcgtacaggcagtaggtcttcttcttgtcggcgctcaagaacgaatacagccagcggaccccgacgtcgtcgttgatgcgcatgatgctggccgcgccctcgggcgagacctcgagtgcatcggcaaaggtgcgttcgatcagatagagaggcatggcaactccttcgtacgggtgaggctgacatcgtaggacgggcaggcgccaggcgttgcatgtgtttcccccgcctggccattcgtactaccctgccatctacccatgcttcgcgccaaaaagcaaaaagccgtacggcgctttgggcaccgtccggctttttgttgttgctggggcaagcggcgtgctgccgctgttcccgagcctgccctgattacaggccggcctggcgcgtgaagctgcgagcttgcgaagggatcacgctgcctgcgaaggcttcgcggcgcagattctggccgggtgcgtgcgcggcggcaacggcttcgttgcgaacttcggcgcggtcggccgaagccagcaccggagccacgacggccgaagcagcgtcgctgtaggcgttgccttcgcgggcggcggctgcggcttgcggtgccacgtcggcacggctgtagccggcgctcaggggctgcacgccttcgtaggtttctgcgtgggcgccagcggcggcgagcagggagagagcggcggcggcgaggatgttcgaggtcttcatttcaatttccttcttgatcgggctttggatgcctcgaagtttgcgcctcaattagcagggaaaaccctagccaatcgaatcgcagtgttcatgaaactgaaacaatgacggggaactttctggacgggagggcgaaagtgctcatcacgagcgatgggtcttcgtccaggcgacgagtatcgcgcagcacagcgatgcacgttgcatgccagccaccgcgccctgcaatgcggcgttcgccctatgccttggcgcctgacaagtacgccactgcgcgcgcggcggtcaagagcggggccagccgcgcaccagcgtccggatcgccacggcgccgcttgccttgacctcggcgcggtagctgcccaccagtgcttcgcgctcggccgcggcctgcgcatcgttgcgccatgcgagcaaggcggccacgtccgcatccggcagggcagcgagcaacgcctgcgtgacctgcttttcgaactcgcgcgccacgatcagcaggttgcgcgggcgcggcgacgtgacgccgcgcgaccacagcgtgtcgacggccatgtcgagcgtgcggtcgggcaaggaagtgaactggctcgcgttgccgcgcgccagctgcttgacgacggagctcagcagcagctggctcgaaaaatcgacttcgcgcacgtcggccacggccatgcgctcgagcagttccgtgcgtgcgggatcggccagcttcgcgcgctcacggttgaagaactccagcttgcccgcgtcgtccatcgcggcgtagtcggcgcgcagcttcgagaaccgggccacggcggcctgcacctgcgggcccggcgccgcgccgcccttgccggcagccgccacttcctgctggattgccgcaacggatgcggccacgtcgaacgaccgcgcagcagccgcgtccagcgactggagcgccttgtcggcaatggcctggtcggagggctccagcagctggcgcgcatcgcgcgacactgcccccggcgcataggccgcctggtagcgcgcctgcacgccctcgaactgcagcagggcctgggcacggtcttgcgcccagcccatgacgggtgcgagcaacaacgacaggagaagaacgacgggtgcgaggaagaagcgtctcggtgaaactgaaaaggcaaccatgcgccattattgattggcgcttgccatggccgccctctcccgccccgggcttcaggcggtcgccaattccttgcgcagcagcttcgcagccgccaccatgttcgacagcgcggcctccgtctcgggccagccgcgggtcttcaggccgcaatccggattgatccagaggttctcgagcggcaccacaccggaggccttgcgcatcaggcgcacgatctcttccaccgtgggaacgcgcggcgaatggatgtcgtacacaccggggccgatctcgttcgggtagcggaagccgcccgcatcgttctcgccacccaatccgccgaacgcgcgcagcaactccatgtcggaacggctggtctcgatggtgatcacgtcggcatccatggccgcgatctccggcaggatgtcgttgaactccgaatagcacatgtgggtgtggatctgcgtctcgtcgcgcacgcccgaggcgctgatgcgaaaggcccgcgtggccgacttcaggtaggccggccagccggcgcggcgcagcggcaggccctctcggatcgcgggctcgtcgatctggatgatgccgatgccgacaccctcgaggtccaccacctcgtcgcggatcgcccaggcaatctgctcgcaggtggtgctgcgcggctggtcgtcgcgcacgaaggaccattgcaggatggtgaccggcccggtcagcatgcccttcatcggcagcttggtgaggctctgcgcataagcagtccactcgacggtcatgggcgcggggcgcgccacgtcgccgaagatgaccggcggcttgacgcagcgcgagccgtacgactgcacccagccgttggcggtgaaggcaaagccgtcgagctgttcgccgaagtactcgaccatgtcgttgcgctcggcttcgccgtgcaccaacacgtcgatgcccagttcttcctgcttgcgcacggccagtgcaatctcggcgcgcatcttctcgcggtagcctgctgcatcgagctcgccgcgcttgaaggtggcacgcgcggcgcgtatctccttggtctgcggaaatgagccgatagtggtggtgggcagcgcggggaatgcgaagcgcgcgcgctgcaccaactgccgccgaccgaatgcggacgtgcgctggtcatccccggccacgctgcgtgccagccgcagtgccacgtcgacgcggtgcacccgcgggctgctgcgccgcgcggccactgccgcgcgcgcggccttgagttcttcggccaccgagccttcgcggccgtcgagcacggcacgcagcacgcgcagctcgtcgagcttctcgattgcaaaggcgagccatgacttgagttccgcatcgagcttgttttcggcggccaggctgaacggcacatgcagcagcgagcaggacggcgcaatccacagctcgccgcggttcttgtcgaccaccgggcgcagcgtggccagcgccgcgtcggggtcggtgcgccagatgttgcggccgtcgacgatgccgacggacagcaccttgtgtgcggagagccagtcggccacgccggtcagatcctgcggcgcgcgcacggcgtccacgtgcaggccggccacgggcagctggcaggcgaggcgcaggttgtccgagagcggcgagaagtacgtggccagcaacagcttgggcgcgctgcgagccagttgccagtaggcgcgctcgaaggcgttgcgccaggcatcgggcaggtccaggccgaggatgggctcgtcgatctgcacccactccacgccctgctgcttgaggcggttcagcacctcttcatacacgggcagcaatgcgtcgagcagcgagaagcggtcgaagccggcttctttttccttgccgaggtacaggaaactcagcggcccgagcagcacggccttgaccgcatgcccggcctgctgcgcctgcgccacttcgtcgaacagccgcgtcgatgcgagcttgaactgcgtggccgcggtgaactccggcacgaggtagtggtagttggtgtcgaaccacttggtcatctcgagcgcgaaggtgccttcgtggccgtggttgcagctgacatcgtgcacgtggtcggcctcgtcttccacgccgcgcgccatcttgaagtagcgcgacaactcgggctcgtcgcccttgaacccgaagcgctcgggttcgcagccgagcagctggatgtggttggccacttggtcgtagtacgcaaagtcgcccacggccacgtagtcgagccccgcgtcgcgctgggcctgccagtggcgttcgcgcagctgttcgccgacggcttcgagcgcggcgcggtcgatctcgccgcgccagtgcttttcgagtgcgaacttgagttcccggttggcgcccatgcgcggaaagccgagggtgtggatgcgggtggtcattgcaggtaatccggtcgctgtatcttgagaatccgcaatggtcgggctttggggcatatgattcaaacgaaacgttttgccctttcacttgaaattcattcatgttgcagtcgatcctcgagatacgccacctgcgcacgctcgttgcgctgcgcgacaccggcagcctggtgcgcgcggcgcaattgctcaacctcacgcaatcggcgctgtcgcaccagatcaagctgctcgaagaccgctacggcgcacagctcttcgagcgaaagtcggtcccgccgcagttcagcaccaccgggctgcggctcttgcagctggccgataccgcgctgccgctggtggaagaagccgagcgcgacgtggcgcggcttgccttgggacgcagcgggcagctgcgcatcgtggtcgagtgccacacctgcttcgactggctgatgccggccatggacgccttccgccagcgctggccggagatcgaactcgacatcgtctcgggctttcaccccgacccgatcgcgctggtgatgcagaaccgcgccgaagtggcgatcgtctccgaagaggaccccgacgagacggtggactaccacgcgctgttccgcttcgagatcgtcgcgctgcttgccaacgaccatgcgctcgcggccaagacgcatctcacggcgcgccattttgccgaccagacgctcatcacctacccggtgccggacgagatgctcgacatcgtgcggcaggtgctggcaccggccggcgtggagcccgcgcaccggcgcacgaccgagctcacggtcgcaatgctgcagctggtggccagcggccgcggcgtggcgaccttgccgctctgggcagtgcagaactatctggaccgcggctacgtgacggcgcggcgcgtgagcagcaagggcctgacggggcggctctacatggcctgcacgcagggcacttcgggccagccgtggctggcggacttcgtgcgcatcacgcgcgagagctgcttcaagagtttgccgggcatcgagctgctctgacgcggcggccgcgaccgcaaggtacagtcgggaatgaacccacacacgcccagcgcccctaatccgcccgaaacggctcccgccgaggtcacggagacccaggcgttcacacgcgcatgggtcgtgtttctgctgctgttcgtgggcgtgctggcccttctgtgggccaacgacgcgctgttcggctagaggctagagacgctaggacgacgacttctgcaccagcttcagcacgcttgagaaatcgagcgcgccatggcccgcgaggctgtgcgccgcatagaggctgcgcgccagcccgccgagcggcgtggctgcacgcacggccgtggcgttttcctgtgcgaggccgaggtccttgagcatcaggtcggtgccgaatccgcccgcgtagttcttcgatgcgggcgcggtttccatcacgccgggcatcgggttgtacttttcgagcacccagttgccgccggagctgcgccgcatgatttcggacagcaccttgggatcgagcccgttggcaacgcccagcgccagcgcctcggatgtgccgatcatcaggatgccgagcagcatgttgttgcagatcttcgcggtctggcccgcgccgatgccgcccgcgtggaagatgttggcgcccatcttctcgagtaccggacgcgcgcggtcgaggtcgtcggtttcgccgccgaccatgaaggtcagcgtgccggcaatcgcgccgcccgtgccgccggaaaccggcgcatcgatcattgcaatgcccttggcggcggccgcctcggccaccttgcgcgaggtggcggccgcgatggtgctgctgtcgatcacgagcgcgccggcgcgaatgctgtcgagcagcgccggcttgcccgcgctgccgagaaacaggccttccacgtgcgcgctggccgggagcatgctgatgaccacgtctgcatcggccaccgattcggcagccgatgcggcaatgggcaggccttcggcagcgtatttcttgcaggcctcgcccgagaggtcgaaggccttgactgcgtaacccgccttgcgcaggttcagcgccatggggccgcccatgttgccgagtccgatgaatgcgattttcatttgcttgtctccgttgtatttgtgaagaggctcaggccagcgcagccagttccgcgggcatctctccgcgcggacgcaggtggtcttcgatgaacgcgggcgtgatctcttcgatggtggcggggttccagcgtggattgcggtccttgtcgatcagcaccgcgcggatgccctcggcaaagtccttgtgcgcgcaaaagcccagcgaggcccagtattcgagccggaacacctcggccagcgacatgcggtgcacgcgctgccaaagctcgaagctcagcgcggccgagctcggggcgcccttcatgaaggtcttggacgcggactgcagccacggatcgtcgctctgcaggttgcgcaggcgcttcgcgatgtcgagcaggtcgtcgccggccatcagcgcgttgatggtgtcgtagtgctcgcgcaccttcgaggccggcattgcggcgccctcaccggcgcgcgcaagaatgcgcgagagttcggcgcggtcggtcttctggtccccactccagcgtgcggccgcaatcgcttcgagcacctggcccttgcgctcgtgcggcaccagcacgtcggccaatccgcagaagatggcatcggccgcattgaggttcgcagccgtcagcgccaggaagaggcccgtgcggccgggcgtgcgccggaggaaccagcttccgcccacatcggggtacaggccgatggcgatctcgggcatggcgatgcggctctgcgccgtgaccacgcggtgcgagcagcccgacatcagacccacgccaccgcccatcacgatgccgtggccccagcacaggaagggcttgggaaaggtgtggatcaggtggtcgagctcgtactcctcgcggaagaaatcttcggcgtaggtgttgcgtgcgggaccgcattcaagcagggtttgatacagctggcgcaagtcgccgccggcgcagaaggctttctcgcccgcggcctgcagcagcacgccgacgatgccattgtcggccgcccattcgcgcagcttgggcgtgagcaggcgcaccatgtccacggaaagcgcgttgagcgaggccggtgcgttgagcgtggcaacgccgaagcgctggccgccggcggtcttgatttcgtcgaagagaactacggagtcggtcattgtcttgagaggttctggatgcggggtttcagcggatgtcgctgtccccttccagcaattttcgcgcaacgatcacgcgcatgatctcgttggtgccttcgaggatctggtgcacgcgggtatcgcgcaccagccgctccagcgggaactcgctcaggtagccgtagccgccgtgcagctgcagtgcgtcgttgcacacgttgaagcctgcatcggtcgcaaagcgcttggccatggcgcaataggtgctggcatcggcatggcccgcatcgagcttgcttgccgcgagccgcaccatctgccgcgccgcgaccagctcggttgccatgtcggccagcttgaactgcaaggcctgaaagctcgcgatcggcttgccgaactgctggcgctcgtgcaggtagcggcgggccgcatcgagcgcgccctgcgccgcgcccaccgagcaggtcgcgatgttgatgcgcccgccgtcgagccccttcatggcaatgcgaaagccctcgccttccttgcccagcaggttctcggccggcacgcgcacgttgtcgaagttgatggtgcgcgtgggctggctgttccagcccatcttgtgctccttcttgccgtagctcacgcccggcgcgtcggccggcaccgcaaaggccgagatgccgcccgcgccgccgccgcccgtgcgcgccatgagcaccagcatgtcggtcgcgcccgcacccgagatgaaggccttgccgccgttgatgacgtattcatctccctgcagctcggcgcgcgtcttgagcgagcccgcatccgatccggcgcccggttcggtgaggcagtaggaagcgagcttgcgcccgctcgtcaagtcttcgccccactgcttggcaaccgcatcggtcgcccaggtgccgagcatccacgtggccatgttgtggatcgtgatgaaggccgtggtcgacggatcgaccgcggccatctcctcgaacaccagcgccgcgtcgagccgcggcaagccgaggccgccgacgcgctcgggcgcatagagcccgcagaagcccagttcgccggccttggcgatggcctctttcggaaagatggcctccgcatcccaccgcgctgcatgcggcgcgaattcggcctgtgcaaaatcccgcgcactctgcgcgaaggcgcgctgctcttctgaaagttcgaagtccattcgcccggtttctttacttgaggctgatggtcgtattcacgccatgggacacggtgctgtcgtcgaaccagcgtgccgtcacggtcttggtctgcgtgtagaacatgatgacctgcttgccgtaggggcccaggtcgccgagcttggaagcacgcgaaccggtgaacgagaacatcggcaccggcaccggaatcggcacgttgatgccgacctggcccacgtcgatgtcttcctggaagcggcgcgccgcggcacccgactgcgtgaagatggccgtgccattgccgttcgggttgctgttgatcagctcgatcgcctcgtcgatgttctcggcgtcggccacgcagagcacgggcccgaacacctcctggtcatagatcgtcatgccgggcttcacgcccgagaagatcgtcgggccgacgaagttgcccttctcgtagccgggcaccgtaggcttgcggccgtcgagctcgagcttggcgccgtcggccacgccgcgttcgatgaggccgttgacgcgctcaaaagcagcgcacgagaccagcgggcccacgtccacgcccttctcggtgccggcaccgatcttcagcgtcttggccttctcgatgagctcgggcacccagttgcgggcctcgcccaccagcaccgccaccgacaccgccatgcagcgctggcccgccgcaccgaagctcgcgcccgccagtgcgttgagggtctgctccttgttcgcgtcgggcatcacgatggcgtggttcttcgcacccatcatgcattgcacgcgcttgccggccagcgtggcgcggttgtagacgtgcgtgccgaccttggtcgagccgacgaagctgatcgccttgatgtccttgtggtcgcagatgccgttgaccacggcttcgccgccgtgcaccacgttcagcacgccgggcggaatgccggcttcgagcgccagctcgcaaaggcgcatggtcaccatcgggtcttgctccgaaggcttcagcacgaaggtgttgccggtgacgatggccatcgggaacatccacagcgggatcatggccgggaagttgaacggcgtgatgccggcgcacacgcccagcggctgcagcagcgtgtaggtgtcgaccccgttggccacgttgttggccagctcgccgagctgcaggttgccgatgttcgatgcgtgctcgaccacttcgaggccgcggaacacgtcgccctccgcgtccggcagcgtcttgccctgctcggccgtgaggatggcagccagttcgcccatgttctcgcgaatgagctgctggtacttcaggaagatgcgggcgcgcgcgccgatgggcgtcttgcgccaggtcttgaaggcgtctttggcggaggccacggcggcgtcgagttcggcctgcgtggcaaagggcacgcgggccagcacctcttgcgtggccgggttgacgatgtcgcgccattcggtggtcttcgattcgacgaacttgccgccgatcaacagcttgacggtggcgacctgggtcttgggggtggtggtggcgtccatggggttttgtctcctgtgaatacgggcctggatggcaggttcaagccgcatcctagctttgcagatttgccatgacaatagacaaatatgcgctatcgctttgcaaaaatgcagagccaacgccacgggacgcacgcacatggactgggacaaccttcgctactttctggagctggcccgctcgggcacgctgatgagcgcggcgcgccggctggaggtggatcacaccacggtggcgcggcgcatccaggcgctcgaaaaggaagtgggcgcgccgcttttctcgcgtgaggcgggcggccaccggctcaccgaagcgggccgcaagctgcagccgcaggtcgaggccatggagagcgcgttccgggcggtggaaagcaccgcgccggcctcgcaggagggcctgtcggggctgatccgcatcggcgcgaccgaaggcttcggcaccgtggtgctggcgccgcagcttgcacggtttgcgcagcagcaccccaaactcaccatcgacctgctggcgatgccgcgcctggtgcatctgtcgcgccgcgaagccgacatcgtgatttcgctggagcggccggcacgcggcgccgtggtggtgaccaagctcaccgactacacgctgcggctctacgcgtcgaaggagtacctggccgcgcacaagcccatcaagacgcgcgaagacctgcgcggccacaccttcatcagctacgtggacgacctgctcttcagcaaggaactgcagtacctcgacgaactgcatcgccccgacgcctttgcgctgcgcagcaccagcgtgctcgcccagcaccaggcggtggtggcgggcgccggcattgcggtgctcccggccttcgtggccgagcgggacccggcattgcgcccggtgctggagggccaggcgaacttcacgcgcacgttctggatgtcgatgccggccgagaccaagcacctggtgcgcatgcaggccgtgtggagcttcctgcgcgagacggcgcaggcccagcagccgctgctgctgttgccgcagaatgcggaagaatccgaagacaggcacggcgcgccgccacggtcgccgcgcccacgcaagcagggtctgtagccaccaggagatcgcatgccacgccatcgtcccgcaaggctcgaacacattgcaggcatcggcgtcgaccgcatgggcgccattgccgacgatgcggacgggccgccctttctccgcctcgaaaacctcgacgtcgacattccgccggaccccgaggccatcgcgcgcaccgtgcgcgccgcttcggaagatgcggacaacagctacctgcccttcgtcggccagtcgcgcctgcgcgaggttgccgcgcggcatgtgtcggcgctctcgggggtggactacagcgcgcgcaactgcgtgatctcggcgggcggcctctcgggcatcctcaacgcgctgctcgcgacggtcgaggtgggcgacgaggtgctggtgaccgacccgacctacgcggggctgctcaatcgcatccggctcgcaggtgggacgccgaagtacgtgcccttcgtcttcacgcccggcggtgaatggaagctcgatcgcgcagcgctgcaggccgccatcggcccgcgcgtgcgcgtgatgctgctgatgtcgccctcgatgccgaccggcggctacttgggcgaagacgactggcgcgccattgccacgctgtgcgtgcggcacgacctcacgctcatcctcgacaccgccatggagcggctgctgttcgacggccgccgggtgattcatccggccggtcttcccggcatggcggagcgcacgatcacagtgggctcgtcggccaaggagctgcgcatgatcggctggcgcgtcgggtggaccatcgcgcccgaggcgtacatgcccgacctggtggctgtgtcgctcgccaacgtggtagtgccggtgggcattgcgcaggatgcggtggcgacggcgctcgaacagtcggcgaacacgctcacaccctatgtggccgaactggaacggcggcgcgacacggtgctcgacgaactccggggcctccctgtcggcgtgccgggcggcggttggtcgctgctgctgcgtaccagcgatttcggcatcgacgggcaggcgttgtccgaacgcctgttgaaggcacgtgtgtgcgcgaccgcgatgaaaggctggggcgaaacgcacggcacgcaatacctgcgtttcgtgttctccaacgaaccggtcgagcgcctgcgcgggctcggcgagaaggtgcgggccgcactgggcgcgtgagctcggcgcgaaaagacagtgccctcccccaacgacaagggccgcgagagcggcccttgtcgatgtcgtcgcagtgcgtacggcctactggatcagcttggcccccgtcttcgcctgcagcgtatcgaagctcacgcccggcgcaagctcgaccaccttgaggccttcaggcaccacgtccatcacggccaggtcggtgatgatgcggtcgaccacgcccacgccggtcagcggcagcgtgcacttctcgaggatcttcaggtcctcggtgccgtccttcttcttggccacgtgctccatcagcacgatgacgcgcttcacgccggccaccaggtccatggcgccgcccatgcccttcaccatcttgccggggatcatccagttggcgaggtcgccctgcacgctgacctgcatcgcgccgaggatcgagaggttgatcttgccgccgcggatcatcgcgaagctgtcgtggctgccgaagatggccgagccgggcagcgtggtgacggtctgcttgccggcgttgatcaggtcggcgtcgacctggtcttcggtcgggaacgggccgatgcccagcataccgttctcactttgcagccacacttccttgtcgccgacgaagttggccaccagcgtgggaatgccgatgcccaggttcacgtagaagccgtcttcgagttcttgcgccgcacgcgcggccatttggtcttgggtccagggcatctcaggctcctttgttgttcttgacgggggcgggcacttcactgccggcggcggcctgcgcaatggcggcctgcgcttcgaccttggcggcggccgcatcggtcggggcggccgcgctcacggtgcgcttttcgatgcgcttctcgggcttggcgttcagcacgatgcggtgcacgtagatgcccggcaagtgaatgtcgtctggggccagttcacccacttcgacgatcttctcgacttcgacgatgcagatcttgccggccatggcggcggcggggttgaaattgcgcgccgtgaggcgaaaacgcaggttgcccgacttgtcggccacgtcggccttgaccagtgccacgtcgggcaccagcgagcgttccatcacgtaggtttcgccgtcgaactcgcgcagctccttgccctcggccacctgcgtgccaacgccggtcttggtgaagaaggccggaatgcccgcgccgcccgcgcgcagcttttcggccagcgtgccctggggcgtgaactccagcgcgagctcgcccgcgaggtactggcgctcgaactccttgttctcgcccacgtacgacgcgatcatcttcttgatctgccgcgtctcgagcagcttgccgaggccgaagccgtcgacgcccgcgttgttggagatgcaggtgagatctttgacgccggagtcgtgcagcgcatcgatcagcgcctcgggaatgccgcacaggccgaagccgccgaccgcgagcgtctgcccgtcggccacgacccccttgagtgccgcgtctgcggagggataaatcttgttcactcgggctccttgatggatggtggagagttggcgaaagcttttgaagagccttgaacgatactacgtactcatatacgtagtatttcgtaatggtgacccccgatgcaggagatcgattaccgcctggctttcgaacatgcccccgtgggcatggtggtttcgcgcaaccgcaccatcgtggcctgcaacgagcgggtgtgcgagatcttcggtgcaacgccctctgcattggtcgggcattcgttcagcattctctacccgagcgtggccgagttcgagcgtatcggcaagcgcatggagcccttcctcaacgccagcggccgctatgccgacaaccgcatgatgaagcgcctgggcggcctgcacggcgccattgccggggaaaccttctggtgccacgtcaccggccacgccatgaaccgggccgcgccgcacgaggccggcatctggaccttcgaagacctgggatcgcgccgcgcggtcaaagccgagctcacgccgcgcgagcgcgaggtggcggcgcaggtgatgcgcgggctcacgtccaaggagatcggcaaggcgttgggcatcagccaccgcacggtggagttgcaccgcgcgcggctgatgcgcaagtacgcggcggcgaccacggcggagctggtgcagaagctcattgccggctaattcttcgcagctactctgacctggttccgcggggatcgttgcaaaaacggaaacgcggtgtcgcgcaaaggcccgtgccgcggtgccttgcgatgactatctttgaggcatgcgggcaagtcgcccgctgccattcaggagtatcgatatgaccacacctcttcattccgaaaagaacctgtttctcgcgtcgaagctgtcgattgcgcgggtgcaagccctggcgtcgcaccgactgccagtcacgctgaccttggcagccatcattctctcggtgctcggcgtcaagccgtagcgcgttacggccaagccgggtcactctggcttgatgtccgccgccttgatcaccttcgcccaggccgccagttcctggtcgacgaacttgcccaatgcggccgggtccatgtaggtggcgaaggcgccctgctcgtccaccttcttgcggaacggctcgctctcgacgattttcttgatctcggcgctgagcttggcaacgacgtcgggcggtgtctttgccggtgcgaacaccgcgaaccacgattcgacctcgtagcccgggagcccggcctcggccgaggtcggcacgtcgggcatcgacggatggcgcttgctgccggtgtaggccagcggcttgatgcgcccgcccgcgaagtggccgatgaccgagggcggcgtggtgatgaacatgtcgacgttgcccgcgatcaggtcgttgatggctggacccgagcccttgtagggcacgtgcgtcatcggctgctttgcctgccgcgacagcagctcgcccgcgatgtgctggatggagccgttgcccgacgaggcgtagaacaggccgccctctttcttcttcttgccgtattcgaccagctccttcatcgagctgaccggcagcttgccgctcaccgcgacgacgtgcggtgcgcgcatcaccagcgccacgggcacgaagtccttggtcgggttccacttgatctgcggaaagagcgcggggttgccgacgtggtagcccgaatactgcatgagcagcgtgtagccgtcgggcgcggcgcgcgccacggcctcggtgccgatgttgccgctggcgcccggtttgttgtcgaccacgatgggctggcccaatgcgcgctgcagcgggtcggccaccatgcgcgcaatgatgtcggtggaccccgcgggtgcggtgggcacgatgaaggtgatcggcttggcgggccatgtgtcggcgccggcagcggaggccgcggaagcagccgaggccgtgagtgcgaggccaaggcttgcggtggccagaatgcgatgaatgggtttcatggttttgtctccgatgttttttgcagcttgtcttcccggccggcccgtcagggcgccagctcggatatctcgatgagattcaggtcggggtcgcgcatatagaccgagcggatgcgcgacgtggcgccggtgcgcatcaccgggccttcgaggatcggcacgcccttgtccttcagccgcgcgatcacgtcctcgagcggcacgctcgcaatgaagcacaggtccagcgaacccggcgtgggcagctgcgccttgggctcgaactcgtggcccttcacgtgcaggttgatcttctggttgccgaagcggaaggccttgcggttggcgccgaaagtctccagcgccatgcccatcgcatcgacatagaagcgggtgcaggcctcttcgtcggtggtggtcagcaccaggtggtccagatggtcgatcatgcgttcagctccttgccgcggcgcgcatgcgcacgcgccgcgatgtcgttgaaatccggcggcggcgcatgccgcgtgagccgatgtccggcacgggcgacctggctcggcaagtcgtgctgcaccagggcctcgagctccgacgcggcgccgatcaggccttcgagatccatgccggtgtcgtagcccatgcattgcagcatgtgcaccacgtcctcggtggccacgttgccggtggcgccgggtgcgtaggggcagccgccgatgccgcccagcgacatgtccagccgctcgatgcccgcctcgaccgccgccaccgtgttcgccagccccatgccgcgcgtgttgtgaaagtgcgcggtccattgcaggccggggtgccttgccatcacggcctcgcagagggcctgcacctgcgtgggaaacgccatgcccgtggtgtcgcacagcgtgatgccctgcacccgcagcgccgcgaagcggtcgatccattccagcactgcagccaccggtacttcgccttccatggggcagccgaacacgcacgagagcgagacgttcacgggcacgccggcctgcctggccaaagcgatgacctcggccaactgcgcgaacgactgctcacgcgtcatgcgcaggttgctgaggttgtgggtttcgctcaccgacatgacgacgttgaattcgccgatgcggctctccagtgcgcgctcggccccgcgtaggttcggcaccagcgcggtgtagaccacgccaggccggcgcgcaatgcgctgcatcacctcttcgccgtcgcgcagcgccggaatcgccttggccgaggtgaacgaggtcacctcgatcttggcgtagcccagcgtgctcaaacggtcgaccagcgcgatcttgtcgtcggtcggaatgaagcggctttccatctgaaagccgtcgcgggtggctacttcgttgatgaagagccgcttgcccttgccttctttcatactcatacggcctcgctttcttggccacggcgcaccggccagcccgcgccctgcagatcgccggtgtgttcgccgagccgcggcgcggggtgcgcgatgcgccctggcgtcgcgctgagcttgggcacgacgccgggcaccttgagcatttctccgtcggcggtgctcgtctccacgatcatctgccgcgccaggtattgcggatcggtggcgatgtcggccaccgtgtagatgcgcccgaccggcacgccggccgcatcgagcaccgccagcacctcgtcacggctgcgctgcagcgtccaggcttcgatggcggcgtcgatctcttccacgcgccgcacccggccgtcgttgtgcaccagttccggatcgctctccaggtccgtgcgctcgatggcccgcatcaaccggcggaagatgctgtcgccgttgccggccaccagcacgtagtggccatcgctgcacttgtaggcattggtcggcgcaataccgggcagcgcactgccggcacgctcgcgtaccgcgccgaaggcgtcgtactcgggcagcaggctttccatcacgttgaagaccgactcgtagagcgccacgtcgatgaactgcccttgcccgccatgcgccgtgcggtggtgcagcgccgtgagcacgccgatcacgccatgcagtgcggccagcgtgtcgccgagcgagacgcccacgcgcaccggcacccggcccggctcgccgctcaggtagcgcagcccgcccatcgattcgccgagcacgccgaagcccggcttgtcgcggtaggggccggtctgcccgtagcccgagatgcgcagcatgatgagccgggggttgagcgcgtgcagctgctcccagcccagaccccagccttcgagcgtgccgggcttgaagttctcgatcagcacgtcggcttcgagcgccagtgcgcgcaccgcctcctggccttcggcgctgcgcaggtccaggcacaccgagcgcttgttgcgcgactgcacctcccaccacaccgaggtgccttcgcgcagcagccgccacttgcgcagcgggtcgccgacgcccgcgggttcgatcttgatcacgtcggcgccgaactccgcaagcgtcttgccggcgaacggtccggcgatgagctggccgagctccagcaccttgaggccttcgagtgcgttcatctgcgtctgtctcctgtgggaatgccccaactctaagaacagatcgcgttcgccggaattgctctgacggcagcaaggcttcgcaaaacgcgaaggcccgggaacttattttctttttgccgctgatgacttggcggcaggcagcggcggagcctccggtgccttgacccagccgcgcagcaagacgccaaggaagagaccgcccgcgaagatcgcccagtacatccagactggcatgttctccataccgctgtgcaggttcatgccgaatgcggcgccgacggccatgagcggaaaggtcagcgcggcaatggtgttgagcttgtgctgcgcgcggctgacttcgcgggtcgagcgtgcctgcgcctcggctgcgtgcgcgagccggtagtcgagcgacatgcgggtgtcggccagcagcagctccaggccgcgcgtgatctctaccgccagatcgcgcaggtcgatcagcatgaggtcgtccttgacggcatcgcgcgccgcctgcaacgcggcctgcatgttcatggcggcgcgggtcagcgggatgagcgggccgagaacctggaacagatcctctgaagtttcagcagccgcgtgcctggcctcgaaggtgcccagcgccgtgcgatagctttcgagcagcttggcaaaggcccgttcgccagggttgtttcccttgtggaaccatgcgccgtccggcttgcgcaagaacactgcgggcttgcgctccgcgccggcaccggcgggcggctcgtgcaggatcaccatcaggtggccctgctcgtggatgacgcgctgtgcgccgtagctggcgcctcccagccgttgctgcatttcgggcggcagctcccagtcgtagtcgattcttcttggcatcaggcggcctgcagttctttccacaaggtgtcgaactcgtccgcaaagcggcgaacgagcgagggatcattgctcagcaccaggttttcctcgttgtagtcgcaggcgctgcgggtccagttgtagctgccgttgagcagcctcgcgccatcgaagatcgcgaacttgtggtgcatgtgcgcttcggtgcgatccaccgcaaccgggattccagccgcgcgcagctggcccacgtcgctgccgcggtcgaattccttgtcgttgtcggtaatgaagcgcaccgccaccccgcgccggtatgcggccagcacctcggtggtgatgcggtcgtccgacagcgtgaagacacacaggtcgaccgaccgcttcgcggccttcagctgttggttgatcgcctgcaggcagcccgttcccggactgaagaaggcctgcgaacgcactgcaaccgaatcgggcgaacggccggtgtcgatcgagcggaccacgccttcgagccatttgagcagggccagctgctcggggtcggtggtgcgcgatcgcaccaggtcgaacgcacggttgcgcagctggcgcaagccgtcttcgggtggcgaggcctcgcgcagggtgtggaccagcacgcggcgctcgtcgtcgctcaggcgcgcatcggccatggtggcatcgagctgggcgagcagctcgggcagcgccgcctgcggctcgagaacggaagatgaagatgcctgcatgttgtctcagtggtcctgctcgggtttgggcgcgcgcctgggcgccgcgcgggtcgcctgcacctcggcggccaggcgctccatgtcctgccgtatcgaacggtcgagttcgagccggcgttcggtggcggtcaccagcggcaggatcagctcgcggtaggtcacggcaatctgcagcatggcatcggccagccgctggccttcgttcggcccttcggcaaccggctcgggcttgggcttgagcgcatcgaccgcgcgcgccacgtcgagcatgctgctggcgatgcgctggctgccgtcgacgtcgtcgccgccgagctttcgctttcgcacgaactcttcgcagatggacgtccagcgcgcgctttcctcgggcgtcgggctgcccagcagctgggcgagccgcaagaggttttcctcggcgccggtggtcagggtttgcgcctcgccgcggtagtggtcgcgcagcagcgcatcgagctcgtcgtcgcgcatcagcgcggtgatcttgcctgcgagcttggtcatgttgcggtagctgccctgcagcttgaacggcggcgcggtgcggtaggcctcctgctgcgcggccgattcgatgtaggcgagattgaccttgagcagcaggtcgcgcgcacggaagagtcgctgcagcagcgccttgatttcttccagttcgaccgcgctgtaggcatgcgagagcgcgctgctcggcatctcgtgcccctgcgccatcttcaccagcagctgcacgtccttgggatcgcgcgaggccagcggcatcagcgtggggttggaggtcaggctgttttcgatgtacgagagcgcaaacgccgcctctcggcccgaaagcacgtcgcccaggttgtagatgtcggcgcggttggccagcatgtccggaatcttgaacacgtcgcccgactcggtatacgggttgcccgccatcacgatcgcgaagcgcttgccgcgcatgtcgtagctgcgcggctcgccgttccacacgccttcgatgcgccgcgtgccgtcggccagcgcgatgaacttctgcaggaactcggggctggtgtgctggatgtcgtccaggtacagcatcacgttgctgcccatcgcgaggccgaggttgagcttctccagctcctgccgcgcggcgctgttgggcgcattggccgggtcgatggcggtcacgccatggcccagcgccgggcagttgatgcgcacgaagatcaggccgagccggtccgccacgtattccatgagcgtggtcttgccatagcccggcggcgagatcagcagcagcaagcccatgcggtcggtgcggctgcccgcgcccgccgagccgatctgcttggcaaggttgtcgccgatgatgggcaggtagagctcgtcgatcagctggttgcgcacgaaggtcgagagcggcttggcctggaactggctcagcttgaggcgagcccgctcccgttcgagcagttcgtggcgcaggctgtgcagcgcctcgtagcccggcacggcgtgcgcggcatgaaacaggaagcggcgccagaagtcgttgaggttcagcgtcacgcggccctcggccacgcgcggatgctcgccgcgaaggccctccaccgtgcggtcgagcgctgcattgacgcgggtgcgctgcaacggcatggccagcacgctggcagcgtcgtccacccagtcgaccgactgcgatgcctggtgggtggcgtaggcgcgcacccagtcgcgcgccaggcgccagcgctccgcgggcggtgcggcgtcgaggtcgtgctgccaggcgtcgcgccggccgccgcgctcgagttcgcgcagcaatgcggccgcaaggtcttcgcccgcacccgaaacggcccaggtctccccgccgtggtcgccggccagttcgcgcacgaggtatgcggcggcctggtcgcacagcgtggccacgcggccctcatgagcgtctcgctcttcctcgctggcactctccgcgagcggcagcaggtcgggcacgacgtcgcgcgcgaagtgcttcagcgcgcgcgccgtatcggcttcgagctgctccagcgcatcgcgccggccgaacagggcttgcatctgcagtgcggcccgcgcgcgccgcagcagcgattcgcggtgcgcaatgaggtggccgtgctgccagtagagcaaggccagcgcgcgttcggtcggcccccaggccagcagcccggcctggtcctgcatggcgacgagcgcacccaacaggcgcagcgcatcgtcgtcgtgaatacccttctggtagccctcctggtagcgcgcggcagcaaagcggcgaaccatgtcgagcagctgcggatgcagcgggtcctcggccagcagcgtgagcacgtcgacccagctgcgctcggacttgccgtcgagcaatgcctccagcacgcggcccgcaaggtattcggcgcgcgacagttcggacgtttccgacaccagcgactggttccagtagcgctgcaacggcagcagccggggttcgtcgacagggctctggtagtcggtgcccgtcacctggtaggccatgccttcgtcgcgggccaccagcgtcaggtcgaccggctggcggtgcacggtgaaggcatggcggcccaggcgaagcgtgtctccgccctcgctcacgagctcccgcttgtcgcggatcgaacgcagggcctggtcgcgcgcggtcttcaggcgcgtgtcgagttcgtcggcaggcaccgcggcgcccagcgtgcgcaaatcggcaatcaatgcatgcagcttgccgagcatcgggtcggccgcgaagtagctgtggacctgcgtgaggtcgccgaactgggcgatgcggcgtggaatgccgtccaggatgcggcccgccgcatcgatcagcccctgggcgcggcgctggcgggcttccaccaggctctggcggcgggcagacagcgcctcgtagacggtctcgcgcttttcggcgatgtcggccaggaagtcttcctgttcggcgaatcggccttcgacttcttcgagctgggcgagcaggcgcgtgagcgcgtcgtcgcacttctcgggcgtgtccgcgaactccagcgcgttttccaccgcctggctgaagagcttgaactgggccccgaactcggcgcgcgcctcggtcgcgcccagcgacttgcgccgtgcgcgcgcatcggcgcgcatgcggttgatgtcggcgtagatcagcgagatgcggtcgagaatcgaggtgcggatcaccgcatcgccgcccggcaggctgccgagctgctcggtcagcaggtcgaggccggcggcctgctcgtcgagcgtcgccagcatctggccgagcgcgggcgaggtggaaaggttcggcaggtcgagcgccagcttgtcgagcgcctggcgctggccgttgaaggccgtgtcggccgccaggaactgcatcgcgcgctcgccgatgcgctgctgctcggtctccagcgcagcgtccatggcggcgatgcgcggcaggtgggcgtagcgcagctccttgagcatctgcagcgcgccgcgccgttcgcgcagccggcccagcgccttcacgaaatcgtcgggtgcgcgccagagggtgctggcaatgtcgaccagcagcgcgtgctgctcgtcctcggcccgggccagcgcgcgcgcggtttcgcggcggatggtatccaccttctcgaactcggccagcgtgctgcgcgccacgtcggcaatgctgcgcagctcggccatgagcccggcggcgtcgggcgcgtcgagccagaagtaggcgtcgcttacgcgggagcactggcgaatcaggtcgtcgtaggcggcccgcgtgggcgcctgctcgcgcaccgcgcgggcaatgcccatcaggtcggacacgccgcgcaccagctctgcattgccgatcttgccgaagaaaccggtggccggtggctgcgcgctcacatgctcttcgctggcaaacggcgtctgccacagctgcatctggtgaacgcgcgcaggctcgccctggtcgccgtgaaacaccagcatgcggccgtcggcaaagcgcgcatacccgttggcgatgatcggcgttgcgagcttcttgtcgatcaggttgtagttgaagaaggcatagcgccccggcttcgggtcgtagaagacataggccacgtcttcgccgttgggcgagcgcagcatgcgcttgaagcgcaggctttccaccacctcgcccggcaggtcgaagcgcttgtattcgcccgactgcagatagtagccacccggaaaaatgatgccgtggtcttcgggcagctgcacgcaggagccgccgatggcgtcgatgcgctcgacctgctgcgtgcggatgttgaacaccaggtagcgcgtgacctgctcgcggtagggcttcacgcgcagcaggatcagcatgccgagcttggcccaggcaacctcggcgtcggcaagcgactggttcttgtcttccaccggctcgctgtagatgcccaggccggtttccgtgttgttctcgatcttgacggtcaggtcgccgcccagcgtttcgacgaacaccgtgtcgagcacgttcacatggggatgcttgcctcccacatggtcttcgcgcgtggcgacggtccattcgaagtcgtggctcgcgggcagcgcgatgtcgcgctcgccgcggttgtcgatgtagtggatgccgccattgcgctcgatggcccagcggaacacgcgcacgtcgtgcggctgctgtccgatcttgaaggacgccagcagcttgtcttgcgtgacacgcagctgcagcagcgtggcctgcttgtagtaggcgtaaagctcgcgaaagtcggaggcgaagcgcgtgtcttcgagaaaggtgccggccaggggcaccgcctgcagctcgtcgttctcggtggcggcctctcccggcaccgccaggcggtacaggccgaacacgtcgcccaccgccgtttccttgcgcaggccgatgaagacgttgtagccgaacagcagcaggtcgccaatgcgcacgatgtcgcgtgccacggcattgttctcggtgcgcgcgcgggtgcgcagcaccagggtctgctcggagcggccgaactcggtgaggcgccgctcgttgagcgcctgcgtctttttcagcaagccctcgccctgggtttcaagccgcttcttcagcaggtcgtagctgccgctgccggacaccagggcctcggtcgggtcggtctgggcctgggcgccggccggcgctcccgattcttccgtgagttgcatagatcggcgcggtcagtccgcgcgcagcaatgcgagcaattcgtcgcggtggggctgggtgtcgagccaggcgcggatgcggtccagctcgtcgatgcagtcattgccgtagcggcggcgcagtgcggcaagtcgcacctcgcgcacttcttcggtctggaggcgccgctgccatccgtctgacagcaattcatcgagccggccggccaagccgcggctcaccagggcacgccactcgcccgcgtcgaaccagaggttctggcaagcgatgcaacggtcgatgcgaaagtcgggcccggcgctcacgcgcaggcgctgcatgagccggtcgcattccggacagggtcgcacggcggcggcgtcgaacacctcgatgacttcatcgtcgaccggatggggatttcgcgcgggatcggccgccttccaggcgcgccagtcgtccatgtccatgaccatgccgccgcagtcggtgcagtgcaccgccagcagcgcttcggccagtgccacggcttgcatgggggcgtgtgcggagcaaccgcatttcaggttcggattcatcgcgcgcccactcagttgcggaaggtggagatcaggttgtggagcgcggtcttctggctttcgctgccgtcgctgctgatgcggctcatcagcgcggcaacgctgaggttctgcatctcgccagacgaggtgccaagtgcgccgacaagctcgcgcaggtccttcaccacgtcgcggtcaccggagagctggtccttgaaggcgaccttcagcgtgttgctcttggagatgacgccatcgatgcccttgcccacggaaagcgagcgcacgaagctgtcgaagtagtcgccctgcccgcccacgatgtcgatcttggcattggccagcgcggtgcccagcacctcggcctgctctttcgcgatggaggtctgcgcgtcgatgcccttcatggtttcggcgtgcgacttttcgaggcgcatgcggaattcctcgtggtcgcgggtgtccgggctcatcgccttcatggcttcgaacttttcatgcaggcccttggcctcggcgctgaagcgggcttcgatcacctgcgcatcggcctggccggacttcagggtggcttcggcatcggctgtgcgcacgttcacttcggccaagccgagcttttccttgcccgaggcctcggcgtcgaacttggcgcgcatgccggcggcttcggcctgcgaacgcgcttcgatcacctgcgcatcggcctgcccggccttgaggatggcgtccgcatcggcctgacgcacatgcacatccgcaagacccagcttttccttgccggaggcttcggcctcgaaagtggcgagccgggcttgcgcggtggcgatctcgaccttggcggcggccaggcccggtgcggcggagatggcctccatgccctcggcctcgcgcttcttcgactcggcatcgcgctcggccaccttcagcttggcatcggccagcgtgagttcttcggctgccttgtggcgcgcgcgcttttcctgcgtttcggccgctttcacgtcgatcaccatcttctcgtcggcctggccctcggccatgatcaccaccgacttcttggtgcgctccgcctcggccaccacgcgcagttccttgatggcttcttcctgctcggcgacggtgcgctcgaccacgatgcgttcgcggatcacgtcggcaatggccttcttctgtatttcgaccgccttgtccttctcgatgcgctgcagcgtcacttccttctcgcggtcgacaatttcgaggtcgcgggcgcgcgtgactttttcttcctcgatggccaccgcgcgcttgcggttgttctcggccacttccttctcgcgctgcacgttctcctgctgcaccgagacggattgctcggccatcagccgggcggtttcggacttggtgcgctcttcggactggatcttggaggtttcggcttcttcgcgggcgcgcacgctggcaatttcgcgctgctggcgcgcggtggcgtcggcctgctggcgctcgagctcgagcatcgcttcctgcgtctcgacgttcttcttcttgatctgcatttcctcgttgcggcgcagctcgttggtgcgcacatgctcgaccgccgtgagttcggtgatcttcttgatgccctgcgcatcgaggatgttgttggcgtcgagctccgacagcggcgtttgctcgaggtagtcgatggccgcgtcttcgagcacgtagcccgagaggtcgttgccgatctggctgatgatctggtcgcgaaagccgtcgcgcgcctggtacaggtcgacaaaatccatcgacttgccgacggtcttgagcgcttcggagaacttggccgagaacagctcctcgagcgtttcatggttcgacgcccgcgcgcagccgatgccctgcgccaccttgagcacgtcgtccgcggtcttgttgacgcgcacgaagaacttcaccttgatgtcggcgcggatgttgtcgcggcagatgaggccctcgttgccggagcggtcgatctcgatggtcttgaccgaaatgtccatcagttcggccttgtggatgatcggatagaccatccgccccgtgaaggtgacgtcgggctcggcgcgcagcgtgttcacgatgagcgcgtggccctgttcgatcttgcgatagaacttcgcgaacatcgcgaacaggccgaggatgaccacggccaggatggccacggcaaagaggatgggctccattttttctccagagatgctttgagagcgaaacagttgatcgggtgggccgcgctcagacggcgtcgtcgtgcgccgcgatgaggtagcggccggccacctcgtcgtattcgagaatcagcgcctgcgatccgcgcgtcaggctgttgggcgttggcgcccagacgcggatgttcaggctggcaccgcggcgggccacttcggcacggccgtctttctcgttcaccacgccggtgacgacgcggcaggcctgcccgaccagtgccgcattgctcacggccgtgtggctcacgaacaagccgcgaaggggccggatggccacggccgtcacgggtatggcgatggcggcgctcgccaacagcagcaccgtgccggccaggagcttgagcggcagcgtgggcaccagcggcagcagccactccccgccaaggcaggacagcgtccacgacaccagcaccagcaggctcaccgccaccgagaacggcacgccgttgaggccgaacgcaaccacgtagctcgcgagctgccccacgtcgctggtgtcgccatcggcatgggtctgcacatcgacatcgatgccgctgtgctcgatgtcgaccatgccggccacggcaagcacccaatagatcaccacgacgcccagcagcaccgtgtagatcgcggtggggtaccccgtcaccgcatccatgaaatttcccattgaccctcccgcgtgcgggttgtgtttttttatctgcggcccggcttccctgcgccggtgcccttcttctttccaccacttgcaaaagcaatcagatctcgcgtggccctctccttgatggccagccggtcgtccggggcgagcccatatctcgccgcaagaaactcgtagtctgccgcattcagcgacacggtcagccgcggccgcttgggcttggccgttgtcgcgaggcccagcacctgccggatctggtcggaggtggacacgtgctgctcgaaagccgccgtgcgcaccgcctccagcacggcctcttccacgtcgaacgccacctggacggcgcgtatcgcctcgtccgagccttgccagcgaaccggcttgacccgcacggtcattttgaatcgggcgccgccgggttggcctggcgggcgcggatgcgttccatcaccttgccggtgcggtcgacatcgctgccgatgcccgccgccgccagtttcttctcgagcgcgctgtggccgagttcgttttcgagcgcctggcccgcggccatccggtcggccaggtcttcgtgccgcttgcggatgcgctccagcgattcacgcgcgttggacaggcgcgaaccacccgcgccgatgttctcggagatcgactgcgtggcgcggtagacgctctcggtggtcttggcgatgccgatctcgcgttcatgctcgcgaatgcgcgcttcggccgtcttgatgaggtccttgagcttggacacctgcagcgaataggaggcatgcgccttggcctgctcctccagttcgctttcgagcgtgccgaccttggccgccacgtcgagcgccaggccttcctgggtcttgttgagcgcctcgagcgcgagcccttcgtagcgggacacttcgttcttcaggcgttcgatctcgcgggccgactgcatctccttggccatcacaccggtgagatcgcccttggccttctcgatgctgtgcttggcgtcgatgatttcctgctcgtagatgcgcgtggcgttgctgtcgaccacgctctcgccgatttcgcgggcactgccgcgcagcaaggtgaccagcttcttgatgactgtcatgatgatctccgcttagttcaggaattcggacagggcgtccagcgcatcgagcgcgttgtcgctgagcaccgccacttcgcgggccacgtcttccacgcccgcattgcgcccgagcgcgccggtgagaacgtagcggccatcgacccgcccgaaggaagacagcggcaccgaagggttcaggtcgagcagcgattcgagcagttcggtgcggcgctcggccttcacttcttcctcggtccatagatagcagatgcagatgacctgcatgtccgaactggtgatgaagatgggcagctcgtcacggccttcgatgctcacctggatcacgggcgtctggcccggaatcggctgcagttgcacggccagcccacccatcgcggcaccggccaggacgtccagccccttcagttgatcgagcagtgattgcatacctctccttggagttgataccgacggaagcgaacggtgcttcgatgagcccactataggtctgccgacataacatgtcaaagaatcttttggcctatgtcccatggctgtcggcgccggcacgatctctagaatccggcgatggccagccttatcaaccccgcacgtgtcgatttcgtgacgctgcgcctgttctgcgccgtggcccagtcgggcagcatcaccaagggcgcggaggcctgccacctggcgctctcggcggccagccggcggctgtcggacttcgaggcggcgaccgggtcgaagctgctcgagcgcagctcgcaaggcatcgctctcacgcccgccggccacgtggccatgcagcatgcgatgcggctcttccagggcttcgagcagttcagcaacgagcttggcgactactcgagcggcgtgcgcggccacgtgcggctgtgggccaacatgtcggcgctcaccgaattcctgccggccacgctggccgcctttctgggccagcacccggacatccgcgtcgaggtcgaggagcaactgagcggggacatcgtgcgcgcgctggtcgacggcctggccgacgtcggcgtgttcgccgagaacacgccggcctacgggctcgacgtggcgccgttccagaccgacgagctggtggtgctgtgcgccaggcagcatccgcttgcgcgcacacgccggacggatttcaagacctgcctcgcgcacgagttcgtgggcctgaaccgcagcagctcgctgctcgaactcacctcgcgcgcggccgagcaggcgggcattccgatgcgcctgcgcgtgcaggtgcgcagcttcgatgcgatgtgccacatgatcgcggccaacctcggcattggcgtggtgccgctcgcagcctgcaaggcgcaggtgagcgcgctcggcctgaaggtggtgcggctcaaggacgcctgggccgttcgccggctgctgatggccaccaagaccggcgaaaccttgtcgccggcggcgcagctgctggttgcgcagctgctcgcgtcgtcgacctgaagcgaagcctggttcaggccatccgcttcaccatgccgatccacttctcgaacgacttcatctggtcgccgacgaacttgcgggtggtttcgtcggtgcagtttccttccgcatcgaacttgccgcccgcaccgccgatgaagatctcgggcttgaccagcaccatcgcattcacgaacagcatcacgcggcgcaggtcgtactgaacgcgcgcgccgcccagcgggccgggagcggccgagagaatggccacgggcttgttcgcgaaaggctggtcttcgccgcggctgacccagtcgatcacattcttgaacacgcccggaatcgagaagttgtattcaggcgtggcaatcagcaacccgtcggcgcggcggatccgctcgcgcagcgcctgcacgggcgcgggatatccgtgggccagaaggtcggcgtcgaacggcggcacctcgcgccattcgacgacctccatgcgcatggaatcaggcatcagcgaaccggcgaggttcagtgccgcgcggttgatggaaccgctgcgaaggctgccgcagaggccgacgatgtcgagtgtgctcattgctttcctttttcctgggtcattcgaatgtgaagaagtggggccgggcgcgtggcgtcacggcagctggaatccggccttgagagtttccctcaagtggctcacgaacagattcaccgcgcgcggtatgtgcagcgagtacgggcgtatggcgtagatctggtccgcgaaggcgcccgtgggctgccagtcgggcagcacctcgaccagcttgcccgcctgcaacgccgactgggcgctgaaatcgggcagcagcgcaatgcccagcccggcctgggcggcatcgcgcaatgcttcgctgttgttggctgccagcggaccggcaatgggcacggtgacccgctccccaaggcgcgtgcggcccgtgcggcgctcgaacgaccagacgttggtttcctgcccgcgcggatagtgcaggcagtcgtggtcggccagcatgggcggcgccagcggcgtgcccttgcggcgcagataagcgcggctggccaccagcaccgatcgcgtgtcgcacagccgccaggccacgtgcgtgtcgggtggcgatgccgcgtgccgcaccgccaggtcgaagccttcggtcgcgagcgaactcagccggtcggagagctccatctcgacgcggatcgacggatgcgccagcagaaagtcggccagccgcggcagcaactgctgccgccccagcgccaccggcgcggtcacccggatcaggccgcgcggttcgccggcatggtcttgggcctgcaggaagctgtgggcaatctgctcgaagggttcgcgggtctggtcgaccagctgttgcccggcctcggtcagccgcatgctgcgggtggtgcggcgcacgagagtgacgcccacggcccgctccagctcggcaatgcgctgactcatggccgccttgctcacgcccagacgcgccgcggcggcggtgtagctgccctgctggccgagcacgatcagccagtgcaggtgtgcccagagagattcggctttttgcagatccatggccgcattgttcaccatagcgaacaaacagttcaacttccaggtctaggcaggtgcccttcccttttctagactacgcctcacttcattcttggcggtacccaatgacccagcagattgcccatttcatcggcggccagcacgccgccggcagctccacccgcacgcaggacgtcaccaacccggcgaccggcaaggtcacgggcaaagtggcgctcgccgtccaggccgacgtcgatgccgcggtagccgccgcgcaagccgccttccccaagtgggccgacacgccgccgatccgccgcgctcgcgtgatgttcaagtttctggagctgctcaacctgcacaaggatgagttggcccacatgatcaccgccgagcacggcaaggtgttcaccgacgcgcagggcgaggtctcgcgcggcatcgacatcgtcgagttcgcctgcggcattccgcagctgctcaagggcgacttcaccgaccaggtttccaccggcatcgacaactggacgctgcgccagccgctcggcgtggtggcgggcatcacgcccttcaacttcccggtgatggtgccgatgtggatgttcccggtggccattgccgcgggcaacaccttcattctcaagcccagcccgaccgaccccaccccctcgctgcgcatggccgagctgctgaaggaagcgggcctgcccgacggcgtgttcaacgtggtgcaaggcgacaaggccgcggtcgacgcgctgctcgagcaccccgacgtcaaggccgtgagcttcgtcggctccacgcccattgccaactacatctatgaaaccggcgcccgcaacggcaagcgcgtgcaggcgctcggcggcgcgaagaaccacatggtggtcatgcccgacgccgacatcgaccagacggtggatgcgctgatcggcgccggctacggctcggccggcgagcgctgcatggcgatcagcgtggcggtgctggtgggcgacgtggccgacaagatcattcccaagctcgtcgaacgcacgaagacgctccaggtgctcgacggcgagaacctggcggccgagatgggcccgatcgtcacgcgcgcagcgcacgagcgcatcacgggctacatcgcccagggcgagaaggaaggcgcgaagctgctggtcgatggccgccagttcgacgccagcaaggccggcgcgggttgcggcgacggcttctggatgggcggcacgctgttcgaccatgtcacgcccgagatgcgcatctacaaggaggagatcttcgggccggtgctctcttgcgtgcgagtggccaacttcaaggacgcggtcgacctggtcaacgaccatgagttcggcaacggcgtgagctgcttcacgcgcgacggcaacgtggcgcgcgagttcagccgccgcatccaggtgggcatggtcggcatcaacgtgccgatcccggtgccgatggcatggcacggcttcggcggttggaagcgctcgctcttcggcgacatgcatgcctacggcgaggaaggcgtgcgcttctacaccaagcagaagtcgatcatgcagcgctggcccgagagcatcggcaagggtgccgagttcgtgatgccgaccgccaagtaggcggcgattgccgggtggcgacaacgggcgccgccgaagcggcatgggcgcgcccagggttaacgaaaagctgacttgccccccgcccggggagcggccagacttgcgcatgaccctgtgccagcgcccatgacaacaaacaagaagcccgcgcgaagcctgtcggccgtgccctccaccctgcggattcccctcgccgcgcgcgcctcgggcgatgcgatgtttccccagatggcggtgcgggacgcctacgccgcatccatcctcgagaagatccgcgatgacgggcaggcccttcccgaagatcggacgaccatctacggcatcctgagccgcacgcggcgctttcgcagccttgcgcaggagttcctcaagcagcacccgggctcgcgtgtggtgaacatgggctgcggcctcagccactactttcaatggctggacgacgacaagtgccgcatgaccgacgccgacctgcccgaggtgctcgcgctgcgccgcgagctcattccggaaaccaatacgcgccacgatgtgcgcgcgctcgacctgacatcgccccgctggtgggagcagctcgacctgccgcgcaagcgtcacgggcaaccggtgttcctgttcgccgaaggcgtgctgatgtacctcgagccgcagcaggtgcaggccgtgttcgcgaccttcgacgagcgcgcgcccgcaggctcggtgctggccttcgatgcgatgtgctggctcggggtgggccgcgcagcgcagcatccatcggtgcggcccaccggcgccgagtttcgatgggggctgcgcagggccgctgagttgacgcaaggccatccacgcctgcgcctggactcgacctaccgggtgctggaaggcttcggcctgccctacaccttgttcgcgccgctgctcctgatgctgcttggcgtgtcgatctatgccgtctatgcgctgagcgcggcggacaacgccgatacataaacgcacaaatttctcctcgaatgctcaaatcccggccttgtccggcccggagtgcgcaggttggctgacgcggaatgggccgccgcccaggcatgctcggcgctcttcgccgcgaaatcccggcgcgggctgcgctaggatggttttcttccgaagcaaccggccggcacccgccgacgatgccgcgccgtcccttgcatcccttgcgtctttcccaacgtatttccaagactcgcaaccctcaagaaacacatgcctgatcgccgatccttccttgccgcaggtggtgccgccgccgcactcgccgcccttggactgcctgaagaggcgctggccgccaatggcctgcagctgagccagccttcgcccttctcgttcgaccgcctcgtggcacaggccaagcgcctggcgtcgcagccctatgccgccgccgcgccgctcgcgcccgacgtgctggagcgcatcgactacgacgcgcacggcaagatcaagttcgaccccgccaacgcgctcttccgcgacggccccggcgcctttcccgtcaccttctttcacctcggccgcttcttccagacgccggtgcgcatgcacgtgctcgagaattccgacggcgatgcctttgcgcgcgaggtgctctacagcccctcctacttctcgatgccgcccgacagccctgcgcgcgcgctgccgcccggcgcgggctttgcgggcttccgcctgcaggagagccgcctgggcgaccagggcaagctggactggcagaagaacgactgggtcgcgttcctcggcgcttcgtacttccgcgccatcggcgagctgtaccagtacggcctgtcggcgcgcggcctcgcgctcgacgtggcggtgcccgacaagcccgaagagtttccgaccttcacgcgctactacttcgaaacgccggccgccaacaacaccacctcgatgacggtctacgcgctgctcgaaggagcgagcgtcacgggcgtgttcaagttcgtgatgcagcgtggcaaggcggtcatcatggacatcgacgcgcgcctgttcctgcgccgcgacgtgtcgcgcctcgggctggtgccgctcacctcgatgtactggtattcggaaaccatcaagcccaccgccatcgactggcggcccgaagtgcacgactccgacgggctggccatctggaacggcgcgggcgagcgcatctggcgcccgctcaacaacccgacgcagacccgcgcctccgcgttcgcagacacgaagccgcgcggcttcggcctgctacagcgcgaccgatcgttcgaccactaccaggacggcgtcaactacgagaagcgcccgagcctgtggatcgagccgctgggcgactggggcgaaggctcggtgcagctgatcgagatcccgaccgacgacgagatccacgacaacatcgtggccttctgggtgcccaaggccgatgcgaaggcgggcgcgagctacagcctgcagtaccgcctgcactggaccgaccaggagccctttccgtcgccgctcgcgcgctgcgtggccacgcgcatcggccgcggcggacagccgggccagccgcgccccccgggcgtgcgcaagttcatggtcgaattcatcggccagccgctcaccaccgtgcccttcggcgtgaagcccgaactggtgctgaccgcgccgcgcggcaagttctcctatgtctttgccgaagccgtgcccaacggcgtgcccggccactggcgcgcgcagttcgacttcacgcctgaaggcaacgagcccatcgacatgcggctctacctgaagaccggcgacaagacgctcaccgagacctggctgtaccagtaccaacccggttgatcgtcatcaacgagcccggcccgatcagcgcttcttcaccgacaccagctcgacttcgaagttgagcgtggcgttcggcggaatcacgccgcccgcgccgcgcgaaccgtaggcaatggccggcgggcaggtcagcttggccttgccgcccggcttcatcttctgcacgccctcggtccagcaagggatcacgccgttgagcggaaactcggtgggctcgccgcggctgtaggagctgtcgaattccttgccgctgtcggggaaggtgccgcggtagtgcaccttgaccacgtcggtcgccgcaggcgatgcgccggtgccttctttcagcgactggtagaccaggccgcttggcgtggtgacgggcgcggattgcgcccacgcggtggacacggcgcacacggacaagaaagcagcgcagaagatcgacgaagaagaactggacttcactggatacctcagaagaatggggaaagcatgattatggccagcgttggaacagcccttgctttgctgcatatgcactgtcaacatccgcacagagaggaagccccatgcagtccatcgacgccacaccggccgcaatcgccgttccggccggcaccggccacctgaagaaggtgctcggccccatccagctctggggcatcgcggtgggcctggtcatatcgggtgaatactttggatggagctatgggtggaacacggccggcacgctcggcttcctggtggccacggtgctggtggccacgatgtacaccaccttcatcttcagcttcaccgagctctccaccgccattccgcatgcgggcggccccttcgcctatgcgcgtcgcgccttcggtccgaccggcggcttcgtggcgggctttgccacgctgatcgaattcgtctttgcaccgccggccatcgcgctggccatcggcgcgtacctcaacgttcagtttccgggcatcaatccgaagtggttcgcgctgggcgcctatgtgatcttcatcgggctcaactggatcggcgtcggcattgcggcggcattcgaactcttcgtgacggtgctcgcaatcttcgagctgttcgttttcatgggcgtggtcacgccgggctggtcgatggccaacttcgtcgccaacggctgggccgggggcagcgtgctcaacggcgcggccatctccggcatcttcgcgtcgatacctttcgcgatctggttcttcctggccatcgagggcgcggccatggcggccgaggaagcgcgcgatccgcaccgcaccattcccatcgcctacaccacgggcatcatcacgctggtggtgctggccttcggcgtgatgatcttcgcgggcggcgtgggcgactggcgcaagctcgccaacatcaacgacccgctgccgcaggccatgaaggcggtggtgggcgacaacagcggctggctgcacatgctggtgtggatcggcctcttcgggctgattgcctcgttccacggcatcatcatgggctactcgcggcagatcttcgcgctggcgcgcgcgggctacctgccgcgctacttcgccggcctgagcccgcgcttcgacacgccgcaccgcgcgctgctggccggcggcgtgatcggcgtggtcgccatcttcagcgacgagtgggtgcagttcggcggccagacgctcaccgccaacatcgtgaccatggccgtgctcggcgccatcgtgatgtacctggtctcaatggccgcgctcttcaagctgcgcaagagcgagcccgacctgctgcgcacctaccgcgcgcccttctatccggtgtttccagccatcgcgctcgggctcggcgtggtctgcctcggcgccatggtgtggttcaacgccatgctcacgctgctgttcctggcgctgatggcggcggcctatggctatttcctgctgacctccgcacagcgcaaggcggcggcgcccgacgagatgctttcttcgagcaccatcgcgtgaacgaaagatgcgctatcgcaccaccatcgccggccaggtcttcgccttcgacgacctgaagcaggtcatggccgtggccagcccggcgcgctcgggcgactacctggccggcgtcggcgctgccaccgcgcaacagcgcatggcggcgcgccacgtgctggccgagacgccgctcaagcggttcctgaccgaagcgctgattccctacgagagcgacaacatcactcgcctcatcatcgacagccatgacgccaaggccttcgcgccggtgtcgcacctcacggtgggcgacttccgcaactggctgctgtcggagcaggccaccaccgaagcgctgacaacgctggcgccgggcctcacgcccgagatggtggccgccgtctccaagctcatgcgcaaccaggacctggtgtccgtcgccaaaaaatgcagcgtggtcacgcggtttcgagacaccatcggcctgccgggccatctggccgtgcgcctgcagcccaaccacccaaccgacgacctgcgcggcgtggcggcctccacgctcgacgggctgctctatggggcgggcgacgcggtgatcggcctcaacccggtgtccgacagcatgcaggtgctgggccggctgctgcacatgctcgacgaagtgatccagcgcttcgagattcccacgcaaagctgcgtgctcacgcacgtcaccaacacgctcaagctcgccgaagcgggcgcgccggtcgacctggtgttccagtcgatcgcgggcaccgaaaaggcgaacgtctctttcggcatcacgcccgagctgctcgacgaagcctatgccgcggcgctggcgctgaatcggggcaccgtcggcaacaacgtgatgtacttcgagacgggccagggcagcgcgctctcggccaatgccaacttcggtgtcgatcagcagacctgcgaagtgcgcgcctatgcattggcccgccgctacaagccgctgctcatcaacacggtggtcggcttcatcgggcccgaatatcttttcgacggcaagcagatcatccgcgccgggctcgaagaccactgctgcggcaagctgctgggcctgcccctcggttgcgacatctgctacaccaaccatgccgaggccgaccaggacgacatggacaacctgctggtgctgctcggcaccgcgggcatcaacttcatcatgggcgttccgggcgccgacgacgtgatgctcaactaccagagcacctcgttccacgacgcgctgttcctgcgccagacgctgggcctgaagcgcgcacccgaattcgaagcctggctgcagcgcatgcagatcaccgatgcagccgggcagcttgcgccgccctcggccaaccgcttgctggcggacatgagcgggctgaccgcactcgggcaatgagcagcggcaacaaagacagcgtcacgccgaacccctgggcgcagtggcgttcggccacgcccgcgcgcctggcgctgggccgcgccggcgccggcatgccgaccgacgagacactgcgcttcggctgggcccatgccatggcgcgcgacgccattcatgcggcgctcgacgtcgacgcgctcgaggccgcgctgcaagaacagcattggcaggtgatgcgggcacgcagccgcgcggaagaccgcaccacctacctgcgccgccccgacctcggccgccagctcgaccccgccgacgcggagcgcctgcgcgcgggtgcgagccgcggttgcgacgtctgcctggtcatcggcgacggcctttcctcgctcgccgtggcacgccacgccgcaccgctcttggccgcgctgcgctcgcagctgccggccgagacgcgctttgcccccgtcgtcatcgccacgcaggcgcgcgtcgcgttggccgacgaggtgggcgaactgttcggggcgaccttgtcggtcatgctgatcggcgagcgcccggggctcagctcgcccgacagcctcggcatctacctgacccattcgccaaaacgcggccggcacgacgccgagcgcaactgcatctccaacgtacggcccgaaggcctgccctgcgaagccgccgcgttcaagctggcctggctgatgcgggaggcgctgcaaaaagggctgaccggcgtcgggctcaaggacgagagcgatctcgcggtgctcgagccgggccgcccggcgccctccttgcccggacaggggtctttgccttcataagaatagtcaatagaatggttgttaagccacttaataaccattttattgatgccaagaagcagcaacagcctttctgccctgccccagcagaccgctccgccattgaaaaacctcggtctgcgccttcgtgctcaccgggttcatcgcggctggacgatcgcagaaatggccgaacgcctgctgtgctcgcccaccacgttgcgcgcgctcgaatcgggcaggccgggcaccagcatcggcttgctggcccacgcactgtggctcttcggcgagatcgattcgctcgaagcattggctcccgcacccgcgggcctcacggccaggcgccgtgtccgcaggtccgctgcgcacgggcctgcaggggtgatcgcggaggacgaacgtgatttctgacgaggccccggacgaacggcgcatctacgtcgggctcgcgagccgcacggacgacgaggtgcagcccgcagggctgatgaagctcgttcgccgcggcgtcgtggagtcgggcgaattcgcctacggccgacgctacctcgaagattccgcggccacaccgctcaaccctgagcacttgccgctgcgcgatgccgctttcgcgcttgcggagcggcgcatccgcgagggcggcgccatgccgctcacgctgcgcgatgccctgcccgacagctgggggcgcaaggtgctcgagatccgccatggcaagccgctgtccgacatcgatgcattgctgctgaccaacgaggaccgcatcggcgcgatggtgttcgccgaatcgctgccgatccggagcgaggaaccgccctccatgctctggtcgctggaggagctcgccgaagcgtcccaccgtgtcgaagccggcatggagatcgggcccgacatgcaccggctgctgcgcggcggcagcctgggcggcgcgcgccccaaggccgcctttgtgcacgagggccagcgctacatcgccaaattttcgtcgcgcggcgacgaccacgacgtggaggtgatcgaggcggcgactctctggctggccagcgcctgcggcatccacgtgcctgcgttcctgttgcagcccctggcatccggccacgccttgctggtggagcgtttcgatcgaaccggccccgtgaaagacgagcagcgccatcactacctgtcggcctcggcgctgctcgatgtgccctatgactccagccgcggcagctatgtcgaactggcgcagctgctgcggcgcatttcccggcagccgcaggaagacctggccgagctgttccgccgcctggttttcaacctgaccgtgggcaacagcgacgaccacgtcaagaaccatggtgccttgcggcacgaagacggcctctggcgcctggccccggccttcgacctcgtcatgcagttgggcggtcacacgggctaccaggaactggccattcttccggggcagcacgcatcgagcctcgaactggcgcgcgccgcctctccccatttcggactgtcggcagcgcaggcggacgagatcatccgcaccaccgaagaaaccgtcgccgtgcaggccgccgcgagcgtcgaggcagcagggggaaaccgcgaactcgtgcgccgggtggcggcgttcatcgaacagcagcacgcacgcatccgcacatagctggcatggctggcatggctgatgcgtaggtcgaggcgggaagtgtctcgggcgctgaatgcgctcgctgcttctcatcgacaaacgcacaacaacagggatcgcatgcaacgccgcctcgtcctcctcaccccgctcgccactgcgctcgtcgccaccggctgcgccagcctctcgcccgccaagggcctttcgcccgcccactgggacgccttcaaccgcgcccagatcgaaggactgatcgccagcctcggcaaaggaagcccgggctacagcgccgccaggccgccttacgtcgtcttcgactgggacaacaccagcgtgtttctcgacatcgaggaagcctcgctgatctaccagctcgaaaacctggcgttcggcgccacgcccgcgcagctcgaagtggcgctgcgcaagaacatcccgaagaaggacttcgtgccggcgcacaacaacgcagccggcaagcccgtcaacatcgatctgctggtgcccgacatcgtggccagctacacctggctctaccagaactacaacggcctcaagggcagccagccgctggccgcggtgaagctgagcccgcactacatcgccttcaccaccaaggtgcgctacctgtatgaagcgattggcgacaccttcgaccacgacacggcctacccctgggtgacctacctcttcgtcggcatgaccgaagcgcaggtgcgcaagctcacggccgagacagtggcgtggcaattgaaggagcccgtggccaaggtcaagtggacctcgccggccgcgctgccgggccaggcgggcgtggtctcggtcagctggaagaacggtttgcggctgcagcccgagatgcaggagctgtacgccgtctttcgcaacgcgggcttcgatgtgtgggtgtgctcggcgtccttcgtcgatgtgatcaaggagatctcgtcgaaccccgccttcggctacaacaacccgcccgagcgcgtgctggccatggaactggagcgcgacgccaacggcgtgatccagcccgagttccgccgtggctacgaccagacccagggcccgggcaagaccaagaacatccagcgcttcctggtcagcaaatacggctatggcccatgcttcattgccggcgacagcgagggcgaccagaacatgatggccgacttcgccgacacgaagaaagtgctgatcgtgaatcgcctgcgcgacccgaagaccgccatcggcaagttctcggccatggcggtgcagaactacggcaagcccgacacgcgctacctgctgcagggccgcgacgacaacctcggccagtgggtgacttcgcagctgcacacgccgctgggcgctgcacagggcaaggcgctcaagtaggcgcagaagccctggggcggggcaaggggccgcggttgcctatgatcgatcctggcattccacccaggagacgaaaaatggccgaccgctaccctcttgccgagctgaaaaacctgcccgaagacatccgcaccgcgattcttgcggtgcaggaaaaagccggcttcgtgcccaacgttttcctcgcgctcgcgcgccgcccggccgagtggcgggccttcttcgcgtaccacgacgcgctgatgctgaaggaggaaggttcgctcaccaagggcgaccgcgagatgatcgtcaccaccaccagcgcggccaaccagtgcctttactgcgtggtggcgcatggggcgctgctgcgcatctacgagaagaagccgctggtggccgaccaggtggcggtgaactaccgcaaggccgacatcacgccgcgccagcgcgcgatgctcgactttgcgatgaaggtctgcgaacgctcgcacgagatcgacgatgccgacttcaccgcattgcatgcccacggcttcgacgatgaagacatctgggacattgcctcgatcaccgccttcttcggcctcagtaaccggcttgcgagcttcagcggcatgcagccgaaccccgagttcttcttgatggggcgactgccccgggagaagaaatagcgcgctcgctaacccaggaacccaggaactcaagccttgtttctgcaggacgcgagtgcgtccaatgcgggcttgtaggtggagttgcccacgtccatcagtcccagcacggtgtgaaagaggttgtcgtgcgtgagcggcgcatcgagccccgcttccatgcacgggcgcgagagcttgcggcgctggctcatgccgtcgctgaaccaggtgaccatgggcacgtgcttctgggcctccggagcaaagctgtagggcacgccgtgcaggaacaggccgtactcgccaagcgattcgccatggtcgctcacgtagagcaaggccgggtcgtactggttcgactgcgccttgagccagtcgatggtccggccgaggaagcggtcggtctgggcaatcgagttgtcatacacgttctgcagctccgcatgtccgcactcggccagcgcattggtcttgcactcgggcaggaagcgcttcatgtccggcgccgagcgcttgtagtaggccggcccgtggctgcccatctggtgcatgaccagcaccacgcccttggcgcggcgctcggccggcagcgccgcaatgcgcgcatcgagccccttgagcatcacgtcgtccaggcattcctcaccatcgcacagcgcgctcttctgcgccgatgaaagactgtcgaacgcagatgcgttcggaatgcgggtgcagacatccttgcagccggcctggttgtcgagccacagcaccgccagccccgcggcctggagcacgtcgacaaggttctcgtagtcgtccttgcgcgattcatagccctgcttgcccagcggcgagaacatgcacggcacggaggccagcgtattggtgccacatgaatgcacatcccgatagctcagcacgccgcgcgcggccagttcgggcgtggtgtcgcgcgcatagccgttgaggccgaagtggtcggcccgggccgtctcgcccaccaccatcacgaacatcggcggacgcgcctggcccgcatagctcgcacccagggccgtgccggcggtgatcggaatcagcttgcggctgcgcttgaacatcggcttgaggagcaccgagccggccgaatacaggctggccaccggattcatcatgtagcgcaggtggatgttgttgcgcatcagcggggcaagctgccggttcatcgacacggcggcgaccagcgccaccgccaccgccagcagcagcagcgccgcattgcgccagagcctggagacgaagcgcatcggcacgatgcgcgcccgccagagggcgaggcccgggagcaggacgaccaccagaacatggaaagccatgcgccagctcatgaggtcgcgcgcttcgttcgggtcggtctgcagcacgttggcgatcatggtcggatccatcaccacgcggtactcgatcatgtagtgctggacgaacgcggccagcagcaccaccgcgaaccacagcggcttcatccagcgcgaccacgcggtgaaggacagcagtgccacggtggcgcacaccacgagcactgccatggcggcggtcgttggcaggtaggcgctgggtgcaccgccgatgcgcgccagttcgttccacagcggccagttggcggccgccgcgagatagatcgcgagccacaccaccacccgctgcgccgagcgcggccgtgtgagccacaggtcgatgcgcgcccaaagcgcgtgtgcaaacgccaggtacggcgcactggctgcgggcagttccatgccgcgcgcgggcgcgggttcgattcgcgaaatagacatgcgccgactgtagaaagcgcaactgaaggaagcctgaattgcgcgttcagccggcgttcagactcgagcccttcttgctctcaacctgggccgcatgtaggccctgagcgccaggttcagcggccggctgacgccgcgctccaccacgatcgacaccagggcggccaggatggcgccgaccaccacgtcgaacggaaagtgcagccccaggaacacccggctccatccgaccaccgcggccactgccagcgccgcgcacatgggcgcgcgccagggcaggcaccagagcgaaaacgccgcagcgaaggtgcacgccgcatgcaggctggggaaccccggccgtgcgccctgcggcgcccactggatgcccaggccgtagaaagcgggccgctggaacggcatggccgaacgaaacacgttcacgatgagccagaccgccagcacgctgaccagcgcggtgaagcaggcatagcgcaggcgccggtcgagcgccgcaccgccgacgatcgcgacggccagtaaagccggcagcacatcggaggcaaagcgcgcgaaatagatgctccacgccggtgccgcggcgccagcgttgatcagcgcgaacagggagacatcaagagcctgcatgcaggaccgcaggttcggcggcggacagtcgggaagtgcggggtgcggcggccaggtcgatggcaaagcccaccacccagcagatccacgccgtccacagcgtgtggctcatgtagtgcgcgccccgcagctgctgcgacagccccagcgcaagacccgcggccagcgacacgccgagccacacgagcgcggcgcgcggcgacaccctgcgcagcacgaaatagccgcccaggtaggcgaaggccgcagaggcatggccggccggaaaacacccgcccgggccgccgtcatagaccctccatgcccaatgcgacacgtggcttgcgacgccgccgaattccttcaggtcccaggggcagctcgtgtggcttgctcgcttgagcacgctgacagcaaccaccgaaagcagcacggtgaaagccagctgcgcccgggcgcgaaccggcagccgccgcaggatgcccagcggccagcggatgccggcaaacagcgcaatcacgaacagccagctcaggttcttggcgctttcgtgcatgacatggaccagaaaggcgttgtcgcgcagcggaaaccccatgggcgtgcccgcgagcctcgccaggacgaggtcgcccccggtggcgtcccagcccagcaggagtaccagcgccagaagggtcatggcccccggacgaagattcgaaacagtcggcagattcagcacacgcgtcatgagcagggaaacaagcagcagaaaaacaagtccgggaaaccccatgagcctacgttcctggtctgaaccgatcctgaagcggcctgaacgaaagctgacgcactccccgaccacgcggcggtcggcgctagactcggttttttgaaagaaagagtgacctcgcgtgcgcatattgctcgtcgaagatgacagtgcgttggcagacgccgtttgcagctacctgattgcgaaggctttcgtggtcgacgtggcgtccagccttgccgaggcccggggcgccctgcattcggtgcaatacgccgctgtgctgctcgacctgcacctgggcgacggcgacggcctttcgctgctgccgcaggtgcgcgcgctgcgcgagccgcccatcgtcatcgtgctgaccgcgcgcgaccaggtcactgaccgcatccgcgggctcgatgccggcgccgacgactacctcatcaagccttacgacccggccgagctgctggcgcggctgcgcgcggtcgagcggcggcgcagcgccggctctgcgccggtgctccacctcggcacgctggagatcgacctggcgcaggaccgggtccgcaaggacgggaatcccgtcgtcctgacccagaaggaatgggcgctgctgcgcgtcatggcgacgcggcccgaacgcatccacacccgcgagaacctggccgatgcgctctacggcttcggcgacgaggccgacagcaacacgctcgaggtgttcatcagccggctgcggcgcaagctcggcaagagccatatccagacactgcgcggcctcggctatcgcctgtcgacttcggcagacgacgacgaatgaacgcagttctccccccaccggccccgacacgctggccggccgcctgactcgcacgctgatcgtctgggtgggcggcgtgtggatgctgtgcgtgctggccgtggtctggtatgtggaccgcgagatcaaccacaacttcgacaatgagctggtggaggtgtcgcaccgcatgttcgacatggcggtgcaggaactcgacaagcggcagcaaggcggcaccccggccaccatgccgctggtcgcgcccaagcagctgttctcggaagacgccgtgaactaccaggtcgtggacatccacgagcatgtgctgctgcgctcggccgaagcgccgaatgatgccttcgacgttccgctggccgccggcttcgcgaacagccagacctggcgcatctacaccgtgcggcatcccacgcgaggcctctacttccaggtggccgatccgctcgacgagcgccgcacggcgctgaaccgcacgctctacggcctgatcattcccctgggcgccgtgctgccgctgctggcgctggtgctgcgcagcgtggcgcgcaccgagctgcgcgtgctgcagcagcttgcgggcgagatcgagaagcgcagcggctccgacctgcggcccatcaccctgcccggcctgccgagggagctgcgttcggtgggcgaccacgtcaacagcctgctggagcgcctgtcgcagtcgctcgacgtggagcgcgcgctggctgccaatgcggcccacgagctgcgaacgcccctggccgcggcgcggctacgcctgcagaccgcgctcgagcacgacctgcggcgcaacgatgtccaggccgcgctcgacgcgctgcaaatcctcagccaccgcaccgagaagctgctccagctctcgcgcgccgaatccggcgcgtcgcttgcgcgctcacgggtcgacctggtccagcttgcgggcgcggtggtgcaggaattctggaacgacccgcagctcagcgaacgcctggcgctcaaggtgcccgacgccatcgcgcccgttacctcgggcgacgtcgacgcactggccatcgcgctgcgcaacctggtggaaaacgcgctgcgctacagcggcagcggccgcgtggtgatcgaggtgatggcaccctgcacgctcgcggtgcgcgacttcggcccgggcgtcagcgcagagcagctcgccacgctgcagcagcgccacgtgcggcacagctccgaccgcgcgggttacgggctgggcctgtcgatcgtgggcaccatcgtcgagaagcacaacgcgaagctcgaactggcttcgccgccggcaggcgccgccagcgggttcgaggcgcgcatcgtgctgcggccggcctgaggctaatcgcagagcccttgcatctgggcaacgatgtgcatgaagacccagacatttcccttgccgtaggtcgaaggctcgccggagccacccaggaacgggtaaggctctgggacatagatctcctcggtcttcaacggacccgctcgcttgcggacctgtgccacgtgatcggcacgcagcacgtagccagcgaagccggggtccttgagcaccttttcctcgaaccgggcgacgctcggaaatacgccataggactttgcgcccttcgagaagggatgaaggacgatgtactcatcactcgcacgcgcgcgaagaaagaaatggcccagcttcgagtacccgacgatctcgtcgtatttcttgaaatgccgggaccagcactcgagctttgtcgcaggcagcggtgccgtcagcgtgtacagcgtatccgcggttaccgctgaagcggcgcccaatgaaaatacgagtgtcagcagctttcgcagcatgggttctccaagtgaaactgaggtttgcagtggcgagcaagcaccagcagtcttctcggcatctcgccctattcgctcaccagcgcgcgcagccagtcaggcaaggccagcgccttctgcttcggaaaatcgacccagatcgtggtcgctccacccgccgcgcagaccacgtcgggcgcatcggcgcgcgccatggtggcccagctctcgaaggtggttcggcccgggtcgctcacgtacatcttgagcagcacgtcacccggatattcgatctggcgatagaaattgcagaaggcattgacgatcaccatgccttcgccgcccggctcgggctcgaagcctatggagtgcatccagtcgattcgcgcggtttccaggtagcgaaagtaggtgccgttgttgaggtggcccatggcgtccatgtcgccccagcggatggggatgaacatctcgtacacgagcttcttcttttcggggatttcgattctcatcggtggatcttgcgtgaggaaagctcagagcgcgaacccgtcgtccgcggcaatcaccgcgccgttcacgaagtggctctgcccgctggccagcagcacgatcaggccgtcgaggtcttcgggcttgcccacgcgcttgcgcggcagcatgttcaccagcttggcgccgccctcggaaagccagtggtcctcgttgagttcggtcgtgatgtagcccgggcacagcgcgttcacgttgatgccgaagcggccccattcgagcgccatggccttggtcatctgcaccacggcggccttgctcatgcagtaggtgccgagctgcggcagcaccttgagcgccgccaccgaggcgatgttgatgatgcgcccgccgatgtaggtgcccggcgccgaaccgtcggcgcgcgccagcatgcgcttgcacacctcctgcgcgacgaagaacgaacccttcacgttggtgtcgaagatgtagtcgtagtcgccgggcgccacgtcctgcaggcgctgggtggtgctcacgcccgagttgttgaccaggacatcaatggggcccacctcggtctcggcgcgcgccacggcggccttgatgctgccgatgtcggtcacgtcgagctcgaccacatgggcgtctccgccctcgccctcgatgcgtgcgcgcagctccttgagcttctcgacccggcggcttgccagcaccaccgccgcaccggcgcgcgccagcgtcttggcaaactgcgcgcccaggccgctggaagcgccggtgacaaaggccacgcggcctgaaaggtcgatgctgtaagccatggaagagggtcctgttgaatcgttgccgagtcgccgaggcgacgccccgcactccacataaaatgtttcgcgccctcgaagcgtccgagcctcaaatcattatcgacgagacccacatgacccacgacgaaatcctcgcccagttcggcccccgcgaatccatggaatacgacgtggtggtcgtcggcggcggcccggccggcctctcgaccgccatccggctcaagcagctggccgcccaccacgaaaaggaaatctcggtcgtggtgctcgagaaaggctccgagcccggcgcgcacattctctcgggcgccatcatggacccgcgcgccctcaacgagctgctgcccgactggaaggaacagggcgccccgctcaaccagcccgtcaccgacgacgcgatggtgttcctcggcgaaaagtcgggcctgcgcacgcccaatgcctttttgccggcctgcttccagaaccacggcaactacatcatcagcctgagcgacttcaccaagtggctggcgcagcaggccgagaacctgggcgtggagatcttcccgggcttcccggctgccgaagtgctctacaacgagaacggctcggtgcgcggcgttgcgaccggcaacctgggcgtgggcaaggacggcgaacccaccgagaacttccagctcggcatggagctcctgggcaagtacaccgtgtttgccgaaggcgcgcgcggccacctgggccgccagctgatcgccaggttcaagctggacgaaggcaaggacccgcagacctacggcctcggcgtgaaggaagtgtgggaaatcgaccccaagcgccaccagcccggcttcgtgctgcacaccgcgggctggccgatgaagagcgacacctacggcggcgccttcctctatcacatggaagacaacaagatctccatgggcttcatcaccggcctggactacagcaacccgtacctgagcccgttcgaggaaatgcagcgctggaagctgcatcccaacatccgctggtacctggaaggcgacgaagccaagggcatcaagcccgccaagcgcattggctacggcgcgcgcgccatcacggccggcggcctgatgtcactgcccaagacggtgttcccgggcggcgcgctggtcggctgcgaggccggctacctcaacgtgagccgcatcaagggcagccacgccgccatcaagaccggcatgctggccgccgaagccgcctacgacgccgttcaggccggacgccagcacgacgaactcacggcctacccggccgccttcgagaagagctggctctacaccgagctgaacaaggcacgcaacttcaaggcctggttcaagaagggcctgggcgttgccaccttcatgaacggcatcgagcagtggctgctcaagggccacattccatggaccctgcaccgccacaagcccgaccacctgtacctcaagcccgcggcggagtgcaagcccatcgtctatccaaagccggacggcaagctcaccttcgaccggctgtcgagcgtgttcatcagcaacaccaaccacgaggaacagcagccggcccacctgacgctcaaggatgcgtcggttccggtgaacatcaacctgtcgaagtttgccggccctgaaagccgctactgcccggccggcgtctacgagttcgtcggcaccgaagacggcaagcagcgcctgcagatcaatgcgcagaactgcgtgcattgcaagacctgcgacatcaaggacccgacccagaatatcgtctgggtcacgcccgaaggcggcggcgggccgaattacgtggggatgtgagaaggccagcgcgatggatgaagccctcttcggagggctttttcgtttctggagcagatttttttcgcgccgatgcatccgatccgaaccccacggcgtaagtgtgagcaggacggcgatgcatgtcgccatccgccaacccattcaacgacccttcgagaggatattcagccatgaacaccatgctccaccgcatcgccatcgccgccaccctggcgctggccgccgcccacgcccttgccgcggaccctgtgcccgccgcgccggccgccaaggccgcgccggccagcaacctgggcgtcgcccgcgcgctcatcgccgacagcaagtggccggccgccatcaccgagctggagcgcgtcaacgacagcggcaacgccgactggaacaacctcatgggctacacgctgcgcaagtcgggcgcgggcaagtggacggcttcggagaagtactacgacaccgcgctcaagatcgaccccagccaccgcggcgcgctcgaatactcgggcgagctgtacctctcgatgggcgacctgaccaaggccgagcagcgactcgccgcgctgggccaggcctgcaacatgagctgccccgagtacaaggacctgaaggcatcggtcgagggcttcaaggccaacggcggcaagaagagctgaagcccggcagcggccgctcgaccgcagtgccgcaaacgccgctacgggtgcaatactcgcgcgcatgaatggacatcttccggacagcctgcaggcgctgctcgccggcgcggcgcgcggcgaccatgcctgcttcgcgcaggtctacgagcgcacgcaccggcacctgttcggcatcgcggtgcgcatgctgggccatgaacagtccgccgaagacgtactgcaagaggcctacgtgagcatctggaagaacgcgggcagctaccgcgccaccgtcgacgggcaggagatccagccgatcacctggctgatcgcgatcgtgcgcaacaaggcgctcgatgcgctgcgcgcccgcacccgccgcggcgctcacgagcaactgcaacagcacatcgacgatgacgaggacgatgccgccgcaacgccgcagggcacagacaccgcccccggcgcgctgcagctcttcgagcaggccatgcacgcgctgcgcatcgaaggctgcatggcggcgctcgacggcagctttcgccagagcctcgcgctcgcctactaccagggcctctcgcacaccgaggtggccgcgcagatgaatgcgccgctgggatcggtcaaggcctggatacgccgcggcctcgacaagctgcgcacctgcctgatcgcgcagggggtggcgccatgaggtacaccgacacccgattgctcgatgcgctggcatcggcctatgtgctgggcacgctggccgggggcgcgcggcggcgcttcgagcgcctgcagcgcgaccgcgccgacgtgcgtgcgcacgtggcgcagtgggagcaacggctgggccagctggccctgccggtgccggcgcgccagccgtcggccgagctctggcgggcgatcgccgcgcgcacgcggcccgtcggagcacgcgaaaccgcaagctcgcgctggcccgcctggcttcgtcccgcaggcttcgggttcggcggcctcgcagccggcgtgatcgccgcgagcgcgctgtttctctcggcgcccggcctcttcctgtcgagcgaccagctcgcgatgcgctcgggcgagcggttgccgcaaagctatgtgggcgtgctgaacgacgcgcagggccagggccggctgctcgtgagttcgctgcggcacggcaagacgctcacgctcaaggtgctgggcaccgcgcctcttacgggccttgcgcccgcgctggctgccgacgagcggctggtgttgtgggccttgcccgccgacggggcgcccttcgccatcggcacggttccggcgggcggcacgcaggtgtcgacgctccccgacacgtccgagaagcttctgttgaaggtttcgcgcctcgtcgtcacgcgcgagcgcacggccacgccctcggcgccgagcgccgatgtggtgttgagcgggagctgcgccaagctctggtgaggctcagcgcaccgcctcgccccacccgccgccaccaggcgtctcgatcacgaacacatcgccagggtgcatctgcacctgcccgatgtggtccagcgtctcgaccgtgccgccggcccgctccacgcggttgatacccaccgcgccggcgtcgccgcccgctccgccgaacgcaccatagagccggccattgctgaggatggatgccgtcatcggcgccaggaagcgcacgcgccgtacgccgccgtcgccgccacgccagcgccctgccccgcccgagcctgcgcgcaagcggtagctgtcgagccgcaccgggtagcggaattcgagcacctcggggtcggtcagacgcgaattggtcatgtgggtctgcaccacgctcgtgccgtcgaagtccgggcccgcgcccgagccgcccgagatggtctcgtagtactggtgctcgccgtcgccgaaggtgaagttgttcatggtgcactggctcgcggccatgacgcccagcgcgccgtagagcgcattggtcacgcagctcgaggtttcgacgttgcccgccaccaccgcggccggcggcagcggattgagcatgcagccattcggcacgatcacctcgatgggtttcaggcagcccgcgttgagcggaatgtcgtcgtccaccagcgtgcggaacacgtacagcacggccgccatggtgatggcgcgcggcgcattgaagttgttggccagttgcgcgctggtgcccgtgaaatccaccgtggccgagcgcgcgactgcatcgaccgtgacccgcacgcggatctgcgcgccgttgtccagcggcagcgtgaactcgccattcttcagcgccgtgatgacgcggcgcaccgactcctcggcgttgtcctgcacgtggcccatgtaggcggcgacggtctcgcggccgaactgcgccaccatggcctgcagctcctgcacgcccttctcgttggcggcgatctgcgcacgcaggtcggccaggttctgctcgatgttgcgcgacggatgcgcgccgctccccagcagtgcgcgcagttcggcctcgcgcaggcggccgccctcgaccagcttgaagttgtcgatcagcacgccttcatcgccgatggtggccgaaaacggcggcatcgagcccggcgtgatgccgcccacgtcggcatggtggccgcgtgaggccacgtagaacgacggccgcgcatcgcccgcttccaggtacaccggcgtcaccaccgtgatgtcgggcaggtgcgtgccgccgtggtaggggtcgttcagcacgaagacgtcgccgggcttcatgccggggttgccgtcgatcacggtcttgatcgactcgctcatcgagcccaggtgcaccggcatgtgcggcgcattggcaatcaggttgccctgcacgtcgaacagcgcgcaagaaaagtcgagccgctccttgatgttgaccgagtaggccgtgttctgcagccgcaggcccatctgctcggcgatgttcatgaagaggttgttgaacacctcgagcatcaccggatcggcgctggtgcccatggcctgcgtggccacgcgcgggcgcacccggtgcagctcgatgccggcagcggtggcgcgcgcctgccagccgggctcgatcaccgtggtcgcattgcggcccgcgaggatggcggggccgtcgatggttgcaccgggcttgagggccgcctcgtcgaacagcgcggcgtcgcgccagccggcggctttttcgtcggcctcgcaatacatccgtacggccgccagcggttcgggtgaattgaaggcaacctcggcctgcacggccggtggcgcgccacgttcgccggcccccacggcctccaccgtcaccgcttcgatcacgagtgcgcgctcggccatcaggaaggcgaagcggcgccggtagccggtttcgaattcgtcgcgcatcgcggcgatggcctcgttgaccgtgcccgccatgggcagcgtgcaggccagcgcggtgtcggtgccttcgtagcgaagctgcacgcggtgcaccaaggcgatgaccgcatccgccacgccctgctcgcgcagctcgcccttcgcctgcgcggcaagggtgcccgcggcatcgcgcgccgcggccagcccttctgcatcgagcctgcgctccagcgccagctcgcgcatcgccagctgatcggccagccccatgccgaaggccgagagtacgcccgccagcggatgcaggtagatgctgcccatgcccagcgcatcggccaccaggcaggcgtgctggccgcccgcgccgccgaagcactgcagcgtgtactgcgtgacgtcgtagccgcgcgccaccgaaatgcgcttgatggcgttggccatgctggcgactgcgatgcgcagcgcgccgctcgccacttcttccgcgctcacgcggcggccggtcgcttccgacatgcggcgcgccatggcgtcgaagccgcttcgtgccgctgccaggtcgagcggctcatcggcgctcggaccgaacacacgtggaaagtgcgaaggctggatcttgccgagcagcacgttcgcatcggtggtggtgagcggaccgccgcgccggtagctggccggccccgggttggccccggccgactccggccccacgcgcagccgcgcgccgtcgaaggcgatgaccgagccgccgcccgcggccaccgtgtggatgctcatcatcggcgcgcgcatgcgcacgccggccacctgggtctcgaaggagcgctcgaactcgccggcatagtgcgacacgtcggtggaggtgccgcccatgtcgaagccgatcacgcgcgcatgcccggcgtccagcgcggtgcgcaccatgccgacgatgccgcccgccgggccggaaagaatcgcgtccttgccctggaagcggtcggcctgcgtgagcccgcccgaactctgcatgaagaacagcggcacgcccggcatctgccgcgacacctgttccacgtagcgccgcaggatcgggctcaggtaggcatcgaccaccgtggtgtcgccgcgcggcaccagcttcatgagcggactggtcttgtgcgacacagacacctgcgtgaagccgacggcccgtgcgatgcgctcggccgcgagctcgtgcgcggtgtagcgccagccatgcatgaagacgatcgcgcaggcgcgcaggccggcatcgaaggcctcttgcagcgcagtgcgcaaggcgccctcgtccagcggctgcacgacgccgccttgcgcgtccatgcgctcgccggcctcgatcacgcgttcgtagagcagctcgggcagcacgatgcggcggtcgaacagccgcggccgcgcctgcgtggcgatgcgcagcgcatcgcgaaatcccgctgttgtgaccagcaccgtgggctcgcccttgcgctccagcagcgcgtttgtggccaccgtggtgcccatcttcacgcactcgacacgctcgggagtgacgggctcgcccggcttgagcttcagcaggcggcggatgccttcgacggcggcatccttgtattgctcggggttctcggacagcagcttgagcgtgtgcagctcgccctcggggtcgcggccgaccaggtcggtgaaggtgcctccgcggtcgatccagaattgccagcggttgccgaggggggtgggttggtcttgcatgatgaggtggtcgctcagcgtttgctgtcgacgtagtagggaacaaagatgcggttggcctcgttgccgaccgagcgcacccattcgagcgagaacttctcgcccatgcgcttgaggtcggcctcgaaatccggcggaacgcgaccgacctggaggcctcggctgcgcaattcgttggtggcgtcggcggcggcagcctggctcagggcccatccgcgcgtctcggcttcctgcccggcggccagcagcatctgctgcagatcgggtgcaagcgcctcgaaggccttccggttgacgaaaacgatgttcttcggataccaggcattgatctcgtagtagtacttcgcgcggccccacacctggttctccacgccggtgaccgccgaggtgatcatgctggtgatgcggccggtggcgagcgcctggttgacctcgaccatcggcacgtcgaccggcgttgcgccgagcagctcggcaatgcgttcggtggtctggttgtaggtgcgcatgcgcgcgccgcgaaagtcggccgccgtacgcaccggcgtgtcggtgtagagcccctgcggcggccacggaacggcatagagcgcctggaggccacgcgccgcgaagtgctggtcgatcagcggccgctgcagcgtccacatgcgccgtgcgtcggcgtagctgcccaccacgaacggaatggcgtcggccccggcgatcgggatctccttcaccatgctggtcatgatggtctcgccggcctgcaccttgccgtcctgcaccgcctgccggatgtccgccagcttcaccagcgcgttgttcggcttcacttcgatgcgcaggcggcctgcgctggcacgcgccaggtcggccgccatgcgctcgatgttctgcgtgtggaacgattcggcgcggtagccggtggccagctgccattggacggcggtttgcgccaggcaaggctgtcccgacgcggctgcgaacgcagccgcgatccagatgtgcttcatgcggttcccctaaaagcgcagcgggtggcgttgcaggtgcgtcacttcgccggccccatcaccaggtcgggcacgatcgtcacgatctgcgggaacacggtgatcaacccgatgcagaccaccaggcaaaggaagaacgggatcgcggcccgtgcgatgcggttgctgtccttgccggtcatgttctgcagcacgaagagattgaagcccacgggtggcgtgacttcggcaatctccaccagcaggatcacgaagatgccgaaccagatgagatcgaagccggccttctggatcatgggcagcaccacggcggcggtcagcacgatcatgctgatgccatccagcgccgtgccgagcaccaggtacaccagcaccaggcaggcaatcaacgcgtagggcgacaggtgcatcgaattgacccactcggccagctcgcgcgggatgccggtgaaggccatggtcttggtcaggaaggccgcacccgcgaggatgaacatgatcatgcagctcgtgcgtgccgatccgaagaggccttccttgaagttggtccatgtgagcgagcggctccaggctgccagggccagtgcgccgaccacgccgtaggcagcacactcggtggccgtggcccagcccgccaccagcgaccagcagatgaaaacgatcagcaatgcgcaggggatcaggttcttggagaggcgcagcttttcacgcaggctggtcggcggctcttccgcgggcatcagtgccttgttgcgcagcgcccaccaggcgatgtaggcgcagaacaggaacatcagcaccaggccgggcagaaagcccgccaggaagatgcggatgatcgatgcatcggcagccactgcgtagaccaccatggtgatcgacggcgggatcagaatgcccagcgtgcccgccgtggccagtgagccgatggcgatgttctcgtcgtagccgcgcttcttcagctcgggcagggaaactttggcgatcgtcgcgcaagtcgcggcggatgagccggacaccgagccgaagatgccgcagcccaggatcgtggtgtggaacagccgtccggggattcggccgagccagggtgccaggccggtgaacatctcctggctgagcttggtgcgaaacagtatctcgcccatccagatgaacagcggcaacgccgccagctcccagctggcgttgctttcccagaaggccgagaacaggttcaggccgggctggctggtcgtgaagaaggcctggccgacccagccgcagatcgccagcgtcatggcaatccagacaccgccggacagcatgagaagcatcagcagcaggagaatggcgccgacggtaaggatgtccatgatcttgacctttcagagatccgaagagaagtcgccctgggcgtggcgttcttccaccagtcgcacgtaggtcggaatgccgccacggacaacgatcagcagttcgtcgaccagcgccaccaggaacagaaccgaaccgatggcaaagctcatctggggaatccagatcggtatcgcccagagcccctgcgccagctcgttgaactgccagctctcgaacgtgaatcggcaggcccaccaggcgaggtatcccatcgcgacgcaagcaaccgcgaggcagaccagttcgaagcggcgccggttggacgcggagagcttttccagcaccagcgtgacccggacgaagtcgccgtgcttgaaggcatgggccatcgtcatgaaggcagcggcggcgcacagccacgacaccacgtcggtgatggcaccggtctgaaagccgaactgccgccccagggtctggacaaccatcaggatgcagatgagcgcaatacagcccgcgcccaatgcgccagccatcaggtaggtgcggtcgagcacgcgccgcagcgcatgcggcgtcgccgtcggggtggtggcgatgccgtccaagggggtggccatatcggcggtcagcgacatggggcgctcacttccgggagtaggcgtcgatgaccgcctggccatcggcaccggccagcttgatccagtcggccgtcatgcggtcgccgatgaccttgagctccttcttcaagccttcggcgccgacgtcgacggtcatgccccgggcggcaagctccttgatgtactcctcgttcttctgctcgctgagcttccagccgcgctgctcggaagccgcggcctgttgcagcactgcgtcctgcgtcggcttgtccagggcctcgaatgccttctggttgaccaccacggcattgcgcggcagccaggcagccacgccatagaagtacttgatgctctcgtacaacttgctgtccacgccgctcgcgctggacgtgaggaagttgtccaccccgccggtggccagcgcggccggcagctcggccagttggatcgtcaccggctgcgcacccacggccgtcgcgatgtacgaggtggccgggttgtaggcacgcatcttggtgcggttgagatccttgagggtcgataccggcttgctggagtacaggctctgcggcggccacggcaccgtgtagagcagcttgacgccctgcgcggccagcgtcttcaccagcagcggccgggaagcctcgtccagccgtttcgactcggcatagctcgtggccaggaacggaatggagtcgacgccgaagaccggcgcttcgttcgcggcgcccgacaggaggagttccccggccggcacctgggccgactgcacggcgcgcttgatttcgttcgccttgaagagcgaggcattggcgtgaaccgcgatcttgagctttccgccggtggccttctccacgccttctgcgaactgctgcaggttctgcaccgggaacgtgttgacgccgtagccggacggaagatcccatttgacctgggcggaggcggtgcctgcagccgcgaccgcggccaggatgagcatgagttttttcattgggggttcctagttcagaagctggcgagttggtggttgaaaagatcggtgatgagcatcgcgcccggagcgtgagtgatgcagaacgaggggcgggcctgcgcgatgaccgcctggggcgtgacgccgcaggcccagaacacgggcagctcgccgggcatgacctcgaccgcgtcgccgtagtcgggatcggcgagcgagcggatgccgatcagcgccggatcgccgatgtgcaccggcgccccgtgcacggccggaaagcgcgaggtgatctgcaccgcgcgaatcgcatcggccgcgcgcagcgggcgcatcgacaccaccatcggcccatggaaaggaccggcgggcgtggtggccaccgaggtgcggtacatcgccacgttgcggccttgctccacatggcgcagggcgatgccctcggccatcagcgcatgttcgaaggtgaaggagcagccgatgacgaagctcaccaggtcgtcgttccacaggacgcgaacatcggtgggctcgtccaccagttctccgtcacgccacacgcggtagcgcggcaggtcggtgcggatgtcgatgtcttcgccaagcgccggcagtgccgggtcaccggcctccgacacgccgagcagcggacacggcttggggttggcctggcagaagcgcaagaaatcggcggcgtacgcccgcggcaggatcacgagattgccctgcacgtgggcactcgcgagcccgctggtgtgggtgcggagcgcaccgctgcggcacgcctggcgcacggcctgcgcactactgccggggccaggctgttcttcgaaggatggagagttcgacatttggcgttctcgatgcccgatgcatcgctttgatgtgatgcgccggattgtgggaatccgcgctcacaaacgccaacgcaaagtttctttctcaactcatcgatttttttgatgaccctgggcggtgcgacgcatgcaccacggcggagctcagcgcggcctccggcaacggggacgacgggtcgtcgcggtagctcgcgtagatgggcaagggctccagcgtgtcgtcgcagggcagcacgcgcagcggcaggcgccgtgccagcggctcgaccaccgcacgcggcagcgtggccacgccgaagcccgcctccaccagctgcgccatcgccgagatcgacgagatcgcatgcacgcgcggcggcgggctgccggcttcgcgaaacagctcgagcagcgccacgtgcggctgcgaaccgcgctggaaggtcagcaggtcgagcgagagcaggtccggcaggcggtagcgccgcttcaggtgcaggtcgcggtggccgacgaagcacataggcatcggtggcacggcgcgggtgcgcacgccgtcgccgatggccggcagtgcggcaaagaccaggtcctgcttgccgcgctggagctggtcgaccagcacgggcgtggtttcgacggtgagctccagctcgaagtccggatgcgtcgcctgcatgtgcttgagccagccggtgagccagctgtgcaccaccgattcgatggcgcccacgcgcagcacggcttcccgcaccgcacccgaccccatctcggccttgatgtgcatctgcatttcgagcagcttctgcgcaaaggcgtgaaagcgctgccccgccacggtgaggcggaattgcttgtcgcgccggtcgagcagcagcacgcccagctcgcgctcgagcgcggcaatgcggctggagagcgccgactgcgtgatgtgcagcttctcggccgcgcgagtaacgctcttgagcgccacggcccagtgaaaggcttcaacgaatcgcaggttcatcgttttccggtcgtccggctccttgagtgcgcgagccgcgagtgtcgcctctgccgggctttgtgctgcgctatgctcgttgcagaaggagacaagaccatgcagatcgtcatcacgggcggggccggctttgtgggcgcacgccttgcccgcacgctgctgaagcaggggcagctttcgctcgcgggtgcaccggcccgggccatttcgcgcatcacgctggtcgaccgcgcccagccgccggccgatcttgcggccgacgcgcgcattgccagcgcgctcggcgacctgaacgaacaactggcatcgcccgatgcggcgctctggcgcgaagccgacgccatcttccatctggccgccgcggtcagcggcgaatgcgaggccgacttcgacttgggcatgcgcagcaactttgccgccacgcatgccctgctcgagaaggcgcgcgccatgggcactcggccggtggtggtgtttgccagctcgctggccgtgttcggcgattcgcccgatcagcccttgccgccggtgatcgaagaccacacgctgccgacgccgcagaccagctacggcatccagaaattcattggcgagcagctggtggccgactacacgcgcaagggcttcatccgcggccgcagcgtgcgcctgatgacggtgagcgtgcgtcccggccggcccaacggcgccgcatcgggctttttcagcggcatggtccgcgagccgctcgcgggcattcgcgccgcctgcccggtgcccgacgaaacgcccgtggccatcgcgtcgccggcgcgcaccgtcgaaggcatcctccgcgcggcggaagccggcgacgccgaatggggcccgcgcacggctctcaacctgccctcgctttccaccacggtgggagagatggccgccgcgctcgagcgcgtggccggcaaggccgccaccgacctgctcgaccgcacgcccgatccggtcatccagcgcatcgtgaaaacctggcccggccgcatcgaaaccgcgcgcgccagacgcctgggactttcggcagatgccgatttcgagacggttattcgcgaatacgtccgtgaaaatcccgacgcggtgaagctcccgattgcggcatagtcgcatgcgcctgacgcattcctgaccacaccccccggagacaccatgaaactcggccacatcgccgccgcctgcctttcgcttgccctgggcacttccgcccttgcacaacaaccgacggtgctgaagatcggctacgcgacctccaaggagtcgcactacggcgtgggctccgcggtgttctgcgacgaagtcgagaagggcacgcaaggccgctacaaatgccagcacttcgccaactcggcgcttggcggcgagcgcgaacagatcgaggccgtccagctcggcacgcaggatctggtgaacacctcgaccggccccgtgggcaatttcgtgcccgaggtcaagatcgtcgacatccccttcctgtttcgcgactacgaccatgcgcgcaaggtgatggacggccccatcggccagaacatcctgaccaagttcccgagcaagggcatcatcgcgctggcctggaccgagaacggcttccgccacatgacgaacagcaagcgcgacatcgtcaagcccagcgatgcggccggcctgaagatgcgcaccatggaaaacaaggtgcacatggacggctaccgcaccttcggcatcctgccgacgcccatggccttccccgaactcttcggcgcgctccagcaaggcacggtcgacggccaggaaaacccgatcccggtgatcctggcttcgaagttctcgcaggtgcaaaagcacctgtcgctcacgggacacgtgtattcgcccgccctgctgctgctctcgcccaaggtgtggaacaagctctcggacgccgacaagaaggtcttcgtcgatgccgcgaaaaaggcttccatcgcccagcgcaagaaggtcaacgacgacgagaacaacggcatcgcccagctcgagaaagacggcatgaaggtcgtgaagaccgtcgacggcgccgcgttccgcgaagccctgaagccggcctatgcgggctacgccaaggagttcggagccgataacatcaagaagatcacggacgtccagtaagcctgcgcgccagcttcttccgacgaccgcgcccggcccgcttcagtgcgccgggcgcttcttttttttccaagacgacagaacagagaacaacacagtgcaagtcttcgagcgctactttcttgccgccaaccgctgggcgctgatccttttgctggccgccatgtcggtcatcatcttcaccaacgtggggctgcgctatctcacgaaccagtcgctcgaatgggccgaagaggtgtcgcggcacatgatgatctggctcaccttcatcggcgccgggccggtgctgcgctacggcggccatatcgcggtcgagaacctgcaggacgcgctgccgcgcagcgcagccgttgcgctgcgcatcgtcgttgccgggctgctgttcgccttcttcggcttcatggtctggtacggctggctgtacatggaacgcacgatgttccagctcacggcagtgacgcagattccgttcgcctatatctacagcgccatgctgttcggcggcctgctgttgatcgtgcactggctgctggtggtgcggggttatgtgatgcgcagggagttcgcttccgacgcccacttcgacgccaacgcctcggcgtcgctgtaaggaaacgaccatggatgccagcatcgttctgatcgtctccgcctgcattttcctggccatcggcgtgcccgtggcctttgcgctaggcctttcgactgccgccacactcattcttgcggagaactacccgctgatggtgctgctgaaggaaaccttcaccggcatcgacagctttccgctgatggccgtgccattcttcatccttgcagccgagttgatgagcggcggctcgctcaccgaagtgctgctgcgcttcgcgggccagttcgtcggccaccggcgcggaggactcggctacaccaacgtggtgtcgctcaccttcttctcgggcatctcgggctcggcgctggccgatgcggcgggaccggggtcgatgctcatcaagatgatggacaaggccggctatgaccgctcctacgcggcagcgttgacggcctcgaccgcgatcgtcgggccgatcattccgccctcgatcatcatgatcatctacgcgctgcaggacgaaaccgtttcggtcggccagctgttcgtggccggcctgctgccgggcctgctgatcgcggtggcgatgtgcatcgtgaacttctacgtctcgaagaagcgcaactacaagggcgatggcgagacgccgccgctgcgcgagattctcatcacgacctggaaggcgattcccgccatcctgctgccggtggtcattttgggcggcatgcgcgccggctggttcacgcccaccgaggcctcggtggtggcggtgttctacgcgctggtgtgcggcaagttcgtctaccgcacgctcgaatggaagatgctgcccgacatcctcgcgcgttcggccctgctgtcggcctcggtgctgatcatcatcgggctctcggcctcgttcgcctggattctgaccatcgagggcgtgccgcagcaaatggcggaatggctcgtgagcatgaacctctcgccatggatgttcctgatcatcgtcaacgtgttcctgctactgttcggcatcttcatcgagccgctgcccggcgtgatggtgctggcgccgattctcgcgccggtggcaatgaaactcggggtcgacccggtgcacttcgcgatgatcgtgatcttcaacctcacgctcggcatgatcacgccgccggtgggcgggctgctgttcgtgacctgcaacgtgtcgaaggtgcctatgtcggcgctggtgaaggagctggtgcccttcctgtgggcgcacggcgccgtgctgatgatcctgaccttcgtgccgacgctcagtacctggctgccgcgggcgctcgggttcaagtagcggggggagccggctggatcgatttccacaacgaaaaccggtccggaaaaagtgacgtgtcatgagaccgatgcccctgtaaggcaaacgttttcacgaaaatgtcacctcttgcaacgatgctgcagccttcgatccccgaaagctgttgcgccatgtttcccaccaagaccgacaaggcacgcgacgaactccaaagcggccaacgcacgctcagccagcgcgaacgcgcattgctgctgatggccgacggccggcgttcgctgaccgatttcagccccctgttcgccaaccgcagcgaagccgagcaggcattgcaggccttgatgagccgcggctacctgcactatccacaggccgcccccgcgcccactcccgcgccagccgccccggcggcggccatggacagcgcggccgagccggcccaggccgcgaccgccgccgaccatttcgacggcaagcgctccctggccaccacgcgcatgttcctgttcgacatctgcgaacgcatgttcgtgcggcgcgaccccaggtttgcgatgcagatgcgcgacgcgctgcgcgaagcccgcgaccgcgacgccatgctgacgattgccgcgctgatgctctcggaggtcgagaaaagcgccggggcggaacgcgctgaatcgctgcgcgagcgtatcgagaggttacttccgctctcctccgagaccgtgcactgagcccgtccaccccccggccgccggaccggggcgccgcgatccactacactcgccatggtcaggagagagcttcgccatgcgaggccgccgaaggcgcaggggtttcccgaacgctcaggcaaaaggactgacacagcgctggcggatgccggcgtttccttgctggagagaggctgtcgcctgcatcgacgcgatgcggcaggcagcccaccgaaggagcaaacctcgatcgtggggcgaatctctcaggtaaagcggacagcaggggtggcccatggcttgcgccatggaattcgactgcccctttggagtgccccgtggccgcttccgcttcatcatccgacgcccaacttctcaagacgccgctccacgacctgcacgtggagctgagcgcacgcatggtgccgtttgccggctattcgatgccggtgcagtaccccgccggcctcatggccgagcacaagcacacgcgcgacgccgccgggttgttcgacatctcgcacatgggccagctgcgcctggtgggcccggacgccgcggccgccttcgaaaccctgatgccggtcgacgtgatcgacctggcgcccggcaagcagcgctatggcctgctgctgaacgacgaaggcggcatcctcgacgacctgatgttcttcaacgaagggcacggctcgatcttcgtgatcgtcaatggcgcctgcaaggtggccgacctggcccacatccagcagaagatcggcgcgcgctgcgatgtgcagcccatgcccgaccacgcgctgctcgcgctgcagggaccacaggcggccgcggtgctggcgcggctgtcgcccggcgtcgagcgcttcgtcttcatgaccggcggcgcagtgcagatcggcggcattcccgcctttgccacccgcagcggctacaccggcgaagacggcttcgagatttcggtggccggcaaggatgccgacgcgctcgcccgcctgctgctggcccagcccgaggtcaagcccgtcggcctgggtgcgcgcaattcgctgcgcctggaagccgggctctgcctctacggcaacgacatcgacaccaccaccacgccggtcgaggcctcgctgaactgggccatccagaaggtacgccgcacgggtggcgtgcgcgaaggcggctttccgggcgcggccaaggtcctggcccagctcgccgccgccatggccggcgccgcgggccggaccgaccacgacacgctgaagcgccggcgcgtcggcctcgtggcactggagcgcattccggtgcgcgacggtacggtgctgcaatcgttcgaaggccacgacatcggctttgtcacgagcggcctgctcggccccacggccgaccgcccgatcgccatgggctacgtggccaccgcattttcggaacccggtacgcgcgtgcaggccatcgtgcgcggcaagccggttccgatggaagtctcgaccctgcctttcgtgcccacccgctactaccgcggctaggctcggcatccccgatcattttttccacgaggagtttttcatgagcatcaagtacaccaaggaccacgaatgggtctcggccgaaggcggcgcagccactgtcggcatcaccgtgcatgcgcaggatgcgctgggcgacgtggtgttcgtcgacctgcccgaagtcggcaagacctttgcccagggtgaagtggccggtgtcgtcgaatcggtcaaggccgcggccgatgtgttcatgcccgtctcgggcgagatcaccgaagtgaacgaagccctgcgcgccgatccctcgctcgccaacaccgatccgctggccaccggctggttcttcaaggtcaagctcagcgaacccgcgcagctcgacgcgctgctggacgccgccagctacgacaagtttgccgccgaatcctgatccgccgagttcgcaagccgcctttcctcatctccgagccttcaccgccatgccgattcccgcccttccctctttgcaacaactggagaacgccgaagagttcctcgcccgccacatcggcatcgatgcagcggacgaggcgcgcatgctgccggtgatcggttcggaaacgcgggcggaactcatcgacggcatcgtgcccgcggccatccgccgcgccaagccgatgcgcctgccggcccccatcacggaagccgatgcgctggccgagctgaaggccatcgcggcaaagaacaaggtgttcaagagcttcatcggccagggctactacggcacgcacacgccgggcgtgatcttgcgcaacgtgctcgagaaccccgcctggtacacggcctacacgccgtaccaggccgagatttcgcagggccgcatggaagccttgctcaatttccagaccatggtgtgcgacctcacgggcatggccatcgccaacgcctcgatgctcgacgaagccacggccgcggccgaggccatgacgctcgccaggcgcagcgtgaaaagcaagagcaatgtgttcctggtgtcgggcgactgccatccgcagaccatcgaggtcatcaagacgcgcgccgcgccgctgggcatcgaggtcaaggtcagcaccgtgtccgagacgctgccacacctgatggtgagcggtgagttcttcggcgtgctcgcgcagtaccccgccaccaccggccacgtgcacgacctgcgcccgctcgcgggccatgcgcaccagtgcgacgcggccttctgcgtggccgccgacctgctggcgctgacgctgcttgcgccacccggcgaatgggacgccgacatcgtctgcggcaccacgcagcgcttcggcatgccgctgtgcaacggcggcccgcacgccgcctacctggcctgccgcgacgagttcaagcgatcgctgccgggccggctggtcggcgtgagcgtcgacacccacggccagcccgcctaccgccttgcgctgcagacgcgcgagcagcacatccgccgcgagaaggccacctccaacatctgtaccgcgcaagtgctgccggccgtggtggccagcatgtacgccgtgtaccacggccccgacggcctcacgcgcatcgcgcagcgcgtggccgcgctcacggccatcctcgcgcagggcctggcgcagatgggccgcgagccggtcaacgccacggctttcgattcgctgaccatccgcaccggcgaagacacgccgaagatcatcgagcgcgcgcaggccgcgggcgtcaacctgcgccagcggctgcagcagcacctgggcatttcactcgacgaaaccaccacgcgcgccgacatcgagacgctctgggcgctgttcgttcccaccggtacgccgatgccccgcttcgacgacctggccaacaccgcgccgcgcctgcccgaagacctgcgccgcaccagcgcctttctgacgcacccggtgttcaacacccacaagagcgaaaccgcgatgctgcgctacatccgcagcctgtcggacaaggacctggcccttgaccgcagcatgatcccgctcggcagctgcacgatgaagctcaacgcgaccagcgagatgatcccgatcacctggccggagttcgccaacatccatccctttgcgccggccgagcagctggtgggctatgcccagctcgatgcgcagctgcgcgcctggctgtgcgaagccaccggctacgcaggcatcagcctacagcccaacgcgggctcgcagggcgaatacgcgggcctgctggccatcaagtccttccacgaagccaatggccaggggcaccgcaacatctgcctcattccctcgtcggcgcacggcaccaaccccgcaagcgcgcagatggtgggcctgcaggtggtggtgacggcctgcgacgcgcagggcaacgtcgacatggaagacctgaagttcgcatgcgagaagcacagcgacaagctggcggcggtgatgatcacctacccgagcacgcacggcgtgttcgagacccgcgtgaaggagctctgcgaactcgtgcatgaacacggcggccgcgtgtacgtggacggtgccaacatgaatgcgctggtcggcgtggccgcgccgggcgagttcggtggcgacgtgagccacctgaacctgcacaagaccttctgcattccgcacggcggcggcggcccgggcgtgggcccggtgtgcgtggtggaagacctcgtgccctacctgccgggccatgcgacgggcggcattgcatcgaacggcgtgggcgcggtttccgcggcgccgctcggcaatgcggccgtgctgccgatcagctggatgtactgccgcatgatgggcgccaagggcctgcaagctgcgaccgaaatcgcgatcctgagtgccaactacatcagcgcgcgcctcaaggaccactatcccacgctgtacgcgagccccaacggccacgtcgcgcacgagtgcatcctcgacctgcgcccgctcaaggacacgagcggcgtcaccgccgaagacgtggccaagcgcctgatcgactacggcttccacgcgccgacgctgagcttcccggtgcccggcacgctgatggtcgagccgaccgagagcgagccgctggccgaactcgaccgcttcatcgacgcgatgatcgccatccgcggcgagatccgccgggtggaagaaggcgtctggccgaaggacgacaacccgctgaagcacgcgccgcacaccgccgccagcctgcttggtacggaatggccgcatccctattcacgcgagctgggcgccttcccgctggctgagctcaagcacgccaagtactggccgcccatcggccgtgtcgacaacgtctacggcgaccgcaacctgttctgcagctgcgtgccggtaagcgactacacggaaaccgaagaggcctgaaggccgggcgcgaacggccgggcgcaggaggacggcggctcggcgccgccgtgctgcggtgccgttctacgcctagtcctcgcggcgatacatcgcccatttcacggtcaggatgtccgccgcgatcttcgcggcattgacgccggcgtaactttcggacgggtcgaattcgaatccctcgcggtatttgacaacctgggcgtagtcctggtcgaaggtcatcggacccatgagctcggcgggatcgatgcccgcgggaagcgccaggaatttcattggatcggtggcactctggtagaggtcgacgctcatcaggttcatacgggtgtcctcgcaatcttgcaaatcgccgaggcagatcatccacgccatcggcgccgcacgcaatcggcccgcgcctacacggcggcacaccgccgggtcagcgctgctgctgcttcttcttcaacatctcgccggtggcgatctgctcgcggaagccgcgcaggctggccttcagcctgcgctcgttctccagccccatgcgcaccatgatcttctggccggacgagagcgactcgagttgcggatcggcgtactcgtagcgcacccacggccgctgcgacgacaccttgcctttcacctcgacgaggcgaacctgcaccgggccgtcgggctccggcgcctgcagcagatggtcgatcacggcgatgagccggtcattgaaatagcgcccgggaaagccgagctcctcatacgatttctgaaacagcggatatagctgggcgtaagtcttggccgccttggccggattgatcgactcggcaagctgcacgatgggcgtgtagcgcgcggcattcgcgggcgcgatggtctgcgcttcgcccttgccggcggtggtgaagcgctgccgggtgggctgcacgggccatgtgctcgcgggcgagtgctctcgcggcatgttgtcgaccgtggccacggtgcggcgcacgatgccctcgaactgcaggaagtcggccacgttcttgctgcccatcaggtcgaccagcgccttcatcacgcgggtatcggaatccgcgaccgtgggcagccccgaggcgggcagcgcgatcgcatcgatcgggttctgcggctccagcgattcgggcagtggcggaggcgccggtgcgggcgcaggcccgtcattcggcgcggtggcaacgggtgctaccggctccacatgcagtggttgctgctgctggtaccagcgccagccgaggaatgcggccgcaagcgcgagcagcacgatgacgatgagggtgccggtcgacgattcgcggcgcggcttgtacgtgggtgcgtcgcgcagctcgggcacttcgcggatttcgggtgtgtctctgtcggacatgtgggcagtttccttttgagaggattgcagtgggagacgaactgctatgttgcaccaacagagcccgcaccacggccgcgtcctcgtaacgccctgtgacgcgccaaccgcgcgaaaagttcagccgctacggtgcgctcgctgtaagcgattgcagccacgccagcgagccctgcagctcggccggccggatctcgtgcccgcccggaaaatcgccccccgacagcgccagcggaaggccgcgggccagctcgcgcgaggccgccgcggcgctcggcggaatcacgttgtccgcgcttccgtggctcacccacagcgccttgccctcgaaaacctctggcggtgcaatgtgcggcaccacctgcggcagcagccggctgtgccacaccattgcggcgcgcactttgccgggctgggtcagcagcagcgacagcgccatgatgccgccctggctgaagccgccgaccaccacgcgctccggcggcacgcccagctgctgcgctgccgaggcgatcatctcgccgaccaggaagcggctttcgcgctcctgctcctcgttgatgcgccgctctccatcggccagcacctggaactcgaaccacgcatacgcatcgggcgagagcacatacggcgcgcgcaggctcagcacgtgaaactgcggcggcatgagccgcgcgaggccgaacaggtcctgctcgttgctgcccacgccatgcatgagcaccagcagccacggctcgcggacatcggcctgggcgccgtgcgccaggaacttgaagggcagatggagttgggtcatgggtgattcacagagatgcgcgaaagccttgtgccagcgcctgggtcacctcggccgaagacacctcgcggcagcccgtcgcgttctggccggaccacagcggtgaaaagtcgccactgcccgccgcctcggccttggcgcgcagcggcgcaatgcccgaagtggcgagcggaaactcgggcgccaccgcaccgatcggccccagctcgcgcatcacgcggttgacgatgccgcgcgccggccggccggtgaacaggttggtgagcgccgtgtggcgcgcggcttcgctcttgagtgccgcgcggtgaatcgcggtggtcgtggcttcaggcgtcagcatgtaggcggtgccaacctgcacgccagcggcccccagcgccatcgccgcggccacgccgtttgcatccgcgatgccgccggccgcgatcaccggcaccttcacggcgtgcaccacctgcggcaacagcgcgaatgtgccgagctgcttcgtcaggtcgtgcgaaagaaaatggccgcggtggccgcctgcttccaggccctgggcaatcaccgcgtcgacgccatgcgcttcgagccacaaagcctcttcgaccgtggtggccgaggccagcaccttcgcgccccagccgtgcacctgcgccatcagcgcctctgaaggcagcccgaaatgaaagctcaccaccgctggacggaactcggccagcagatcggccacttcggcgctgaacgggttgcgccccgggccggtgggaatgccggccgcatcgatgccgaattcggcgtagtacggtgccagcgcggtgcgccataccgcctcacgctcagcgctcggctcgggtggcgtgtggcagaagaagttgacgttgtagggcttgccggttccagcgcggatggccgccaactcgctgcgcatggcatcggggctcagcatggcgcatggcagcgagccgagcccgcccgcgttgctgaccgcgatggccatcgcactgccttgcacgccggccatcggggcctggatgagggggagttcggtgccgagaatttgctttagcgtcgtcatgcgaaaggtctcttgatgtgtcgatgccggccattgtctcgccaagccggtggtcacttctgtggcggggtcatggccgaggcgcaccgcgggacggacacttcgcgcagccgctgatgcgcagcgtcaccccacgccacgggctgctggttcttcgcgcgcagatagtggtgcgtgaacaccaccagataagcatgcagcgtctgttcagcaacatgctcgcctgccaggttcatgcacatcgcggccacctcgctggtgcagaagtggtcgtcgcggccggagttgcgcagcttgtattgcgtgatctgctccggctgcaggctcaacaccggcagccggtcgaggtaagggcttctgcgaaacatcttgcgtgcctcggcccatgtcgcgtcgaacaggatgaagagtgggcgtttcgcggtgccactgcagttcggttcaggcgcgggaacggtcaggaccacgcgctcgggcgccgcatattgccccgggaacaccacgtatggctgccattgcggatcgttcaacagcgccagcagcgcgggatcggtttcggtgcgggcccagccgaaggcgaaggtatcggccaccacgtcggcgaccagccaccccgtgttggtgggcttgagcggctcgatgtcggccatgagcagacacacccccgcgcgcgttgtcaccgaagggcgcacagtgcacatgcagtggctgggcaccaggcggcagcccgcgcagcgctcgcgcttgaagccaccacgtgcaagaaagggtttggcgcttcgcgccaggcgcgcggtgcgaaggagggagacggcgtgaggcatgcgccgattctcggcgctcctgaacgccggcgcgctggaatgctccgggcagctagaccagctgcagatccttcggcgccaccccgtcgaacacccgcgcgagctgtgccggcgagaggccgtacatccgcttgaacagcccgccaaacaccgcgcggtattcgttgagcaccgggtagtcgcggttctggaacagcgtggcctgcgtcacttcctgttgctcgcccacgatgcgcccgccggcctctgccgagagtccgccgccgagcacccagtacacgctgccgtgcccgtggtcggtgccacggttgccgttctcgcggaaggtgcggccgaactcgctgatgacgaccaccacggtctggcgccacgcgtcgtcgcccatctcctgtgcgaagccggccacgccgcggcccagttcctcgaagcgattggcgaggtagccggtggccccgccctgccccacgtgcgtgtcccagccgccgacgtcgacgaagccgaggtcgaagcggtctcgcatcagcaaggccatgcggcgcgccaccagttcgaagcctttggcggtcatggcgttgcggctggcggcgtccatctcggcctgcaccgcgcgcgtcacctcgtcgcgcagctggaagccttcggccaccggcttggccagcggggtgttgcggtacatggccgcaatgacctcgctctgccgcgcatcgatgcccgcacgcgcattgccagcgagcgccatgttggcggccttggcgccgccgcgcagcgcaaggggcagctgctcggtgaaggcgatgggggacacgtcggtgacgggccccgcgccaagcacgccggccaggcgattgagaaaacccgagcggtagtcgcggcgcttgccgagcgcctggccgagttcgatggagtcctgcgtttcgaagtggctgcgggtgaggtcatcggtgccggcgaaggcgatgaaggaggcctgcttctgctggaacatcggcatcacgctttgtgccagcgcggggtgcaggccccagttgccgtcgagcggcagcgcgccgtcgggcgtgccggggcgggcgatggcgatgttggggcgcgaggcgtagtagaagtcgctgctcgtggggacgagcaggttgctgcagtcgtacgcgccgcgcaggaacacgaccagcagcttggcgccttcggctgcgggcgcggccatcaatcggccagcggcgcccgcgaacggaacggcggccgtgagcttgagcagttctcgacgttgcatgaccatgtgtcctttcttctgtcttgccccttccccctttgggggaaggttgggatgggggcacggcggcgttcgatcgacctcggtgattcatcaaacgccgcttgcccccacccctgccctcccccagagggggagggagaaatacattcaacggcgcatcaattccggcgacgccagcaggaaggtgttccactcctgcgggttcttcgcctgcgccagcgcctcgcgcgtgtccgcgcccaggcccgcctgcattgcgcgcaccgcgcgcgaatcggccagtggcgggaatccgggtttctcgagcggagccctgtcgtccgcgcggaacagcacggcgccgttcgcaccgatggcgcgcgcgatttcgaagcgcgtgttcatctgtcccgcgctggcccaggccgcttcgttgagcggatagccgttgggcgtctcgtggccgtacagctgttcgcccatgcgggtgatccagccgagcatcggattcacgttggacaccacgcggtcgtcgtacgcgagccgcacgccagcgatcacgtagtgcaccgggtcgcggaacttgcggccgagcgaagcggcgaactcgggcgactcgaacatcgccttgagcgtgacggcgatgtcgccgtcgctgcgcgtgaaggccgcagccatgcgttcgaccaacgcctgcggcggatcgtcggagacgaaatacacggcgagcttgcgcgagatgaagcgcgcggtggccggcgcgcgcgccaggcggtcgagcgcctcgtcggcctcggccaatccacggctctggatgggctggcccagcagcgtcttggccccgtagtcgtgccggctggggttgaactcgaacaggcccttgcgcacgtagtcggcgcggagggccggccgcacgttcggcggcggcgcgtcgagcggctggtagctcacgcccacgccggtgagcacgcgcgccagctcctgcacgtcggtttgcgaatagccgccgtccacgccgagcgtgtgcagctccatcagctcgcgcgcatagttctcgttgatgcggttggcggcgttctgcgcgttgtcgaggtagcgcagcatcgcggggtggtgcagcgtgactccgagcaggtcgcgaaacctgccgagcgcgtgcggacggattgcgttctcttcgtagtcgcccaccatcgcgcggatgatgtccttgcgcaggctgacgttgaagtggttcatccagaaccatgtcatctgctcctgcaactggttgggcgaatagagcgcgcgcagcacgaagcgctgttgcgcctcgcgcaccagcccgttgagccgctgctggtaggcctggcgcgcggccttcttctcgtcatcgcccggcaacgcatcggccgccttgcgctgcgcgtcgagctcggtgacgagctggtcgagcggcgtgcgcgaaatggccatggcatcgatctgcgcctgcgcggccggcggcagcggcgcgggccgcggattgagctggtcgcgcatccacggcgacaggccgcgccgcgccagttgcgcttcgctgctcgcattggcaccccagcccacgcggtcgagccagcgcagtcgcgcggcttcgttcaccgatgcggaggaaggcaacgacaccgaaaccagcggccgacggtcccccggcgcgctcgcgcaggccgtgagcagcgccactgcgcatgcacccagcgccatcggcacgcgccgcatggagaacaacagcgaagcggcggccggcaccgcgctcactccctctgcatatcgtggtggcgcacgtcaccgatggcgtgctgcgcggtgtcgagtgcagcgtcgacgtgcgccaggccgcgctgctggaacggccgcgagcgcgggtcgtcttcttcgcgcgccacgtcgacgcgcaccttgcgcagcaggtcgaccgccgcatgcagacggccttggcgcggcagccacgcatcggtgggctcgcgccattcgacgggcttgccgtcgagccatgccgcatgctgcaggtcagcgatggcggcatgaatctcgtcgaccaccacctgctcgtcgcgcgagacctgcccgtcttcggggcggcggtgctccaccttccaggcggccgtgcgcaggtcggacaaggcgtggaggtagaacgggtgcctgccgtattcgtcggccaatgcaggcagcgacgccgctgccatgagaaccaatgcggcgatgaggcttttcttcttcacttcggagctcctgtgagtgacgacggttcgaggatgcctcctcaaccgccgtgccctgctccgcgttgacgcactttaccttcgcagcgccgcgcaaggcagcgcctaagcgccggctaagtcaggctaccgacaggctggaaggcgcagcgccggcgatctgccgcagcgcccgctcgaacacctcgaccggctgcccgcccgagatcaggtgctggtcgttgatgatgatcgcgggcaccgagtggatgcccgcgtccgtgtacatgcgttcgcgctcgcgggtttcattggcgaattcgtcgccggccaggatctcgcgggcacgtgcggcgtccagcccggcctcggtggccgcgcggaccagcacctcggggtccgaggggttctgcctgtcggtgaagtaggccttcagcagcagtttcttgagcgccgcctgcttggccgggctttcgagttcggcccagtgcagcaagcggtgcgcgttgaaggtgttgtagacgcgcgggcggccttcggggctgaactcgaagccgacctcggccccgcgctggcggatcatctcgcgcgattgcgcctgttgttcacgggtggagccgtatttctggttcaggtgctcgaaagtgtcctgcccttcgggcggcatctgcggattcagctcgaaaggctggaaatgcagttccgccgtgacgccgggggccacgcgctggagcgccgcctcgagtgaagcgaggccaacggcgcaccaggggcaagagacatcggaaacgaaatcgatcttgagatgggaagtcatgggcgccattcttcatggcgccgacgcccttggtgcgcgcaaggtcttcaggccgcggccttggccatgcgggccgtttcaagcgtctgctcgcgcatcaggtcgtactcgagcttgtcgaccggaaccgcatcgggcttgcccaggtcgttcatgtgcacgcggtaggtctcgcgtgcggtcatggccgagatcgcggcaatggcgcagatcgccagcgtgatggcaccgacggtcagcgggatgttggcagcaccggggggcgcgaccgccacgaacagcgccggcagcagcgccgtgattgcggtgccgatgttctgcgagatcgccatgcccgaaacgcgagtgcgcgtggggaacatctccggatagaagctcgggaacacggcgttgtagccctggtagaccacgccccacatcaggagcgacatcacgatggccagcggcacgttgtggatgctgatggcgtacaggtaaccgaacgacagcaggcccgaaccgatggcgccgaccatgatcggcaggcggcggccgaccttgtccgacaggttgccgacgaacgggatcacgatcacggccaggatgttgcccatcaccggaatccagaggtagatgtctttctcgaagttgatgccgtagcccggctgcaccgcgtaggcggcgccgaagatggtcgcgaccaccgggatcacgttcatcagtgagcacagcagcacgcgcagcatgtcgcgccagctctcggtcacggcctggatcaccggcgccttcggcaccttgccactcgcgtcgacttcggtgaaggcgggtgtctcgtccacttccttgcggatgatgtaaccggccacgatgacgatgaagctcaacaggaatggaatgcgccagccccaggagttgaaggcgtccttgtccatgtagtgcgcgagcggcaggaacacggcggccgccatgatctggccggcctgcacgccctgcagcgtgaagctcgcgaagaagccgcgtcgcccgaacggcgcgtgctccaggatcatcgagctcgccccggaaatctcgccggccaccgcaaagccctggatcagccgcagcagcaccagcatggcgggtgcccacaggccgacctggtcatacgtcggcagcaggccaacggcaatggtcgaaaagcccatcaggaacatgcagagaatcagtacggtcttgcgcccgtgcgtgtcgccccagtggcccagcagcagtgcgccgatcggccgtgcgacgtagcccacgccataggtcgctagcgacgcgatgatcgcgatctgcgggtcgcccttcggaaagaagatctgcggaaagatcagcgccgcggcggtggcgtagatgaagaagtcgtagtactccagcgccgagccgatccagccgcttgcggtggccttcttcgattggtgcttgcctttcggctcgtgggccgtgggatttgccatggtttgtctccagggttgacgaaaagaatctatgcctgcgcctgcgatgccatgcgggccggtgcgttgagggcgccatacgcgtcatagcccgcggtgcgctgtgccagttcgaagaagagtccgccttcgatgttctcggtgtagatgtgcaggtagtcgcccgctggcgaacggtcgaacagcacccccgcctcgcgcagccgtgcgagcagcgccgggtcgaggtcgatgcgcgtggccaggtcgtcgtagtagttgtccgaaatgggcacgaagcgcgtgccggcggcgcgcagccgcgccacgctgtcgaagatgtcgtcgcagcgcatcgcgatgtggtgcaccgcgccgccgccggtcacgctcagcgtgcgcgcggtgcgggtgcgctggctcagcgacacgttgagcaccagccgcacgctgcgatcggcgttggccacgccccggctgcggatgagcccgaagggatcggccagctccaggctttcgcccggctccaggcccagcaccgcgcgcgtgaacagcacccaggtgtcgagctgatcgaccgccaggcccagcgccacgtggtcgatctgcgtcaggccggcatctgcggcggcggccgatgcatcttcctcgaggacgaagtcggcttcgtacagcccgttggtgcccagcgactcggcaatgaaatggatgaggttgccgcccggcgccacgatggcaggcacgcgcaattcgtccgggcctagggggctgtcgtggcgctgcgagcgcatggccgtggcacggtcgacggccgccagcggatcggcgcagcgcacgcccagcgcgcagaccgaggtgccatgcgcctcgaagcggctgcgcgcgaacgaatccggctgggcattgacgatcaggttgatctcgccctggcggtacagcaccacggctttggagcggtgccggccgacacggcggaagccgagctgcccgaacagcgtgccgagggtctgagccgacgcttcatccgccgcgaattcgatgaacgacaggcccgagagcgccggcgcggcgggcgggctgaacagctcgacgctcagcgcgcgcgcaggctcatcggcggctggcgccagccgccgctgcgcctcgctttcgaggtacagcagcgagcgcatcgcgtccaccgcagtgcgccggttgggtgtttcgcggaacacgtcgttgaagatctccagcgacagcggcccggtgtagcccgcgcgcagcacctgctcgaagaacccgatcacgtcgaagtcgccctgccccggaaacgagcggtgatggcgggcccactgcagcacgtccatcgagagcagcggcgcgtcggccatctgcaggaagaagatcttgtcgcccggaatggccgcgatgcccgcgggatcgtccttcagcgacagcgtgtgaaagctgtcgaggatcaggcccaggttcggatgatcggccttgcgcacgatgttccaggcctggccatagagcgaggtgaagcggccccaggccagtgcctcgaagcccacgcgcaggttgcggcgggcggcgcgctccgcgagttcatgcagctgggctgcggccagggccgggtcgtcgacggccagcggcgaggtgttggagcagcacagcatcgtcggcgcgcccatcgcctccatcaggtcgaacttgcgctcggcgcgctccaggctgcgccggaactgcgcctcgggcatgccctcgaagtcgcggaacggctggtacaggtcgatcgagaggcccaggtccgcggtgatgcggcccagctcgtcggcgctgcccttgaagttgacgaagtcggcctcgaacagttcgatgccgtcgaaccccgcggccgaaacggcctcgagcttctggcgaagcgtgccgctgagagagacggtggcaatggagcgatgcatgggggtgactgtaaaaacacccgtcacccgccacaacgctttgcccccaggttgcgttcgataatcgaacgtctacgtccattgttcgcacgaaacaggggttacacctaggcaagccgcccccgccgcaagcggcttttttcagaggctgcgccagtaatcgatcagcagctgcgcgaactcgaccggccgctccaccgcgctcaagtgcgccgcatcgatggtggccaggcgcgcatgggggatggcggccaccatggattcggacatggccggcggcgtcgcttcgtcctgcagcccggcaatcaccagcgttggtacggcgatgcggtggttgctctcgcgaaaatcaatggcggccacggcgttgcagctctcgatatagccctgcggatcggtgcgcaccagcacgtcgttcagcgcctgggccgcggccttgccctcccccgtggtgacgaaaccgtgcgtgagccagcgcgccaccgcgcccggcgcaatggcggccacgcccttggtggccaccgtttcgacgcgggcacgccacggcgactggtcgggatagtgggccgacgaattcgcgatcaccaagctgcgcagcagctcgggatgccgcaccgccagcgcctgcgcggtcatgccgcccatcgacaggccgacgaagtgcaccggctctctgcccgcctcgcgctggatgagctcggccacgtcctgcgccagcgtttcgacgcgcagcgcgccgggcaccacctccgagccgccatggttgcgatggtcgtagcggatcacggtgtgggcgcgcgcaagctgctcggccacgccgtcccacatgtgcaggtcgcagccgagcgcgtggctcagcacgacgaaggggccgctgccttcgcggacgacattcaaacgggtcatggtgattcctttttcatcggatgttgaagacgcggcagccacaggaacgtgatggccagcagcacgcaacccgcgagcagcatcggcacgaccatcggccaggcgccgttcgaaaaatcgttgtcgacgaactgtgccgcaagttgcccggcactgaacgccaccatcatcatgccgaagcccgaccacgacacggcccggcccgccaggtgcggcaaatcgcccacggcgccggcctgtccgcagggctggtggatgccgtggccgagagaatagatcgcgtggcccgcgagcagcggcagggcgctgtgcggcgccagccagcagcccagcgcctggatcgatgcgccggccatgctcagcgtggcgcccagctgcacggtgcgcaccggcccgtgcttgcgcagcaggcgccggcacagggtggtgctgaagatgtagaccagcgagccgcccgctggaatccagccgtacatggcgggcgaccagcccagatagccgatgtagaccatcggcgagagcaacaggaagcagaagaggccaccgtaggttgttgcggccaacgaggcccaaacgcgaaagctgcggctcgcgaacacggcgcgggcgctgccgcgcggcgccgaaagatcgctcgccagcggccgccgcgtttcgccgaacgagtgccagcaaagggcaagcagcagcagcgcgtagagcgccatcgacgccatcacccagcgccagccggcgccctgcaccagccatgcgcccagcagcggcgccagcaagcccaccacgcccaggcccgtgagcccgcgcgccatgacgtgcgggccttcgtgcgcggggtagaggtcgcgcaccgccgcgcgtgcgcagacgaggatggccgccatcgaaaagccctgcagcgtgcgccagcccgcaagcaccggcacgctgccggcgaacgcaccgccgagcgcggcgaccacatagcagcccagccccgccagcaacaccggccggcggccgaagcgatcggccagcggaccgcagagcaattgcgcaaagccgaaggccagcacgaacagcgtgaggctggtgctggccgagcccagctcttttgcgatggcgggtagcgcgggcaggtagctgtcggtggccacgggctgtgccgccagcagcagcggcaacagaaggccgaagccgacctcgaaccggcgccgctcgcgaagcccgggccgcgtcactgcgcaggcgcggccagcaatcccttctcgcgcaggatgccggttgcgatgccgaaggcgtggttggccaccggcacgccgcaatagatggccgccatcatgatgacttccttgatgtcctcgggcgtcaggcgcgactcgggcggcccgtcgagcgcggcgcgcacgtgcatcgcgaattcttcataggcatggatgcccagcatcatcgacagcaccatgtagcggcgcgtcttgtcgcccagcgccgggcggccccagatgtcgttccacgcatggcgcgtgatgagctcctggaactcggcgttgaactcgttgcggttggccagcgacttgtcgacccaggcatcgcccagcacgcggcggcggttgacgagcccggcttcgtagtcgttggcgggaggtgtgcttgcctggtcggtcatcgggatgtgtctttcgcagtcagttgggcgcgcaatgccgccacttgccggagcgccgtttcgccggcaggcccggccagggcggggtcgaaccattcgtccgccgcctcgcgcggcagctccgcgcgcagggtgtcgatgttggcacgcatgcgcgccgcgtcgatctgcaggcccggcagcgcaccggccagcgcacgcgcgctgccgtgcgcggacatgagcagttgcggccattcggccagctcggcctgccagccgccgagcgcgcgctcgtgctcctgcggcatggcggccagcagcgcggccacgcgctgcggcgcacgctgggccgccgccagcgccaccatcgcggccacgggattgcgcttgtgcggcatcgccgaggagccgccgcggcccggctcagtgggttcggccgcttcgccgacttcgtactggcccatgagcgagatgtcgcgcgcgatcttgccgaggctgcccgtgagcagccccagctcgcagccgagcgcgacccattcgtcgcgttgcgtatgccaggtcgcgccggcattgccgaggccgagctcgtccgccacgcgctgcacgaccgccgggccctgccccttcatctgcgcgagagtgccgacggcgccgccgagctgcacgttcagcgcgttgcgcgcggccgtttgcagccgcgcacggctgcgcaccaagggcgcggcccagccggcgcacttgaggccgaagctcgtgaccgaggcgggctgcatcagcgtgcgcgcaagaatcggcgtggccgcatgctgcgtggcgtgctgcagcagcgcttcgatcgcgcggtcgacatcggcttcgatcagcgcgatgccttcgcgcgtgaccagcgccatggcggtgtcgatcacgtcctggctggtgctgccgaaatgcacgaagggcacggcggcgggattgaacaggcccacggcctccttcaatgccttgaccagcggaattgcgacgctgccggcgcggccgctgtcgcgcacgatctttgccacgtcgaacaactcgaccttgcagctgccgacgatcgaatgcgcagccgcttccggcaccagcccgagcgcggcctgcgcgcgggtcaatgccgcctcgaagcgaagcatggcatcgacgaagttgtgatcgctgaaggcggagagcgtctcggacgtggaaaggaagccttcgaaaatactcatggtgaacgcctcagtagctgatcttcgccgtggcgcgcagcgcgtcggccgtggcggtgccgaagccgaaaaattcgaggtacgcgggaatcatctcgaacagcatatcggtacccacctgcacggcgcagcccttgtccagcgcggcgcgcagcagcggcgtgtattcggacttcatgaccacctcgccgacgaaggtcgacggcgcgatgcggtcgacgtcgaatggcagcggatcgccttccttcatgcccattggcgtggcattgacgaccacgtcgaagccggccggatcgttcgagcccgtggacaccaccagcgccggatagtgcgtgcgcagccgcccggcaagcgcatcggccgaggcggtgttggcgtcgaagagcgcaatctgcgccacgccggccgccgcgagcgaggccgcgatcgcggagccgacgccgccgcttccggcgaccagcacgcgcgcgccctcgagcgcgcggcccttgcgcagaacgccgcgcacaaagcccgcgccgtcgaactggtcgcccaccagcgtgccgtcggcgcgcttgagcacggcgttgcaggcgccggcgatccgcgccgttggcgtcacctcgtcgaccaggcccatggtggtgatcttgtgcggcatggtcaccagcgccccccggatgttggtgagccggaacaacgcggcgaaagccgcgggatagtcatcgggcttcacgcccatcggcaccacgaccgcatcgatgccctgcttctcgaaccaggggttgtaaatcatcggcgccttgaagctttcggtgggaaagcccaggtgcgctacgagggtggtcttgccggtgatcatgaagtccttcgcttgcctgttgaatttactttcgaaccttggcgatctcggccatcagttccttcacggtcgcctcgcccaccgtggccgtgtacttgtcgatcaccggcttgaccttgtcacgcagcttggccatttcggcgggcggaagttcggtcacggtcatgccggccttcttgagcgtgtcgagtgcggtgtcggccgcggcgcgggacgcctcgcgctggaacttggtggcttcggcagcggcatcgctgatgatcttcttctcctcggcgctcatgccgtcccaggccttcttgctgatgatcagcgcctgcgggttgtagatgtggcgcgtctgcgtgatgtgcttttgcacctcggcgaacttcgacgatgcgatcacggtgttggggttctcctggccgtcgaccgccttctggtccagcgccgagtacagctccgggaagggcattggcgtggcattggcgcccagcgtattgaacaggtcgatgtagatcggcgactggatcacgcggatcttgaggccggcgatgtcgtctgccttggcaatcgcgcgcttgctgttggtcaggttgcggaagcccaggtcccagtagccgaggccgtgcaggttcttctcgtccagcctggcaagcagcttctggccgaaggggccatcggtcacggcgtcggcttcctgcgcgttgttgaacaggaaggggaagtcgtaggcggcaaactccttgacctgcgcggtcaggatgccggcgttgagcaccgtgatctcgacggtgccgccctgcagcgccgaaactgtctgcaggtcgccgccgagcgtgccgcccgggaacagtttgacggtgatcttcttgcccgacttctcggcgacgaggtcggcgaacttctgcgcgccttgcgcctgcgggtggccggtctggttctggaacgcgaacttgagcgtgcgttccttcacctgggcggcggcgccgcccatggcagcgaccgcgaccacggcgatcagcgtcttgcggaaaaagttgttcatgtgaaagtctccttgggttgaaattagggaagcgaatagcgtgaaagtcagccgctgagcagccgggccggccagatgatgagttggggaaacatcaccatcaggaacatcattgcgaactccgcgatggcgaagggcagcacgccgcgcgtgacctcgtccatcttcatgcgcgcgacgccggccaccacgttgagcacggtgcccaccggcggcgtgatgaggccgatcgagttgttgatgatgaacagcacgccaaagtagatcggatcgatgcccgccgccttgatgaccggcatcagcaccggcgtgaggatcaggatggtgggcgtcatgtccatcgcggtgccgaccgccatcaccagcaccatgatcacgatcaacagcagcgtcgggctcgcgatcagcggttcgagcagcgcgaccagcttggccggcaggtcggccacggtgatgagccaggccgagaccatggccgccgcaaccaggaacatcacgatcgcgctggtcttggcggccgagacgaacatggcgtagaactgcgagggcttgagctcgcggtagaccaccgtggccacgaagatcgcgtagaccgcggccaccacggccgcctcggtgggcgtgaagatgccgaagcgcaagcccaccaggatgatcagcggcagcagcagcgcccaggtcgcttcgcgcagcgcggtgagcatctcgcccttggacttgcgcggcggcggcagcactttttccttgcgcaccagccaccaccaggtgaaccagagcgaggcaccgatcaggatgcccgggaagatgcccgcaagaaacagcttggagatcgacacgttggcagcgacaccgaagatcacgaatccgatcgagggcgggatgatcgggccgatcacgccggacgccgcgatcaggccgcccgagcgcgccttgtcgtgcccggcggccaccatcatcgggatcagcagcgccgacagcgcggccgcatcggccaccgcggagcccgacagggccgacaggatgcaggccgcgacgatcgccacgtagccgagcccgccgcgcacatggcctaccacggccagcgcgaggttcacgatgcgccgcgacagcccgccctggttcatggcctcgccggccagcatgaagaagggcacggccaggagcggaaagctgtcggcgccgttgatcacgttctgcgccaggatctgggcatcgaacaggtcgaggtgccacatcagcgcgacgccgcacagcagcagcgaataggcgatcggcacgccgatggccatggcacccagcagggcaccgagaaagatggcgatcgtcatgtcagttgcctcgtgcgttgttgctgccgcgctggcgtgcgatggcctcttcggcatcgcggcgcgcgagttcggcgttgatgcggtcgatgtcgccctgctcttccgactcgtgcaccatcacgagttcggcgtcgctgagcttcccgctcagtgcaagccagaggtcgtacagcaggaacacgatggccgagacgccgaacaccacgccgacgaaatagaagatgccgacggaggcgccggtggtgggtgcgctcacgtcccagttgatcagcgtctgctgccagctgcccgtgagcagcaggtacgaggcgaacagcatcaacccgtgcgacagatacaggcacagcttcttgccccaggtgggcagcttggagatcagcatgtcggtgcccaggtgggcgtgctcgcgcaccgcgacgatggcaccgagaaaggtcatccagacgaagagccagcgcgacacttcctccgacacggtgatgcccgaattgaagccgtagcgcagcacgacgttgccgaacaccatgaccaccatgatggccagcatcagcgccatgagcccttcgagcccccggcagtaccacgagaagattcttgtcattgtttgtctcctgttgaaattttttctgctcggtcgtgttgcgcaggcatatcaggcgacgttgtccgagtgatagcgcaggggggtggcaatctccgcgtgcatggccggcggatagacgatctcgcgcagaaagtcggcgtcgtcgcgcacgccctgcgccgcatcggcatggccaaagtacccgaggtagtgcggcatctgctggatcagcatctcgaagccggcctgcgcgttgaggccgcgcgcacgcgccgcgcgcaccagaggcgtcggctggttgcgcagcaggatgtcgaacagcgcggcatggcggtccatgcgggcgacgtcgacaggcagcgcgtcgttctcatccagtccaagcggcgtggcgttgatcaccaggtcgtagccttcgggcgcgttgctgtcggcgacagtcacgtcggcatcgaagaacgcgtcgagcttggccgcgacgccggcggccttgccggccgaggtgtcatagaaggcaatgtgctcggcgccatcgaccgtgccgccttcggccagcgccacgccgatggcggccgcgctcacgcccgcgccaagaatcagcacccgcttgccgcgaaacggaatgttgaagtggtccagcgcgcccacgaggccttcgccgtcgaacaggtcgccctccagttcgttgttctcggtgcggcgcaccacgttgaccgagcccgccacgcggccgaacaggccacagccgtcgagcaggtcgaccaccagcggcttgtgcggcggcgcgatcaccatgccgcgcacgttgcgggcaaggaaggccgatttgaagaacaccgcgaagtcgcgcagcggcacctgcacgggcagcagcaccgcatcgatgccgaaatggtcgaagacggcattgaacaacctcggcaggcgcacgttgcgcacggggtcgccggggatcaggtacgccagggtgctgccagtgatggaggtggtcatgtcttgcctcgtttgtgcggcaatcgctccaaggccattgccaagccgaactctatccatctcgccacgccggtcaccctcgggctaggcctaatttggccgacaatcgtgccaatgcgttcgtttatcgtacaaaagccgggtttatcccgatcgaggccagctgcggtgacggccgccgcgcctgcacacttccggccatgagcaccgatctcaccgatctttctcccgcgccggccggcctcgacaagcgcgactggatcgccggcctggaacgcggcgtgagcatcatcgaagctttcgacgacgcccatccgcgcctgaccgccagccaggccggcgagcgcaccggcatgacgcgcacggccgcacggcgctacctgctgaccctgcagcacatgggctacgtggcgagcgatggcaagctgttctggctcacgccgcgcgtgctgcggctggggcagtcgtatctcgactcggcacgcctgccgcgcatcgttcagcccttcttgcagcgcgtggcggccggcacgcacgagatcgcctacctgagcgtgatggacggcgacgaggtggtctacatcgcccgcaacggccccaaccgaagcatgagcacgggctacgtgctgggcgcgcgtgtgccggcgcaggtcacggcggccggcatgctgatgcttgcgctgcgcggcgaggccgagttgtccgagtggctggccacccggcagctgcaggtgttcacctcgtacaccattggaagcatggaacgcatgaagctcgaactggcgcgcatccgcgcgcagggctgggcgctgtcggaacagcagctcgacctcaactcgcgcggcattgcggtgccgctgcgcgaccggcacggcacgctggtgggagcgctcaacatcaccatgcccatgggccacgaaagctccgaagatgcagtggcgcgcgtgctgccggtgttgcgcgaaactgcgcaggccatgcgcaacctgatctgactgacaactatccgacagcctccgtcgggcaggatgcaggctttcttaaacacaaacgatggagacaagcaccatgtccgacaacttcctggacgacctccaacccacgcgccgccagtggctgcagggcggcagcgcaatggccctgggcggcctgctgccctcgatggccgcggcccaggcgggctggcccggcaaatcggtgcgcttcgtggtgcccttcgcaccgggcggcagctcggaaatcgtggcgcgctcgacggcggcagagctctcgcgcacgctgggccagagcgtcttcgtcgacaacaagccgggcgctgcgggcaacattgccatgagcgaagtggcgcgcagcaccgaccagcacacgctgatcctgggccacatcggcacgctggcggtcaacccgtacatctttgccaagctgccctacgacgccaacaaggacttcaagcccgtgagcctgctggccaaggtgccgagcctctacgtggtgcaccccgacgtgccggcaaagaatctgaaggagttcatcgcctacgccaaatccaagccgggccagctgagctatggctccgcgggcaacggcagcgcgggccacttggccttcgagtacctgaagatgaccgccaacatgttcatgctgcacgtgccctaccgcggcacggggccgatggtgaccgacctgctctcgggccggctcgatgcctcggccatcggcgcggccgccatcattcccttcatcaaggccggcaaggtgcgctgcattgcaacaggctcggccacacgcctgccgcagttgccggacgtgggcaccgtggccgagcagggctttcccggcttcgagatgacgcagtggtacggcatgctcgcgccggccagcattgagcccgcgcaactggccaagctgtcggccgagacgatgaaagccgtgaagtcgccggagtcgatgcagcggttgaccgccgatgcggccgaggccatcggcggcacgcccgagcagttcgcgcagttcatcgcggcggagcaggcacgctggcagaaggtgattgcgagagccaacatcaagcccgactgagcgggcaacttgccggtcagcgcgtcagcgttgccagcttcttcttcgcgctttccaggaggcccatcttctcggcaggcggcttggccttggtgtcgccgggcgcgatgatctcgaacgcgcaacgcgctgccaacttcgacgcaagcggatcgcgcggcgcgaggccgttgaacctggcgttcgagatgacgtgcatcttcagatggcgatggatgtttttcgacagcttctggcacgcggccttcatggcggattcgtcgggtgtcagctcgccatgcacgacaagaagctccacggtgccgtccttgtcctcccccaggacgaaggcgcgcaacactgaatccctgaacttggtgcgcagcatcgagcgaaccggctcggcggcggcgaacgacttcagcgcgatgccgcgcaactcgtcatggaagatgaacgcgcgatcgaccgaaacggtttcggcctcttccgccttcggcttttgccgcttgaggatgccgctgccgacaaggtgctccagggtgcgcgcggcatcggcggggtcgagcttcgaacgctgggccagctcgctgcaagaaaactgttggtccggcgccgcgtaggcgaccatcaggagcttttgtacctcaggtgcgaaaagaaaatctgcagagctcattgtttccggttctcgacaagtggatcgcattatcgagagaccggggtcagcgcctgacgatgcggttttatccgcggcgctttcgagacgatttccgtcggagcacatggtgcaggcctacagctgtgttcaatgccagccatcaagaatggctgaacacgaacaacgagcttcagttcagccatgcaccaggaaatcgacaagctcaagcaagcggacgttgcgagcggcaggtactgggccccttgcatggccatcgcattggttgcggtgtttcttttctatgtggcattgaaaggcctggtgaatgagagcgcggcgcgcgcgccaaccttgccacccgcggtcatgccagccaacgtcgagaccaccgtgccgggtactgcgacacgctcgtccgaagaaccggccttgcccccaccccgcgcgccgctggcgaacgcgacgctcgaggccccggtaatcgccccggtaatcgcccccgcggttgccgccgcggagccgcccgtcaaggctgcgcccgccttcgtcgaagtacacaagtgcgtaatgcctgagggcgatgccggctataccgatcggccttgtcccgagggcgcacgcgcgagcacgctgcgattcccacgcaacctgcgcgcagcggcgacgccgtaagcggctcaggccgccttcaggaacacgtcgtggtcgggcgcgaagttggcgtgcagcggcagcatcgcgccgcccagcgcgcaggcctgcgcacccgcccttcccccgtgcaggcgcggctgccagatgccttcccagttgcaccggcccagagccgcgcgtgtctgctccagcagggcctccagcagcgaacgagacatggacccgtccatcaccacgtcgcccaggtcgagcaccgccgtgccgcttgcaatggcgtaggccagcgcaaccgaagccgacgcaagccatgcctgcgtggccgccgcataaggcgcctccaacgcgcggtcgtcgtaggcggcggtggcatcgaggccttcgctgcgcaggcgttgctccagctcccagagcgaggcttcggcaatcagctgttgtgctggcgcaccgcctgctgctgcggactgcatgggcagcgaggccaatgcgcccgcgttgccgtgcgcgccggtatgcaggtgcgagtcgatcacgagcccgccgcccacgaaggtgtcgacgaacacatacagaaaactcttgaggtcgtggccccggcccgtgaccagttcggccacgcaggccgccacggtgtcgcgcgcataacccaccggcacgtcggtgcgagcccgcacctcggcggccaggtccatctggttccacacgtcggactgcgccttcgacagcccgagcgtgcggtgccagccgcccagctggaagggcgcggccagccccgcccccacggtgcgcaccgcgagcggacccagcccgtcgcgcagccggtggatgtgctgtgcaatggcgggcagcagttgctccgcatcgggaaactcgtagctgatggcatggcgctcgcgcacctgcgcggcaaagtcgatgagcagccattcggcaccgcgccgcccgaccttgatgccgatggcaaaggccccgtcggggttgagcgccagcggcaccgaaggctgcccgatgcggccgcgcacgcggccctgcttgacgatgagctggtcttcctccagccgcgcggtgatgagcccgatggtctgcgcgctcagcccggtgagccgcgcgaggtcggccttgggcaggctggtgtgaacgcgcagggcctgcagcaccacgcgttcgttgaactggcgcatgccgacctggttggagccgcgcgggcgcaacaggtcaggtgggcgcgcagcaacagcttctgcatcaggcatgggcctccgcgggcagctggtcggcagtcatggcgccggtcatcacggccaccgtgtcgctcatgctgatcttcttcgggttgagcacggccgcgcgcttgccgagccgcgccacgtggatgcggtcggccacctcgaacacatgcggcatgttgtggctgatgagcaccaccggcaggccgcgatcgcgcacgcggcggatcagctcgagcaccatgttgccttccttcacgccaagcgcggcggtcggctcgtccatgatgaccacgtgccgcgcgaaggctgcgctgcgcgccacggccacgcactggcgctggccgccggagagcgtttcgaccgcctgcgtcatcgactggatgccgaccttcaggtccgccatgcgcgcgctgctctcctgcagcatcttcttcttgtcgagcatgcgcagcacgttgcccatgaagcccgggcgacgcagctcgcggccgagaaagaggttctcgtagatggtcatggccggtgccacggccaggtcttgatagaccgtctcgatgcccgcgcggcgcgcgtcgagcgggttgcgaaagtgcaccggtgcgccgtcgagcaggatctcgccctcgtcgggcacgaccgcgcccgacaacgccttgatgagcgacgacttgccagcgccgttgtcgccgatcaccgcgaggatttctccttcgcgcaattcgaagtcgaccccgtcgagcgccgtgacgtggccatagcgcttcaccaggcccttggcctgcatgatgattttcggatttgccacggtgttcatcagcgggctccccggcgcgacagttgatcggccgccaccgcaagaatcaccagcacgcccgtcaccagcacctggtaaatggacgacacgcccatcagcgtgagcccgttgcggaacacgccgacgatcagcacgccgatgagcgaacccagcaccacgccgcggccgccgaacaggctggtgccgcccagcaccacggccgtgatggcgtcgaggttttcggtctgtcccgcgttcgggtcgcccacgccggtgcgcgccaccgacagcagcgaggcaatgccgtagagcacgcccgcggccacgtacgcgcccagcagcacgcgctgggtgggaatgccgaccaggcgcgtggcctcggcgttgttgcccaccgcatagatgtgccggcccgcggccgtttcgcgcagcacgaaccatgcgagcgcatagagcaccagcatcagcaccgcgccccaggtcacttcggcgctgccgatggtgaaagtggtgcccagccccgtgaggccggcgggcagatcggtgatggtctgcgaggacgaatacagctgcgtgatcgcgaacgcgatgttcagcgtgcccagcgtcacgatgaacggcggcagcttgatgcgcgtgaccagcaagccgttgagcaggccgaacaacgtcgtcacgccgatgccgcacaagatggccaccggcaccggcagcccgagttcggtggcgaacttggtcatgatgatgctgcccaacgccatcaccatgccgcacgacaagtcgatgcccgccgtgaggatgatcagcgtctggccgatggcgatgacgccaaccaccatcacctgctgcatgatcagcgagaggttgccgcccgtcagaaagcggtcggactgggtcgcaaagaaaatgcatgcgccaagcagggccagccacggccccagggcgccccacgggatgtggtgcgttggagatttcgccatcaaggtgctccgggccttgattacttcttgccccagcacagctcggcgcccgtcttggtgtccttgctgtcgacgcccgccacgctcttgccggcgatgagcgtcacgcccgtgtcgacgtagcccgaggccttcttgcccgttttggcatattccacgcccgccgccacgcccatggccgccatcttgagcgggtactgctgcgaggtggctgcaatcacgccggcgttggtgtccttgatgccctggcagccgccgtccacggaaacgatcatcacgcccttctccttgcccgcgcgcttcagcgcgttgtaggcaccggccgcggcgggctcgttgatggtgtagaccaggttcacgtcgggcgccttctgcaggcagttctccatcgccgtctgcgccttggcctggtcgccgaagctgtcggccatgcagacgatttcaggcgacttcgacagctcgttcgacttggcgtcgttggctggcaggccgaagcccttcatgaagccgttgtgccgctgcgcgcccaccgggtgccccggcagcaggtcgagcgcgacgatcttcgccggcttgcccgccatcgcggccttggcgtattcgccgatcagcacgccggccgtgtagttgttggtggcgaagagcgcatcggtcgcatccggcggatcggccgggctgtcgagcgcgatcaccatcacgcccttgtcgcgcgccttcttgatcgccggcacgatggccttggcgtcgctcggcgtgatgaggatggtcttggcacccgcggcaatcatattttccatggccgtgatctggcccgcgttgtcgccgtcggccttgcccgagcctgaaagcagcttggcgccgagcttcttggcctcttcctgcgcgccctccttcatcttcacgaagaaggggttggtttcagtcttggtaacgaggccgatgaccggctggtcggcggcaaaggcggccgacgatgcagccagggacatggccgccagggccaggatggagcgggagctgagcatgtgtgtgtctccgtgggcagacggcgtgcgcctgcggtcttgggatccggtagcgggtccgacgaaggacgcggcatccgggcgcagggagactatcggacaggagagggactaaatcaagtggatttagttatcggaaacccggaggctgaagcgccggacgctcgcaagacgcgcctcgatggcgagtcgaacatcatctttgaagctatccctgtctgctcatccacttggcgcgagccatgcccgccttgtcttaatttgcgacgccttctggtgaaacttaattgatcccattggaggaaatcaccagctcatttgaagagaatttgacaaaaaacacctgcgtatcgcattttcggttttttcgggaaaatccgtagaactccgaaggactaaaatccccaattttgatgaatttttccaacagaaattctgcatactcgaaagcctcatcactcatgccgagcgccagacgcccgtcgctcatttcgagcctttccttatcttctttttttatttcaatccgagcggcgacaattgtgcgcctggaatattggaagcaatcgataattatcgactcgccttcgccttcgcctttggaaatatccgcaattgccgacaagaatttggccgcacccttggcatcaaacctgattgttaactcattcttgctgagtggtccgaaattaaaaactatcatggacaccccagtggcacatgcacattcttcattgccaaaaaattccccggtggcgttccgttattcattttcggcgacaagaactcaaactggacatgggatgtatttgaaacattcggcgatcccatgccatgtcctccagcatagtcgccaggtccgactttaaattgccgagtgccatcgatgctgcgccacttcccttctccaaccttcacaaactggtccccgagaaatttattcctggcggcaccaattgcagatggacatattcttctgcgccactccgacggttgccgggtcgaggttttacttgagctgtccttgcctgatacaacggtgaagatctaagaaactcacttttgctcatctcttaatttttcggctccgcggggaaacgacttcaaaataaacagcaacgcagtctcaacatctggcaattccgctcgtacatacgcgtcgtagaggccgactgcatcttcatatttttccagattctcatcgaatccgatactcactgcttcacctagcagcttgacgaaacactcccaatggacaacttcgcttcgcgaaagtattcaccattgatccagaagatctttttggctcggattattgatccaagccttgaaagaatggctgcatcgctcattttttcctcgccaaaggccatttggagggacgatcgaatcacgcgagcacgtcgccgtcccatccgaacgcgacgagattgccgcgctcgtcatggcgataggtggtgcctgcgcattccttcagcgctggctcaagccgtttccctgctccctggccacttcgcggtgcagatcgtctcgctcgaagccgaaaggccctcgtcatcgaggcgcaaacagactcaatgagcttgcagagctcgttcgatcaatcggctatttgccagccgatctccgtacgcacgcacggactcgagtactgcatcggcggactcatgtgtgcgtgcagccttggcgtcatcaatcaagcctgcaacagatcgtccaatgaaaaccacacttctcgcgccacggtggtcctccatgaacacccccacggaacggcagtgagcgatcaagcgcttcaagcattccgcaaaactcccaagctgaactgcgtcctccactaccgagttgacatcctcacccccgatgagaaggaacccggcagttgagttgtaaacagctctcagatagtttttccaatcatcgtttgaaacagcaggagcaccatccaaaaagaagctttccgaagtcccgatcagttttcttcgaaaagttctgtgtcgattcatttccagtaactttgctcggccaaacgcaccttgaaactcgctaagtttgggatttaccgcacccggcaggatctccgtcaacaagaaggcggtgattgcgcctgcaagcggcagctcttcgagcgtcaacctgtacatctccattgctgattgaaaccgaagccaaacagcatcgacttcacaatcgaccgctgtcacttcgcgaaaaatttttccgcctgcgtcatcaaatatcgaaaagttgctcatcgtccgtacttgttagtagggcgcacgcgccctcgttcataggagatgtgctcgccatcggggccatggtagtgagggagctcgtaagttgggcaaggcgtctgctttgtcggtggaaactgatggccttggggatgcaccttgacctcgccggtttttctcggcccgcctgttttgcggccgccttcgcgaatttcttccacgtgcatttttgcacctgagccgtctaccccgtcggggctcaacacagtggagtagcttcttgaagtcgggatattctgggccctcatcgcagcacgtcgagcggccctcgcagtcggcaaagtgacatcgccttgggtctgctgtcgtcgttgcatgcccaccggacacagccccaaagggtcaacccattcaaccgcgctgggcgcatacacgtgagcgttttccccacccgacagcccaatcggatctttggacacaaagcgtccagcgattggatcgtagtaccgatgtcggttgtagtgcagccccgtttcctcgtcaaagtactgcccctggaaccgaatcggattcctgaaccccgcccttctccccgcctcgctgatggcctcccgcgcctcgccccacgccttgtactgcgctgaccacgcaatgctcccctcatggtccgtcaactcctgcggcgtgcccaggtggtcgcattgatagaacgcaatctccttcctgtcgaaggcgctcggcacgcttcgctgttcgccattccacagcggatcctgctcgatgtcataggcaccgccgttcgcctccatcagcgccttcacgtcggtcgtcttgctcagcgccattgcgcgcggctgcctgatctgcaccagcggcacgaaggagccgcgctcgtggatgtagtgcacgctccaaccctgcccttgctgctcgttctgcgcggcagtgctttgggtgctctcgaacgcaagcacgtcgccgtcccatccgaacgaggtggtcgcatcgcctgaacgcttggcgatgcggcggcccagggggtcgtagctgaaggtggtggtaacgccgtcacgatcggtggccgccgtcatgcggttgaaagcgtcccacgcgaagaccgtcttgcgaccgttcttcacacgctcgatgagattgcctcgctcgtcgtagcgatagctggtgccggcgtattccttcagcaggttgtcgagcagcttgttcgcggtgcgctgcagggggccttcagtctgagcggggtcgacgatgttgcccgcggggtcgaaggcgaacgtctcgcggcccaggcgactgttggcttcgagcaggcggccgacggggtcgtagcggtagtccagccggccgcggcggctgtcgccgatggcggtgagttggccggccttgtcgtaggtgtagcggcggctgagctccagcgcatcgacagggccgcgcccggtttgcgagatgcgttgctccagcaggcggccggcggggtcgtacttctggcgttggctcaggccgttgccctgctccctggtcacttctcggtgcaggtcgtcgcgctcgaagccgaggatgtcttgcccgtcgacaagaaggccgtgcacgtggccagaaccataggtgagccattgggtcacgtggccgtcagggcgagtggtggcaatgcgctcgttgagttcgtcgtagcggtgctgccagaccgcggtgcgcgcactcgcaaggtagtggtgatgctcgcgcgtcaggttgcccgccgggtcatggaaccactgcaagcgcgcatcgcgattggcggcctccaccagtcggccgttgcggtcgtatgcaaagtgctccaactggccttccccggcattccgctcgacaagacggccgagcgcgtcgaactgcaattgggtcgcgtggccggcctcgaccactgtggccagcgtaccagtggttgcctcgtgacggtattgcgtggtcttgaggtcgaagccggtttcttccagcaggcggcccacagggtcgtagcggaagttgtaatggctgccgttctcgttctgcagctccgtgagccggcccagcaagtcccagtggtatttgagtgagcggcctgccgcgtcggtgcggctggcaatgaggcctgcacgcgtgtagctgtagcgcgtgcgccggccgagcgcgtcggcgtgtgcgagcaggcgcccttcggcatcgtgcgtgaagtgctcgctggtttcgtcgggcagcacgatttcttccaactgcccagcggcgtagcggtagctggtggtattgccggctgcatccacggccttggtcacgcggctgcgctcgtcgtactcccatcggctggtcttggcggagcaatcggtgtggctgagcaattgcccagacggggaataagcgagcgccttcacgccgcccttcgcgtcggtaatgcgcacgggccgcccggctttgtcataggcgtactcggtcttgtggcccagcgggtcgatctcttccgtcaggtggccctgcgcgtcgtagtcgcgcttccacacgccgccctcggcgtcgcggatgcccgtgagccggtgctggttgtcgtactcgaagtgcacctggctgccgtccgcacgggtgtgcgtctgcaggttgccgtcttcgtcgtacgtgtagtcgtcggtggttccgtccgtatgcacgtggcgcgtgacgttcttcgcgtcgtcgcgaaagaaccattcctccagcttgtcgggatggatgattcggtaggtatagccctggatgtcgtagtagtgccaggtctcgccgcccagcgcatcggtcacgtaggtcaggcggatgttcgagtcccactcgagcaaaagcgcgaagctgccgtcgtcggaccattcgcgcacggccttggcatcggcaccggtgccgctgtactccaggttcatgccccggccggtgcggtcggtgtagcgcgtgatcaggtggtgcgagtagctgtagctccagctggcgccgtcctcgtcctgtgccgcgaccagatcgcgttcggcagcatcatgcgtgtaggcggccagctggcgaacgacttggccgtccttcagctcccacagcgattggatgaggcccatccgcgcatcgggctgcgtgccgacatgcgccatgacgacatcgccctgcttgctgacgatgtcgctcagcacctgctcgccggtggaggcgatcacatggtcgtaacgcaggccgatcgacatgccgtccttcgcttgctgcgccacgagacggaagtgcggctgcttgctgtccaccagctcatagagttcgcgccactcgctttgctctcccgcaggcagcggcttgccgaagtccagcgccagcaaggtctcgctgagacgcgagatcgttacttcctcaatcgcatcgcgatacgcctgcccaaccgccaaagccggatacgcatggctgcgcccgtcagccgcgtgatagacgaggctcgcacgtccctgacgggcgccgcgcgagggcgtcgcgatgtccacccgcatgctgtagggcgtgatccatcgggcacccaggctgcctcggtcgaaggcatcgagatcgctggcgtaggtgcgcgcccattcgatcggcagcggcgcggcaagcacaaaatcggtgtgcgtgaagctctcgttgccggtcgcgaggctgatcgaagagcccttgcgcgctggggccgggcagttcttgcaacctgccgcaggtcctcgtacttccgcctgcctgctgatgtggccgagcgccgcacccggcttggccttctcggccttggcccccgcctgcggcgacacgatggccgaacccttgcctttcttgcgcagcagcgcatctcgcagcttgttcagcaaccacatgatgctggcctgggcctcccggtcagccagcttcgataactgcccgcgcagcagccgcttgaagtccagcatctgcgtgatgacgccgtcgacccggctcgcgacgcccgcgggcagttggttcgccgccgccttggccacgtagttcgccgactgcttggtgtagcgcaccgcagtgccccacatccggctccaggtgctttgggtcttcgggtcatgcaccttcgtttccgccgccccgggcctggccacggtaaacaggtccttctgccccagcacgcgccgaaggatgtcgacgaggttgtcgatgatcttgtcggccaggtccgcgcagctcttcaggatgccgtcgagtttggcgatcgcgccgtcgatgaacttgtcgagctcccccacgatggtggcgttcaggtgccccaccagcgtggtcacgatggcctcgcccagattcgaggcggcgctcttgagctgctgcttcaccaggtgcagcgtgggccgcaggctcatgcgcgctgccgccatggtcggcggcagcgggatcagcccgatcaggttgatgcccagactcacccaggtcaggaacgcttcgacgccgtccttggtcttcttttcgacaatggtgatgatgtccaggaacacatccaccagcgccatgatgttgccgacgatgggaatgctgccgagcaccatcgtgagccgctccagcgtgacgtagccgccgctgaacgagcgcagccagttgtccaccgccttgctcgccgccgcgatgtcttccttgacgatggtgttgagcggcgccactgccgtctgcggttcgcgctgcgccggcgccttggttccttccgtccctgacatttttttatgttccctctcaattgatgttcgcgccctggaactccagctgctcgaaggtgctgttcgtgaagtccacgctgcgcccttgcagcccctgtgcgtgcaccactgtgccgctgcagttcagcacgccgacgtcgttccactgcccgcgcgcaaagctgatgtcgtcccagcggcactgcgtgaaggtgctggcgccgatgctgccgccgtcgaagttcgcgcgcgtgaagctgcaattgacgaaggtgcagccggtgatcgagatgccgccaaagtcgcattgcgtgaagctgcagcccgtgaactggcaagcgctccagcccgcctgcttgaagctggtagcggtgaagctggtacccgcgaaagtcgagccggcgaactgcaccaggcccaggtcgagccccgcgtagacgaagctgtcggcttgcccgacgaggccggccggcgcaccgcccgcgcctttgcgccacatgtcgtgggcaaggatgatcaactgcgagctcatgtcagcgggctccacccggatacgaccttctccgtctctatctgcttcagcagccagccggcttcgtcattgccgtttttctgggcctccgccgcccagtacgcggccttttcgaggtccgtgccgtccatgtacaggtcgtaggcgaggttgtgctgcgcaacgccatggccgcccttggccgccatcgacagccagtgcatcgactgttcggcgtcggagaacgtgaaggtgtagtacagcgagaggcggaaggcagactcggtattgccggcctcggcctttgcgatcagcgcaaggcgctgctcgtcggtgagcgcgaagctctgagcgcccgagatgggagagagagacgagatcgaagcgggggcgtcgttgtccatgaaactgttctccgttgtgtaaggcgctcagcggcttgccgcttcgcgcaggatctcgccagtggtcttcgacgcgatgtagagaaccgagcggccgagacggtttgcattgcccaggcctttcctgcccggttccagcttcgcgacaaaagcgatcccgatggtgttctcgccgttctcgtcctcgccgttctcgcgcgtccgctcgctgatctggatctcgaagttcttcaggtcctgcccagtttgcgcaaagcgctcgcaggcgcggctcagcgcgatggcgaggggtgggttgagttccgggtccaagatcggcacgtcccggttcaatcgatgtcctgatagatgctccaccccgaaatgtcggcaccggactcgtcctcgaactcctcgcaaatcacctcgatcgagtttccggacggatccacgatcctcgcgatgtagaaggttctgatggccgggaatcctcagcacgtccatatccgggtccggctcgtagccgagcgcgttctcgtagaacgcagtcatcttctcgggaatccccttctttcgaagcatggggacatgaatggcgaatggcctcatttccgtaccttccttgcgacccgatgagctccaaattcatggccgaggcttacgggccgccgcagatcgggccgcctcgatttccttgagcagttcgcctgcattcgagttgccgttcttcagtgattccgaggcccagtgcgtggcgccctcaagatcctggtccttcatgtacagctggtaggccaggttgtgttgtgccacggcatggccgcccttggctgcgatggacagccagtgccgctgctgtgcgtagtcctgacgcaggaagccgtagtactgcgaaagtcggaaggctgattcggtgtcgccggcctccgcctttgcagcgaatgcggtgcgctgctcatcggtgagcgcaaagctctgcgcgcccgagatgggcgacggcgaagatggggatgcaggggtgtcgttgtccatgaatttgttctccgcggcgtgtgagatcgaaagcgcgagtgccagcagggtcggcactacgcgtgtgaggtgaggcttcgtcatggcttgggattgaaggtgtgccatcgtccgatgtcgcccgtatccatcgtcttgtcctccttcatgcccgctggttgaaccttgccgttgggccagatccagaggaacttgtcgggcccgctgaccggtgcgccgagttcgttggccaccttctgcgcgtaagggtcggaaccgttgccggtgttgcaggacatgagcacgacgtgctggccttgggtatacgaagggtgggccttgatgcggtccgccatttgcttgggcgtgatcgggtcgtgcaacgcgccgaccatgacatccgaattgccgtggccacccaccgtgaaggtgcctttcggattcgggatgttgtcggccgattgccggatcccctcgtcgtgcggaaacagattgagatcgaccagccccagcggatcgatgccgcgcaccgggttgttgcccacgtacacatgcaggttgcgtccacccgccagtcccagcggatcgcgcgacacgtagcggccgcttgtcgggtcgtagtagcggtagcggttgtagtgcagcccggtttcggcatcgaaatactggccctggaagcggatcgggttcgcaaggcccgcgcgccgccctgcctcgctgatggcttcgcgcgcctcgccccaggccttgtactgcgcggaccacgccacgcggccttcatggtcggtgagttcgtgcggcgtgccgaggtgatcgcactggtagaaggcgagctcgtccggcgtgaagccgtcgagctcgggctgctgttcgccgttccagagcggatcctgctcgatgtcgtaggcgccgccgttggcggccatcaacgctttcacgtcggtggtttcgctcagcacgatggcccgcgcctggcgcacctgcaccagcggcacgaaggagtcgggctcgtggatgtagtgcacgctccaaccccggccctgctgttcctgcgcgccggaaatgctctgcgtgctctcgaaggccagcgtgtcgccgtcccatccgaacagcgtcatggcatcgtgcgagcgcttggcgatgcgccggcccatcgggtcgtagctgaaggtggtgccggtgccgtcctggttggcggccgcggtcatgcggccgaagccatcccatgcaaaggtggtcttgcggccgttgcgcgtgcgctcgacaaggttgccgtgctcgtcgtagcgatagcgggtgccggcgtattccttcagcaggttgtcgagcaacttgtgcaccgtggcctgctgcgttgccggctcggcgttcgcagggctgacgatattgccggccgggtcgaaggcaaatacttcgcggccgagacggctgttggcttccaccagacggcctaccgggtcgtagcggtaaccgagattgccgtaccggctgtcgccgacggcaatcagctggccgatcttgtcgtagctgtagctgcggcgcacttgcaacgcctcgatggcgctcggacgggtctgcgcaatttcctgttggagcagccggccaccgctgtcgtagcgcaaccgctggtggaggccgttgcgctgttcacgcaggacttcccgatgaagatcatcgcgctcgaatccgagaatgtcttcgccgtcgagcagcaagccgtgcacatggcccgagccataggtcagccactgggtcgtgtggccatcggggcggatggtcgcgatgcggcggttgagctcgtcgtagcggtgctgccaaaccgcggtgcgcgcattcgcgaggtagtggtgatgctcacgcgtgaggttgcccgccgggtcatagaaccattgcaggcgcgcgtcgcagttgacggcttcgacgatgcggccattgcggtcgaacgcgaagcgctcggcctgctcaccggccgtgcgctcgacaaggcgccccatcgcatcggattgcagttgcatcacgcgcccgccctcctctacggcaaccaaacggccggtgctctcttcatggcggtagtgggtggtcttgcgatcgaagccagtttcttcgagcagacgacccaccgggtcgtagcggaagttgtagcggctgccgttctcgttctgcagttctgtcagccggcccagcagatcccattggtagctgagcgaatggccggccgcatcgatgcggccagacaccaggcccgagcgtgtgtagctgtagcgcgcgcggcggccgagcgcgtcgacatgcgcgagcaggcggccttctgcatcgtgcacgaagtgctgctgcgtgtcgtcgggccaggtgatctcttcgagctggcccggagagttgccgtcgccgcgctgcacgatgccttcacctgaagggctgtaacggtagcgcgtggtcagccccacagcatcgatggccttgatcatccggcctcggctgtcgtattcccagcggcgggtcttgcccgagcaatcggtgaagctcgcaaggcggctgccaggcgtgtagctcaacagcttcgtgccacccttggcatcggtcacgcgcaccggccgccccgccttgtcataggcgtacccggtcttgtggcccagcgggtcgatctcttcggtgaggtggccttgcgcgtcgtagtcgcgcttccacacgccgccctcggcatcgcggattcccgtgagccgctgctggccgtcgtactcgtaatggatgcggctgccatccgcgcgcgtgtgcgcctgcaggttgccgtgttcgtcgtacgtgtagtcgtcggtggttccgtccgtatgcacatggcgcgtgacgttcttcgcgtcgtcgcggaagaaccactcctccagcttgtccggatggatgatccggtaggtgtagccctggatatcgtagtagtaccaggtctcgccgcccagcgcatcggtcacgtaggtcaggcggatgttttcgtcccactcgagcttcagcgcaaagctgccgtcgtcggaccattcgcgcacggccttggcatcggcaccggtgccgttgtactcgaggttcatgccccggccggtgcgatctgtgtagcgagtgatcaggtggtgcgagtagctgtagctccagctggcaccgtcctcgtcctgcgccgcgacgaggtcgcgctccccatcgtgcgtgtaggcggccagctggcgaacgacctggccgtccttcagctcccacagcgaccggatcaggccggtcttcgcatcaggctgcgttcccacgtgcgccatcacgacatcgccctgcttgctgatgatgtcgctcagcacgcgttcgcccgtcgacgcgatcgcatggtcgtaacgcaggccgattgacttgccgtccttcgcttgctgcgccacgagacggaagtgcggctgcttgctgtccacgcgttcgtatatttcttgccactcgccttgcttgccgaagtccagtgtcagcaaggtctcgctgagctggctcaatgtcaggttctcgatgggatcgcggtgcacctgtcccacggccagcgcgggataagtgtggctgcgcccgtcgaccccgcggtagacgagccctccctgcggtgcgatgtcgatgcgcgtggtgtacggcgtgatccaacgcgcacccagcaggccggggtcgtatgcatcgagctggctgcggtacacgcgcgaccacgtgatggacagcggcgcgctcagaacgaagtcggtgtgcacgaagctctcgctgccggtcgcaaggctgatcgagccaccgacggccgcgcgcgccggccggttgcggcagcccggatcgttgcgggccggcgcctgcttgttgatgtggccgagttgcgcgcccgggcggtccttgtcggccaccgcgcctgcgcgcggcggcacgatggccgcgcgctgccccttcttgcgcttgatggcctccagcagcttgtgcagcagccacatgatgctggcctgcgcttccttgtcggccagccgcacgagttgcctgcgaaagttgcccttgaaatcgagcatgcgcgcgatcacgccgttgacctgtcccgccacgctggccggcagctggttggccgccaccttcgccacgtagttggcagactgcttggtgtaacgcaccgcgctgccccacatgcggttccaggtgctctcggccttcgggtcgtgcacacgggtttccggtcgaggcggcgtaccgacgctgaacatgtccttctgcccgagcacgcggcgcagcacgtcgaccaggttgtcgatgatgctgtccgacagcttcgcgcagctcttgagcatgtcgtcgagcagcgagatcgccttgtcgatgaacttgtccagctcgcccacgatcgtggcgttcaggtgccccaccagcaccacgacgatggtctcgccgaggttcgacgccgccgtcttgagctgctgcttcaccaggtgcagcgtgggccgcaggctcatgcgcgcggccgccatggtcggcggcagcgggatgagcccgatcaggttgatgcccaggctgacccaagtcaggaacgccgcaacgccgtccttggccttcttctcgacgatgttgatgatgtccaggaacacatccaccagcgccatgatgttgccgacgatggggatgctgcccagcaccatcgtgagccgctccagcgtgacatagccgccactgaaagagcgcagccagtcgtcgactgccttgctcgccgccgcgatgtcgtcaccgacgatggtgttcaagggcgcgaccgcggtttggggttctctctgcgacgtttgctgttgcgatccttcggccattgccttgttttccctctttgcctggtatttcttgttattcgaagagcacgcggcagccccgcgtcagcccatgaaaccgggcgtgcgccccgcgagcgcgggctgcgtggcggcggtggccatgcccgtcttgacgcccgctggcacgccgccgctcgcaacgctgcccgccacgttcgccatgccggcgatcggcacgcccatgggcccgagccgcgcccccgctgcctgcatcgccatgcccgtggcggcctggctcgcctggccgagcagcgccttggcgccgccctgctggatggcctgggccgcgctgacggcctgctgcgccatgcccgccgcctgcgtgacctggcccagcatgcccgcggccttgctgttcgtgcctgcaacgccggccagggcgcccgctgcgccgccggccgaaccggccatgccggccaagccgcccgcgccggccagaaagcccgaggtccccgccgcatcggcaccgccggcggtcggctctttcgccttccagtccttgggcgtgccgaagtagctgccctcttcccatggatcgcgcgggtccttgccaaaggtgaccttcgcggtaccgatcggcaggcccgacacggtcgcgaaaccgttgcggtcgaaggtgccggcgtgcgagccgccttccgaatcgaccacggtgaagtcgccctgcgcaacgccctggtgcttttcgcctgtcggcttgatgtactggtggtacaggtcgagctgccccttgggcagttgcggcgggttgggcagcgaaggcttgccctcgctggccgggcccacgaggctgtgcaccgcggcgtgctcgcgccaggtgcccgaggtgccgtgctcgatgccgcccgagctccagcggctgtagctggagccgccgttgatgaccacctcttccttcgcgtggatggtgatcttgttggcggtctgcgtgatgttgagcttggccagcacgttgacgctgtccttcagcgccttgatgtcgatgtcggcgctggccgccaccagacgcatgccggccttggaggcgaacatgcggatggcgctctgcacgctcaccaggaagctcttgcccgcgctcacgctggtgtggccgccgctggtgagcgcgttgtgctcgttgctcaccatgtgggtggagccctgcgccacggtctgcaggcccttggcgctggccagcgtgaggtgcggctcctgaaactctgggaagtcgccttgctcgcggttgccaccctgacccttgatcgcgtcgttctgctccttcaggcccttggcaacttcgtcctggtcgccgctctcgtgcgcctctgcggcctgggcggcttcgctcaggccttcatgcaggtcgcgcgcctgcgtgagccggccgacggtctcgcccatgtcggtggtgtgcgcctgcgcattgggccgcggctcggtggtcaccagcagccccctggccgcgcgcgccacgccatgtccgtcggtgcgcagctcgaagccctgcccgcgcggctccttgcgccccgcggtgtcttcgatgcggccgatgtgccccacgctcagctggctggcctggtggtcgctgcgcagctgcgcctggatctttccgtgcgtatcgtcgagcaccaggtgattgccgcgcccgccgccgagttcgcggctgcgaatgcccgacaagtgtttttgctccggcagctgccacgccgccatcgtgtctgcgttgtagacgcagccggtgacgatcgggtaatccgggtcgccgttcaggaagtcgacgatcacctccatgccgatgcgcggcaccgacaccgcgccgaaggtggcgcccgcccaggcggtggacacgcgcacccagcagctggagttctcgtcgtccttgccgaggcgatcccagtggaactgcaccttgatgcggccgtattggtcggtccagatttcttcgccggccggcccgaccaccatggcggtttgcggaccgcgggtgcgcggcttgggcgtggtgcgctgcgggcgccacgccaggctggtgggctgcacgtcgaaggcaaagcgctgcaccgatccctcggtggcatccgccccctcgctcgcctgcaggttctcctgcaggtggtagctcacgctcagcaacaggtactgctggttctggtcggcgcgggggtggccggtcaggcgcagcgtgtggcccgtcgcaagctcgcgcaggttggaacggccgctggcgcggctgcgctgggtcagctgctcttcgttgcgaagacgcgcgtaggtttcgccatcggcgtgctgcacgaagccaccgggccactcgtagttctcgtagccatcgtggtcatggccgggcggcatttgccgcaggtgcgagaggtcggccttgggcttctcgaagtcgtagtcgttgttgtagtgatggcccgcgcgcacctcttccgcggtttcccaggcatagatgcgttcgcgctggcccatgccggatttttcaagcgggtggtaacgcaccgactcgccgccgggcagcggaccgtgcgagcttgcgatgtcgtccgcaaacaccagaacgtgctgcgacgcctcatgcctgaagtagtagtagatgccttcgagctcgcacaggcgcgagatgaagttgaagtcgctctcgtggtactgcacgcagtagtcccagcggcggtagtcgccccggctgagcttcttctcgatgggatagccgtagcttccgagcacctccgtcaatatctctggaacggtcttgccctggaagatgcggaagtcgctgcgccgcgtggcaagccacagccagggccgcagctgcaggcggtagaaggaatggcgcgcatcttcctgctgcaggccgaagcgggtcgcaatgccgcccaggtatcgcacgccgccgctttcggtttccaccgccacggcggaggccttgccgagcagggctttcgggtcgatggcgttgctgctgcccagcagctcgatgtcgaaggcgtagagctggctgagcgcctcccggcccaccagttggcgaaattgcaacgcctcgcccagcggcgtctggatcgtgacgcggcggctcattgcagatccgcagccagccaataagacaaattggctaatgccaattcattcaataagaatattgttttcagatcgagcttcatgctcagctccccttccattatttgacaattattttaaatgttgatttatcgtaagagccaatgcaaaggttaatctttcaggggagatgtggaagatttccgcctttttctcccagcgccgaggccatcggcacgcaccgcgccctaccgctgcaattcggaaaacaattcttgtaagaagaaatagcgcatgaagcgcgagaattcgaagcgccgaattctttttaaatcaggctcagcgttgcgggcagtttgccgcgctcttcaggcagcgctcggcgcaattggccgtcccggctgttccagcttcatcacccgccacgcacacaggctgcccactgccgccagcaccgcggccagcgcgaacatggaccggtagccgacctcctgcgccacggcaccgcccagcagcacacccagcacgccgccaaatccatagccgatcaccgtgaagagcgcctgcccgcgcccgcgcagccggccggggaagcggcgcgagacgacggcaatgcaggtggtgtggtgcgccgcgaagctcagcgcatgcagccactgcgcgacgatcagcgccgcgatccagcctcccagcccggcggtcaggcccagccgtgccacggcggcaatgccgcacaccagcatccagcgcggcatcggcaagaggccgatgagccggccctgcagaaagaaccagacgatctcggccaccaccgacagcgcccagagcaggccgatgacgcttttgccgtagccgagcgaatcgaggtacagcgagaagaatgcgtagaccgagaagtgcgacatcacatggaagaacagggatgcaaagaaccaccgcacggccggaattcgcagcaccggcccgatgggctctttcaccgcatcgtgcgccgccaccggctcgcggatgtcgggcagcttcatcgtcgcgatcagcacgacggccagcgtgcccgccgcccaggccggaaagtgcttcatgccgaagcgctcgaaccactcgcccgcaaagaacaccgtcaccagaaagccggccgagccgcacagccggatgcgcccgtagcgcccccagtcgccggccaccagttgcgccatggcggcctcggtgagcgacatcatcgagctggtgtgggtgaacatcaccagcagcaccagcgccagccaccacgcgccgccgtgccaccagagcccgaaggagctggccagcgccaccgccgcgctgaagcgcagcagcttcacgcgctggcccgtgtggtcgctgagcgcgccccaggcatagggggcgaacactcgcgtgatcgactgcaccgaggccagcaggctgatcgtgaagatcggcagccccaggtccttgagccacagcggcaggtaggggttgaagaaaccgatgtgcgcgaaatagctggccgacagaccagcgaacgccagcaggtggccgcgtccggcggccactggtggcgggagaggcactagaggaaggacgcctgcggggacgcggcttcggtcgtttcgtcttgcgctttttgctgttgctgcgcgtcgccgcactgcgcgcggttgcgcagcgcgtgctccatgaccaccagcgcaagcatggcttcggcgatgggcgtggcgcggatgccgacgcatgggtcgtggcggcccttggtgaccacctcgaccgggttgttgtgaatgtcgatcgactggcgcgggctgatgatcgaactggtgggcttgatcgcgatgctcacttccaggtcttgccccgagctgatgccgccgaggatgccgcccgcgttgttggtgacaaagccggtgggcgtgatcgagtcgccatgcgtggtgccgcgctgggtgatgctgtcgaagccggcgccgatctcgaccgccttcacggcgttgatgcccatcatcgcgtaggcaatctcggcgtcgagcttgtcgaacagcggctcgcccaggccgatgggcacgttggtggccgtcacgcgaatgcgcgcgccgcacgaatcgccggccttgcgcaggcggtccatgtacgcctcgagttcgctcacgtcggcaatgggcgcaaagaacggattgttgggcacatggtcccagctctcgaacggaatggcgatttcgccgatctgcgtcatgcagccgcgaaacaccatgccgtatttctcggccagccacttcttggcgaccgcgccggccgccaccatgggcgccgtgagccgtgccgaagaacgcccgcctccgcgcggatcgcgaatgccgtatttcttccagtaggtgaagtcggcatggccggggcgaaactgctgggcgatctggccgtagtccttgctgcgctggtcggtgttctggatcagcagcgcaatcggggtgccggtggtcttgccttcatagacgccggaaagaatctgcaccgcgtcgggctcgttgcgctgggtaacgtggcggctggtaccagggcgccggcggtcgaggtcgccctggatgtcggcttcgctcagttccatgcccggcgggcagccgtcgatcacgcagccgatggccgggccgtgcgactcgccaaaattggtgaccgcgaagagagttccgaatgtgttgccgctcatggcggggattatccccacaaagcggcggccactcagtctgtcgtgttttccatgcgcttggtgagcgtgcccaactgcagttcgatggagaagagccgctcgttcagaacggcggtctgcagccgtatcgcctcgatgatggccttggtctgcggatccgaggtgttttcggacagttccgccaggtcatgcagcttcttgcgaagttcgttgctcatgggaggctccgttcatcgtctcgtcgtggagcctgcagtatgggtcttcgtcagcgctcgggcaatgcatccgatggcgccttgggctgcgcggcctctccggcgctgcgcagccgcacggccaccagcgcacctaccgcaagcagcaccgccgcgcaaatcccggccgtcagccgaaggccatgcagcaaggcggcccggcccgcgtcgagcagttcggtgctggcagtgcctccgagttgtcctgccagggccaccgccccgccgagcgtgctgcgcgccgcttccacctcggcggcccccgccaaccccaccggaacggcgtcggccatcgtgctacggtagatggccgcgccaatgctgcccagaattgcgatgccgagcgcaccgccaaactccgaactcgtttccgaaatggccgaggccacgcctgcgcgctcgggcggcgcgctgcccaccaccaagtcggtggccagcgtaaaaacaggtgccaggccgagggaggaaatgacggtgctgctcaccatccacgccaggccgccctcggcaggaagcaccacgagcatcgcgaatcccaaggccgcgacacccaacccgccgcccatcacaaacgcgggccgcatgcggcgcaccagcgcggaaaccaccatggagccggcaatgaaggcggccgcactcggcacgctccaaaggcccgcatgcagcggcgagagcccgagcaccagctgcaggtattgcgcgttgtagagaaagatgccgaacatcacgaagcaggccagcatgtaggccgccagcgagacgctgaaggcaggcaaccggaacaggcgcaggtcgatcatcgggtcgacgagccgccgctgcctgcgcgcgaatgcccacccaagcgccacgcccgccgcgatggccagtgccgacacggcatccggcccgtgctccgccacctgcttgatgccgtagatggctgccagcaccgcgccgagcgaaagcgccacgctggccaggtcgagccgtcccgcttccgggtcgcggtattcgggcagcaggatggggccgagcaccagcagcaacaccatcaccggcacgccgatcaggaacaccgagccccacggaaagaactgcagcagcacgccacccagcaccgggccgatgaccgcgccggccgagtagctggaaatccagacgccgatggccaccgtgcgctgccccggatcgagaaacatgttgcggatgagcgagagcgtcgacggtgcgagcgtcgcgcccgccacgccaagcagcgcccgggtggctatgagcatgttggcgctggtggaaaacgcggccagcaccgaggcgatgccgaaggccgccgcgccaatgagcagcagccgccgccggccgatgcggtcgcccagcgtgcccatggtgaccagcagcccggcgacgaagaagccgtagatatcgacaatccacagcaactgcgaggcggtgggcttgaggtcttcgctgatcgagggaatcgcaaggttcagcaccgtgagatccatcgaatacagcatgcacggcagcgcgatgacggccagccccgtccactcgcgcgccgttgcgcgggccggcgtcggtctgccggcaggctcgtcgcgccggccggtcattcagccgctttcgccaaccatcgctcgagcttgagcatggcgccggtccagccgtagttgtgtccgtcgcgcgcggcttcgtcgaagaactgctcgtgccgcaggaccagttcgcagccgttgccgtcgggctcgatcagcacggtcacgcgcgactcacgctccggcgtgctgcgccaggcccagctgaagaccagcttgcggttgggcacgagctcctggtagacgccgctcacgtcgtgcgtctcgccgtcggccgcaagcatggccacgcgaaagcgcccgcccacgcgcaggtcgacttcggccacggggacggaaacgatctcctcagggccgaaccaggctttcagcgcttgcgggtcggtccacgcgcgccagaccttttcgggggcgacggggtagtgcctgcggagggtgagcgaggggcgctctttggcgggggcggcaggttttgccattcggtctcctcttgatgatagagatagcgcgccagcgcatcgaggcgcccggtccagaatttctcataccgcgacaaccacacggcagcctcctgcatgggccgcggcgagagttcgcagcgcacgatccggccctctttcgtgcgcgagatgaggccggcatcctccagcacccgcagatgcttcatgaagccggtcagcgacatcccatgcggctcggcgagctcggtcacgctgaggctgcgctcgcccagcgtttcgagcacggtgcggcgcgtcgggtctgaaagcgcggcgaacacggcgtcgagcgtggcagcatctgggtgaaccatgtggttgagtatctcgcacccggcgccgtttgggaacgctttatgcgtgctgcagcgcagcaccaccctcaaaacctgcgaaggagcgccccatgctggaccgaaccgccacccagttctcccacgtcaaacccggcgacaccgagtacgtctcgggcggcctgcgcgatttctttctctaccgcgacctgggcattgcagaggccaccaacggcaaggtcattgcgcacctcgtcaaggccaacatggcaccggaaacgggcacgggctggcaccgtcacgaggccgacttccagatcgtgctgatgctcaagggttgggcccgctttatgtacgaagacaaggaaacgctggtcgaggccggcgacgtggtgcaccagcggcccggcatccggcattttctttttgactactcgccggacatggaatacctggagatcgtctcaccggccgacttcaagagcatcgacgtcgatccggtgtgcgagattccgccgcccacgccctggccctgaccatggcgcagggcctgcagggtcaggccgagaccagcatcccgctgaccagcagcgccgcgaacagggcggtcaccgcgcgccacgatgcggggcgcacttcgacccagcggtacagcagcagcgcagccgccaccgaaagaccgaaggtggcggccatgcccagcgcatcgatccaggccgcatgcggcctcatctggccgaccgcggcattggtggccagaagcaccggaaagtggatcaggaacagcgagtacgagatgcggcccagccgctgcagcggcatggctgcgtccggccagcgtgccatcgacagccattcttgccgctgcgcgatggcaatcagcaacgcgctcacgagcgccgtggcaatgcggctgcgccagtcgatggcgagtgcgccggcgccggccagcgccagcagcacgatggcgccctgccaggtgctggcgcgggtcgcgcgcccgatccagaacaccagcatgccgagcccgtaggcgccgaagaagtagagcgccgtggcgtcgagatcggcgttgcggttgaaaagcaccagcgaggccagcacaacccccagcaccagcgccacggatatccagcgttcgcgcgaggccggtgcggccggcgtccgccgccacaaggccggcaaccccatgagcgtcagcgccagcacaaagagctggaagtcgatggccacgtaccagaccccggtggacagcgactcgtatccgagcaggtcctgcatcagcaatccatgcgcgagcaactggccgatgctgggcgaggccggcacgtcgtcgccactcatccaggggcgcacgatggcggccaccagcacgcacacggtgagcgcggccaggtaaggcatgaccaggcgcccgtagcgctgaaagatgcgcgccaggggacgatcgacgcgcaacacgccgtcgggtgcgaggctggccgccgccagaaagcccgcgatcaccaggaagacctggacggcaagacggccgtcatcggccagccagcccaggaaatccggcgccagcggaaaggcccccaccggcatcgagccgtagcgcgacaggtgatgcccgacgatgaccgcgcaggcgattccttttgcgatgtcgagcagcggcatccgcccgcgttgcgcaggctgctgggcggcagccgccatgttgccagcgccgctcaaagtgcgagccgctgccttgcttcgaagtattcgcgcttgagcttttcgatgaacgcagccgcgctggccacttcggtcacggcgccgatgccctggcccgagccccagatgtctttccaggccttggccttgctgccgtcgccgccgccgaagttcatggtcttgacgtcgccttcgggcaggttggccgggtccatgccggccttgacaatgctgggcgccaggtagttgccgtgcacgccggtgaagaggctggaatagacgatgtcgtcggaggtgccgtcgacgatggcctgcttgtagtcttcgctggcgcgtgcttcctcggtggcgatgaaggcggtgccgatgtaggcgaagtcggcgcccatggcttgcgcagccagcaccgcgccgcccgtggcgatggaccccgacagcgcgatggggccgtcgaaccactggcggatttcctgcaccagcgcaaaggggctcttcgtgcccgcatggccgccggcaccggccgccaccgcaatgatgccgtcggcgcccttctcgatcgccttctgcgcgaacttgttgttgatgatgtcgtgcagcgtgacgccgccgtagctgtgtaccgcgtcgttcacgtcggtgcgcgcgcccagcgaggtgatgacgataggcaccttgtacttgacgaccatttccatgtcgtgctcgaggcggtcgttgctcttgtgcacgatctggttgatggcgaacggcgcggcgggcttgtccgggttggccttgttgtaggccgcgagttcctcggtgatttcggccagccagtcttcgagctgcgccgcgggccgcgcattgagggccggcatcgaaccgaccacccccgccttgcattgggcgatcacaagcttcgggttgctgatgatgaaaagcggcgagccgatgatcggcagcggcaggttggcgagcacggggggcagcttggacatgtcgtctccgggataaggtttcggttttatataagaggaaggccgtatcgcccgtcaggtgggcgacacggcgggccgtgggtcagaacgcgtcgagcgccagtgccgtcacgctctcggcgccttcgacgatgctgtcgcggatgcccggcaccttgttgaggatgtgctcggcgtagaagcgcgccgtggccaccttggcctgcatgaaagcggtatcgacgctgcgggacgccaggtcttctgcaatgagcagcgagcgcgccagctgccagcccgccacgaggttgcccgccagcatcaggtagggcacgctgcccgcgaacaccgcattgggcgatgccttggtctggcccgcgacgaaatcgaccacgtcgacgaacgccaggcgcgcggccttcaggcgcttcagcacggccgccgctgcggcgctgtcgctcttcgcgagttcagcctcggtcttctcgatctgcaccgcaatggcctttgcggtctggccgccgtcgcgcgcggtcttgcggcccacgaggtcgttggcctggatggcggtggtgccttcgtagatcgtcaggatcttcgcgtcgcggtagtactgcgccgcgccggtctcttcgatgaagcccatgccgccgtgcacctgcacgccgagcgaggccacttcaaggctcatctcggtgctgtagcccttgaccagcggcaccatgaattcgtagaacgcctggttctgcttgcgcgcatccgcatcgggatggtggtgcgcggcgtcgtaggccgcagcggccacggccgccatggcgcggcagccctcggtgtaagcgcgcatcgtcatcagcatgcgcttgacatcggggtggtgaatgatgggggcgctggcgttgatggagccatcgaccggccggctctgcacgcggtccttcgcgtaggccacggcgtgctggtaggcgcgctcggcaatcgcgatgccctgcatgcccacggcatagcgggccgagttcatcatgatgaacatgtactccaggccgcggttctcctggcccacgatgtagccgacggcaccgccgtggtcgccgtactgcagcacggcggtgggcgaggccttgatgcccatcttgtgttcgatgctcacgcagtgcacgtcgttgcgttcccccagcgatccgtccttgccgacgaggaacttgggcaccacgaacaggctgatgcccttcacgccttcgggcgcgccggtcacgcgggccagcaccaggtgcacgatgttctcggccatgtcgtgctcaccgtaggtgatgaagatcttggtgccgaacaccttgtaggtgccgtcgggctgcggctcggcgcggctgcgcaccatggcaaggtcgctgccggcctgcggctcggtgaggttcatggtgccggtccactggccgctcaccagcttctccaggtacaccgccttgagttcgtcggagccggccgtgagcagcgcctcgatggcgccatcgctcagcagcgggcacagcgcgaagctcatgttggccgagttgagcatctcgccgcaggccgcgccgatggtcttgggcaggccctggccgccgaagtccgccggatgctgcagaccctgccagccgcccgacacgtactgcgcaaaggcctccttgaagcccggcgtggttgcgacctcgccgtccttgaaggacgacgggttgcggtcgcccgccacgttcagcggcgcgaccacgtcctggttgaagcgcgcgcattcctcgagcacggcctgcgcggtttcgaggcccgcgtcttcaaagccgggcagcttggcgatctcgccgatgttggccaggtgctcgatgtcgaacagcatgtccttgaggggggcggtgtaactcatctcatgtctccagatacagcggatacgaaaagggcatcgcgaacgatgccctctggctcagtgcagcgatgcgatcagagcgccttgacgagttccggcacggccgtgaacaggtcggccacgagaccgtagtcggccaccgagaagatcggcgcttcttcatccttgttgatcgccacgatcaccttggagtccttcatgccggccagatgctggatggcgcccgagatgccgcaggcgatgtacagctgcggcgccacgatcttgccggtctggcccacttgccagtcgttgggtgcgtagcccgcatccaccgcggcgcggctggcgcccaggcccgcgttgagcttgtccgccagcggcgtcatcacctcggtgaacttctcggcgctgcccagagcccggccgcccgagacgatgatcttggcggcggtgagttcggggcggtcgctcttggtgacttcgcggcccacgaagctggacttgccgctgtcggccacgccttcggcggtttcaacagctgcgctgccaccggtggcggctgcggcgtcgaagccggtggtgcgcacggtgatcaccttggtggcgtcggtgctctgcacggtggcgatggcgttgccggcgtagatcgggcgctcgaaggtgtcggggctcacaaccaaagtgatgtcggagatctgcgccacgtccagcttggcggccacgcgcggggcgacgttcttgccgttggcggtcgaggggaacaggatgtggctgtagttggccgcgatggccagcacctgggcggcgacgttctcggccaggttctcggccaggctcgggctgtcggccacgatgaccttggccacgcccacgatctgggcggcggccttgccggcttcggcggcattggcaccggcgacgagcacgtgcacgtcgccgccgcaggccagggctgcggtcacggtgttgagggtcgcgggcttgacggtcgcgtggtcgtgttcggcaataactagtgcggtcatgtcgttgtcttcctcagatcactttggcttcgttcttgagcttgtccaccagggtggcgacgtcgggcaccttgataccggcgccgcgcttgggcggctcgctgaccttgagggtcttcaggcggggcttgacgtccacgcccaggtcttcaggcttgaagacgtcgagcgtcttcttcttggccttcatgatgttgggcagggtgacgtagcgcggctcgttcaggcgcaggtcggtcgtgatgacggccggcaggctgagggagatggtctccaggccgccgtcgacttcgcgcgtcacggtggccttgccgtcagccacttcgaccttggaggcgaaggtggcttgcggcaggtcggccagcgcggcgagcatctggccagtctggttggcgtcgtcgtcgatggcctgcttgcccaggatgacgagctggggctgttccttgtcgaccagcgccttgagcagcttggccacggccaggggttgcagctcttcggtggtctcgaccaggatgccgcggtcggcgccaatggccatggcggtgcgcagggtttcctggcacttggcatcaccgcaggagacggcgatgacttcggtcacgacgcccttttctttcaggcgaaccgcttcttccacggcgatctcgtcgaacgggttcatgctcatcttgacgttggcaatgtccaccccggtgccgtcgctcttcacgcgcaccttgacgttgtaatcgacgacccgtttgacaggcactagaaccttcattgacttgactccattgggattgcaaaaagggggcttcgagggcaaccggtcattttagagtccgaccttcgccgcctctgcgttcgtatcggtttgtaccgtggggcaacaaaaaaagaacggtcgtgctttttcgagattatacggcagcgtcgcgcggtccggaaacgcccggtggcagagactccacgcgcagcacgcgctggggatacggaatgtccacgcccgcgctgcgcaggccttcgagaatggcgatgttgatggccgagcgcacgttgtccttgcccttgtcggggtcagcaacccagaagttcagaacgaactcgagtccgtcgggggcaaagttggcgagaaaggtcaccggctcagggtccgtcatcactcgctcttgcgacttggcggcgctgcaaagaatggactggacctgcgccacgtcgctgtcgtagcccaccacgacgctggtcgtgatgttgaacttgcggtccgccatcgagaggttctcgacgcggctggtgataagcgattcgttcggcacgatggcctcgcggccgttgcccgcgcggatgagcgtgtagcgggtcttgatgtcggtgatgcggccttcgaaggtgtcgaccttgacgttgtcgccaatgcggatggagcgttcgagcaggatgacgaagccgctcacgtagttggccgccagcttctgcagcccgaaacccaggcccacgccaagcgcgccgcccagcaccgagagcgccgtgaggtcgacccccaccgccgacagcgcgaacagcagcccgaccagcagcaggatggcgcgcaccgcattcgaggcgaccttgcgcatcgaaagatcggacacggcctcgaacaggatgcgcttctcgatggtggcggcaatccacagcgcgatcaccagcaccagcccggccgacagcgcgccctggacgatggtttgcaggctgacgcgcgtcttgccgaacgacagggtgatgttgtcgagttcggccagcaccggcggcagcagcccgacgatccagagaatggcggcaatccaggccagccacgagatcgtgcgctccagcagccgcaccaggttggaggtgggaaacaccgccctcatcacgcgcgcgaacaggcggatgaccaagagcgacaggaaaaccgacaccgcgatgcgcagcaccagcaccggctggaagccgttcaccgcgcggcgggcgagctcggtgaaaaccagcgccagcagcggaaacagcacgccgtcgaaggtgcgctcgccgaaccagatcgaatccttgggctggtcgcgcccgaaccagcggcttgccacccaggccagggccacgcaagccaccagcgcggccaactcgatgcccaggccgcgcgcgtcgacctggcccaggcgttgtgtgaaatcgttgaagttcatctcttgggaaaacatggcgccgtcatggcgccgtatttgcgcctgcggctctacagatcggcaaggacgcggatgtgcgcttccacgctgcgggccagcgcatcgaggttgtaaccgccctcgagcatcgagacgatgcggccgcgcgcatggcgcctcgcaacgtcctggatgcggctggtgatccaggcaaagtcgttctcggtgaggccgagctggcccaggtcgtcctcgcgatgggcgtcgaagccggcactcacgaagatcatctccggcgcgaattcctcgagccggggcatccagctggcctcgatcagctcgcgcacgtccatgccccgggtataggccgggatcggcaggttcagcatgttcgaagccgggcgctcggtgccgctgtacgggtagaacggatgctggaagaaacccaccatcagcacgcgcggatcgttcgacaggatgttctcggtgccgttgccgtggtgcacgtcgaaatcgacaatggccacgcgctccaggccgtgcacctcgagcgcatgccgcgccgcgatggccacgttgttgagaaagcaaaagcccatggcctgctcgcggcaggcgtggtgcccgggcgggcgcaccgaacagaacgcgttctcgatctcgcccgccacgaccgcgtcggtcgcggcaatggcggcgccggcggcgcggcgcgcggccagcagtgtgaagcgagtcaggatggtgtcgggatcgagctgcgcatgggtggggccgcccgccggctcgtcggccaccaggcgctggtgaagctcttcgagatattcgaggtgcgcctcgctgtgcgcccgcgtgatctgcgacagtgtggccagcggcacgtcccggtgttcgagggcatcgcccacgccggtgagcagcagcctgtcttcgatggcatcgagccgttcgggacattcggggtggccccggcccatgtcgtgcttccagcagtcgcgatgtgtgaagtacccggtcttgcccatgtctttgccgtgtctctgtcgtatctagacctcacacagcatggggccgggcggtcttacggtatcgtttgcatatggatacaaatatggacgtcgctgcgaagcttgccactttgctgagtcagcttaacacggtgatcgtaggcaaggagccccaggtgcgcgactgcgtggcatgcctgttggcgggcgggcacctcttgatcgaggatgtgccgggggtcggcaagaccaccctcgcccatgcgctgtcgcacaccttcggcctccagttctcgcgcgtgcagttcacggccgacctgatgccgggcgacctgtcgggcgtggccatctacgaccggggccagcaggccttcgtgttccaccccggcccgatcttcgcgcaggtgctgctggcggacgaaatcaatcgcgccagccccaagacgcagagcgcgctgctcgaggcgatggaagagaagcaggtcaccatcgagggtgaaacgcggccgctgcccacgccgttcttcgtgattgccacccagaacccgcaggaccagctcggcacctttgccctgccggagtcgcagctcgaccgcttcctcatgcgcatttcgctcggctatcccgaccgcgccgcggagcgcgagttgctcgcgggcgccgaccgccgcgaaatgctggccaccctgcccgccatgctgaccgccggcgagctgacggcgctgcagcagcgcgtgcagcaggtgcatgccgccgatccgctgctgaactacgtgcaggacctgatcgccgccacgcgttccggccggtggtttttgcagggcctctcgccgcgggccggcattgccgtgctgcgcgccgccaaggcgcaggcgctgctggccaaccgcagctatgtcgcgcccgacgacgtgcagtcgatattgccgcagaccatcgcgcaccgcctcaccccggtgggcgatgcgggccggggcgccgtggagcaggtgcgcgcgatgatcgcggacgtgccgctgccataaagatgaatccgcccgtgaaccagacgcattgccaccgatgatcgcgtcgctacgctcgcgcatcgacggctggttcctgtcgcgccggccgccttcggacacgctggagctcacgcagcgcaatgtctacatcgtgcccacgcgcgccggctggctgctgggcgccacgctgctggtgctcttgatcgcgtcgatcaactaccagctcaacctcggctatctgctgaccttcctgctcgcgggcagcgtggccgtgggcatgcatgtgtgccacgccacgctgcgcggcctggccatgcacctgacgccgcccgagccgcattacgcgggcgccgccgccgtctttcgcgtggtgctgcacaacacgcggcgcagcgtgcgctacggcatcggcatggcggtgcgcggcagcggccaatgggcctggaccgacgtgccggccgaaggcagcgccacggtcgagatcgccttccagcccgaaaggcgcggcctccacccggtgccgcccctgacggccgaaacccgttttccgctcggaaccttccgtgtctggacggtgtggcggcccgccgcgcagatgctggtctacccaacgcccgaggcgcatccgccgccgctgccgcccggtgagcccctgtcgggtccggcggccacgtccgctgccctgcgcgcccaggccgccggggaatacgacggcctgcgggcctaccggcgcggcgacccgctcaagctcgtggtttggaaaaaggcggcccgcgcgcaagccaccgggtcggaagacctggtgagccgcgacacgcagcaagcccagcgcgaagagctgtggctcgacgcgcaggcggccaacgtcgccgacaccgaagcacgtctttcaaggctttgcgcatgggtgctgatggcagaccggctgggcgtggactacggcgttcgcgtggccggacgggtggtgcagccgtcgcagggcgaggcgcaccgcagagcctgcctggaagcgctggccctatgttgaccgcccgcttcttccgcccggagcgccgcgcatgaacaagttcatgcgcgaaatctcggcgctgccacgggacgccagggacaccctgttcctgctgatggtcatcgcactcatcgtgcttccacaggccgagaacctgccctggtggtgcacggccatcaccgcgatgatcctggtgtaccgcggcacgctggccatcgaagcccgcccgctgccgggcaagtgggcgcgcgtgggcctgctggcgctgacgctggccgccacctacgccacgcaccgcaccctgctgggccgcgacgccggcgtcacgctggtcgtgatcctgctggccctcaaaacgctggagctgcgcgcgcgcagggacgccttcgtgctgttcttcctgggcttcttcgcgatgctcacgaacttcttctactcgcagtcgctgatgaccgcggtcaccatgctgcttgcgctgctgggcctgctcacggctttggtcaatgcgcacatgccggtgggcaagccgccgctgaagctggcggcgcgcaccgccagctggatggccttgctgggcgcgccgatcatgctggcgctgttcctgctgtttccgcgtttcgcgccgctgtggggcacgcccgcggacgccatggcaggccgcaccggcttgtcgaacaccatgcgcgtgggcaccatcgccgaactggcgctggacgaccgcattgcggcgcgcatcaagttcgagaacgaccgcgtgccgccgcagagccagctttatttccgcggcccggtgctcacgcagttcgacgggcgcgagtggacggcgctgccgagctggtcgcgcggcgggccggcttcgggcaacctgcgcaccagcggccagccggtacgctacgagatcacgctcgagcccagccaccggccctggctgctcacgctcgatgcggcgcaaagcccgcccgaagtacccggcttcgaagtgctgggcacgcccgacctgcagtggctcgcgaaccgcccgatctccgacctggtgcgctaccgcgccgaaagccatacgcagttcgcgagtggcccgacgcggcagacggccgcgctgcgcccatacctggcgctgccgcccggatcgaacccgcgcaccgccgcgctggccactgaaatgcgcgcccagcccgccatggccaacgccgacacgcaggccttcgttcgcgcggcgctgcagcggctgcgcaccggcggctacacctacacgctggagccgggcttttatggtaacgacacggccgacgagttctggttcgaccgcaaggaaggcttctgcgagcacatcgcctcggccttcgtggtgctgatgcgcgggctgggcgttccggcgcgcatcgtgaccggctaccagggcggtgaactcaacagcgtcgacaacttctgggtgctgcgccagagcgatgcgcatgcctgggccgaggtctggcaggaaagcgtcggctggatgcgcgtcgacccgaccggcgcggtgtcgccggggcgcgtcggccagcagcagcggctcgtgccccagccaggcctctttgccggtgccatcggcgcgatgagcccgacactggcgcagaacgtgcgcgccgcctgggaagccgtgaacaatggctggaaccagtgggtactcaactacacccagagccgccagctcaacctgctgaagagcatgggcttcgagacgccaagcctcgaagacctggcctacgtgctgctctacctgctggtgggcgcaagcctggccggcgtgggatgggccttgtgggaacgcagccagcatgacccatggctgcggctgctggcccaggcgcgcgcgcgcctcgccaaggcaggcctccaggtgccagagacggcgccgccgcgccagatggccgcgcaggctgaagctcgcttcggccccgctgcccaggcggtgcgcgactggctgctgaagctcgaagcccagcgctacgccgaggcctcgcccaattcgctgggggcactgcgcaccgagttccgccggctgaactggcccgtgccgaaccccaagcgctgaaaccgcatgtgtcccgcgaaggcgggctcgcgggcggacggcacaatcgcgcccatgcgattttttctacctgcgccgccgcgcgccgctgccgtcatcctgctcgccgcttgctgcgcgtggtccctgggtgcacaagcccagaaaaccggcaacggccgcgcggtgaaaaccgtggccggcagcacgccctacgccacccgcgacgacgccatgcgctttgccgacgacgtggccgaacgacgcggcctcgaccgcgaatgggtgcgcgccaccatcggcagcgcccgcttcctgccgaacgtgccgcgcctgatgttgcccgggcctgtcggctcggtgaagaactggcaggcctatcgcagccgcttcatcgacgcgacgcgcatcgccgccggcgtgcgcttctggcgcgccaatgccgagacgctcgcgcgggctgaagaggtgtacggcgtaccgccggaaatcatcgtcggcatcatcggcgtcgagaccatctacggccgcaacatgggcaacttccgggtgatcgatgcgctgtccacgctggcgttcgactttccgcaggcccacccgcgcgcggccgagcgcgaagctttcttccgcggcgagctggagagttttctcagcaccaagagccgcacctccgacgatcccctgcggcccgtgggcagctacgcaggcgccatgggcatgccgcagttcatgccgagcagcatcgccaagtacgcggtcgatttcgacggcgacagccgcatcgacctggtcgacaaccccgccgacgtgatcggctcggtcgccaattacttcaaggcctttggctggacacccggtatgcccgccgtctaccccgtgcatttcgaagaggcccgactcaagaaggcgatgcttctggcacccgacatcctgccgagcttcagtgccgacagcttcgtggcggctggcgcggtgcctgaaggcgagggcctgctgcacaagggcctgctcgcgctgatcgagctgcagaacggtgccgatgcgccaccgacctatgtggcgggcacgcgcaacttctacgtgatcacgcgctacaactggagcagctactacgcgatgtcggtgctcgaccttggccaggaggtcaaggccgcgatggagcaatgacgccgtgacacccgaggtgctgctggccaactggaacgccgcgtggcgcgcgctgggcgtggcctctgctgacgaggcgctgtgcatcgagctccagcgccgctacagcgagccgcagcgccactatcacaccctgcagcatctgggcgaatgcctgacgtggttcgagcgcgagcaagcgctggctgagcgcccgggcgaagtcgcgcttgcgctctggtttcacgacgcgatctacgacgtgcatgcccacgacaacgaggcacgcagtgccgaatgggcgcgtagtgccctgctcgcgtccggcgtgcaagccgagtcgaccgaacgtgtgcacgccctggtgatggccacgcggcacgatgccgtgcctgaaggccgcgatgccgagttgctgatcgacatcgacctgtcgatcctcggtgcggagcgggagcgcttcgacgaatatgaacgtcaggtgcacgccgaatacgccttcgtgcccgacgcggtgcgcttgccgcgccgccgcgccatcctgcagcgcttcctggcacgggaagcgatctacgccacgccccggatgcatgcgctgctggaggcacgcgctcgcgccaacctggcgcggtcgatcgcggcaacagcctgatcctgcaaagcgcgggcgagactgcggtgcttcaggccggcaccagccgccaccattcggagcgcggcatttcgccattgcgctcctcttccaccacgcccagcagcaagccggcgctccccgcgccgatccgcgaaagctgcagcagctgctgcgggtcgcggcacagcgcaaagcccgcgtcgccctgccagtcgagacagcggccgacctcagccagcatcaatgcgggctggccctgcatgaaggtgaacggcatcagcgcgcctgcgtcgagctgcgccaagcccgcatgcgtcgcgccccaggcaccgcgcatgctcgacacgcgcaggcgggcgcccgtgggcagcgcatcctcgcccgcggcatcgaggcagcagcgcgcgccgtacatcgcgagttcggtccagaggccgacgcgccgcggccgacggccaagccgatgcgccagctggtcgcgccaatccgcaggcagcggatcggcactgaagtacgcaacggtgcgccacgcgacggaggaaccggcgttcatgcggtgcaatcctccagcaccagcgaggcgtgtccaccgccgaatccgaccacgttgagcaggatgttgcgcagcctggcgggcgcctgtgaactcaatgcgatgccgagttcgccgtcgaccgcgtagccggtcgaaggccatgccccggcttcgatacaggcgacgagcagcgccagttcggcggcccccgatgcacccagcgtatggccaagcagcgacttgagcgacaccagcggcggcagcgtatcgaagacctgcttcaacgcctgcgcctcgatcgcatcgttgaccgggctgcccgcggcctgcaccttgatcaggtcgatatcccgcggactcagcccactctgcgacagggccccatggcacatggcaatcaacgcgctggcttcggtgcccgaggggttgcggccatcgaccacgttggacccaccggcaatgcgccagcgcgccgcgcgcgagccgaggcgcaatgcggccaccgcctcgccgagcaccaacccgttgcggccggcgccgaaaggccgcgcgccatcaggcgagagcagttgcatggcgccgaagccggccacggtgaagcgattgccgagttcggccccgatgaccagggcctcgtcggcttcgccgctgcgaatgaagtcgcaggccgccagcacggcgttgagcgccgaggtgcaggccgtggagatggtgaaaaccggcccctgccagtcgagcgcgccggccacgaggccggcaaagtcctgcaggtcgccgcccaggcggaggtcttgcacctcgtgctccatgttgccaatgtccagcgaagacgatgccacgaagagcgggccggaacgtccgcctgcgccctcgcctgcctgcgccgcgacgctgcgcacggtacgcgccaagcgctcggcccagctgccatcctgcgtgggcagcatgaacacaggccagcggacgccttcggagacggcgaccggacggggctgcacaccgccgcgcgcaagtgctgtcacggaggacgcgagatcgttgcccagtgcacaggccaggcccatgccggcaacatacacgccctcgatgctcattgaatgaccttcgtgcttcgcactgcggtgcgagcccccttcggagcggccgggcggcggctcatgccttgcccgcttgcaccaggtggtcggccaggtgggcaatggacgtgagcgcgcgccgcgtttccttgctgtcgggcatgcgcagtccaaagcgctgatggatcgtcatcgacacctgcagggcgtcgagcgagtcgaggtcgagccgggcttcgggcccgaacagcggctcgtcgtcgccaaggccacccggtggcgcgtctttttcgacggcctcgagcaccatggccttcaggctggcaatgaattcagcggatacagagtcggtcacgatgcgggcctgcgaaacagaaagacggcaagcaggaacatggcggccgcgaacaccacgagccggccgacctgcggcaaggtgtcggccacgctgccgccgcgcaacagcacggtgagcagtgcctccaacccccagttcatcggggagatttcgaccagccgctgcatgaagcccggcatgacgaacttcggcaccatgatgccgcccgcggccgccatcagcacgttgaccatcggcccgatggtcgcggcctgcgcatggctgcgcaccaggcatgccagggccagcgacaggctgaccgcggccaggctcaccgcggccagcgccagcaccagcgcgtcccaatggatgcccgcgagggagagcgcatcgccgccgatgagcggcatcagccagatgccggccgccagcatcagcacggcctgcagcgcgttgacgccgaggtaaggcagcgctttcgacatcagtagcatgaagcgcgacacgcccaggctgcgcaggcggcccagcgcgcccgagctgcgctcctgcacgaacaggctggagagcgaggccaccacgaagaacatgccgaacaccagccacgccggcacgttctgctgcaccgaggtgggccgcggcccggcggtggaataacgctcggcatttaccagcgcctggatcgaggcgcccggcggcgggccggaagtgccgggcaccgccagcgcgaggcgcgccttcagttcgccggacgcgccgaccagttcggcgcgcagggcgttgaacaggttggcgtcgatgcccggctcggtcagcagacggatgtgggccttggtcgacagcgcggccgactccagttccgccgagaggccgggctccaggacgatgacgtacttgagcgcgccgctgcgcaaccgtgcctgccagtcggcatcgagcgcttggggtgccccatggccgcgctgccagatctgctgcagccattgcgcaggggtctcgttgtcgcgcatgtccaccgcatagctcagttcggccagcggcgggcgatagatgtctttcagcgtgagcgacatcagcacgatgaagatcatcggcatgagaaacagcgccgcgagcccgtgcatgtcgcgcacgagtgcgagcagttccttcttgatgagcgcaagcagcatggcgttcagtcgcgcagggaacgatgggtgagcgccatgaaaagctgctcgaggtcgtggcggccgaactcggcgtggcgcacctcgatgccttcggcttccagggcctgcaacacgggaccggggccagtgccctcgttgaggtgaacgcgccaatgcacgccgcccggctccacggtgccgaagcgcgagagcttctgttcgtccagcccgtcggccgccagcgtgagcagcatcgcgctcttcgacagcagctcttcaagcgagccttcgcgcagcacgcggccgtggtcgaggatggcgacgcggtcggcgatggcttcgatctcttccatgtagtgcgaggcgtagatcacggccgcgccctgctccgccaagctcttgatggcgtccagaatgaaggcgcgcgattgcggatcgacgcccaccgtgggttcgtcgaacagcatcagctcgggttcgggcaaaagagcaatggccaggttgagccggcgtttcagcccgcccgagaggcgctcggcgcgcacacttgcaaactgctcgagctgcgaaaatcgggtgcaggcttcgatacgcgccttcttgcgcgcaccggtgagaccgcccgccgccgcgaagcatgcaaggttctcggtcaccgtgagcatgggatagaaggcctggtcctgcggcgccaccgcgatgcgcgtgggtgccttggcgcgaacctgctggagcgcttggccgtcgatgaggatctcgcccgactgcacggccagcgcgcccgagaggtgagagatcagcgtggtcttgccggcgccgttggggcccagcaaacccatgacgcaacctctcggtaccgcaagcgacacatcttccagcgcaggccttccggcatgcggatagcggtagccgaggttcttcagttcgagcatcggcgtgttgcttgttcggagtggtggttgttcgagccgaacaacgacagcgccctgtgtgcgcagggcgccgggtgctccccgcagcgaaataaaggaggagccgaaggcgggggacattcgcggaggggagtacccggtggcctgtgcacgcgccctgaacagaagcgccctgaacagaaacgtcctgaaccacgcaccatacgacctgcgcaccgaatcgagaaacgatgctccatctcaggcaacagcagccttcaggtcgcgaaagaacgtttcctcctgctgcgcctgctcacgcagacgctcggccagcgccgccggatcgaccggctcgcgccccttcaccatgcgcgctgccttgagcgcgaaggcgcgccagccgtcgccgatggcgatgagccgctcggacatctgctgcagctgcggtttgtcgagcaactgcgccgcctcctgcaggaagcccgcatagatgaaacggaaacccgccccacccgtgccgatttcttcctgcatgcgcaccacgtggccgatgaaatcgacgctgcgtgagtcggttggcgacagcttctgcatgcgcttggccagcgtgcgcatgccgcgcacaccgacgatgggaatgggcgcgagcatgtttcgcacggtcttgcggatggcctttgtcaccgatgccgcgtcgaccgtcttgcgctcgatcgactgcgggtaatacatgaggcccttgggcgcaagcacgcccttggcgaagcgcgcacgcgacaggtcggcgctggcgcagcgcacaggctcttcgaacaccggatcgctgatcaggtagtcgtcgccgtccttgccgtagaccagcaggttgtgcgcattgaagtgaaagcgcatgttgggcggaaagtaaggcagccagtagaccgaggtctgcagccccacgatctgcccgctggccagcagggcgtcgaggcgctgggcacccgcctcggggctgcgaaaggtctcgaagcggaagcgcgcggccattggtgccaagaggcccttgatgatggccttgggcggcatgcggtacgagatgagcggcaggcccgagagcttgatgaacggcaggtaggcgaacgacaacgcagacgacaggccgagcgccatgctctcggtcatgggtgcaccatggtggcgcatcaggttcgagatgacgccgctttcgcaatgcgccgcttgttgatgttcgaagttcacgacggcaggccttgcaaggtggaaacgggcaggcccagcgcctccgaatagcgcgccatgtgcttttgcgacagcgctgcgaagtgtttgggcttcaggtggcgccgtacgcgccattgccagaagccgctggtctgcgagagcagcgccacgtccatgcggcgttcgtacatccagtattcgagcggcgacgcgagcccctgggccacgcgctccttggccgcctgcgcctgcacgacgagcacgtcgaccgcatggctggtgacgatttcttcagcctcccagccgcgcgaggtggtggtgacgacacggccctgcgcgtcgcgcgcgtacatgagcttggcatggccgccgagggtggcattgccttcttgcggaacggcgtcgacgtccatggctacacagcctccatatagatgaagccgctcgaaaaacggccgctttcgggcacgaacatcaagagcttgtggccgggcttgatgcgcccggaacggaacagctcgtcgagcatgatgtaaggcgatgccgccccggtattgcccttgcgcgccaggttgctgaaccagcgctcgcgcgggattgcgaagtccatggcttcgaggcagcgggcaacgggttcggcgaaatagttcgatgacaggtgcggcaggaaccagtcgatgtcggccgccttcaggccgcgccgctcgacgatggctgcgagcggctcgcccagcgtggcgcgcacgatgttctcgttgagcaggcgcacgtcctgcttgatcgcgaaggtcgagtcgcggtgccaatcctgcggctgcgtgcgcgcccagccgtcgaggccgccctcggcgttccggtcggcgcccgagtacatgcacaccggcagctcgtgcgctgccgacgacaggtcgatccattcgatgcgcagcgacagcggcccgcgcggcacgcgctccagcagcacggcgccggcgccgtcggacagcatccagcgcaggaagtctttctcgaacgcgatctcgggccgcttctcgagggcttcgagctggtgttcgagttcggcctcgaagcgcgaaccgcgcatcaccggtgacaccagttccgagccggtggcaacggcgcgttgcgcatcgcccgcgcgcaccgagagccaggcatgcttgagcgcggtggtgcctgcaaggcagatgccggcgcaggccaccacctcgagccgcggccagccgagctcgccatgcaccatcacggcgtggttgggcagcagttggtcgggcagcgaggtgccggtaacgaggcagtcgacgcggccgatgtcttcggggtcgccgagagcgcggacggccgaggccgtgagctgtgcgttggtcatggcctgcaggccggtggaccggtcgatcgcatagtggcgcgattcgatgccgttgctgcgaaggatcaggcgccgcgctcgcgacgccttgccgccgatgcgacccagtacttcttcgatgtcttcgttgccgaccggcgaaaaaggcaggaaagcggcggtacgggtcaggaaaacatcagtcgtcatagaggtgggagcggtctgtggccgagcccgaggggcgctcgaagtgagccgtcattttagtcagccaccccttgaacaaaggccgcagcagcgcctgcagcgtcaagctcacgggcacgaccgtgacaatcagcacaagaaggaagaccacatagagcagcagcaacggcttgcgttgccatgcgccgggccgccccgccgccacgatcagcttgccccagaggaagaagctccgcgtgccggctttttcgctgatcaagagccgggcatcggcccgcactgcgcccaggcccgcgagcagcggctgcgatccgcgctcgagatcgttgtgcagcgcctcgcgcagcgcgcggccgaagcgacccgcgccctggacctgttcggcgctgaggccggcgtcgggcatgccccagaacccgcgcttgcggccccagatgagccaggccggcgtggtgaagaaagtcgccagcgtcgggccggggtcggtcagcaccacgttgtcgatcagccgcgcgcctaccgcgtcgagcaggcccttgagcttttcgtgcgccagcagccacatgttgcggcaggcgatgacggtgaccacgggcttgccccggagcaggcggcttgccagcggatgcttgagaaaggcggtaatgggctgcgacggcgccaggaaccagacctggtaaggcaggatgacgagatcgaagtcttcgtccccggtcagcgaaagcggcgccagcggcgccggcttcaggtgggccgactccggaaaggcatcgaagaaggtcaggaacggccagggaaacggaaaatccgcttgcgggcgcagcgtttcggcgtgcacggaaatctgcggatcggccctgagcggcgcaacgatctggtcggcgacgctgccgagctggcccgtctgcgaatagtgaatcaccaggacacgtttggggcgcgcggcggggctggaaatgcttgaggtcacttgttggggctgagcgggggccgtcgaatgtaagccaagcgtcgcactggcgcatctgccattggtcatgccgtcgcgccgaccccacggatagagacgaaaaaagggccgcacccttcggcgcggccctcgtcggctgttctgcaagaaacgcaggcggtcagcgcgccttgccttccttccaggctgccagcatcttgctgtattcgatggtctcgcccttgggcttttcgttggccagcttcttccacggcgcgttcttgtcgctcagccacttgttgggatcgcccttggcgttgagcttgggtgcgcaatgggccatgccggcgcgctcgaggcgggccatcacgttgtccatctcgtcggccaggttgtccatcgccttctgcggggtcttctcgcccgtcacggcctcggccacgttcttccaccagagctgcgcgagcttcggatagtcgggcacgttggtgccggtgggcgtccatgccacgcgggccgggctgcggtagaactcgaccaggccgccgagcttgggcgccatgtcggtcattgccttcgactggatatccgattcgcggatcggcgtcaggcccaccatggtcttcttgagcgagacgctcttggacgtgacgaactgcgcgtagagccaggcggcggccgtcttgttggcgtcatggccgttgaagaaggaccacgaacccacgtcctggtagccgttctgcatgccctgcttccagtaggggccgttcgggccgggcgccatgcgccacttgggcgtgccgtcctcgttcaccacgggcaggcccttcttggtcatgtcggccgtgaaggcggtgtaccagaagatctgctgggcaatctggccctgcgccggcaccgggccggcttcgccgaaggtcatgcccatggcttccttgggcgcgtacttcttcatccagtcgatgtacttggtgagcgcgtaaacggcggccggcgagttggtcgcaccgccgcgcgacaccgcggcgcccacgggcgtgcacttgtcgtcgcccacgcggatgccccattcgtcgatcggcatgccgttcgggttgccgatgtcggcggtgccggccatcgacagccatgcgtcggtgaagcgccagcccagcgacgggtccttcttgccgtagtccatgtggccatagatcggcttgccgtcgatggtcttcacgtcgacgctgaagaattcggcgatgtcttcgtaggcgctccagttgagcggcacgcccaggtcgtagccgtacttggccttgaacttgtccttcaggtccttgcggtcgaacaggtcggcgcggaaccagtacaggttggcaaactgctggtcgggcagctggtagagcttgccgtccggtgccgtggtgaacttggtgccgatgaagtccttgagatcgagtcccggattggtgaactcttttcctgcgccggccatgtagtcggtcaggttcatcatcttgccgtagcggtagtgcgtaccgatcaggtcggagtcggaaatccagccgtcgtagatcgacttgcccgactgcatcgaggtctgcagcttctcgaccacgtcgccttcctggatcaggtcgtgcttcaccttgatgccggtgatctcctcgaaagccttggccagcgtcttcgattcgtattcatgcgtggtgatggtctcggacaccaccgagatctccttcacgccctttgcctgcagcttcttggccgcatcgatgaaccacttcatctcggcggtctgctggtccttgctgagggtcgacggctggaactcgctgtcgatccatttcttggcctcgggctctgcggcccatgcaccgtgcgcggcgaacatcgccgctgccattgccaatgccgtgtagcgcatcttcatgaatgtgtctcctcggttgaaagcttccccggttttttcgatcgcggctccggggaggcggagagccggtcgcgtctgaaaacaaattcttgggcctagcccttgcgcatcaccagcgccaggagaaacatcgacagcacgaagctgatccagatcgaaggctcggcctgcaggcccagccattcctggaatttgccggccaggccgatgaagaccaggttgaagtaggccgccgaaagcaggccgatgaaaagccgatcgcctcgcgtcgtggcaatgggcagccagccgcgccgcatcgtggtgggcgacttgaactcccacaccgtcatgccaaccagcatgagtgcgatgcaggtgaagaaaacggccacgggggtggtccagaccatccaatcgaacatttctcagctccttttcttttcttgctccttccccctctgggggaaggttgggatgggggcatcggcgctcgatggaaacgccgcttgccctcacccctgccctctcccagagggagaaggagtcaatacctaaacccgtcccatcgcaaagccctttgcgatgtagtgccgcacgaaccagatcacgatcgcgcccggcacgatggtgagcacacccgccgcggccagcgtggcccagtccatgcccgaggcgctcaccgtgcgcgtcatggtcgccacgatgggcttcgcgttcacgctggtcagcgtacgggccagcagcagctcgacccagctgaacatgaagcagaagaacgccgccacgcccacgccggccttgatgagcggcaggaagatccggacgaagaagcgcgggaacgagtagccgtcgatgtacgccgtctcgtcgatctcgcgcggaatgccgctcatgaagccttcgagaatccacaccgccagcggcacgttgaacaaaaggtgcgccagcgccacgcccaggtgagtgtccatcaggcccacggtgctgtacagctggaagaacggcagcaaaaacaccgcgggcggcgtcatgcggttggtcaacagccagaagaacacgtgcttgtcgcccaggaacgaatagcgcgagaacgcataggccgccggcagcgccacggtgagcgagatcaccgtgttgatcgccacgtagatcaggctgttgatgtagcccgagtaccacgactcgtcggtgaagatgcgcgcgtagttggcccaggtgagctcgtgcgggaagaacgagaagctcgagacgatttcctcgttcgtcttgaagctcatgttgatcatccagtagatgggcaacagcgcgaacaggatgtacagcatcaggaagatgctgcgcttgcggaatcgcttttcagacatgttgacccccttggcgctgcgcgccgtccccccgagggggagcatccgccttgaggcggctcagcgacggattcattgttctttctccacttcttgcgtgccgacccgctgcatccagttgtagagcacgaagcagaacaacaaaatgatgaggaagtagatcagcgagaaagctgccgccggccccaggtcgaactggcccacggccttctgcgtgaggtactggctcaggaaggtggtggcattgcccggccccccgcccgtcagcacgaagggctcggtgtagatcatgaagctgtccatgaagcgcagcagcaccgcaatcatgagcacgccgcgcatcttgggcaactggatgtagcggaacaccgcgaacttgctggccccatcgatgcgcgccgcctggtagtaggcatcgggaatcgagcgcagcccggcaaagcacaagagcgccaccagcggcgtccagtgccacacgtccatcaccagcaccgtgagccaggcgtccgccgcgctgccggtgtagttgtagtcgacgcccaacttctgcagcgcgtggcccaggaggccgatgtcggcacggccatagatctgccagatggtgccgaccacgttccacggaatgagcagcgacagcgccaccaccaccagcaccgcggaagacttccagcccttggccggcatcgacaaggcaaggcagatgcccagtggaatctcgaccagcaacaccgagagcgagaagcccagctggcgccacagcgcctggtgcagttcgtcgtcgcgcatcaccgaggcgaaccattcagtgccgacgaacacgcgccggtcgggcgagatgatgtcctgcaccgagtaattgaccaccgtcatcagtggcacgatggccgagaaggccacgcagatcagcaccggcagcacgagccaccaggccttttgattgatgggcttgttggttgcgttcatggtgttgctccttccccctttggggctgagggctgcggctccagttccgcctgcgcggaactggacagcccgaagagcggcagcctctggctgcctgcaccgaggttgggatgggggcgggcagagcgcgcaatggatgcgccgcttgcccccacccctgccctcccccgggaggggagggagaaagacgaaggcatcaggcccagtttgatcggggtgttcatgccaccagttcctcgtccttgtaatagcaagtgtgggtgtcgagcacccgcaaccacaccgtgtcgcccaccgccggcggctggtcttccgagtgcagccgcaccttgatcacactgccatcgacctgcgcgctcagcatggcgtgagtgccgacgtcctgcacctgcttcaccacggcgggcacggcaccggcagcgcccgcgttagaaaggcgcaggtactccggccggatcccgatcttgagcgcgccctgcggcagctcgcgcgtgggtacgagcggcgtccccgcgacctcgagcgcgccgttcgcgttcttcgcagaaagaaagttcatgcccggcgagccgatgaagtggccgacgaaggtatgggccggacgctcgaacagcgcctcggcgctgcccacctgcacagccttgccgcgcgtcatcaccaccacttcttcggcgaaggtgagcgcctcgacctggtcgtgcgtgacatagatcagcgtgagcttgagctcgcggtgaatctgcttgagcttgcggcgaagctgccatttcaggtgcgggtcgatcaccgtcagcggctcgtcgaacagcaccgccgacacgtcgttgcgcaccagcccgcggccgagcgagatcttctgcttggcatcggccgccaggcccgccgcgcgctggttgagctggccgctcatgtcgagcatctcggcgatctcgcccacgcgcttcttgatctggtcctcaggcaccttgcggttgcgcaaggggaacgcgaggttctcggccacggtcatggtgtcgtagatcaccggaaactggaacacctgcgcgatgttgcgttcctgcggcgtggcgcgcgtcatgtcgcggccgtcgaacgtcaccgtgccctgcgaaggcacgagcaagcccgagatgatgttgagcatggtggtcttgccgcagcccgaggggccgagcaaggcgtaggcgccgccgtcgcgaaagctcatcttgagcggcagcagcgcatagtcgctgtcctgcgtcgggttgggtcggtaggcgtgggccaggtcgagatcgatgcgtgccatagcgaggctcctagtttcctttgcgccatgccggcgcgagcgccagcttttcgccggcatcgaacacataggcttgcgacgcgctgaaatacagcgtgatcggcgtgcccaattcgaagcggtgcaccccggtgagctgcgccaccagttcgccgaccgccgtgtcgacgtgcacaaaggtgtcggagcccgagatttcggccagctccaccttgcctggcaaggcgatgtcgccctcccccgccccgacgttcaatgcgcttgcgcgcaggccgaccgtcaccgcgcccgagacgttctccggcacggccagcgcgagcttggggccgccggccaattgcacatatccagcggttgcggtaccaggcaaaaggttcatcggtggatcgctgaaggcgcgggccacgcgcagcgactgcggcgcatggaacacctcggctgtcggcccgtactgcagcagttcgcccgcatccatcacggccgtgtagccacccagcagcagcgcctcgccgggctcggtggtggcgtagatcaccgtcgaatcgccggtggcgaacagttgcgtgagttcttcgcgcaggccttcccgcagcttgtagtcgaggttcaccagcggctcgtcgagcagcatcagcggcgcgttcttggccagcgcgcgcgccagtgccacgcgctgctgctgcccgcccgacagctcggccggcaggcggtcgaggaacatgccgatgtgcagcttgtcggccagcgccttcacgcgcgcctcgatgttcttctcgccgcgcagcttgagcggcgaggcgatgttgtcggccaccttgagcgacggatagttgatgaactgctggtacaccatggccacgttgcgctcgcgcaccggcatgccggtcacgtccttgccgtcgaccagcaccttgcccgtgctgggcgtgtccagccccgccatcaggcgcatcaggctggtcttgccggcctgggtggcgcccagcagcacggtgaccgcaccgcttctcggcgcgatgctctgttcgtagagccaggtttgcgcgccgaccttcttggtgacgcgctccagagtcaattgcatcagcgcttcccgttgatcatgtagaggttgttggttgcgcgcgcctgcagccagtcggccacctgctggcgctcttcggccgtgtagcgcagcccgagcttcgaccggcgccagagcacgtcgtcggcgctcatggcccattcctgttcttgcaggaagcgcagttcgcgctcgtgaagccccggtgccacggcttctcccatgtcggccatcgcctgcgcatctccaagcagctcggacacgcgtgcgccgtaggcgcgggccagccgcctcgccagcttggcatcgagccatgcatggcgggcctgcaccgcggccacgaagcgctcgaaatcgtcgtcgggccgcgtggcggcaccgatccacgccgacagatcgccgccggccaggaaggcgccgtcggtccatggcgggcgctgcgcgctcgattggccgagcatcttgccgacctcgtcggccgcgtcttcggccagcttgcgaaaggtcgtgatcttgccgccccacacggagagcagcggcgccgccgcggtgttcgactcgagcatgtagtcgcgcgtgaccgcggacgggtcgcccgacgcatcgtcgagcagcgggcgcacgcccgaataggtccagaccacgtcggccggcttgatcggcttgtcgaaatagcggctcgcctgcatgcagagatacgcgatctcttcctcggcaatgcgcgccgcgccgggatcgtcgccgttcagctcgatgtcggtggtgccgatcagcgtgaactcgtcctggtaggggatcgcaaagatgatccgcttgtcgggattctggaagatgtaggcatggtcgtgctcgaacaggcgcggcaccacgatgtggctgcccttgaccagccgcagatgccgtgtggccagcgcctcgcccttggccgattgcgccacgccgcgcaggaacgattcggcccacggccccgcggcattgaccacggcgcgcgcgcgcaccacgcgaatgccaccgtccgcgccttccagcgtggcggtccagccgtcggcgtcgcgctgcgcatggacgcagcgggtgcgcgtgagcacctcggcgccgcgcgtcctggcgtcgatggcgttgagcaccaccagccgcgcgtcgtcgacccagccgtccgaatagacgaagccgcgcttgaactgcggcttgagcggcgccccggccgcgtggcggcgcaagtcgatgctgcgcgagcccggcagcacttcgcgcttggcaaggttgtcgtacatgaacaggccgatgcggatcatccaggccggccgcatcgacgggtcatgcggcatcacgaagcgcagcggccacatgatgtgcggcgcgctcttgagcagcacctcgcgctcctgcagcgccttgcgcacgagcgagaactcgtaatactccagatagcgcagcccgccgtggatgagcttggtcgacgaggaagacgtgtgcgaggcgagatcgtccttttcacacagcaccacgcgccagccccggcccgccagatcgcgcgcaatgccgcagccgttgatgccgccgccgacgatcagcacgtcgcattcggttgccggcagaggcggattggaggagaaatcgctcacaggaaatgggcccgttgattcgtgactttggtcacggaagggcgccattgtattttcgtgtcttttcatttgggttccttttgacgcgattttcccccgagttttcccttagaaatcttcgttttctttcgctttaaagtggcacggcctgtactctccaaagagtcttcacgttctttacgacgcccctgtgaactccaatccgcgccagatcaaccttctcgataccgtgcgcacgcgcggctccgtcaccgtcgagcagctggccgacatgctgggcgtcacgctgcaaacggtgcggcgcgacgtgcagcggctggccgacgaaggcttgctcactcgctttcacgggggcgtgcgcgtaccgagttccaccaccgagaacatcggctaccagcagcgcgaaacgcttcatgccgaaggcaaggcgcgcatcgcgcggcgcgtggccgagctggtgcccaacgactgctcgctgatcctcaacatcggcaccaccaccgaggccattgccaaggcgctgctgcggcacaccggcctgcgcgtgatcaccaacaacctgaacgtggcgaccatcctgagcggcaacacctcgtgcgaggtgatcgtggcgggcgggtcggtgcggccgcgcgaccgcgccatcgtgggcgaggccaccatcgatttcatccgccagttcaaggtcgacatcgcgctgatcggcgtctcgagcatcgaggccgacgggtcgctgcgcgacttcgatctgcgcgaagtgaaagtggcgcaaaccatcatcgcgcaggcacgggaggtgtggctcgcagccgatgcaagcaagttcaaccggcccgcgatgatccagctcggcacgctctcgcagatcgaccggctgtttaccgatgcggagccaccaccgccatttgccgacctgttgcatgctgcgcaggttcggcttgagattgcgcgcgattgagatgagagctcgtcgttttgcttgccgcgctttaaggcattcggggggcgctcccgccgacggggtaccttgctccgcgaatgtcccccggcctgcggcctcctcctttatttcgctgcgcaaggcaccccatcgacgggatcgttgtccagagcggttattgatcgagctgaacaagcgcagcgcccagtgggcgcagggcgccgggtgctccccgcagcgaaataaaggaggagccgaaggcgggggacattcgcggaggggagtacccggtggcctgtgcacgcgccctgaacaagagcgtcccaaaaaccggcgccaagaacgcaagacaagaccccaaggaacacccaacccatgacctacctgctcgccctcgaccaaggcacctccagctcgcgcagcatcgtgttcgaccgcgaaggccatatcgtcgccatcgcgcagaaggagctcacgcagatctacccacaacccggttgggtcgaacacgatccgatggagatctggaacagccagctcgccaccgcgcgcgaagtgctcgccaaggccaagctccagcccgccgacatccacgccatcggcatcaccaaccagcgcgagaccaccgtgctgtggaaccgcaagaccggccagccggtgcatcacgccatcgtctggcaagaccgtcgtgccgagccgctgtgcgcaaagctgcgcgacgaaggcatgaccggcaccatccaggaaaaaaccgggctggtcatcgacgcgtatttttccggtaccaagctgcgctggctgctcgacaacgtacccggcgcgcgcgcccaggccgagcgcggcgaactcgccttcggcaccgtcgacagctggctcatgtggcagcttaccggcggcaaggtgcacgtgaccgacgtgagcaacgcgtcgcgcacgatgctcttcaacgtgcaccgcaacgaatgggacgcggacctgctcaagttgctggacattcccgctgcgctcatgccgaaggtgcaaccgtcgagctcgcactttgccgacaccgatgccgcgctgctcggccgcgcgctgcccatcggcggcgtggccggcgaccagcagagcgccctcttcggccaggcctgcttcgcggccggcatggccaagaacacctacggcaccggctgcttcttgctgatgcacacgggcgccgcgttccagccctcgcacaacggcctgctcgtgaccagcgccgcgcagaccgacgccacgccgcagtacgcgatggaaggcagcgtcttcgtcggcggcgccgtggtgcagtggctgcgcgacggcctcaaggccatcaagggcagcgccgaagtgcagtcgctcgccgagagtgtgcccgacgcgggcggcgtgatgatggtgccggccttcaccggccttggcgcgccctactggaacgccgacgcacgcggcaccatcaccggcctcacgcgcggaaccacggtggcccacatcgcgcgcgccgcgctggaaagcatcgcctaccagagcgccgcactgctgcaggccatgagccgcgatgcagtcgccgccggcggcacccccgtggcggagctgcgcgtggatggcggcgcgagcgtgaacgacctgctgatgcagttccaggccgacctgctgggcattcccgtggtgcggcccgaagtgatcgagaccaccgcgctgggcgccgcctatctcgcgggcctgtccaccggcgtctacagcgacgcgcgccagctctcgaagctgtggaaggtggagcggcgcttcatgccgaccatgggccgcgcgcaggccgaggagtcgatggcccgctgggagcgggcggtgcggcaggccaccgccacctgaggcgcatcggctcgcggttcttttttactactgcgccggaaccagaaagtcctggctgatccgcccaccgagttcgttcacgcgatcaaggaactgcgtgagataagcatgcagcccggtcgcgagaatttcgtcgacccgcgcgtactgcaggtcggccagcagcttgccggcgcggcgctgggtttcggcgctctgctcgttctgcaccttggcgaggttgttcaccacctcgaccaggctcgcgtgcagcgaacgcggcatgtcggcgcgaagaatgagcagctcggccacgcgctcgggcttgatcacgtcgcggtacaccttgcggtagacctcgaaggccgagacgctgcgcaagatggcgctccagtgatagaagtcgtactcttggtcttcctcggtggcggtgccgaagaactcgctgttgagggcgtgaaacttcacgtccaccagccgcgcggtgttgtcggcgcgctccaggaaagtgcccaggcgcgagaagtaaaaggcctcgtcctgcagcatggtgcccagcgtgacgccgcgcgagaggtgcgagcggaacttgacccattcgaagaactgggccgggtcgcgctcgaaatcgcccgcgcgcagcatgcggttgacttcgagccatgtggtgttctgcgtttcccaggcctcggtggtgagcgcgccgcgaaccgcgcgcgcgttttcgcgcgcggctttgaggcaggagacgatcgaagacggattgctctcgtccttgaccatgaactccatcacgtcgtggggcgtgatctgctcgtacttcttgttgtacgaaggcagcagctcgctgatggacagcacgccctgccagccgtatttggccacttcggccgattggggcaggagcgaggtctggtagttgacgtcgagcatgcgggcggtgttttccgcgcgctcggtgtagcgcgacatccagtagaggtgatcggcagtgcgtgacagcatcgttttgttctcctgattccttgcttgcttgcctgctgcgctaggccgattgcgtttgactttgcgactgcgtcgctttcggcttggcgccgcggtccgcctcgagaatccaggtgtccttggtgccgccgccttgcgatgaattgaccaccagcgagccttccttgagcgccacgcgcgtgaggccgccgggcaccatctgcacctcgctgcccgagagcacgaaggggcgcaggtcgatgtggcgcggtgcaatgccggcgtcgacaaaggtcggcgacgtggaaaggctcagcgtgggctgcgcgatgtagccgtcgggcttggcaatcacggctttcttgaagtcttcgatctcagcctgcgtggccgccgggccgatcagcatgccgtagccgccggcgccgtgcacctccttgacgaccaggtccttcatgttgtcgagcgtgtactgcagctcgtccttgttgcggcacatgtaggtgggcacgttcttcaggatcggctgctcgccgaggtagaactccaccatcttgggcacgtaggggtagatcgacttgtcgtcggcgacgccggtccccaccgcattgcagatgacgacgttgccgtcgcggtaggcgcgcatcaggccggcgcaaccgagcgtcgacgtggggcggaacacctcggggtcgagaaaatcgtcgtcgacgcggcggtagatcacgtccacgcgcttcggcccgcgcgtggtgcgcatgtagacgaagttgtcgcggacgaacaggtcttgcccctcgaccagctccacgcccatctgctgggccaggaaggcgtgctcgaagtaggcgctgttgtacatgccgggggtcagcaccaccaccgtgggctcggccgtggcggccggcgcgctggcgcgcagggtttcgagcagcaggtcggggtaatgcgccaccggcgcgatacggttctggttgaacagctccgggaagagccgcatcatcatcttgcgattctccagcatgtagctcacgccgctgggcactcgcaggttgtcttcgagcacgtagtactcgccgttgccctgggcgtcgggcgcccggacgatgtcgatgcccgagatgttcgagtagacgtcgtgcggcacgctgacgcccatcatttcggggcggaactgcgcgttgttcaggatctgctcggccggaatgatgccggccttgatgatttcctgatcgtggtagacatcatgcaggaagcggttgagcgccgtgacgcgctgcaccagccccttttccatgctctcccactcgtgggcgggaatgatgcgcggcagcaggtcgaacggtatgagccgctcggtgccggaaccgtcctcgtccttggcgccgtacaccgcaaaggtgataccgacccggcggaagatcatttccgcttcctcgcgacgcgcccgcatcacctcgccgggttgcttcgcgagccattggtcgtagcgcttgtagtgttgcctgattgcagcccccgcatagggcaactgctcatacatctcatcgaatttgtgcatggaacgaccaatctccttgagccatagcttagcaagttcgaggccagtgaaagccctaagttggcgcggccgcgcgtcttcaaggcaggcgatggtgccagtaacgggcctggcgctcccgttcgcagccgacctcggcaggcgcccggctgtgccatgaagcggcgccgcagggcacgttttcgaccagccgcacgccatacgcagcatagcgctcgaccacctccgggaccggatgaccgaagcgattgcgatagcccgcctggaccagcgcgatgcgcgggcgcaccgcctcgagcagcaccgcgctcgacgaggttttgctgccgtggtgcggcgccagcagcacgtcggcctgcagcgcgggggttcgcgacaccagcgccgcttcctgcaggcgctcgatgtcgccggccagcagcaccgtggcgcggccgttggcaacgcgcagcacgcaggaaatggcattgggcttggtgaaggaaagatagtcggccggcatgggatggaggatctcgaaatccacgccgtcccaggtccaacgctggccggcttcgcagcgccgggccgggcgcaccgactgcagcggatgcgcggcttcgatcgagctcaggagcgcggcctgcggctgcatcgcgagcaccgcgggcgcgccacccgtgtggtcgctgtcgcggtggctcagcagcagcatgtccagccgttcgtcgaaggcgcgcagcaaaggaacgagcacgcgatggccggcgtcgctttcgaggctatagcgcggccccgcgtcgtacaggaggctgtgcgttgcggtacgcacgaggaccgaattcccctgcccgatgtccgcggccagcagttcgaactcccccgcaggcggccggggcgcctgccacagcagcaccggcagcaggaacggcagccccagcgtgcgcagcgaccacggcagccgcatggccagcaggacgcccccggccaccccgcaggctgccatccacgccggcggagcggccatcgacagcgtggcgtacggcagcgcggccagccagcgcaggagcaaggccagcgcctggaccgcccatgcggcaacatcccagaggggcgccaccgcggtgcccagcatggccagcggcgtgatcaccagcgtgacccaggggatcgccacggcattggccagcaggcccaccacagagacctgctgaaacagcagcaggccgagcggcgtcagcgccagcgtgatcacccattgctcgcgaaaaaacgccagcagccgggccgacggccccgtcttctcgtcggccgcccgcatgaagccggtcgtgaacagcaccccgactgcgacgaagctgagccagaagccggcctgcatcagcgcccagggatcgatggcgaccaccaccgccgcgatcagcagccagacatggggccacggccagcgccgccccgtgagtcgcagcagcgccgcggtggccagcatccagaccgtgcgctgcgaaggcacgccccacccgctgaaaagcgcatagagcccggccaggaacacgccgccgaccagcgcggcctgcggtgcgggaaagcgcagcatcagccgcccgctgcggcgccacagcgcgccgaccgcatgcgccgcgagccaggcgaacatggtgatgtggaggcccgaaatcgacatcaggtgagccacgccggtggcgcgaaaaatatcccagtcgttgcgctcgatggcgccctggtctccggtgacgagggcagcgatcacgcccgcctgccgggggtcggcgacgcgttcgaacaccgcgtctcgcaccgcttcgcgcgcacgttcgagcgggtgccgccacgtggcctgcaaacgtgccggcgccgcgtcgcgggcgcccgttcgcacgtaaccgctggcatgcacgccctgctcccacagccacagttcgctgtcgaagccatgcggattgagattgccgtgcggcgccttgagccggaccgtgagtcgccagcgttcgcccgcgtgcagcggggcggccgcgtctcccctggccgcggcgcgcccttcgggagcgcgtccccagaggctggtgtcgtcgcgataccagccgagcgcaatgcgtgccggaacacgcggcggcgatgcgaggggctcatcggcccagcgggccgactccaggtcgagccgaaaccgcgtaccgccctcgttgcgctgcggcatctgtgccaccacaccgaccacctgcaggtctcgtccttcgatggccgggtccagcgcgccgctcgcataggcagccgcccgccaccctgcgagcccgcctccggcgaaggttccgcaggccagggccccgatcaccggcagcccggccagcatgcgccatgcacgaggccaatggaacatcggccgccatcgccgcgaaagcagggccagccccgcgagacccgtgaagaacaaggccgcataggcacccccgctccacagccctgcctgatgcaactggcatgccgcgccgagcagcgttccgcccagcgcggcaaaggcccacgacccggccatgacgacaccggacgcccgcgccggcgtcaacagcaaactccggaacacatgatgcaaaccctcccaggcccgcgctcaatggcgcgttaattgctttgcttctcggctagtatgcgtctcacaagagacatcttttcgatgcaatctcgcagtactgcacacaaaacgcatgtccattcacgccgcactccaccacgtcacccactacaaatacgaccgcctggtgcagctgggcccgcaggtcgtgcgcttgcgccccgcaccgcactgccgcagcaaggtcatctcgtattcgctgcaggtcgaaccggccgatcacttcgtcaactggatgcaggatccgttcgccaactaccaggcgcggctcgtgtttcccgagaagacgcgcgagttcaaggtcacggtcgacctcgtggtcgagatggcggtctacaacccgttcgacttttttctggagccgcaggccgagaactttccgttcaagtacaccgcctcgcaggccgaagagctcgcgccatacctcgtcaccgaggaacccacgccgctcctgtcggcctacctcgacaagatcgagcgcaaggaacagcgcaccatcgacttcctggtcggcatcaaccagcaggtccagcaagacgtcaactacctgatccgcatggagcccggcgtgcagacgccggaagaaacgctcaccaacggcagcggctcctgccgcgactcgggctggctgctggtgcagctgctgcgtcactgcgggctggccgcgcgcttcgtctcgggctacctgatccagctcacacccgacgtgaaggcgctcgacggcccgagcggcaccacggtcgacttcaccgacctgcatgcctggtgcgaagtgttcctgcccggcgcgggatgggtcggcctcgatgccacgtcgggcctcctggccggcgagggccacattccgctcgcgtgcacacccacgccttcgagcgccgcgcccatcgaaggcggtgtcgacgaagccgaggtcgatttcggccatgaaatgaaggtcacgcgcatctacgaatcgccgcgcgtgaccaagccctacaccgacgaacagtgggccgaggtgctggcgctcggcgacgcggtcgacgcgcgcctcacggccggcgacgtgcggctcacgatgggcggcgagcccacctacgtggccaccagcgaccgcgacgcgcccgaatggaacaccgatgcgctcggccccaccaagcgcggctatgccaccgaactcgtccacaagctgcgggccgagtacggccagggtggttttctccacttcgggcagggcaagtggtacccgggcgagcagttgccgcgctgggcgctttcgatcttctggcgcgccgacggccagacgctctggcacgagcccgagctctttgccgacgagcgcgtgcccacgcactacacgagcgaagacgcacgccgcttcaccaccgtgctggcgcacaagctcggcatcaccgagcgctacgtgcagcccggctacgaagacgtttattactacctctggcgcgaacgccgcctgccggtcaacgtcgaccccttcgaatcgaagctcgacgacgaactcgagcgggttcgcctgcgccgcgtgttcacgcaaaagctcgacgccgtcatcggctacatgctgccgctcgaacccgccaatgccgatgtggacgctcccgcgctcgaaggcccgggctggaaaaccggcccctggttcctgcgcgacgaccggctctacctgatcccgggcgactcgccgatgggctatcgcctgccgctcgattcgcagccctgggccagcaagggcgactacccctacctggtcgagcgcgacccgaccgcgccgcgcgcagcactgccgagttcgtccgactaccgcgcacgctatgccgtgcctgccggcggtgcaatgggcgccgatcttggcgccgtgccctatgaattcggtgcgccgcccgtggtgcccgcggccctgcgcatgcaggcgccgggcggcagcggaaccgcgagcggcgatgccgcagccgcaggcgacggcaaggccccggccgatgcagccgaccgctccgcgacaccagccacgcggcagccccagcgcggcgaatcggcccactgggtcacgcgcaccgcactgtgcgtcgaggtgcgcgacccgcggcgcgccaacggccccgcggccgagaaaaaaggcagcgcctcgggcgtgctctacgtcttcatgccgccgctcgcccgcctggaagattacttggacctcgtcgcggccgtcgaggccacggcgcagcagctgggcatgcgcatcgtgatggaaggctacccgccgccgcgcgacccgcgcctgaagatgctggccgtcacccccgatccgggggtgatcgaagtcaacatccatccggcccacaactggaaggaactggtcgcccacaccgagtttctctacaacgccgcgttcgaaacccgcctctcggccgagaagttcatgacggacgggcgccacaccggcactggcggcggcaatcacttcgtgatgggcggcgccacgcccgcggacagccccttcctgcgccggcccgagctgctcgcgagcctcttgctctactggcacaaccacccgtcgctgagctacctgttctcgggcatgttcatcggcccgaccagccaggcgccgcgcgtggacgaagcgcgcaacgaccaggtctacgagctcgagatcgcgctgaaggaaatcgcgaagaaccgcgagatccacggccagaacatgccagcgtggatggtcgaccgcacgctgcgcaacatcctgatcgacgtgtcgggcaacacgcacaggagcgagttctgcatcgacaagctctactcgcccgactccagcaccggccggctcggcctgctcgagttgcgcgccttcgagatgccgccgcacgcacgcatgagcattgcgcagcagctgctcatccgcgcgctggtggcgcgcttctgggacgacccgtacaaggcccccgtcacgcgctggggcaccgagctgcacgaccgcttcctgctgcccaccttcgtcaagatggacttcgacgacgtgatcagcgagatgcgccaggccggcttcggcttcgacgtcgactggttcgcgccgcatttcgagttccgcttccccttggtgggccaggtgcaggccatgggcgtggagctctcgctgcgcaacgcgctcgagccctggcacgtgatgggcgaggaaggttcggccggcggcacggtgcgctatgtcgattcgtcgctcgaacgcatcgaggtgcgcgtcaccggcctgaacgaaagccgccacgtgatcaccgtcaacggcaaggtgctgccgctgcagcccaccggcaccgtgggcgagtttgtcgcgggcgtgcgctacaaggcctggaacccgccttcggcgctgcatccgagcatcggcgcccatgcgccgctgaccttcgacattgtcgacacctggatgaagcgttcgctgggcggctgccagtatttcgtcgcccacccaggcggacgcaactacgacaccttcccggtcaatgcctacgaagcggaaagccggcgcatgtcgcgcttcaccgagatgggccatacgcccggcctgatgcgcacgccgccggccaccatcgagctcgcgggcagccgcgaattcccattcacgctggacttgcggcgctgagcacgggcattaaaagggcgcaaagggacatttggcacatcggccgtcacaccacccgtgacggcaatgtgacaatccatcccctgtggaacctttgaacgaatccctgttcgacgcccaggcgctggaatttccagccgccctggcgtcggcgctcgccccggccgcgctgcccggccacttcgacgagctgcgcggcgaggccacgcccgcggcgccggcgcggcctgccatgggcattccgcccatggcgccaatgccgcccctgctctacgacgccacggcggagcgcccggccgtggtgccaggcgcgccgcaggcgcagacccagacgcaaacgcagtcccagggtgtccagccagcgccgccccccagagagaagccgcccctcacgccaggctggaacgccttcttcgaccagctcggcccgggcgggttcggcgacctgccacggcgcgcggtcagcctggagcggcagatccgggacaacggcgtcacctacaacgtctatgccgacgccaacgggccgcagcgtccctggtcgctcgacctctttccgctgatcgtctcgcccgagagctggagccagatcgaaaccggcgtgctgcagcgcgtgcgcgtgctcgaccgcgtcatggccgacgtctacggcccacagcagctgctggccgaagggctcttgcccgcggcgctcgtgcgtggccatcccggctacctgcgcgccctgcacggcgtgaagccgccgggcgacacatggctgcacatcgcggccttcgacctcgcccgcgggcccgacggcaactggtgggtggtctcgcagcgcacgcaggcgccgtcggggctgggctacctgctggagaaccggcttgccatcgcgcgccagtttccgcaggccttcgaggcgctgcacgtgcagcgcctggccgccacctacagcgccatgatggacggcctgcagcacatgtgcccggccggcgtaccaccgcacatcgcgctgctgactcccggcccctacaacgagacctacttcgagcacgcctacctcgcgcgctacctgggcgtcaccttggtcgagggcagcgacctcaccgtacgcgaccagcggctctacctcaagacgctgcaggggctgcggccggtgcacgggctcatcaagcggctggacgaccagttcctcgatccgctcgaactgcgtcccgactccacgctcggcgtgccgggcctgctgcaggccattcgcgccggcaacgtgctggtggccaacatgccgggctcggcgtttctcgaatcgcccgcgctgctgggcttcctgcccggcctcgcgcgccgcctcatcggcgaaaagctcaagctgccggcgctgccgacctggtggtgcggcgagcgcgccgcgctcgaggcggtgctgccgcagctgggcgattgcgccatcaagcccacctatcccggctccgacggccagaccagcttcgacgcggtgctgggcagccagctgagccggcgccagctcgacgaatgggccggccgcatcgtgcgcgaaggcgaagcccacacgatccagagctacctcccgctgtcgcaaatgcccacctgggccagcgacatgggccccggccacatcgcaccgcgcgcggtgctgctgcgcgtcttcgcggtgagcgacggcgcgcagtcgtggcgggtgctgcccggcgggctggcacggctcgcgggccgcgatgcgcagatcgcctccatgcagcgcggcggcagcagcgccgatgtatgggtgcagacgcatggcgaagtcgaccgcaccaccctgctgcagccgcacgccacgccggcctcgctggcgcggcaccgcgcgcccgtgaccagccgcgcagccgagaacatgttctggctcggccgctacaccgagcgcgccgaaaacgcagtgcgcctggcgcgcctcacgctcaacctgctgggcagcgaagaccagtcgtcgcgcccgctgctcgactggctgcatcgcatggcgctgcgcaatgcgctggtgccggccgaagtgcccaccgcgccgcagtcgcgccgcgtgttcgaacgcgcgctggtcgccgagctcggcgatgtggagcgcggcggcagcgtgggcttcagcctgcgctgcatccggcaggctgccgccgccgtgcgcgagcgactgtcgcaggacaactggaaccagatcatgcgcgccgaagccgagtttctgcggcgcgcggccgagcaggccggcgaaggcagctttgccaccggcgcggcactgcgcgcgctcgaatccgccagcaccgcgcttgccgccatgaccggtgcgcagaccgaccgcatgacgcgcgacgacgcctggcgcctgctgtcgatcggccgccacatcgagcgcctgggctttctctcgagtgcgctggaggccggcttcgagaacggcgcggtgcacgaagtgagcggcttcgaagccatggtggctctgttcgacagcaccatcacctttcacgcccgctaccagcaacggcgcgacgtggccacgctggtcgacctgctggtgctcgatgccgagaatccgcgctcgctcgcgtgggtcacgcaaacgctgcgcgggcgcattgcgcgcctggccggcagtgcgcccggcaagctcaccgcgctgtcctacgaactgcccgatccggccacctggacgctcgagcatctctgcgtggtgggagccgacgcgaactaccctgcgctggccgagctgctggccagttgcgagacggcggcctaccatgtgtccgacgccatcggcacgcgctacttcacgctcacttccgaatcgctgcgctccgtgggcgcctgatgacgcgctccccgcgaggttgcaaccgaagcagccaaagagaaatttcatgctccttcatgtcacgcacgaaacccgctacgagtattcgcccccggtcgaaacggcgcagcacctggcccacctgaagccgctggccaccggctcgcagcggctcgtgagccacaagctcgccatcgagccgcagcccgcgcagcgcagcgagcagcccgacgtctacggcaacatgcgcgcgttctttgcgctcgaatccacgcacgacagcctcgtcgtcaccgccgaaagcgtggtcgaaacctcgacgccgctgcttgcgccgggcattgcgcgcgacatgccctgggaggccgtgcgcgagcgcttccgctaccgcaaggacgccaccttcgacccggcctcggagttcgtttttccgtcgccctacgtgccgcgccacgacgacttcgcggcctatgcgcgcgcgagcttcgcgcccgagcggtcgaccttcgacgtggcgatggacctcaccgagcgcatgtaccgagactttgcctacgacgccgacagcaccgagatcaacacacccgccgtggaggccctcgcgcagcgcaagggtgtgtgccaggacttcgcccacatcatgatcgcctgcttccgcgccatgggcctgcccgctcggtacgtgagcggctacctgctcacgcagccgccaccgggccagcctcggctggtgggcgccgacgcctcgcacgcctgggtctcggtgtacctgcccggtgaaagtgatggcggcaacggcgacggcaacagagacggccacgacagcgccggcggctgggccgaattcgaccccaccaacggtcgccagcccggcgaggactacgttgcactcgcgatcggccgcgactactccgatgtctcgcccatgcgcggcgtgctgcacggcggcgcgcgccacacgctcaaggtgggcgtgacggtgcggcccatcgaagagctgcggacccaggccgcggaggcggcgcagtcacaatcacagacacaatcgcagattgaatcgcaacccatagacaaggacctccaatgagcgtttacgacaagctttccagcctcggcatcaccctcccccctgtcgccgcccccgccgccgcctatgtgcctttcgtgcggaccggcaatctcgtttttctctcgggccacattgccaagaaagacggcaaggtctgggccggccagctcggcgcaaacatcggcaccgaagaaggcaagcaggccgcacgcgccattgccatcgacctcttgggcacgctgcatgcggccgtgggcgacctgaacaaggtcacccgcatcgtcaaggtcatgagcctggtcaattccgtgggcacgttcaccgaacagcacctggtgaccaacggcgcgagcgagttcttcgccgaagtgttcggccccgagaagggcgcgcatgcgcgcagcgcgttcggcgtggcgcaagtgcccatgggcgcctgcgtcgagatcgagctgatcgccgaagtcggctgaccggctctgcgcaggcagcaacagccatgagcgtgcaggccctgcgctcgtccttcggcaacaagtgccactggtgcgggctgccgatggattttgcggagcctcgcagcgcgccggagtcggccaccatcgagcacctgaacgattcgacgctgggcggcgtccgcaagcagaagcaccggcggcttgcccacgccatctgcaaccagacgaggaacgagttcaagctgcaggccgaacgcggcttccagcgctggattgcagagcgcgtcgaggccggcctcgcccgcgccgcggatcagcccgtcatgccggccgggacgagccccgcaccaccagttgtcccggcagcagcagttgccgcggcgctgcatccagcccccgcagccgttcgatcaggcaggtagcggccgagcggccgatggcgtcggtcggctgcgccacggtgctcaggccggggccgatcagcgaggcccattcgggatcgtcgaaaccgacgaagcccaggtcttgtccgaactgccagcccagccgcgccatcgattgcgcgatgcgcagcgtgaccaccgcattgcccgcgaccaccgccgcccggcgccccctttttgcgcgctgccgcagcgagcgcaaggcttcgtcgagcgcatcgccgtcgccttcgacgctctcgaagacctcgcccgccacccgcggctcgtgcgcggccacgcaggcaccgaaggcggccgtgcgttcgcgccgcgagctcacgcccttctgcggctcggtcacgtagagcagttcgcgaaagccgccttcgaccaggtggccgcaggtgtcgcgcatggccgaatggttgtcgagcgcgacgaagtcggtgtgcatgccaacatggcggcggtcgaccagcaccgcgggcttgccatgcagcgtgaccgcgtcgaccacgttgctgccgcggcccagcgtgttgaggatgaagccgtcgacctggtagcccgcaagcgcatcgatggcctcgcgctcgcgttcgctctcgttgcccaggttgaacagcatcacgaggtagcccgcttcctggcaggccttctcggcaccgcgcagcaccgccaccgaataagggttggtgatgtccgccacgatcaggccgatgagccgcgagcgtccatggctcagcgcctgcgccatcgggctgggcgtgtaggccagcttggcgatggccgcctccacgcgcgccgcgatgtcgcggctcaggaggcggtcgcggtggttgagaaaacgcgagacggtggctttggaaacgcctgctgccttcgcgacgtcggcgatggtcgcgcggcccgcggggttcatgcgcggctctcgctccctctccccctggggagagggttggggtgagggccggcggcgatggcgtgggtagcgtttgcacgacggccgacgccctcaccccaaccctctccccggggggagagggagcaagacaccgggttcatgcagccgccgtgtcgtacgccgccgtcggcttctcgccggccagcacctgcagcaggttggtggttgccagctccgccatggcatgccgcgtctcatgcgtggccgagccgatgtgcggcagcggcgtcacgcgcggatgggtgcgcaagggcgaatcggcggggagcggttccttcgcgaacacgtcgaggcccgcggcgcgcagcgtgccgtggtccagggcgtggagcaaggcggcttcgttcaccgtggcgccgcggccgccgttgatgaaggctgctcccggcttcatgcgcgcgaagaaggcggtgtcgatcatgccgcgcgtcgcgtcggtcagcggcagcatcgccagcacgatgtccgaacgcgcgagcaggtcgtccaggggcgtgtgcgtggcacggccctgcagctcgggtgcctgcgtggccaggtcgaccggccggcgcgagtgatagagcaccggcatgccgaacccgagcgcgccgcgccgcgccacggcctggccgatgcggccgaagccgagaatgcccagcgtctttccatgcacgtcggtgccgaagagttcgtcgccgatgttcttcgtccaccggccttcgcgcacgaggttcgaaagctcgaccacgcgccgctgcgtcgccatcaggatcgcaaacaccgtatcggccaccgtttcggtcagcacgtcgggcgtgtggcacagcacgacgccgcgcttgtgcagttccgccagcgcgtagttgtcgacgccgaccgatatgctcgaaatgacctcgagcgcaggcgctgcgtcgagcagcgccgcatcgaccgtgtggctcgcgccgatgagcccgttcgccgtgcgcagcgcggcggcgaaagcctcgggctccttgcgcggatcggccacggtcacatggtgcgcagcctgcaggcgcgccagctggtcttcgggcaagggccgaaagacaagcacgttcttttttgtcgtcatggtcagagtcctgcttcttcgagttcggcgcgcgtgggcaagccttcagtgtcgcccagaacctgcacggcgcgcgcgccgatccaggcaccgcggcgcacggcctcgggcacgctcttgccttcgagcaatgcgctcaccacgccagccgcaaagccgtcgcccgcgcccacggtgtcgatcacttccttcaccggaaagccatcgacgcggccggtgccggccacgtcgctgtcgtagtaggcgccttcggcaccgagcttgaccaccaccagcttcgcgcctcgctcgcgatagaagcgcgccacgtcctcgggcctggtgtggcccgtgagcagcaggccttcctcgatgccgggcagcacccagtcggcgcgcgaggccagctcgttgacccagtggcgcatcgtttcggtggaagaccacagcgtcggccgcaggttggtgtcgaacgagatcgtgcggccggccgcgcgcatcacgtccatgctcttgagcgcggcctgcaggctggtgtccgagatggccgcgaacacgccggtggcatgcaggtgccgcgccgaacgcagccaggcttcatcgacatcggccggccccatctggcttgcggccgaacccttgcggtgatattcgacgggtgggtcgctgccatcggtgacgcggcccttgaactggaaacccgtgcgctgcgccgcatcgcagatgacgtgcgagcagtcgatgccctcggccctcatggcggcgatcaggtggcgccccatcgagtcggtgccgagccggctggcccagcccaccttgagccccaggcgagaaaggccgatggccacgttggtctctgcaccggccgtgcgcttgtggaacgcctctgcgttctccagtggaccgggccggtcggccaccagcagcagcatggcctcgccgaacagggcaacgtcgaaagcggtgggttctgtcatatgtggttctgcctacgcccgcgcggcgcggatgaagtcgatctgcgtgcgcgtggcggccagcaggtcgtcgccgaccaaggggtattcgatggcgtgcggcacgtcggcgggcaatgcacgcagcaccgcgcgccacggcgcggcggagtcgcccagcggcaccgccacccacttgtgcggcaggcgctgcgcgcccttgcaatgcacgtagcgcacgcggcggcccagcacctctgcggcctgcaaggggcactcgccaacccagtgccagttgcccatgtcgaaggtcatgcccagctcgacgccggcacgctcggccgcatcgaagaatgcctgcagcgcgggcagcgtgccggcacgcacggtctggtcgttctcgatcagcagctcgacgcgggtttgcgacagttccactttcaggccccagagcgagccgtgcgaagaaggctggaaatcgccgatggacatcttgagccgcttcgcaccgatgcgcgtcgctgcggcgatgccgcgcttgagcgcggcgctgtcgagccagccgccttcggcccagaggccttcggggctggagtacacggaggcgaggcccttcagcgcgggcagttcggcgtccgcatcacgcagcatctcgccacgcacttcaacggaatcggcgcccgctgccaatgccatttgcgcgcaccagagctggccatgccgccccacttcggccgcgccgaaggacgacagggaaatcaaaacggaaaaggacattcagtgtgcttggtgggagctgaggatctggccgaggaattgtcgtgtcctttcgtccttgggattgccaaaaaagtcggcgggcggcgcctgctcgacgatcttgccgtcggccatgaagatcacgcggtctgccacgctgcgggcaaagcccatttcgtgcgtcacgcacagcatggtcatgccgtcttcggccaggccgatcatggtgtcgagcacttccttgaccatctcggggtcgagcgccgacgtgggctcgtcgaacagcatgatcttgggcgtcatgcacagcgcgcgcgcaatggccacgcgctgctgctggccgcccgagagctggctcgggtacttgtgggcctgctcgggaatgcgcacgcgcgcaaggtacttcatggccacctcttcggcctgtgcacgggtcatgccgcgcgagcgcatcggcgcgagcgtgcagttttccaggatggtgaggtgcgggaacaggttgaactgctggaacaccatgcccacttcggcgcgcaccgcgtccacattcttgccgccggccgtgaggtcgatgccatcgaccacgatgcggcccttctgcaccgtctcgagccggtttatgcagcggatgagcgtggacttgcccgaacccgagggcccgcagatcacgatgcgctcgccctggcgcaccgacaggtcgataccggtcaacacctggaattcaccgtaccacttgttgaccgcttccatgcggatgatcgattccgtcgtcatgccaggattcctcgtttttctctgccttggcggctcaatgcatcttgggcaggtcggcctgcagccacttttggtagagcttgttgagctcgccgttggcagtgttcttcgcgacgaattcgttgaccgccttgtgcaggtcgtcctggcccggacgcatcgcgatgcccatcgattgctgcaccagcgtgaacttgttttcgtaggtgccggcgggcacgcgcttggcgatctgcgctgcgacggtgaccgagcagccgatggcatcgacctggccggagatcagcgcctgcatggccgaggcatcgtcgtcgaagcggcggatctcggtgccttcgggcgcggccttggtcacggccacgtcttgcgtcgaggcgcgggccacgcccacgcgcaggcccttcaggtcgcccgccgccttgataggcgtcttggtggcaccgtacagcacgatggtcgcggccgcatagggctgcgagaactgcacctgcttcgaacgctcgggcgtgatggccagcgaggcgaccagcacgtcgaccttgttggtcagcaggaagggaatgcggttcgggccggtcaccggcacgatgttggccttgacgccccactccttggccagcagcttggccacgtcggcgtcgtagccgtcgggttggttctgcacattggtggtgccgtagggcggaaagtcgaccagcatgccgatggtgatctcgcccttcttcttgatgtcggcgacggactgcgccgaggcaaagggtgcgaacaccgtgagcgcggcgcccaggccgagagctgccagcgcaacgcggcgggtggtgatacgggtcatggggatgtgtctccgggaaaaagaaagaaagcgacgagaaaagggaatcagcgggccagggcctgcgcgcgcctgcgctccatgcgggcagcgagcagcgacagcggccagcagatcgcgaagtagatggcggccaccaccgagaacacgacgagcggctggaaggtggcgttgttgatgatctggcccgcgcgggtgatctccgcaaagccgatgatggccgcgagcgaggtgcccttgatgatctgcaccaggtagcccaccgtgggcgcgagcgcgatcttgaaggcctgcggcagcaccacgtcgcgcatgcgcgcgctgtacttgaggctcagcgcctcggccgcctcccattggccgcgcggaatggcctggatgcagccgcgccagatctcgcccaggaaggccgcgctgttgagaacgagcgccacgcccgcggcaatccacgggttgatgtcgagcccgagcaccggcgcgccgaagaagatcaggaacagctgcagcaacagcggcgtgccctggaagatctggatgaacaccgtcgacacggtgcgtgcccaggtcgaatcggaggtgcgcatgagcgcgatggtcagccccaggatcgcgccgccaatgaaggcaatggccgacaacgccagcgtccacttggccgcttcgagaatgaaaaggaattcgggaaagccgaaggtacgcatgattgtttgtgctcgggtgcgtggcctgttaccggcggtccgggtagttgagcgtgcgcttgtagatgagcttgaacagcgccgagaacgccagcgccagtgccaggtagatggcagccaccacgatgtagatctcgaaactgcggaaggtctgcgactgcaggttggcggccaccgaagtcaggtcgtcggccgagatgaccgacaccacggccgagctcagcatcaagaggatgaactggctcgtgagcgccggatagatggccttgagcgcgggcttgatgatcacgaagcggaagatctcccagggcttcaggttgagcgccctgcccgcctcgatctgccccttgggaatcgactcgatgcccgcgcgaatgatctcggtcgcatatgcgcccaggttcaccaccatggccaccagcgcggccgtttgcggcgaccagcgcagcccgatggcgggcagtgcaaagaagaagaaaaacagctgcacgaggaacggcgtgttgcggatcacctcgatgtacgcattgacgatgaagcgcaaccagcctggccccgatgtcttgccccaggcgcagaagatagcgaccaccaggcccagcagcgtggccaccagggagagctggacggtgatccaggtgcccttgagcagcagcggccaggcagcgaagacggcgtcgaattgaaactggtaattcatgggtgcggcaaacacggcgtggccgcgcgcatgcctcggaagcaatgcttgcagcttatatgaaaccggtttcaggcctacctagggattcccctaggtcagccttttgacagtccttctgcctacactcatgcgatgctgaatacacccgaggctcctgtccgcgcagaggcaagcgcatccctggcgggcgcctatgcgccgcctgccgtgcagcatttcaggcaggccctgctctggcccctgcggctgatgccggctccggacgacaagccttcgcaccacggtccctggcacgtgctgcgcgagatgggcgatgcctcgccatggcgcgaagagatcgatgaatacaccggcgacagcagccgctttcacgaacggcactacaacgagttcgtgagcttcctgccgtacgtgcagcgctttctctacggcgagggccgctccaagagcaagagcggcaatgaagacggccacggcggcgattcgccgatgcgcgtattccgccgccacgacattgcggcagtgcgcgtggtcgcgcaagccggcgatgcgcccatcacactcgacgtggtgcattgcgacctgtatttcttcttcgacatcgacgtggtgatgctcaacctcgaagttggcgcggaccacctgagcctggcgcaggcgcaagacctgctctaccgtttcggccgcgcgtatccggccggctggaatgccgagggcggcgcgctgcattgcatggccagcgtcgaatggctggctgccgatggcagcgtgctcgcgcgttcggatgcgcagcaacgcgaagcctttctttcgcacgtggcccagcaccgcgcgccgcgcatctcggcccactgggcctatctgatgcagccgctggtgagcgaccattccgacgaccctggccttctgcgttaccgccagatcgagtactaccgcatgccggtgatggcatatctttcgctcgacgatcccaagcgcctctcgcgcaacgacttcatccggctcggactggtcaccggcgccgccgaggccgatgcggcgcagcagtcgcacctgccctatgccgaccagcatcttgccgacttcgagaagcgctattgctacgaccgcttctgggtcgatgcgggcgcggcgcccaacacgcgctacctgtgcaacggccacgcactggtcgtggtgggcgatgcacgctccgagttcttctgttgccgcgaccgcggcgtgctcgcgcagttcaggcaccagcacttcctgctgtttctcatcgcgcacttccagaaggcctcgctcctgatgttctcggaccagctcgtggaggccctcaagcggctcgacatccgcagcacgccgagcgtgaagcagttcaagcgcgccatccgcgcgagcttcgaacgctttctgcgcttcacgcaccgctactggttccacgagatctcggagcaggcgcaggtgcgcgcgctctcccacatgtgcaccgcgcacctcgggctcgatccgctctacgacgaggtcaaggcgcgcatcgccgacatgaacacctacctggatgcagacagcctgcgccggcaagccagcaccgtggtccgcctcaccgtggtcacgctgttcggcctgatcggcacggtgacgacaggctttctcggcatgaacctcctcgccgaggccgacgcgccgctgtggcgcaaggtgatctccttcggcgtggtgttcgggttcacgacctggctgaccatctacaccatggtgaagtcgcagcggctttccgacttcatcgatgcgctctcgaacgaccggctgggcttcaggggcaagctggccgcgctggcgcgggtgtggcggccgggctcggactaagatcgcgcccctctcccctctctccgttgcctgcacagggtttgcgaatgcgcattgcgatcgtctccgacatccatgggaatcttcctgcactcgaggccgtggtcaaggacatccgccgccgcggcgtggacgccgtcgtcaacctgggcgacagcctctccggtccgctgatgccgctggagaccgcgcagttcctgatggcccaggactgggttcatcttgccgggaaccatgagcgccagcttcttaccctgccctccggccggcgaggaccgtcggacgagttcgcgcattcgaggctcggcgggaaggaattcgcatggatggcgtcgctggggccgagctttcgcttcagtgcggaagttttgctctgccatggcacaccggcgagcgatctcgagtactttctggagaccgtcgagtcctcgaacttccgcgcggcaaccatgccggaaatcgatgcgcgccttggcaaggtcgatgccgagctgatcgcgtgcggtcacacgcacgtgccgcgcgtggcccgcgcatccggcgggcagctgatcgtcaatccgggcagcgtcggcctgccggcgtatgacgatatccatccctatccgcacgccgtcgaaacaggttcgccggatgcgcgctatgccatcgtcgagcggtcggaaggtgcctggatctcgacgctcattgccgtgccgtatgaccacgcggccatggctgcgctggctctggagcacgcgcgtccggactgggcctctgcgctctccaccggacgcatgccgtagcggcactcagtcgccgaacgcgatctccgcgctgtcgaccgcgcggatcggcacgccaaagctcgtgatgtccgagagcgtggcattgtggtgcgcacgaatgaaggcgcctgtggcgtgcggcttgtcgtgcgaggtgtgcgcgtcggccgcgagcgtgacctcgtagcccagcccggcggcgcggcgcgtggtggtgtccacgcaaaactccgacgaatagccgcagaccaccacgcgctgcacgcctttcccggtcagccaggcctcgagcggcgtgcgcaggaaagagtcgggcgtggtcttgcggatcttggtgtcacgcgcatcgacgtgcagcgcatcggccagctgccagcgctcggaatcgaactccaggtcgacggcgttctcgtgctggatgaaggccaccggcacgcctgcgccacgcgcgcgttcggtgagcgcattgatccgctgcacgacctctccggcctcgtgagggcgaggcggatcgtcacagaggccacgctgcatgtcgatgacgaggacggcagttttcatggtgatggaaagcaggaccttgggtcacagagtatgaccccggagccggccttccggggcgccgcttcagctccaggcgctcacctcgagccgcaccttgccgctgatgcccggcgccgcaggtgccgcgcccaggcttgaaagcggcacgatgaactgcagcttgccattggccagctgcttcgggctgatcggcagcgacgcctgccccgcggtgtcggtctgccagccgtacttgacgttccagttctgcgccggatcgtccgcccggggcggcgcgatctcgatgaccagcgtgtcgcggaacagcgaactgccttcgtagtggccgtcgagccagaacttcttgttcacctggtagtcgggcacgcgcacgcccagcgtcatggcgtaggccagcgtcggccggtcctgcttcacgcgggccttgttggcaaggaacacggtcgagagatagatcgagcggcgctcgggcttttccggatcggtcagttccttgtgcgtgcggcaggcgggcgagtcttcctcggccacgcgccggctcaggtaccagcgcttgccgcgcggcgcggccagcagctcgacctggtagagcgcatcgacgtcggcgtccttgggcaggtcgggcggcaaggtgacgccatcgacgtcgaaccagagatcgacgcgcacgtcgccgaacagaaagcgcacgaggttctggtaggcctcctcggaattgacgatgccgaagtagcccgagtgcgaacgaaaggcgtaggcggtggccacgggcttgctgcgtttcagctcgtcgatggaccagagcgaggcattctcgatgcgcaccagcccgtcgctgccgtggcccgcgaacatgcgcgaaaggcccttggccgcttcgtagtcgccgcggttggagcccaccatgcagaagaagcgctcggccggaaaggacgcggccggcaggtagtccatgcggccgtcgaccggcgccgtgtccagaaactccgacatcttctcgcggttgaaggtgttcatctcgttggccgtgagccaggccggcacgttgacgccgcccatgtcgatgccgttgtgcggcgtggcataggtaaacaccttgtccacgcaggcgcgcgccgccgcatcgccgagcgccgggttctgcaggaaggcccgcaccaccagcccgcccatcgaatgcgccaccaggtagcagcggaagtcggccgccgggaaagcgggcccctcgcgcagcgccaccaggtcgcgcacgcgaaggatcagcttgctcaaaccctgcgcgtagatcttcacgtcccgcgacttgccgtcgccgagcagctccgagccgctgtcgtagtagcggtagatgacgatggaggcagccggaatgccgtccacgtccttgccggtttcgtcgggcgaaggcttccagtcgttgtccaggatgtccaggccgttttgatagacgctctggtattggtagtcggccagcagccgcaccaccggagattcgaagacgaacttctgcgccggcgcgtccttcttgaccgtggcgcggtacacggtggagcccacattgaagccgcagaacggatcggcggcagtgtcgtcgcgctcggcttcggtcatcgcgtagccgcgcacgtagatgatgggatagcggttgctgctcatggtgtgtgcacctcttccatgctcgcaaaaccgcaagacgcggcgcttttcagtgtgccgcgccaggtccttgccatccatagaacgcatggcatacgacaggtggcgggccgcgcaaatgcccctttgcgccgaatgtttctgccgctgaaaccattcggcgcggcgcccgggctaagctcgcgccgcaaaacccgaccacacccgagcccatgaacgaagacgcccgccccgcgaatctcctccagcgcagcttccgccgctgcggcaccctgctgttcgcggccagctgcacgctggtggccgcatgcaccagcaacagcggctgcgaggtgcgctacgacgggtcgccgcagttcaagggctgcaccttccagaatctgccgaaccccgaagtcatgccttccgcgagcgcatggcgaatctggtcgcgcttcatcgtcggcagcaaggtcgacaccgtgccggtcgatccgattccggtgcgcatgctgagtaccgccgacctggacacgctcgacaacaaagccaaccacgtggtgcggctcggccattcgtcgcacctgctcaagctgcagggcaaatactggctgatcgatccggtgttcagcgagcgggcctcgccgttcagcttcgccgggcccaagcgcttccacaagccgccgctcacgctcgagcagctgccgccgatcgaaggcctgatcctctcgcacgaccactacgaccacctcgacgtggccaccatcgagtacctggcgcagcgcgtgcagcgctacttcgtgccgctgggggtgcgtgcgcggatcgtggccatgggcgtgcccgcggagcgtgtgaccgagctcgactggtggcaaggcggcgaacacgacggcgtgaagctcaccgccacgccggcgcagcacttctcgggccgcacgttgaccgaccgcgaccgcacgctgtgggcctcatgggtggtgcaaagcggcgatcagcgcatcttctacagcggcgactcgggctatttcccgggcttcaagcagattggggagcgcttcggcggcttcgacctggcgctgatggaaaacggcgcctacgacgcctactggcccgccgtgcacatgacgcccgagcagagcgtgcaggccttcgaagacctgcgtggcaaggtgctctattcagtgcacaacagcaccttcgacctcgcctttcacacctggcacgatccgctcgatcgcattgcggacctgtcggaagccaagaagatcgaactggcgacgccggtgatcggcgaagtgctgacggtgggcaaggcgcgcaccaacgagcgctggtggcagggcctgcattgaggcctgcaacagccctctaattgcgctccttgcgctcgcgcgcccggcgctgctgccgggtttcgttggcctgcgccgcgatgcggtccttctcgcgctgcttggccccgcgcttcaggcgcatgcggcggccgaaccagaagctggcaaggccggtgaccaccgcaatgaagaggccgatgacgctgatgtcgatgccgcccatcacagcaccctcacgatgctggccggcttgaagccgaggtcggccgccttgcccttgcgcgcgcggctgccgcgcgcgttgttgagcgtgcggatttccagcgtctcgtcgcgctccttgccaccgcggccgatgccttcgatcttcacgctgcgcgtgtaggccgcggcgcccgccagcgtgtccttcgcttccaggtcgatcagcgtgaggccgcggccgcccttgggcaggctcttgagctcggtgatgtcgaaggtcaggatgcggccgccggtcgaggcgcaggccacgtgcgtggccgccggcatcggctccgcgccgctcgcgccgcccaccagcgagggccggcagagctgctcgccctcgcccacgtcgatgaaggccttgccgccgcgctggcgcgacatcatgttctcgaccgtggcgatgaagccgtagccgcctgtattggccagcagcacgcttgcgcccaccggccccgcgaagaaatgcgtgacgtgcgtgccggcatcgagttcgatgagcgtggtcacgggttggccgtcgccgcgcgcgccagggagcgacgccaccggcaccgtgtagacgcgcaccgatttgtccttggcgctaccgaagaccagcagcgtgtcgacgctgcggcattcgaaggcgccgtaaagggcatcgccggacttgaagctgtattcgggtgccgcagagccgttggcgccgttcttctcgctggcccagcccttctgcgcacggacccagcccttctgcgaaacgatcacggtgacgggctcgtcgaccaccttgacttcggccacggcacgcttctcggcctggatcagcgtgcggcgcgggtcttcgaaggtcttggcgtcggactcgatctccttcaccagcaggcggcgcagcgcggtcgggctgccgaggatgtcttcgagctttttctgatcttcgcgcaggcctttcagctcctgctcgatcttgatggcctcgagccgcgcgagttggcgcagccggatttcaaggatgtcctcggcctggcgttcgctgaggttgaagcgcgcgatgagcgcggccttcgggtcttccgctgcgcggatgatcgcaatcacctcgtcgatgttgagcagcaccagctgccggccttcgaggatgtggatgcgctccagcaccttgttgagccgatgtcgcgagcgcttttcaaccgtgatctcgcggaacgcgatccactcgttgagcatctggcgcagcgacttctgagtgggcttgccgtcgatgcccaccatcgtgaggttgatcggcgacgaggtttcgagcgaggtctgcgcgagcagcgtggtgatgaactcgtcctggctgatgcgcgaggtcttgggctcgaacaccaggcgcaccgcggcgtccttgctggattcgtcgcgcaccacgtcgagcaccgagagcatcgcggccttcagctgggtctggtcggcggagagggccttctttccggccttgaccttcgggttggtgatttcctcgatttcctcgagcaccttctgcgtgctgacgccgggcggcaactcgttgaccacgagctgccactggccgcgcgcaagatcttcgatcttccagcgcgcgcgcaccttgagggagccgcggccggtgcggtaggcgtcggcgatgtcggccgggccactgatgatctgggcgccgccgggatagtcggggccgggcacgatctgcagcagctcctcgtcgctgagcttgccgttcgccttgatcagcgccacgcaggcatcggcgatctcgcgcaggttatggctcgggatctcggtggccaggccgaccgcgatgccgctggcgccattgagcagcgtgaacggcaggcgcgcgggcaagaggcgcggttcttcggtgctgccgtcgtaattgggaatgaagtcgaccgtgccttcgtcgatctcgtcgagcagcaggctggtgatgcgcgcgagccgcgcctcggtgtagcgcatggccgcggcgccgtcgccgtcgcggctgccgaagttgccctggccgtcgaccagcgggtagcgctgcgaaaaatcctgcgccatgcgcaccagcgcgtcataggccgcttggtcgctgtgcggatggaagcggccgagcacgtcgcccaccacgcgcgcgctcttgacgggcttggcacccacggtgccgttggcgccgccaaagcccaggcccatgcgcgacatcgaatagaggatgcgccgctgcaccggtttctggccgtcggacacgtcggggagcgcgcggcccttgaccacgctgagcgcgtattcgagataggcggtttgtgcgtaatcggccagcgtgagggtggtgtcgccgtcggtgggaccctggagatcgagcggaggttgggagtccatgtagaagagaaaaagaaaaacagttgtcgggccgtgcgccttttatgcgctcaacccagtgatcggcgacgaaaaacgcggatgcggcatgttcaggacagcggcacttccgctgtgccgtccgataccgtcggctgctcgggcatgtcgggcatggccggcatgccgcttggcgagtcgggcggcaggttgccacggcccagggcgccgcccttcggcaccgtgagctccatgcgaatgcgccccggcgccttgccgccgcgcgcattgctgccacctccaccgcccagcgccgccgacggcttgaggtaggcgtagagctgcagcaccgtctgcacgtagttctgcgtttccttgtagttcggaatcttgttgcccgcgcgctgcacggcgccctcgccggcgttgtaggcggccagcgccagttcgatctggcccgggaacatggcgatcaggtcgcgcaggtagcgcgagccggcggcgatgttgatgcgcggatcgaacagcttcttttcgatgctgctgcgcttgtccgccgagacgccgtagcgctgcgcggtgcctggcatgagctgcatgagccccatcgcgcccttgggcgacacggcctgcgcatcgaagcccgactcggtggcgatcagcgcctgcagcaattcgtagtcgatcgaatgcttgtccgccgcatcgcgcagcgcggccttcgcggtcttgtagctgggcgaggcttcgaaaagagcgagcagggtctgcgacgcttgcggcaccttcccatcgagcttgcgcccgccgcgtccgaatggcgacacgccctgcgaggtgtcgaagctctggccccggcgaaagaagatctggtagcgctcgtcgatcttttccgccgcgaaatgggccacgcccttgctgtcgacgtagccgtagatgtcagcggcgtgcgccagcccctgctgcgtgcaaagcagcagcaaggccaggaacaacggacgcatgaaatctgaaattttcacgagggtggtcaaacatcgatgtcgacatcgtcagcgcgcagttccatcagctcgcgccgagccgctgcctcgcccttgcccatgagcttggtgatctccccttgggtggacgtgaagtcgaagcgtcccagctgcaccttcatcaggcgccgggtgtccggattgagcgtggtttcccacaattgttccgcgctcatctctcccagacccttgaagcggctgatgttccaggcgccttcgcgcacgccgtccttgcgcagtttatccagggtggcggtcagttcgccctcgtcgagcgcatagaccttggaagccggtttcttgccgcgcgccggggcgtccacgcgaaagagtggcggctttgcgacataaacatggccggcttcgatgagtttcggaaagtgccggaagaacagcgtgagcagcagcacctggatgtgcgagccgtccacgtcggcatcggaaaggatgcagatcttgccgtagcgcaggccgctcatgtcgggcgtgtcggcggggccgtgcggatcgacgcccacggccaccgagatgtcgtggatttcggtgttggcaaagagccggtcgcgctcgacttcccaggtgttcagcaccttgccgcgcagcggcaggatggcctggctttccttgtcgcggcccatcttggcgctgccgccggcggagtcgccctcgaccaggaagacttcgttgtggctgatgtccttgctctcgcaatccgtcagcttgccgggcagcacggccacgccggagcccttgcgcttctcgaccttctggcctgcgcgctggcgcgtctgcgcggccttgatggccagttcggccaacttcttgccgtagtcgacgtgctggttgagccacagctcgagcgcgggacgcacgaagctcgacaccagccgcaccgcatcgcgcgagttgagccgttccttgatctggccctggaactgcgggtcgagcaccttggcactcagcacgtacgaagcgcgcgcgaacacgtcttcgggcaggagcttcacgcccttgggcagcagcgagtgcagttcgatgaaacccttcaccgccgtgaacaggccgtcgcgcaggccgctttcatgggtgccgccggcgctggtgggaatcaggttgacgtagctctcgcgcaccggctggccgtcttcggtgaaggccacgcaccagtcggcgccctcgccttcggcgaaattgtcggcgttcttgtcggcatggccgctgccttcgaagagcggaatcaccgggtcgccgctcagcgtctgcatcaggtagtcgctcaggccgcccttgtagagccactgctgcgtttccttggtcttctcgaccgtgagcgtgacgctcacgcccggcatcagcacggccttgctgcgcagcaggtgcgtgagttcgctcatgggcagcgcggcggtctcgaaatacttggcgtcgggccaggcgcgcacggtggtgccctggcggcgctcgccggcctcgagcttgcggatttcgagcgcctcgatcacgtcgccggcgctgaacgccagcctggccacggagccttcgcgatgcgagacgacttcgagccgcttggacagcgcattggtcaccgacacgcccacgccgtgcagcccgcccgagaagctgtaggcgccacccgagcccttgtcgaacttgccgcccgcgtgcagccgggtgaacaccagctcgaccaccggggccttttcttcagggtgcaggccgaacggaatgccgcggccgtcgtcttcgatgctgaccgagttgtcggcgtgcagcgtgaccttgatcttcttgccgtagcccgccagcgcctcgtcggctgcgttgtcgagcacttcctggatgatgtgcagcgggttgtcggtccgggtgtacatgcccggtcgctgcttgacgggctccaggcccttgagcacgcggatggagccttccgaatacccggaggacgcggacgatgaactggggggagtcttgaggggagtcgccatgggggcggattgtagtcagtcgaaccgaaatgactggatacccatacaggaacatcgcccggcaactgctccatgccatcgaatttcgcggcgttcacggcgccggtctgctttgatgcccggggcgcatcaaagcactggctataaatcatcaatggcgcaaggcccctccacctgccagaggatgcaagtcgctacattcgacgcaatgcaagcctcccctcccactctctcgatcaagcaggtgctgatctgcggcgccatgatcgtcacgctttcgatgggtattcgccacggcttcggcctctggctgcagccgatcacccaggcgcaggactggacgcgccagaccttctcgttcgcgctggccgtccagaacctgtcgtggggcatcttcggcgtgttcgcgggcatggtggccgaccgcttcggtgccttccgagttctgatcgcgggcacggcgttctatgcgctgggcctgctgggcatggcgtattcgcccacgccgctgctgttcacgctgagcgccggcgtgctgatcggcgcggcgcaggcgggcacgacctatgcggtcgtctacggcgtgatcgggcgccagattccggccgagcgtcgctcgtgggccatgggcgtggcggcggcggcgggctcgttcggccagtttttgatggcacccatcgagggccgattgatcggcagccttggctggcagaccgcgctggcggtggtggcggtgctggctctggtgatcgtgccgctggccttcggcctgcgcgagccgcagcgcggggcgctggccggccgccgcgaccaatcggtgctgcaggccgtgggcgaggccttccgctaccccagcttcggcctgctgatggccggatacttcgtctgcggcttccagcttgcgttcatcggcatccacatgccgacctacctgcgcgaccagcgcctggcggccgacgtggcgggctacgcgctggcgctgatcgggctcttcaacgtgttcggcgcctacacggtcgggctgctggggcagaagctggccaagcgcaagatcctggcggccatctaccttgcgcgggcggtgtcgatcatgctgttcctgctgatgccgatttcgccgctcagcgtgtatgtgttctcggcggccatgggctttctgtggctttcgaccgtgcccgccaccaatgcgatcatcgcgggcatcttcggggtggcacacctgtcgatgctcagcggcttcgtgttcctgagccaccaggtggggtcgttcatcggcgtctggctcggcggctacctgtacgacaccaccgggagctacgacatcgtctggtacatcgccatcgccctgggcgtgttcgcggcgctgatcaacctgccggtcaaggaaagcgccattgcgcgcggcggccggccggccgcggtgccgggctgacgacggagaatggaccgatacatgacttcgcagttgcgccatcgcctcgtgcatgccggctggctggccggcgcgctggcggtgctgggcggcgttttcgcgctctacgttcacccgagctttctggtgacactggtcgaccaggtctggtcctgcttctgatcgccatgaaagacatggcaaacccgcacgccggactggcgccctcggaatggatcgtgaagtggtcgcacctgctcgcgcccggcgccaccgtgctcgacgtggcctgcggcccggggcggcacatgcaatggttcgcggcgcgcgggcatgcggtcaccggcgtcgatcgctcaccggaagccacccaggccgcaggtgccttcggccataccctgaccgccgacatcgaatccggcccctggcctttcgcgggcgaggctttcggcgcagtggtcgtcaccaactacctgtggcggccgcgcttggctgacatcgtggccgcggtcgcgccgggtggcgtgctgctctacgaaacctttgccgccggcaacgaaagcgtgggcaagccctcgcgcccggacttcctgctgcagcccggcgaactgctggccgcctgccgggagctgcgcgtggtggcctatgaagacggctttcttgacgagccgccacgcttcgttcagcgcattgccgccgtccgtgccggcgaggccggcccgggccagcccgcgcgccatccgctgcggggaaactgaccccaccggggggccggtttccgccgaccccagagtaagtagaatcggcgctttcgtccaccgacagagagattcccccttggagcaactgacaggcagcatcgtcgctctcgtcacgccgatgcacgacgacggcagtgtcgactatcccgccctgcgccggctgatcgactggcacatcgacgaaggcaccgactgcctcggcgtggtcggcaccaccggcgaatcgcccacggtcgacgtggaagagcattgcgaaatcatccgcgtggcggtcgagcaggccaagggccgcgtgcccgtgatggccggctgcggcgccaactcgaccaaggaagccatcgagctcgcccgcttcgccaagggcgtgggcgccgattcgcagctgcaggtcgtgccctactacaacaagccgacgcaagaaggccagtaccagcacttcaaggccatcgccgaagccgtgggcgacctgcccaccgtgctgtacaacgtgcccggccgcaccgtggccgatatggcgcacgacaccgtgctgcgcctggcccaggtgccgggcatcattggcatcaaggaagccaccggcaacatcgaacgcgcgcagtggctcattcgcgacctgcccaagcactttgccgtgtattcgggcgacgatccgaccgccgtggccctcatgctctgcggcggccagggcaacatcagcgtcacggccaacatcgcgccgcgcaagatgcacgaactgtgcgttgcggccattgcaggcgacgtgcggcgcgccatggagatccagttcgagctcatgccgctgcatcgccatctgttcgtcgagcccaatccgatcccggtcaagtgggccatgtccaggctcggcctgtgcggaggcacgctgcggctgccactcaccgagctggccgaagcgaaccagcccgtggtcgaggccgccctgcgcgccaccggcctgctgaagggctgagccggcgcgccgctcctcgacaccccctgcacttctttttcgcctgccgcaccaaggtcaagcaaccttttgcccgaaccgtgctcagagagtgcgggcaatgcggcccctagattgatcgaacccattccaacaaggaagacgacgttgaagaacctttcgcacatctcgcgattcgcactgctggccctcgttgtcagcctcgccgcctgctccgtcctcgagagcgacaagatcgactacaagagtgccggcaaggccccgacgctcgaagttccgcccgacctgtcgcagctttcgcgcgaaaaccgctatgcggtgccgggcggcgcggtcacggccaacgcctaccaggccggcgttgccaacgcgccgggcattccgaccgcggtggccaacatcggcgacgtgcgcatggagcgctcgggcacgcagcgctggatcatcatcaaccgctcgcccgaccagctttgggacccggtgaaagacttctggcaggaaagcggcttcctcctgaccaccgagcagcgcaaccttggcatcatggaaaccgactgggccgagaaccgcgccaagctgccgcaggacatcatccgtggcacgctgggcaagctggtcgattcggtctactcgaccggcgaactcgaccgcttccgcacccgcctggagcgcacgcccaccggcaccgagatcttcatcagccaccgcggcatgcaggaggtctacaacaacagccgacaggaccagaccgtgtggcagccccgcccgagcgaccctgaactcgaaaccgagttcctgcgccgcctgatggtcaagctcggcgtctcgcaagagcagtcgaagatcctggccgcaaccaccgcgccgaccaagaccgcaaccgttgccgccgtcagcggccagccggtcgtgcagatcagcgaaggcttcgaccgcgcatggcgccgcgtgggcctggcactcgaccgcaccggcttcaccgtggaagaccgcgaccgcagcgccggcctctactacgtgcgctacgtgacgccgaaccccgacaagaaggaacccggcttcttcggcaagctgttcagcagctcgagcaagaacgagtccccgatcaagttccgcattctcgtgaagagccagggcgagagcaccaccgtctcggtcctgaacgaatccggcgcgcccgaaacctcggccaacgcacagcgcatcgtccaggtcattgccgacgacctgaagtaacccgcatgctccgcttccgaagcctcggcagcggcagcacgggcaacgccgcgctggtcgaatccaccagcggcggccgcacctctcggctcctgatcgactgcggcttcggcctgcggcagctcgatctgcggctcgccaaggcgggcctcgcggccggcgacatcgacgcgatcttcgtcacccacgagcacggcgaccacatcggctgcgcccattcgctgtcgcggcgcagccgcattcccgtgtggatgagcgaaggcacctggctcgccaccggcgcacgggatttcgaaggccggctcaacctcgcgcgggacgatgcggaatttgcggtcggcgacatcgcggtgcggccctttaccgtgccgcacgatgcgcgcgagccgctgcagctgcgctgctccgacggcgcccgcaccctgggcgtactcaccgacctgggccatgccacggcccacgtgctttccaggctcagcggcgtgcatgcgctgctgctcgagttcaaccacgacagcgaactgctggccaattcggcctatccggcatttctcaagctgcgcgtgggcggcaagcatggccacttgtcgaacacggcggccgcggacattgcgcgcgcggtgcgccacgacggcctgcgccatgtggtcgcggcgcatctgagcgagcagaacaaccgtcccgagatcgtgcggcgcctgatggccgacgccctcggcggccacgaggccgagatgctcacggccagtgcgtcggaaggctcaccctggctggacgtctgagcgcaacagcccgcctgcccttttcgagccccatgcaaaaagccgccccagggcggctttttgccgggcgcatgaaacgccccgtgcgggccttgcttactgctttggcgcctggttcttcttggcagcctctgtcgcggcattggcggcgtccagagccgacgaggcgcccggcgaaggcgttgcagcggcgggatcgctggtcgacggcgccggggcaaccgcaggcggcggaggcgccggctcggtgaccggcgcgggcggtggggtcacgaccgccggcgcggcatcctctttctttccgcaagccacgagtgcggcagcggcgatcagcgaggcgagcaggacggaagacgacttcttcatggaaactcctttggcgatggacatctgaacgaaaaaattctagacccgcatcactgcccgtttgtgtctcgcagcctcattcgcggcattggcttacaagcccagtgtcgatgccggaaatgcgggccgacctgcccgccaagattcatcaattgtttctcgaagttcgcgccgcgcacgcgggtcgaagccacacacgccgcggctgcgttccggatcgtgccggtgcgcgaaccaatcgggagtccagatggcactcggcaccgcggggctccccgcctccggccggaccgccctgcattcgatgatgtggtcccacatgcgccgccagggcaccagccgcgtgtgagcacgttcgatgacgtcgaagcgctgtcccagcaggatgaaccggcggccggtggccgaccacgcctgtagcgcctggatgctggcccgctcgccgagcggccaatcggcaaagtcggggtcgctgagaaccagttccctccagccttggcgcgacgcgttctcgagcgcagcccgcacgatgccctcgaaggcctcgcggccatcgaaccgtccttcgggcagggacggttccgaaggcacgggcgtctcagcctgcatgaacccaccccgcttcgcaccactcggccaagagcgccagcgcaccctcgctcgcacgcgccagttcgcgtggaccgagcgcgcgccggtcggccagccgccgcatcagcgttgcatcggccccgccggcgcgaaagctctcgccgttgatgtacaggtgccgcgcgtcgtaaagcatgcgcgtgcggcggtcgagcaccacctggttcaacccatccggcgcttcggcaccttcgtcgaaccagacattggccttgggctccgtgagcgattcgcccagtgcgcggtcgatcgcgtcggggtcgcgcagtgcggcatcgacggccttgcgcgcgaaggcctgcagcgcggccggcatggcggccggcgcatcgaccgcgggctgcgtcggatcgcggtagcgcgccagctcggccgggcccgcatcttcgagcgcctccgaataggcctgcgcgatgcgtgccagcaggtcggcgccaagctcgcccaccgcggacgaacgcaggccgatggagcaggtcatgcagtcgtcgccaaccgccacgccatcgtgcgcatagcgcggcggcagatagagcatgtcgcccggctcgagcacaaaactttgctcgggctcgaaatgctcgaggatcttgagcggcacgccctgctgcaggcgcaggtcgctctgcttgccgatcgaccagcgccgcgtgccctgcgcctgcagcaggaacacgtcgtagctgtcgaaatgcgcgcccacgccgccctggtcgctcgcgtagctgatcatcaggtcgtccagccgtgcgtcgggcagaaagcggaactgctgcagcaatgcatgcacgccgtcgtgatgcaggtcgacgccctgcaccagcagcgtccatgcgggctgcttcagcggcggcagcgcacgccgcgcaagcggcccgtgcctgagcgtccagccggccttgccttggcggatgaggcgcgattccacgtcctcacgctcggccagggcgaacagcgcgccgcgctcgatcggtggcaccatggcggggatggcctggcgcaccagcaacggttttttctgccaatactgccgcatgaactgcgcggcgctcaggccgccgagcaacggcagcggttgtgaagtctccatgggagaattctgcaatggaaatctctgaacaatgcgtggtcggcctgacctggacaatgaaagacactctgggcgaagtgttggacgtgctcgacgaaccggtggaattcatggtcgggggcgatgacctcttcgacgtgatcgaagccgccctgcagggccatgagcccggtgcgcgggtgcaattgcagctcgagcccgagcagggcttcggcgacttcaacgatcagctgctctttctcgagccgcgctcgctgtttcccgaaggcaccgaggaaggcatgaccttcgacggcgcggcactgcccaagggcgtgagcgacgccatgcccaaggacgtgatctacaccgtggccgaaatctacccggagcacctggtgctggacggcaaccatccgctcgcgggcatcgcgatccggctcgacatcacggtgcgctcggtgcgcgaagccacggaagaagaagtcggcagcggcactgcgggcacggcctttttcaaggtgcctccaacggcgccgggcaacgatctgctgcactgaccgaaaggcggacgtaccgctgccgcagccagcaaaaagccgggcactgcccggctttttgctgctcgcgaaaaccgccgcaaggcgggttacatgcgcgagatctggccgttgtcgatgcgcacgcggtcgccgatgcgcaagtcgcccgggtgctgcacgtcgaaggcccgatagccgccgcgatcggtctgcacggagatgcgatagctctcgtaggcgcgcgggccgttgcgctgtgcctcgatggtgttgcccagcagcgcaccgcccacgatgccgagggcggttgccgcggcgcggccgctgccgtgcccgaactggttgcccaccacgccgcccacgacaccacccgccacggcgccaccgccggtggtgccggtgccgccggtttcactgcgcatcacttcgatattggccacgtggccatactcgacatacgccgcctcctggtacggaacggcctgtggcggcgcctggtaggggtagcgcgtggtgtgatagaccggcgcgggagcgacgcaggccgtgagcgtggcaagcgccagcgcggaagcgccgatggaaacgaagcgcgttgaaattttcatgttgaaggctcctcgaaataatgggtgcattcggatgcaccaagcctgtgtctaacgcccttcccgcaagagggatgacgcgtgacacacaccgaaacgtaggagcgggccgcgaactgacggttccgatctttaccggcccgatacgcgaagacgaggtcagtgcttgccggtggacccgtagccgccctcgcctcgttgcgaagctgcaaattctgtgaccacgcgaaactccgcctgcaccacgggtacgatcacgagctgcgcgagccgctccatcggctggagcacgaagggcgtgtcgctgcggttccatgcgctgatcttcagttcgccctggtagtcgctgtcgatcaggcccacgagattgcccagcacgatgccgtgcttgtggccgaggccggagcgcggaaggatcagcgccgcatagcccgggtccgccaggtggatcgcgatgccggtgcccacgagctgccacgcattgggctccagcgtgatgggtgcatcgaggcaggccctgagatcgagccctgcgctgccgggggtggcataggcgggcaattgatccaccatgcgtggatcgaggatacgaacgtctactttcacttctacttgccttgcttgtgttgctgttctttttgcttgcgggcggcttcctcgagcacctgctgccacttggcgacaccgggtgaaagcttcaggcccttgaacttgctggcgagccagagggccgcaccgaacaagaccaccagcacgaccacgggcacgccggccgaccacagcgccaggaggaccagcgcgcccaccacgccgatgatcttgagcgccgcaggcgggaacgccccgaagcctggcgccgaggtatcgccgttcgaggattcgcgccgctgtgccgcagccgccgcggcgccctgcgcgcccggtgcacccggcgcaggcgtcatgcccacgtcgagcccgtgatcgccttcgtgcgctgcccgcttgggcaatgcagcctgagcggacagccgctccacgtagctggcgaaatcgccattgggcggtgtgttccattggggattcatcagaccctccagtcaggcagtcgtgcggcgatctcggtcatgagttcgcgcgccagggtgagcttgggcgcgcgcggcagctcgcgcgtgcgctttgcgtccacgaggagcagcgcattgtcgtcctgcccgaaagtcagcgggccgatgtttccgaccaggagcggaattcccttgcgctcgcgcttggccttggcgtgctccaccaggttctcgctctcggccgcgaagcccacgcagaacagcttgcgcgactgggcgcgctcgctcttggcgacggcaagcaagatgtcggggttctcgacgaaattcagcaccggcgtcttgccactgccgtccttcttgatcttttgctcgctgtgcgtcgcggggcgccagtcggccacggctgccgtcgctataaaaatgctagcagactgcgatgcacgcagggttgcttcgagcatgtcctcggccgaaagcacgtcgatgcggttgaccccgcgcggggtgggcaggtgcaccgggccggccaccagcgtcacttcggcgccggcctcgcgggcagcgcgcgcaatcgaaaaacccatcttgccggatgaatggttggtaatgccgcggatggggtcgagcggctcgaacgtggggcccgcggtcaccagcactttctggcccgcaagcagtttcggcgcaaagaaggccgtgacgtcctcgagcagctgcggcggctcgagcatgcgtccgtcgccggtctcgccgcaggcctgccagccgttgcccacgcccagcaccgtggcaccgtcggccgccacctgcatcaggttgcgctgggtggcgggatgcgcccacatctcgcggttcatggccggcgcaatcaagagcggcacgcggtccatcggacgggccaggcacatcaggctcagcaggtcgtcggttcttccctgcaccagccgcgcgatgaagtcggcgctgcagggcgcgagcacgatggcatcggcctcgcggctcaggttgatgtgcggcatgttgttgggctcgcgcgtgtcccactgcgaggtgtagaccgtgcgccccgaaagcgcctgcatcgtgaccggcgtgatgaactgctcggccgcctcggtcatcacgacctggacggtggcgcccgccttgacgaacaggcggcacaactcggccgacttgtagcaggcgataccgccagtgaggcccaggacgatgtgtttgccggcgagatcttgcatggggcgtattgttgctcacccccagcccgcccgcacttcgggcggccgtgcgcagcggccccttcgaaagatgtccttggcggaaggtgtcgcaatgggcacacctataatcagcatttcccactgcccggtcctcgcgtccggaactggcatgaccaaatttgtcttcgtcaccggtggtgtcgtatcttcccttggcaagggaatcgcctccgcctctctcgctgcgatcctcgaatcgcgcggcctcaaagtcaccctcatcaagctggatccgtacatcaatgtcgatcccggcacgatgtcgccgttccagcatggcgaggtgttcgtcaccgacgacggtgccgagaccgacctcgacctcggccactacgagcgcttcatcaccacgcggatgcgcaaggccaacaacttcaccaccggccagatctacaagaccgtgctcgaaaaagagcgccgcggcgactatctcggcaagacggtgcaggtgatcccgcacatcaccaacgagatccaggaatacatcaagcgcggcgccggcctgggcaccgcgcatgaagtggacgtggccatcgtcgaaatcggcggcacggtgggcgacatcgaatcgctcccgttcctcgaagccgtgcgccagatgagcctgcgcatgggcccgaacaactcggccttcgtgcacctgagctacgtgccctggatcgccgccgccggcgagctcaagaccaagcccacccagcacaccgccaaggaactgcgtgccatcggcatccaggccgatgcgctgctgtgccgcgccgaccgtccgattcccgacgacgaacgcgccaagatctcgctgttctcgaacgtgcccgaatggggcgtgatctccatgtgggacgtcgacaccatctacaaggtgccgcgcatgctgcacgagcagggcctggacggcctcatctgcgacaagctgcgcatcaacacgccgccggccaagctgcagcgctgggacgagctggtgtacgaggtcgagcatccgcagcaggaagtgagcattgccatggtcggcaagtacgtcgacctgtccgacagctacaagtcgctgaacgaagcactgcgccacgctggcatgaagaaccatgcccgcgtgaagatcgactacatcgattccgaaaccatttcggcgcaagacgtctcgcggcttgccaagtacgacgcgatcctggtgcctggcggcttcggccagcgcggtgtcgagggcaagatctcggctgcccgctttgcacgcgaaggcaaggtgccctacctcggcatctgccttggcatgcaggtggccaccatcgaatacgcgcgccacgtggcgggcctcaagaacgccaacagcaccgagttcgaccccgagacgccctgccccgtgatcgcgctgatcaccgagtggaaggacgccgacggcaccgtcaagacacgcaacgagaagtccgacctcggcggcacgatgcgcctgggcgcgcagagctccgacgttacggccggcacgctggcccacagcatctacggcgacgtggtgaccgaacgccatcgccaccgctacgaagccaacgtgaactacctcgacgagttgcgcgccgcaggcctcgtgatttccgcgctgacgcagcgcgaacacctgaccgaaatcgtcgaactgccgcaggacgtgcacccctggtacatgggcgtgcagttccaccccgaattcaaatcgacgccgtggagcgggcatccgctcttcaatgccttcatcaaggcggcgctcgagcacaaggcccgcagcgcgggcggtgcaaagaacctgaaggcagtcgcatgagccgccgggccgctcccaaggcgaatgacgaagtgcgcagcacggagacatccctatgaaactttgcggattcgacatcgggctcgaccagcccttcttcctgattgccggaccctgcgtggtcgagtccgagcaattgcagatggacacggccggcacgctgaaggaaatcacttcctcgctcggcattccgttcatcttcaagagcagcttcgacaaggccaaccggtcgtcgggcaccagctttcgcggcccgggccgcgagaagggcctcgagatcctggccaaggtgaagcgcgagctgggcctgcccgtgctgaccgacgtgcacaccgaagacgacatcaccgaggccgccaaggtggtcgacgtgctgcagacccccgccttcctgtgccgccagaccgacttcatccgcgcggtggcgcagtcgggcaagccggtcaacatcaagaagggccagttcctcgcgccgcacgacatgaagaacgtgatcgacaaggcgcgcgcggctgccaaggaagcgggtctgcccgaagacagcttcatggcctgcgaacgcggcgcgagctttggttacaacaacctggtgtcggacatgcgttcgctcgccatcatgcgcgagactggcgcaccggtcgtgttcgacgccacccactcggtgcagctgccgggcggccagggcacgagctcgggcggccagcgcgaaatggtgccggtgctgtcgcgcgcggccgtggccgtgggcgtggccggactcttcatggaaacgcaccccgaccctgccaaggcgctgagcgacggccccaatgccgtgccgctcaagcacatgaaggccctgctcgaaacgctcgtggcgctcgaccgggtcaccaagaaaaacgcattcctggaggacgtcttccaatcatgagcagtggttatgtcatcgcccacgtcgaggtcaccaacccggcgcagtacgaggaatacaagaagtggtcgagcgcggccatgcaggcgcatggcgccgaagtgtgcgtgcgcggcggccaggtcgaagtgctcgagggcgactggtcgccttcgcgcatcgtcatcctgaaatttcccagcttcgagaaggccaaggccttctacgaatcgcccgaataccttaaggcgcgcgaagcgcgcgccggtgccgccgtcatgcgcatgatcgcggtcgaaggcatttgattatttgagttcgagactgaaaagagaaagagaaacgcatgagtgcaatcgttgacatcgtcggccgcgaaatcctcgacagccgcggcaatcccacagtcgagtgcgacgtgctgctcgaatcgggcaccatgggccgcgcggccgtgccctcgggcgcatcgaccggttcgcgcgaagccatcgagctgcgcgacggcgacaagaaacgctatctcggcaagggcgtgctcaaggccgtggaaaacatcaacaccgagatctcggaatccgtgctcggcctggacgcgagcgaacaggccttcctcgaccgcacgatgatcgacctggacggcaccgacaacaagggccgcctgggcgccaacgccaccctcgccgtctcgatggccgtggcacgcgctgcggccgaagagtcgggcctgccgctgtaccgctacttcggcggcatgggcggcatgcagctgccggtgccgatgatgaacgtcatcaacggcggcgcgcacgccaacaacagcctcgacctgcaagagttcatgatcatccccgtgggtgcgccgagcttccgcgaggccgtgcgctacggcgccgaggtgttccacgcgctcaagaagatcctgggcgaccgcggcatcagcacggcggtcggcgacgaaggcggtttcgcgcccagcgtcgagagccatgaagcagccatccagctgattctcgaagccatcgacaaggccggctacgtggcgggcgagcagattgcgctcggcctcgattgcgccgccagcgagttctacaaggacggcaactacgtgctctccggcgagaacctcacgctgtcggccggcaactgggccgacatgctggccacctgggtcgacaagtacccgatcatcagcatcgaagacggcatgcacgaaggcgactgggacggctggaagctgctcaccgaccgcctcggcaagcgcgttcagctggtgggcgacgacctgttcgtcaccaacaccaagatcctgcaggaaggcatcgacaagggcattgccaactcgatcctgatcaagatcaaccagatcggcacgctgaccgagaccttcgccgccatcgagatggccaagcgcgcgggctacacggccgtcatctcgcaccgctcgggcgaaaccgaagacagcaccatcgccgacatcgcggtgggcaccaacgccggccagatcaagaccggttcgctctcgcgctccgaccgcatcgccaagtacaaccagctgctgcgcatcgaagaagacctcggcgacatcgccagctaccccggccgcggcgcgttctacaacctgaagtagcgcccgaagccggcggcaatgcgctcgcgcctcgttccacccatcgtgctgttgctgctgctggtcatcctgcagtggcagctgtggaacgggcgcggcagcgtgcgcgacgtgtctcagctgcagaccaagctggcggagcagaaagaggccaatgccaaggccacggtgaccaacgagcggctggcctccgaggtcaacgacctcaaggtcggcctcgagatggtcgaagagcgcgcgcgacaagaattgggcatggtcaagcccaacgaagtgttcgttcaggtgacacactgaacacgcactgaacgagacttcaccgctgtgcccgagttcttctcggcccccgccttcgcgctctggggctcaccggtcagctggctcgaactcgtggccgccgtgctggcgcttgcgatggtcggctgcaacatgcgcgaagtccattggggctggccgctcgcgatcgtcagttcgctgctctacgtggctgtgttcgcacaggcgcgcatctatggcgacgcctcgctccaggtgttcttcgcgatcgtcgcgttctggggctggtttcagtggctgcggggccatcgcgccgatggcagcgcattgcaggtcagccggctttcgccgcgcggcatcgcgttttcgctggtggcctgcgcactggcgtggcccgcggtcgcgctcttcctgcaccgctttacagacaccgacgtgccctggtgggacgggttctcgaccgggctcagcctcgtcgggcagtttctgctcgggcgcaagttcatcgagaactggcttgtgtggctggcggtgaacatcgtgagcgtgggcctgttcatccacaagggcctgtggctcacggtcggtctctacgccatattcgcggtgctcagcgtggcgggctttcttgcatggcgcacgcgcatgcccgaggccgcgcgcgcatgactcccatgctgccagtcggatgcgtcattgcgctgctcggcgccgagagcaccggcaagaccgaactcgcccgcgcgctcgtgcagcgcctgcaagagcgcggcattgccaccacgatggtgggcgaatacctgcgcgaatggtgcgaccgcgaaggccgcacgccccgccccgacgagcagcggtccattgcccaagagcagacccgccgcatcgacgccgcggccgccgcgggcgtggtggtggccgacaccaccgccctcatgaccgcggtctacagcgagcagctgttcggcgacacctcgctccatgccgacgcgctggcggcgcaggcgcgctatgccatcaccctgctgaccgcgctcgacattccatgggttgccgacgcattgcgcgacggcgaccacgcgcgcgaacccaccgatgcgctggtgcgcgcggcgctgacgggcgcaaggctttctttcgcggtggtgcacggcaccggcagcgaaaggctctccagtgcgtggaacgccatcaattccattgccgggagcgaaggccggccccgcgcacgaggccgcttcgattcgaaaccggcctcctggtcatggccttgcgagaagtgctccgacccggaatgcgaacatcggctcttcagcgatctgatcggacgccgcgacaatccctcgacccccagctcggagatctgatgttcccgcttcgtttctctcatcaccccgctggctgcgccagcctcttgcttgccgcactgctcgcagccggcgccgccacggcagcgcccgtcgccgccacggtggaaaacgccaccacgcccacggcctgcgccgaggaagacaacgtctcgctggtgctgcacggcgcaggcatccggcgcatgcgcatcgaggcgctgcagccggcttacctggacagcatcggcaacgacaccaccgcacccgacttctcgaactgcaacttcgacggcggggcacaccccaccgatccggcccacaaattcaagccccgccgcgtggtgctgctcgacgatgcgcagtggcgcatcgtcggcatgaccttgccgagtttctggcggccgcagcaggtgccggtgcgggtgggcgcgcgcacggaccgcggctttcacatgctgcagatcttccgcaaggaggaaggcaaggcgctcgaagcgctggtgctctacccggccgacggctactggcgcatcaagccgctgccggaagaacgcttcggcgacggggtgtacggctcttcgttcctgctcggcccggtcgaacagggcagccggccggtggtcgacatcgcgtcgatccgcatcgtgcccaagcccctggccattcacctgcgtttcgtcgggggcggcagcgccgtggccaaggtgtccgagatcagccgcacgcgcaccgcgctcgacgtgcggctctcgtcgccgacggccaatgcccggccctttgccgtgctgcgctcgatgtacgtgacgcccgacaacgccgacgtgagcgaggtgcggtggcaggagtcgcccgatgccgcggagcaggtgatgtccctgtccgaactgaagacgctgagcggcacgcacctgcgtttcggacgcagcctgccttcgcgccacaacaccagcgcacccgacatcgtgttcagcgacttcgacgacaaggtgccgcgctgatcgaggctgccggcttcgccgagggcgctgccgttactggacgacggagctgcccggaacctggtcgcccggcggcttgaagagctgcgcggtatcgaccgcgtcgaagcggtactgcttgccgcagaagtcgcagcccacctcgatgtcgccacgctcgacgaggatctcctcggcttcttccacgccgagcccgcggatcatctgcgccacgcggtcgcggccgcaggtgcacgcgaaatgcggtccgagcaagcccgcctggggttcgaagcgcagcaacttttcttcccagaacaggcggcgaagaatggtctcgatgtcgagcgtgagcagctcgtcgcgcgtgaggctcgaggcgaggatcgagatgcggttgtagtcctcgttcaggccgatctggtcctggttggcctggtcgtggtccttgtcggcggtgccggactggccttcgaggttgccctcgcccttcaccggcaggcgctggatgagcaggccggccgccaccttgtcgtcggcggcgagcaccagcgtggtgtcgagctgctcgctttgcagcatgtagtgctgcagcacgtcgctgagcttgccgagtttctcgccctcgtcgtcgaagagcggcaccacgccctggtaaggcgtcgtgcccggcagcttgtccttggggtcgagcgtgatcgcgcagcggcccttgttgttctcgttcaccatctcgggcaggcgcgcatcggccggcaggtcgccgatcaccttggcggtggcgcgcaggctcaggtcgggcttggcctcggccaccgccaccttgaccgggccgtcgccgaagatctgcaggatcaatgcgccgttgaacttgatgttcgcctgcatcagcgtggccgcggcggtcatctcgccgagcagctcggccacgggcggcgcataggcgccggtcgcggtgttggaggcgcgccgcgccaggatttcctgccacgcatctgtcaggcgcacgatcatgccgcgcaccggcaggccatcgaacaggaatttgtgcagctcgctcaaaacggattcttctttctgttgggcctgcgcggggtcaggcaatcttcttgaggcccttcgcatagcgaacggcgtttttgacgtaatggtcggagccgtggcgcaaacgggcggcgtcttcgtcgctgatcgtgcgcatcaccttggcgggcgaaccgaagatcagggaattgtcgggaaactccttgccctcggtcacgacgctgccggcaccgacaatcgaattgcggccgatcttcgcgttattcaagaccacggcctggatgccgatcagcgagttgtcgccgatggtgcagccatgcagcatgacctggtggccgatggtgacgttctcgccgatggtgagcgggctgccggggtcggaatgcagcatggacatgtcctgcacgttgctgttgcgcccgatggtcatcgtctcgttgtcgccgcgcagcaccgcaccgaaccagatgctcgcgttctcgcccagctgcacgttgccgatcacttccgcgctgtcggcaacccatgcgccggtgccgagttgcggcgcaacgccgtcgagttcatagagggccatcgtggagtctccggggggcaaaaactagaattgtagggatgcacccccgattgagcgcgctggccgcgctgcgactgaccgatcctgaagcaaaggtggcggcaacacgcaccaccgctgcgcgagccgctaccgattccatagcaaccgaacccctgcgcactgtgggcgatgacatcggcgtgccgggccgccccgaaaggccgctgcgcgtggccgccaccgccgtgcaaaaacgctcgcccttcacgcccgaaggccgcgccgcgttgatccattcgatctgccacatcgagttcaacgccatcaacctcgcgctcgatgcggtctggcgctacgacggcatgcccgaggcctactaccgcgactggctgcgcgtggccgatgaagaggcgcagcacttcacgctgctgcatgcgcacctgcaggacatgggctggcgctacggcgacttccccggacacgacgggctgtggagcatgtgcgagaaaacgaaggacgacgtgctggcgcgcatggcgctggtgccacgcacgctcgaagcgcgcgggctcgacgccacgccgctgatccaggccaagctgaagcgcgtcaacacgcccgatgcactgcgcgcggtcgagatcctcgacatcatcctgcgcgacgaagtgggccacgtggccatcggcaaccgctggtaccgctggctctgcgagcgcgagggccgcgaccccgaggcggcctaccccgaactggtggcgcgctacgaggcgccgcgcctgaagccgcccttcaacctcgaagcacgcagacgcgccggcttcagcgccgaggaactgcgcgcgctctcggccggcagcaaggactgaacagaaggcctacgcgggccgggcgtgcaccaccagcttcggcgtgaagtactggaccacctcgccgagctggttgagcgtgcggcagcgcatcgtcaccatcgcgcggccgggcttggagcgcgagggcgtgatctcgaggacctcgctcaccacgtgcagcacatcgccgggccgcgtcggcttgggccattgcaattcgccgcccgagccgatgatgccctcggccagcgggatgccgctttccaccagcagcttcatcgtgagcgccgccgtgtgccagccgcttgccgcgaggccgccgaagaaggtgttcttcgcggcttcttcgtcgatgtggaaaggctgcggatcgaactgaagcgcaaaggccttgatctgcttcacgtccagcgcatgttcgccgctctggaaacgatcgccgatcgacaggtcttccaggtacagcgcgcgcttcgcgccggtgtcgtcagtgagtgccaccatgggagttccttgtagtgcttgtgcgcattctcgaactttcagcgcgccaggtcgcagggtcaatcggccttgatgttcgcggccttgacgatgcgcccattgctctcgaactccgaggcgatctccctggcaaaggccgcgggggtgccgccggtcggcacgttgtcggtggccgtgagcttggcgcgcaactcggggctggccagcgccttgttgatctcggcgttgtactttgcaacgagcgcgggcggtgtcgccgcgggcgcaaagacgccgaacagcgagttgatgttggccgcgttgtagcccagctcgcccagcgtgggcacctgcggcaggctttcgagccgcgcgggcgcgcccaccgccagcggacgcagcttgcccgactggatgtgcgaagtgagcgtggggctcgcattgctggagagaatttcgaactgcccgccgagcgcgtcgttgagctgctggccaccgcccttgtacggcacgtgcgtgatgtccacgcccgccgccgaacgcacctgctcgagcacgatatgcccaagggatgccggaccggacgtggcccagcgcaccgcccccggctgggccttggcatcggccagcagcgcgcggaagtctttcgccttgctggctggcgtggcaatcagcagcaccggcgaatacatcacgctggcgaccggtgccacgtccttcagtggatcgaagggcagcttgccgaggtgcgggctgagcaccagcgggctgatggccgagaagccgagcgtggcaccgtccggcgcggccttggccaccgcatccatgccgatagcgccgctggcgccggcccggttttccaccaccacggtggttcccaactgggtggcgagcttgtcgccgagcgcacgcgcgaccacgtcgctgacacctccggcagggtacgcgacgatgatgcgaatggtcttgggaacggcttgagcctgtgcaccggcggcagcgaacagcgctgcaccggcgaagagccacgacggcttgaatgggaaatgcatggatttcatggcagtctggtggatggagtggaaggccgcggcgtcttcagccgcgcgggtggtgcttggcgtgcagttgcttgagccgctcgcgcgccacgtgggtgtagatggtggtggtcgaaatatcggcgtgacccagcagcagttgcaccgcgcgcaggtcggcgccatggttcagcaaatgggtggcgaacgcgtggcgcaaggtgtgcggcgacagcggcacgtgaatgccggccgcggtggcctgcttcttcacgatgatccagaacatcacgcgcgtcatgcccgcgccgcgcgaggtcacgaacaggtcgggcgtctgctgaccgtcgaggatggcgggccgcgactcctccaggtagcgctcgatccagcgcctggcctcgccgccgaagggcacgaggcgctccttgttgcccttgcccagcacgcgcagcacgccgtcgttcaggctcatgtcgatggccttgagcgcaacgagctcgctcacgcgcagcccgctcgcatacatcagctcgagcatggcgcgatcgcgcagccccagcggcgtctcgacgtcgggcgcggccagcaggtcgtcgacctgcttttcggacaaggtcttgatggcgcgcggcatctgccgcgccggcgcgagccgcaggctcggatcggccgcgatgcgccgctcgcgcagcgcccagcggtaatagcgcttgaacaccgtgagccgccggttggccgaggtggccttgcccttggtggagagccgcacacccatgtaggcctgcaggtcgttctccttcgcggcatcgagcagcgcgccgctgcgttccttgcgcagccacgctgcgaacagtgccaggtcgcgccggtaggcggccagcgtgttcttcgacagtccatcttcgagccagagcgcgtcgatgaagtcgtcgatttcaggggtttgtgtggcggcggcctcggtcatgcctgcaagatagcaaaaagaaaatcaccaaagaaaaaggccgcctcgtgcgggcggccttggctcagagcaacaccggtcagtcgagcttcagcttctgcttggccaccacctgcttgtagacctcgtactcggccttgatctgcgcggcaaactgctcgggcgtgttggccacgatcagcgaaccggtgtcttcgatgcgcttcttcacggccgggtcttccacggatttcttcacgccggcattgatcttgtcgaccacttccttcggcaggcccttggggccgaggatgccgtagtaggccatgcgattgaccggctcgagccccacttccttgaaggtcggcacgttgggcagcgcggcaaggcgctgcggcgcggacaccacgatgggaaccaggcgaccgctctggatgaacggcatggccgacggaatgttgtcgaacatgatcggcacctggcccgccaccacgtcgttgagcgccgggcccgcgccgcggtagggaatgtgcgtgacgaaggtgttggtgaggctcttgtagagctccatcagcagatggccgatgccgccggtgcccgacgaggcatacgaatacttgccggggttcttcttgagctcggccacgaactccgcgtagttcttggccgggaagctcgggttcaccgcaatgatgttcggcgtggccgcgatgttgatgatcggcgtgaagtcgttgatcgggtcgtacggcaccttgggattgatggccgggttggccgccgtgctcgagaccgtggccacgccgagcttgtagccgtcgggcgtggcgcgcgccgtttcggccgcacccacgatgccgcccccgcccgcgcggttgatcaccaccaccggctggcccagcgctttgcccagggggtcggagatgacgcgcgccacgatgtcggtcgtgccgcccggtgcaaagggcacgctcagttcgaccggcttgttgggatagccctgcgcgaagctctggccagcgaccgcgaccagcgcggcggcacccaccatggcgccccattgacgacgttgcatcgaaaactccttgattgactgtatcgaaaaagcaaagccccggatgctagcggcttcgcactgcgcccgtgctgtggaatacccatggttcgccacggtttatgctcgaagcggtgaacttcgcccagctgctcttcccggatttttcgctcatcgccatcggctggctgctttgccgctacaccgcgctcgaccgccgcgtgtgggaccaggtcgaaagcctggtgtactactttctttttccggtattgctgttccattcgatcgtgcgcagcccgctcgattttggcgccacctcgagcctgctcaccgcgggcgtgggcatcggcatcagcggtatcgcgctggcctatgcgctgcccttcattccaggcctgcgcacgcacatcgaccgccgcgaccatgccgcaagcgcgcagatcgcgtttcgcttcaactccttcatctgccttgcgcttgccgaacggctggccggcccgcaaggcctgttactgatcgcagtgctgatcggcgtgtgcgtgcccatgttcaacatcgcggccgtctggccgatggcgcggcacgccaagaccggctttgcgcggcagctcgtgcgcaacccgctgatcgtcgccacgctggcggggctgctcgcgaacgtgctgggcttcaccgttccgaactgggccacgccaacgctgacgcgcatcggcgccgcatcgctcgcgctcggcctgctggcggcaggggcgggcatgcagttcgcaaccttggggcgcggcaaggtgctggcggtttcggtgctggccatccggcacctggtcttgccgctggtcgcctggggcctctcccttgcgctgcgcctggacgccacgcaggcttcggtgctgatggcgttttcggccgtgcccacggcctcgagcgcctatgtgctggcagcgcgcatgggctacaacgggccgtacgtggcgggtctggtgaccctgtctacgttgctggggatggcgagcctgccgtttgcgctggcgttgccgcgctagccggcgcgggccgctgcgccagtgcccatgccacgtgctcgcgcaccagctcgctgggatgggccgcccgcgtggccaaggcctcggcggcgccgccctcgccggcgcgcagcgcgttgcccagcgcgacggcgatgttgcgcagccagcgctcgtgaccgatgcgccggatggggctgccctcggtgaagcgcaagaaatcttcctcgctccaggcgaagagcgaggccagcgcctggccggtcagcccttcgcgtgcgtcgaagtcgggcagcgcgcttttctttgcaaacttgttccaggggcagatcagctggcagtcgtcgcacccgtagatgcggttgcccatcaacggccgaagctccagcggaatgggtccgccgtgctcgatggtgaggtacgagatgcagcgccgcgcatcgagccgatacggcgcaatgatggccttcgtcgggcacacgtcgatgcaggcgctgcaactgccgcaatgcgcggtgaccggctcgctttcgggcagcgccatgtcgacgtagatctcgccgagaaagaacatcgaacccgcgctgcggtccagcaccagcgtgtgcttgccgcgccagccctggccgctgcgcgaggcgagctcggcttcgagcaccggggccgaatcggtaaaggcgcgatggccgaagggccccacctcctcggcaatgcgctcggccaattttgcgagccgcgcgcgcagcaccttgtgatagtcgcgaccgcgtgcatagaccgagacgatggcttcaccggggcgcgtgaggcggtcgaactccacggcctgccaatcgtccagcggcgtatcgcgcggcagatagtccatgcgcgccgtgatgacgctcacggtgccaggtaccagctcggccggccgcgcgcggcgcgtgccgtgtgttgccatgtatttcatctcgccatggaacccatgggccagccattgcatcagaccttcctcggcgctcgatagatcgacgcccgcgattccgatttgggagaatccgagttcccgggccaatgcctgaatacgagcaacgagtggatggctgacgatcacttgccgattgtagaaattccgaagaacgccagccgcagactgcactggcgcagcgaggacgacaccgccgccttcgcacgcgcgcttgcggcctcgcccgccttgcgcgatgccttcattgcgctgcatggcgacctcggcgccggcaagaccaccttcgtgcgccacctgctgcgcgcgctcggcatccacggccgcatcaagagcccgacctatgcggtggtcgagccgcacgaggcacccgacgggctcgccatcttccatttcgatttctatcgcttcaacgatccacgcgagtgggacgacgccggtttccgcgacatttttgccggaccggggctcaagctcgctgaatggcctgataacgccacgggccgtacgccaattgccgacctcgctattaaaatagaagcaatgacagacgacacacgcagcgtgaccctcctggccaacaccccccgcggcagcgatctgctggcgcgcatcggcgtatgaaggcgagcggcctcaagcggcgggtgctgctgcagggcggcagcattgcgctgatgctcggcgtgcaccagattgcgcgcggcgccaccattcttgccgtgcgcgtctggcccgcggccgactacacgcgcgtgaccatcgagtccgatgcccggctccattcgcagcagctcgtggtgggcagtccgccgcggctggcggtggacatcgaaggcatcgacctgaaccccgaactgcgcgagctggtcggcaagatcaagcccggcgatccatacatcaatggcctgcgcgtcgggcagaacgcgccgaaggtggtgcgcatcgtcttcgacctgaagcaggccgtggtgccgcaggtgttctcgctggcgccgatcgccgcgtacaagcaccggctggtgctcgacctctatcccgaaaaagccatcgatccgatggaagcgctgatcaccgaacgcctgcgcgaggcgccgcgcggcagcggcagcggcggcaacgacgccgccgtggccagcgcgccctcggtgccgccgcccgccgcgccctcttcgggtctcgcgcccgatggagggccgccgatcctcgtgcggccttcgcccaacgtgcccgcgccgcgccctgtgcctggcgccaccgcgcctcccgcccggccaccagccgcggcggccgcgcccgcacccgatccgctcggcgaactgatggcgcagcagtcgacgcggcccggccctgccgcgccaccaccgcccgctgcgcccatcgcgcctgttgcccctgctgcgccgcccgtcgccgccgcgcgcaacggcgccaccgcgagccgcaccgaccgcatcatcatcgtggccctcgatcccggccatggcggtgaagacccgggtgccatcggccccaatggcacgcgcgaaaaagacatcgtgctgcaaattgcgcaccgcctgcgcgaccgcatcaacgccagcagcgtcaacggcaatccgatgcgtgcgtttcttacgcgtgatgcggactttttcgtgccgctgggcgtgcgcgtgcaaaaagcacggcgcgtgcaggccgacctgttcgtgagcatccacgccgatgccttcaccacgcccgccgcgcgcggcgcgagcgtgttcgcgctgagccagagcggcgcctcgagcagcgccgcgcgctggctcgccaacaaggaaaacgaagccgacaaggtgggcggcgtgaacgtcggcaaccacgaagcgcaggtgcagcgcgcgctgctcgacatgagcaccacggcgcagatcaacgacagcctcaagctcggcggcgccatgctcggcgagatccgcggcatgggcgcgcggctgcacaagccgcaggtcgagcaggccggtttcgccgtgctcaaggcgcccgatattccgagcgtgctggtcgaaacggcgttcatcagcaaccccgaagaagaggcgaacctgcgcagcgtcagctaccaggaaagcctctccgacgcgctgatgcgcggcatccagcgctactttgcgcagaacccgccgctggcgcgcagccgtcagctttgactgccttgcgccgccctgctgtcccacgccgggcggcccgtggcaccgcacacccaggcgcggcaggctcctacaacgctgacaggccgcttttgcccatcatgattccatcactctagaaaggtggacgacatgatgaaggcacgaatctggatggctgctgcggcggctaccacggtcatggcagtggcgggttgcgcctccggtcccaaccagaacctgggcaccggggtcggcgcacttggcggcgcggcagtcggccacgccatcggcggcaacacggccagtacgctgggcggtgcagccattggcggcgtgatcggcaaccaggtgggccgcagtgtggacgagcgcaactactacgagcgccagcgcgtctatccgccgagcacgtactacccgcgcaacggtccaacctattgaccattcccaaccctcagctgtgaagcgcgcctccaacggcgcgcttttttttgagcgtcgatcaggccttggacggcaactgcgcgcgcgctttttccgcgcgcgacgcacgccaggcaccgaagatggcgatcaggccaggcacgatgatcaacgcccagatgatcttgtccaggtgctcgcgcacgaagggcaggttgccgaagaaatagcccgccgttgcgatgccaagcacccagatcagcccgccgaccacgttgaacatcgtgaactttgcgcggctcatttcggccacgccggccacgaagggcgcaaaggtgcgaatgaagggcatgaagcgcgcaagaatgatcgtgacgccgccgtagcgctcgtagaacgcatgcgcctggtcgaaggccttgcggttgaagaagcgcgagttctcccacttgaagaccttgggcccgaagtagcggccgatgctgtagttgcactggtcgcccaggatggcagcggcaatgagaaccgcgcaggccagcggaaagctcatgagccccacgccgcacagcgcacccacgatgaagagcagcgagtcaccgggcaggaacggcatcaccactgcgccggtctccacgaacacgatcaggaagagcagtgcatagacccacggtccataggcaatgacgaaggcctcgaggtgtttgtcgacatgcaggatgaagtcgatgagaaagctgatgatttccatggtggcggattatccgtgctgagtgccgcatggcttcgccgtgatggattcagagaccctggatgacagctcgatacatccgggggaggcttctagaatgctcgcgtgagcgcccttccctcctccattccctctctcgatcgacgtccgatccgcgaacttcccgacgagctgatcagccagatcgccgccggcgaagtggtcgaacggccggcatcggtggtgcgcgagctgctcgacaacgcactcgatgcaggcgcacgtcaggtcacggtacggctggcctcgggcggcgttcggctgatctcggtcgaggacgacggccagggcattccgcgcgaagaactcacggtggcactgcgccgccacgccaccagcaagatcgccaacctgaacgacctggaaaccgtgggcaccatgggttttcgcggcgaggcgctcgccgccatcaatgccattgccgagctcagcattctttcgcgctttgcgggcgccgacggcgcttttgcgctcgacggccgcaccggcgagctgcgcccggtggcccgcgccgtgggcaccacggtcgaggtgcgcgagctgttcttcgccacgccggcgcggcgcaagttcctgaagaccgacgccaccgagctggcccactgcatcgaggccgtgcggcgccatgcgctggcgcggccagaagtcggcttctcggtgtggcacgacggcaaactggtggagcagtggcgcgccgccgaccagcgcgagcagcggctggccgatgcgctcagcgacgacttcgtggcgcaaagcgtggcggtcgatcacatcggcggcccggtgcgcgtggtcgggcgcgcgggcattcccgacgcggcgcggtcgcgcggagaccagcagttcttctacgtcaatggccgtttcgtgcgcgacaaggtgctttcgcatgcggtgcgcagcgcctatgaagacgtcctgcatggccaacgccagccggtgtatgcgctctacctcgaaatcgatccgtcgcgggtcgacgtgaacgtgcacccgaccaagatcgaggtgcgctttcgcgacgggcgcgaggtgcatcaggcggtgcgccacgccatcgagaacgcccttgccgcgccgcgcgcgggcgatgcggtggcgcctgccggcgtgcagcaaccctttttcaagccgaacctgccggcttcgggcgccacctgggcgcagcccgccatcaacttcacggccagggagcgcggtgccggcgatttcgaggccatgtggccgcgtcgggcggacgagtcgacccactcacccgagcccgctgcctcgggctggcccattgccggcgcatcgccgatggcgttccgcgcgccggccgcgttgccgggtgcatcgtcggcacccgaagcccttgccacccacgaggaagcctggccgctcggccgcgcgctggcgcaactgcaaggcatctacatcctggccgagaacagccagggcctgatcgtggtcgacatgcacgccgcccacgagcgcatcgtctacgagcggctcaagacgcagctggacggcgccgccatcaccagccagccgctgctgattccggccacgttcgcggccacgccccaggaagtggccaccgccgaggcctgcgccgcggtgctgccgacgctggggctggaaatcacccccttttcgccgcgcacccttgcggtgcgtgcggtcccggggaccctggccgacggcgatccggtggagctcgcgcgcagcgtgctggccgaactggcccagcacgacgcaagcagcgtcgtgcagcgggcacagaacgaattgctgtcgaccatggcctgccatggcgccgtgcgggccaaccgcaagctcaccatcgacgaaatgaacgctttattacgtcaaatggaagctaccgagcgttcggaccagtgcaaccatgggcgccccacctggcggcagctgtcgattcgcgagctggacgcgctttttatgcgcggcagataaccaatcgggggcttttgagggtttttccggggtttttggcggtcatccgtgaagcgggcacgggcgttgcatgtgtagaacaaagtgccgcctgagcactgcggggaggggtgctgaggcgcagtgtcggcgcgtttcagacgaaagtgcatgaactttctgccggcttcgctgtccctctagcccatgaaacgctggtccctgcttgcctccgttctttcgctgtgcgcccttctggcggccggttgctccacgttcgatgagcagcagcgcgagtggatctttcaacccagcgaccgcagctggggcaataccgccaccatgaccgagggcatgcaggacgtctggatcgacttccagtcgtccatcaccggcgaatccgcacgccttcacggcctctggctcggcggcgagcccgaaaccaccgaccggcccgtgatgctctacctgcacggcgcccgctacaacgtcgccgggtcggcgccgcgcatccagcgcatgcacgaactgggcttttcggtgctggccatcgactaccgcgggttcggcaagagctccaagggcctgccctccgaagaatcggcacgcgaagacgcccgcgccgcctggacctggctcgccgcccgccatccccggcagcaccgttacatcttcggccattcgctgggcggcgccatcggcatcgacctggccgcgcacgtcaacgacgaaagcggcaccatcgtcgaaagcaccttcacctccattgccgacgtggtgagcagcttcaagtggggctggctgccgttcggtccgctcatcacgcagcgcttcgaggcgatcaaccgggtcaaggacatcggcgcgccgctgctggtggtgcatggcaccgccgacagcctcatcaaccccacgctgggccgcaagctctacaacgcggccacggttcccaagcttttcgtgctggtcgagggcgggtcgcaccacaacaccaattcggtcggagaggcccagtaccgctcggcgctctcgcagctgttccgcatgaagcccgaggccaccatggctgtgcggcagacggaaggcatgcccatgcccgcgacgcgcagcgcgcaaccggtgcccgtattgccgccgccccagcgcgcggattcggcccctccgccgcaagaagcgcgcgccaaggccgccgccagcgcgcaggccatctgacgcaaggcccggcttcgcttttgttgttaccctcgggcgcttatgccgccctcccttgccgccaccggccatcctgaaaacctgaaatacatagcgctcgcggggccgaccgcctccggcaagaccgcggttgcgctggcgatggcgcgcgtgcggccggtcgagatcgtcagcgtcgattccgcgctcgtctatcgcggcatggacatcggcaccgccaagccgagcctggccgaacaggcggccgtgccgcaccacctgatcgacatcctcgaccccgccgaaagctacagcgccgcggctttcgtggccgatgcgacacggctgatcgacgagatccgcgcccgcggcgccttgccgctgctggtgggcggcaccatgctttatttcaaggccctgttcgatggcatcgacgccatgcccgccgcggacgccgcggtgcgggcccgcatcgacaccgaagcggccgcgctgggctggcccgccatgcatgcgcggctcgccaaggtcgatcccgtgacggccgcacgccttgcgccgcaagacagtcagcgcatccagcgcgcgcttgaagtctgggagagcagcgggcagcccttgtcgagctttcatgccggggaaaacaaggctgcgaaaggcctggccgggggcctgctcttttcgctcgaacccaccgaccgcgcctggctgcatgcgcgcattgccgatcgcttcgacgccatgctggccgccggctttctcgacgaggtcagggcgctgcgcgcacgcggcgacctctcgacagagctcccctccatgcgctgcgtgggctaccgccaggcgtgggaaatgctcgacgcgtgcggcggcgcatcgcccgacgccaaggccatgaacgagctgcgcgaacgcggcatcgcggccacgcgacagcttgccaagcggcagatcacgtggctgcgcagcatgccggctcgcaccgtcatcgcctgcgatgcgcccgacgccgtgcagaccgccgttcaacgcattgcaaccgccgaatgacgctgcgcatttccaagctcgccaagcactatggcgatgtcccggtcttcgagaacgtgacgctcaccgtcgagcccggcgaattcgtcgccatcgtcggcgaatcgggtgtaggcaagtcgacgctgctcaactgcatggccgggctcgacagctgggacgcgggcaccgtcacgcacgaaggcaccgacatcggcgcgctcgacggcgaagcctgcgcgctctggcggcggcgccacgtgggcttcgtgttccaggcctttcacgtgctgccgcacctcgacgtggcgcagaacgtgtcgctgccgctcatgctgctgggccggcagaaggacgacggccgtgtcgcgcacatgctcgaagcggtgggcctgcccggcatgggcgcacgcctgccgcaaacgctttcgggcggccagctgcagcgcgtggcgattgcacgtgcgctggtgcaccgccccgccctgctgctggccgacgagcccaccggcaacctcgaccccgccaccgccgccaaggtgatggagctgctgatcggccagacgcgcgagcacggcgcctcgctggtgctggtgacgcactctgagagcgcggcggcccgtgcggaccgcctgctgcatctcacggccgaaggaattcgcgcctaaagctacgcgagcagcgcggcgtagcgcgcgaggtcgacgttgccgccgctcaccacgatgccgacgcgctggcccgcaatggccttgcctgccgcgatggcccccgcgaaagcgaggcaacccgtcggctccaccacgatcttcatgcgctcggcaaagaagcgcatcgcctcgacgagctgcgcgtccgtcacggtgaagatgtcgtccacgtcgcgccggatgatgccgaaggtgtactcgcccaggtgctgcgtctgcgcgccgtcggcaatggtcttgggcgtgtcgatgtgcacgatcttcccggcgcgcagcgactgctggccgtcgttgcccgcttcgggctccacgccgtagaccttgcaacttggcgccagcgcgcgcgccgacagcgccgaacccgacagcagcccgccgccgcccaggcacacgaacaattggtcgagcgggccggtctcctcgatcagctccttcaccgcggtgccctggcccgcgagcacgtcgggatggtcgtagggcgggatcatcgtcatgccgcgctcttgcgcaagccgcttcgtcagcgcctcacggtcttcggtgaagcggtcgtacgtcaccacttcagcgccatagcccttggtggctgcgaccttggcggcgggcgcgtccttgggcatgacgatgacggccggaatcgacagcagccgggccgacagcgcaatggcctgtgcgtggttgcccgaggagaacgcgatcacgccgcccttgcgctgcgcagcgctgaacttcgacagcgcattgaacgcaccgcgaaacttgaatgcacccatgcgctgcaagttctcgcacttgaagaagaaactggcgccccagcgctcgtcggccgtctgcgagcgcagcacgggcgtgcggtgggcatggccttggagccgcgcagccgcggcaatgacgtcgtcgtaggtaggtagttgcatgggccgagcttagcggcggcttgcgatttgttgcagcgccgatgggtaaaaacccgggatacgcggcagcccggcctttcgtattctgtatacagagttcagaaagaaggccgccatgccagcccagctcgtcagcatcgaaaccgcgcccgacctcgtcgaccaggtctaccgcgccctgctgggcgccatcagcagcggctcgctggcgcccggcgagcgcatcacgcaggaagacatcgcgcagcgcctctcggtgtcgcgccagccggtgctgcaggcgctgcggctgctcaagaaagacggcttcgtgctcgacgcaccgggccgcggcgtgctggtggcgccgctcgatgccgagtggatgcgcaaggtctaccaggtgcgcggcgcgctcgacgtgctggccgcaaggctcgcggccgggcaacgctttcgcatcgaccccaagctgctggagcgcggccgccgcgcggcgcgcgggcgcaacgtcgaagccatgatcgatgccgacatggcctttcaccaggccatctacgaagcctcgggcaatccgctgatcggccagagcgccggccagcactggcgccacctgcgccgcgccatgggcgcggtgctgcaggccgagccgcagcgcgaatcgctgtggaacgagcacgaggccatcgctacggccattgccgcaggcaacgccgaacgcgcggcgcgcctgagcgaggaacacgtcgcacaggccagcgaggcattgagccggcggctcgcgcaccagcttgcgcgcaccgcatccacccaccaaggagacaaggcatgaagttgacccccgagcaacgcgcgcggttcgagcgcgatggctacctgttcttccccggccatttttcgcccgaagagacaaagacactgaccgatgccgtgcccgagctctacagccggcgcgaagccttcaacgtgcgcgagaagggctccgacgcggtgcgaaccaactttgccgcgcacctgatcagcgagccctttgcccgccttgcacgccatccgcgcatggtcgagccggtgatggctctcttcggcgaagaggtctacatgcaccagttcaagatcaacggcaagatggctttcgaaggcgacgtgtggcagtggcaccaggactacggcacctggctcaacgacgacctgatgcccaccgagcgcgcaatgaacgtcgcgatttttctggatgacgtgaacgagcacaacggcccgctgatgttcattccgggcagccaccgcaagggggtggtcgatgcgaagcatgacctcacgaccaccagctatccgctctggacggtggacaacgagctgatcgcgcagctcgtggagcgcgcgggcggcaagaacggtggcatcgtctcgcccaaggggcccgccggttcgatgatcctgttccacagctgcctcgtgcatgcctcgggcagcaacctctcgccgttcaaccgcgtggcggtgtacctgagcctgtgcgccgtcagcaaccacatccgccgccacaagcggcccgagtacatcgcacacagaaatttcactcccatcgagatgctgcccgacgattgcctgctgaagccctaccccgtcgaagtgccgtggaagaacggcctgcccgagagcgcgctgcagacctcgcttgaaatcctcgataccgcggaggcctgacgccatgagcctctacacccgcctgcagcagcgcgccgccgaaggccgtcccatccgcatcggcctgatcggcgcaggcaagttcggctcgatgtacctcgcacagattccgcgcacgccgggcgtgcagctggtggccattgccgatctctcgcccgatgcggcgcgcaccaatctcgagcgcgtgggttggaagccgggccgcgccgcggcaggctcggtgcaagaggccctcgacgccggcaccacctggatcaccgacgactggcaggccgtgacgcgcgagcccgccatcgacatcgtggtcgagtgcaccggcaatccggtggcggcggtcgaccactgcctggacgcctttgcgcacggcaagcacgtggtcaacgtgacggtcgaggccgatgccttctgcggcccgctgctcgcgcgcaaggcgcagcaggccggcgtgatctattcgctggcctttggcgaccagcccgcgctgatctgcgacctggtcgactgggcgcgcacctgcggctttccggtggtggcggccggacgcggccacaagtggctgccgcacttcaccgaatcgacgcccgaaacggtgtggggcaactacggcctcacgcccgagcaggcgctgcgcggcgggctcaacccgaagatgttcaacagctttctcgacggctccaagccctccatcgaaagctcggccgtggccaacgccaccggccttggcgtgccttcggacggcctgctctacccgcccgcgagcgtggaagacattcccttcgtcacgcggccgcaaagcgagggtggcgtgctcgagcgcaagggcatggtcgaggtcatttcatcgctcgaggccaacgggcgaaagattccctacgacatccgcatgggcgtgtgggtcaccgtcgaggccgagaccgactacatcaagaactgcttcgaggaatacaacgcccacaccgacccgagcgggcgctacttcacgctctacaagcgctggcacctgatcggcctggaggtcggcatgtcggtggccagcgtggccttgcgcggcgaacccacgggcgttgccacctgctggaacgccgacgtggtggccaccgccaagcgcgacctcgcccccggcgaaatgctcgacggcgagggcggctacaccgtctggggcaagctgctgccggccgagcgctctgtgcgcctgggcggtctgccgctcggcctggcgcacaacctcaagctggtgcgggcggtgaagaaggggcagagcctctgctgggccgacgtggcgatcgacacctcgaccgccgcctacaggctgcgcagcgaaatggaggccatgttcgcgccctccgtcaaggccagggcggcctgaagacataggtggcgcaaccgttgcaccaaacggcaatcgcgtaaaaaataatctgctcggcacggcgcttcgtgtcgaaatgagcggctgcgggccgtcattgtggtgagcgatcttgctcagcctcttttccacgacggagagacaccatgcagtacatgttgatgttctatcagcccgcagccgagttcgaacagcgcgacgacgcctcatcgcaggcctatcgggccagctggatggcatatgccgatgcggtgcgcgcgtcaggcatttcgctcggcggccacggcctgtttccgcccatgaccggcaccacgctgcgcgtgcgcggcgacaagcgccaggtgcaggacggacccttcgccgataccaaggagcagctcggcggctatttcgtgatcgacgtggccgacctcgatgcggctctcgagtgggccgcgcgggcgccgtgcgccaccagcggcggcgtggaggtgcgccccgtattcaccgcgaccgcggccgccgcctcgtgaacgacccggcggctcatcgggccgccgaacgggcagcgcgcgagtcgtatgggcggctccttgcgatcctgtcggcgcgcacgcacgacattgcagcatccgaggatgcgcttgccgatgcgtttgcgcgcgcgctcgagcgctggcccgccgacggcgttcccgaccagcccgacgcctggctgctgagcgtcgcgcggcatcgcaggctcgacgcctggcgccatacccgcgtgcaggatgcagccacgcaaaccctgctactgctggccggtgaggtggacgtgggcgccgccgacggcgcggccgtgcccgacgagcgcttgcggctgctcttcgtgtgcgcgcatcccgccatcgacgcggccgcccgtgcgccgctgatgctgcagacggtgctcgggctcgacgtggcccgcatggcgggcgccttcctgacctcgccctccacgctcggccagcgcctcgtgcgggcgaaagcgcgcatccgcgccgcgggcattcccttcgaatacccgcaggctcgcgacctgccgcaacggctgcaggacgtgcaggatggcatctatgccgcctacggcaccggctgggacgacatcgacggcgcggatgccttgccccgcaacctcactgccgaagccatcgacctcggccgcattctttgcagcctgatgccgaacgagcccgagccgctcgggctcctggcgctgatgctgttctgcgagagccgcgcggcgtcccggcgcagcgaggccggcgcctatgtgccgctcgaccggcaggacatggcacgctgggatcccgcactgctcgcacaagccgaggaatgcctgcggcgcgcctcgggcatgcagcgcatcggcgcgtaccagctggaagccgccatccagtcggcgcactgcgagcggcgcgtgggagcaccggtgccgcccgaagcgctggtggcgctgtatgagggcctgctggccctccggcccagcgtcggcgcgcaggtcagcctggcctgcgccttggcgaatgcgcgcgggccggacatcggcctgcaggcgctcgacgccattccagcggacgaggtcgcgagctatcagcccttctgggcagcgcgcgcgcacctgctggcggccggcggtgcgcgtgccgcagcacgccaggctttcgaccgcgccattggcctcagcaccagcgcggccgtgcgcgcctatctcaacgggatgtccgagcggctttgacatttccgccttctcccgagcgaaggccacaatcgcagcatgcgtgccttgctcaccaccttttcatggcaggaactgcgccatcacccttggcgtaacgccgcggccgtcctggccgtgatgctgggcgtggcgctcgcgttctcggtgcagctcatcaatgcctcggccctcgacgaattctcgagcgcggtgcgttcggtcaacggccagccggacctcgaggtgcgcgccgtgcagggcagcttcgacgaagccgtgttcgcgcgactggcgcagcatccacaggtgacgctggcgagccccgtgctcgagttccaggccctggcgctggccggcgaacgccaggtgccgatgcgcgtgatcggcatcgatgcgctggcgctgcccaccattgcaccggcgctgatgccgcagccccgcaagaacgccaaccgtttcgcgatgctggcgccgggccatgtgtttctcaacgccgcggcgcgcaacgtgctcggcctgccggccgaagcggtggaaggccgtgcggagacgattcggctgcgcagcggcagcgcctggcagcaactcgaagttgcaggccatgtcgccgccagcggaacggccctggcggtgatggacatcgcggccgcgcaagacctgttcgacaagctcggccagctcagccgtgtcgacctgaggctggcaccgggcaccgaccaggcggcgttcatcgcatcgctgcagcggtcgccgggctggcccgccggcttgcagtttgccgagccgggcgacgcggccgagcgcgtgagcaatctctcgcgcgcctaccgcgtcaacctgacggtgctggcgctggtggcgcttttcaccggggctttcctggtgttctcggtgctggcgctcagcgtggccaagcgcgcgcagcagttcgcgctgctcggcgtgctgggcctgacgccgcgcgagcggctgcgcctggtgctggtcgaatcgctggtgctgggcctgatcggaagtggcgccggcctggccctgggcacggcactcgcggccttcgcgctgcgcgtgctcggcggcgacctgggcggcggctacttcgagggcgtggcgcccgtactgcactggagcaccggctcggccttgctgtacggcgggctcggcgtgctcgcggccctggtgggcggctggtggcccgcgcgcgcggcacaggcgctgcccgaggcgcagacgctcaagggcctgggtgccgcaccggtcccaagccagagccactggctggcgctcggcctcattgccgcgagcgcggcactggccaacatgccggccgtcggcggcatcccggtggcggcctatctctcggtgggctgcctgctggtgggcggcatcaccgcactgccctggctgatcgcgctgctctacgaccgcgtggcacccgtgtttgcgcagcgcgtgttgccgatgctcgccatcgagcgcgcgcggcgcatgcgcggcaccgccgccgtggcggtcagcggcgtggtcgcgagcctgagcctcgcggtggcgctcacggtcatggtcgcgagcttccgcgattcggtgacgcgctggctcgacgtggtgctgccggccgacctttatcttcgcgccacgtcgagcggccgctccggcaattcgggcacccagagcagcagcgacacggccacctttccgccggccttcgtgcaggcgctggcgcaactgcccggcgtggaacgcaccggcacgctgcgcacccggtcgctgcagctcgaccccgcacagcccgcggtcacgctgatttcgcgcagcctcgacggcggcgcggcgcaggccctgccgctggtgggccctgcgctgccggtgcccgcgggacagatcggcatctacgtgagcgaaccgatggtcgagctgtatggcgccaagccgggcacactgttcgcgccgctgtcctcggcattgggcagcagcagcaccacaggcgccacgccagccgccttcttcgtggcgggcgtgtggcgcgactatgcgcggcagttcggcgccatcaccatggacgcgcgcgatttcgaacgcctgaccggcgagcgcaacgtgagcgatgtgtcgctgtggctcgcgccgggcgcatccgaaggcgcggtccgggccgcggttcgcgagcttgcggcgcgtcgcgtcggcgtgagcggcgaatccggatcgaacatcgagatctccgccgtcgggcagattcgcgcgacttcgctgcgcatcttcgaccgcagctttgcagtcacctattggctgcaggccgtggccattgccatcggcttgttcggcatcgcggcgagcttcagcgcgcaggtgctggccaggcgcaaggagttcgggctgctcgcgcatctgggctttacgcggcggcaggtgctggcggtggtggcgggcgaaggcgcggcatggaccgcaatcggtgccgtggccgggctcttgctcggcctcgcggtgtcggtggtgctggtgaaggtcgtcaatccgcagagctttcactggacgatggatttgctggtgccttgggagaggctgctggtgctttgcgctgcagttgtggccgcggggacggtgactgcgtggatggctgggcgtgcggctgccgggaaggatgtcgttcttgctgtgaaggaggattggtagttttttgtcttcccgaggccgggtctcgccccggcctcgggaaacaaacaagacccttgtagactgccagcgatatgcagcaaacccctaccagctggcaaggcacagccatccgccgcatcgaagccgactaccaccgcagcgccgacacgcacctcatcccgctgccgctgccaacgctcgccgcccagggcatcgacctgtacctcaaggacgaatcgacccaccccacaggcagcctcaagcaccgcctcgcgcgatctctctttctctatgcgctgtgcaacggatgggtgcgcgaaggcaccaccatcgtcgaagcctcgagcggctcgacagcggtcagcgaagcctatttcgcgcgcctgttgggcctgcccttcatcgccgtgatgccgcgcagcacctcgcccgagaaagtggcgcaaatcgccttctatggcgcgcgctgccacttcgtcgaccacgcggcgcaggtctacgaagaggcgcgtgcgctcgccgagcagaccggcggccactacatggaccagttcacgtatgccgagcgcgcgaccgactggcgtggcaacaacaacatcgcagaaagcatgttccagcagatggcgcgcgagcggcatccggtgccggcctggatcgtggtgggcgcgggcaccggcggcaccagtgccaccatcgggcgctatgtgcgctttcgctgccacgacacgcaggtgtgcgtggccgaccccgagggctcggtgttctcggcctaccaccgcacgggcgacccgacgctgacggcggcgggctcgcgcatcgaaggcatcggacggccgcgcgtggagccgagcttcatccgcacgctggtcgatcgcatgatcgaagtacccaatctcgattcggtggcggcgatgcatgcgctctcggcgctgctggggcgcaaggtcggcccttcgaccggcaccaacttcatcggtatgctggccattgcgcgcgagatgcgcgcggctggccggcagggttccattctttcgctgctgtgcgacgcgggcgaacgctacctgccgagttatcacgatgcggcctgggtgcaaaacgcattcggcgacatcggaccgtcgcagcagcgcatcgacgcgctggttgcggagtgatgccgccgcctgccttcctcagtctctcccggcgcagcctgctgctcgcggcgctggccgccgcagcgcccgcaagctgggcattgcctgcgcgcgcgctgcagttcccgcgcgacttcggcagccaccccgaactgcaaaccgagtggtggtacatcacgggccacgcgaagacgccggcgggacgcgagttcggcttccaggtgacgttcttccgctcgcgcgtcgatgcggcgcaaggcctgcgctcggccttcgcggccaagcatctcgtgttcgcgcacgcggccgtcaccgacctcgaaggccgcgtgctgctgcacgaccagcgcatcgcacgcgcgggcttcggcattgcgtcggccagcgaaaccgataccgacgtgcgcctgcgcgactggtcgctggtacgcggggcggacggcagctattgggcgcacatcccggccggcgagttttcgatcgacctgcgcttcgcgcccacgcagccggtgctgctgcagggcaaggccggactctcgcgcaagggcccggaagaggcgcaggcgagctactactacagcgaaccccagctcaagacccggggcaggctgacgctcaggaaaggccaggccttcgacgtcgacggcaccgcctggctcgaccacgaatggagcgaggcgctgatgcatcccgacgccgtgggctgggactggatcggcatgaacctggatgacggcagtgctctcaccgccttccgtttgcggcgcagcgacggcggtgcattgtgggcgggcggctcttttcgcacacgcgacggtgcgctgcgcatcttcggcagcgacgaggtgcgcttcgacggtgcgggcgcgtggacgagtccgcgcacgcaggcgaagtacccgacgcagtggcgcgtgcagaccccatcgggcagcttcgaggtgcgcgccctgctcgacgaccaggagctcgacagccgtggctccgccggcggggtgtactgggaaggcgtgagcgatctgctcgatgcacaggggcgccgtgtcggccgcggctacctggagatgaccggctacgccgcaccgctgcggctctgaaagcccgcgcagcctcctcccgtcatcacgctgtcatgccgagcccctgaactcggctttcgacattgcacgacggccgtgcgccaaggctcgaatgaagaagaacagaccccggatcatcgcgctgctgatgcttgtgctggccgctgcagcaggcatcgcatgggcattcgcagccgcgcggcctgcctcgccggcaaacggcgccgtgctcgaaatccgctggcatggcaacggcatcatcctgcagggcgcggtgagagatgcggccacgcagcacgcactggtcgaaggcgcaaccgcacggctcggcggcgaggccgaccaggtggtggactggctggacatcgcgcccgaggcgctgcccgtggcggacgccgcggcacttgccagcctcatccgggtggggcaagagggctggcatctgcagcggcgagccgccagtggatggctcgccgtgcagtcgcccgacgacgcgcgcagtgcgcaggccggcgagctgctgcaacgcgccttcggccccgacgtggccattcgcctggttcccctgccctgagaactcgaacgaaaaaaaggcggcggtcacggcgacgtcatctgccatcttcagcatgcgctgcattccacaaagaggagaggctcatgcacgcatcgttgaaaccacgtctcgcgctggcggggattgccctggccgcgctgtccgcctgcggcggaagcggtaattcgaacggcttcattccgttcttcccgtcgcccgcaccggctcccgcgccgccagccccgccgccgcccgccacgcccggcagcatggaggtgaagctcattgccttcaacgacctgcacggcaacctcgagccgcccaggctgtccatcaccgcaccggccaagagcggcggcacggtcgcggtgcccgccggcggcgcggcctacctcgcttcggccattgcgtcgctcaaggccaaaaacgagaacaatgccgtggtgtccgccggcgacatgatcggtgcctcgccgctggtgtcggcgctgtttctcgacgagccgaccatcgaggccgtgaacgagatgaagatcgacttcaacgcggtcggcaatcacgagttcgacaagggccagaccgaactcctgcgcatgaagaacggcggctgcgccaagaacacgccgctggagccctgccgggtgaacaaggcgttcccgggcgccaacttcggcttcctcgcggccaacaccgtgaagaccgacggcaccacgctgtttcccgccacgggcatgaagaccttcacgaaggatggggccacggtgaaggtggctttcatcggcatgaccctcaagggcacgcccagcatcgtgacgccgtccggtgtcgcgggcctgagcttcaaggacgaagccgacacggccaacgcattgattccgcagctgaaggcccagggtgccgacgccatcgtcgtggtggtccatgaaggcggcacgaccacggtgggctacaacgacaagagctgcgccggactgagcggcgacatcctgccgatcctcgacaagctcgacgcttcggtcgacgtggtgatctcgggccacacgcaccgctcgtacatctgcgactacgcaaagacgaacccggccaagcccttcctgctgacgagcgccggccagtacggcaccttgctgaccgacatcaacctgacgatcgacacgcgcacccgcaaggtcacggccaagtcggccgacaacgtgatcgtccagggcgaggcctacaccagcggcgccaacacgattgcgctgaccgaccaataccctgcgttcggcaagaaccagcaggtggccgcgctcatcagccagtacctttcgatcgccgccccgctggtgcagcgggtggtgggcacgctctcggccacggcaacgcgcacgcagaccgcttcgcgcgagagcgtgctcggcaacctgatcgcggatgcgcagctcgatgccaccagcgccagcaacaagggcggcgcgcagatcgcgttcatgaatccgggcggcgtgcgcgccgacctcgtgccggccggcgacggcagcgtgacctatggccagatcttcagcgtgcagcccttcggcaacagcctggtggtgaagacgatgaccggcgcgcagatcaaggccgtgctggagcaacagttcaacagcggcaccaacacggtcgcttcgcccagggtgctgctgccttcgcgcagcctgagctacagctacagcctctcggcgcccgccggctcgcgcatcagcagcatggcgctcaacggcaccgcgatgaccgacggcacgagctaccgcgtgacgatgaacagctttctggccaccggcggcgacaacttcacggtgttcaaccagggcaccgacacgctcggcggcgaccaggacgtggatgcgctggaggcctacatcaaggcgaacagcccgttggcgccgccggcgaccaaccgcatcaccgtgctgccctgaacgggcctgtcccagatgcaaaaaaggcggacactgtccgccttttttttgttgcatcagaccttgctttttcggcggtcgatgaaggcgatgacctcgcccatgatccccttgcggaatgcgagcacgcagatcacgaagatcaggcccgtgaccatggtcaccgattcgccgagcgtgttgaaccagtcgacgccggtcacgcgtgccatgaaggtgccgaagtcgcccaccttgttctcgagcagcacgacgaccgccgagcccaccagcggacccgagagcgtgccgaggccgcccaccagcgtcatcaggatcacgtggcccgatgcggtccagtgcacgtcgctcagcgacgcgaagccgagcaccagcgtcttgagcgagccggccaggcccgacagcgcggccgagatcacgaaagcgagcagcttgaagcggttgacgtcgtagcccagcgaaatggcgcgcggctcgttctccttgatgcccttgagcacctgcccgaaaggcgagtgcacggtacgcgcgatcagcaggaaggccgccaccacgatcaccagcgccacgtagtacatcgtcaggtcgtcgcgcagatcgacgacgccgaacagcttgccgcgcggcacgctctgcaacccgtcttcgccgcccgtgaagggcgcctgcagcacgacgaaatacatcatctgtgccagtgccagcgtgatcatcgaaaagtagatgccctggcggcggatggccagccagccgaaaaccagccccagcagcgcgccggccagcgtgcctgcgatcaggccgatctcgggcgtcaggtgccagaccttgagcgcctggcccgtgaggtaggcggcgccgcccagaaaagcggcgtggccgaatgacagcatgccggtgtagcccagcagcaggttgaaggcgcaggcgaagagcgcgaagcacagcaccttcatcacgaacaccggatagaagccgatgaagggcgcgacgacgagcgccagcagcagcaccccgtagacgacgagcgatattttcttcatggatttatttctcgctgccgaacaggcccgcggggcggatcagcagcaccacgaccatgatcacgaagaccacggtggccgaagcctcgggatagaacaccttggtcagcccttcgatcacgccgagcccgaggcccgtgaggatggcgcccatgatcgagcccatgccgccgatgaccaccaccgcgaacacgatgatgatgaggttctgccccatcagcggcgaaatctggatcaccggcgcggccagcacgccggcaaaggccgccagcgccacgccgaagccgtaggtcagcgtcaccatcagcggcacgttgacgccgaaggcttccaccagccgcgggttctcggtgcctgcgcgcaggtaggcgccgagccttgtcttctcgatggcataccaggtggcaaagcacacgaccagcgacgccacgaccacccaggcgcggtaattgggcaggaacatgaagcccaggttggtgcctccgctcagcgcctcgggcgtgctgtaggcgaggccggacacgccgtacaccgagcggaagccgccctcgatcagcagcgtgaggccgagcgtgagcagcaggccgtagaggtggtcgagcttgtagatccagcgcagcagcagacgttcgatcagcacgccgaacaggccgacgatcaagggcgccaccaccagcatgacccagtagtcgatgttgaagtaggtcatcgccatccacgacagcaccgcccccatcatgaacagcgcgccgtgcgcaaagttgatgacgttgagcagaccgaagatcaccgccagccccaggctcaggatcgcgtagaacgacccgttgaccagccccaacaggagctggctcaacagggcaggcatggaaatattcatcgtggaaacgaggttcagataggcgtcattgacttcgcgtgagggccgctgcgcacggccgcccgaagcggccgaacaacagttacttccagagtgcgcaggtgctctcttccttggtcgtgtagacctggtcgcccggcaccttcttgatgatcttcagcaggtcccacgggcccttggattccgaaggcttcttgacctcggccagcagcatgtcgtgcaccatgcggccgtcggggcggatcacgcccttggcgtagaagtcgttgatcggcgtcttcttgaggtaggccatgaccttgtcggcgtcggtgctcttcaccgcctcgacagccttcaggtaggtcatggtggccgagtagtccgccgcctggatgtcggtcggcttgttcttggtcttggcttcgtagcgtgcggcccacttgcgcgactcgtcgtccgcgtcccagtaccagctggtcgtgtgcagcaggccctgcgtggccggcaggcccaggctcttcacgtcggtcaggaacaccagcaggcccgcgaccttcatcgacttgtcgatgccgaattccttcgacgccttcatcgagttgatgaagtcgccgccggcgttggccaggcccagcacctgcgccttggagttctgcgcctgcagcaggaaggacgagaagtccgaagcattgagcggtgcccgcaccgtgcccaccaccgtgccgcccttggccttgacgaccttggcggtgtcgccctcgagcgcatggccgaaggcatagtcggccgtcaggaagaaccagctcttgccgccggtgtcgaccaccgcgccgccggtgctcttggccagcgcgacggtgtcgtaggcgtagtgcacggtgtaggggctgcactgcgcgttggtcagcgccgaggtggccgcgccattggtgaagaacacgcgcttcttctcctgagccaccttggatgtggccagcgcgacgcccgaattggtgcccgcgaagatcatcgtggcaccggcggtgtcgatccattcgcgcgccttcgaggccgcgatgtcgggcttgttctggtggtcgacgctcagcacttccacgggctggccgagcaccttgccgcccatgtcgtcgatggccatctggatcgccgctgcgccgcccttgccttccaggtcggcgtacaggcccgacaggtcgctgatgtagccgatgacgaccttctcctgcgcctgcacggcatggctggcgagacccgcggctccgagcatgagtgcaatgattttgagcttgttttgcatggtgtctcctgggatggttgagagagtcaacggaaaaaaagcgatggcatggccgcggctacacgcccagcagctcgctgagcacgggcatcttggcgtcgagctccttggcgccgaaggcctcgaccatgcgaccgtgctccatcacgtagaagcggtcggccagcggtgcggcgaagcggaagttctgctccaccatcacgatggtgtagcccttggcgcgcagggtgtggatcatccgggccagcgcctgcacgatcaccggcgccaggccttcggaaatctcgtcgagcagcagcagcttggcgccggtgcgcaggatgcgcgccaccgcgagcatctgctgctccccgcccgaaagccgtgtgcccgggctgttgcggcgttcggccaggttgggaaacatctcgtagatctcggccaccgacatgccctgccccgcacccttgagcgccgggggcagcatcaggttttcctccgccgagagactggcgaagatgccgcgctcttcggggcaatagccgatgcccaggtgcgcgatgcggtgcgtgggcatgccaatggtctctttgccattgacctcgatgctgcccttgcgcgtgccggtcaggcccatgatggcgcgcagcgtgctggtgcgcccggcaccattgcggccgagcagcgtgacgacctcgccgggctgaacgaccatgtccacgccatgcagcacgtgcgattcgccgtaccaggcttgcagccccttgatctggagtgcggcggtcatggagcctcctgccgggccgccccaaaggaggctcgcgccccctcggggggcagcgcatacacgaagtgaggagcgtgggggttcatgtcagtgagccccctgcagctggccgtcggtggtgcccatgtaggcttccatgacctgggggttgttcgaaacctcggcgtaggggccttcggccagcacggcgccgcgctgcagcacggtgatggtgtcggcaatggtcgacaccacgctcatgttgtgctcgaccatcaggatggtgcggcccgcagacacgcgcttgatgagttccgccacgcggtgcacgtcctcgtggcccatgccctgcgtgggctcgtcgagcagcatcagctcggggtccatggccagcgtggtggcgatctcgagcgcacgcttgtggccgtagggcaggttcacggtgagttcgtcggcctggtcggccaagccgacttcggcaagcagttcacgggcgcgcgcatcgagcggcttgagcgtcttctcgctcttccagaagtggtacgaggtgccgagcgcgcgctgcagtccgaggcgcacgttctcgagcagcgtgagatgcgggaacaccgccgagatctggaacgagcggatgatgccgcgccgcgcgatctgcgccggccgctcgccggtgatgtcgtgcccgttgaaaagaatggtgccggcggtcggctcgagaaacttggtgagcaggttgaagcaggtggtcttgccggcgccgttgggcccgatgagcgcgtggatcgatccgcgcacgaccgacaggttcactttgctgaccgccgtgaagcccttgaattccttggtgagctggcgtgtttcgaggatgacgtcgctcatctcgcgaagtcgcccgggttcaggaaagatatgtcggtcatgcggtccatctcgatgcgccactaccgagcgcggcctgattgttcgtgggtgcctcccgcttgcatactggggcaaatgcctatgctgcagtgcaacctgtgcgcacccgcggtccctggcatcgggcaactgtcgtcacaatgacaatgactcgccggatctgacctctacgcccatgccgaacttccgctcgcccgatttcctgacggaccacatcctgcacacgctggctttctacgcgccggtcagccgcgactcgtcaggcggcttcttccacttcttcaaggacgacggcacggtgtacgaccggcgcacgcggcaccttgtgagcagcacgcgcttcgtcttcaaccatgccatggcctaccggcgcttcggcaggccggaagaccttgcagccgcgcgccacggcctggctttcgtgcagcatgcgcacgcgcggccgggcggcggctacgcgtggcagatcgactggcacgacgcacgcgccacggtgcaggacgacaccaaccattgctacggccttgccttcgtgctgctcgcgcatgcgcacgcgctgatggccggcatcggcgaagcgcgcgcggggctggggcagacctgggagttaatggaacagcgtttctgggagccgcaacatgcgctctatgcggacgaggccagcgccgattggcatgtcaaaccctaccggggccagaacgccaacatgcacgcctgcgaggcgatgctcgccgcgttcgaggccacgcaagaggcgcgctatctcgatcgtgcgctcacgcttgcggaatcggtcacgggccggcaggccgcgctggccgacgggctggtctgggagcattaccgcgaagactggtcgatcgactgggactacaaccgcggcgacaagagcaacatcttccggccctgggggttccagaccggccacctcaccgagtggaccaagctgctgctgcagctcgagcgcgcgctggttgccgcaggccgcgaggcaaagtggatcgtgccgcgcgcacggcacttcttcgacatcgccatgctgcgcggctgggacgccggcaacggcgggctggtctacggattcggccccgatggcgcggtgtgcgacggcgacaagtacttctgggtgcaggccgagagctttgccgccgccgccctcctggccatgcgcaccggcgacgccggctactgggcctggtacgaccgcatctggacctacagctgggcgcacttcgtcgaccaccggcatggcgcgtggtatcgcatcctcacgcccgacaaccgcaagctgagcgacgagaagagcccggccggcaagaccgactatcacaccatgggtgcgtgctatgacgtgctgcgcgcactcggcgcctgaagaagcgcgcctttcttctccgcgagcttggtgcgagcctagtgcgccccggccgcggcgtcgccgcccgcaccgccgcgctgcggccttgccagccacaccagcggaatcagcagcaggaacaggattgccgatgcatagaagatgtcgttggtggccagcatgaacgactgctggtcgaccacgcggttgacctgccccagcacctgctccgtgctgaggccgctgctcgtcaggccggacatggcgctggccgctgcgttgttgcccaggttcaccgactccgccagctgcgaatgatgcagcgccgcccggttctcccacagcgtggtggtgatcgacgtacccatggcgcccgcggtgatccgcaggaagttcgacaagcccgacgcggccggaatgcggtcgggcgtgaggcccgacagcgtgatggtcaccagcgggatgaagaagaacgccatcgcaatgccctggatgatcgtcgggatgatgatcgtcacgaagtcggcctgcgtgttgaagttcgaccgcatccacagcaccagcgcaaacaccaggaacgagaaggtggcgtagcggcgcggatcgatcttggcgaccgtgagcccgaccaccggcgagaagaggatggcgagcagcccgaccggcgccatgatcatgccggcctgtgtggcggtgtagcccatccactgctgcagccacagcggcagcagcaccacgttgccgaagaacaggccgtaggccacggcggtggccaccgcgcccgaccagaagttgcggcgcttgaagagcgacaggtcgaccaccggatgcttgtcggtcagctcccagatgaggaagaacgcgaagccgaccacggcaatgaccgccatcgtgacgatctcgggcgaatggaaccagtcgagttccttgcccttgtcgagcatgagctgcatcgagccgacccacagcaccagcagcgcgagtccgatggcgtcgatcggcaccttgtgcgtggtgctttcacgcttgcgatagagcgcccacgtgatggccgccgccacgatgccgaccgggatgttgatgtagaagatccacggccacgagatgttgtcggtgatccagccgcccagcagcggccccatcaccggcgcgaccagcgtcgtcatcgaccacatcgccatcgcaaggcccgccttggcgcgcggatagctcgacagcagcagcgtctgcgacagcggaatcatcggaccggcaacgaagccctgcagcgcgcggaacaggatcagcgtcgtcatgttgggcgccaggccgcacaagagcgaggcgatcatgaacaggatcacgctggccatgaacagccgcacctggccgaagcgctgggtcatgaaacccgtgagcggcaccgcgatggcattggccaccgcgaagctggtgatgacccaggtgccttgcgtggtgctcacgcccaggtcgcctgagatggccggcagcgacacgttcgcgatcgacgagtcgagcacgttcatgaaggtggcggccgaaagcgcgatcgtgccccagacgcgggcggcgccctcgagcggcggatgcgcaacgtacgcgggagcagcagtggccattggctttgcctcgggaaccgttaacggcgatcagccgggatgggattgcgaagcagcttgcgcagcggtcccggcattggttgccggcgtggccgagcggcccgttgccggtgccgcggaacctgccggcgcaccgcgcccgagattcgcggccacgatgcgatcgacttcggcgtcggcgccctggtcgagcttgctgtagacctgcgtctgcgacatggcggtggcgcgcggcgcatcggccagcatcttgccgcccttctgcgagatgtcgatctcggcaaccatcgagaggccgatgcgcagcggattggccttgagctgctccgggtcgagcgcaatgcggaccggcacgcgctgcaccaccttgatccagttgccggtggcgttctgcgcgggcagcagtgcgaatgcgctgcccgtgcccacgcccaggccggccaccttgccggtgtattccaccttcttgccgtagacgtcggccttgagcttcacgggctggtcgatgcggatgttgcgcagctgcacttccttgaagttggcgtcgacccacagctggttcagcggcacgatcgacatcatcggcgtgcccgccgccacgcgctggccgagctgcacggtgcgcttggccacgtagccgtcgaccggcgccggcagcgccacgcgctgcgtggcgaggtaggcctcgcgcaccttggcggcggcggccagcacgctcgggtgccgggccacgctggtgccttcggtcagcgactggttgctggccagcgcttcgcgcgcggccaccacgccggcctgcgccgcagcaagctggctcttcgcattgtcgagcgacgtctcggcgtggttgagttcttccttcgagaccgcgccgttgcccgacagcgcgcggcggcgctgcagatcgtcctgcgccttggcgatgtcgctctgtgcccgggcgatgtcggactggcgcagcgtgacctgcgcggccagcgagccgttgttggcgtacagcgtgcgcacctggcgcacggcctgcgccagcgcggcctcggcctgctcgagcgccaccttcgcatcggccgggtccagctgcaccagcggctggccggccttcacgaagtcggtgtcgtcggcgttgatggccatgacggtgccgccgatctgtggcgtgatctggatgacgttgccctgcacgtaggcgttgtcggtgtcttcgtagtggctggcaaccagccattcgtagaggccccagccgccaccggcgacgatgaccaccgcggcgagcgcggtcagcgcgcggcggcgcttgccgttgccggcgggttctgcgggtgctgcggtggaggctgcggaagcagcgggcgtcggagtgttgttgtcgctcatgatgaagttctttccgaagacgaagaagtcggttcagttcagttcagtgcggacggcgtgggcgccgcggcggtggcggtcgccggcggctgccagccgccgccgagtgcgcgcgccaggcccacctgcgtgtcgagcgcgcgggcggcaagatcgaccgccagccggcgctgcgcgagcacggaggtttccgccgtcagcacgttgaggtagttgccgaggccagcgcggtagcgctgcaccgcgatgtcgtaagccccttcggccgccgtttgcgcggcgcgctgttcggcctgctggcgggcgatcgactgcgcgctcgacacctggtcggccgcgtcacgcaccgcgtccagaacggtggcgttgtagctctcgatcgcgccgtccaggtcggccgccttgccgcgcaggttggcgcgcagccggccgccttcgaagatcggcaggtggatggccgggcccacgccccactgctcgctgcccgacttgagcagcttgccgaatcccaggctctggaagccgacgaaggccgtgagattcacgttgggatagaactgggtcctggcattggccacgtcgctggtggcggcctcgacgcgccagcgcgcggcggcaatatcggcgcggcgccccagcaggtcggccggaatgttggcctgcagcgcgatgggcttgacggcctccagcatcggaggcttgagcgatgcggacacattgggctggcccacgagcgcatcgagcgcgtgctgctggagcgcgatctgctcgttgagcgcttcgatctgctggcgcgcttcgggcagcccgccctcgctctggcgcagttcgaggcgggtgtccaggcctgcggacacgcggtcgcgcacgagcttgagcgtttcgtcgcgctgggccagcgtgcgccgggccacgccgagctgctcgttcaggcgcgcccactggaagtagctgcgcgccacgttgctggccagcagcacgcgcgcggcgtcggcatcggccgccgcggcattggcgctgccgatggcggcttcgagcgcggtgcggttcttgccgaagaagtcgagctcccagcttgcgccgagctgcagcaggccgatgttctgcgtcgagccgcccagtggtgcgggatagatgtagttgctgttgaacttctgtcggctcaggtcgagttcgccattcaccttgggcttcagggccgactcggcgatgtccgcggaagcctgcgcccgcgcgaggcgcgcgcgtgccacctggagattcggattgccggccacggcctggtcgaccagcgtgtcgagctgcgcgtcgccgaaggctcgccaccattggctgtcgacgctggacacggccgcggcgctgctgtcggcagcaatgccgagtgacgaagcatcgcgaagcctggcctccgagccgatgccggccatgtcggcacaaccggccagcgcgaccacaaggagtgcagcagcgacgacgggggtgcggcgcaccacgcgcgcggcaagagattcagtcatttttttctccacgggctgcgagggcttgcgcgttgtcgaggatgcggcgcaggtaacccttgagctgttcccactcttcgttggtgaaacccgccaggtgctcgttctgcacgcggctcagcacgtgcgggacttccttggcggcggcgcggccctcttcggtgagttcgatgttgaccacgcggcggtcttcgagcgagcgaacacggcggcacaggcccttggcctcgaggcggtcgagcaggcgcgtcatggcgccggcgtcgagctcgcaggcgcgggccagttcggccaccgtggtggccgcgccgacgtgcagcttgtacagcggcagccactggggaaaggtggggccgccgggctcgctcatgcgggtttccaccgcctgggccacggcgctcaatatgcgccgcatcaaatacccgatgctttcctcggcctggtaggtctcggcacggtagaagtccgccggccggagcttggggtcgccggaagctggcgggactttcggagtatctgtatcgctcatggccagattattaattgcccaagcaattattgtcaaggctgcctttgtggtggcaagggtcggtagaatccgcgccatggcttcttcccctctgtctactccagccaagggctcgccccggtcgctctcgggcttgagcccttttcttcggccataccgcgtccagatcgtgctggcgggcatctttctggtgttcgcggcaatcacgacgctggtctttccgctggcgctgcgcagcctgatcgacggcggactcgtcagcaccgacaagggcgcccagaccatggcgctgcgcgagcacttcggcgctctcttcgcggtggccgtggccctgggtcttttttcagccgcgcgcttctacacggtgagctggctcggcgagcgcgtcacggccgatctgcgcaatgcggtgtacggccacgtgctgcgccagagcccggcgttcttcgaaaccacgcagaccggcgaagtgctgtcgcgcctgacggccgacaccacgttggttcagacggtggtcggatcgtcgctgagcatgggcctgcgcaacgcggtcatgggcgtgggcgccctggcggtgctgatctggaccaacccctacgtgatggtccaggtgctgggcatcctggtgctggtggtgctgccgagcatgtggttcggccggcgcgtgcgcaagctctcgcgcgccagccaggaccgcgtggccgactcgagcgccatcgcggccgaggtgctcaatgccattccggtggtgcagagctacacggccgagtcgcgcgaagccggccgcttcaatgcctcgactgaaaatgccttcaggaccgccgtgcgccgcaccaaggcgcgttcggtgctggtggccttcatcatcatcgccacctcggcagcgctgctctggggcctgtaccagggcacgcaggccgtgctgcgcggcgacatcacggccggccacctgggccagaccgtggtctacgtggccattctcgcgagcgcgaccgccgtgctcggcgaggtctacggcgacctgctgcgggcggccggcgcaacggagcgcctgatggaactgcttcatgcgccggcggcaatcgtctccccacgggatccggcggctgcgcccgttcccgtggcgggcagcgcggtcaagttcgaggccgtgacctttcactacccctcgcggcccggcacaccggcgctgaagaacttcagtctcgacatcgcgcccggcgaaacggtggcgctggtgggctccagcggcgcgggcaagagcacggtgttccagctgctgctgcgctactacgacccccaatcggggcgtctgctgctcgacagcgtgccgctggcctcgctcgcgctgtccgatctgcgcacccgcatcggcctggtgccgcaggatgccgtgatcttctcggccagtgccttcgagaacatccggtacggccgccccgacgccaccgccgacgaggtgcatgccgccgcccgcgcggcctttgcgcacgactttctgcaggcgctgcccgagggctacgacaccttcctcggcgagcgcggggtgcgcttgtcgggcggacagcgccagcgcatcgcaattgcgcgcgccattctcaagaatccgccgctcctgttgctggacgaagcgacgagcgcgctcgacgcggagagcgagcgcatggtgcaggcggcgctcgaatcggcgatggaaggccggaccacgctggtgattgcgcaccgcctggccaccgtgcagaaggccgaccgcatcatcgtgctggaccatggcggcatcgtcgagcatggaacgcatgccgcgctggtggcgcaaggcggggtgtatgcccgcctggcggcccttcagttcacggcttgaatctgctgcaggagcagcgagagcggcaagggcagcagcggactactgcagcgtttccttgagcgcggcgggtatcggcagcggcatcaccggaatgccttcttcgagcagcgcttcggtctgctcgcgggtggcctggccgcggatcccgcgctcttcggcttcgccgtagtgcatcttgcgtgcctcgtcggcaaagcgctcgccgacgtcttcggtcttcgcgagaacctcgcgcacggcgcgcatccagcgtgcctcgggagacatttcggcggagagctgcgccttggtatccggggcctgggcgggaggtgcggcggcctccgcgggcgccttggcgttgccgagattgaggcgcggcgcactcaagagcttgacgatgcgcgtgtcggcacagatcgggcactcgaccaggccggccgagagttgggtttcaaacgcctcgttggacgcaaaccagccttcgaagccgtggccatgcgagcagcgtagatcgagaaccttcatgcgcggattatcccgcgccgccttgcgcagcgggggcctgccaatcgagttcccatgcgcccgaaaggacgttttgcagccagagcgcgcaagtgagcgacttggcatcggtgatcgtgccgtcgcggcaccagccggccacttcctgcggcgtggccgtgaacacgtcgaggaactcgccgtggtcgagctggcgcgtgccgagcgaaaggccgcgcgcaaagtagatgtggatgatctcggtggaatacgccaccgccaggtgcatggcgccggcatatgcccattcgcgcgcggtgtagccggtttcctcgagcagctcgcgctggccgcaaaggaacggatcctcgcccgcgtcgagcttgccggccggaaactcggtcatcacgtgcgcgaccgggtagcggtactggcgctccagcaccacgcggccgtcgtcgagcagcggaatcaccaccaccgcacccggatggatcacgtactcgcgcgtggcggtgtggccgtcgggcaggcgcacggtgtcgcggcagacctggaggaaattgcccttgaccagcacctcgctggcggtgcgttcttccttcagatgcgattcggccatggaggtggaagtcatgtcagtgcctgtgcttcatgaggtagcgccaggtaaaccctggaaatgccagcacgatgaaaagcgcgccggtcaccgcgtagaactcccaaccctgcggggcgatctgccctgccctgcgttcgaacagcagccccacgccgccggcaacgaagtacagcaccaccagttcggcaaggcggatcgccagcgacttggggtgggcttgcagcggtatggcaccaaacagccggtcgttgaggaacgggaggttggccgccagcagcgccaccacgagcacgacccagaccgaagcggtttgcgacaccgtgctcaggccgggatcagttggccagcgtcgccacgatggcgttggcgcacagcgtcatgaggccgccgggaacgatgcccagcacgagaatcagcaagccgttgatcgacagcacggtgcgcacgtcgcgcggggccgacacggtgctggccgtgacgggcgcgtcgaaatacatgaccttgaccacgcgcaggtagtagaaggcgccgatcagcgacgtgatcaccgcgaacacggccaacccgatgtagagcgcctggcccgacgcgatcagcgcctgcaggaccgccagcttggcatagaagccgaccagtggcggcaggcccgcgagcgagaacatcgcgatggccatcacgccggcatacagcgggctgcgctggttcaggccggccaggtcggtgatctcttcgctttcgaagccctcgcgcgccagcagcaggatgatgccgaagctcgccagcgtggtcagcacgtaggtcacgatgtagaacatcgaggcgctgtacgcgaactgcgcgttgtaggtgttgccgttgaccacgcccgccaccaggccaagcagcatgaagcccatctgcgcgatggtcgaataggccagcatgcgcttgaggttggtctgcgcaatggcggccaggttgcccaccaaaagcgaggcgatcgccagcagggccagcatctgctgccagtcgatggccagcggcagcagcccttccaccagcaaccggatgatgatggcgaaggcagccagctcgggcgccgcgccgatcagcagcgtgacggccgtcggggcgccctggtacacgtcgggcacccacatgtggaaaggcgcagcccccaccttgaaggccaggcccgcgacgatgaacaccaggccgaacaccagcacctggtggttcaccttgccgcttgcgatgatcttgaacacttcgttcacgtcgagcgaaccggtcgcgccgtacagcatggagaggccgtagagcaggaagccgctggccatggcgccgagcacgaagtacttcatggccgcttcgcttgccaccgcgttgtcgcggcgcagcgccaccagcgcgtagctcgagagcgtgagcagttcgaggcccaggtagatcaagaggaagttgctgcccgagatcatcacgaacatgcccagcagcgcgaacatgctgatggtgaacatttcgccgccgcgcagcatgccgcggtccgccgcgtagggccggccgtagaccagcgtgaccatcagggccacggtcgcaaagcacttgagccagttgcccatggggtcgctcacgaccatgccgccgaagccgtagaccgtcttgccgtcgttggcggcgatgccggtcaagacggcgaccacggccagcgtgagcagcgtcaggatgtaggtgcgcgtgcgctgcgcactggtgctcgacaggtcgaccagcgcaatgatgcaggccatgaccagcagcacgacttcggggtagatcgcaatccagctgagtttgtcaatcatctcgttctcttcttcagcgtggaatcaggggagtttcgaagttgccacgtggcgcaggagctccgtcacggaagcatccatcgcagcggtgaacggcttcggatagatacccatccacagcacggcaatggccagcagcgacagcatcaggaactcgcgggcattgatgtcggtgagttccttgacgtggtcgttgccgaccgggccgaggtacacgcgcttgtacatccagagggtgtaggccgcaccgaagatcagcgccgtggcagccccgaagccgagccagaagttggctttgaccgcgccgaggatgaccatccactcgcccacgaaaccggcggtgcccggcaggccgcagttggccatggcaaacagcagcgcgaacgcggcgaacttgggcatggtattgaccacgccgccgtagtcggcgatctggcgcgaatgcacgcggtcgtacagcacgccgatgccaaggaacatggcgcccgacacgaaaccgtgcgcaatcatctgcacgatgccgccggacacgccgagctcgttgaagatgaagaagccgagtgtgacgaagcccatgtgcgcgacggacgaatacgccacgagcttcttcatgtcttcctgcaccagcgccaccaggccgacgtagatcacggcgatcagcgacagcccgatcatgagccaggcccattcgtgcgaggcgtcgggcgcaatcggcatcgagaagcgaaggaagccgtaggcaccgagcttcagcatgatggcggccagcacggccgagccgccggtgggcgcctcgacgtgcacgtcgggcagccaggtgtggaccggccacatcggcaccttgaccgcaaaggcggcaaagaacgcaaagaacaggaaggtctgcgccgtggaacccagcggcagcttgtgccagctcaggatgtcgaagctgccgcccgacttgttgtacaggtagatcagcgccaccagcgtcagcagcgagccgagcaaggtgtagatgaagaacttgaaggccgcgtagatcttgttcgggccgccccagatgccgatgatgagatacatcggaatcagcgtggcttcgaagaacacgtagaacaggacgccgtcgagcgcggcgaacacgccgatcatgaagcccgagagaatcaggaacgcggccatgtactggttgacgcgctcggtgatcacttcccaggccgagatcacgaccaccacggtcgtgaacgaggtcaacagcaccagccagagcgacaggccgtcgatccccaggtggtagtggacattgaagcgcgcgatccagctggctttttcgacgaactgcatcgcggcggtgccgttctggaagcccgtgtaaagcggcacggtcaccaggaaactcaggatcgcgccgaccagcgcgacccagcgcacgccgcgggcgtgctcgtcacggccgaacgccagcagcgcgacaccgaatgcgattggcacccagatggcaaggctcaacaaacccatttttctttttctccagcgctaaagctcagcgtttgaaccagacgaagtacgtcatcaggatgaagatgccgagcagcatcgcgaaggcgtagtgatagatgtagcccgactggagccagcgcaccgcacccgagatgcggccgacgaccttccatgaaccgttgaccagggcaccatcgatcagcgcctggtcgccgcccttccacaggccggtgccaaaggcacgcgtggcacgggcgaggacgttctcgttgaaccagtcgaggtagtacttgttgtccagcaggcgatagatcgggccgaaggcgcgcttgatcgcggccggcagcgccggattgaccatgtacatgtagaacgagagcaccacgccggccagcgccagccagaacggcggcgccgtcaggccgtggatcgccatggccagggggccgtggaaggcttctccgagctccttcatggcatggtgcttgttggcgtcgaccgcgatggcgcccttgaagaactcgccgaagagcatcggctcgatcgtcatgaaaccgatcaccacggacgggatggccagcagaaccagcggcagccacaccacccagggcgattcgtgcggcttgccgtgatggccatggttctcgtcgtgctccgcatgttcgtcgtggtggtgcgcgtcaggattctggtcgtagcgctccttgccgtggaacaccaggaagtacatgcggaacgaatagaacgccgtcacgaacacgcccgccagcaccgcgtagtaggcgaactgcgcgccccacaggtggctttcgtgcaccgcttcgatgatgctgtccttcgagtagaaaccggcgaagagcggcgtaccgatcagcgcgagcgaacccacgagcgacgtgatccaggtgatcggcatgtacttgcgcacgccgcccatccagcggatgtcctggttgtggtgcatgccgatgatcaccgagcccgcgccaaggaacagcagcgccttgaagaaggcgtgcgtcatcaggtggaacaccgcgaccgaataggccgatgcgccaagcgccaccgtcatgtagccaagctgcgagagcgtcgagtacgcgaccacgcgcttgatgtcgttctggatgatgccgaggaagcccatgaacagcgccgtgatggcaccgatcaccaggatgaagctcaaggcggtgtcgctgagctcgaacagcggcgacatgcgcgccaccatgaagatgcccgccgtcaccatggttgccgcgtggatcagcgccgagatgggggtcgggccttccatcgagtcgggcagccacacgtgcagcgggaactgtgcgctcttgcccatggcaccgatgaacaggcagatgcagatcacggtcaccagcatccactcggtgccggggaaggtgatgccagccagcgtattggccttggcaaaggcctcgccgtagttcagcgtaccggcgtaggccgcgatcaggccgatgccgagaatgaagccgaagtcgcccacgcggttgaccaggaaggccttcatgttcgcgaagatggcggtcggcttgttgaaccagaaaccgatcagcaggtacgacaccaggcccaccgcttcccagccgaagaacagctggagcatgttgttgctcatgacgagcatcagcatcgagaaggtgaacagcgagatgtaggcgaagaagcggttgtagccttcgtcttcttccatgtagccgatggtgtagacgtgcaccatcagcgacacgaaggtcaccacgcacatcatcatggccgtgaggccgtcgaccaggaagccgacttccatcttgaggccgccgaccaccatccattcatagatggtggcgttgaagcgggcgccgtccacgacgaccgacttcagcgtcatcgccgagatgatgaaggcgacgaacacgccgaggatggtcagcgaatgcgtgaccttgcggccgatgtggttgccgccgaacttggtgccgaacaggccggcgacgacggcgccgaccaggggtgccagcggcacggccagcagggtggatgcggaaagggttgcgctcatactggtttcaacccttgagcgagttgagttcgtcgacgttgatgttggacttgttgcggaacaacaagaccagcagcgcgagaccgatggccgattcggccgcggccaccgtcaggatgaagaacacgaagatctggccatgcatgtcgcccaggtagtacgagaacgccacgaagttcatattcaccgcgagcagcatcagttcgatggccatcagcagcacgatgaggttcttgcgattcaggaaaatgccgatcaccgagagcgcaaagagcatggcgccaagcgatagaaagtgtccgagcgtgagcgtcatgccttgttttcctttgccgctgcggcgtcggccggtgcttccaccacgggctcggcggcgcgcgtgaccgccatctgcacgatgcgaacgcggtcgcgtgccttcacgcgcacctggtccgacgggttgacgtacttgctgtccttgcgggtgcgcagcgtcagtgcaatggcggccacgatggccacgagcaggatgaccgcggcaatttccagcggatagaggtattcggaatacagcagcttgccgagctcgagcgtgttcgagctgttgggagaagtggtcgccatggcgcgcggcgcttcaccgagacgaaagccgcccatcagcacggccgccatttcgagcgcgatgagcgcgcccacgccggctgccagcggaaagtgcttccagaagccctcccgcaagccgtcgacgttgatgtccagcatcatcacgacgaacaggaacagcaccatcaccgccccgacatagacgagcacgagcgagatcgccaaaaattcggcgcgcagcaaaagccagatcgccgaggcctggaagaaggccagcaccaggtacagcgcggcgtatacgggattgcgggcggtgatgacgcggaaggctgcaaacagcagcaccgcggcaaacagatagaacagaccggtcttgacgtccatttggaattcgaattggtacggggttcgggctgagcgggatcagcggtacttggcgtcggccgccttgttcgctgcaatttctttttcgtagcggtcgcccacggccagcagcatgtccttggtgaagtacaggtcgccgcgcttttcgccgtggtattcgaagatgtgggtctcgacgatggagtcgaccgggcagctctcttcgcagaagccgcagaagatgcacttggtcaggtcgatgtcgtagcgcgtggtgcggcgcgaaccgtcgtcgcgcacatcggattcgatggtgatggcgagcgccgggcacacggcctcgcagagcttgcaggcaatgcagcgctcttcgccgttttcatagcggcgcagcgcgtgcaggccgcgaaagcgcggcgacagcggcgtcttttcttcgggaaactgcaccgtgatcttgcgggcgaaggcgtacttgccggtgatggcaaggcccttgaacagttcgaacagcatgaagctgcccaaaaaatccttgagcgagaacggagcggacgttgttgcggtatgcgcagcagacatgatgttggcgcttccagttatttccagatattgaacggggtctgcatccaggcaccgaccacgaccagccacacgagcgtgaccgggatgaagatcttccagcccagacgcatgatctggtcgtagcggaagcgcgggaacgtcgagcgaacccacaggaacatggtgacgacgcagaaggtcttggcaccgagccagatccagccgggaatgaagctcaggaactcaaacggcggcagccatccaccgaggaacagcacgacgcacaggatcgagaccagccacatgttggcgtactcggccaggaagaacatggcaaagctcatgcccgagtactcgatcatgtggcccgcgacgatttcggactcgccttcgaccacgtcgaaggggtggcggttggtttcagccaggcccgagatgaagtagacgacgaagatcggcagcagcgacagccagttccacgacaggaacccgatgcccatcgacgcgaaggtgcccttgccctgccctgtcacgatgtcggtcatgttcaggctggccgagaccatcagcaccacgacgaagcagaagcccatcgcgatttcatagctcaccatctgtgccgaggcgcgcagcgcgcccaggaaggcgtacttcgaattggaagcccagcccgcgatgatcacgccatagacctcgagcgaggtgatggccatcacgaacagcaggccggcgttgatgttggccagcgccacatcggggccgaagggaatcacggcccacgcggcgagcgccggcatgatggtcatgatcgggcccagcaggaacaggcccttgttggcgaccgtcggaatgatgatttccttggtcatcagcttgagcgcgtcggcaatgggctgcagcaggcccagcgggccgatgcggttcgggccgatgcggatctgcgtgaagccgatggccttgcgttcccacagcgtgaggtaggccacggcccccatcagcgggagcacgaccacgatgatcttgatcagcgtccagatcacgggccagaccacggctgtccaccagcccgcatggaccaggcccaggccgaaagcatgcagtgaatcgatcatgccaatgcctcctcggcacgggccggtgctgccagtgcgttgcgcgcatcggcggtgagttgcagcgacggtgcgcggcgcacgatcgagtcgagctggtagatgctcgcgaccacgggtgcgggaaccgcgccggtggaagccacggcttttgcggcggtcgtattgcgaagcgcatcggccggcacggcgccgttgtcgccgatggtgcgcagcacgtcagcggtcgattcgaaggcaaagcccggcaggccgagcaggttggccagcacgcgcagcaccttccaggccggacgcgcctcgccgtgcggcttcacgacggcatggaagctttgcacgcggccttcggcattgacgaaggtacccggcgtttcggtgaacggcgcgatgggcagcagcacgtcgctgaactcgaggttggccttgaaggggctcagcgtgacgaccatttgcgcattgccgatgacatcggcggctgcggcgcccgcggccgagtcgaacaccggctcggtattgagcagcagcaccgccttgaggccggaacccgccgccagcatgtggccggcatcgaggccgccattcctggggaacgcgccgacgagttgcgcgcccacggtgttggcggcttcggtcaggtagccgacggtggcgccggtctgcgcgccgatccagttggcgagggccagcaggctgctggcttgcgcgtggtgggcagcggcgttgccgagcaggatggccttgcgctcgccgctcagcagcgaggctgcgatggcttgtgcggtggcatccggtgcattcttcggtgccagcggcgcagcggcgccattggtctggccgatggccgcggccacggcggccagcgcctcgacccactggtcggcttcggcgatcgtcgattgcgccacgttcatggcccacgcgtcgcggtcggccatcaggctggccgaggcaatcaccgacagcgcggcgcccttgcgcacggcctggcggatgcgctgcgcgaacagcgggtggtccttgcgcaggttcgaaccgacgaccagcgcgcgctgcagctgcgtgagcgatgcgatcgaggtgccgagccagcgcacgccttcgaacgccgtgaattcggcgttgcgcaggcgatagtcgatgttgtcgctgccgagttcacgcgtgagcatggcggcaagctgcagctcttcgagcgtgctgtgcgggctcgccagcgtgccgatgctctgcgcgccgtggtcggccttgatctgcttcaggccgttggccacgtattcgagcgcggtctgccagtcgacctggtgccattggccgccctgcttgagcatcggctgcgtgaggcgttccgggccgttgagcccttcgtaggagaagcggtcgcggtcggcgatccagcattcgttgacttcttcgttctcgagcggcaccacgcgcatcacgcggttgttcttgacctggacgatcaggttggcaccggtggaatcgtgcgggctcaccgacttgcggcgcgacaactcccaggtgcgggcgctgtagcggaacggcttgctcgtgagcgcaccgaccgggcagatgtcgatcatgttgcccgacagttcggagtcgaccgagtcgccgaggaaggtttcgatttcggagtgctcgccgcgttgcgtcatgccgagctccatcacaccggccacttcctggccgaagcggacgcagcgcgtgcaatgaatgcagcggctcatttcttccatgctgatcagcggaccgacgtccttgtggaagacgacgcgtttttcttcttcgtagcgcgaagaagaaccgccgtagcccacggccaggtcttgcagctggcattcgccgccctggtcgcaaatggggcaatccagcgggtggttgatcaggaggaactccatgaccgactgctgcgccttgatggccttttcgctcttggtgcgaacgatcatgccctgcgtgacgggcgtggcgcaggccggcatcggcttgggcgctttttccacgtcgaccaggcacatgcggcagttggccgcgatgctgagcttcttgtgatagcagaagtgcgggatgtaggtgcccgccttgtcggccgcatgcatcaccatgctgccttcggtcacttcgaccttcttgccgtcgagttcgatttcgatcatgagtatgtttcttctcgcgctcaggccttgacgggcgctttcgggacgtagcccggaatcaaggcctcgaactcgtgacggaagtgcttgatcatggcgcgcaccggcatggccgccgcgtcgccgagggcgcagatcgtacggccctggatgttgtctgccacggagttgagcagatccatgtccgacgccctgccctgtccgttgtggatgcggtcgaccacgcggtagagccagcccgtgccttcgcggcaaggcgtgcactggccgcaggactcgtgcatgtagaagtacgacaggcgccgaagcgactcgaccatcgagcggctgtcgtccatgacgatgacggcgcccgaaccgagcatggagccggccttggcgatggagtcgtagtccatcgtgcattccatcatgatggcggcgggcagcaccggcgacgacgatccgccggggatcacggccttgagcgtacggcccttgcgaacaccgccgcacagctccaacagcttggagaacggcgtgcccatgggcacttcgtagttgccgggcagttcgacgtcaccgctcaccgagtagatcttggtgccgccgttgttcggcttgccgcattcgaggtaggccggaccgccgttgttgatgatccagggcaccgccgcgaaggtctcggtgttgttgatggtggtgggcttgccgtacaggccaaagctcgccgggaacggcggcttgaagcgcggctggcctttcttgccttcgagcgattcgagcagcgcggtttcctcgccgcagatgtaggcgccgaaaccgtgggcggcgtgcaactggaagttgtacgtgctgcccatgatcttgtcgccgaggtagccggcggcgcgcgcttcttcgagggcttcctcgaagcggtcgtagctctggaagatctcgccgtggatgtagttgtagcccacgctgatgcccatcgcatacgcggcgatggccatgccttcgatcacgatgtgcgggttgaactgcaggatgtcacggtccttgcacgtgccgggctcgccttcgtcggagttgcagacgaggtacttctggcccgggaactggcgcggcatgaagctccacttcaggccggtcggaaaacccgcgccgccgcggccgcgcaggcccgaagccttcacttcggcaatgacctggtcgggcgtgaggccctcggtcaggatcttgcgcagcgccttgtagccgccgcgcgcttcgtagtcggccaggcgccagttggtaccgtcgaggccggcatagatctgcggctcgatgtggcggtcatggaaacaggtctggacgcccgtggcctggaattgctggagcacttgttcgggcgacatcacgcggcctcccctttggtggtgccggtggaggcacgcaatccgtcgatgagctggtcgagcttctcgttgctcatgaagctgcacatggtgcggtcgttgaccagcatcacgggcgaatcggcgcaggcgcccaggcattcgctctgctgcagcgtgaacaggccatcggccgtggtctcgcccatcttgatgccgagcttcttctcgaggtggacgagtgcggtgacgccgtcgcgcagctggcacggcaggttggtgcacacgttgagcttgaacttgcccaccgggtgctggttgtacatgttgtagaaggtcgtgacctcgtgcacggcgatgggcgccatgccgaggtactcggcgatctcgcgctcgcgctgcatgctgatgaagccttcgtcctgctgcacgatggccaggcaggccatcacggccgactgcttgccggcttcaggatacttggcgacttcgcgcgcaaagcgctcgagaatcgcaggcttcagaggagcagaaggcgccgtaggcgccgtgtcatggtgggtcgaggaagtcgtcattcgctctttctcacctgtcgatttcgccgaacacgatgtccatcgtgccgatcaccgcgacagcgtcggcgatcatgtggccgcgcgacatttcgtcgagggcggcaaggtgcgggaagccgggggcccggatcttcaggcggtacggcttgttggcgccgtcgctcaccagatagatgccgaactcgcccttcgggtgctcgacggcggcatacgcctcgccttcgggcacgtggaaaccttcggtgaagagcttgaaatggtggatcagctcctccatgttcgccttcatcgattcgcgcgctggcgctgcgaccttgtggttgttggtgatcaccgggccggagttgacacgcagccatgccgagcactgctggatgatcttgttggcctggcgcatttcttccacgcgcacgaggtagcggtcgtagcagtcgccggtcttgcccacgggcacgtcgaacagcatctggtcgtagacgtcgtagggctgcttcttgcgcaggtcccattcgatgcccgagccgcgcagcatggggcctgtgaagccgaggttcagcgcgcgctccggcgtcacgacgccgatgcccacggtgcgctgcttccagatgcggttgtcggtgagcagcgtttcgtactcgtcgaccatcttcgggaagcgcttgcagaagtcgtcgatgaagtcgagcagcgagccctggcggttctcgttgagacgttcgatcgccttcgcgttcttgatcttgctgaccttgtactgcggcatggagtccggcaggtcgcggtagacgccgcccggacggaagtacgccgcatgcatgcgcgcgcccgacacggcttcgtacatgtcgaacaggtcttcgcgctcgcggaagcagtagatgagcatgttcatcgcaccgcagtcgaggccgtgcgcgccgagccacagcaggtggttcagcaggcgggtgatctcggcgaacatcacgcggatgtattgcgcgcgaatcggcacgtccaggcccatcatccgctcgatggcgaggcagtaggcgtgctcgttgctcatcatcgacacgtagtcgagacggtccatgtagggcagcgactggatgaaggtgcgcgactcggcgagcttttcggttgcgcggtgcaagaggccgatgtgcgggtcggcgcgctggatcacttcgccgtcgagctcgagcaccaggcgcagcacgccgtgcgctgccggatgctggggaccgaagttgagtgtgtagttcttgatttcggccatatcagtgcaaaccgctgccgtagttgtcttcgcggatcacgcgcggcgtgatttcgcggggctcgatcgataccggctggtagacgacgcgcttctgctcttcgtcgtagcgcatctcgacgtggccggacaccgggaagtccttgcggaacggatggccgatgaagccgtagtcggtaagaatgcggcgcaggtcgtcgtgcccctcgaacacgatgccgtagaggtcgaaggcctcgcgctcgaaccacgtggcggcgttccagacgggctggagcgaatcgaccaccggtaggtcttcgttgggggcgaacaccttgaggcgcacgcgctggttgaggcttaccgaaagcaggtgcgtgacgacgcaatagcgctcgccctgccactcgccttcgcgatagtcggaatagtccatgccgcagaggtcgatcaactgctcgaagcggcagccgggcgcgtcgcgcagcagcgtggccgcctcgatgtaggcgtctgcagcaaccaccacagtcacctcgcccaatgcgagcgtcacgctcttggcgcgggcgccgagcgcctcggcgatggtggcgcgcagcacctccggcgatattgcaaagtcagtcatcgtcggcaatccctcaggcgcgcgcaatggtgttggtgcggcgaatcttctgctgcagctggatcacgccgtaaagcagggcttcggcggtgggcgggcaacccggcacatagacgtcgacaggcacaatgcggtcgcagccgcgcaccaccgaatagctgtagtggtagtagccgccgccattggcgcacgagcccatcgagagcacccagcgcggctcaggcatctggtcgtagaccttgcgcagcgccggcgccatcttgttgcacagcgtgccggccacgatcatcagatcggactggcgggggctgggccgaaacagcatgccgaaacggtcgatgtcgtagcgggccgcgcccgcgtgcatcatttcgacggcacagcaagccagaccgaaagtcatcggccagagtgatccggtcttcgcccaattcaccaccgagtcgtaggtggtggtgacgaagccctctttcatgacgccttcaatggccattttgtcgattccttgtcattcccagtcgagcgcgccttttttccactcgtagacaaagcccacgacgaggatggcgagaaagatcatcatggcccagaagccgacggcgccgatttccttgagcgcgatggcccacggaaagagaaaggcaatctcgagatcgaacaggatgaagagaatggcgacgaggtaatagcgcacgtcgaatttcatgcgcgcatcctcgaaggcctcgaagccgcactcgtagggagcgttcttcgctgcgtcgggccgattgggacccaggatgtagccgatgacttgcggtgcgacacctacaccgacaccgaccagaatgaacaaaaggacggggagataggaatcgaggttcatcgggagatttttcaccgcttgccaccggcagaaaaacactcggatgaggtttctgccagtgagatttggtgcggtcggcgagactcgaactcgcacagctttcgccactaccccctcaagatagcgtgtctaccaatttcaccacgaccgcggttttttgttcggatggcatgaggtacctggaaaggtgtttggctttccgaacagctttagagtttaccctgaaatgaagccgtttctcgctggcagcttcatgaaaacaacttgattatttgttcgggatctgacccgggcccgaaacaggtgcggcaggtgccgaagctggtgccttggcaggcgccgcaccggatgtgcccgaaggaatttgccccgccgcggctgacgcgggggttgcgggcgtgccgacggccgcgcgctccagcaggctgccgccgcccgtgggccgtgcatggctgaagtaggccagcagcagcgtgctcgcaaagaacaccgccgccaggacagccgtggtgcgcgaaaggaaattcgcgctgccgctggcaccgaacaggctgccggcactgccgctgccgaaggccgcgcccatgtcggcgcccttgccgtgctggatcaggatcagcccgatcattgcaagggccgacagcatctgcacgccgaccagaagattgaggaccacattcattcgttcttactcctaattgatgacagccgcggctcgggttcagcgagcggcggcggaaatgatctgcaaaaagtcgggggccttgagcgacgcgccaccaatgaggccgccgtcgatgtcaggctgcgcgagcagctctgcggcgttggccgcgttcatgctgccgccatagagaatgcagatgccggccgcgtgttcgctggcggcgtggtgcagctgcgcacgcagcacggcatgcaccgcctgcgcctgctcgggcgtggccgtcttgccggtgccgatggcccagacgggctcgtaggccaccacgatttcgctgatgcagtggccgttgacgtggatcaccgccgccagctggcgcttgacgacttcttcggtatgccccgcttcgcgctcggccagcgtttcgcccacgcagacgatcggcgtgatgccgttcgccagcgcagccgccgtcttggccgccaccgcttcgtcggtttcgccgtggtactggcggcgctccgaatggccgacgatcgtatagcgcacgccgaattccttcagcatggccgccgattgctcgcccgtgaacgcaccttgcgggtgcgccgagatgtcctgtgcgccaagcgccatggccgcagagcccgccagcagcgattgcagctgggcgaaatacggggccggcgcgcaaagcgcgatatcgcagctggccggcgccgcggccaggccctgctgcagggccttcaccagcgactcgttggcagcaaggctgccgttcatcttccagttgcccgcgatcagcttctttttggtcgttgtcatcgtgttgttgcccgtcaccatgtcagcacgatcttgccgatgtgctggttggattccatcagcgcatgcgcctgcgcggcgccgctgggttcgccgcccgccacaaaggtgctgtggatcacgggcttgatcgcgccgctttcgagcagcggccagaccttctcgcgcagcgccttggcaatggcccccttgaaggccaccggccggggccgcagggtcgagccggtgatcaccagccgcttgcgcagcaccaggcccgcgttgaagtcgctcttgaccccgccctgcaccgcgatgatcaccagccggccgtcttcggccatgcattcgatctcgcgggccacgtagtcgccggcgaccatgtcgagaatcacgtccacgcccttgccgccagtgagcttctttgcctcctcggcgaagtcgctcgtgcggtagttgatggcgtggtcggcgcccagcgccttgcaggcttcgcacttgtcatcgctgccggccgtgacgatcacggtcgcacccagtgccttggcgatctggatggccgtcacgccgatgccgctcgagccgccttggatcagcagggtttcgcccttttgcagacggccccgctcgaacacgttgctccagacggtgaagaaagtctcgggcagcgaggctgcctcggtatcgctccagcccttgggcaccggcaggcattgcaccacgggcgccacgcacagctgcgcatagcccccgcccgcgatcagcgcacagacgcggtcaccgatcttgaaacccgcctcggccaaggccgcggcgtcgcccgacacgatctcgccggccacttcgaggcccggcaggtcggaagcgcccggcggcaccggataatgccccttgcgctgcagcacgtccggacggttcacaccgctggccgccacgcgaatcagcaactcgcccgcaccggccaccggatcgggacgctccacggcgcgcagcacctcaggggcgccgtacgaagtgatttcaatggctttcatggtctttggcctgcaacgcccgcggaacgggcgtggttagctgttcaaaaagatggcaacggcagccatggccgccgttgcgcccttcttctctacttactcttgcggttcgcgcggtgcgtactgcggctcgccaacgggcgcctgcggctgctcgttgcgcggctgctgttgctgctcgttgctgaaacgcggcgcacgttcgccacgatcgccaccgcggtcaccgccacggtcgccacggtccgaacgctcgcggcgctcgccgccgcgatcaccacggtcgccacggtcttcacgcggcgcgcgttcctggaactccatgccggccggacgctcggtcagggccttcatggacagcttgacgcggcccttttcgtccgtctcgaggaccttgaccttgacgatctggccttcgctcagatagtcggtcaccttctcgacgcgttcgtgcgcgatctggctgatgtgcagcaggccgtccttgccgggcaagaggttgatgagcgcgccgaagtccaggatcttggtgaccgggccttcgtagaccttgccgatttcgacttcggcggtgatctgctcgatgcgccgcttggcgaactctgccttttccggatcggtcgaggcgatggtgatggtgccgtcttcgtcgatgttgatcgtcgtgccggtttcttcctgcaggccgcgaatgaccgcgccgcccttgccgatcacgtcgcggatcttctcggggttgatcttcagcgtggtcaggcgcggtgcgaattgcgacacctcggtcttggcctcgcccatggcttcctgcatcttgcccaggatgtgcatgcgcgcctccttggcttgcgccagtgcgacctgcatgatttccttggtgatgccctggatcttgatgtccatctgcagcgcggtgatgccgttggtcgtgccggccaccttgaagtccatgtcgcccaggtgatcttcgtcgcccaggatgtcggtcagcaccgcaaagcggttgtcttccttgatgaggcccatggcaatgccggccacgtgggccttcatcggcacgccggcgtccatcatcgacaggcagccgccgcagaccgaagccatcgacgaggagccgttcgattcggtgatttccgacaccacgcgaatggtgtacgggaattcttccttggtcggcagcacggcgacgagcgcgcgcttggccaggcggccgtggccgatttcgcggcgcttggtcgagcccatgcggcccacttcaccggtggcgaagggaggcatgttgtagtggaacaggaagcggtcttcgtactcgccggccagcgcgtcgatgcgctgtgcgtcgcgttcggtgccgagcgtggtgatgaccaggccctgcgtctcgccgcgcgtgaacagcgccgagccgtgggtgcggggcagcacggagttgcggatctcgatggggcgcacggtgcgcgtgtcgcggccgtcgatgcggggttcgcccgagagaatctggctgcggacgatcttcgactcgatcgagaacagcaggtcgttgaccttgccggcgtcgaagggttcgccgctttccttcagcgtgttcatcacgctggcattggcttcgcgcagggcttgcgtgcgggcttgcttgctgcggatctggtagacggcgcgcagcttttcttcggccaggctcttgaccttggcaacgaaggcttcgtcttcggccggcgcttgccagtcccacaccggcttgccggcgtcgcgcacgagttcatggatcgcgttgatcgcgatgttggcttgttcatgaccaaacaccacgccgcccagcatgatttcttcgctgagttgctgcgcttcggattcgaccatcagcacggccgcttcggtgccggcgacgacgaggtccatctgcgaatccttgcgggcggtctggcccggattcagcacgtactggccgttgatgtagcccacgcgcgcggcgccgatcgggccgctgaagggaatgccggaaatcgacagcgcggcgctcacgccgatcatggcggcgatgtcggcgtcgacttcggggttgagcgacagcgtgtggatgaccacgtgcacttcgttcaggaagccttcggggaacagcgggcggatcggacggtcgatcaggcggctggtcagggtttcatgttcgctgggcttggcttcgcgcttgaagaagctgccggggatcttgcccgcggcgtaggtcttctcgatgtagtcgacggtcagcggaaagaagtcctggcccggcttggcggtcttggaggcaaccacggtcgcgaggatcacggtgccgtcgatgtcgaccaccacggcgccgctggcttggcgggcgatttcacccgtttccatgacgacggtcttgtcgccccactggaaggacttggtgactttgttgaagaggctcatgttttgctcctgttttgatagcgaaacacctgtattcggtacaggttccgcagggacggaggcttctcagaacacgatgccattccagcgaagctcggcgggaacttcattggaatgacacagcttcgctctgttttggcactccgaaagtggatcgcgaagtaaaaaacgcctgagctagcggactaacccaggcgttttttcatgcgattcggtttacttgcgcagacccagcttggcgatcagcgcggtgtagcggtcggcgtccttggacttgaggtagtccaggagcttgcggcggcggctcaccatgcgcagcaggccgcgacggccatggtgatccttggcgtgcgtcttgaagtggggggtgagctcgttgatacgggcggtcagcagtgcaacttgcacttcggggctgccggtgtcgttggcggcgcgggcgttgtctttgacgacttcggccttgatggaggctgcgatcatgttgaatttccttgttccgggatgtttgacttgcggtgagcgctggaactgccctcaccgtgcgccttgcggcatgcaaagccatggaattatagctcgcccccaggctccgcgcacttcgtgtcgctcctccctccccctaccgggggcgacgccagcggcccggcaaagccggttccgcggcatccctggaatggacggctcgccttcggcctcgcggcggttcttcttttttttattgctcggcgagccaggttttcaggcgctcgacgccttggactagtcgctgcgggtctttggaggcaaaacaccagcgcagccagccttgggcttcgggggcaaaggcattgccgggggcgagaccgaggccggcttcgacgaccaggcgcttggccaggtcgagggaatcgccgaagccctcgaggcggaagaaggcgtacatgccgcccttggcgggagccacctgcacgccggggagctcggccagcagcggcaccagggtgtcgcggcactgcttcagatgggccaccacgcggggcgtgatctcggcggtgtgttcgatggcggcaacggcggcgcgctgggtgaagacgctggcgcacgaagtgttgaactcgatcagcttgccgatgccctccaccagcgcgggcggcagcacgagccagcccaggcgccagccggtcatgaggaagctcttggagaagctgtgcgtcaccaccagccggtcgtcgggcctggagatgtcgagaaagctcggcgcgcagccattgggcgtgggctcgaagtaaaggcgctcgtacacctcgtcggccaggatccaggtgccggtctcacggcaatggtcgagcacggcctgctgctcttcgcgcgtcatggtccagccggtcgggttgttgggcgcgttgacgatcaggagcttggtctttggcgtgaccgccttgcgcagagcggccaggtcgagcgtccattgtccgtcggcaggcaccagccacaccgtgcgcacctgggcgccgaggatggcgggctgcgccgtgaggttgggccacaccggcgtgaccgcgaccacctcgtcgcccgcatcgaccagcgcctgcaccgcgagcatcagcgcgctgacgccgccggaggtgacggcaatgcgcgacgcatcgaccgccggatgaagcatgctggtgtagcgcgcaatggcctcgcgcagttcaggcaggccgaggttgtgcgcatagaaggtttcgccgcgctgcagcgagtcgatggccgcctggcggatcacctcgggcgtgacctcgtcgctttcgccgaaccagaacgcgagcacgtcgtcgcggccgagcccggcattggcaacctcgcggatcttggaggcttcgaggttgtgaatggcttcgcgcatgttttcgtttcctagattcttttcattttgcagctggtcggcagttcggcgcgttcgggcgcaatggtcttgatcacgcgaaagccgtaacccgacccttcgacatcgaactgcacgcccggccggccctgtctgtccatcacaccgaccacgagctgctgctgaaactggtggtcggccgcgcgcatgcggccacgctgtccgtagaggctcacgtcggcctgctcgagcgcgcgcgccacggccacggcttcgacactgcccgcgcgttcgatcgattgcgccagcgactccatgagcagctgcatgcgcatgtgcacgtagtcgtcggccggcttgggaaagcgcgcgcggaaggcgcggtagaacgcctcggactgggcggtctgcacgttgggcagccagtcggccaccgcgatgacgcggccgatgccggcatcgccgatggccgcgggcgcaccgagcgcgttgccatagaaggtatagaaggtgccgttgaatccggcctcgcgcgccgccttcaccagcagcgtgagatcgttgccccagttgccggtgaacaccgcctgcgcgccactcgcaaggatcttgctggcgtagggcgcaaagtccttcacccggcccatcgggtgcaactcgtccccgacgatttccacgtccggccgctgcacgcccagctggcgtttcgattcgcgcagcaccgcctggccgaagctgtagtcctgcccgatgagatacgcgcgcttgagcgccgcatcgtccttcaccacttccatcagcgcggccacgcgcatgtcggcatgggcgtcgaagcgaaagtgccagaagctgcagcgctcgttggtgagcaccggatcgacggccgcgtagttgagaaagatcacgcgccgcgaaggatcgcgttcgttgttcttctcgatggcatcgaccagcgccgcggcggtggccgaggagttgccctgcagcacgatgcgcgcgccatcgtccatggccgcgcgcaatgccgacagcgcttcttcgttctgccccttgctgtcgtagcggtcgagctgcagcggccgcgcgccaccgggcacacccggcagcttgacgccgccgcgcgcattcacgcgctccacggcccacagcaggttgcggaagaccgcttcgcccgtgttggcgaacgggccgctcatgctttcgatcaacgcaaggcgaatgggcgcaggtgctgcggacggcgcctgcgccagcgcggcaaagggcgctgcgcatagcgccagcgccgcaaatttcaaggccttgcgacgccaaataaaggggtgagtcattgtcttgaaacgggtgcggccatgcctagatgaggtgtcaagcggcactcaggattgaatggccgcgcagtgtaagggacacacattccttgtccccattgtgttcattcaggagttctcacatgtttttcgcacccacccttcgcacggcccgtttcgctccccgttcgtacgaccgcgccttcgagcgcttcgtcaatgaagcctttgccggagcaagccgctcgccgctcgtcgaacaggacgacaagagctggaccctttccctcgacgtgccgggcctctcgcgcgaagacctcgccatcggcatcgaaggtgccgtggtccgcatcgacagcaaggccgaagccaagcgccaattcaaggctgcgtatgagctgccgctggacatcgacgtagctgccagcgaagccaagctcgagaatggcgtgctcacgctgaagctcggcaaaaaggtgccggccagccagatttcggcgctgcagatcaactgatcttgcaaagcccacgagaggaaagtgtcgttaacttttgtttttgactttgttcgcactccctattcacaatagggcagcggataacgtcacatgatgtgacgttttcacatttttcttcttcgtgggcgtctcgcaagcgcaccgaatcctcgcggtgcggattcgggtgccccctcaaggcacaccatgatcacgcacctcaagtcagccaaagacaatgaacggtccgagacgctcctggtcttcctgccgggcgcctatctgaaacccgacgaattcgagcgcgaaggcttcatcagcgccgtgcgcgagcgccatctggcggccgattcgctgctggtggacgccgacgtttcctactactacgaccagacgctcagcgagcgcctgcatgcggacgtcatcgaaccgcagcgggccaagggctacaagtcgatctggctcgtgggcatttccatcggcggcttcggcgcgctgatccatgaactgtccaggccgggttcggtcgacggcatcgtcgcgctggccccctacctggggcggcgcgttctcggcgccgaaatcatcaaggctggcggcctgcgcgcgtggcaggcacccagcggccccctgcccgacgaagaactcgaccgcaagctgtggccgtggttcaagcaatacctggaaccccagcaagcccagaggctgccgcagctctatctcggcttcggcctggacgaccgctttgccagcaaccacaagctgctggccgatgccttgcccgaaggccgcgtcttcacgaccgaaggcggccacgactggccgcagtggcgccagctgtggcgcaacatgctcgatgttctgccggtgccgtcgctcggccgctcgccgcgtcctgcggctaggcgagcacccgcgggggtgtctcgggcgtcatcagcgaagccatgggccatcgcggcttgacgtcgaaggcatagcgctcgctggcctcggccagccccgactgcagccgcatggcggccgccatggcgatcatcgcgccgttgtcggtgcacagatgcagttccgggtagtgcacgcgcacgccgcgcttcgcacaggcggcattcagctgctcgcgcaggcttcggttcgcccccactccgcccgccacgacgagccgcttgaggccggtctgctcgagcgccgccatcgacttcttcagcagcacctcgacgatcgccgcctgcgtcgatgcggcaaggtccgccttgctcgcttcgagcgcggtgccgagcttcttggcctgcgtcagcacggcggtcttcagcccggcgaaggagaaatccagatcgccgctgtgcaaaagtggccgcggcagtttgaaggcggtggcgctgccctcctccgccagcttggccagccaggggccgcccggatacggcaggcccatgagcttggcgctcttgtcgaaggcctcgccggctgcgtcgtcgatggtttcgcccaggagttggtagcgcccgacgccatcgacccgcatcagctgcgtatgcccgcccgacaccagcagcgccacgaacggaaattccggcgggtccgcgctcaggaacggcgacagcaggtgcccttcgaggtgatgcaccccgagcaccggcttgccgagcgccgcgcccagcgcgcaggccacgcccgcgcccaccagcaaggccccggcgaggcctggcccgcgtgtataggcgaccacgtcgatttcggccagcgagcgccccgcctcggccagcacggtttcggtcagcggcagcacgcggcggatgtggtcgcggctggccagttcgggcaccacgccgccataggcctggtgcatggcgatctggctgtgcagcgcgtgcgcacgcagcagcggcagcgcgttgccgtgcgattcgaccagcgccacgccggtttcgtcgcaagaagattcgatacccaggagaagcatgctgcgagtgtaggcggcgcagaatgtccgcacggcacggatgttgcagcgaggctgtggctccccctccccaccatgaaatccggactgagttttctgatcgccgccagaaagtgcgaaatcgacgagctggaccagctcgcgcgcaccagcgacctggtcggcctgatcgcgcgtctggttcatgcgctgcagcgggagcgcggcatgtcgaacgtctttctcgcctcgcgaggggtccgcttcgccgagcagcgcgacccgcagatcgccgaatgcctggcactcgaacaggcggtacgcgccggattcgaccagctcgagaccgaggcgcgtcctggggccaccgccggcaacagcgcccgcctcttcagccgcattgcctgggtgctccccgggttcgacggcctgcctgccctgcgccgccgcgtcggcgcgctcgagctgacgcccgcgcaggccactgcggcattcgccaagctcgtcgccggtttgctggccgtggtgttcgaagcggccgatggcgccaccgaccccgaaatctcgcgcctcctggtcgcgatgttcaatttcatgcagggcaaggaattcgcgggccaggagcgcgctttcggcgccgcctcgctggccgtgggccgccgcgacgagtcacagcgccagcaatggctgcatctcatcgaactgcaggaacgctgcttccaggtcttcaccgacttctccagcagcagcgtgctggcgctctggcatcacagccagtccgacgcggccacggccgagatcgaacgcatgcgccggatgagcgtgacgtcggcccaggcggcttcggcggccgtgcccgactcccggttgagccaggcgtggttcgacagctgcacgcgccgcatcgacaccatgaagaccgtcgaggaccggctggccaccgacttgcgcgagctctgcgcccgcaagaccacgcaggcgcgcagcgaactgcagaggtacgaggaggtgcttggtgccctggcgccccaaaccgaaggcgcggccttcttcgacgacgccggcacccaggccaccgagcccgcccagtacggccggcacctggagcgctcggtgctcgacatggttcaggagcaatcgcgccgcctgcaggccatgagcgacgagctcgagaccgtgcgggcctcgctcaatgagcgcaagctggtcgagcgtgccaagggcctcttgatggcgcaccgccggatgaccgaggccgaagcccacaagatgctgctcaagacagccatgaaccagaagcgccggctcgtcgacgtggccgagtcgatgctcgccatggccgactaccttcccgtggccgaggcgtcccaacgctgaagaagcgggcacgggcgttcgaattggtgcggcgcacaacaatcgtgcatgcagccgactttccggtccaaccccccgtgccgcgcacaggcagtcgatcttctgctgcctatttgatagcggctggagtgccgaaaagctggcacacagtttgctgaagtagtacatggaccctcgggtcccaggcaggcagcacccaacggcgggtgtttgactaccgacatcggacaaaggcgtccccaccccgcaagggctcgttttcgagcggccctcgcgcggtgcggacgccttttttgttttttgcttttcctttttgtctgtccttcaaccggagcccgtcacatgaccgacctgctgaaaacccgcctcagccgccgccgcgtactgcaagccgccgccattggcgccgtgggaatcgatcccgccctgcgcgccgccgtctgggcccagggctccgacaagccggagaaggaggaagtgaagatcggcttcatcccgctgaccgactgcgccagcgtggtgatggcctcggtgctgggcatcgacaagaaatacggcgtgaagatcgtgcccagcaaggaagccagctgggccggcgtgcgcgacaagctctccaacggcgatctggacatggcgcacgtgctctacgggctggtctacggcatgcacctgggcctgagcggtcccaagaaggacatggccgtgctcatgacgctgaacaacaacggccaggccatcacgctgtcgaagaagctggccgacaagggcgcggtggacgcggcctcgctcgccaagctcatcgccaccgaaaagcgcgaatacaccttcgcccacaccttccccaccggcacccacgccatgtggatctactactggctggcctcggcgggcatcgacccgttcaaggacgtcaagaacatcacggtgccgcctccgcagatggtggccaacatgcgcgtcggcaacatggacggctactgcgtgggcgagccctggggccagcgcgcgatcatggacggcatcggcgtgacagccatcacgacgcaggacatctggaaggaccaccctgagaaagtgctcggcaccacgggcgacttcgtcaagaagtatcccaacaccgcgcgcgccgtcaccgcggccatcatcgaagcgggcaagtggatcgatgcgggcctgcagaacaagaacaagatggccgagaccattgccgacaagagctacgtcaacaccagcgtggacgccatcaaccagcgcatcctggggcgctacgtcaacggcatgggcaagagctgggacgaccccaaccacatgaagttctacaacggcggcgccgtgaccttcccctacctgtccgacggcatgtggttcctcacgcagcacaagcgctggggcctgctcaaggagcatccggactacctgaaggtggctaccgagatcaaccgcatcgacatctacaagcaggccgccgccgccacgcagacgccggttcccaaggacgtgcttcgcaccagcaagctgttcgacggctccgtgtgggacggcaaggacccgaagaaatatgccgactctttcaagatccacgtctgagacgcctgaggagaaacacaccatggtcagcgctgtatttcattcgccgatggacgcatctctccctctcccacgtgcgggagagggccggggtgagggagcgccccgcgccgaagctgcccccctccccatcccactccccaaagtggagagggagcaaaagccacgcatatccatcgacctgcgcgccttctggatgcgcgttctgccgccgctcgcgggcttcggtctcctggtgctgatctgggagctggttgccatgaagagcaccaccggctttccctcgccgctcgccacctggcagcaggcgctcacggtgttcagcgatccgttctacagcaagggcccgaacgaccagggcgtgggctggaacgtgctctcgtcgctgcagcgcgtggcgctcggcttcgggctcgccgcggcggtcggcattccggccggctttgcgatcgggcgcttcgagtttctctcgcgcatgttcaacccgctgatcagcctgctgcgtccggtgtcgccgctcgcatggctgcccatcggcctcctggtgttcaagggcgccaacccggcggccatctggaccatcttcatctgctcgatctggccgatggtgatcaacaccgcggtcggcgtgcagcgggttccgagcgactacatgaacgtggccaaggtgctgaacctcagcgaatggaagatcttcaccaagatcctcttccccgccgtgctgccctacatgctgaccggcgtgcgcctggcggtgggcaccgcgtggctggtgatcgtcgcggccgaaatgctcaccggcggcgtcggcatcggcttctgggtgtgggacgagtggaacaacctcaacgtcgccaacatcatcatcgcgatcttcgtcatcggcatcgtcggcctggtgctggagttcgcgctcatcaagcttgcaacggcattcacgttcgaagaggtcaaatcatgaacgacgattcgaagtacatcgagatccatggcgtcgagcagcgcttcaagaccgccaagggcagcttccttgcactgcagggcgtcaacctgaacgtggccaagggcgagttcgtcacgctgatcggccattcgggctgcggcaagtcgacactgctgaacctcattgccggcctgaccacgccgaccgagggcgtgctgctgtgcgcgaaccgggaaatcaagggcccgggcccggagcgcgcggtggtcttccagaaccactcgctgctgccctggctcacctgtttcgagaacgtgtacctcgcggtcgaacgcgtgtttgccgccaccgagaacaaggcgcaactgcgcgcacgcaccgatgcggcgctcgcaatggtcggcctcacgccggccgcgcaaaagcgccccggcgaaatatcgggcggcatgaagcagcgcgtgggcattgcacgcgcgctgtcgatggaacccaaggtgctgctgatggacgagcccttcggcgccctcgatgcgctcacgcgcgccaagctgcaggacgagttgctcgccatcgtgcaaaagacgcagagcacggtcgtcatggtcacgcacgacgtcgacgaggcggtgctcttgagcgaccgcatcgtgatgctcaccaatggcccggccgccaccatcggcgaagtgctgacggtggacatcgcccgtccgcgcaaccgcgtcgaactggccgaagaccccgtctacgtgcacgcccgcaaggccgtgatcgattttctctacacgcgccaggcgcacgtggagaaggtcgcggcctgaaccagcgagcgcggcacaagcggcgtcaggacatgatgacctgcaagctgtgctcgtaccaggccgtgaggcgctcgaaggtgtcgaccagtgcttcgctggaacgcaccagcgtcgcccggccctcggcgctgtcgagcgcctgcacgccacccaccaggcgcagccattcgtcgcgcgcggcaaccagcgcggcgcggatctcgggcgagctgaggggcgcacgctccagttcgcccagcgccgcctcgaactcgctcatggtcggcaacagccggccgcgcgaagcctctgccgcgatggtcgatgcaagcaatgcgtctttcgcaaggcgctgcgcacgcatgcgctggcgcccgcagatgttcacgatgcgcagcgcgcgccgcgcaccggaggcttccaacgcatccgtcatggcctcggccgccaacagcaaggcctcgccgcgcgcatcgatttcggccaacccctcgggcgccggccgcgcggccagcaaggcggccaatccgtcccaggccgttcgcacttcgcccagcgcctgcacgccggccgcgcccagctcgagggtggccagatgatccaggttctgctgcacccgctcggtcgattgcgtgcgcaggacccgcgcgcgctgcacgtcgatgccggcgagcaactgcgccgccacgcgcaccagccgctgcgagagcatgcgcagctgtccggcgcggttgatggcgtcggcccattgcgcggcctcgatcaccgagcgcgacacctcgcccagcctcaggttggcatgcatggcggcaccgcgcagcaggccgaaggcttcgtcctcgccgatgccccgtgcggacatcagaaggcccttggcgcgatcaacccacttgcgctcgtccatgcgggtgcgcaggccctcgagttcggtacgcaatgcggcgtcgcgctgccagcgggcctgcgcccgggcggtcagcccggccagcgaagcgccgtcgagcgcatcgagcggcatccacgcatgcatgccgagcgcaaccagcgcttcgtgctgcgcgctgtcgagcggcgcactcaccaggctcagtgcgcacggcggggcgccgttccattccttcagcgcatcgagcagcgcctgcagctgctgcgccggtgccggcagccaggccagcgcctgttgcggtgcaagcgcccccacccgctgcaccagcgtgtggcaagtggcccgctcgccggcgccggtgccggcactcgccagggcctgctccagcggctccggcaacggcgcgggtacggcgaattcattgggcaggacgacgagaagggacatcatggcaaagcggttgaaggcagggcaagcataggccacgccggctcgttttcgcaggcacgcctcttgcgtcaatcggggcgcggtgtaacgaagcaccgctttggtgaggttgcaggctcctgcaaccgtcccggcattccccatgccgggaagcacccccacgccgacagcgtccgctgccggcactccgccccaaccccgtccgtcgacacggccctcgaagagccgcgccgcggcatttcgcacgattgaacgccatgtccagtttcaggaccttcttgcaatcaggccacggcccgacgctgttctcggcctttctgtacttctcgttctcctgctgcatctgggtgctgaacggcgccatggcgcccttcatcggcgagaccttcaacctctcgcccgcgcagaagggcctgatgctttcggtgcccatcatcgcgggcgcgctgatgcgctttccgctcggcatcctctcgcaatacatcggtcgcaagaatgccaccctggtcgagatgggcatgatcgcggtggccatgctgttcggcttcttcttcgtgaagagcttcaacgacctgctggccatgggcgtattgctgggcattgccggcgccagtttcggcgtggcgctgtcgctcggctcgggctggtttccgccgcagcacaagggcctggccatgggcctggtgggtgcgggcaatgtcggcaccgcggtgtcggtgctggtggccccgccgctcgcgcaatggctcggctggcaggccgtgtatgccgtggcggccgccgccatcctggtgccgatgatcgtgatggtggtgttcgccaaggagccgcccgacgtcgacagccacgcgagcttccgcgagcacatcgcctgcctgttcgaaaaagacggctgggtgttcagcctcatctacggcgtgaccttcggcggcttcatcggcctcatcaccttcctgccctcctactactacgaccagttcggcgtgagcaaggtgcaggccggacagctcacgatgctggccgccttcatgggcgctgcggtgcgcatcgtcggcggctggctctccgaccgctggggcggcgtcaacaccctcacggtggtgctgctggtggtggctgtcggcctggtgctggtgggcatctcgtcgtcctccctggcgctcaccacgctgctcctgatcctgtgctttgccgcgctgggcgcgggcaacggcgcgctgttccagctggtgccgctgcgctggcccacgagcacggcggtggccggctcgatgatcggcgagatcggcgcgctgggcggcggcctggtgcccaacgccatgggcctgtcgaagcagtacctgggcagctatgtctggggcttcgtgttcttcggcgcgctctcgctggtgatgctgggcgtgatgcgcgtcatgcagatccgctggacccgcacctgggccgaaaaaggcggccgtgcgcgcacctcgcaccagccggcggaaatgaagaaatacgtcccaccacggaaagcggcacgcccatgaccttcttccgctcgccgtcagcgtggcaggaagagaagccacaccacgagcagtgcgttgaacagcagcgacacggccagcgcgatcttgtagagcgcggccggatcgcggcggatcagcggcgtggcggcgggcgcgctgacggggcgggaagcgccccgctccagggcgagcagcatttcctcggcggtttcgaagcgctccctcggatcgcgcgcgacggccttgcgcaccaggtggtcgagccacacgggcacgtcgggccgaaggcgcgagagcgcgaccggatcgcgccggtagcgcgccacctggtagggctcgatctcgccgtagggcaagtgcccgccgagccactggtacagcgtggcgccgagtgcgaacaggtcgctgccggggtcggcatgggcgccctcccattgctcgggattgatgtagctcggcgtgccggcatgcagctcccgctgggccgagccttcgcgtccggacagcgccacgccaagatcgaggatgcgccagcgtccgtcgtcgcccaggtgcaggttgccgggcttaatgtctcgatgcaccacgccatggcggtgcagccggcccagcgccttggtcacctcgatggccgccgtgaccacttcggccacggtgccgcgggcgccggacttgcgcatctgctccagcgtgcgcccgccgtgccagtcgaacacgatgtagagcgcgctggcgttttcggcccgctcgtgcacccgcacgaatccgccgctccccacgcgctggcccagccaggcctcgtgcgcgagcatggctcgctcctgcggatcgctggcgcgcgaggggtgcagcgtcttgagcgccaccagctgtcgcgtggctgcattgcgcgcctggtacagcagatgcacgccggtgtcggccaccagcccggtgatgacgtagccgtcgagtgcatcgcccactttcaagaagggcggcggcgccagacggcggccgtcgccgagctcgtcgtccagttgccgcgcgtccaggccgaccacgcgaatgaccagcgccgtcgcgttgtcgcgcgtgcctgcatcgagcgccgcccgcaccagcgcctcgctcgcgtcctcggcaccgccctgcaaggcgagctcggccaggcgctgcggcttgagcacgccgtgcacgccgtcggacgtgagcacgaagcagtcgcccacccgcacgtcgccctgcacgtagtcgacgcgcacctggtcgtccaggccgatggcacgcgtcaaccggctgcgcatgtcgggatgctcgaaggcatggtcctgcgtcagcagcatggcgggctcgccgtctgtgcgcacgcgccatgcgcgcgtatcgcccacgtgcgccagcgtgtagctctgcccatgcagcaccagggccgtcaaggtggtgagcgcggtgcccccgccctgccgacgacggttgtggtcggcaagccaggcgttctgcgcggcgaccaggcggtcgagcgcggcggtcggctcccaggtgtccggcgtggcgaagtaatcggccaagaggcccatcacggtggtctgcgaggcctccagcccgcggccgccggtggacacgccatccgcaatggccgcgatgagcccgcgcgcctcgtcgccgggcggcgcgttcacggcgccggcaaagtcttcgttcacttcgcgcggtccgcgctggctgctgtagccgatgtccacttcaaagctcatggcgcgattctccacgcgccgcgtgcttcccattgcttgatccgaacccgctgattccccgaaaggccccaccccatgcagaaactcaaactcgtgatggtcggcaacggcatggccggcgtgcgcaccctggaggagctcctgaagctcgccccggagctgtacgacatcaccgtcttcggtgccgagccgcaccccaactacaaccgcatcctcctgtcgcccgtgctcgccggcgagcagaccgtggaggagatcgtgctcaacagctgggagtggtacaccgagaaccacatcaccctgcacgcaggcaagaaagtcgtcgaggtcgaccgcgtcaagcgcatcgtgcgcgccgtggatgcgcagggcgccatcaccgaggccgcctacgaccgcctcctcatgtgcaccggctccaaccccttcatgctcccggtccccggcaaggacctccaaggcgtcatcgcctaccgcgacatcgccgacaccgactacatgatcgagaccgccaagacccacaagcacgcggtcgtcatcggcggcggcctcctgggcctggaggcggccaacggcctgatgctgcgcggcatgagcgtcaccgtggtgcacgtcatgccctggctcatggagcgccagctggacgacgtggccggcaagctgctgcaaaagtccctggaagaccgcggcctcaccttccgcatcggcgcccagacccaggaactcgtcggtggcgacgatggccgcgtcaaggccatccgcttcaaggacggcaccgaagtggccgccgacctggtcgtcatggcggtcggcatccgccccaacaccgagctggccgagaagatgcgcctgcactgcaaccgcggcatcgtggtcaccgacaccctgcagaccgtgaccgacgcgcgcatctactcggtgggcgaatgcgcggcccaccgcggcatcgcctacggcctggtcgcgcccctgttcgagcaggccaaggtcgcggccaaccacctggcccagttcggcatcgggcgctacctggggtcgctgacctccaccaagctgaaggtcaccggcatcgacctgttctccgccggcgagttcatgggcggcgaaggcaccgaggagatcgtcatgagcgaccccttcggcggggtctacaagaagctggtgatcaaggacgacaagctggtgggcgcgtgcctgtacggcgacacggtggacggcagctggtacttcaagctcttgcgcgacgggcgcagcgtgcacgacatccgcgacaagctgatgttcggcgaatccaacatcggcgacaccggccacgagggccacagcaaggccgccagcatgcccgacgaggccgaggtgtgcggctgcaacggcgtgaccaagggcaccatctgcaaggcgatcaaggacaagggcctgttcacgctggacgaggtcaagaagcacaccaaggccagcgccagctgtggttcctgcaccggcctggtcgagcagatcctgatgttcaccgccggcggcgactactcggccacgcccaagaagaaggcggtgtgcggctgcaccgacgcgaaccaccaggaggtgcgggaagccatccggaaggaacactacctgacccacgatgcggtctaccgcaacctgggctggcgcacgcccaacggctgcgcgacctgccgcccggcggtgaactactacctgatctcgacctggcccaaggaggccaaggacgatccgcagagccgcttcatcaacgagcgcagccacgccaacatccagaaggacggcacctactcggtgatcccgcgcatgtggggcggccacaccacgccggacgagctgcgccgcatcgcggacgcggccgacaagtacaagatcccgacggtgaaggtcacgggcggccagcgcatcgacctcctgggggtgaagaaggaggacctggagggggtctggaaggacatcggcatgccgtcgggctttgcctatgccaagagcctgcgcacggtgaagacctgcgtgggcagcgagtggtgccgcttcggcacgcaggattccacccagatgggcaaggacctggagcgggcgctgtgggcgatgtattcgccgcacaaggtcaagctggcggtgtcgggctgtccgcgcaactgcgccgaggccgggatcaaggacgtgggggtgatcggggtggactcgggctgggagctgtacgtggggggcaacggcggcatcaagacggaggtggcgcagttcctggtgaaggtgaagacggcggccgaggtgatggagtattcgggcgcattcttgcagctgtaccgcgaggaaggctggtacctggagcgcacggtgcactacatcgggcgggtcgggctggactatgtgaagaagaagatcctggaagacgccgaaggccgcaaggcgctgtgggagcggctgcagtttgcgctggatggggagccggatccctggttcgcgtccagccaggcgcaggtggatgtgcggcagttcacgccactgacggcgtaaacgaaaagagcggagaaaaaacttgaaaagaagactcttcatcgcttcctcggcgttcgccgctgcaggcgtccgtgcgcaggtggccgacctcaacgacgccatcaacaaggcgggccgccagcgcatgctgtcgcagcgcgcgagcaaggcctatctcgctctggcgcagaaggtggaaacgcgcaacgcccagcaggtgctcgacaagtccatcgtgctgttcgaaaagcagctggccgaactcaaggcctttgcgccgagccccgccatccgcagcacctacgacgcactcgacggcgcctggggcgagttcaagcgcgagctcaccggcacgacggccggcaaggaagaagccgcccggatcgtcaagctcgacgccgccgtgctcgcgcttgcgcaccagggcaccacgcagtacgaagccgcgtcgggcaagtccgtgggccggctggtcaacatcgcgggccggcagcgcatgctgtcgcagcgcatggccaagttctacctggccggtgcgatgcagatcgacgcggccggcagcacggccgaaatcgccaagtcacgcaccgaattcctggccggcctggacaccctgcgcaacgcgcccgaagccaccgcccagatccgccaggaactggtgctggccgacgcgcagtggatgttcttcaaccgcgggctccagcgcctcgaaggcgccggccactcgcccgccctcatgtccgacgtgttcgtgaccagcgaaaacatgctggccatcatggaccgcgtgacgggcatgtattccgacctcaaaacctagagaccccatcatgagtgaatggaaaaccatctgccgcatcgacgacatccccgtgctgggcgctcgccgcgtggcgcgcccggtgggcgtggacgtggcggtgttccgcaatgccgagaaccaggtgttcgcgctgctcgaccgctgcccgcacaagggcgggccgctgtcgcagggcatcgtgttcggcaccagcgtggcctgcccgctgcacaactgggccatcggcctggacgacggctgcgccaagtcgcccgatgagggatgcacccccaagttcgcggtgaaggtcgaagatggccaggtcatgatgaacgcgctcgaactcaagacgcacgccatcgatctggccccgccgcgtgccggccccggcgccgcaacggcgggcaagctgggtgacgagagcttcgacgtgcaggcgccgcacggcagctaggcgcacaaccaaggcatcgacccatggaagaaactcgctccacctgcccctactgcggcgtgggctgcggtgtgatcatcgagtccgacggcgcccagattaccggcgtgcgcggcgaccccgaccacccggccaacttcgggcgcctctgcaccaagggctcgacactgcatctcacggccacggccacggtcacgcgccagacacggctgctgcaacccatgcggcgcgccgcgcgcggcgccgagccggcgcccatcgcatgggacaccgcgctcgacggcgccgtcgacaagttcgaacaggtcatccgcgaccacggccccgacgccgtgggcttctacgtctcgggccaactgctcaccgaggactattacgtcttcaacaagctcgccaaggggctgatcggcaccaacaacatcgacaccaactcgcgcctgtgcatgagcagcgcggtggccggctacaagcagacgctgggcgccgacgcgccgccggcctgctacgacgacctgaagcatgccgagtgccttttcatcgtgggcagcaacgctgcatgggcgcacccgatcctgttccgccgcatcgaggatgcgaaggccgcgaaccccgggatgaagatcatcgtggccgatccgcgccgcaccgacacggtggaaatcgccgacctgttcctgccaatccagcccggcaccgacgtgatgctgttcaacggcatgctgcacctgatgctgtgggaaggctggaccgataacggctacatcgcggcccacaccaacggcttcgatgcgctgaaggccacggtgcgcgaatgcacgcccgacaaggtggcgcagatctgcggcatctcgaaggaagacctgctcaccgcggcgcgcatgttcgcgacttcgccggccacgctgagcctctactgccagggcctcaaccagtcgtcgagcggcaccgcaaaaaatgctgcgctgatcaacctgcatctggcgaccggccagatcggcaagcccggcgccggcccgttctcgctcaccggccaacccaacgccatgggcgggcgcgaagtgggtggcctcgccaatctgctgagcgcgcaccgcgacctggccaatccggcgcatcgggccgaagtggcggcgctgtggaacctgccctccgtgccggaaaaacccggcaagaccgcagtcgagatgttccaggccgcggccgatggcgagatccgcgcgctgtggatcgcctgcaccaaccccgcccagtcgatgcccgaccaggccacggtgcgccgcgcgctggagcgcgccgaattcgtcgtggtgcaggaagccttttcgaccacgtcgacctgcgcctttgccgacctgctgctgcccgccaccacctggggcgagaaggaaggcaccgtgaccaacagcgagcgccgcatctcgcgcgtgcgccccgcggtaccggggcccggcgaggcgcgccacgactggtcgattgccgtggacttcgcacgccggctcgaacagcggctcggccgcacggccaccctgtttccctatgaaagcgccgagcgcgtgtggaacgagcaccgcgaatccacgcgcggccgcgacctcgacatcaccggcatgagctacgccatgctcgacaccgcgggcccgcagcaatggccgctgaaagaaggcgaaaccaccggccgcgcccgcctgtatgaagacggcatcttcccgacgccggacggccgagcgcgtttcgcggacacggtctacaagccggtggccgaggcgcgcgaggcgcgctatccgttctcgctcaacaccggccgcctgcgcgaccagtggcacggcatgagccgcacgggcacggtcggccggctcttcggccacgtggctgaaccggcggtgcagatgaatgcgcaagacatggcgcgccgccagctgcaagacggcgacctcgtgcatctcacctcgaagcgcggctccatcctgctgccggcgcgcgccagcgccgagatcgggctgagccaggccttcgtcgccatgcactggggcgaggaatacctgagcggatgctcgtccaccggcacgccgctggcaggcatcaatgcgctgacctccccggcctactgccccacctcgaagcaacccgagctcaagcacacgccggtcaagatcctcaaggccgagctgccgtggtcgctgctcgccatggcgtggctgccgcccgacgcggcgcttgccgcgcatcaggcgctcaagccgctgatggcaatgttcccgtttgccacctgcgtgccgttctcgggcaacacgccgggcgaggaacgcagcggcatcctgtttcgcgccgccgcgcacgacgcaccggcagacgaactcatcgaccgcatcgaaggcctgctcggcctcggcagcagcgatgcgctgcgctacgccgaccgccgccgcggccagcgccgcgtggcacggctggtgcggcgcgccgacggcaacgccggcctcgaggccttcctgctgggcggcgacaccagcgccgaggcctggatcggcaccctgctgcgcgaggaaatcccggcgcagagctacggccgcctgctgctgtcgcctggcgctcgcgcgcccgtggcggtgcagtcgcgcggccagccggtgtgcacctgcttcaacgtgaccgacctggcgatccgggccgaactgggccgctgcagcggcacgcccgaggagcggctggcttcgctgcagggcgcgctcaaatgcggcaccaactgcggctcctgcctgcccgaactcaagcgcatggtgcgggccaccccggccgaaaccgtggtggagggtgcataagccgccttgctttccggcataagcattgcgggacaatccgtgcacccatgggaatcagccaatacatcaaggaaatcggccgcggcgcgcgaggcgccaagccgctgacgcgcgaacaggccaccgacctgttcggccaggtgctggacggcaccgtgaccgacctggagatcggcggcttttgcctcgcgatgcgcatcaagggcgaaacgccggaagaaatggccggcttcctcgacgccacgcacgccaggctcaaccgcctgcccgccgccgaccgcccgctcatcgtgctgccgagctacaacggcgcgcgcaagctgccggtgctcacgccgctgctggcgctgctgctcgcccgcgaagggctgccggtgctggtgcacggcagcgccacagaaacatcgcgcgtgctggcatcgaacgtgctggaggcattggacatgcccatgctcacggccatccgaaaaatcccgtccggcgaagtgggctttgcacccaccgagctgctcaaccccgccctcaagcggctgctcgacgtgcgccgcgtggtgggcttgcgcaaccctggccacagcgtggtcaagctgatgcagccgaccacgggcccgtgcgtgatcgtggcaagctatacgcatccggaatacgcgcgcaccatgggcgaaactttcgagctcatgggcatgaccgccttgctctcgcgcggactcgaaggcgaagtggtgtccgacccgcgccgcaccgcgcaggtcgacggcttcgtgcgcggcgtgcgcagcgaactgcaggcccaggccgcgggcacgtcgagcgaggtgcccggcctgccgaaagaaatcgacgtcgcgaccacggccgagtacacgcggcgcgtattgaacggcgagcttcccgtgcctgaagccatcgccacgcaggtcaggcacatcacgcaactggcgtcccacgcatgaacagaccgatctcttcttttgccaccggcagctgcacgctggtgggcgccggccccggcgaccccgaactgctgaccatcaaggccgtcaaggccatccaggccgcaaccgtgctgctggtggacgatctcgtgagcgaaagcatcctgaactcttacgcccggccgggcgcgcgcatcgtgcacgtgggcaagcgcggcggctgcaagagcacaccccaggctttcatcgagcggctcatgatcaccgcggcacatgaaggcgaaacggtggtccggctcaagggcggcgacccgttcatcttcggccgcggcggcgaagaggtcgagcacctgcgcgaagccggcatcgagtgcaccgtgatcaacggcatcacggccggcctcgcggccgccacctcgctcggcgtgccgctcacgcaccgcgaccatgcgcagggcgtggtgttcgtcaccggccacgccaagaccggcgccggcgcgcacgaagacgcgaccgactggcgcgcgctcgcggccacggcgcacaacgcccggctcacgctcgtcatctacatgggcgtggcgggcgcgggccacatcgaacgcgaactgctccatggcctgcccggcgacacgccggtggccgtggtgcagcatgcgagcctgccgcagcagcgccacatcgcgaccacgctcgatcggctccaggccggcattgccgaggccgggctcgcgagccccgcggtgatcgtggtgggcgacgtgctgcgcgggctggccgcggcggcgctgccggcgggcacggacgccggccgcttcggcacctgaacggcgatcagaaagagagtgccccggccatccggggccgtgcacgaagtgccgcggcttccggcgcatgcggcgcgtgcaacacgatcggcgtgcggcttccgaggctggccatgagggcgatccagccgatggccaggttgccattcgacatggccagccgctgcaggtcgagcatcagcgcctgatactcctcgagcacctggacctccgacatctcgccgcggctcattcgcgccttggcctgctcgaacgacgccttcgcgtcgcgcacgcgacggttggccgccgccgccgcatcgttggtagcctgcagctttcgcagggcctcggcgacctcagcgcgaccctgcgccacggcctccgggaagagcgggtagccggggagatcggcgtcggcgtcctggccgctctcgcctgtgtcttccgcggcatcgatcgtgccgcctagcccggcttgcggatcgatgccatacagcgccgcggccaactgaatatcgtcccggttggcaagcaatgccgccggcagggcctgcggcagcgggagcgccatacgaggctgcttgcgcgctgcgacttcatcggcgatggccttctgcagcgcctctgcggacaggcgcgagcgcgcagccagaaaggcgagctgaacgtcgcgctgcgcatcgatcttcttcatcgatgaagtcgcgtcggcttcgcggtgcttcaactcctcgcggaaatcgtcgtgcggtgcggggctggcgaagacgagttgcaactggcgccgtgcggcggcacgcgcactgtcgatgtaggtcaggctcagcgtctggaccagcaacccgacatacgccgccgacacgccgacctccggcgcctgcatgtccaggcggccatcggaagccgcgccgcgcgatgcctccgcaaccagcgcattcagcgtttcgctctcgaaggccagccaccagggacccgccgacgcacgcgaggcagacgccacgggctgccccgcgccatgcgtcaacgacgggcgcgccatggcgtggctcgcgctcacgccggagcctgcgcacgcgatgcccagcgcgccgatgagcatcgcaaccattgaccgacttgccaccattcgtgcgctccagaggatttcgacagccacgatggtcccccgcaaattcggagaaatcgaagaggtggcgcagcggggtcgcgaggccgccggcgcggcccattgcatccatgcaacacaagttgcgatcggtcgctgttcggcgagattcctcccacattgaacgaaaccattcaacccgtcatcgcggagcgcgcatgtcgctcgcgccccgctcaagaaagacggagagaaccatgaagatatgtccgcgctcgccgagcgccctgcgacggtggaccggtgttgcgctcgtctcgctggcctcgattgccgcgcacgcacagaacgccatcgaggcggtcaccagcactgcaaggggcgacgtggaactggtgcggatcgacttcacgcatccgctggccgcgcttcccaccggcttcgtggtgcaggagccggcgcgcattgcgctggattttccgggcgtcgccaatgccgtgggccgctcggcgatcgagttcaacctgggcaacctccgcaccgccaatgtcgtgcaggccggcgagcgttcgcgcgtggtgctgaacctcaaacacgcgaccacctaccaggcagagatccagggccgctcgctcctggtttcgctgcagcccggaacgggccagccccccaggacgccgtccaacgccggttttgccgaaggcagggagcgccaggcgacgccgctgcgggacatcgatttccggcgcggcggcgacggcgccggccgcgtgctcatcgccatgggcagcagccagctcggcgtggacgtgcggcggcagggctcggcgctggtggccgatttcatgcgcgcttcgctgcccgacgcgctgcggcgccggctcgacgtctccgactttggcacggcggtcgacgcggtgcacgcggagcagctcggcgacagggttcgcctcacgatcagttcgcacggcgactgggagcagagtgcctaccagaccgatgagcagttcgtcatcgaggtgcgcccgcgcaagacagacccgtccaagttgacgcagggcaccgggtacaccggcgaaaagctcacgctcaatttccagaatgtcgacgtgcgcgcgctgctgcaggtgatcgcggacttcaccggcttcaacgtggtgacgtcggacacggtatccggcgccctgacgctgcggctcaaggaggtgccgtgggaccaggcgctggaagtcatcctgcaggcgaagaacctggggctgcgcaagaacggcagcatcctgtggatcgcgccgcgcgacgagatcaacgccaaggaaaaggtggagctcgaagcgcaggccgcgctggagagcctggccgcgcttcgcacccagtccttccagctcaactacgccaaggccgccacggtggtgcaaagcctgacgggcggcggcgcctcgggcggcggcggcagcgcgtcggccacgcgcatcttgagcacgcgcggcagcgcgatcgccgaagtgcgcacgaaccagcttttcgtcacggacacgccgcaacggctggccgaagtgagcgagctcatccgcaagctggatgtgccggtgcggcaggtgctgatcgaggcgcgcatcgtcgaagcctcggacaccttcggcaagtcgctgggtgtcaagctgggcggcggggcctccggcaagaacagctcgttcggcaccagccccacgggcacggacaacgcctttacctcctacaccagcagcaacttcgtgaacctgccggccggcgatgcgggcggcaccggcagcagcgcgggggccttctcgctgtcgcttttcaactcgagcttcacgcgcatgctgaacctggaaatctccgcgctcgaagccgaaggcaagggccggctggtgtcgagcccgcgcgtggtgacggccgaccagaccaaggcgctgatcgaacagggtgaagagattccctaccagcaggccacctccagcggcgccacgtccatctcgttccgcaaggcggtgctgaagctcgaagtcacgccgcagatcacgcccgaaggcaacatcatcctggcgctcgacgtgagcaaggatgcgcgcggcgtcaccacgtcggccgggccggccatcaacaccaagcacgtgcagacggaggtgctggtggagaacggcggcaccgtggtgatcggcggcatcttcgagctgacggaaaccaacgacgagtcgcgcgtaccggtgctgggtgaggtgccttacctcggcgccctgttccggtcgcgggaacgcgtggtgaacaaggtcgagatgctggtgttcatcacgcccaagatgatcgcgcgcccgaacgccgcgctgtagcaccaagatgtggcatggagcgtgcttaacgccagcatgcccgttttccgatcgttttcagcgccacgcgcccgttcatgaacgccgtcgccgcgcctccgcccgccgccgttgaaatcgttgccctgagcaagcgctacgccgcaggcacgccggccgccgtcgaccggatcgacctgcgcattgccagcggcagctactgctgcctgctgggcccttcgggctgcggcaagagcaccacgctgcgcatgatcgcggggcatgagtcggtcaccagcggcgacatcctgctggacaaccgcaacatcacgaacctgcccgcggccgcgcgcggcacggccatgatgttccagagttttgcgctgttcccccacctgtcggccacggacaacgtggccttcagcctcaagatgaaaggcgtcggcaaggccgagcgccagaagcgtgcgcgcgacctgctggaacgcgtggccatgggccacctggccgaacgcaagcccggtgaactctccggcggacagcagcagcgcgtggcgctggcgcgcgcgctcatcaccgagccgcgcgtgctgctgctcgacgagccgctgtcggcgctcgaccccttcctgcgcatccagatgcgcgccgagctgcggcgctggcagaaggagctggggctgactttcgtgcacgtcacgcattcgcaggaagaagcaatggcgctggccgacaccatggtggtcatgaaccacggggtgatcgagcaggtcggctctccgcaccagatctacaaccacccggcaaacgaattcgtggcgcgcttcatgggcggccacaacgtgttcgacacgcccgccggcccgatcgccgtgcgcaacgaccacatgcggatcgccccggcttcggacggcggtgcgccaggcggccttgccgcggcggtgaccgatgtcgagtaccagggcacctacgtgctgctcgggctggcgctgcaagcggccccgcccggccgccagaacgtgtcggtcctgatgggcgaagccgccttcctcgcgagcccctatgcacagggccaggcggtgagcctggcctgggccgaggccgacgcgcgcgcactcgccgcggccccgtaagcgccgccaccacacacagcttttccccgttccttcatctgccacttttcatacggaggctctttcatgaccgaccccatcgactcgtccgccggcgtccagcgccgcacccttctgcaaggcactgccggcatcctggccacgggcatcgcgcccttcgtgcatgcacaggaaaaagtcgtgctgcgctaccttggcaccgcggtgaaccaggacaaggcgattgccgagaagttcaaggccgacaccggcatcgagatccagtacgtggccgtgaccaccgacgacgtgaccaagcgcgccgtgaccgcgcccaacagcttcgacctgatcgacacggagttcttctcgctcaagaagatcgtgcccaccggcaacctcaagggaatcgacaccaagaaaatcaagaatgccgacaagatcaccacgctcttcaccaagggcgaagtcggcggcaaggccgtgggcgaccagggcaccgcgcccaagaaggtgatctacctcgagggcgagaagagcaagaagttcgcgaccgcgccgacgcagttcatgtcgctcattcccacggtctacaacgccgatacgctgggcatccgtccggacctgatcaagcggccgatcagctcctgggccgaacttctcaatccggaattcaagggcaaggccgcgatcctgaacattccgtcgatcggcatcatggacgccgcgatggtggtggaggccaagggcatccacaagtacaaggacaagggcaacatgatcaaggccgagatcgacctgacgatcaagaccctgatcgaagccaagaaggccggccagttccgcgcgctgtggaaggacttcaacgaatcggtcaacctgatggcttcgggcgaagtggtgatccagtcgatgtggtcgccggccgtcacggccgtgcgcaccaagggcattgcctgcaacttccagccgctcaaggaaggctaccgcgcctgggccgccggctttggcctgccggccacgctgtcgggcaagaagctcgatggcgcctatgaattcatcaactggttcctcgacggctgggccggcgcctacctgaaccgccagggctactacagcgccgtgctcgacaccgccaaggccaagatggaggcctacgagtgggcctactggatggaaggcaagcccgcctcgcaggacatcaagagccccaatggcgacgtgctcgccaagaccggcgcggtgcgcgacggcggcagctacgagcagcgcatgggcggcatcgcctgctggaacgcggtgatggacgagaacgagtacatggtcaaaaaatggaacgagttcgtcgcagcctgaccctgtgagcgctccaaccgccagcgcgcatgcgcccagtccgtccctccatgccgtgaaggcatggtggcaggcggcgccgttcgcgctggtcttcttgctgttcttcctgattccgctggggctggtcgcgatggtcagcttgtggaatttcaacgagtacgagctgatcccggcggtgacgctgcgcaactacctgagcctgttcgagggctgctctcagctcacggacaacggcgacctgtgcgtcacgctcaacacctacctgagcaccttcaagttctgctttctggtgtggggcatcacgctgctgatcggcttttcggtggcgtactttctggcattccacgtgcgctcgtcgaccatgcagacggtgctcttcgtgctgtgcacggtgccgttctggacctccaacgtgatccgcatgatctcgtgggtgccgctcctggggcgcaacggtctggtcaaccagatgctggcgggcctcggcctcgtcgaccatccggtcgagtggctgctgttttccaatttctcggtggtgctcgccttcgtgcacctctacacgatgttcatgatcgtgccgatcttcaacagcatgatgcgcatcgaccgctcgctgctcgaagccgccagcgacgcgggcgcctcaagctggcaaacgctctggaacgtggtcgtgccgctgtcgcgcaccggcattctcatcggctcgatcttcgtcatcaccatcgtgatgggcgacttcgtcaccatcggcgtgatgggcggccagcagatcgcatcgatcggcaagatcatccaggtgcagacctcgtaccttcagtttccgctggccgcggccaacgcgatgatcctgctggcggtggtgctgatgatcatctgggggctcacgcggctcgttgatattcgcaaggagctctgatgagccaacgcatcggagaacaacgcgcccccggcttctggccgttggcgatcgtgttcgccctcttcgtgctgttcctctacggcccgatgatcacgatcttcatcctgagcttccagggccccgaaggcggcctgacctttccgctgcgcggcgtttcgctgcactggttccacaaactggcggagggcctgggcaccgtcgacatcggcgcggccttcaggcgctcgctggcgctcggcgcggtggtgatggcgttcaccgtggtgctgtcggtgctggccggcctcgccttccgcaagaagcttgcgggcagcaacgcgctgttcttcgtcacggtggccagcctcatcatgccgtcgatcatcatttctctgggcatcggtctgcagttccggctcatcgacaccggcatcaagagcctgctcacggccatggacgccaccaccctgctcgaagggtacggcaccgcgctcggcctgttcagctccgcactcggcgcccacctgacgtggaccctgcccttcgggctgctcatcatgttcgcggtgttcaaccgcttcaacccggcctacgaggaagccgcgcgcgacctcggcgccacgccctggcagaccttccggcatgtggtgctgccgctgatcggtccgtccatcgtcggcatcggcatgttcggcttcacgctgtcgtgggacgagattgcccgcacctcccaggccatcggtgacgtcaacacgctgccgctcgagctgcagggcctgacctcgaccgtcacgacgccttcgatctatgcgctcggcacggtgaccaccgtggtgtcgctgctcgtgatggccgtggcgctgggcacggccgcgctgctgcgccgccgcgccgttcggccgcgctgagaccgggaccggcctcaaccgaaataagggtgctccaggggaaacagtgcccgcttgacgaacgtgcgccattgcacaggcgcgcgttgacccaacacgaccaagcctgcgctataggcgtaggcccggaattgcggcgtcaggcctgcgagcgcttcttcggcttggcgcgggtccctgctggtccgcagcacggtcacgaaggcacgcaccctctgtgcgtcgtcgggcgacatgtatttgagcaactccatctgcttgtccatcgagcccccatgcttgattgccaggccgatgccgggcaacagagactcgaagtcgccgatcgtcatcgcctggctggcatcgagcgccttcgccacctgcttcgggctcgccccatccgacgcgccgatgaacaccagcaggcggacgggcggctgcgtgcccgacgtcgcgatagcagaggctttgtccagattgccgcgactcatctcgatgtagccgaacgcggagctctccggaggaatgtccttgccgttgccaaggacctgctgcatctgcaggaagctcgacttggccgcaagatcgtcgagcgacacggtttcgccctgttcgatgcgccggatgcgcgccaggtcgtccgtggtgatctggctcaggagaggcgacttggctcccgccctttcgtaggcccggcgcgcttcgggccaggcctgttctcccgcccaggcatgcccggcggcaaaggcgaaccaggcactgtccgggtgctcggccgcgcccttcttgaaagccgcgtccttggcaggactgtcgtccatgcagcgcaccaccagatagccgagatcgctcgcagcctgatgggcttgcgccaatgcgcgatgctgcccgcaaacgcgttcgcgcgcttcgggcgtgctggcgtggttctgctgttcgcgcagcgaggtgacttcgagcggcgcgcgctccaaccgcgcggcgatgatctgcgcgcggttttccggggcgtactgatcggcggccgccagccattcgagcaggtagggtgacttttccgaatcccacctggcgtgtgcctcgatgagcgccttgcggtcgctctcggcgtcgatcatgcccagtgcgttgttcgcggagcgggtctccgggccgctgatgaccgagcgcgtgccgccggcgctgcccttgggagtggtgatctgctgcggcggtggttcgaacagcgcatctgcggactgcatcgaccagcgcggcgccccgagctttctttctgggggtggcgatccacgtccgtacatcgcggtccaagcaaccattggcgcagcccctgccacgttgtaaacgtaacgcacgccgatcagctccgggttggccgaaaacgattcgatcttctgcccctcggtcgtgtgcgaactgagttcgatcgtcttgtcggcctcgacttcgaaagtctgcctgccgcccgccgggagtgttgcgctgctgccgccgatgcggaccttcacctggcggtcaagcccattgaatgcaatgacgcgggcgctgcccagcgaggtgctgatacccatcaggcttgcgatcacaccgccggccacggtcaaccgcgccgcgccggcccaccagccgtccgccgtttgaaacctcgaccaggcatcgagctttttctgccgtggtctttcctggccacttgtcagcgtggcataggtcgatggcaccacgggcgcgtctgatgctccgcccgccgcctccggcgacaacggctcggccgcgatccgtgcttcggtgtgcagcagctgatcgagtgcggcacgccgcaaatgccccagcgcgcgcagcatcggcttcagccagctgtccacgtgcttgatccattcgttgaggttttcgcgcgtcgggtacccgaattcgaatttccccaccagcgaagcccagctgtcgtggcccaacaaggccaatgcatcggcgccggcctggatgtcgggtgcatcctttccgatctcggccatggcggtgaaaagcgcgccggcatcggcgtgcacgcgctgagcctcggcgtcattgactttgcgtttggcagtgaccattgccagggtgttggacaacgtggattgcagatccgccaggttggcttcggcatgttcggcatagtgcagaagccgcaactgcccaagccacgctgcttcccattcaggccccttgacgacggccaatgcatgtagcgtggagcggcagcggcggtcttgcgtttcgagctcgcgctcgacgtcggcgatgtcgcgagagacctcgtcgatggcgccgggcagttcgcgcttcttgatgcccttgccccgatgttccaggcgcggaccttcggtgcgggcaatgccctcctgaacggcgaccagcgcggcgcgctcgtgcagcaacgcatcgagccgctcgagcatgcccgacagcgaatccggatagagctcaggcagcgaagccgcggcgtccgaagcgctcatgcggtcgaagagctgctcgaccaggttttgcgtgcgcgtaacggtccgcgccagatagatgccgcgatagcgccttttgtaggactcccggtcgtactcggcgtcgagtgcctccgccgcggcctcgcgcgtgccggtcagcggcggcggaacgatgtggctgatcatgcctgcgcagatgcgttcccggaatgacaaagcctcgtcgaacaggtcccacgcggagctttgccgggcttcggccgcgaggtaggttttcttggcgttctcctcgcgctcgtggctggctggatgcgtggcccacatccgcgacaccgaaaccttgtcgcgcttgaagatgcgatgcgcctcggggccctgcgttggcggtggcggtggaatcccgtagccgggatcgtcaaggatcacccgcagtttctgcagaatcttcgactggatctcatagagatccgggacggctgtgcctttgtgcaattgccggtttgcgaaatcgagcgtacggtcccaggccgcatcggccgcctgcatcctgtagagcgcctcgatcagcgcgtcgctacccgccaggctcaccgaaacacgatcggcctggaattccatctccctggacagcgcacggtcggccagcacgacgatgcgaaacaggctgtccacgacggagcggatggaccacaccaacagcgagaaaagccaacccacccaggcaatgcgaatgtcggtacgcgaaagaccttcgagaaagcgatcgagccggtcgcgcttggccacgacatgcgccgcgatctgctgcgccaggtagacccaacggccgaccgccatgctgcgctgcgcgaagtgcccgaactcgtgcgccagcaccgccttgaactcggagacggtcagcacattcaccagtggaaggccgatctccaggtttttcttcgaggggaagaagaagttgagcagcgaaaggtcgtagaacaccgccgcattgacgcgtgacgacacatataccctcgcaggccgtggggcccgggcttcgtccgccagacggtgcagaaaggcgaacagcctggggtgctcggctgccgtgatctcgaccgaaacgcccgtctcgccgcgccgtacgaacaccagcgccttcagcatgaacacggcgaggaacgcggcccccaggcccactcccatcagcaataggccgtcgccgccggacccatagaccgaagcccggatggactgatacgctttccacgccagccagcccgagaacagcaggtaagccgcgataaatgccatgagcgcgaacattgcgagccaggcatgccgccgataggcaggcgacgctttcgcgagttggctgccggtgccagcgggacccgctggataaagttgatccatgttgttccctcttcctcgcacaattgattgttctgcgggtggcacttcggtccggcagcaacacccaacggccagcccagccgataattccacgcattgtttacagattcttgcatctgcaaaagaagaccagagggaaaaaatgctcgaaaaactcaatgaattcacagaaagccacggcgagctgcgccgcggccgaggccttgtcacgggaaccattgcgctgagcctgggcatcctgtgcttcctgggcgtgctggcgttccactttccgcagtacctcacgacgcccgagttgcgcaagagctacaacgtcgacgtgatgcgcttcatcctgctggcggccatggtcgtcgcgggcgggatggcgctggtgaacatcatcttcaaccgctcgcgctggctgtcttctgccgcgttcctgctggtggtcgcggcggcgctgctgggcgggcacaaggtgccggtgaacgactttgccgacaacacgccctacatcggcctggactggttcatcctcgacctgctgggctcatcgctgatcttcatcttcatcgagaagctcttcgcgctgcgcaaggaccagccggtttttcgcgccgaatggcagaccgacttccaccacttcgtggtcaaccacatgatcgtgggcttcgtgctgctggccaccaacctgatggtgcacaagttcttcggctgggcggccaacgacggcattcgcggctgggtgggcaatctgccgttctgggccgggctgcttctgatcgtcctggtggccgacctggtgcagtactggacccaccgcgcctatcacgaggtgccggtgctctggcgcctgcatgccgtgcaccacagcgtgaagagcatggactggatggccggctcgcgccagcacatcctcgagctgctgatcacgcgcacgctggtgctggcccccatctacgtgctgggcttctccaaggaagtgatcgacgcgtacatcgtggtggtgggcttccaggcggtgttcaaccactgcaacgtgagcgtccggctcgggctgctgcgctacatcatcgtgacgcccaacttccaccactggcaccacagccaggacgtcgaggcgctcgacaagaactattcggcgcactacgcttttctcgactatctcttcggcaccgcggtgaagagcaccaagctctggcccgagaagtatggcgtgctcggcgactacgtgcccaacggcttcttcaagcagttgaagtttcctttcgtctggaaaggatgatgcggcgccatctcggcgcggcggcgctcggcgctgccgcaatgctgctgctctcggcctgcgccacccgcgtcgacctgccgtcgaaagacgcgggcctgcgcctgcgcgtgcagagctcggtcatcgcgcccggcaacggcggcgagctgatcgccgccgacgcgctgcagcccggcgacatcctgctgacctccattgccaccgtcaattccttcggcatccggctgggcaccttctcgcccgtgagccacgccgtgctctacctgggcgacggcctgatcgccgaggcagtgggcagcggcgtgcgcgcgcgtccgctggccgacgtggtggacgaagaacagatggtggtggcctttcgcgtgcccgggctcgatgccgcgggtgcccagaaactccgcacctgggccaactcgcaggtaggcattcgctacaacaccaccggcgtgctgctgaatgcgcctttcgtgctgaaccggcgcctgtgcgaactgccgctgattccatcggccgtcagccactattgcatcagcggcatggcaatggtgcagctgggcgcgagccgcgacgaccagttcttctgttcgcagttcgtgctcgaggcctaccgccgggccggcctgccgatcaccgacgccgacccgcgctgggtgagcccggccgacctgctgcacatgcgcgagggcgacgtgccctcgattgccgccacgcagccgctgcgctacgtgggccacctcaagtacaacccgccgccgctgcttgccgctgacggcccctgaccgccttgagcaattcttcttcggatcatttcgacgtcgtcgtggtcggcgccggtgccgcaggcctgttctgcgcggcgctggccggccagcgcggcttgaaggtgctgctggtcgaccacagcgaaaaagtggccgaaaaaatccgcatctcgggtggcggccgcgccaacttcaccaaccgcgacctcgacgtgcgcgcgccgcagcgccacttcatcggcgacaacccgaatttctgtcgctcggccctgtcgcgctatgcgccgcagcagttcatcgaactggtgcagaagcacggcatcgcctttcacgagaagcacaaggggcagctgttctgcgacggctcctcgcagcagatcatcgacatgctgctggcggaatgcgacgcgggcaacgtcacgcgctggcagccgtgcaagctcggaaagatcgtgttttccacttccggctgccctgatgcgacgagcccaggcagctaccagatcgatagcagcaagggcttcgtcgaaacgcccaagctcgtggttgccacgggcggcctgtcgatcccgcagatcggcgccagcgatttcggctaccgcctggccgagcagttcggcctgcgcgtcgtcacgccccgcccggccctggtgccgctgactttcggcggcgaagcctgggcgccgtatgccgaactggccgggctggcgctgccggtgcgcatcgaaaccggtgccaagaaggaaaagatgaccttcctggaagacctgctgttcacccatcgcggcctttcgggcccggccgtgctgcagatttcgagctactggaagcccggcaccccgctcacgctcgacttcgcgcccggcgtggacgtggccgaagccctgggcgacgccaagctccgctcgaagaagcgcatcgccaacgaactggccatgctggtgccctcccggctggcggatgcctgggtcgggcaggatccgggcctgcagcgccccgtcaacgaggccgccgacaaggccctggccgccctggccgagcgcattgcccgctggcaaatcacccccagcggcaccgagggctataaaaaggccgaggtcacggccggcggcatcgacacccgcgatctgtcctcccagaccatggaatccaggcagccgggtctgtatttcatcggcgaagtggtcgacgtgacgggttggttgggcggatacaacttccagtgggcctgggcgagcgcacatgcgtgcgcaaccgcgctataatcgcgggctaactttggcctcccctcaacggccgcaaaaatttttcagttgaggaaccccggcttggggcctcgatctccccgagccaaattcagttcaacgattcatcaatgaccaccatccgcgttaaagaaaacgagcctttcgacgtcgccctgcgccgcttcaagcgcaccatcgaaaagctcggcctgctgaccgacctgcgcgcccgcgagttctacgaaaagccgaccgccgagcgcaagcgcaagaaggcagccgccgtcaagcgccactacaagcgcgtgcgcagcatgcagctccccaagaagctgtactgatgcccgttggcaacaggatcgccggcctttgacgcaagtcggcccagcgatccgattgctgcctcagccgcgccagggaaacctgccgcggcttttgtttttcccgaaccaggagccccgagcatgagcctcaaggaacagatcaccgaagacatgaagaccgcgatgcgcgccaaggactcggagcgcctcggcaccatccgcctgctgctggcagccctgaagcagaaggaagtcgacgagcgcgtggaactcgacgacgccatggtcgttgccatcgtcgacaagatggtcaagcagcgcaaggactccatcgcggcgttcacgaccggcgggcgcgccgacctggccgacaaggaagccgccgagatcaaggtgctcgaggtctacctgccgcagcgcatgggcgccgacgaagtggctgccgaagtgaaggccatcgtggccgagctgggcgccaagggccccggcgacatgggcaaggtgatgggcgcggtcaagacgcgcctcgccggcaaggccgacatgggccaggtgagcgcggcggtcaaggcggccctggcgagcgcctgatgcgcagcggcggcgccggcgccaccacgacgatcccgaaggcttgcgcctgcctggtcgatgccaggggccggctgctggtgttccgccatcccggcgacgggaacatgcagctgcccaagggcaccatcgagcccggcgagtcgcccgagacggcggtgcgccgcgagctgctcgaggaatcgggcatcgaccacgtcggcgaactgcagccgctcggcaccctgcagcgcgactgcgaggccggcatcgagggcaacacggtgcgccatccccagctgtggcatcttttcctgatgcgtgccgacggcccgctgcccgaaaccttcgagcacgtggccatgggcagccccgaggaagacggcctggtgttttcgttcagctggctcgcgcccgacgacggcatcgagaacttcgccctgccctacaggcaggccatcgcacgcgttcgcgcggccttgctcgccccctgaagatcgcaccggggttcttcggaggctcacctggctcaggccagcgcgtgcgccaccatgtagacccccaggagcgccaatccggccaggaagcagcgccggaacaccgccaccgacaagcgctggcgcagccacgttcccagcaccatgccggcgagggccggcagcaacatcgccaccgacccgccgaccgccgaagcgggatagctgccgttgccgaccagcccgatggccagcaccacggtcgaggtggtgaacgaaatacccatcgcctggatcaacgcatcgcgctgcaaacccagggcctgcagatagggcacggccggcaccacgaacacgccggtcaccgccgtcaccagacccgtcgcggcgcccaccagcggccccagccagcgctcgtgcgccgcgggcacatgcagctgccgccccgtgagcccccagagcgcataggccaccagcgccacgccgagcgccaccgaagcccaggcgccagccggcaccccgagccacagcgcgccgcccagggaacccaccacgatgcccgcctgcatgccaccgatgcgccgcagcaccggccagaaggtcgcgcgcggcccggtctgccaaagattggtgaccagcgagggtgcgatcaacaacgcggccgcgcgcaccggcggcatccacagcgcgagcagcgccatcgacactgtcggcagcccgagcccgaccacgcccttgatcaccccggccaggagaaataccgcggcggccgcggcccagtggcctgttgccagttcgttcgagatcgtcattgcggcgcagtctgccggcctgtgccgaggctgaaaatgcggcattcgcgcagccagcctcaggcacaggctgaggctcccgtgctaccttgcggcctcaccatgcgattcgatctcacagacctgcggctcttcctccacgttgtggaggccgggagcctgaccgccggcgcacagcgctcgcacatgacgctcgcctcggccagccagcgcgtgcgcggcatggaggacgcccttggcagcccgctgcttacgcggcacgcgcagggcgtgcgccccaccgaggccggccgcacgctgctgcaccatgcgcgtgtcgtgctgcagcagatggaacgcatgcgcggcgaactcggtgaatacggccagggcctcaagggccacgtgcgcttcatgtgcggcacctcggcgctgaacgagcacctgcccgaggtgctgagccgctttcttgcgcagcatccgcgcatctcggtcgatctcgaggagcggccgagcccgcaatcggtcgatgcgctgcgcgccgggctgtgcgacatcggcatcgtctcggacgcggtcggcaccgaggggctcgaatgccaccccttccgccgcgacgatctggtgctcgtgatgccgcgtggccatgcgctcgcggggcgccggcgcgtgcggctggccgaggtggccgacagcgaattcgtcggcctgaccgaggacagtgcgctgcagcagctggtgacgcagcatgcccgtgcgctcggcaagcaactggcctaccgcgtgcgcgtgcgcaacttcgaggccgtgtgcggcatggtcgcgcatggcatcggcgtgggcatcgtgccgcagaccgcggccgcgcgctgcgcccgctcgatgaagatcgcgcgcgccaacctcagcgatgcatgggccgagcgcacgctgatggcctgcgtgcgttcgtcggaagatctgccgctcaacgcccggcggatgctcgagcacctgttggcgccgcccgagaaggctgcggcgaagtaacctgaacgcgaggccggctgcggctcagcgcggctggagcgcaagcagctccgccatcttccgcagcgcttcttccggcgtcggcgcgatgtggatcgaacaggccagcatcaggttcagcggctggccgaaatcttccaccgcgatgccgctgccggtctcgcgcagcaccccggccgcatcgggcgcgcactgcaagagagaccgggcccggtccgcatagctgcccgcaggcacgccgtaggccacgaccggaatccccagcgccaccgcagcgcccacctcgaacactgtccctgaatcgggctccaggccgcggaagcacgcgaggttggccaccacaccgtccgcgccgcgaagccgctgcatgttggcctcgtagatctgctcttccggcgcgccggcgcctggctgatcgttgccatcggccggcagcagggccgcaagccccagcgcatcgcaagccgccgcgagcctcacgaagtggtccctggcgtcggggcgaaagacgtccgggcccgcaaggtagatctgcgggcgggcctgtctttctgggtcttgattcattgaaagcacatcttagccgcgcgcttctgaagggccgttgcgctctatccgctgagggcgatcaggcaaaccatcaaatagcacggtccgcaagtgctcagctgccggccaccttcatgcggttgaccagcaccgaccccgtggtcttggcgccgaaggtgtaggcatcggccccgatggcctcgatgcccatcagcatgtccttgaggttgccggcaatggtgatttcatgcaccgggaaggcgattcggcccttctcgacccagaagccgctggcgccgcgcgagtagtcgccggtgacgtagttcacgccctgccccatcagctcgatcacgaacaggccggtgcccagcttggccagcatggcgtccaggtcgtcgcccggcttcgtgaggcgcgaattcagggtcaggttgtgcgagccgccggcgttgccggtggtcttcatgcccagcttgcgcgccgaataggtcgagagaaagtagccttcgagccgccccgcgtccaccaccttgcgcgcgcgggtcaccacgccttcgtcgtcgaacggcgagctgcccttgccgcgcagtacgtgcgggtcttcggccacgtccacgtgcttgggcagcaccggcttgccgagcgaatcgagcaggaaggtgctcttgcggtacagcgccccgccgctcacggcctgcaccagcccgcccaagaggcccacggccagcggcgactcgaacagcaccgggcactcggtggtcttgatcttgcgcgacttgagccggctcagcgcccgctcggcggcgtagcggcccacggcctgcgggctggccagttcgccggccgagcgcatcgagctgtaccaggagtcgcgctgcatgtcgtcgcccttgccggcaatgggcgcaaccgaaatcgaatgccgcgagctggcatagccgccgcggaaaccgtgcgtgtgggcgctgaaaaagtggctctgctgggccgaaacgcccgcgccttcgctgttggtgatgcgcttgtcggtcgaaagcgccgccgcttcgcactcgagtgccagcctggcggcctgctcgctcgtcacatcccaggggtggaacaggtcgagttcggggtgttccttggcgatgtcttcctcgtcgggaaggccgctgaccgggtcttcggccgtgaagcgggcaatgtcgtaggcggcctgcaccgtctgggcaatggccgcctcggagaagtcggaggtgctggcgttgccgcggcggtggcccacgtagaccgtgatgcccagcgacttgtcgcggttgcgctcgacgttctcgagttcgcccttgcggaccgagacgctgagaccgcagccctcggaggcctcggcgccggcatcggttgcaccgagctttttggcgtgggccagggccgagtcgaccaggttttcgaagaaggagcggctgtaggcgaagccggaatcggcgcgcgaggaggatgtcgtcatgtggtggctatgatacttgcgccccccacattccgttttcccttcagcttcccactgcgcattgcacgcgttgcaacgccgcacggtgcggcccagaatccaccccatgtcccgcaaacccaaaaaaggctatttcgtccgtggccagttcgtcgccgaaggcagcgagctcgacctggagctcaagcgcgagctcaagggcaccgacgaagccagccgcaccgatctcaagcgcgaaagcgacgaactgcaaaagctcggaaccgaactgctcggcctgcgcgccggcctgttcgatgcgctcccgctcgacgaaaaactggtcgacgccgtggccgaggccaagcgcatcaccaatttcgagggcaagcgccgccagatgcagttcatcggcaagctgatgcgcaaactggagcccgaggtgctggaggccgtgaagctcgccctgaccgagcagaacagcgtgccggcggctgaaaccgccgcgctgcacgaagccgaacgctggcgcgaccggctgattgccgacgacgatgcgctgggcggctggatcgaaacccaccccgccaccgattcgcagcagctgcgcgccctggtgcgccaggcccgcaaggacatgaagtccggccccgccggcgaagcgccgcgccagggcaaggcttatcgcgagatctttcagctggtgcgtgcccagctggcggtgcatggtggcgccgaccacgctgcggaggctgccgcgcaagaccgggaagacgacgcatgagctttctgacttttgactttctccctctcccgcttgcgggagagggtcggggtgagggtcgacggcctgtccacgcgtacgctctttccaccgccagcagccctcaccccagccctctcccgcaagcgggagagggagcaagaggcatgagaccatgagcacacccgaccccgtacgcatcggcatcgtctccatcagcgaccgggcctccagcggcacctacgaggacaagggcctgccttcgctgaaagaatggctcggccgggcgctgaagaaccccatcgatttcgaggcccgtctgattcccgacgaaacggccctcatcagcgccaccctgatcgagctggtcgacgccggctgttcgctggtgttgaccaccgggggcaccggcccggccctgcgcgacgtgacgcccgaggccacgctggccgtggcccacaaggaaatgcccggcttcggcgagcagatgcgccagatcagcctgcgcttcgtgcccaccgcgatcctttcgcgccaggtggcggtgatccgcgacaagagcctgatcatcaacctgccggggcagcccaagtcgattgcggaaacgctcgaggggctgaaggacgcggacggcaagcaggtggtgcccggcatctttgccgccgtgccgtactgcatcgacctgatcggcgggccgtacctggagaccgacgacacggtctgcaaggcgttccggcccaagtcggccatcaggaactagcccacgggcctgttctcttcgctccgccggtgcgccatgcggtagagcagcggcagcaccaggagcgtcagcatcgtcgacgacaggatgccgccgatcaccaccgtggccagcggccgctgcacttcggcgccggtgccggtggcaatcgccatcggcacgaagcccagcgaagcgaccagcgcggtcatcagcaccggccgcagccgcgtgagcgcgccttcgcggatcgcagcatcgagcggcagcccaccctcgcgcaggttgcggatgaacgagatcatcaccagcccgttgagcaccgccacgcctgaaagcgcgatgaaccccaccgccgccgagatcgagagcggaatgccgcgcagccacagcgcgacgatgccgcccgtgagcgcgaaggggatgccggtgaacaccaggagaccatccttcaggttgccgaacatcgcgaacagcagcgtgaacaccaggagcagcgacaccggcaccaccacctgcagccgctcggtggccgaggccaggttctcgtactggccgccccaggctgtccagtagcccggcggaatgctcaccttgcgcatcgcttcctcggcctcggccacgaaggagccgaggtcgcggccgcgcacgttggcgctcaccacgatgcggcgcttgccgttctcccggctcacctggttggggccgggcgccagctccagcgtggccacctcgccgagcgggatgaagctggtgcgctgctgcgcctccgcgcccgcaccccggggcagcgccacggggaggcgcttgatcgcctccaagtcggtgcgcaggtgctcgggcagccgcacgaggatgtcgaagcgccggtcgccgtcgaacagcgtgccggcctcgcggccgccgaccgcgatggagacggcgtcctgcacgtcgcccacgttcaggccgtagcgcgcggtcttctggcggtcgatgttgaccgtgagcatcggcaggccggtggtctgctcgaccttcacctcggccgcgccggggatcttgcccagcacgcccgacacctcggccgccgtcttgttcagcacctccatgtcgtcgccgaagatcttcacggccacgtcgctgcgcacgccggagatcagctcgttgaagcgcagctggatcggttgcgagaactcgtagttgttgcccggcagcttttcgacctcttcctgcacggccgccagcagctctgcgcgtgtgcggcgcggtgtaccttgcgacttgggccactcgctctcaggcttcagcatgatgtagccgtcggaaatgttcggcggcatcgggtccgatgcgatctcggccgtgccggtgcgcgcgaacacgcgctcgatctccggaaacttcgccttcagcgtgcgttcgatctgcttttgcatctcgaccgactgcgtgaggctggtgcccggaatgcgcagcgcctgcacggcgaagtcgccctcgcccaggctcggcacaaactccgtgcccaggcgcgtggccagcaggcccgagagcaccaccgccaccaccgcagtggtgatgaccagcggcttggctcccatggcgcgcgccagcagcggcgcgtagccgcgcctggcccagtgcatcaggcggttctctttctcgcccaccttgttgccgatgaagagcgccacggccgcggggatgaacgtgatcgacaggatcattgcgcccagcagcgcaatcaccacggtgaaggccatcgggtggaacagcttgccctccacgcccgtgagcgcaaagatcggcaggtacacgatcatgatgatcagctggccgaacaagagcggccgccgtgcctcctgcgaggccgcgaacacttcatggaaacgctcgctgcgcgtgagcggccgcccgtgcttggcctgcgcatgcgcgaggcgccgcacgcagttttccacgatcaccaccgcgccgtcgatgatgatgccgaagtccagtgcgcccaggctcatgaggttggcgctgattttctggttcaccatgccggtaaaggtgaacagcatcgacagcggaatcaccagcgcggtgatcagcgcggcgcgcatgttgccaagaaacaggaacaggatggcaatgaccagcaccgcgccttcgagcaggttcttcttcaccgtggcaatggccttgtcgaccagcacggtgcggtcgtacaccgtcacggccttcacgcccgcgggcagcgttcggttgatttcctgcatcttcttgtcgaccgcctgagagacggtgcggctgttctcgccgatcagcatgaacacggtgcccagcaccacctcgcgcccgttgtcggtggccgcacccgtgcgcagctcctggccgatgccgacctcggccacgtcctgcacgcgcagcggaatgccgttcgcgttgcccaggatgacgttgccgatgtcttccgcggtcttcacctgccccggcgcgcgaatcaggtattgctcgccgcgcttctcgatgtagcccgcgcccacgttggcgttgttgcgctccagcgcggccaccaggtcggtcatcgcgaggccgtgtgcctggagctttgcagggtcgggcgcgatctggaactccttggcgtagccgccgatggagttgatctcggtcacgcccttcacgttgcgcagctgcggcttgatgatccagtcctggatctcgcgcaggtcggtcggcgtgtagggcttgccgtcggccttcttcgcgccctcttccgcttccacggtccagagatagatttcgccgaggccggtcgagatcgggccgatcaccggcgagatgccgttcggcatgctttctcgcgccgactggatgcgctcgttcacgagctgccgcgcaaagtagatgtcggtgccgtcctcgaagatcaccgtcacctgcgagaggccgtagcgcgagagcgagcgggtctgctgcaggcccggcaggccggccatcaccgtctcgatgggataggtcacgcgctgctcggcctcgagcggcgaatagccgggcgccgccgtgttgatctgcacctgcacgttggtgatgtcgggcaccgcgtcgatcggcagcttctggtagctgaagatgccgagcgcggccatgcccagcaccgcgagcaggatcagccagcgctgttcgatggaaaaccggatgactcgttcgaacatgcggcgtcctcagtgggtgtgcgtggcagagctcttgccctgctgagacttcacgacgaagctgccgctcgccgcatacgcggtgccgggcacgaggccgctcacgatctcgacgcgccggccgtcgctgcgcccggtctgcaccgcctgtggcatgaagccgccgggcaccttggcgaagaccgtgggtttgccttccaccgtctgcaccgcctcggccgacaccgtcaccggggcctcggcttcggacgaagcaagctccacgttcacgaacagtccgggccgccacacgcgctgcggattcgtcaccgtgacgcgcgccgtcgctgtacgcgtctgcgcgccgatgagcgagcccaggtacgacaccgtgccgctggcggtctggtcgaaagcgctggagcggatggtcaccggttcgccgatgcgaacgagattgaggttgttggcagccacgctgatctcggcccagaccgtggagaggtccgaaatggtgaacacgctggcgtcttccttgaccgactcgccgagcgagatgtgcttctcgaccaccatgccgtcgaacggcgcgcgcagctcgtagcggccaagcgccgacgagcccggcgtggcgcccagcgccagcagcttctggttcgcgttggccacggcaatctgcgcctcctgcatggcctgctccgcctgcaggtagtcctgctgggcggagatcttttcttgccagagttttttctcgcgctcgtaggtggtgcgggcaagcgccagccggcgctgcgccgactgcagttcgctgcgctgctccgagagccccgggctcgacagcaccgccagcacctggccgcgcttcacctcctggccaaggttggccggcacgctctcgaccacgcccgccacgcgcggcaccacgtgggccgtgcggtcttcgttgaacttgatctcgcccggcagttgcagcaacgaccggatgcgcgcggggccggcgctttcgatggccatgccggcggcctggacctgctcgtcggtgaagacgatttttttctcgtcttctcgttcttcgtgcgcctcgccggtgtggcccttggcctcgccgtggccatggccgtgttcgtcgccctcttcatggtgctcgccctcggcgtgctctccggcttccgaatgtccggcggcttcgggttgggcgggcgtggtgcgcaggatcattgcgccggccgcgaggcccaccaccagcacggccacgatggccagccactgcttcttgccgatacgttcggcaaaggtcttgcgttcttgcgtgttcatgattcgtggagtccttgtcagcgcggagcgggtgccgcatggagggtgtcgccgccgccggtgccgagcagccggtcgagttcgccggccgcgcgatgcgcctcggccagggcgagcaggtgctggttgcgcacctggaacagcgtgcgctgggcatcgagtgcgtcgagaaagctgaacttcccgagctcgaagccccgggcggcggcctggcgggcggcttcggcgccgggcagcgcgtcgcgctggagcatctgtgcggtggcgcgcgccgaacgcaggcgctcggtagcctgcgccacgtcggcacgcagctgaagttcggccgccagaagatcgtcgcgcgccttctcttcgcggctcagcgcctcggcgacgttgccgcggttggtgtcgaagatcggcagcggcaccgacacgcccaccacgacctggttgcggccgctgccgctgcccatgccttcatcggccggcacgcgcttcgcgccgagcgacacggtgatgtcgggcacgcgccgggcctgctccagttccgacagcgcctggcgccgttcgacctcgagccgcgcctggcgcagcaccggtgcctcggaaagccggctctgcacgtccgcaaccgctgcgggcaacgagtcgagcgcgccgtctgcgtgcgtgaagcgtggcgacgcattgccccagagcgcagcgagttgccggcgcgccgagcgcagcgcgccctcggcctgcagcagctcgacgcggatgccggcctcggccacgcgcgcccggttctcctcgagcggcgaaaccttgccggccgccacccggttggcggccgcgcgggttgccacttctgcaagtccgaccgagtcttgcgccagccgcaagcgctcctgcgcggccagcacctcgaagaacagcgtgatcgtcgacgcacgcaactcggaacgccgcgcaagcaacgccgattcggcctggtcgcgggcacgctccgccgccgtcacgcgcgccgcgcgcttgccgcccagctcgatgggctggctcagctgcagcgtggtggtgcggttgtcgcgccgcaggtcttccacctgcgcgccgaacaccgggttgggccaggcgccggcctgcaccacggccgcatcggtggcctcccgttcgcgcgcggcggacgagagcccggggttgaactgccgtgccagcgcgagcgcgctgggcaggtccagcggacctgcgggttctgccgctccgggggcggcgtgcccgagcggcgaaggattggaaccggcagtggattgtgaaaatgccgggaacaccgccaaggccatgacggccagcggcacgaagagcgtgcgcatcgaattctcctgggttgcaaaacaacgggcgggggaattcggcgagagctcagctgatgatgagtatcaggaaaatgggttgttctctcgccgaatcaaagggcgagaggccaggcaggaggcacgggcacttcggagatgtgcgagacgaaatgttccgcgcgcatggcgcgcagtgcctgcgccattggcggtgcatgcacgcgatcggccatcgccggcaggtgttgcgcgtggcccaggtggcagacggcgcaatctccgagcacggcgttgggctgggtgccggggctcttctgcgcgtcgtcggtggtgcgcaaatcgcccgcgctgttgctcggctcgtgctcgtgatgcccccagtggctcggttgcacatcgcgttcatgctggcaataggccgccgacgccgcccagctgaactggaacggaagcaaaagcagcaagaagatctgaagccagcggcgcatggtgcaaaaagtatatcggcgccgtggggcccgccggtctgcaatgcccttgcagtttgcaggttgcggcgcaatgtacgacaagcgcgcggcgtttcggctgtcgttcggcgtgcgaatccataacttccgccgggccactccacggcggacatttcatcgatgagaattctcgtcatagaaggcgagcccggactgggcgacgatctgaagaagggcctggaagcaagcggccatgtgctcgacaccgcacgcgacggcgtcgaaggccgcttgctggccaccctggacgggtacgcgctgatcctgctcgacgtgacgcgccccgggatcgacggctttgcggcgctgcaagccatccggcgcaccagcaacgtgcccgttctggtgctcaccgaccgcgacaaggtcgaagaccgggtcagcggcctgcagcacggcgccgacgactacctcgtcaagcccttctcgctttccgaactgctggcgcgcgtggaggccctgctgggccggggcacgcgccaggcgtccaccatgctccggcttgccgacctggcgctggacccggccagccgcacgtgcgttcgcaaccgcacgcgcatcgacctcacggccaaggagttcatgctgctggcgctgctgctgcgccaccacggggagatactttcacgccgcacgctcggccaacaggtgtgggatgcagccttcgagaacgaaagcaacgtggtcgaagtgaccattcgcaggctgcgcagcaagatcgacgacgctttcgacgtcaagctgctgcacacggtgcgcggcaggggctacgtgctcgaagatcgctcctgatcgcgagccccgggccgcccccatgcggcaccggctcacgcatccccggtgtcagggtttggcaggcgcctctggcttgccctcggcgtcgccggcacgcggcgccttgcggccaatgcacagcgtcatcagcggccccgtcatcgcggtggtggccagggccatcaccagcagcatggtgaacagctcggggccgatcagtcccacgtcgaacccgatcttgatcacgatcaactccatgagcccgcgcgcgttcatcagtgaaccggtggccaggctgtcgcgccagctgtagcccgcgatgcgcgcgccggccgcgccgccggcaatcttgccgacggtggccacgcccacgatcagcagcatcgcacccaggctcgcaccggagaaggcattcgccgtggtgcccagccccgcaagcgcaaagaacagcggcatcagcacgacgatggaaatcggctcgatgcgttcgctcagcgagcgcagcaggcggtcgtcgcgcggcaggcaggcaccgaacaggaaggcgccgaacaccgcgtgcaggtgcagccattcggtcagcagcgcggtgagcaacaggccgatcatgagcgaggccatcaccgtggtcgaaggctcgccgtcgggcgccttcacgcgcagcagccaggcaaaggcgggcttcaggccgaagaacaggaaggcgagcatcacgaccacgccgacggtgatcttgatcaggctctcgtagccctcgcccgcgccaaccagcgccaccacgaaagccagcaggatccaggcgaacacgtcgaccacggccgcggcactgagcgagagctggccgaaggccgtgcgcgtcatgccgcggtccttgaggatgcgcgccatgacgggaaaggccgtgatggaaagcgcagccgccatgaagagcgcaaagggccagaaagcgacaccggccggcgcgagcgtggggtacagcgcaggcgagatcgcaatgcccagcgccagcggcacgatcacgctgagcacgcccacggcgcccgccgccttgagttgcgcccgcatgttccgcgtggcccgcaattccaggcccaccacgaacatgaacagcaccagccccaccgtcgacagcgaagaaaggccctgcagcgagtccttggcaaacagctgcgcgtgcagcgaggggaagagcgcgcccatgaccgccgggccgagcatgaggcccgccgccatttcgcccaccacgcccggctggccaaggtagcgaagcacccagccgcagaggcgcgcggtggtcaggatgacgacaagttgcagcaggagagaggtgacggacatcgaggggctggggtcggcaaggggaaacagccgatgttagttccaagccgtgtcgccgaaccagcggttggcccactggttcagcgcgaggcgcttggcgcccccccgggcaactcacctggacgcgcgcatcagccgcaagccgttcgccaccaccagcaggcttgcccccatgtccgcaaacaccgccatccacatcgttgcgccgccgaacaccgcgagcacgaagaacacggccttgatgccgagcgccagcgtgatgttctgccacagcaccgaatgcgcgcggcgcgagaggcgaatcgtttcgggaatgcgccgcaggtcgtcgttcatgatgaccacgtcggccgcttccatggcggtgtcggtgccggcgccgcccatcgcaaagccgatgtcggcctgcgcgagcgcgggtgcgtcgttgatgccgtcgcccgccatgccggccatgccgtagcgctgctgaagcgccttgatggcatcgagcttctcctcgggcagcaggttgccgcgcacgtcgtcgatgcccgcatgaacgccgattgccttggccgtggcggcgttgtcgccggtcagcatcacgggcgtgacacccagcgcgcgcagctcggccatggccgcctgcgaggatggcttgatggtgtcggccaccgcgaacagcgccagcaccgcatggccagaggccagcagggtgacggtgcgcccggcctcctcatgccgcttcagctcggcttcgagcgcggggctgcacagcttctgttcttcgatgaggcgatggtttccaagcacatagctgcggccttcgtgcgtggcctgcacgccgcgtcccggcagggccgcaaagttgccgaccggccggggctcgcgcttcaggccctgggcaatggccttcgacaccgggtggtcggagcggcccgcgatgctcgcggcaatggcaaggatttcgccctcgtccgccgtcttgtcgagcaggctggtttcgaccagcttcggcttgccttcggtgatggtgcccgtcttgtcgagcgcgacggccttgagcttgcgcgcctcttcgaggtaggtgccgcccttgatcaggatgccgcgccgcgcggccgatgccagcgcgctcaccaccgtgacgggtgtcgagatgacgagcgcgcaggggcatgcgatgaccagcagcaccagcgccttgtagacggcctccatccaggtccagcccatgagccagggcgtgagcgccgccacggcgattgccagcgcgaagaccgcgggtgtatagacggcggcaaaccggtcgacgaagcgctgcgtgggcgcgcgcgtgccttgcgcttcttcgaccgcgtggatgatgcgcgccaacgtggtgttggcagccacggccgtgacgcggaattcgagcgcgcccgtctggttgatggtgcccgcaaacaccgcatcgcccaccgacttgtcgaccggaatgctctcgccggtaacgggtgcctggtcgatggcgctcatgccctccgtcaccacgccgtcgagcggaacgcgctcgccggggcgaatgcgcaccagggcaccgagcgccacggtgtctgcctttgccgtcttccagctgccgtcgggctgcctgacatcggccagctcgggcgccagcgccaacaggccctggatggcattgcgggcgcggtcgacggcacgcgcctcgatcatttccgcaatggcatagagcgccatcaccatcgcggcctcgggccattggccgatgacgaaggcacccgtgaccgccaccgccatcagggcgttgatgttcaggcgcccgcgcaccaatgcggcgaagcccttcttgtaggtgtcgagcccggccagcgcgatggctgcgagcgccaaccccatctccaccgccgtgaacccgatgccctccggtgcgagaaaggaaatcgtctcggccgcgatggccagcaccagcgcggccaccagccgccagagctccggcgtcatgaggccggcggcgcgcgccgtgccgggagcgggcggcgcaccggccacctcattcagcggctcaggcttgaaccccgccttgcggatggcttcgagcgcattgggcaaggcagtgtcgtcggcggtgatcgccatcgtccgttcgccgagccgaaagcgcagcccgctgatgccgcgaaccggctccagcgcgcggcggatctcggactcttccacggcgcaatccatggtgggaattcggaagagcaaggcgcccttggggatgtctgcggtattggcggcagcgacaactgccgccgatccacatgcggaactgccgcagcaggcggtttcggccggtgcatgcgaatgagcatgcgcatgcggcgccaccggtttcagagcgttctggttcgtcatgaagtgcattggaaaccctgaagcaggtgtagagtcaaacgctagattcctccactccccttcttgccgcatcatgaaaatcggagaactggccaaggtcgcgaacacgccggtcgaaaccatccggtactacgagcgcgagcagctgctgcccgagccggcgcgcaccgaaggcaactaccgcatctacgacgacgagcatgcgcagcggctgggctttatccgccgctgccgttcgctggacatgacgctcgatgaaatccgcagcctgctgcgctttcgcgatgcgcccggcgaagactgcggcgaggtcaaccagctgctggacgaccacatcggccacgtggccgcgcgcatttccgaactcaagacactggaaaagcagctgaaggcgctgcgccagcaatgctgcgggcctgaatcggcgcagaactgcggcatcctgcaagagctggacaccgccgcgctcgcaacggagccgttcgggcagcacgcgggccatgtgcatgggtcgctgcacacggccgcgaaacgatcgacctgaaaggcctcgctacctgccgatgagctgcgtgagcttctccgcctcgaagctctcgtcacgcgccgcatcgcagggcacgcaatccttggtgccgggatgcgcagacagcttctcgatggcctgccacaagagcgcgatctggtgttcctggctcgcggcactgtcgacgaggccgcgcatggcctggctcagcgggtcgtcgtcctgcgtgatgccgtaggcggagaacttctgcggcgcggccacatcggcgctctcgccggtcttcgacgggatgatgcgtgcgggaatgcccaccgcggtcgcccctgccggcacaggcttgatgaccaccgcgttgctgccgatcttggcgccatcgccgacgacgaacccgcccagcaccttggcccccgcgctcaccaccacgttgcgccccagcgtcggatggcgcttggtgcccttgtagagcgaggtgccgccgagcgtcacgccctggtagatggtgcagccgtcgccgatctcggcggtttcgcccaccaccacgcccatggcgtggtcgaagaacacccgctcgccgagcttggccgcgggatgaatctcgatgccggtgagccagcgggcccagtgcgcgatgaagcgcgccggccacttgaaaccgtgcgtccaacacgcatgcgcccagcggtgcagcaccacggcatggaagccggggtagaccgtgatcacttcccaggcgctgcgggcggccgggtcgcgttcgaggatgcaccggatgtcggcgcgcattcgagaaaacatcgctgcctttgttgtcgttatatcgataggggccgggcagtctaaagcgcagggtcttcgcgtacgggcgatggggttttaggcgcatgcgcggcgtcggccatggccttggcgatgccgcggaggatgtgaatttcctccggcgtgggctgggcgcggttgaaaagctgctgcagccggggcatcagcttcttgggcgcctgcgggtcgagaaagccgatttccaccagcgaccgttcccagtgctcgagcatgccggccaccgccttcgcatcggccgcctgcacgggcgcggtggcgtcgcgcacctcgtagccacccagggccagccgccattcgtaggcaaccacctggatggcggcgccgaggttcagggagccgaacttcggatccgtgggaatgctcagcgccacgttgcagcggtagacgtcttcgttgcgcatgccgaaacgctcggagccgaagaggaaggccacatgctggtcgccctgcttcacgagcggctccaggtgctcgcgcggggtgcgcgtgggcgggccgaagtcgcgcgggatcatggcggtggcgcacaggtgggtcacgccgtcgagcgcctcgtccagcgtttcaacgatgcgggcgttgttcagaacgtccagcgcgccgctcgcacgctgaatggtttcttcccgccgcagcacgttggcccaccgcggcgccaccagcactaggtcgtcgaaacccatggtcttcatggcgcgggcggcggcgcccacattgccggcatggctggtctggatcaggataaaacgggtgcgcatgggggtttggagacacaaagcgggcggagccggtaaaatgcccgattctcgccgcccgcatcgccgggccgctcatcggggcgccagccgctccttccgccgttcttctcacaatccaatgtcgtcccccaacctgcatcccatgctcaatgtggccgtcaaggccgcacgcgccgccggcgcgatcatcaaccgcgccgccctcgacgtcgaggccgtgcgcatctcgcaaaagcaggtcaatgacttcgtcaccgaagtcgatcacgccagcgagcaggtcatcatcgaaacgctgcttggcgcgtatccggggcacggcatcctggccgaagaatcgggcacccagcatggcgccaaggattcggactacgtctggatcatcgatccgctcgacggcaccaccaacttcatccacggctttccggtctactgcgtttccatcgcgctgtcggtgcgcggcaagatcgagcaagcggtcatctacgacccgagccgcaacgacctcttcaccgccaccaagggccgcggcgcctacatgaacgagcgccgcatccgcgtttccaagcgcacccggctcagcgaatgcctggtatcgaccggcttcccgtttcgcagcggcgacaacttcaagcagtacctggccatcatggccgacatgatgccccgcatggcgggcctgcgccgccccggcgcggcagcgctcgacctggcctacgtggcggccggctttaccgatgccttcttcgagaccggcctcaacccctgggacgtggccgcaggctcgctgctggtgaccgaggccggcggcctgatcggcaacttcacgggcgagcccgactttctcgaacagcgcgaatgcctggccggcgcgccgcgcatctatggccagctggtgccgctgctcgccaagtactcgaaatttgccggcatcgacgacaagatgcgcgcgagcgaccgggtgcgcgctgtgtcggccgccgcgcggcctggtgccgatgaatcggtcgacctgtatgcccgcagcaccgtcaccgaactgacggccgcgccgctcgacggcgaagcgcccgcgccggccgccgcagcagcgccggtgtcgcgcaagctcacgcgcattcgccgcgacgcgcctgccgacggcagcccttccgaaggcgacacttccgccaagtgatgcaggggccacgtgccgccctccggctccgtgcggcgctgcgcatcgcgctgagccagtacgtcgccagcgggctcacggtcgcgctcggcctgctcgtcatctcggccggcgcgcacctgtggctcggcgccattgcggcggcgtcggccgcggtgggcgtgatcgtcacggccccgccggacctgcccggcccgcgccgcggcaagttcttccagatgctgccggcgccgctgatcggcctgccgctcttctttttggtgcagctgctgcacgccgcgcccatccgcctcggcctggtgctggtgcccgccaccttcatcgccttcctggccatggcgtggggcaagcggggcatcccgattgccatcgcggtgatgttctcgatgattttctcgatggccacgccggcgcccagcggcatggccgaggcgctcgaacgcacttggcacttcggcctgggcgcagggctttacgtgatctgggccacgctggccaaccacgcgctcaacacgcgctttcgcgtgcagtcggtctcggacgttctttattcgctggccgcgctgatgcgcaccgaggccagccagttcaccccgctcgacgacaccagcgacatccgcgaaacccccgcgccgttgctgggccaactgctgcgcgaacaggccgcgctggccgaccagctgcaggccacgcgcgacatcgtgctggagtcgccgcgcacgccgcgccggcagcggctggcggccatgctggtgatcgtgctcgagatgcgcgaccaactgctcgcgagcgagctcgacctggacgcgctcaagagccatcccgcgcatgccgaggcgctgatcgaaatgcgccgcgtgctcgaagagctggccgacgaaaccaccgcgctaggcgatgcgctgctgatgggccgccagcccgaagcggtggccgaccggcggccgcggctcgcgtcgatccatctttccggcgaggacgatggcgcgggccatggactgcccggcccgaatgccgccatgctcgcgcgcggccttgcgagccgcatcggccacatcaacgacgaggtgctgcgcctgtcggccatggcgcgcggcgacgccgagcccaaccttgccgtggtgcgcgccaactggcagatgttcgtgagccccaccgattggtcgctgcggccttttctcacgctgtggcgctgggacgcaccgccgctgcgccacgccattcgcgcggcgctggccattgcggccggctacgccattgcggtgtcgctgccctggggatcacacgactactggattttgctgaccatcgtagtggtgctgcgcggcagcctctcgcaaacgctcgagcggcgcaacagccgcgtggccggcacgctgctgggcagcgtgctcgcggtggggctgctctccgcgcatccgtcgccgctgatgctgctggccatcatcacggtgtcgcaggccattgcccacagctttgcggtgcggcgctatctgatcacggcggttgcggccaccgtgctgggcctggtgcaggcgcacatgctcaacaccggcgccgcgcccatcttcgcgctgttcgaacgcattgccgacacgctaatcggcgccgcgctggcctggggcttctgctatgtgttgccctcgtgggagcgcgggcagattccggcgctcgtggcgcgcacgctcaccgcgcaggcgcgccatgcacgcctggcgctcggtctcggccagttgaaggccatcgacagcagccccgagctcgaatggcggcttgcgcgccgtgaggcctacgacagcctctcggcgctggtgcaggccacgcagcgctcgctgtccgaaccgcgcgcggtgcagccgccgctcgagccgctcgagcacctgcaggcgcacagctaccagttgctggcgcagctgagcgcggtcaagtcgatgctcgtgctgcggcgcgaccggctcacgccggccgatatcgagggcccgctcgcgcgcacggcacagcgcatcgacgccgccatcggcaccgccccgaccaccggcccctcgcttcccgaaagctccgcctccaccaccgtaggcgggccgattcccctgcccgacccgttcgacaacgacatcagcccctggctgctgcgccgtctcgacctggccacggcgcttgccacgcagctgcgcgacgacgcggcgcgcattcttcaacctctgaacgagacacagaccaccacgaccgccaccgtccaatgactcaagagatccttgcccacccctggttcggcacctggctcgcagcctttgtcggcgttccggtcgccctcttgatccaccgcgtgggcggcctcgtgctgttgcgggtcacgcgcccgacaccggcgcttcacgcgatggtggtcaactgcaaggcggtggcgcggctggtgctgccgctggtcgcgctgctgctggtgtttcaggccgcgcccgacaacctgcgcttcattggcagcgtgcggcatttcaacggcctgctgctgattgccgccaccacatggcttgccgtcaaggccatcagcggattcgcggacggcgtgctggcgcagcacccgcacgacgttgaagacaacctccatgcgcgccgcgtgctcacccagacacgcgtgcttgcgcgcaccgccatgtcgatggtgctggtggccggcggcgcgatgatgctcatgacctttccgggtgcgcgccaggtcggcgccagcctgctggcctcggcgggcgtcatcggcatcgtggcgggcctggcggccaagccggtgttcagcaacctgattgccggcttgcagattgcactggcccagcccatccgcatggacgacgtgctggtggtcgagggcgaatggggccgtgtcgaggagatcaccggcaccttcgtggtcgtgagaatctgggacgaccggcggctgattctgccgctcagctatttcatcgagaagccgttccagaactggacgcgccagtcgtcgcagctgcttggcgcggtcttcatctacgtggactacggcatgccggtggccccgctgcgcgcagaggtcgagcgcatcgtgaagggcgcctccgagtgggacggccgcttcttcaacctgcaggtaaccgacgccaccgagcgcaccatgcagattcgcgtgctttgcaccgcgggcaactcgagcctcgccttcgagctgcgctgcaaagtgcgcgaagggctcatcgacttcatgcagcgggagtattcgcagttcttgccgaagatgcgcattgagggcgacgcgatgcaggccgcacgcgcggaccacccgctgggtcaggaagccgcgcctccacaccaagcgccgcgctaacctgcgctaacctgcgtgaaggctgcggcgcatcgccggaagccggaggttggtgaacgcccgcagcagccactccgccggcccgtaggcaaagcggcgcatccaccacccgctgagcagcaggttgcccgcgaagatcgccagcgcgacgccgaaagtggccagcggccccatggtgccgatccaccgcagcccgtaggcgagaaagagccacgcgcacaccagcgattgcagcaggtagttcgacagcgccatccggcctgccggcgcaagcatccgcgccagcacgcggccgcgcccgctctggaacacgagcagcatgccggccgcgtatgcgcccgccaggaacggtgccgtcagcagcgtgaccgcaaggccctggacctcgcgtaccgcgttcaggcgaagggttggaagcgcataggccagcgcacccggcaggccgatggccagaccccaccacagcacccgccacagcagggcgcgatgcgcttcgacgtgcgcaagaagcccgcgccggccggcaatgaaccccaggaagaacatggccagcgcctccggcgcctgcaccagcgccgtcatccaccaggtcagcgaaaggtcgcgcacatgctgcgccatcaccaaggccggcgtggcgcggtaggcggccagcgccgcggcggcgtcgccgtaggccgcctgcacggccatctgcatatccatttgcgaatacatgcggccgacgccggcccacaacagcgaagtgagcagcaccagcgcgatggccgcgcacgccagaaacacatcgccgcgccgccgcagcatgagcagcacggcgcccagcaccgcataggccatgaggatgtcgccgtaatagagcagcacggcgtgcgccacgcccatgacccacagcccgaggtgccgccgcaccatgcgcggcacgaagggtttgccatcacgctccgccgcccgcatctgcagggtgaagctgtagccgaacaggaacgagaacagcaggtagaacttggtctcgaacgcaaaggcccggacgaacgaggcgatctgatcgggcagcgacatacccagcggatcgggaatgcccagggcgtagtaggtcgaggcgaagctcgcgatgttgaccaccaggatgcccatcagcgcgaagccgcgcagcgcatcgaccatctgctggcgctcgttcgatgcactggccgggtctggtgcggaagggttctggtgcgccatgtggcgttgcgggttagtttggaggatggtggattagatcaatcgaatgtagcgtctctacagtcgttcgagatcgaacgccaacccgagaagacccgggaacgccccccaacggccgaatgattcaatgattgactgactgaacgaggaggatccccatcatgctgaagaacacccccatcacccgccgcctggccacgctgcttgccgcggccggcttcatggcgtccattgccaccatggccaccacggcgggggcgcagacgacgctcgacagccccctgcacatcgtggttggctatgcgcccggcggcgccaccgaccgcgtggcgcgcatcgttggcgacaagctcagcgcacgcctgggcgtgccggtggtcgtcgacaacaagcccggcgcgggtggccgcctggcggcgcagcaggtcaagaccgcgaccgccagccagaacgtgctgatgctcgccaaccccgccgtgatggtggtggcgccgcttgtcttcaaggacaacaactacgaccccgagcgcgacttcgtgcccgtgtcgcacgtcaatgcctacgactttgcgctgtccgtgtcgccccacctgccggtgcgcgagctgaaccacctgctcgcctggatgcgcgccaaccccttgcaggccaacgtgggcgtgcccgccaccggcagcctgccgcacttcttcggcctcatggtgggcgagaaggccaaagtggagacgcagatcatcggctaccgcggctcggccccgctgctgaacgacctgctcggcggccaggtgccgatttccatcgacaccgaagacgtggtgctgccgcagcacaacgcgggcaagctgcgcatccttgcgatctccggcgccaagcgctcgccctttgcgccgaacattccgaccttcaaggaagccggcctcgacctggccgccaccggctggaacaccttcttcgcgcccgccagcatgcccaaggagaaggccgaacgcctgtccaacctgatccgcgaagtcatgcaagacgccgacacgcagcgcaagttcaaggacgccggcatgacgccggtggtgagcacgcaggcgcagaccgccgcaatgctcaaggcctaccgcgcgcagtgggcccccgttgtccagaagtccggctaccagccctgaaccgtttcagacacatgaccagacccaacatcatcttcattgtggccgacgacctcggctatgccgacctgggctgctacggcggccgcgatgccgccttcggacccgtgtcgcccgtgctcgacggcctggccgccaacggtttgaagctcacgcagggctattcgaattcgcccgtgtgctcgcccacgcgctttgcgatgattaccgcgcgctaccagtaccgcctgcgcggcgcggccgaagagcccatcaggagcagcagccgcggcagcaccacgctcggcctgccgaccgaccaccccaccctgccatcattgctgaaggccagcggctaccagaccgcgctcatcggcaaatggcacctgggctacccgcccagcttcggcccgctgcgctccgggtacgacgaattcttcgggcccatgtcgggcggagtcgactacttcacccactgcgactccaccggcggccacgacctgtggcttggcgaagaggacaagaaggaagagggctacctcaccgacatcctctccaaacgcgccgtggactacgtggagcgcatggccaagcaagaagcccccttcttcctcagcctgcactacaccgccccccactggccctgggaaacccgcgacgacgccgagaaggcgccgaccgtgaaggacaacctcttcgacctggccggcggcaacattcatgtgtaccgccgcatgatccatcacatggacgaaggcatcggctggatcatggccgcgctgcaaaagcacggcatggccgacaacacgctggtggtgtttaccagcgacaacggcggcgaacgcttctccgacaactggccgctggtcggcggcaagatggatttgaccgaaggcggcatccgcgtgccatggatcgcgcactggcccgcggtaattgccaagggcggcgagagcaagcaactttgcatgaccatggactggtccgccaccatgctcgacgcggccggcgtgaaggccgatgcagcctacccgctggacggcgtgtcgctcatgcccgtgctgaaagacgcgaagcacagcttccgccgcccgctgcactggcgcatgaaccatcgcgggcaggaagccatgcgcgatggcgactggaagtacctgaaggtggacgggtacgagtacctcttcaacattccggcagatgagcgcgagcgggcgaatctcgcgaagaaagagccggagcggttggcggttatgcgggctgactggctggcttggaatgcgacgatgcctgggattccggaggatgcgacggttagtttggggtattcggttagggatatgccgcagcggtaggggtgcagcggcgcggggaatacatgccgtgcatgttgcttccgaagacgactgattggaggtttctcaagggctgcttaagactgtacccaggacccctgtcgcaatcaccggccattcgcggtcaagggtatcgaccggcggctgcgagactgctcgctttcgcttgcctgaagtcgttacaaggctatctcaagcggcgtccgactctcttcgtgagtgcgggacgccttcgctgcttcaggcgactgccacttcgcctgcctgagacaggatcgcctcgcagtcggccacaaggctctccagcgcacggcgtccccaccgcgtttgcccaccttcgccggtgccctcttcaagggttgcaagcgtggcatggcaaaccagcggacccaccgggatgccgacttctcgggcgatgcaggcctgcagtcgagcaaggcccttgaagttccccagcgccttctggatgaagaattgatagcgatagacagcagtcaggtaaagctcgtgcttaggccccagcttcaggctgacgtgacttaggcactggccaccacgcccgttgtcgtagtcgttctcagcgtcatagaatttcagttctagcggctccagggtcatgtccaattcatagaccgcccgtggaggtccgttcttgacacgcttggccgcagccatggccgccttcaacttgtcgatcacgatctcgagcgggttgatagtcctgccgtccgaacaagtgcgctgcgtcaacctcagagcgtaggttccccagcggtttgcggggatgcccttgatgtgcgggtaaacgtcagtcgggtatgcaaagacctttttcagccccccggacttgtactcagccgccgggaaaatcgtgtctgaaactgtttgcacgggcaggcagttgtgctcagccaagaacgcatccacacgccgctcgatggccttcgtcgcttccgtttcaagtccgggctcctggatctcgacgatgaggttgtagatgcgctcgtgctccttgtaaagcagacgagcggacttcaaccaagcttcggcacgggacgttgcgggcacgggtttcatatgttcctttgactacgcggcaagcgctagcggcaccagagttcttgagccaatgagattcccggtcaagtagctcaagggcagccaggcgtacccgccgaagccccacctgaacccccagctgtttcgcaaaagcagcaggtcgatggcgcccgcggcaattgaggctccgagcccaacgcccagaacgctgtgtccgccgacgggagtgccggacgtgtcgatgatgtacgggctctgctgcacacggttaaagccgggcaccagccgcaaaccaagcacaaccggcagcccggcttggagcgcgtcgacaacttcgtatgccgcgcacggatccaagccaccgtaccaaagcgtcgtcaatgatggcggcgcccaagggcttggcgtcttggtctggtacggccactcgagctcgtttggctgaccatcgctgcgcagtgcctgatccgccgcgccaagtgtcaaacccttggccgggttcagcgacggcactctcttcaggccagcatagaagaggtactcggcggacagcggttggccgagaccatgcgcatgggcgtgggcgtccgaaaccgcgcaagcgatgcacgtcgggcgcgcgccttggtcccggacttccgtccatgcatggcgtgcgtctgcttcaacgacgatgcctccaacgtcgctcatgtcgcgttcagtctttccgcgcgcagcaggccaaccggctctttccccagaagcgccaggttgaattccatcgagttgatagcactgtctccactttcccacggccggcgctcagccagacgcaatttcgtgcgcgccggtgcgctaccttggacgacgacgcgcctggtcacggtgctccccatggcgtcgtcggccgagtcggctcgcctgtccttcctgacttccaggccgttggatggatccggttcaatctcccactcgtagccgcccgccaagtgctcctcgaggttcagcacgaggaagtcatccgggctcccgacaagctgcgcacccttgtctcggtcggaaagcagccacacgtcgggatgccaagacgccggctcaacgtcggacatcgcgcgctgcttcgcctcttttgggggacgggcggcaagcgctcgagcttcgttgtgggtgaggaaatctgcggaagccagggcccagcaggtggctgaatagctggcggccagccgcagggacaactggtagatgaccccggagtacctgaacgactcaagaccccagccttgccgccgggcgtgtgctgcgatcagccacttcgggagcatgaactcggcggcaaacgagtccgcctcaagctcctgctggccatagcccgtcttctcaccgcggccaacgtatccgacgttgatgtccagactcatggtccgatgctgaaggacgtggtggccaagctcatgcgcagccgtgaaccgctggacgtgatggtcacgccgcgtggtcacgagcattccggcggagttcggcgtcggcacgtacgccccgagcagcccatccagcggacggaacagcaccatgatcttgagcgcctcgatggccgcgaagacgtccatgggacggctaccatctctcaactgctctcgaatgcccatcgcgtgatgcagctccgccgcacgcgctattccactgaggatggcgtcgcgcttagccattgctgccgtccccaggctgcgaacgctgcatgaggaactcggtgaatctcagtagctcagagcggtccttctcagacaacgtcgatgcttgacgcgccaacatgttgacgtcggccggataagcaagctggtcctcgcccgtgaagtaggcagtgggtcgctgatagagacgagcaagggccgtcaactcttgggcgacgacactgcgcttcccgctttctataagtgagacggcagaacgaggaatgcctgtggcgtcagtgacctcttgctgcgacaggccgaggtattcgcgagcttctctgagccttgaggcaatagcggcttggtcgtcggacattttcaggtctcctgctctagtggaccgcgtctgccacttccgttgcaggcgcagaaaccggcgcggccggcacagccacgcggtgctgtttgatttggctaatgatgtgcgcgacagcttcttcaaccgtgtgatagccgccgcgctggatccaacgcgggtcgagggactcgccggtcaactccttgacggccggcgacaacttcgcgacggtcttcgagtccacctctggcgtgtcccacaacggatccttcttgaggtcaggcagtgcgcagtcctcctgctctcgctggagatcctttgtcagccggtccatcagtttaggcagcaggcccgagaactcggacgggctcaacatctttggcttgctcatgcgcactcctgttcggaattcaaacgaagcgtatcacatgttgttcgattttccaacattaacgacaaatcgcctgtcgccggcgtatgggcgaatcagggcggcgattgcgccgcgatgatggcgaaagcgagcggcgaggcgcccagggccaggcgacgcaccacgacgcgctttaagaccgcagcagtgagcgcggctacgcgccagcccgcgacggacatgacgccggcatcgctctggccggccagcagacgtgcctgcagatgccccagttttgagttcaatgtcagtggatactgacatttgaagatggcctccttcgccgaaaaggcgaagttttgggctgccgcgtggtcggcgagacccatggcgcgctggacgcgcgagacctcagacatccaggtcacacccgccgcagccgcgtcgccaagtggccgtgcgtcgtcaagatcgacgcctaaggagcagtaatcaacggcgaggccgaccagcgcgacggcgtgctcgcgcgtgtgactgatgcttccgcgcagctccgctggaaagagtggctccccttcagctccctgcccgatgccaacggccggtacacccaagacggccatcgcctggcgggctgcgtcacgacccgccgcgaactgcgcgcgacgccgcgcggtcgcgccaacgacgaggagttcctcgtccggccagagcatcgcaggggtcggagaaatcggcacaacacgagcgaccaagcgctcggcgacccaatgcagtccgataggtggcaagtccgacttcctcgtggttagctgagtacattcaatcatgcgcttcaccttacccgccgagccggaggcacttgctcgctatctgcctgagttcatggccctggtcggaacggagaggtggctcaagcgagccaaccagctcgccgacgagatggatcgctccgcctacctccacaagatcgtgctcgactatcactggctcgagatgaacgtctgccatcagtgggaggtgctcacccgggaaaaccgcgtggacctgactgtgcgcccgcacctaagcctggctgcgctgaacttcgcagcaacggccgtcgtggttcatcggcagttagggcccaagggcaagcgcgtgctcgaaggtcgcctcttcgatgccctcaaggccgagaccggcttcgccgcactctatctcgagctctcgctcgtgcaacggcttttgacatgggacttcgatatccagctgccggacatggagggtactggtcagttcgacttactgataactcgtgacggcttctccgctgaagtcgagtgcaagagtcagtcggctgatgcgggccgacagattcaccgcaagcacttctatcgcttcatggcgttgctccagccggggaccaatccggggctgcccaagcgtcgggaggtggtcctggtgacgctgtccggtcgcttgagcgccgacctcgcccaacagtcgctgcttgcgaatgccgtcagcgccttgatcgactctgacgcgacatctgcgatgaagggcagcggatttgagctgcgcaaagctcgcttcgaagatgtccccggcgtcgaagagaacctccgagaccccaagctgcttcaagcggctctgaacaaggcgttcggcaaagaccttcatgccgccggctggcagggatcggacagcgcgtacctacttgtgatgagaagtacgaaggaagacgatccttccttccccacgctcgaagcgatgcgcaaaggcgccagtcagcttagcaagacaaggcctggcttactggctttgcaggaccacggcatggagccggccgacctattcctgccacatgtacagcgacgagccttcatcctgtcgggcgcgctattcggtcaatacaaggcgcggcacgtcaatgcggtctacatcaccggctatggcgctgtcgtcgacgaccagcacacgctccgcacgccaggtttcgccgtcaccaacatgcttgccaagcaccccattcccgatgagcacacaagggcgctgctgacagggctcctgcaggagaggccaccggccgacttgccgcccacatgacggagtgtaccgaccaggttcctgcgactgaggaaactccgggcggaactgcgggccgcccccgaaggcgttaccaacctgctaactcggcgccgtcgagaccaactgtggccgactcaccgcccacgcgacgcgacgcgtgttggccaggcggctcaacacgccctcgacgttggagaagtccttggtagcgcgagcaaaggtccctgcgccttgctttctgccgagggacatcaacgcctcgtcaaccgttgcgtcgacatggacgggtacatgcgccaagacatccaacgagcccatgcgaaccttgacgggcaaacaaccctgctctcgccattgttcgatggcgttggcaacctctttgagggacggatcgagcacgacagcaatcgaacctcgccggtgggccaggacgaccgcggtaatagcgacatccctcacccaagcgaccgtgactatcgctcgcgcctcattcgcaggctcgcagcccctccagccgtccttcaccgagggaggcaggtccaatgcatatcccggctcttgcgcacaagaactcgagcgcgcgatggcgaccggcagcgaccgtcgatgcttcgagtcgtgggtgtctgggtgagcgttcatggaggcccttcgcagtccgaagtcgctgttagatcggtatggcgctcaaggcttaaacgcgcaccggcgctgtgcgacgccatccattggaccgtgcgggctgccgcctgacgttgatttaaagcaaagaaggggacgccaggggcacgttcggcagcgcatgagacaatgaaacgctggcgcggggagcgtctcaaacgccccccagacgacctcactaagctacttgagaaatgtaacggtgaccggcaagaatcttgggcccaagcgctcttccccagctaagaacgggctgaccacgtttgcacggcgcaccgcgccaacctccaccgtcgtctatgactcctactggcgcttcgctaccgaacgccagcagctgtacttcaaccggctcacggctgaacacggaccgtggacacaggacccagtgctctccaagtacaagttcaccaacgcgtatcgcgcagccgaccgtgtgagccagtacctcatccgggtcgttatctatcagggagctttcgacgagctagacgtggcatttcgcatcctgctcttcaagcttttcaacaagatcgagacctgggagctactgacagctcgcttcggcactctgtcgagggctaccttcgacgttgagcgatttgacgctgcgcttagcgaagcgctacgggcgggcattcggatctattccgcagcctacatcatgcccaacgctcctcgcctgctagagggctcatataagcaccgcacccatctggacttgctccattccgtggtgaagagcggcctactgcaacagctggttgaggccggctccatgcagcaggtctatgagctgcttctctctctgccaagcattggaccgtttttggcttaccagtacgcggttgacctcaactacagcgccatttctgaattcagtgagaacgagttcgtacagccaggaccaggtgccttgaacggcttgacgaaatgcttctcatcgcttggcgactactcccctgccgatgcaatccggtgggtcaccgaacgacaagacgcagagctcaaggccagaggtcttgcgttcaggtcgctgtggggacgaccactacagctcatcgactgtcagaacctcttctgtgaggttgacaagtatgcacgtgtaatgcatccagaattcagcgccctcaccgggcgtgcacgcatcaagcagaagttctcgagcaacggtgacctgcctgcgccgttcttcccaccgaagtggaacctaatactggatctgccgaaagacacaaccgtctggccattcccaaaggtgagcaagcggaaggctcagaacgagctctttgcctgaggatgcggtctcgctaggcaagccgcagtggcggcaggatggtcaccttggttcgaataccaacgtgtgctggtcaaggtcgaccgtcacccttccgccgcggtgttccttcagcaagcggaagacgcgatatccctccaggattgcgatctcccactgccacataggccgggcttcaacctcgtagccctgaacaaactctcgaacggacttcagcagctcaaagtccagcgaggtagtcgagcgatagaacatcgcatgggcggcgtggttgaaaatccaggaagagatgccctcctcgataaggatggcgcgggccccatcttcgttctggtccacctgggggttggacttccgcttgcgcctgagcatgcccctcagcgttggcgaccagcccaacaccgcagcatgcgcaagatggaacacgtcgtgaaagcgatagtcgtcctgaaggctgcggttgtcggtcagccggtcgccaacgttgacaccgtccaattcaaccacgacgaaggtattcccgttctctgtccgctcgaagaagtcgaagaccatgtgacgcgggaactgctcttgcaccggaaacacttcgtcgaacgaaccaccccaggacttctggcgaggccagcgcccttcggacttggcgacgttgcgccgggcagcgatgtcaagactgatgtctgcatcgtctgctgcgcgaaccagagaccggaagacctcgaccaggtcggcggcgaggcggtcacggttgttgtcgatgcgtccgctagcgtagctgtcgaggagtccgccggtcttggcggccagctcaatgagacggtgctcaaaagccgtgccggacgaagctgcgaggttgctggtgttctggaggtgggcgaatgtgtggacgacaggccggccatggtagctccagtcagcgtgactggccaccactcgccctgcaagatccgacagcttgagcccgacccgacccgccgcgttggccaaataccaaagagcgtcgccgaactcttctacgacggccgcgtcataggcgaggaaggcatccttgtcgcgctttttcttcttgagcgcgctcagaagactgccaacctcaccgaacagccctagaagcacaaacccaagcccgtcggcccctgcaaggccagacctgtctgacattgctgtaaagtcctggtactcgtcgagctggagcgcgtcgcggacgtcgtcaaacagctgcgcttggttgagtggcaagtaggtgtctccaccatcgcccgattaggagcataggtcgtggacccgcgagtacgggcgttccggtaaattctagagcaacaacgccggaggaggcgccatgacgcgagcagcgcgttttctgcacatcaccgacacgcacctgaaacctggcggctccgcgttcgagatcgacgacagaaagcgggacattcagctcgagccccagacgcgcgaaggctcgcttgagggtgggctcgagcgattagcggagaggctcactcaagacaaccagcgtctggatggcgtcatcttcagcggcgacgcgttgagtggtggcaaagccggcggcgacaagctgctcctcgatttgatcctccgccatcttggcccccacggcatcacggcgcagtgcatcgtcgcggtgccaggcaaccacgatgtccctcaaggtgctgagcccggctcagacgcgcgctacaaggaattcctcgaggcttggcgcgctgcaggctgcataacgccgtggctagatggtatcgacctgccgaagccagattttgcgaaccacatcctgctcggacctgacaacgcctgggccattatcgccgtcaactccagcaactggtctcatgtcaacgccattccgcccaagctggcaagcatgtgggacaggattccggccacactggcaccgggcgactcggacctagaggcagcgctccgcaaggagctgaacatgctggcaaggtacgacgtggcgcgggtgtcaccgaatcaacttgacgctctccgatggatgctcaaaagtcttcctcgggctgaccacggaaagcagctcaggatgatggtgctgcaccatcacttgcgtgcgccatccgttgctgaggaggtgaagccattcgccgacatcagcaacctcgagcagattcgcacgttcattgccgagcagaacattcgagtcgtgcttcacggtcacaagcacgtggggcgggtccactccgatgtagttgaaccaggtctcggccgtcccccgcacaaggtgcttatggttgctggagcatcgttcagcgcgtccgaccatgccgacgcgatgcggattctcgacctcaccggcttgccctgggtaccgtcgctgggcgttgagccgctcgctatcccgcgcggtggtctagatccggcgccggcgccagcgtcgagttcgcgactgtgggccgccaccgatagtgccgctgaagcgccagtcgtcattcagggtagcaacttcgacgaggtttacgctcgagtcattctggcggcacgcgaggaagccaaggacaagacgctcatcgttcagcttgacctttcggacttcacagcagtaaagcgccttcccgacgactacccgagcaacatcactgcgggggccgaaagggccgcatggttaaaggacctggtggactggtggcaactgccccaatcgcagctgcaggaacgcgtgccttacattcacggcacgcgactgcgcaactacgggagcaacctcgaccagatagatcgggttcgcaccctgctgaaggaccggcagacgacacgcgcaatagcattgctggtggacccatcggtcgacttcaaggaggcgtcgggcgccaagaacgacttcgcgtcgttttgtctggtgcagttcacgaggcgcgatgagccaggggccgtctttatcgactgtgtcggttactaccgcgcgcaggagatggtcaagtggtggccgattaacgtggctgaacttttggatctgcagacccaggtaggcaagcccttcaatggacggccgggacgcataacgactatcactgcttgtgcccggtccttggcccgctctccaacacatgttgcgatgccggtcatagaccggtggctcgaccaaacccctgagaagtactttgtgcttgcgtccattttgctgagcgacgcccctatgccggccaacgcccgaaaggtgctccgtgaatgggtcgcagcactcgacgagctcaatgaggctgccaccatccccacgccagatggcggccctgtagtagcaattgaaggtccaattcggctggcgaagtacctacgcatcggtaacggaccgcgcgccgacgaatgcgcccgtcttgccgagaaccttgaggaaattgctcgcattggcaagagccccccaccatcgagcgaagttctgcagcgccacacttggggtgttcagctctcccggttgctggggcgagccgcggagcagtgcagagccctcgagatcaagtcgtgacttcgagcgccaagctcgcatcaccagccaaaaagccctacgtaagctacagaagccgaagacgaactccttcttcaccctcacccgccaaaaccgtgaactttttgccgggcagcgccgcctgctcttgccatcgcccggacgctttgccggcgtagttgaaaagcagccgggcgtccggcctgctctcaacaacgcgcgcgattgcgacgtcatccggatggccgtgatgatcgccgttggtcgaaaccacatagttcaatgcggagtaggcccttagcaaggactcagtcacgttcttggcactgccgtggtgcggcagcttaaaaacgtgaagatccttacggacctcctccgccacgtgcagcgacgccgcaacaaggtcctttggattggcgtcggcgcccagcaggagacgcttcccgccaaactcgaaaaggaatgcaatcgagctcgcatttgttgctgacccgtccaattgggtcttggtcgccgccaagttcgaaatgttcatcgcttcgccacccatacgctcgagcccaggtggcgcaggctcggccttggatggttgttccttcttggcttcctctacggttcgcaagtacctatcccaaaggtgccggactgccgtcaaacgtgggagggtcggggatagaagggtaatcttggctcctgaatctaaggtcttcttcactggaacgtcagcatctaggcaaaccgcattcttgccgaaagcacggttccacgagatgccgtctgcacagagcgcctcttgcagttcgatcccttgagcaacaccgagtgactccgtgccgggcggatcaagatggtgtctgccgttgaaccaaatgtcttgaaatcgaccagcaacagacttgtcggccagcaaggtgaggactccgccgatgtggtcggcgtcgatgtggctgacaaccagcaactcccagatggcgttcggatcctcgtttaggacctttttcagtcgctccgctgttccctcaacacctgcgtccacaacaattcgatagtcgtgtccttcatcgccgtagctcagaacgatgcagtcaccgtgttgagcggcgagcgcatggaagttgagccgatgctttcccggcaaggcggcatcatcgtgcgacatcgaatacgcagaagggttggtcagggtcaacgcgcagcaacagctccctgacgtagcgttgcgccgactggagctctcgccgaatgcgggtgatccgtgccgattcggcttccgcagtgagtatttcgaggttcgttgccaacaacttcaatccgtagcgaaacagtggcggccctcgtcggaccgcctcaagggtcgcgtcgagcgacgagcggaaaggctcgtagcctggacccatgaactgcaacccttcgctgacacggggcggcccctgcagcaaaagggtggagtagagaatggccccatcgggaaggcccgtatagcggcttgcaaggttgagcacccactgtcgccagttcatccagccctctccctgtggcaatcccgcattcaagagcacatagccagcgactgcggcagcatacgggttcctccacttcgcatacagaatctccagcgatcggttcacgacgctcacagagcccgccaggtcgccctgttgcaggaagtcgatgagcccaccaaagtcggggtcgtcgacctcaagccgtagagcgcggtacctgcgttgaccgacctctctgacgtgataactggcgctcactggggccaacgttccgtcctgagtcatccagcggccgggcatgcacgccacttgaagcggatagaagtcgtcggtcgcgcgataagacaaagcgaagtagcgagctcctttcccttcatcggagacgcgcccgatgatcgactggttgcgcaacggatacttccagtgcgcgtgcaactcctttgggttgccatacagccgagtagcttggacggcatcaatgtcccctaccaaatacgacgaaaggtcctcctgctgctggaaagcggtgctgcgagtccgtgtcttgagccttgcgacacccatgaaatcctggcgcttgttcacaacctcgcggactggcaagcctggcaggtagttcaaagccgcgggcacaagacccggctcaattagtctggcagtccagcgctccctgtccgcagagcccgacgacaggtcgcccgaagagggaagcctgtcgcctaactggccttcaacgacgagacgctcccccccgtcttcatagctgtccacgccgcgggctgccgtcctctcgggaacgaattcaagcgcagtgtcgtggccctcgtctcggacgcgcacccgtttttgcagcacctgtccggtagggacgcgcaggcggacgagatactgaccaggcgggaccctctccttgaccggccctcgcctgaggttgactgcgatacctgtcttgacctgccgctcttcggctcccccatcgctcaactcgacgatatccgccacggccacgcgcgggcgcgctgcgttgagaggaagaactcggctgaaatcgacgtctacggtggtgctcatggcttgtctccacaagatataaacaccgtctcgtagggtggagaaacatgttctgccagcgcctggccatgcaccgttggcgcgccggagaccgactcgatcgcctcaaaatcgtgaggtccccgtatcaggtccacattccaaggcgattggcctgcgccaaaatgttcagtctggtcgacgtgcaaacaggaaaacgcttcgaagtcctccggttgacacaacaccttcacaggcacgagcggcgcaccgggcaactcatggaagtccacggcagacgaaaaaccggcgccatacatgacttcctgcccttggccgtcgggacgtcgctggatgagccagtcgagcgcagtttttagccggtccgtcttcacaacccattgggtcgccccttgcttcgctgcagctgcgcccttcatggcttccaagaatgcggtcatgaagagtgacggcgcattgacaacgccgtaagccttggtgccaaactcgctggcccgaacgtagacgggcctcacgatgccaaggttattgtttgtcgctggagtgatgacggagcgaggttgcaccttctcgtagtcctccggcagtgggacgcgggtactgcaagcatcaatcaaatagatctgccgtctggccttggctttgaccatcgcgccagcaaagcgctcgggctcgaaggcatggtcgaacggcacgtcactgttcgaaccaaagtcttgcgctagaagggcgtgcacatcgcctacgcgcaggccatgcccgcagaagtaaaacagagctaagttctcttcgtgcgaattgacgtccttgaaccaagctctgatgtacttctggatgttgtcgaaagtcggctcgctgttcagccagggcgtttgcttgtccggagacgatgcaagtagacgtagggaacgcagtggtgcgccacttacacgcaaatccgcttcaatccagtccgcaaacgcctcgaccgagtgcaacggcgatgtgagctccttcagtccagcgtctggggcgaactccccgagttcgtgacctggttgcaagtgcgggtaccgccccaccccgataagcaatgcgtgaactccaggctcacctggaacacgcttgtcgaccagcaatgccatagctctccctacgctttacttggcgcggtctcgtgcgcttccgggacgctctgccgctctgatggccgattatgggggacttgtgctctggatgccggcggcgaaccctgcgtcgccaagatcgagagcttcgggcacaaagcagcgtgctgccctttagcggataaattttgggagcaatatggcatgtcgtctctgaaaaagccatgcccacttccatccttcaatctctcgcgctgaagcacatttcatcatctgtaagggtctacagatggcaatgcgatatggttctcctgggtccttggcccaagccttcaccgttagctttttcttttcccaaaaatcggccgtcggaccggtgagtgcctcgatgcacggatgactgctgttgggctgtcacgacaagacgacgactggcagcaaccgctgcctagtggaacctcgaagtcgtcgcctcgacttaagcaccatgaatgcattgcgcaattcagctggtggaagtcgacggcagacgcggccagttgagggcgcgcgcagccgacgcgcgggtggcgccgattcgaagggccagggacctgcgttaacgacactgcccctaagtgcaacgcttcagtcctcccgaacaagcacatccccctcaaaccgataccgaaaataaaaccacttctcagtctccgacttcgcctcgatgcgaaacgccgtgatcaacctttccccatccgtcttcagatagatcgcgccgtacacctcgacattgctgcgcgcgagctctttcacgtcggccttgagctgagcgaccttgtcgggcgagagcgtgcccgcggccagcttgtcgatggcggccagcagcttgtcgaccgcgttcttgtcttccattgcccgcgaggagcgctggagctccgttgaaagaatcaccggtgcgccgccacggccaaagcgtcccaggcggcccagcaggtcgggcctcgggtggatgtggccctcttcgtctcccgacgagatgatgaaggcggccgggttgacggcatccagaaacgcatcggtgactttctcggagccgtggtggcacgacttcatgacgtctgacctgaaggtgtcgcgcgccttggtcaccatgtcgtcgtaggccggggtgccggtcttcggaaacttgctcgcgccggtgtagtgctgcagcagaaatttttcggcgccctcgttcaggtcgccgccgaacagcacgctgaactttccatactggagccgcaggatgacggaatgcccgttcttggtttcgctgtaggagcccagctgccgcaacgccggggtgccatcggggccttcttcgacgactggggccagcacccgcatcgtgtagccgcggtcgtccgacggggcgaagtcgggcatccaggcggcgccgtcttcgatcgtcgcgtgctgtgccgagagcatgcggatgtcctggatcttcgggttgtcgagtgcggctttcatgacttgtggaaagagatggctggtgccggagttctcgaagatcgtcttgacggttgcgtagtcggtggccaggtcgcctatgtaggcaatggaggcgccgtcttccttcacgggcttgccgcccagcttctcccaggttcctgcaacgggccgctcgaccagcccgttgtgatagaccgcgccaaagccgatgccggggtcggcaaagacgtccttgaagccgaggtagtgatcgctgtccggatgcgtcatgacggcggccgcaaagttgaagccgcgataggtctggaaccttccggcgagaaaggcgcgcatgttgccgccctcgccggcgtcgatgaccacgatacgctcttcgtcgtcggtctcgggcgagatcagcacggcgccatcgccctgccctacgtcgacaaagatgatttcaagcggccggcgggcgaccgtgtcttccttgcggatgtagagcgtgcgccgcttggtgggcgagcgggcggcccagtcgatctcgagccatccgtcgccgagatctttcttgaccttgaggtagtcgccccagatcacctcgcgaaattttttcttcttgtcatcgaagagatggatcggacttccgtccgcgcgcaagttgacgaatcgatgtgccatgccccgcccctcgtttgacgaatcccgtgctttttagcagtgcctgatgcaaaagcgcatccgacgaaagcggtatggcgcaaacagtcgcggcaagggtagtcacatgtccatcgttctcggtgcggggggacgaggcgtaccaaccaacggcctcgctcgcccctcctccgccaagcttcatccgttcacgccaagctggaacctgcgcgcgaagcttccagcccagacgcgccggccttcaccgagggccctgccgcagcacccgcctccagcgaacaccatgcggctgacggtttgcctgcttcgagtgagcaccatgcggccgaaggtttgcctgcctccagcgaacaccatgcggccgaaggtttgcccgcttcgagcgagcaccatgccgctgaaggtttgcctgcctccagcgagcaccatgccgctgaaggtttgtccgcttcgagcgaacaccacgctgccgaaggtttgcctgcctccaccgagcaccacgcggctgtgggcttgcccgcctccagcgagcaccatgcggccccatccttgcgcggctcgtgtcgggccgcgggcgtcggctcgccgaattcttcggcggtcaagcgctgcatctccaggaaggcatcttgcagggccttggcgtcgtcctcgccacgcaggccaaggtacggaaagtggtgcagaaaatagccgaaagtggtttcgcaatcagcggcgtactttctcgtgtcgaggatgtgcatgtgccagaagcggtcgacgtcctgctcgggagcgagcgtcaggtcggggtgcttggcgtgcaggatcaggtagcgcttgtaggccacctccatctggtccgcgtagccggcagaccagccgtagccgtcttctttgcggcaggccttgaacttgatcggcgtgaggtcgagcccctcgattgcagcgatcgtttgcgccagtgtcttgcattggggggaatgaatcatgaatgctcctgtgaagttgccggaaggtccgagcgaacgtgcccggtgacgattgcttcgaggtttggccgtcgggtcagaccaccaccgatgaagcaaactgggtgcgcagatgacgcgccatgaaattgcgtgtgtcgtcggcagacacgggcttgcagagccaatatccttgggcctcgtcgcatccgcggctgcgcagatagtcgagctgggccgtggtctcgatgccctcggccaccaccttcatccgcaacccatgggccagcgtgatgatgccgtcgatgagcgctcgcgcgtcggcgtcttgcgaaaggtcgttgatgaaggagcggtcgatcttgaccgtcgacagcggaaagtgcttcaggtaagagagcgaggaataaccggttccaaaatcgtcgatggcaaggccgacgcccatgtctcgaatcatccgcagcaacttcgccgcacgctcggggtttgccatcaccgcgccttcggtaatttccagttccagcagcgacggctccaggcccgaggcttccagcacggactgtatgtcggcgatgagcgtgcggctttcgaattggcgcggcgacagattgacgctcatcaacacctcgggcaaaccgtctttctgccacgaccgcgaatcggcgcaggccctctccagcgcccacttgcccaaaggcacgatcaagccgatctcttcggcaatcggaatgaacttgaccggcggaatcatgcccaggaccggatggtgccagcgcatcagcgcctcgacgccgacgatgcgctgggtctgcaggttcatcttcggctggtagtgcatttccagctcgccgcgttccagggcatggcgcagcgcgctttccagcatcagctgttcggtgctctgcgcattcatcttggccgcgtagaaccggtaggtgttgcggcctctttccttggcccggtacatcgcggtgtcggcgttcttcaagagcgcttcggcgtcgccgccgttgtcggggtagacgctcacgccaacgctggcggtaacgtgcagctcgcgccccgtgatgacgaaaggctcggcgcaacaggccagcactttttcggcgagcatcgcggcctcgttcgcactggagaggttctccaggagcagcacgaactcgtcgccgccgaaacgcgccacgacatcggcctcgcgcagcagccccgtgaggcgctcgccgcagatcttgatcatctcgtcgcccacgccgtggcccagcgtgtcgttgatgtgcttgaagcgatccaggtcgacaaatatcaccgcaaactgcttctggtggcggttgctgcgcttgatggcgcgagcaagctcgtgttgcagcgcggcgcggttgaacaacccggtcagttcgtcatggctcgccatgaaacgaagacttctctccgccagcttgcgttgcttgtactgggcgatctgcaaggcaatcacgcgcagcgactccagcgtctcggcgtcgacagcgtagggattggagccaaagaactccagcgcggtggtcgaaccggtaatgatcatcggcacgatgacgccgacagtcagcccggcccggctggccagcacatcgcgcgcaaagtggcccggagccgccagggtgtcgatctgcacgatgccgccggctccccaggcgcggcccagcgagccttcgtcgggccggtattcgaacgagcggctgtcgctgacgaattgccgcacggccggggagatgtcttcggcatgccaggtggcggcgcagcgaaccacgccgtcatcgccaacgccccacactgcgccgcagtcccagcgcaggtcggtgcatacggcttccagcgcttgcgtgatcaccgtctcggccccgccatcgccggcaagcagccgggcgatcttgtactcgagctcctggcgcaatgcgtccttgcgcagccgcgtggcgtcgcgcacggtgccgcgcaccatcgtctttccgccttcttcggccgactgcgcgatgacatggagccagcgttcggtgccatcgggcaggcacaggcggtgctcgaattcgctgcgctccatggactgcgaggccagtgcgatctgctcttcgaccgcagcgcgttctgaggttggaacccgcgagagcagcgtgggcaggtccggctgcgaagggccgggttcaaagcccaggatgcgccgagcttcatcggagcattgcagggctccggtttggggatcgaggatccagctgcccaggcttgccaggtgctgggcctcttccaactgccgctcgctggtgcgcagatgaacggtcatcttgttggccagaacctgggctcggctgcgtgaggtggtcaacgaaaaaacgatgccggcaagcagcatgctggtggccagcccgccgaagacaatgaaccacggaatggccttgtcgagcgggccgaagacctggttttcgtcttgaccgacttccacgagccaggagtgaccgcccaactcgaagccgagcatgcgctccaggctgcgcgccggttcggcaataggcttggccgaggctgcgctgtcgaacatcaattgccgctcgccgaacgaagtggtcgctacaaaccgggtctcgacgcgtgtcccgatcgccccctggcctcgaccggcatcgatcaaccgcaagcggaacgtcctggcggcgctggcacccaccacgtcgctcaacattcccgcgacgctgaagcccgcgccaaccgaaccgatataggcactgcgccgctgctcgagagtatcgagcgattgtcttgggcgatagaccggcagccgcattgccaatccgatgtcggactcgcggcccgcgatgcggaccttgcggccggacatgacgagcccgccggtgtcgcgcccctgctcgagcgcgtctcccctgtcgggcatcgcgcccaggtcattgccgagcagcctctcgtttccggcccgcggttcgatgtagatcagtgggtagtacgtgtcccgcttgccgggcggcttgatggcaaagctggaggcaatgccggtgtcgaggctggcatcaccgcgcacctgttgctcgaaggcctgcttgtcgtcggccaagatgcggggcgcatagttgacggcctggaacccagggtaggcggtcgccaggttcagccccgcgacgtagtccgtgaagtcgcttcgcgtgacggtctcggaggtgttgaatcgcgcacgcaggccgatcaggacggcaatgtagtcgtcgaagcgggcttcgaccttgcgcgccaggtcgaaggcggctgcgtcgaagcgcgcttgggcgctgcgcacgatctcctgccgggccgagacgccgagggcgatcgacagcgccgcgccggccacgaagatcaccagcggcaagcgaatcctgacccagacggacaatgacattggatttgatcctgtcgttggcacggaccggttggctctgggtgctgcaatgcagcacggagagaacgcagcattttgtattgttttgtcgcaatatatacaaatggtgcgagagcgtcacgcgaattgtgacgccgagagtgagggcatacacagatcactcgttcggacttgaacagttcgcgtctttgcgcccttgttgctgcgagtgcgggcttccgatgggtatcggtttgactttattttagatatatctaaaataatctagacacacctcggaaaggatgcccgccatgagacatttccacttcggccaccaccaccatcaccactgccacgccccccgcggcgaacacgaagacggcctctccggcggctgcggcccccgccacggcggcggcgaagagcgcatgcacggaggaggccgcggcggacgcggcggcgggcgggtcttcggccatggcggcctgcgcttcgtgctgctgcagctcatcgccgagaagccggcgcacggctacgaactcatcaaggccatcgaagaccgcctgggcgggagctacgcgccgagccccggcgtggtctaccccacgctcacgctgcttgaagaaatgggctacctcagcgtggaaacggccgacaccggcgggcgcaagcgctacagcatcaccgccagcggccaggagtttctggccgccaaccgcgacacggccgacgcgatgatggcccgcatgaacggcggcgtcgacggcgccggcccacgcggcgggcgcccgccgcaggtcacgcgcgccatcgagaacctgaagctcgcgatgcgcatgcgcctctcgggcaagcccctcaccgaacaacaagcccacgatttcgccgcggtgctcgacagcgccgcccagcaactggaacgcatctagaaagaattttcttgaatgactgacttcaccaccacaacctcccctgtcggcgcgcccgaccgcaccccgcgccgcgtgcgccacgagcttcgctttcgccaactcacggtaaagacggtgcagcgcgtgacgccgcatctgatccgcatcacgctgacgggcgacgatctcgcgggcttcaccagcctgggcttcgacgatcactcgaaggtctttttccccgacgcctcaacaggccagctcacgcttccgactgtcggcccagacggcccggtgtggcccgcgagcggccgcccgaccatgcgcgactacacgccgcgccggtacgacgccaaggccaacacgctcgaaatcgacttcgcgctgcacgaggccggccccgccacgcaatgggctgagcaggccaagcccggcgacattctgggcgtcggcggcccgcgcggctcgttcatcgtgccgaccgagttcgactggcatctgctgatcggcgacgacaccgccctgcccgccatcgcccggcgcctggccgagctgccggccggcgcgcgggtggtggtgctggcggaggtcgacagcgaagccgaccagattccgttcgagacgcaagccgaactcacgctgcagtgggtacaccgccgcggtgccgagccgggcctgagccccgtgctgctcgacgcgctggaggcgatgaagctgccggccggcgactttcatgcgtgggtagggtgcgaatcggcgattgcgaaggcattgcgcgcgcacctggtgggcgaacgcggagccaacccgaagtggattcgcgcctcgggctactggcggcgcggcgcggtagcgacgcacgacacgcacgacgagtgacccgcgttgctccttccccctccgggggaaggttgggatgggggcacgcggcctatgaaaaggccgctggctcttgatgcgccgcctgcccccacccccaccctcccccggaaggggagggagaaagacataaaactcagagccagccggctcgcctgaatcggtaatagaggtagctgcaggtgccgatcatcagcgtcagcgccgccgcatacccatagcgcaatttcagctcgggcatgtgctcgaagttcatgccccagatacccgcgaatgcggtgcacaccgcaaagatgctggcccacgcggcaagccgcttggtcacttcgctctcctcgatggtgaccatcgaaaggttcaccgaaatggcggtgccgatggtgtcgcgcatggcgtcgatggagccgttgatgcgccccaggtggtcggccacgtcgcgaaaatattcttgcgatgtgacgcagatctgcggcacccgcccgccgtgcaacttgccggccgcctccgccagcggcgccactgcgcgcttgagaatcagactgcgccgcttcaggtcgtacagctgcttgatcttgtcgcgcgccgcgccgccttgcgtgaagatctgctgctcgatggcctccagctccacctcgagcgcgtcgatgaccggaaagtagcggtcgaccaccgcgtccatcagcgcatagagcacaaagcccgcaccgttgcgcagcaactcgggctcgcgctcgcagcgctcgcgcacacccagaaagccctgcttgctgcggttgcgcaccgagagcacgtagttcttgcccacgaacacgtcgacctcccccacgttcacgcaatgttcgccctccggcgagggctcgaccaggtgcatcaccacgaagagggagttgccatattcctccaccttgggccgctggtggccgtggtgggcgtcttccaccgccagcggatgcaggttgaactcctcctgcatctgggccagctcttgcggcgtggcgtcgctcagcgccacccagacgaagcagccgggccggatgatgtattcgctgatgtcctcgactggaatatcggcgagcttggcgccgttttcataggcaacgcagttgatcagcatcggtactcgtccatggtcaggctggatatggggtcaggtcttcaccgcatccggattcgaagccgcggccaggagggcggtggctgccagcgaggcctcgatagcctctgtctcgctcctgagcagggcaagccctttttcggcgaacgccgagtggcttgcaacgtcggcccacaggctcgcggcggcttcggcgcatgtcagtgacgtgaagcggatgcggcccttcgccagctccacgaagcgtttctcgcgcagggggtccgcccggtcccaggcgccgccgacgagcacgcgccggccgcgtttgacacgaggttcgagctcggcaaagaagggcagcttggcggacacccagcccagcatgccggagttcaacgcggtgtcgaaggccgttggggcggtgtccgacttcgcaaagtcgcgcaaggtgcccagttcgtagagcaccgggtctttcggtccctttgcggcgctttccaccggcttgatgacgggcgggccattgcctgctcgcccatcgggccgtctcgacttgcgcaggtcggcgagctgggccggcgacatgcaaaggtacagcgcggcaagctctgcgggcaaggtggcggtgtcgggcagtgcgtctgcgtcagggccgcctttgaattcatccgggtggaccatgggcgccttgttcttcacgcgggggttcgcgccggcagattttagaacggcggggtgcacgctgattcgcatcggcaagccggccaggttgaccgtcggccgagccgtccggcgtccccgataatcgtccgagtgaaaacgacgactgcgcaaccctccccctcgaccagcgacttctccgggcatacgcccatgatgtcgcaatatctgggcctcaaggcaaaccatccggacaccctgctgttctaccggatgggcgacttctacgagctgttctgggccgacgccgaaaaggccgcgcgcctgctcgacatcacgctcacccagcgcggccagtcggccggccagccggtggtgatgtgcggcgtgccctttcatgcggtcgacacctaccttgcacggctcatcaagctcggcgaatcggtcgccatctgcgagcaggtgggcgaggtcggcgccagcaaggggccggtcgagcgcaaggtggtgcgggtggtcacgcccggcacgctgaccgactcggaactgctcaacgacaagagcgaatcgctgctgctcgcggtgcatgcgggcacgcgcaatttctgcgggctggcctggctcagcgtcacaggagccgagctgcggctggccgaatgcccggccgacgcgctcgaagcctggatcgcgcgcatcgcgccgagcgagctgctctacagcgcagaggtcacgccggccttcgagcagcgcctgaaggccgcgcgcgcggccacgcctttcacgctctcgatccgcccggcctggcagttcgacgggggtctgggcgaacgcaagctcagcgagcagatgggcagcaacagcctggccgcctggaacgccgaatcgctttccaacgcgcatgccgcggccgccgcgctgctgggctacgccgagcacacgcagggccgcgccctctcgcacgtgcagcgcctttcggtggagcgcgacggcgacctgatcgagctgccgccgaccacgcggcgcaacctggaactggtgcagacgctgcgcggcgaagactcgcccacgatgttctcactgctcgacacctgcatgaccggcatgggcagccgcctcctgaagcgctggctgctgtcgccccggcgcgaccgcggcgaggcgcaggcccggctcgaagccatcggcgcgctgcagtccacggtgctgggcggcacggccgcgccctggcgctcgctgcgcgagcagctcaagaacacgagcgacgtggagcgcatcgcggcgcgcatcgcgctcaggcaggtgcgcccgcgcgagctgctggcgctgcgcctggcgctcgccaaggccgagcagctggcgccgctccttcccgcatcggccgcgctgctcgaccggattgccgaacggctggcgccgccgccgggctgcgccgacctgctggtgagcgccatcaagcccgatccgtcggcgctggtgcgcgatggcggggtgatcgccaccggccatgacgccgagctcgacgagctgcgcgccatcagcgagaactgcgacgactttctgctgaagctcgaaatcagcgaacgcgagcgcaccggcatcagcaacctgcgggtgcagttcaaccgcgtgcatggcttctacatcgaggtgacgcaaagcgcgctctcgaaggtgcccgacaactaccgccgccgccagacactgaagaacgccgagcgcttcatcacgcccgagctcaagactttcgaagacaaggcgctgagcgcgcaagaccgcgccctggcgcgcgagaaatggctctacgaacagctcctcgatgcgctgcagccctcggtgccggcgctcacgcaactggccggtgccattgccacgctcgacacgctgtgcgcgctggccgagcgctcgcacacgctgcactggcgcgcaccgagcttcgtgtcacacccgtgcatcgagatccagcagggccggcatcctgtggtggaagcccgcctggccgaaaaatcgtcgggcggcttcatcgccaacgacacgcagctggggccgcagcagcgcatgcagatcatcaccggccccaacatgggcggtaagtcgacctacatgcggcaggtggcgatcatcgtgctcttggcttccatcggctcgcacgtgccggccgcggcctgccggctcgggccgatcgacgcgatccacacgcgcattggcgcggcagacgaccttgccaacgcgcagtcgaccttcatgctcgagatgaccgaggccgcgcaaattttgcacagcgccaccgcccagtcgctggtgctgatggacgaaatcggccgcggcaccagcaccttcgacgggctggcgctggccgccggcatcgcggcccagctgcacgaccgcagcaaggccttcacgctctttgccacccactacttcgagctgaccgagtttccggccacgcaccactctgcggtgaacatgcacgtgagcgccaccgaagcgggccgcgacatcgtgtttctgcacgaaatgcagcccggcccggccagcaagagctacggcatccaggtggcgcggcttgccggcatgcccgccgcggtggtcaaccatgcgcggcaggcgctggaggcactcgagtcgcagcatgcgcaaacccgtgcccaggtcgacctgttcgcaccgccgcccgcggctgaagctcccatggccagcgccgtagaatccgcgctggctgcgctcgaccccgacacgatgagcccgcgcgaagccctcgacgcgctctatgccctccaaaaactgaacacgcgtgaacacagtgccgccggctgaccgggcctgattcatgcgagacgaactcatgacttactgcgtaggcatcaaactcaacgccggcctggtgtttctctccgactcgcgtaccaacgcgggcgtggaccacatcagcaccttccgcaagatgatcgtgtacgagcagccgggcgaccgcgtcatggtgctgctgtcggcgggcaacctgagcatctcgcagtcggtgcgcgaaatcctccagatcgaggaactgcgcgaaacccgcgaagacggtacccagggcgcccccatcaccatctggaacgccacgagcatgttcgacgccgcgcgcgtgctcggctcggccgtgcgccacgtgtacgaccgcgacgccgaggcgctcaagcatgcggggctcgatttcaacgtttcgttcatcttcggcgggcaggtcaagggcgaaggcatgcgcctgttcctggtctacgcggccggcaacttcatcgaagccaccaccgagacgccctacttccaggtcggcgaatcgaaatacggcaagcccgtgctcgaccgcgtgctcacgcccgaaaccccgctcgacgaagccgccaagtgcgcgctggtgtcgatggactcgaccatgaagtcgaacctttcggtcggcctgccgctcgatctggtggtgtacgaggccaacaagctcgagaccgatcgcgtgatctgcatcgacgccgacaacccctactaccgcatgatgcacaacagctggggccagaagctgcgcgaggtgttcgacagcatcgaagacccggtgtgggacgacgccgccaccgaacatccgctgaagatgccggcaacccgccacagcccgctgcggaaaatctccacgcccgacgaaaagctgatctgaatcccgtgcctccggtcgttttttcgcacggcaacagtttccctgcgagcacttaccgcgtcgttctcgacagcctgcgcaaccgcggcttcgaggtcgatgccatcgagaagttcgggcacgacccgaagtaccccgtcaccgacaactggccgcacctggtccagcagctggccgacttcgcgcagcagcatgccgaccgcgcgggcgggccggtgttcctggtcggccattcgctcggcgggttcctgagcctgatgtgcgcggccatgcatccggcgctcacctgcggcgtggtgctgctcgactcccccgttctcggtggctggcgcgcgaacacgctgagcctggtcaagcgcaccccgctgatgaagaccgtgtcgcccggcgccatcagccgccggcgcaagaaccgctgggcgcaccgcgaggaagtgttcgagcactttcgccgcaagaaggcctttgccaagtgggacgagcaggtgctgcacgactacatcgaccacggcaccttcgacagcgaagacacccgcgagctgagcttcgatcgcaacgtggaaaccgcgatctacaacaccctgccccacaacctgagcgccctgctgcgccgcaatccgctcaagtgcaaggtggctttcatcggtgggcgccagtcggccgagatgaagcaggtgggcatgaagatgacccagcaggtcaccaagggacgcattgccatgctcgacggcagccacctgtttcccatggaaaagccgctggccaccgccgcggccatcgaggcgtcgctgcgcaacctgctgggctgatcggcaacggctcggccaacaggtgccgcgtctccgcacgaggcggatttttttcacggcggctgtcggctcgacgcatactcgttcgtccttggggtgacaggaacgatgaagcccatgcgcatgaccgacacggcctggatcgccaccacgctgaccgcttcgcggccgcgcgcggtggcggcgctgctgcgctactttcgcgaactcgacctggccgaggaggcgtaccaggaagccagcctgcgcgccctgcagcactggcccggcaacgggccaccgcgcgacccgctggcctggctgatcttcgtggggcgcaatgccgcgctcgacgaggtgcggcgccgccagcggcatgacgcattgcccgaaggcgaggcttcgatttccgatccggacgatgccgaagcccggctcgtcgaagcgctggaccacgcgcactaccgcgacgacgtgctgcggttgctgttcgtctgctgccacccggatctgccgctgacgcagcagatcgccctggcgctgcgcgtcgtgtcgggcctctcggtacaggaaattgcgcgtgcctttctggtgggcgaaagcgccatggagcagcgcatcacgcgcgccaagaagcgcgtcgcctcggctggcatccccttcgatgcgcccggtgcacgggagcgcggcgagcggctggcggccgtgtgcaccacggtctacctgctgttcaacgaaggctattccgcaagcggcggcgccgagcacgtgcgcaccacgctgtgcgacgaggcgatccggctggcacggctgctgctggatctgttcccggacgagcccgagctcatgggcctggccgcactgctcctgctgcagcatgcccgggcggaggcccggctcgattcccaaggcatggtcgtcctgctcgaagaccaggaccgcagcctctggaaccgggcgctcatcgacgaaggcctggcgctcgtcgaggcggccctgcgccgcgggcagcccggaccctaccagctgcaggcggccatcgcggcaacgcacgcccaggcagccagcgcggcggacaccgactgggccgaaatcgaccggatctataccgcgctcgaagtgctgcagccctcgcccgtggtcacgctcaaccgcgcggtggccatcgccaagctgcgcgggcccgaggcagcgcttgcaatgatcgggccgttggcgcagcctctggccgcctacttccatttccacggcctgaagggcgggctgctgatgcagctcggccgcatcgaagaagcgcgtgtcgcgttcgccaaggccatcgccctcgcccgcaccgccgccgaagccgcgcacatccgcctcatgctcgaccggctggaagacattcgcccaccgcgcggccgcaccaaccctgcggcctgaccctccaagcccccagaaggaagaccgatgctctattccatcctcatctacggttcggagtccgctgttgccgcgtgggcgccggaagtcgaagacgaaatgctcgaacggcacaccgacctgcgggacgagctgcaggccaagggccggctcggcacggtgctgcggctgatgcccgacaccgccaccacggtgcgccgcgccgccaccgcccatccgctcgtcaccgacggcccctttgccgagaccaaggaacagctgatgggcatctacatcgtcgactgcgacaccctcgagcaggcccgcgatgccgcgcgccggctggacttcgaaaccggcgtgttcgagattcggccggtcacctggtacgacccgggcgtgattgcggcgcgcatcccgcaggtctgatcgaaaaaaatctgtcgccattgtcgggtggcgccggcaccgtcgtccttggttcgaacgcccgcattccgctggcgaccaccaaggagaagttcatgtcgtcgaattcgttgcaggacaagtgcgccgtcgttcatggcggtggcggcgccatcggcggcgcggtggcccgggcctttgccggcgcaggtgcaaaggtcttcctcgcgggccgcacgcgcgccaggctcgatgccgtggccgaggacatcgtggccatgggcggcagtgccgaagtggctgtcgtcgatgcgctcgacgaggcggccatgctgcgccacgccagcgaggtggccgaacgggccggtggcatcgacatcgcgttcaacgccgtcggcgtgatgcatgttcagggccggccgctggcggaactctcgctggcggactacttcctcccggtccaggcctacacgcgcagcaatttcctcaccgcgaaggccgtggccccgcacatggcgcagcaaggcggcggcgtgatcatctcggtgtccacgccggcctcgcgcctgcccgggccgggctatctgggccacgccgtggcctgcgcgggcgtcgaggccctcacgcgccacatggcaggcgagctggcggccttcaacatccgcagcgtgtgcatccgatcgcacgccattcccgaggccgccgctgcgggctcgcacagccgcgaggtcttccgcccagtggccgaaagcatgggcatgacggtcgagcagatgctcgcggccaagccggccggtctgctggtgaagcggctgccgtctctggaccagatggcgggcaccgcggtgttcctggcttcggagcacgccggcgcgatgaccggcacggtggtcaacatgagcggcggcgtgacgctggactgacccaccctggaacaatccccgaaaatcagtaaaaacgacctaccggccttgccaccgatcagaatgctccgagcacatgtccatgtcccaaccggaagtcgttgaagccgtttccttgagcccctcgctggtcgtcgaagacgacccggcgatgcgcgagcgcctgggccgcgtgctgtcgatgctcggctgcgacgagccgcagatcgcatgggccgacagcattgccacggccaagaacatgctcgaggcccggagcttcggcatcgccctggtcgacatcggcctgccggacggcagcggggtcgaactgatcggctggatgcaggcgacgcatcccaaggtgccggcggtggtgatctcggcctggcggaccgaggaaatcatcttcgcggcgctgcgtgccggcgccatcggctacctgctgaaggagcgcgacgacctcgaactgagcattgcgctgcgcagcaccgagcaagggggcgcgcccatcgatccggccattgcgcgccatatcctcggctggcttgcagcgcagcagccgccgctacccgccgtggtggcggccgatgcgccggccccgctcccggtggcgctgaccccgcgagagcgcaagatcctcgaactggtggcgcaggggctgagcaatcgcgacatggccgaatcgctgtcgatctccaggctgacggtggaatgccacaccaagaacatctaccgcaagctggccgtcacctcgcgcaccgaggccgtctaccaggcccgaaggcacggcttgctgcactgatcgcgccggcctccttctctgccgcgcctcaccatgcatagcccgcctgcacgcgggcggcaatgcggttgctgctgccgctgctggttgcggtggagacacccaggcccaggttcaggttgtcgctgacctggtagccgaaagcgaagccgatcgccgacgcgccggcgtagttgcccacggcggcacccatccatttcctgcccaccggcagtgtcggcatcgacggcatggccagcgccgccgcaacgccctgcgctgcaaaggcgttcgcctggttggttgcgttgctcaccgcctgctgcaactggttgacgttgacggcatcggtgcccagcagaccgggggcgacattcgcaatgccgcgcaactggccggtggccgcgttgcctaccgagacggtgttgtcgcgatcggccaccgagccctgccccagcgcgaccgcattgctgcccgaagccagtgtgttggcccccagcgccacggcgttgttgccggtggccaccgcgttgttgcccacggcggtggtgggatcggccagcgccttggcgccggcgccgatggcgaccgagcccgcatggttggcctgcgcgccattcccgatggcgacggtgttctcgccattggccttcgcgttggtgcccatcgacgtgctgccggcgccgctggagctggccccgggcccgcaggccacggcgccgcccgcgcccaccgcgcatacaccgctggccaatgcctggttcatcaaggcctgcaatgcggtgacctgctgaacggtgaagttgttggccgtggtgatggcggtctgctgggcctgctgcacctgaccgacattggcggcatccgtcgtaacctgacccgcgccgacgttgctgatggtggtgccggcgccgccgttggcattgagttgcagcgaagtgccgcctgcgccgtactgcgccgagttctgcgccaagccgagtgcggagttggcggttgtctgtgccgcgcccgcggcacccacggctgcgttggcagtggtttgtgcagcagaggcggcggtttgtgccgcggaggcggtggatgccgcggtgctggcggtctgctgcacggtgtacagctggctgccgttgacggcgtcggtgctcgtggaggttaccgaccccgcgctgacgttgaccaggccgcgcgtctggcccgcggttccgaaagacaccgtgttggccgccgtggcgacggagttcgcgccgatggccacgctgccgttcgcaccgctcgcgacctggctgccggacccgatcgccacgctgcccgtggccagtgcggccgcacccgaagcaccgccgctggcgccgccgatcgcggtgctgccgttgccggatgccacggcgccctggctggtgccggaggcgcttccgatggcgatcgccgcattgcccgaagcctgagcgccgctgccgcccgtctggccggtactgccgcaacaaccgtcggtgcccacgcctcccgcgccgagcgcgatcgcgccgcccgccgaggcctgggcgccacgtccccctgcgccgcccgttccccccgcttcgcccagtgcgccagcgccgccgcccccgacggcggttgcgccgcttgcggttgcgctggctcccgccccgcccacgccgccgacgccacccgcggttccgatgccgccatcaccaccggcaccgaccgccgtggccccgtttcccgagacgacggccgcagcgcctccggcgcctgccgtcccgttgttggttgcagggccgacattgcccgccgtgccaccggcaaatcctgccgcgtaggcgcttcccgcgaccagcaacgcaatcgcaggcagatgccgaagtttgcgcaacccttgacgggtgccactggtgccgatctggactggcatggacttcctctttttcgaaagcaaataaaacaaacgtggcaaagtgtgtctttccgggctcgacggggccatccccgaaaattggtaaatgccacaccgagaacctctcccgcgggcatggcttgctgcgtcgattggcgccttccttttcctcttcctcctccttgtcgccgtcccggcgatggcgcgggcgcaacagccggcccctccactccatgtcgaagccgtgcgcagcccgggctggaacgacaccgccccgccggccgacggctggacgcccgttaccctgcccgacagctgggccggacgctggccgggcttcgacggcgtggtctggtaccggctgacctgggagcagccggaacaggtgcgggaggctgggctgctgctgcactacctcaacatggccggtgcggtgtctctcaacggcacgccgatctcgcgcgacgagagcctggtcgagccgctcacacgcgcctggaacacgccgcgctactggctgctggcaccgccgctgctacgaagcggcagcaacacgctgctggtgcgcgtctcgggcctgtccgcctaccaggcgggcctcggcccggtcagcctcggcacgccggccacgatgcaggccgcgttcaccgacgagcacatcgtgcgccgcgacctgcaggtgctgggcctcgcggtgagcgccgcggtctcggccctcttcgccgcgctgtggctgatgcgccggcgcgagaccgcctacggctggttcgcggtaatggacgtgctgtggctgctgttcggctacaaccagatagcaaccagcccctggccctttgcctccaaccacagctggcaggcgcttaacacctcgctgctgctgttgttcagcgcctcctatgtcgtcttcgcactgcgcttctgcgaccgccgcatgccgcgcctggaactggcggcactgctggtcacgctggccggcgtgctcgacctgtggctggccaacggcccgagccttcccatgcatcgcgccttctggaccctggtgggcggcctcatcaccattgccgtcaacagcgcgtccatcgtgcatgcctggcgccatcccggcagtccgatgcgtttgctcgcgccgttcatggcggtgtccgcggtcgcaggtgcccacgatctgctggtgttcacgcaggtgatcgacagcaacgtctactacacgaccatctcgtcgtacctgctgctgctcggcatggcgctgacccaggccgcacgcttcgtgcagagcctgaaacgcatcgagaacttcaacaccgagttgatcgaggaagtgaacgccgccaaggccgagctggccgccacgctcgcgcagcagcacgcgctcgagctggcgcatgcgcgcatcggcgagcgcgtcaacctcgcaagcgacctgcacgacggactcggcggcatgctggtcggcagcatcgcgacgctcgaacgcaagcccgagaacctctccgcgcccgaactgctggccctgctcaagcgcctgcgcgacgacctgcggctgatcatcgacgccaccggccgccacgacggcgcccgggcgttcggcgagctgctcgcgccgctgcggcaccgcacctcgcagtcgctcgacgccaacggcatcgactgccggtggcaggtgtcgaacatcgagacgctagaactcccgccttcgcagtgcctcgacctgctgcgctttctgcaggaggcactgaccaatgtgctcaagcacagcgcaagccgccgcgtggacgtggccgtgacgcgcgccggggccgaactgcagctcagcgtgcgcgacgacggccgcggcttcgtggtggatggcgtcgacaagggggccggcgccggcttgcgcagtctgcgcacgcgtgcccgccgcctcggggccgatcttcagctgcattcgcggcccggcgagacgcaactgacgctgcgcatgccgctggcacccgccgcctgagcgccctgcggtcgccgagcctcccgcgcgcggcgcattttttcgtctacatccgctcggatgggccggcccccgcaaaggccctgtcaagaggggaacaaaccagatgatacaaattgcaatcgcctgtaacattcggcgagaataagtaaaaacgtcccacttcgcaggcccccgttccaaaatgtcccacgaatgtcaacttctcagtcggaagcccttgaagccatctccctgagcccgaccctcgtggtcgaaaacgaccgggggatgcaggaacgtttgcactacgttttgtcgatgctcggatgcgacgagccgcagatcgcgtggaccgacgacgacgcgacggccatccaattgttcgagagccagcacttcggcgtcgccctggtggacatcgggttgccggacggccgcggaatcgaactcatcgaatggctgcaagcgcaccacccgcaggtgtccgcggtggcaatttccgcctcgttgcgcaccgaggaagccattttttcggcattgcgcgcaggcgccgcggcctatttgctgaaggtacgcgacgatctggaactcagcatcgcgctgcgaagcatcgaacaaggcggcgcgctcatcgatgcggccattgcccggcgcattctcgcgtggcatgccgatcacgccagcgacttgctgtccatgccggacgtgatgctgacgctgcgcgaacgcaacatgctggaactcgtggtgcaggggatgacccaccgcgacatcgccgaaacgctttcgacgccccggctggcggtggaacgccgcaccagggacatctatagaaagctggccttcggctcgcgagccggagcggcgcacacggtcaatggaaccattttgctgcgctgaggcgggcggctcttcgcagccccggcgcggcggcgcatcgcgctcactccgcccagaccaccgtgccggtccatgcagtggccagcaccacgatgccgaaggcaatgcggtaccaggcaaacggaatgaagtcgtgcgtgctgatgtacttcagcagccagcgcacgcaaagccacgcgctcgcgaacgaaaacaccagccccacggagaacaacggaacgtcggccatcgagagcagtgcgcgctccttgtagaggctgtaggcgccggcgccgatcagcgtcggaatggcaagaaagaacgagaagtccgtggcggcctggcgcgacaggccgagcagcatgccgccgatgatggtcgagccgctacggctggtgcccggaatcatcgcgaagcactgcaccaggccgaccttgagggcgtcccacatcgtcatgtcgtcgacgtgctcgatgcggatcgagcccggcggccgcttctcggcccacaggatgatgaaaccgccaatgatgaaggtgctggccaccaccacgggcgtgaagagctgctccttgatcatcttgccgaatatcagcccgagcagcacggcgggaatgaagccgatgaccacgttgagcgcaagacgcctggccctggcctgccgcggcaacgccaccacggtggaatggatcttttgccagtacaccaggatcaccgcgaagatcgcaccggtctggatggcaatgtcgaacaccttggccttggcgtcgtcgaagccgagcaacgagcccgcaagaatcagatgtccggtcgacgagatgggcagaaactcggtcagcccctcgacgatgcccatgaccgcggccttcaccagcaaaacgatgtccacgcttactcctttaaagagcatcaattatggcgaggcatcgagtcaggcccggttcagctggcccctgacaattgcgggccttatccggggacttgaccggcgcgcagccgcagggcccgcaccgcactgtcgacggtggtgagcactggcaggccgctcgcttgctcgcaggcggtgcgtgcgcgggccatgctgaactgcgcgagcgcaatgcgcgtgcaaccgagttggcgcagcgccagcgcctgcgcggcaatcaacgcatcgtggcgctgcgtgtcgccagcgttcagcgcatcgagcgcgccttcggcgagcacgggttcgagcgcgatgccggacgggaattcgggtggcatcgacacgagcgtggccgcgaaggttgcgatgaggccgagcttgccctgcccttcggtctgagcttgcgcggcctcggcaaccatggcctcgttgggcttgagcaccggaatgcccgcatgccgccgcgccaccgcctcgatgcacggcccgaaggccgagcaggtgaagagaatgccctctgcgccggtatcgaccgcgtactgcgcgagccgctgaaatcgctcgtgcatggcggcgtcgagcccgtggccgccgcgcgccagatcggccgacaggctgtcgtccagcaaattcatgcgcacggcttcgggccagtcgcgctcgaaggcggcgttgatgggcgccaccgaatgcgaaagcgcgtggatcagtgcgatgcgggtcatgcggaaacggcggtcagatgcccttcgaagacgggttggcgaaagcctctttggtctcggcgttgagcgggtagttgatgttgatgcccttgggcggaatcggcgacgtgaaccacttgttgtagagcttctccatctcgccggacttcatcatgcccgacaccacgcggtccaccagcgccttgaaggccgggtcgtccttgcggaacatgagcgactggttctcggtgcgcaggctctcgccggtgacgatgaagtccttcgggttgcgcgcattcgcgatctggccggccagcaggatgtcgtcgagcacgaaggcctgcgccctgccgctttccaccagcaggaacgaatcgctgtggtccttgccgccgaggttgttcacctcgagattgcggcccttgtcggcttcgcgcagcagacggaacgaggtggtgccggtggtggtgaccaccgtcttgccctgcaggtcggcaatgctcctgatgcccgaatcggccttgaccagcatgcgcacgttgtagcggaagatgtcgggcgaaaacgccacctgcttctggcgttcgaccaggttggtggtggagccgcactcgatgtcgaccgtgccgttctgcaccagcggaatgcggttggccgaggtcacggcctggtacttgatctcgacggccggcagcttgagctcgctcttcactgcctcgacgatgcggttgcagatctcgatgctgtagcccacgggcttcaggttgccatcgaggtacgaaaagccgaacgacgactcgcggtagccgaaggtgatggtgccgcttgccttgatcttggcgagcgtgtcgttgttgtcctgggcctgtgcggacgtgtgcggcaacaacagggcgaaggccaccgcgagagcggcagcaccgaagggaatcggcagacgaagcttgggcatgggagcgctcctcggaacggcggttgaagaaaacggcgaaagaaaatcgaaagtggtcagcgcgcggcggcactcgtcaccgcgtcgatcgaagcagcgaggcgggtggcgatttcccgcaggtcttgccgcgttgcgatgaacggtggcgccagcagcacgtggtcgccctgccggccatcgaccgtgccgccaaaggggtagcacagcaggccgcgcgccatggcgtccttcttgatggctgcgttgacctgcaaggccggatcgaacggcgccttgctcgcgcggtcggccaccagctcgatgccccagaagaagccgcggccgcggatgtcgcccacgtgcgcatggccgccgagcgcgtcggccagcatggcgccaaaggccgcgccgtcttcgcgcaccttggcgaccaggccgtcgcgccggatcacctgctgcaccgcgagcgccgccgcacaggccatcggatggccgagataggtgtggccatgctggaagaaaccgctgcccttggacatggcctggacgatcctgccctgcgccagcaccgcgccgatcggctggtagccgccgcccaggcccttggcaatggtcatcaggtcgggcaccacgccctcctgttcgcaggcatgcagcgtgccggtgcggcccatgccgcacatcacctcgtcgaggatcagcagcacgccgtatttgtcgcacaccgcgcgcacggccttgaagtagcccggcacgggcgtgagcacgccggccgtggcgccgcccaccgtttcggccacgaaggcgataacgcgatcggcgccctgcgcgacgatggcggcttcgagttcggccgcaaggcgcaggccgtattgctcggcgctttcatcggcccgctgctcgcgataggggtagcacggcgccacatgcgtggccggcacgaggatgggcgcgaacggctcgcgccgccatgcattgccgcccacggccagcgcaccgagcgtgttgccgtgataactctggcggcgcgcgatgaagtgcgtgcgctgcggctctccgatttcgacgaaatactgccgcgccatcttgagcgccgcctcgaccgcctcggacccgccgctcaccaggtacgcatggctcatgccctcgggggcgaaagcgatcagctcgtcggccagttgctcggccacttcgctcgtgaagaagctggtgtgcgcgtaggccagcttgtcgatctgcgcatgcatggcggccagcacctcggggtgcgcgtggccgagcgacgacacggccgcgccgcccgaggcatcgaggtattcgcggccttcggcgtcgcggatgaacaatccgccggagccggcggcaacgggcggggtctggcgaaggtgacggtgaaagacgtgcgtcatggcggctgggcggcggtggatggcgattgcgtgtttggaactaacgtttccgccggattattgtttggaacatttgttccgtcaactgttgcgtcgttccatgtccggtacattcgttccaacgaccgccagaagagagacaccgccatgggcgccagagaccagatccgccagcgtttcaacgagttgagcccggccctgcagcaggttgcgcgctacgtgctcgaccaccccaacgaggtggtgaccgcatcgatgcgcaacgtgggcacgcgcgcgcagagcacgccggccacgctggtgcgttttgcgcagcacctgggctatgcgggctggccgcaactcaaggaagcctttgccggcgacatgggcctcggcagcgaaacctacggcgggcgggccaagcaactcatcggccgcgcgcaggaccgaagcctgacggccgagatgttcgaggtgcagcgccgcaacctcgaggccacgcaccagcagagcgagcaggcgctgcaaaaagcctgtgcgctgatcgagaaagcgccggccgtgcatgcggcgggtttcagggcctgctttccgatcgcgttttcgttcgtctacgtgtatcggctcttccgcgccagcgtgcacctggtcgacggccagggcggctcgctcgaaatgcagcagcgcgcctttgccaagggcgacgcgctggtggtggccagcttcatgccctactcgcgcgaggcgctgcaggtggcagaggcggccaaggcggccggctgccgcatcgtcgccatcaccgacagcgtggcatcgccgctgtcgctgctggcggacgaaacgctgcttttcacgatcaacagcccttctttctttccgtcggtggcggcgggggttgccgtgaccgaggcgctggtcgaactgctcgcaagccgcgcgggcaagccggtgatccggcgcatcgaccaggccgaggcgcagctgttcgagtcaggggcctatctggtgccgccggtgccgcgcggaaattaggcctccgagccgaatccgcgtgctgcagtgccgcattggcggaaccccgcccgagcccgaatagtcgaacgactgtcgcggttgtgtgccgcgacaggaggtaatgaccatgaagcaggtgaaacattggcaagacccggtcagcgttgcgctcggtgcgtggctgatcatctcgccttgggtcctggggttccaggacgtcacttacgcgatgtggagcgcagtggcgacaggcatcgtgctcggcgccgtggcgctgggggcgaccctggtaccgcgtgcatgggaagagtggaccgaaggcgccattgccatctggctggccgtgtcgccctgggtactcggctttgccaccgtcgagaaagcgatggtgaatgcggtgctcgtggcggcggcgatcctggtgctcgcgctctgggttctggtgaccgacaaggactacctcggcgggtcgatggaccgtcacgcgcactgagcgcatgaccatcgcgccgtgaagaagaacggctccgagcgctatccgcgccggggctgaggagatgggcagccgcccatctcgcgcacagccagttcactccgctcagcggaggggagtaggctgttgccagccgccgcccaaggcctggatcagcgccaccgcggcggtctgccgattgacctgcagctgcaccagcgtgcgccgcgcgctgagggcggctgcctgcgccgtgaccacctcggtgtagctcacctgggccgcgcgatagcgattgagcaactgctgctcggtcttgtcggcggcggccgaagcctcgcgccgcaggccctcttgctgtgcgagcgcggcgccggccgtcaactggtcttccaccgcctggaacgccgtgagcaccgcctgccggtagcgtgccacgctggcttcgtgggccgccttggccgagtcgacgctcgcgccgatggcgcccgcatcgaacaccacctgcgccaccgagaggccgagcgcccacagcgtgttggatgcgttgaacaggtctttcacgcggctcgcgctgctgcccaccgaagcgctgagcccgaagttcgggaagtacgccgaccgcgcaatgcctatctgcgcattggccgcggccaccgcgcgctccgctgcggcaatgtcgggccggcgctgcagcagggtcgacggcacgccggtggggatgccgggcaccgtgggtgtccactgcgcggcgggcaggctgaagtcggcgggggcgacgcccaccagcatggcaatggcgtgctccagcgtggtgcgggagcgctgcaggcccacgcgctcggcctgcgcggtcacgagctgggtctgcgcctgcagcacgtcggtctgggccgcgatgccggccttgtagcggttgctcgtgatctcgaaggcgcgctggtagccctcgatggtctggtcgagcagaacgatctcggcgtcggcttcgcgcaaagaaaaataattggtcgccaggtcgccgatggccgagaggcgtgccgacgccaggtcggcctcgctggcctgcgcattggcctcggcgctggtcacggcctgccgcaaccggccccagacatcgggtgcccagtcgacacccagcgtggcggaaaaggcattggacgcattgctgctgccgccgatgttgccgcttcgccggccgctgccgtcgagcgaaaccgtgggaaacagcgcggcacgctctccccgcaccagggccttcgcctgcgcgtagttggctacggccgcggcaatgttctggttcgacacctgcaccctggcggccagctcgtcgagcgcggcatcgccgaagagcttccaccaatcgccgcggtcgagcgcgtcggccggggcggcgggcagccagccctcggcggtcttctgctctttccacccggcgggcatggccgagcttggcacctggtatgcagggcctacggcgcagccggccaccatggccgcgaaggcgagcgcggacagcgaagggatgcgggtgcgatgtgtcatggcaagggattcattttctcggaggccgggaacaccgcggaaccggctttgccgggccgccggtgttgcccccttgaggggagagtcgagctacacgaagtgagcgagacgggggtgggtttcatacgggtgagcttgccgcgcggctcaggtggcgctcgttgccggagcgccggcgcagcttgtcgagcagcacgtagaccaccggcgtggtcagcagggtgagcagctggctcgccaccaggccgccgatgatcgccacgcccagcggctggcgcagttcggcgccctggccgaagccgatggccagcggcagcgcgcccagcgcggcggccagcgtggtcatgagaatcggccggaaacgcagcaggcaggcctcgcgcaccgcttccaccgccgagatgccgcgggcgcgctcggcctcgagcgcgaagtcgatgatcagaatcgcattcttcttcacgatgccgatcaggaggaaaagcccgatcagcgcaatgatcgaaaaatccatgcggaacagcagcagcgcgagcaccgcgcccacgcccgccgaaggcagcgtggtcagcacggtgatcgggtgaatcaggctttcgtagagtatgccgagcacgatgtagatgaccacgatggccgccacgatgagcgccagctgctgcccctgcgattgctgcgccgccagcgccgtgccctggaagctgcctcgcacgttcacgggcatggcaatgtcggcctcggcctgcgcgacgatgcgccgcgcctcctgcagcgtgacgccctcgtccaggttgaacgagactgtgctcgcgagctccgtgtcctggtggtcgatggagctcggcaccgcgcgctcgctgaccttggcaatggccgacagcggcaccatcagcgtggtgttcgcggccagcgcctggccggtggacgcggtgcgcagtgccgggttggccgacgtggtggtcgaggtgccggtggtcgcgtcggtggtgttggccagcgaactcacgacggaggcaccgctcgcggtggtgctggtggtgagcgtcgagggtacgtacaggtccttcagcacgacgggcgcgcgctggtagcgtggtgcccattccatgatcaccgaatactggttgagctcgtcgtagatggtggcgaccgagcgctggccgtaggcgttgtagagcgcgctgtcgaccgcgctcgacgtcacgcccagccgcgcggcgctttcgcggtcgacatcgacgtaggtctccacgccgttgtccgcctggtcgctgtcgacatcggtcagcgccgtttcctggcgcagccgatcggccagcttggcggtccaggtgcgcaggtcggccaggttgtcgcccttcagcgtgtactggtaggcggagttgctcgaacgcccgcccatgcgcaggtcttgcaccgggctcaggaacacccgcaggccggtgagctggttgagctgcggccgcagcctgttgaccaccgcggcggtcttctcgctacgctgcgacaccggcttgaggttgacgaacatgaagccgccgcccgagcggctgccacccgcgaagcccaccacggtatcgacggccggatccttgtggatgatgtcgaccgcctggcgcagtttttcgctcagcgcggccgacgaaatgctctggtccgcgcgcaggcccgcattgagctggccgttgtcctgctcggggaagtagcccttgggaatggcggagaacaggtacacgttgagcccgatgacggccagcagcaccaccatgaccacggccttgctcgcgagcgcccagtcgaggctgtgggcataggtgcgcaggctccactgatagacgctttccgccatgcgcgccaggcgccccggcggcttggcaccgggctgctcggcccgcagcagcatggcgcacagcatgggcgtggtggtgagcgagatcaccagcgaaatcagcaccgccaccgacagcgtgaccgcgaattcgcggaacaggcggccgatctgcccgtccatgaacagcagcggtatgaacaccgccaccagcgacaggctgatcgacagcacggtgaagcccacctcgcgcgcgccgcgcagggccgcctcgatgcggcccacgccggcctcgatgtggcggctggtgttctcgagcaccacgatggcgtcgtccaccacgaagccggtggccaccgtgagcgccatcaggctcaggttgttcaggctgtagcccagcaggtgcatcacgccgaaggtgccgagcagcgacaccaccgtggccacggccggaatgatggtggcacgcgcacggcgcaggaacaggcccaccacgagcaccacaagcgcgatggagatcatcagcgtggcctcgatctcgcgcagcgaggcgcggatggagttggtgcggtcggaggccacctgcacctcgatgtcttgcggcagctgcgcgcgcagttcgggcagcagctcgcgcacgccgtccacggtctggatgatgttggcgccgggctcctgcgtgaccagcacgaccaccgccggctggccgttgaagagacccagggtgcgcgtgttctccacgctgtcgatcacccgcgcgacgtcgcccagccgcacggccgcgccgttgcgccaggcgatcaccatgtcgcggtactccactgcgtggcggcccggcgagggcgtgtagatctgcagccggcgctcgtcgttctcgatcgcgcccttgggacggttggcgttgttggcctggatggcggcgcgcacgtcttcgctgctgatgccgaagcggttgagcgagaagggctcgagctccacccgcacggccggcagcgaaccgccgccgatctcgacctcgcccacgccctccacctgcgagagcttctggctcacgatgttggacaccgcctcgtagatctgccccggcgtgcgcgtcttggaggtgagcgccaggatcgcgatgggtgcggccgtcgggttgcgcttgcggtaggtcgggttgctgcgcaaggtggccggcaggtcggcccgcgccgcgttgatggcggcctgcacctcgcgcgcggcgctgtcgatgttgcgcttgaggtcgaactgcaggctgatgcgcgtcgagccgttggaactggtcgaggtgagttcgttgacacccgcgatcacgccgagccgccgctccagcggcgtggcaacgctcgatgccatggtgctcgggctcgcgcccgcgaggctggccgtcaccgagatggtgggaaagtcgacctgcggcaacggcgacacaggcagcacgaagaacgccgcgatcccggccagcgcgatgccgatggtcaaaaggaccgtggcaatcggacgttcgacgaaaggcctggagaggttcatgcggccgcggcctcccgcttgggcccgaagcggcggcccagccggtcgaacgccaggtagaccaccggcgtggtgaacagcgtgagcacctggctcaccaccagcccgccgaagatcgccaggccgagtggccggcgcagctcggcgccctcgccccagccgaacatcagcggcagcgccgcgaaaagcgccgccagcgtggtcatcagaatgggccggaagcgcagcaatgccgcctggtggatggcctcctgcggcgacttgccctcgcgccgctcggcgtcgatggcaaagtcgatcatcatgatcgcgttcttcttcacgatgccgatcaagaggatgatgccgatgatgccgatcacgcccaggtcgttgccggtgaccatcaaggccagcagcgcgcccacgccggccgagggcagcgtcgagagaatggtcagcggatggatgtagctctcatacagcacgcccagcacgatgtacacgcacaccaccgccgccaggatgagccacagctggttggaaagcgacttttcgtaagcacccgccgcacccaggaaggtcatggtcatgctcgacggcatgccgatttccttggccgccgcgcgaatggccgccaccgactttccgagcgccacgttctccgccgtgtcgaagcccacggtggccgccggatactgcgccacgtgcgtgacctgcagcggcgccggctgctcgcgcaccgtggcaatcgacgacagcgtggtcgcaccgccgccacccgtgcgcagctgcaggttgcccagcagctgcggcgacgccagggcttcgcgctgcgcttccaggatcacgcggtactggttggtttcggtgaagatggtcgagacgatgcgctggccgaacgcgctgtagagcgtgtcgtccaccgaactggccgtcaccgacaggcgcgaggccgtgttgcggtcgatgtccacgtacgcggccaggccctgggcacccgccgtggtggtggggttgcgcaccaggggttcggagcgcaggcgctccaccagcttttgcgcccaggcatcgacggtgttggtgtccaccccttcgagcgagacgcggaattcggtcgggccggtttcggcgtcgatggtcaggtcttgcgtgggctgcaggtacagcgtcacgccggccacggcacgcacgcgctcgcgcaggcgctgcattgtggcttcctggttgccgcggtcggcgcgcatgttgatgagcatgctgccggtgttcagcgccgtgttgttggcggcgtcaacgcccaccaccgagctcacgctggccacttcggggtcggccaggatggccttggcggcttgctgctgcagctcggccattcgcgtgtacgacacgtcctgcgccgcctcgatgcgggcctgcagttgtccggtgtcctgcgtgggaaaaagccccttcggaatcaccacgtagagcagcaccgtgagcgccagcgtggccagcgcaacgaggagcgtcagcggctggtggcgcagcacccattgcagccacacgtcataacgcgcgatcacgcggttgaagaagcgctgcacgctggcaccgaagcgcccgccctcctcggcctggggcttgagccagcgcgccgacatcatcggcaccagcgtgagcgacaccacggcggagatcaggatggtgatggccagggtgacggcaaactcgcggaacagccgccccaccacgtcgcccatgaacagcagcggaatgagcaccgcaatgagcgacaccgtgagcgagatgatggtgaagccgatctgcgtggcccccttgagcgcggccttgaacggcgggtcgccctcttcgaggtagcgcgcgatgttctcgatcatcacgatcgcgtcgtccaccacgaaaccggtggcaatggtcagcgccatcaggctcaggttgttgaggctgtagcccagcaggtacatcaacccgcaggtgcccacgagcgagatcggcaccgccaggctggcgatgatcgtggcgcgtacgctgtgcaggaagaagaagatcaccagcaccaccatcaccacggccagcccgagttcgatctgcacgtgcgagaccgaggcgcggatgccggtggtgcggtcgctcagcacctccaccttgagcgagcccgggagcgatgcctgcagttcgggcagctgcttcttgatggcatcgaccgtgccgatcacgttcgccccgggctgccgctgcacgttgaggatgatggccgggtagagcgttgccggctcctcgccggcgcgaagcgctgcccaggcgcccagctgcgtgttctcggcgccatcgaccacgcgcgccacctcggtcatgcgcacgggcgcgccgttcttccacgcgacgatgaggttcttgtagtcgtccgccgtcacgagctggtcgttggcgttgatggtgtaggcccgcttcggtccgtcgaagctgcccttggcgctgttggcgttggccgcggtgatggcgctgcgcagcgtgtccaggccgatgcccaccgacgcgagggcgttggtgtcggcctggatgcgcacggccggccgctgcccgcccgaaagcgacaccagccccacgccgctgacctggctgatcttctgtgcgagccgcgtgttcacgaggttctgcacctcggtgagcggcatggtctcggagctcacggccagcgtgaggatgggcgcatcggccgggttcaccttggcgtacacgggcggcgccggcaggtcggccggcagcagcgagctgcccgcgttgatggcggcctgcacctgctgctcggccacgtccagcgtctggtcgagcgcgaactgcagcgtgacgatcgacacgcccgccgagctcaccgagctcatgcggttgaggccggccatctggccgaactggcgctcgagcggggccgtgacggtgcggcccatgacctcggggctggcgccgggatagagggtctgaacctggatggtcgggtagtcgacctgcggcagcgcggccagcggcagcagccgcaagccgacgaggccggccagcacgatggcgaccatcagaagcgccgtggccaccggccgttcgatgaaggggcgggaggggctcatcgcgaacgcgctcgctggttccgtgtgtcttggttgctcgtcattgcggggggcgctggcgccgccgctctccgccttcgccgcgctctccgcgttgtccgcgcggacccgaagccgcaccgcgcggccccgccgcgggccggtcgccctgcagctgcacgaccgcgccgtccttgatgcggtcgccgccttcggtcaccacgttctcgccgacacgcaggcccgaggtgatggccaccacctcggcgttggcttcgccgcgcttcaccggccgcgtcgacaccttgcggtcttcgtcgatcacgtacacatagtcgccgttggggccggtgcgcacggccgtcaccggcaccaccaccgcccgcaccttgcgcagcagcatctgcacgttgacgaactggctcgggaacagcgtggtctctgcattaccgaagcgggccttggctttgaccgtgccggtggtggtgtcgaccaggttgtcgagcgttgaaaaagtcccggtgtcgagcgtcaccgcgcgggtgcggtcgaacgcggtgaccggcagcggctcacccttggcaagctgcgactggatgtcgggcacccggtcttgcggcaccgagaactgcacgtcgatcgggttcatctgcgtgatgactgcgatgcccgtggtcgcattggccgtgacggtgttgcccgcatccacggcacgcaggccgatgcggccggccaccggcgaggtgatgcgggtgtagtcgaggttcagcttggcggcggcctcggcggccaggtcggtggtgaccgtgccttcgagctggcggaccagcgcggcctgggtgtcgacgtcctgccgcgcgatggaatcctgccccagcagggtgcgatagcgcgccagcgtgacgcgcgcggcttcgagctgcgcctcgtcgcgctggcgggtgccgcgggcctgcatcagcgcctgctcgtagggccggggatcgatgcgcgcgagcagttggttcctggcaacggtctgcccttcggtgaacagcacctcggtcagcacgccgccgacctgcgccttgagcgtgatggttgccagcggcgtgaccgtgccgagcgcatcgatggtgaccggcagctcgacttcgcgcgccgccgcatggccgaccgtgacggtcgcgccgccgaagcccgggccgccggttgggctggccttgcggttgatgaggtaccaggcgccgcctcccagcgccagcagcaacagcagcgcgatcaggcttccgagccagagcctccggcgcgagggcggccgtggcggcggagacgaggaaggttgtgttgccggttgaacagcaggcgaatcgccggaagaaggctcggagttcggagattccatgtgatgtggcagtgcgcaagtacggctgctagtggagcgctgcatcgtagcgcgcctgtcttatgaaccgtaaagcgacggtaaagctgctgcgaacggcgcgtttcgcgcccggtggctgcgtctcgcgccgcggacctgcgtttcgtcgcagacccgtggcccggatgcgggcgcgccggcacagtccggcccatcgaatcacctcttgttggagaaacgccgtgctgctgcaaatcattcttcacaccccgaagtgggtcttcgccgttttcgtgctgctcctgtggctgggctgcaagcagttgatgtccggcagtgtcagcctggccaaggtcacgatggtgccggttgccatgaccggcctctcgctggccggcgtgatctcggcctttggccattcgcccggcgccctgctcggctgggcggtggtcgcgactgcgctggtgctggtggtgctgcagcagcccttgcccgccagcacgcgctacgaccgggccgcacgcgagtttcacgtggccgggagcgcggtgccgctggtgctgatgatgggcatcttcttcaccaagtacgtggtgggcgcggccctggccatgcaccccgaactgcgccagcaggccagcttcgccgtcgcggtgcccatgctgtacggcgccttcagcggcatcttcgcggcgcgggccgtgcgcctgtggaagctggccatccgcaccgacgccatggccgtggcagcccccgcggcctaagatcgccagccgattcatcgactgccctcgaaccattcgttatcggagaaccgtcatgaaccccacacaagcaaaccgttccacccccgacgtcgagaagctcgcccgacgccgcgccggcgccaagatgggctggtacatccatgccttcgtctatgtgctggtcaacctcgggctggtggcgctctcggcatcgcgcggccatagctgggcggtgtacccgctcatgggctggggcctgggcctcctgatacacggcgccgtgatctggttcgtggcgccaggcggcaatttctatgaccggctggtggaacgcgaacggcgcgcgctacgctccggggagcgcggatgagcggagcgcagggccgccccaagcccgctcgctcccgcttggcgggacggcgcgcagcgccaagggtgcaccaatgagtgttgaagcgctctctcgttttcgcgcggagaacgtccggagcatgcttcggcatgggctgatcaccgtcgtcttctgctgcttcattgccgcggcgctggccatcacgcagcacggggactggggctcgcaaatggtgtattcgctgtcgatcgggctgatcagctggctcttcatcgacgtgggccggctgctcatcagcggccacaaggaaatcctctggccgtccggcccctggggctatctgctggtggcggccggtgtgacggtcggcttcctggggggcaatgccattggcgatgcgtggacccatcagcccctgctcaatttccgcagcttcgcggagcgcaggctcgccaccacgatcatcatcacagtgacagccacggtctgcatgtgcttctttttctacagccttggcaggagcaagcacatgcggggccagatcgaactggcgcagcgcaatgccaccgaggcgcggctcaagctgctcgaaacccagcttgaaccgcacatgctgttcaatacgctggccaacctgcgcgccctgattgcaaccgacccgccgcgcgccattgccatgctcgaccggctcaacaactacctgcgcatgacgctcaacggctcgcgcgcgctggcgcatccgctttcggccgagttcgaacggctggccgactacctcgaactgatgtccgtgcgcatgggcgagcgcctgcgctacacgctcgatctgccggaagacttgcgcgacacgcccgtgccgccgctgctgcttcagccgctggtggaaaacagcatccgccacgggctcgagcccaaggtcgaaggcggcaatatcatcgtgcacgcccgccaggaggcgggccggctggtcatcgaagtgagcgacaccggggtcgccctcgctgcaaacccgtcgccgtcggaaggcggcggtttcgggctcgcgcaggtccgcgaacggctggccaccgtgtacggcgaccagggccgcatgagcctggcccccgagcccgcgggcggaacccgcaccaccatcagctttcccttgccggcacgcgcatgaaccccactgccctcatcgccgaagacgagcccctgctcgcccaggcccttaaggccgaactggccgccgcatggcccgaactgcaggtgctcgccatcacgggcgacggccggaccgccgtgcgcgaggccctgcgcctgctgccgcaggtgctgttcttcgacattcgcatgcccggcctcgacggcctgggcgctgccgccgaactggccgacagctggcccaccgacgaggcgcccatgccgcaactggtcttcgtgaccgcctacgacgaatacgccgcccgcgccttcgaaacccgggccatcgactacgtgctcaagccggtgcagcccgagcgcctgcgcaagaccgtgctgcggctgcaacaggccttgaccgcacagcagccatcgaaaccagccccgaacggagccgacgacgtgctggagcaaacccttgcgcagtggcgccaggtgcttgcggctgcgtccggcggtgcgcaggcacccggcactgccccgctccggatgattgcagccagcgaagccggcggcagcaccgtgcgcatggtcccgatcgacgaggtgctgtatttcgaggcggcggacaaatacattcgcgtgctcaccgccacgcacgaatacctgattcgcacgccgctgaagcagctgttgacccaactcgaccccgaggttttctggcaggtgcaccgcgcggtggtggtgcgcagctcggccatagaagcggtgcaccgcgacgaggcgggcaagctgcatctggacctgcgcggccggcccgagaaaattccggtcagccggctctacgggcacctgtttcgcgcaatgtgaaatttgcaggctcgaagcgcgcataaaaaagccggccctgagagaccggctttttcacatggcgggaatccctccccagctaccgcgcttagcgccagtggcgatggccgtggccatggccgtagtgatggcgcggaccgtaatagcggggcgcgtagtaggccggcggcgcgtagtacaccggggccggacggtagtagaccggcggcggcgggcggtagtacaccggaggcggcggcgcgtagtacaccggcgcgggggccgtatagaccggcgccggatagtaggccggagcgcccacaccgattgccacccctggcagacccacgccgacagaccagctcacgtcgccacgggcactggccgaagtggccgcaaacaatgcaccggctgccacgacacccgcggcggcccatttgaaaaaggttgaacgtgtgaggctcatgatcttggactcctagttggggcgtttcctgcccatgtatgtattgaacgcgccaaatgcaaagcggttgcccgccgcaatgtgaagaacgttgccaaaggtaaccggcagggggtgcactctagaatgccgcaatgacctccccgaccgacaaagacagcgcgaaaacgaccgctgcaccgagtaatttcctgcgtcacgtgatcgaaaacgaccttgcgcagggggcctattctggccgcaaatggggtggctcgcccggcgacgccgcccatcacgcccagggcatggccgaccccgccaaggtgcgcatgcgctttccgcccgagcccaacggctacctgcacatcggccatgccaagagcatctggctcaatttcgagctggccagggaatacggcggcgtgtgccacctgcgcttcgacgacacaaacccggagaaggaagagcaggaatacgtcgattcgatccgcgacgccgtccaatggctcggctacgaaacctacctggccgaccgccccagcgcgccaggcaccctgcagccgcacgaatactttgcgagcgactacttcgacttcatgtatcgcgcggcggaatacctgattggcgccggccttgcctacgtggacgaacagacggccgaagaagttcgcgcgaaccgcggcgacttcaacacgcccggcaccgacagccccttccgcacccgcacgcccgacgaaaaccttgcgcgcttccgcgccatgcagggtggccaggtggccgacggcgccgccatcctgcgcgccaagatcgacatggccagcaccaacatcaacatgcgcgaccccgcgctgtaccgcgtgcgccgggccactcaccacaacaccggcgacaagtggtgcatctacccgatgtacacctttgcgcaccccatcgaagacgcgctggagcagatcacccattccatctgcacgctggagttcgaagaccagcgccccttctacgactggctgctcgaccgtttggccgaaggcggcctcattgccagcccgcatccgcgccagtatgaatttgcgcgcctcaacgtcacccacgtgctcaccagcaagcgcaagctgcgccagctggtcgaagaaaagcacgtcgacggctgggacgacccccgcatgcccaccctggcgggcctgcgccgccgcggctacacgcccgaggcgctgcgcctgttctgcgaacgcagcggcaccaccaagtccggcggctggatcgactacgcaagcctggaggccgcgctgcgcgacaccttggaccccacggcaccgcgcgccatggccgtgctcgacccggtcaaactggtgatcaccaactggggcgagctgatgggcggccccaacaaggatgaaagcgtgctcgacgactgctcggcccccgtgcacccgcaccaccccgagatgggcaagcgcgagttcaagctcggccgcgaggtgtggatcgaacgcaccgactacgaagaagtgcagcccaagggcttcttccgcctgttcccgggcaacaaggtgcggctgaaatacggccacgtcatcgaatgcaccggcggtaccaaggacgcgaacggcaagctcgtcgaagtgcaggccacgctggtgcccgacaccaagagcggcacgcccggcgcggacgccatcaaggtgaagggcaacatcacctgggtggccgcggcggatgcggtgcaggccgaagtgcgcctgtatgagcggctgtttgcggcggcgaatccgggcagcggagagttgatggatgagctgaacaagcagagcctggaggtttgcactgcgtacgccgagccctcactggccaaggctcaggatggcgcggcgtttcagttcgagcggcatgggtacttcgtgctcgacgcgaaggctggtgcaggcggcaagcgggtgttcaatcgcgccgcgggcatgcgggacagctggggcaagtaatcccgtcccgcctgatccgcttcaacaagccctacggcgtgctcagccagttcacgcccgagggccgctggcgcgggctgaaagacttcatcgacattcctgacgtctacgtcgccggccgcctcgatgccgacagcgagggcctgctgctgctcaccaacgacggccagcttcaggcgcgcatcgccgatccgcgcttcaagatggagaagacctattgggtgcaggtggaaggcgtgcccactgaagaggcgcttgccgcgttgcgccaaggcgtgcagctcaacgacggcctcacgcgcccggcccgtgcgcgcctgctcgatcctccgcccgatgtgtgggcgcgacaaccacccatccgcgaacgcaagaacattccgaccgcatggctggaactggcgatcagcgaaggccgcaaccgccaggtgcggcgcatgaccgccgccgtggggcttcccaccctgcgcctgattcgcgctgccatcgggccgcacacgctggacggattggcgcccggtacctggctggagtaacgcagcagcgccgccgcacaccttcattcattcgcccttatgcgcagcaaaacccatcttcccgatctcccctcgcccgctctgaatcgccgccgcgcattgctcggcacgctgagcctgctggcgctgcctgctgcaacgcacgtcagtgccgcgccccctgcgaagccgaagcaacagcgccccgacgtctggccgcacgcgtcccaggtgccgggcggcgtagcacgcctgtcgctgggtcccagcgccaaacgaccggccgccttttcaggcgacgtgccattgctcgtgctgggtgacgccatcgagtggacagcgctcgtgggcattccgctcgccgccactccgggcgacgcaagcatcgttgtgcgctccgagagcggcgccgaaaaacaggtcgcctacaccgtggcccccaagcagtaccgcgagcaacgcctcacggtgccaccgcgcacggtcgatctgtcgcccgaagacgaagcacgctatgagcgagaacgcgcgcacctggccaccgtcatggcaacgttcaccgatctgccgcccgatgcctcgctgcagatgcgcgtccccgtgccgggccgccgctccagctcgttcggcctacgccgcgtgttcaacggccaatcgcgcaatccgcacagcggcatggacatcgccgccggtaccggcacgccggtgctggcgccgttgccggggcgggtgatcgatacgggcgactatttcttcaacggcggcacggtgtggctcgaccacggcggcggcctgctgacgatgtattgccacctgagccgcgtcgatgtgaaggtgggcgatgtgctgaagaccggcgagcggttggctgctgtgggcgccaccggccgcgtgacggggccgcatctgcattggtctgtgatgctcaatcgggcgatggtggatccggcgttgttcattgcgacatgattcaaatgggcggcggcactacactccgcagcatgcgtccctctgaagccctgtcacagcatcgcgagcgcattcgcgagattgcactgagtcaccacgtcagcggcgtgagggtgttcggctccgtcttgcgtggagaagacgggcctgacagcgatcttgatctgctggtcgagcccacggaacaaaccacactcctggacctcggagccatcaggtacgaactgaaaagccttctcggcatggaagtcgacgtgctcacgcccaacggattgcctccgaagttccgcgatcaggtgctgcgcgaggctgtgccgatatgagccgaggcgatccgcaacgtcttgcggattatctggggcatatcctggaagccattgacagcattcgcgactacacgagccaagccacgcgcgaaagctatctggcagaccgaaaaacgcaagacgccgtggtgcgcaacctggaagtgatcggcgaggccagcaacaatgtcgtgaagcatcatgcagaatttgcggcggcccattccgatgtcccctggcgctttgcctacgaaatgcgcaacgcgctttctcacggctatttcactgtcgatcacgcgatcgtctggcaaaccattcagcacgatctgccgccgcttcgcgagcaaatatcgaagctgaaggagccctgagcttcatcgctgcctcaaagcggcttcgtcaagtaaaccgcctcccgcccaacgatcacccgctgcgcgggcatgaagatcgtgcagtcgtcgcacggcgcgcggatctcgtccgggccgttggtggcgatgagttcgcccttggcaaaggtctcgaagccgatcagcgggcgcacgaacgcaaagtcttccgacttgatgacgtgcgtctgcagcagttcgaagcggcgctgtgggccgggcgccggcactgcggggtccttgtcgatgaggccgaagtgcgccagaaaatcgagcgagatggcggtggccagttcggaggccgagcgcagaaagtgctggccgcattcagccaccagcgccacgcccttgccttctgaaaggccgtggcgaccgtgctggatcagcggtgtgccggagccgaggccttcgggcatcaccagatgcaccgaggggcggccgatggccattgcggcctcggcattgcggtcgaatgcggggtacacccagaacggaatcaccggctggctggtggagtgaatgtccaggatgtggtcggccgcgctcaccaccggacggagcacgcgcgcgcggcgcagttcggggctgtcctcggtgccgtcgagccattcgggcgaccagatgcggttgaggttgtgcaccagttgccggctgtcgaagggcagcgccttgtcgaaggactcgtacgcttccacgttggcaaagctcacggtgagcgtgccgatcttggggcgcacgttggtgtcgagcagatgcgtggcggcggtcatgccgcagatttcgttgccgtgcgtgagtgcgttgatcagcacgtgcgggccgggcttgccggactcgaagcgatgcacgtagtcgatgccgatgttgcccttgcggtaggcggagaggtcgcgggggaggacttcgagggcggggggcgtttgggtcattggcgttggcgttggcgttggcgttggcgttggcgttggcgaaattgaagcggactggtcgggcgagtttgctacaggctgcgctttcgtgcttcttgtgctgctcgcagctacctcgagcggatgagcgcgtaccgagttgccttgccttgccccgttttttcgagcaagccggatgccaccatctcggtcagttcccgatatgcggtggcgcgcgacacgcccgcaatggccacatatttctccgtgctcatgccgcccaggaatccatcgggaccggcgtcatagagcttgttcaacactttgcgctggctcggcgtaagttgcggatgcgcggtgtccagttgggcccagaacccggccttggcgcctgcggcctggatctgcgccagcgtcgagaggcacgccttttcgatacagccgatgaaccagcgcacccagggtgtgacatccatatgcccctgcgcgctggcagcctgcagctggttgtagtacccggcgcggtcgagccacagctgctgcgagaggctgaacagtcgctggttgctgcgcaggtcctgcgccagcgccaagtcgctcagcgcccggccgatgcggccgttgccgtcttcgaacgggtgaatggcttcgaaccataggtgtgcgatggcgctgcgcacgatgccatcaatcttcgggtgctgccgcccttcttcgaaccattcgagcaacgccttcatctgcgctggcacatcacgggaaggaggtgcttcatagtgcaccgtgtcgggcttgccaatgcgcggcgtgacgatctgcatggggtcttcgtggacacggtagccaccagtgacgatgcgcgtgatgccgcttcgcccgtttggaaaaagcgcggcatgccaatcgaggagcctgccttctgccagtggttcattccagcgcgcgatggccgcttcaacgatgtcgagcgtggcttccgtgcgtgcatcctttggcacgcgatcggcgggcgtgagccccagccgccgggccgccgaggcccgtaccgaattgacctgcagcgtttcaccctcgatctgcgctgtagcgatggcttcctgcgtccactcgccgagttggagttcgctcagatcgatgagttgaaggttgccggctacgcccagcatgcgcccctgtgccaggcgcgcagccgacagcgcgggctgcagcgcctgcgcgtcgacctcgaagtgcggccattctttagcttgccagatccacatgaagcgcattttaggcaaatacgcttcaaaaatgaagcgcatcacggacaaatgcgcttcagcgtcgcgctgggccctaccagttggcctcacgctccggcgtcgccgaaatatggtggatcgacaggtcggccccgtcgtattcctcttcctgcgtgagccgcagccccatcgtggccttgagtgcgccgtacaccgccgcccctgccagcgcagcccaggccacaccgatcaaggtgccgatgagctgcgcccacaggctcacgccgccgatgccgcccagcgcctgcgtgccgaagatgccggccgcgatgccgccccaggtgccgcacaggccgtgcagcggccacacgccgagcacgtcgtcgatcttccacttgttctgcgtgagcgtgaacatcaccacgaagatggcgccggccacgccgcccaccaccagcgcgcccagcgggtgcatcaggtcggagccggcgcacaccgccacgaggccggcgagcggtccgttgtagacgaagccggggtcgttcttgccgagcgccagggccaccagggtgccgcccaccatggccatgagcgaattgacggccacgaggcccgagatcttgtcgatgctctgcgcgctcatcacgttgaagccgaaccagcccacgcaaagcacccaggcgcccagcgccagaaagggaatgttcgacggcggatgcgcgctcagcgagccgtcgccgcggtagcggttgcggcgcgcgcccagcagcagcacggccagcagcgcgagccagccgcccaccgcatgcaccaccaccgaacccgcgaagtcgtgaaactcgctgcccgtggccgaggcgatccacgcctggatgccgaaagccttgttccaggcgatgccctcgtacagcgggtaaacgaagccgacgatgaccgccgtggcgatcagttgcggccagaacttggcgcgctccgcgatgccgcccgagatgatggccggaatggccgcggcaaaggtcaagaggaagaagaacttcaccagctcgtagccgctcttggcggcgagctcggtggcgcccacgaagaagtgggtgccgtacgccacgccgtagccgaccaggaagtacacgatggtcgagaccgagaagtcgaccaatatcttgaccagcgcattgacctggttcttcttgcgaaccgtgcccagttcgagaaaggcgaaaccggcgtgcatggccaacaccatgatggcgccgagaaggatgaacagcgcgtcagcgccctgtttgagtgcgtccatgggagcttcttgcagttttctggtttgaattggtgcgtgcacccgaattgctcggagcagcgccgcaagaaagcaaaaatggtgcctataggctcttcgatggtgcgaaatgagccataaaggggctttacgattcaggctcgcaccggaacaggacactcacgggcctgccccggccactcaagtcgcccctgcgcgcagggcttcgcggtagcggcggctgcacggcaccgtggtgccatcggccatgtgcagccgggcatcgccaccgtcgagtggctcgatctccttgatgcggcccaggttgaccgcgtggctgcggtgcactcgcacgaaatgggcagggtcgagctgggtcagaaaatcggtgagcgtggcgcgcagcaggtagtcgtggccattgacgtgcaggccgacgtagttgccctcggcctggagccagtcgatgtcgcccgcggcaatgagaaattcgcgccgcagcttgcgcaccagaaagcgctccggccgggcgggcggcaccgcgggttccacaagagcgggttgggcgggctcgggcggatcgagcacgcgcgcctcgccttgcagccgcagcatgaagacaccgtagacccagatgccgaacaccattgacaggtaggcgcgcacgtccttcaggtattcgtagccccagcgtccggtccagcccgcaaagtcgtagcgctcgcccatggccgaatagaccatggcacgcagcgcgaacatcgcggccacgtgcaccaggctgaagacgacgctggcggccgcgtgccacgccaggtagcgcagcagattcgtgcgcgccagcggcgacagccggcgctggacggcgaccacggcaggcaccagtgccagcagcaccaagtggctcgacacctcccaggtcacgatttcccaggtggcgcgcggcactgcgcgatcacgcgcatcgaccagcgccaccatggtgttgaacaccgcctgcagccccatgaagacgacccagaagcccacttccacccagcggcggatgggttcatagcgctcgtacaggttcttttttcgggaatctcccatgcccgggattctcgcgatccacgcgttcggcgggaaaatttcgtcccccggagcccaccgctcgtcacaaaagggccgcgatccgtccctcaggcagaccgcgcgcggcgcaagaacgcaaccatcggcccctccttcccacgcgttttcgaggagcgtccgatgagcgcaacccctgacacccggtccgcagcacccgaccgccgccacgacatcgacgcgctgcgcgcgctggccttcctgctggtcatcctctaccacgtggcgatgtactacgtggccgactggccctggcacctcaagagcccgcatgcggccgaatggctgcagtggccgatgcgcgtgctcaacctctggcgcatggacttggtgttcctggtctcgggcgtgtcgctgggcttcctgagccgccaccagggcagctggggcctgctgcgcagccgtggcgtgcggctgatgctgccgctggttttcggcatggcggtgatcgtgccctaccaggcctatgcagagggcgtggccaacggcctggtggcgccgggcttcggcgcgtttttgctgcgctatctgtcgatgggcgatccgtggcccaagcaggcttttgccggcgcggagttcggcatcacctggaaccacctctggtacctgccctatctgttcacttacacggccatcgtcgcgctgacgctgccgctgtggaaatcgcccgccggccagtggatgcgctgccgcttcaacgggctgcgcggctggaagctgctgttgctgccggcgcttccgctgctggtctggacgatgctgctggcccggcactttccgcccacgcacaacctgatccgcgactttcacctgcacagcatctacttcacggtgtttctgtacggctactggatgggcgtggacacgggcgtgtggcgcgaactggaacgcctgcggcgggtttcgctggcgctggctgcggcggtgatcgccactttcatcttgctccggctcggcgccaaggggccaccttccggcgtgctgatggacaccttgcgcatgctctacctgtggctggcggtggccaccatcctgggccatggccaccgctacctgaaccggccgtggccctggctgcgctgggccaacgagtcggtgtacccgtggtacgtgctgcaccagacgctggtcattgccggcgttgcgctgctggcaccctttgcattgggcccggtgctggagccggccttgctggtggcgttgaccatcgccggctgctgggcgctcaccgacgggctgatccggcgcgtcaattggatgcggcctctattcggactcaagcctcggcgcgcgagcacccctccgcgggctacttcgccggaggggcctcttccaccggaaccaggattgcgctccccgtcgccacgagcctgaggccgtcgccctcgccctggccatagagctcggcggtcgcaaacacctgcttgcgcccggccttcaccaccttgccgcgtgcaatgaaggcgcggcccagcgcgggcgacaaacagttgaccgagaagtgcgaagccagcacccgccccgccaccgtggcggccgcaaagccgcaggccgtgtcgagcatcgccccgatgagccccgcgtgaaggaaaccggcgtactggcccatatcttcctcgcgccacgccatgcgcagttcggcttcgccgtcagcggcgcgggtcacttcgaagccggcccagcgattgaaggcggcagtcttgttgatggcctgaatggtgtcgagcatggcggtctttcacgaagaaggatgaagcgtcgaaaaagccactctacgaagcggccccgctgcacgccgtcgcgcccgcgacgcgcaacgcccggccagttgccttggcgacagcgcactttttttgcggaggcttaaccccggtcggcgaggcccgccgtatgagtggaggaacgatccactaccgaggctccgatgaaagctatctcttcctcttctttctcttttcgtgccaatttgcgcgccaccgccgttgctgcggcctggctggtgctcggcatcggtgcccatgcacaggccacggccctcgccaccggcgcggatgcatcccgcatcacccaggtcaaggtctatcccggcagcgcgacggtggagcgcgtggcgcgcgtcgcggccggcagccgatccgtcactttcgcctgcctgcccgcggcgctcgacgtgcagagcctgcaggtttcggccggggcgtctgtgcgcgtgggcgagacctcggtgctcagcgagccgcgcgaactctcggcacgctgcgcgaccagcgcgctcgacggccgcatccgcgaactcgaagaccagaaggcagcgctccaggccgagaacgatgcgctcggcatggtgacgggctatctcaagggcctctcgggcggcggcggcgaatcggcccagggcgcacgcgcgccgttggacgcgcgcaacctcgccgcaatgaccgaggccatgcgccgcaccggtcaggactcgctgctgaagcagcaccagatccagcgcaggcaggccgacatcgaccgccagctcaacccgctggtggccgagcgaaagcgctcgcaaggcaacggcgcccaggtgatggccgtgaccgtcacgctggccgccagcgccgatgccgaggtgaagctcagctaccaggtcaacggccccggctggacacccacgtatcgcgcgctgctcgacaccgccacgcgaaaggtgcgcatcgaacgccaggccctggtggcacaggccacgggcgaagactggcgcggcgtgaaactggtgctctccaccgggcagccgcgccgcgaaaccgcgggccgcacgcccaacgcatggcgcatcggcatcgaaccgccgcagcgtgcgccggcaagcccggccccggccgccatgatggcggcgccggcgcccatggcgtccgccgacaagcgtgcaatggccgaggctgcagagccgctcttcgacgtgaatgtgttcgacaacagctttgccaccgaattcgcggtgccccaaggtatcgacgtaccctccaacggccagcgcgtgacgcttgcgctgggccagcacgaagacacggcgaagcttgccgcacgcaccagcccgcgcgtggacgcgagcgctttcctggttgccgaactggcccagccggcgggcgtgtggccggccggtgcgctgcagctctaccgcgacggcaacttcgtgggcagcggccgctggaacgcgcccagcgattcgaagctgacgctctcctttggccgcgacgagctggtgcgcgtgcagcccgagcccgagcaggacagccagggcacgggcggcttcgtcggctcgcgcgccgagcgcaaggtgcagcgcgcctacgtggtcgagaaccgccaccgcacgccgattgcggtgcaggtgctggaggccgccccggtgtcggtcgacgagcaggtgcgcgtggctgcgcagttctcgccccagcccggcgaactggcctggaacaagcagcctggcctcgcgatgtggagcttcgacctcgacgcgggcaagactgctcgggtggcggccgactacaccatcagctatccgaaggacgcacggctgcagattcgctgagcgctgagcgcgcgcagttcagtgcggctcgggcgtctggccttcggcgggctcggcgcccggtttgcgcttcttgccgcgcgcggccttctttgcctgccgctcggcgtcgatgcgctgcccttccgcgagccactgcccaaactcctcgggtgtctcgagcgtgatgcgcccgaggttgccggcacgaaactcgtgcatcacgatctcggccgccttctgcaggttgacgcgccccttgcctagcagcgcgccgcgcttgcggccgatggtgtcgagcacgtcctcgtccttcatcccggcgatggttgctgcatcgagctcgaccagcttgaatcgctccgcgatgcccgccgcatagtgcgtcttgaggtagttgagcagttcgagcgccacttcctcttcgtcgaaggcattgcgccccaccgctccgctggccgcaaggttgtagccgctcttgggcaccacgatgcgcggccacagcatgccgggcgtgtcccataggtagaagtcgtcggccagcgtgatgcgctgctccagcttggtgatgccggcttcgtcgccggtcttggccttgcggctgccggtcagggtgttgatgagcgtcgacttgccgacgttgggaataccgcagatcagcacgcgcatcggcttggccatgccgccgcgattgggcgagagctcatggcaggcgcgcacgatggcctgtgcgggcgtggtcaggctcgcgtcgagcgggatggcgcgcgtggccggcagcgcgttgtagtgcgcgagccagagcgcggtgcgcccggggtcggccagatcctgcttgttgagcaccttgagcgagggccgccccgccgtgagttcggccagcatcgggttggcgctggagcccggcagccgcgcatcgagcagctcgatgaccacgtcgatgtccttcacccgctcggtgatggccttctgggtcgtgtacatgtgcccggggaaccactggatcgccatcgatggatgctctttctttcgctttgtctgggaatcggcccgaagggcggatgggcattgtggacccggaatgtgcgttaggtcacaccgctatgctttcgatagcctcgagtgccgattctgcctgcgtccggggtgcctcggcctctagaatccgcgcgctgcgccgcagccatcttcaataaataagtaccgagggaaatccatgttcaagcgccttgccgctgccgccctgctggcagccaccgtccttcccgcgaccgtcgtccatgcgcagcgcccctcgccgccgcagggcccgatgctcagcggctacctgtgctgcaacatgcggacctacggcagctcgatcagcgacatcaactacgacgagcaaggcacgagcatcgtggcggtgggcacgccggcgcgcatcacggcctacgacttccgctggttcgaggccgatctcgcgggcaagccccagcgcatcaagaacgactacagccgcaacatcacgctcgccgacttcgcgaagcgctacgtggtgaccgaagatccgaagcagaagatggccgctttcccgcccgccgtccgcgacgccatcgtcgccggaaaggtggcgcccggcatgacgcgcgaacaggtgctgatggccatcggctatccggtggccggcgagaaccccagcatcgacgcacccacctggcgctactggcgcgacagctggtcggagtaccaggtgaatttcgacgacaagggcctggtcaagaccgtcgcgggcaaccccgtggcgctcagccgcgtgctggcgccaacaccttagttcgctcgctggcgcgcggcgcgacgcgacgcgcgcaatcccctagaggtttttgcattgctgggagcggttccaccgatatcgcccctatcatttgaccgagtgcggcgcatggacgcgtcggtcgaagctaaacttttttgatggagttaccgcgatgaaacccgtctccgaactgctcaagcgccacgattccgcggcttggcgcacctcgccggacaccagcgtgttcgatgcgctggccaccctggcacgcttcgaggtgggcgcgctgatggtgatggacggcgaccggctggtaggctttctttccgagcgtgactacacccgcaaggtggcgctgcagggcaagaattccaaggagatgaaggtttccgagatcatgacgcccgacgtgatgaccgtgactccgcagacccacacgcgagactgcatgtcgctcatgagccagcgcaagttccgccacctgcccgtggtcgacggcgacaaggtggtgggcatgatctccatccaggacctgatggacgacatcatcagcgagcacgagcagacgatcgaccagctcaccagctacatccggagctgaaaagccgggtcccggaccctgcccggcccgggggtggggaacacgcctacgcgcagggtcaccgtttagggcgcacagtaggggctcgttcatccatcagcagggacatggcatgcagattcaggtcaacacgagcaacggcatcaacaacaaggacgccctggagcgctgggccgacaccgagatcaagcagcaactgggccgtttcgtcgaagacgtgacacgcgtcgaggtgcatctgagcgacgagaaccacgacaaggccggcggcggcgacaaatgctgcgtgatggaagcccgccttgcccaccatcaaccgcttgcggtcacgcagcacgccaccagcctggacgaggccttccgcggcgcggccgacaagctcaagcgcctgctcgacaacacgctgggccgtctcagcaaccaccgcgaccgcgaatcgatccgcagggacgcgggctttatcgcggagtagccagaaaatccagcagcaggcggctcacttcggcgggctgctcctgctgcacccagtgccccgccccctcgatccagtgcacgccgcgtagctgcgtgcaggccgttgcctgcatggcttcgaagtcgccgggcttctggaacacgccccaatcgccgcagcccgcaatgaaacatgcgggcacgtcgatcgtgcgccccgaccaagcctgcatttccggaatgtagcgcccacccgtgccgcagcgataccactgcaacccgccctggaagccggtgcgcgcgtattcggcggtgtacacggccagatcctcttcgggcagccatcggcaggcggcgatctgttcggccgagggcatttcgtcggccaccgtctcggccatggtctggtcggcccgcatcacgtagtaggtgggcaggcgcgccagttcggcggcgctcattgcggccagcgcgaagggccggttctgcggccagtcggcactcttctggtggtaatagccgcgcaggaaggcatgcagcccttgcggtgcctgccgcatgtcggcatcggcctcggaccccgagtagtaccactggtagtgtttgcgtggcggatgcaatgcggcgaggccatcgagcaggtgccggatgacctgcgcgaacacgggtgccgccccagcgctcggcgggccgggaaacggcgcgctcatcaatgcgaccgagcggaacacgtccggacgggtcagcgcgcaccaggccgccaccggcgagccgaagtcgtggcccaccaccgccgccgtctggtggcccagcgcggacacgagccccgccgcatcccgtaccaggttgagaaggcgaaactcttccagcccggcgtcgtagccctgctgccagcccgtggtccggccatagccgcgctgatcgggtgcgaccacgtgaaagcccgcctcggccagcggcaacatcaccttgcgccagctgtaggccagctccggaaaaccgtgcagcaacagcacgcaaggacgccccggcgcatcgaagccggcttccagcacgtgcatggacaggccattgccgttgtcgacctggcgcgagcggatgcccgcgggcagcgggatgggggcaagttcggcgatggtcatggggatttccgtggttttgacggtttcggcgcgagcgcccggaggcggggtgtttcggcgggaatcagcggcggccggtggccggtgtgcatccactcgtcgtagaagtcgatcttgcgatcgaccagcgacagggcgcgtttccagtcggcaatggtttcggccacgcgcgcacggtgcgctgcgagcatgccgcggcgctgatgcagcgtggccttgccctgcaacgcgagcgcggtgtactcccgcatctcggcaatggacatgccggtgcggcgcagccggtcgatcaggtccagccagccgacgtgcagctccccgtagaggcgccggccgccctcgtcgcgcgagacgccgggcacgagaccctgcgcctcgtaccagcgaatggcgtgcacggtgcggccggtgcgcgtcgcaagctcgccgatgtgaaaaggggtgccgcggtcagccggcatgggcatggagagcagcggcgggcggcgcctcgagcgcctcctggaccagtgcggtgtcgaaatactcggtcagctctttcaccttgcctccttcgagtcgatagatgtagcaatagcggttgttgtagcgcttgccggccttggtgggcacgtcgccgctgaacagcaccaccacccggtcgccctcggcaatgatgccctcggtcttgctcacgtagcggcccgcgaactgcgcgaacagcggtttgatcagctcttcgcggatggccgccttgcccgcgtaggtgcgcgaccacggcgtggtgccttccagcgtccagcgggcatcgtcggccaggctgtcgatgaagagctggccgttgcccttgtccagctcggcatggatgcgctgcaccagcgccttgttgtctgtagtggtcgtgttcatggctgcttgtcctcgtggaatgaatgaaccggaagctccggtcgattcattggaaatgctcgagtgcacttcaggtcaagcgccatgaacgggggtgcgcgtcagcccttgcgcgcgtttgcggccatggccttgccgacctcgttgctgccttgcgcggtgccgctctgcggcacgatctcgccctcgcgcgaagtcacctcggcgagccgcgcagccagttgttccggtgtgtccacaccgatgccgagccaggcgccctgcgtcagggtgatgtgcgccgcctcgaaggtgccggcgcccgcgcaaaggatggtgcggttcggcgcgtccgcggaggccagcaccagcatggcgggcaccacggcctccggcttgagcgcatcgagaacctccggcggcatcaggccctcggtcatgcgggtggcggccgtcggggccaggcaattgacgcggatgtcattctttgcaccctcgatgctcagcgtctgcatcaggcccaccagcgcgagcttggcggcgccgtagttgctctggccgaagttgccgtagaggcccgacgacgaggtggtcatgacgatgcggccgtatttctgctcgttcatgagcgcccagacggccttggtgcagttcacggcgcccatcaggtgcacgtcgaccaccagcctgaaatcggcaagctccatcttggagaagctcttgtcgcgcaggatgccggcgttgttcaccagaatgtcgacccggccccaggcctcgacagcctgctgcaccatggcctgcaccgcgtcgaagtcggtcaccgaggctccgttggccatggcctccccgcccgcggccttgatctcgtcgacgacggcctgtgccgcgctcaccgaggcgccggagccgtcgccgggaccgcccaggtcgttcaccaccaccttggcgccgcgcgctgccagggccagtgcatgctggcggccgaggccgccgcccgccccggtcacgatggccactcggcccttgaaatcgatgatgctgttgctcatgtgtcgctctcgctgctttgctggggaatggggatgtgcgggccatggcggccgcgaggcgttttacctcagaaaagcaggccgaccctgccggccggccgccagctcagtcgcgcgcgtgacgcagggtttcgcaataggcgaccagctggtcgagttcggccgacttgtcgaagaaggcatcggcgcccagttgctcggaacgttggcgcatgtcggccgtggcgtagttgctcagcaccaccactttctgcttcgccttgcggttgcggcaggccttgattacgccaaggccgttgccgcgctccaggaacaggtcgacgatggtcaggtcccagtcgtcgcgatgctggcgcagccagcgcactgcctcttcctcgctgctggcgcaggccaccacgtcggcgtcggccacgtcgtgaaggaaaccgacgaggttttcacggatgagggcactgtcctcgacaagataggccttgaaagtcataccgggatttccggccaaaccgcgggccggaacaaaaaactggagcttgcgggatgcatgctcccatggtcgccaccgtggcggcgcccgcagtgggtcatgccggccaatgcctgtaggccatcggcccccgccgctgtcgtcaggcgggctgtgtgacggtgagacgcgtaggacagggacggttcaggccgcgacggccatccggccgcggccgagccccaggcgtgccggcgacacgtattgctcgcggtagatctcgaacggcatggtgtccgcggcctcgatgcgcttctgctcctggatcgattcctcggtcatgtgctcgaacgcggcctgctgctcggccgagaacggcagcgccagcagcgtggcgcgcgtctgctcggactgggcccgcacgaagccgatgaaggagttgccgtgccgctcctcgacggcagccagcacgcgcgccgagggcaggctgtccgggttctgcagggcggaaagcgctgcgcgcaccgcgtcggcatgctgcgtgccgccattggcagcgtcaagcgccgcggcgatgggcaggcattgctcgaccagctccacgccccagtcggtcagcgaaacgttgcgcccgccgcgcagcagctgcaggcccggctcgcgtccgcgtgcggcggtgaggtgctggttgtgggccagttcggcaatttcctggggcgtgtcggccgggctgtcgctcagaaggcactgcagcaggaacacgtcgaggaagcgcatcgtctgcgcgttgatgcccaccggctcgaaggggtcgaggtccatcagccgcacctcgacgtactcgacaccgcgctcgcgcagcgcatgcagcggacgctcgccggggttgatcacgcgcttgggccggatggtgccgtagaactcgttctcgatctgcagcaggctggtgcccagctggttgtagtcgccgccgaggttctggatgccgatggcctcgtaggcaggccaaggccgcgtgagcgcgtcctgcagcgaggcggcgtagccttcgaggctgttgtagctcacggccagcgaggcttgcgcgtcgctctggtagccgagccggcccatgcgcagcgaggtgccgtgcggcatgtacatgctgccgtcgcccagcgcctggagctcgtgcggacggcccgcgacaaagctcgaacacagcgccggcgaagcgccgaacaggtacagcagcaggaaggcatgccggcggaagttgcggatgagcgcgaaatattgttcgctcgacacgccgggcagcgaccagttgtagtgaatgcccgagatggtctgcatgcgccgcccgtagcggtggctcaggcccatgcggtagacgctcttggcgcgcccgacgttcgacgagccgtagcgcccgatcggaatggtttcgtcggtcggcaggccgcagggcatgctcgacacccagagccgctcgtcgccgagcgaatcgagcacgcggtaggtgaactggtgcacgcgggtcagttcctcgagcgccgactcgacacccgcatgcacgcccgtgatgagctccagctgcgactcgctgaagtcggtggtgatgtgcggatgggtcagcgcggacccgagggcgatcgggtggggcgtgagcgcaagcttgccgtccgggagcgcgcgcaggctttccttctcgatgccgcgccgcattcccttcaaccgcgtggtcgagagtgcacccaacctctcttgcaatctgctgctcatattgttatgacccgtcattctctgaggggctggaaggtagcacggccgcgcgggcattgctggtgcagggaatcccgactttcgctatgctccgcggcgctacggttttgatagcagcattcatgggctcatggaatttcggcaccggcctggattcgatccgcgaacctcagtcgcgcccttctccaagatcgatctcgttgcactcgtagacgaagatctgcggcatgccatcggccatggcggccagtgccttcgcgaacgcgcgcgaggcctcgacgccgaaatgcgccttcagcgccgccatgtcgctccaccgctccacgaaggtgagccgcagcggctgctgcacgttggtggtgacctcgtgcgagatgcagccgggttcggtgcgcgaacgcagcacatgctccacgctgatggccagcatcgcgtgcagggtttctgccttggccatggcgtgtccgatgacgaggatcatggtgtcgtctcctgctttgtggcgtatgcgtgaaggtgccgaaaaaagcgtcaggaagccagaacgcgcagaagaaaccggttcaggtcggcaatttcctccatgcagaccgaatgcgccatcgtgtactcgtgccactcgacgggatgaccgagcgcgatgagcgcgtcgcgcgactgcagcgccctttggagcggcaccaccgggtcttgccggccgtgggccagaaagaccggtgtctcgtggttggccgcgtgccgctcggctgcggtggtggccgcaatgggcagatagcccgagagcccgacgatgcccgccagccgctcggtgtggcgcaggccggtcatcagcgccatggcgcagccttgcgaaaaccccgccaccacgatgcggccggccgcgatgccgcgggccttctcgttggcgatgagcgtctcgatggtggcctgcgaacggcgcaggcccgcctcatcctcgcgcgcggccaggtcggccacggcaatgtcgtaccaggcgggcatctggtagccgccgttgatggtgacggggatgaccggggcattggggaacacgaagcgcaccgggcccacgctcgacaggtcgagttcgttggcaatcggcacgaagtcgtttccatcggcgcccaggccgtgcatcacgatcaccgtggcggtgggatggggagcggtttcgatttcgatcggggagcgggacatggttcggaagaaggtattcagaaacgcgaaaaaccagaccttagcgcattcgggccggccggggcgcggtctcacggaatgcaacacaatggcggtaccgcgaagaacccatgagcctgcacccgaagccccctcccgccgccaaggcgcccgacagcgaaaccctgctgcgccagaggggcctgcgcgtgacgcgcgccgcgcaaacagtgctggaactgctcgcgcgcgcctcgcagccgctcacgcacgacgacgtggttgccgcctacaccgccgccaccggcgaggcgcccgaccgcgtgaccatctaccgcgtgctcgaccgcctggtcgaagcgggcctgtgcgaccgccgcgtgggcgcggaccgcgtcaaccgcttttcgcgccacgtggaagccgcttcgggcaacatcttcgaatgcgaccagtgccacaaggtgctggccctgccctccgaccccgagctgcccaaggtgatgagccgcctgggccgggaactgcgcaagcaaggcatcgacacccgccacaccgcgctcacgctgcacggcacctgcggggaatgcaggggctgaagcccaggagctacgcgttccaggacggaaaaggatcggggaagttcgtccaccacgaagcgccggagcgcatttcgctctctgtcagcaggcaggcgtcgagccgcgcacgcaggccgggctcgtccatgccgatgccgatcagcaccagttcctgccgtgcatcgccggtgcccgggtcccagttcttgcgaatggcgtcgagcgcttcctcgtcggaaggccagtgctcgcgcggcactgcggcccaccacaggccggcgactccgtggcggcaagcacctccggcctgcgaccatgagcctgcccgcgtggcgcggctcgcgagccagaagaatcccttggaacgcaccacgccttcccattcgctttgcaccaggtcccagaagcgctggggatggaacggcagccgtgcgcggtagacgaagctgccgatgccgtaggtctcgctctcgggcgcatgctcgccgcgcagttccgccagccatccgggcgcgcgttcggcctgctcgaagtcgaacaggcccgtgtcgagcacgcggtcgagcgcgacacggccgaactccgaggcctcgatgcgtgcacgcgggttgaggctgcgcaggatggccatcaggcgctcgcgctcttcggccgtgacgaggtcggtcttgttgaccaccagcacgtcgcagaactcgacctgctcgatcaagaggtcgaccacggtgcgggtgtcctcgtcgcccagcgactggccgcgctggcccaggctgtcgggcgagccgtagtcgcgcaggaagttgaaggcatcgaccacggtgaccatggtgtccaggcgcgccacgtcggcaaggctcttgccgtcttcgcccgcgaaggtgaaggtctcggccaccggcagcggctccgaaatgccggtcgattcgatcacgagctggtcgaagcgcccttccttcgcgagccggcccacttcgacgaggaggtcttcgcgcagcgtgcagcagatgcagccgttgctcatctcgaccagcttctcgtcggtgcgcgagagctccgcgccgccgccccgcaccagcgccgcgtcgatgttgacctcgctcatgtcattgacgatgaccgccacgcggcgcccctcgcggttgtgcaggatgtggttgagcagcgtggtcttgccggcgccgagaaaaccggacagcacggtgacgggaaggcggacggtcatgggtatggccctatatgcaacagaattgcattataggaaccaatgcaaccatgttgcgtttggtggacgccggcttttccactgccgtgccggtcggcatagactgttgcgcgccatgcaacaccctgccctgcccgttctctacagctttcgccgctgcccctacgcgatgcgcgcgcgcctggcaatggccgcgagcggcgagcgctgcgagctgcgtgaagtggtgctgaagaacaagcccgccgagatgctcgcggcttcgcccaagggcacggtgccggtgcttgtgctgcccgatgccacggtgctggaacaaagtctggacatcatgctgtgggcactgcgccgcgacgatccgttgcgctggttggaacccgacgccgccaagctcgacgacatgctcatgctcgtgaacgcttgcgacaaccagttcaagccgcagctcgaccgctacaagtacccggcgcgattcgagggttcgtccgccgatgcgcgcgagttgggcgtccggttcctgttggacctggaggcgcggctcgccggctccgggcagctattcggcgcgcgggcctcgttggcggatgcggccgtgatgcccttcgtgcggcagttcgcaatggtcgagcccgcatggttcgaaagccagccctggccttcgctgcgcgcctggctcgcgggctggaccgcttcgccgctgttcgagcgtgcgatgtggaagtacgcaccgtgggtcccgggcgaaattggcgtcgcctacccgccggcctgatcagccgaagttcggcgctcgccgctcgcgcagcgaggccacgccctcgcgcacatcggcgcccgcgaagcccatgaattcgagcgccagcgaagcgtcgaaggtcggcccggcctggcgcagccagttgttgagcgcgtacttggtgaagcggatcgcgctctggctgccggccgcgagccggtccgccacttcgtaggcgcgcggcagcagatcggcctcgtccaccgcgagcgacaccaggccgatgcgctcggcctcttcgccgctcaccggttcgcacagcaaaaggtggtatttggccttggccatgccgcacaagagcggccagacaatggccgcatggtcgcccgcggccacgcccaggcgcgtgtggccgtcgacgatcttcgcgcccttgctggcaatggagatgtccgccagcaggcccgccaccagccccgcgcccacggccgggccatgcatggcgctcacgatgggcttgtcgcagttgatgaggttgtagacgaggtcgcgtgcttctttccagacacgctggcgcaccgcgtcgtcggtggtcatgtcctgcaccatggccaggtcgccgccacccgagaagcccagcccctcgccccgcagcaccgcgcagcgcaccgtgtcgtcggccgacacgtcgcgccatatttccgccagttcgcgatggccgtcatggcccgccgtgggcagcttgccgttggtcgcgcgcatctggatgtcgagcaccgtatcgccgatgccgcggcgcgtgatggcaagggtctggtagcgggcgtagtccatggcgtgtctccacctcgcaatgcgtgcgaggattttcttttttcgtcgaaagacgggacgcctattttcgcgcggcaatctcgcggcagcgctgcacattggcctcgaagcgcggcgccagcccgggctcgcacccgtcgcccgaaggattcagcttgcacatgccgaccaccacatagtccatcaccgcctcggtacacatcgggtacttcgcgaggtcgggattggcctgcgccttgaagccccagcgctcggaaaactgcaccgtgcgcgccatcgcaccgtggaagaagctgcggtccttcgcggcaatggctgcttccatgcgaggcagctcctcgttcaggtagccgacggagtccagcgggaagtccgagggcgcctgctgcgcactggcgatggatgcggccaccatgagaagcggcaaggcgacgaaggtgcgcagccgcgaggacgacgaaggcgcgaaacggttgggcgtgcggtgtgattgcatggcttgggattttgcaacgtctggaagcatcttttcgtggcgggcgccacgcctacctgccttttttcggccggtcgaacttgcgccagtactggaattcgtcctcgtgcacttcgagatcgacttccgaaatgcgcgactggaggcgctcctgcacgtcggccacggccttgttgtagacgatggggccgacctcttcaagaaagaaaccgagcagcgcgccggccgcgatgttgccgatcttctcttccatgttctcgttgaagtagcgctcgatcgaggcgatggcctgctggcgtgcttccttggatatttcgatggtcatgagggctgctcttcgattcctggaaattgggtcaatccattgtgccgctaccatgcgctgcggccgcgcgcggcccgcagcacaaagacctacaacacggagaccgcttcatgaaattccatccggccgcactggccgccctggccctggccgctctcgccggctgcaccaacctgacccccaccgtgccgcagcgccagctgatgctggtggcgaacgacgaaaagcagtcgtggagcgacgccggtgccgtgatcctcggtccgatgggccgcgacacggtgcaggtgctcgacatcggcaccgacccgctcgcaccgaagctcgtgggcacgctgcagctcgacaacaccattgccggcccgccgaccaacctcgcgatcacgccgggcgaaacgctggcgctggtggccaactcgctcaacgtggtggaagagaacggcgtgcgcaagcaggtgcccgacaaccggctcttcgtgatcgacctgaccaccacgccgcccaagctgatcgacacgctcaccgtgggcaagcagccttcgggcctgtcgatcaaccgcgcgggcgacctcgcactggtggcgaatcgcgccgacaactcggtcagcgtgctgcgcatcgcgggcaagaaggtgacgctgatcgacaccgtggccatgaacgattcggtggcacacgtgcgcttcacgcccgacggcaagcgcgcgctcgcagccaagttcccgacccacaagatcgcgctgctcgaggtgaacggcgagaaggtgagctacaacaaggtggaccttgcggccggcctctggccctacaacgtcgacgtgacgccggacggcaagctcgcgctcacggcagacaacggcaactcgggcgcgtcggacgggcagatcgacacggtgagcgtgatcgatctggaggccacgccgccgcgcgtggtcgacaaggtggtagtgggcgacggccccgaaggcctggccgtgagcccgaccggccggcatgcggtggccgtgctcctgcgcggcagcaacgcggcgaagaacgcctacttctacaaccgcaacggctcggtggtgctgctcaagatcgacggcaagaaggtgacgcgcgccaacgaagtggtggtgcgtggcctgcctgaaggcgccgtgtggagtgcggacggcaagtacctgtacgtgggcaacttcatcgaccaggacatcacgatcctgcgcgtggacggcgacacgctggtgccgacgggcaagtcgtttccgctgcaggggcatccggccgcgatgcgcgggacaatgtcgcactgaccgaatagacgctcgacgcaaactgacctgaacgcaacgccatggcgcaacccaaacgacaactccgcacgatcgaacgcggcattctctgcctggcgatcggcgccgccgttctgctggcgccgcgcttcctgcaaggcacgcgctggttcgacatggtggccggtgcctacgtggtcggctggttcgcgctggcgctgggcgtggcgctggtggcggtcggcctctttcagcgcggcaaatagcgcgggcaagcgcggcccacggcccgcgggtcgcaagcgctcaggcggccttcttgccgcgcagcttgcccacgagttccacgcccgccagcacgatggcgcccgccacaatgccgatgccggcgttcacccccatcgagccgagcgcgccgaacacgccgcccgtggccttggcccagtcttcgaccgcgtggccgaatgcgggcacgccgtgcaccaggatgccgccgccgaccaggaacatggccgcggtgcccgcaaccgacagccccttcatgagccatggcgccgcagcgagaatgccacgccccaaagcctgcgcggccttgctggcttgctggctcaggtacaggcccgcgtcgtcgagcttcacgatgccggcgaccaggccgtagacgccgacggtcatgatcagcgcaatgccagcgagcaccgcgaactgcgtggtgaacggctgaccctgcacggtgcccagcgtgatggcgatgatttcggccgagaggatgaagtcggtgcgcactgcgcccttgatcttgtccttctcgaccgccaccacgtcgacggtctcgtcggccacggcgcgctcgtggcgcgcggtgtcggcctcgtgctccttcttgtgcaggaacttgtgcgcgagtttttcgaagccttcgaagcagagaaaggcgccgccgatcatgagcagaggcgtcaccagccagggcagccaggtgccgatggccagcgccgccggaaccaggatggccttgttgatgaacgagcccttgcacaccgcccagaccaccggcagttcgcggtcggccttgacgcccgacacctgctgcgcattgagcgcaaggtcgtcgcccagcacgccggccgtcttcttggcggcgagcttggtaaggatcgagacgtcgtccaggacggtcgcgatgtcgtcgagcagcagaagcaggctggtggccatggcaagaatcggtatgaaaaagaaccggcgagcttagccgcaagcgccgcccgcgccggcaatacccgtacgcggtgggcgcgtcgttggcgtcaggcgacgctgcgcttgaggcggatctcttcgacccgcacggtgcccagcgcggtggtcttggcggtcttcatttcgcgcttgaagccggccagctcgtggaagcgcatggcgcggtcgttgcgaatgggcacccacacggtgaccgtggtgcagccctcttcctcgaggccttcgcgcgcggcgtcccagagggcgacgccgatgcccttgccccagtgctcgggcttgacgtagatggcccagatctcgcccgtggtggacggcgtcttggggtcgcgcgagcggtcgaagccgacaaagccgacgatttcgccgtccagcaccgcgacttgcacctgcggctcgctgaactcgatggcttcgcgccacttggcttcacgcgaggcgggagccagcaagcgcagctcttcttcgggcaggatgccttcgtaggcggccttggcggccagggcatggacttcggcgacggccttggcgtcgcgcatggtggcggggcgaacttcgtaatctgacatggatgcggggaaatcaaatggaaccgcgtattgtcgccgcaccgctaaacttcccattacatacgccgcatacgcagcatcaaaaggagtcgatatggcaaaaggtcaacaacgcgcgaacaaggaagccaagaaaccgaagaaggacacctcgccgcccaagccggtaggcaccggcggcatcgaacccgtccgcacgatcaccacggcggtgattccgcgcggcaagctcaagaacaagtgaccgatgaggcaccagcggggcctgtgccgccaccggcgcccgccaagccggcccagcctcgcaacccgctgcacgggctcacgctggaggccatcgtgacggcgctggccgactactacggctgggagcggctcggcgagctggttcccatccgctgcttcgcgatcgacccgagcgtgggctccagcctcaagttcctgcgcaagacgccctgggcgcgcgagaaggtcgagagcctctatctcttcatgctgcgcgaacagcgccgcgagcagcaacaacagcagcagccgccacagcgatgagggttcgactcgaaccgtcgggcctcggtttcgaggccgaggccggcaccacgcttttgaaatcggccgaggcggccggcatcgagatgccgagctcctgccgcaacggcacctgccgcacctgcatctgccaactggtgtcgggcgccatccgccatgtcatcgaatggcccggactgagcgccgaggaaaaggccgagggctggatccttccctgcgtggccgaggcgcaaggcgacctcacgatcgatgcgccccaggcgttttcggtgttctgaaaaaggccgctgcgccgcttcgcgctatttgatggccgccgccggcattgccaccaccagccgatcgcgctgcgccagcgacgggaacagcttgaaccagcccagcgccaccatcatggtgcccacgccgccgaccaccaccgagcccaccggccccagaagcgccgcggtggcacccgattcgaactcgcccagctggttgctggcgccgatgaagatcgaattgaccgcgctcacgcggccgcgcatggcgtcgggcgtttcgagctggaccagggtctggcggatcaccacgttgaccatgtcggcgccgcccgacaccatcagcgcgatcagcgagacgatgaagctgcgcgaaattccgaacaccaccatgcacagcccgaagagcccgacggccatcagcagcgtgcggccgatgttgcgctcgatgggccggcgcgtgagcgcgatcgacatcaccagcgcccccaccgccggcgccccgcgcagcaggccgagcccccagggccccgtgtgcaggatgtccttggcgtagatcggcagcagcgccaccgcaccgcccaggagcaccgcgaaaagatccagcgacacggcgccgagcacgggcttgcgcctccagatgaaatcgacgccggcaaacacggtggccagcgtgaccggctcgcgcgcggccggcgtatggacatagcgcagccgcaatacaaggccgcaggccaccgcgaagcacagcacgctggcgccgtacaccacctgcatgccggccacgaaaagcaggccgccgagggccggtccgccgatgatcgcgccctgcatgccggccgagctgaaggccattgcgcgcggcagcatgatgggcgacaccaagagcggcgtcagcgcctgctgcgcgggcatctggaaggcccgcacagcgcccagcaccagcgagaggcccagcagcaggccgcgcgtgtcgaagcgctgcaccaccgcgagcagcagcaccagcgccaccagcccctgcaccgcaaagcaggccgccacgatgcggccccggtgatggcggtcgaccacgtggccggcgagcagcgccagcaacagcgcgggaacgaattggtaaaggcccacgagcccgaggtcccaggcactgctggtgagctcgtacatgtgccagccgatggccaccaggagcatctgcgaggccgcggtgccgaagaggcgcgccacccacatccgcatgaaggggcgctcgcgcgtgagttcggaaaagctcgggggcggggaggcggaagcggaggcaggggcggaagcagggccggacattcgttcgaggatagccgaggctccatgagccgcgcatgagcgtgggctctctacactctcggcactcatgccggacaccgacgccatcgacctcgtctaccaggacgcccatctgctcgtgctgaacaagcccgccggcctgctctgcgtgcccggacgcggcgaagacaagcaggattgcctgagcgcgcgcgccatgcggcaatggcccgacgcgctgatcgtccaccggctcgacatggccaccagcggactcgtgctgatggcgcgcggcgccgccatgcagcgtgccctcggcgacgcctttgccaatcgcctggtgcacaagcgctaccaggccatcgtggatggcgcgatgcccgtgcgagacgaatggtcggtcatcgatgcgccgctgatggccgactggcctcggcgcccgctgcagaaggtcgacgcggcgggcaagcccagcgtcacgcgctggcgggtattgcactcatcgccggcaggcgacctcgccgctgccacacacgtgctgctggagccgctcacggggcgttcgcatcaattgcgcgtgcatctgctctcgatcggccatccgatccttggcgatgcgctctacggaagtgaagaggttcaggcgcgcgccccgcgcctgctgctgcatgcgagcgaattgggcttcgtgcatccggcgacgcagcagacccttcgattcgaaagccctccggacttctcgctgctcagccgcccttgaccaccagcacgggcatgggcgcgtcctgcagcacgcgctgcgtgacgctgccgagcagcagcttctcgatgccgctgcggccatgcgaacccatgacgatcaggtcggccgcgatggcaatggcggtgtcgacgatgccttcgtgcaccacgtggccgtcgatcacgcgctggtcgctgtgcaggccttcggccgcaagtgccgcaacgccgcgcgccagggccgcattcgcgctcgcggtggccgccgccaggtattcgttctggcccagtgcgtagtccgcacccacgccgatgaaaggatagttgtcgatcacgtggatcagcgtgatgcggctcccgaacgccagcgccaggccgctggccttgctgaccgcgagcatggaagtttcggagccgtcgatcggaaccaggatgtgattgaacatggcggacctcactttttcgttcgcggacaggcgcggctcgcaaccgaaccgtccctcgaatttaccccctgcgcgggggcctgactgtaggactcaagccagcgggctcaatccccctggaaaccctgagcgcggcaagtgaccacaagggtatcgcgccagccgggggtaccctcttcgagcggctggatgggcgtggactcgtggatcacgcgcgcatcgtcgagcagcagcagcgtccatggctcggtcatggtgaagcgctcgccgcgccgcccattggcttcgaacacacgggtttcgccgcccttgacgccgctgcgcccgaccagcgccaccgccaccaggtcgacaccgtcgcggtgcgcgccttcaggcgtgggccggccgatgccgcccgccgtgtcgatgcggaactgatgcgcttcgacgaaccatggctgcgccgcggcggcgcgcatgttgctggccgcttcgcccaggcgttgcagcaggcgctgccatgccggctgcgccacggtggcttcgtgcatgggcgcaaaccagcgctgcatgccgccgtgcagcgcgttgtattcgaccggctgccagtgcgcgcggtgcggcacctgcgcgattgactcgccctcgaccgtgaaacacgcgtggcgcctcgtgcggtagcggcctccgtccttcaggtattcgtccggtggaagatcgttccagtcggcgtgcagcgcctcgagctgcgcgagcggcacgccgagccagtcgctcacgccttgcgggctcagcaccgcatagccttgttcgcgcagggcggccggcagttcggctggctggatgaacggcggtgcgaatgcggccgtggtcacgacgcgctgactttcacgtctttccagaacgccacgcggtcgcggatttcctcggcttcgggcttcgggtcggcgtagtaccaggccgcgtcagtatggagctcaccgttgaccagcagcgagtagtagctggccgtgcccttccagtggcaggtggtcttgtggttgctgaaggtgacgtggtcgcggttgagcgagctcatcgggaaatagtggttgccttcgacgagcacggtgtcgtcgctttcggcgatggtgacgccgttccaggttgctctcatgtcttgctctctccaagggaggatgcgggggcgcttggctgttttgcggctgccgcacggggaagggatattgtgccttctgcttttggcatgccttctgtccgggtgtatgtgggcttgttttcttcccgaggccgggtctcgccccgctgggcgactcactttctttgcttcaccgcggcgcgcagcgccgcggtggcctggtggccgagcgaagcaaaggcccgttcggtctccaagcccctctgtatgcgccgaggagcgcagggtttcgcggatcagggctcgcagctgtttgagcgaagcgagttctgcgagaccccgcgaaacccgagcaccgcaggttgccccgtagcaaagcgaaggggtcgcagacagtggggtcgccttttctttgcttactttcttttggcgaagcaaaagaaagtgagtcgcccgtcggggcgacacccggcctcggaacctaaatcaggcccctaaccaatgcacactaaaaagcctctccggatccgtccaaaccgccaaaggccgaaaccccgccttcacagccagcgcccgcaacccttcaacggtgaacttgtgcgagtactccgtatgaatcgtctcgccctcatcaaagccgaataactcgccattcaatgaaaccgcctgcgcccgccggctcacaagatgcatctcgattcgctgcttcggcgcgttgtagaacgccgcgtgcgcaaagccgtcgatgtcgaaatccgtgtcgagttcggcattcgcgcgccgcagcaggttgaggttgaacgccgaggtcacgccttgcgcgtcgttgtacgccgcatgcaggcgatccgggtccttcaccagatcgacgccgatcaggagtcctccgccgcgcagcatccgcgccgcaagctgcagaaacgccagggcctcgtcgggttcgaagtttccgatcgtcgagccgggaaaaaacccgacgcgcttgcccgcaccgggcagtggcgcgggcagtaccaggggcatcgtgtagtcggctgcgatcggctgcaccgcgagcctggggtagtcggccttcagccgctcggcggcggcctccaggtgttcgcccgagatgtcgatgggcaggtagcgccggggcgattcgagcgcatcgagcagaagccgcaccttggtgagcgagccggcgccgaactccacgatttccgcgccgggaccgatctgcccggcgatctcccccgcgcattcgccgaggatgcgcagctcggtgcgcgtggggtagtactcgggcaattcgcagatgcgatcgaacagctgcgaacccgctgcgtcataaaaatatttgggcgaaatccggcgcggcttgcgcgcaaggccggcttgcatctcgcggccgaattcggagaggagcggcacggccgcggcgacgggcgccgcgggctggcgctgcgcggctgcagcaaacgaaatggaggacgaagatgttggattgcgcatgattcagacgtctttcgcgagccgcagccccgagaactgccagcgcgcggccggcggaaagaagttgcggtagctgggccgcgtgtgcccggccggggtggccacgctgccaccgcgcaacaccagttgacccaccatgaacttgccgttgtattcggccgcgataccgggcatgggccggaacccagggtatgggtcataggaggaccgggtccactgccagacatggccggccatctgcgagatgccgggcgcgtcgaaggcggcctcccattcgaactcggtcggcagccgcgcgccggcccattcggcgtatgcggcggcttcatagaagctgagttgcgacaccggcgcatcggcttccatgggccgaacgccgtgcaggccgaacacctgccaaccgccctgttgctgctgggctccaagccgcggatcgtccgccgcgagccagtacgccggatgccgccagccctgcgcctgcacggcagcccagccatcggacagccagagctcgggccgctggtagccgccgtcggcaatgaactgcgcgtagtcgccgcagttcaccagcctgtcggcaatggcatagggttgcagcagcgccgcatggcgcggcgtttcgttgtcgaaggcaaagccttgtccttcatggcccacctggaccacgccgccaggccttggcagccagcgcatggctggcggcaaggcagcgagccgcagcgcgggccccgaggcgggcttgtaggctggcagcagcgggttgcacgacagcgcatgaagaatgtcggtgagcagcagctcctgatgctgctgttcgtgatggaggccaagcgtgacgatgggctcgatggcggcccagtcctggtcgccgatgccgccgtcgagcagggccagcaccgcctcgtcgacatggctgcggtaggcatgcacctcgtccaccgaaggccgcgtgagcagcccccgctgcggccgcggatggcgcgggccgagcgcctcgtagtacgaattgaagaggtactgaaaacgggtatcgaaggcccggtagcccacggcatgcggctggagcagcacggtctcgaagaaccacgtggtgtgcgccaggtgccatttggtcgggctcgcgtcgggcatcgactggatgcactggtcttcggcggagagcggcgcggcgagtgccaggctggcggcgcgcacttcgcggaacttgtcgcgcagcgcgcttgccgcctgggtgatcggccgggaaagcgtcatggtgtctccagtcgggtcaaccgcaatttgtagccgatcggtgttgccgcatcacgtaggacaagtgcccgccctgccctgtgccgcgggggccgcccgatcggcgggggagccactttggcacaagatgggctgacgtgcagggcgcctgcgtatcatccgctcgatgcaaacgaacaacgcctccgcccgcccccgtgtcgtcatcgtcggctgcggattcggcgggctcgaagccgcccgcaagctcgaaggcgccgacgtggacgtgacggtgatcgagaagaccaaccaccacctgttccagcccctgctctaccaagtggcgaccgccgggctggccgcaccgtcgattgcggcgccggtgcgcaccctgttccgccagcagccgcgcatcaccacgctgctcggcgaagtgagcgccatcgatacctcggcgcgcgcggtgcagctggccaacggcaaccgcgtcgcgtacgaccatctggtcgtcgcggccggtgccacgcacagctacttcggccatgacgaatgggcgcccgtcgcgcccggcctcaagacgctggccgacgcgttcgaaatccgccgccgcgtgctgatgtcgttcgaggcggccgaaaccgccaccgatccgcagcgccgccgcgccctgctcaccttcgcggtgatcggcgccgggccgaccggtgtcgaaatggcgggcacgctggccgaaattgccaagcacacgctttccggcgagttccgccacatcgaccccggcagcgcccaggtgctgctgatcgaaggcgggccgcgcgtgctgcaggccatgcccgagagcctgagccagaaagcgctggaacagctggaaaaactcggcgtcgaggtgcggctcaatgcacgcgtcacggccatcgacgccaccgggctcgaagtgcagtcaggcggcggcgcggacggcgcaggggccaccagctaccgcatcgacaccagctgcgtggtgtgggcggcgggcgtcgccgcgtctccgctgggccgcatgctgggcgaggcgaccggtgtcgagtgcgaccgcgccggccgcatcaaggtcgagcccgacctgagcctggccggccatcccgagatcagcgtggtgggcgaccttgcggcggccctgagccatgcgcccggcaagccgcccaagccggtgcccggcgtgtcgcccggcgccaagcagatgggccgcgccgcggccgcgaacattctgcgccgcatcaagggcgagccgaccgcgccgttccgctatcgcgactacggcaacctggccaccatcggccgcaactcagcggtggtggacctgggcacgcccttcgggccgttacgcttcagcggtcgcctggcctggctcttctggctgttcgcgcacgcgtacttcttgatcggcttccgcaaccgcatcgtggtgatgatggactgggccagcgcctactggagcttccagcgcaatgcgcgcgtggtggcggacgtgcagggcaggagcgagtcttagcggcgggccggaggcgtctccagagccgtcttgcgagcggcccacgtcccttcccgcatcaggttccgatcacgccgccatcgttcttcgtgatgaccacggtcgccgagcgcggacggcccgcgccgtccggccacttcgacacggccagtggacgatccggatcgctgcgctcgttggccggctcgcccggatgctggatgttgatgaagagcgtgcgcagatcgggcgtggtcgtcaggcccgtgacctcgcagccggccgggccgagcaggaaacggcggatctcgcccttggtcgggtcgcaggccagcatctggttgttggacaggttgccgtactcgcccttgccgagcgtggaggtcgagacgtcggtctcgatccacagcacgccgcgcgcatcgaccatcagcccatcggggctgccgaaggtgtcgcccttgatattgccttgcgcctcagagcgcgtctgcttcggatcgcccgcaagcacgaggtggttccaggcgaacttggtcgcatcgaggtcgccgctttccttccagcggatgatctggcccatcgtgttgttggagcgcggattggccgcgtccatgaaaggctggcccggcgcaccgcggttgctgttgttggtgagcgtgcagtagacctccttcgtcagcggatcgacggaggtccattcggggcggtccatcttggtggcgcccagcaggtcgctggcctggcgcgccttgatgagcacgtcgccctggctcgcgaagcccttgtcggcggtgagcccgttcttgccctgcaccagcggcagccattcgccggtaccgtccacgtcgaagcggcccacgtagagcgtgccgtggtcgagcagttcgcggttggcggcggcgccgcccggctgcaccttgtcgcggctcacgaacttgtagatgtattcgaagcgcgagtcctcgcccatgtagatcacggcgcgcccatcgttggtgagcgcggtggcggcgccttcgtgcgcggcgcggccgagggcggtgcgcttgcgcggcgtcgatgccgggtcctgcgggtcgatctcgaccacccagccgtaccggttcgattcgttcgggtgcttcgccacgtcgaagcgctcttcgtgctcgtgccagcggtacttggcgccgttgcccttcttgatgccccagcgcttctggtgcgcatccggcgtgtcggtgccttcgaaatagtccgcaaagttttcttcgcaggtcaggtaggtaccccacggcgtctggccgttcgagcagttgttgtaggtgccgagcacctgcgtgccggtcgggtcacctgcggtgcgcagcatcgggtggcctgcggcgggaccggtcagcgtcatcggcgtgagcgcggtgatgcggcgcgcgaagcgcgaaggcagcacctgcgaccacttggcgccttcgcgctgcagctcgatcaccgagacgccgtgcgcgttcatggacttgcgcaccttctcggccgtccaggtcttcatgccgtccgtatgcagcaggccgtcgtccacgtattcatggttcagcaccagcaggccgcggttcgatccgtcgagcggaaagaaggccatgccgtcgtggtgcatgccggcctgcagagcctgttcgtccgcggtgttggagccatcggccttgaaggcgggcatgcggcccgcgatgccggtggcgtcgccccagcggtagatcacctgcgtgctgtagccctcgggcacgacgacccggtcgacagccgccatgggcacgctcttgaagccgatggcccggcccagcgtgctcaccgaactgccggtggtggcgcaaccggccagcgtgccggccgccaggggaccgaaaagacccgccacggccgccgccaggccgccgcgcacgaacacccggcgcgacggatcggatacctcgtggatcgtggggttggcggaggggttggagtcctccatctgctcgaaatctttggccatcttcttgtcgtcaggggttgcgagaacccgcgatggtcccgcatccgcatgaatcccccatgacagcggccccggaggctcagaagaaggcgtcgctccaatggtgctcgcgccgctcccgccgccagtcccagggcggcgtcggcttcgaatcggcccacaaccccaggccctgcctgcgcgcggcatcctgcagcttgaagagtccgccgccgcgcctggtcgcgataccgttgtagtcgtacacccaggcccagcccccggacaccatgcggctgcctgcgtcctcgccgttgcagctcacgtcggccacggtgcggccatagcggtcggtgtcgcgctcggtgatgagcgccttctcggcatagcagaggcggctcagggcctgccggctgcgctgaccatggggctgcttccgttcaggcgcatcgatggcggcgatgcgcaccttgatctgctcgtaggcaccgatgcggccgcagcgcgcggtgagcgtgtcgccgtcgctgacgccgaccaccaggcaggttcgaggggcggcctgggacagctgaggcaaaagagcaagacagatggcgaagagaaagcgcaagcgcatgagcggagaaaccgtggcggtcaaaggcacggattctcggtgcgaagtgcccgggcgccggggccggaacccgctgttacgcggcgctgccgttctcgtcttcctgcagcagccgccacatcaccttgccgctcccgctcttgggcagcgcatcgacgaactgcaccttgcgcggaatcttgtagaccgccatgttctcgcggcaccagtcgatgatgtcctgctcggtggtgtccttgtgcgtggcgcgcagcacgaccacggccttgaccgattcgccgcggtagctgtccttggtggaaatgacgcaggcctcctggatggccgggtggcggaacatcagcagctcgacctcggccggccacaccttgaagccgctcgcgttgatcatgcgcttgaggcggtcggtgatgaagaaatagccgtcctcgtccatgcggcccatgtcgcccgaacggaagaagcgcttgccttcgaactcgacgaaggcggcccgggtggcgtcggggcgcttccagtagccctggaacacctcggggccgtggatgatgatctcgcccgattcgccgatgggcatttcggccaacgtatccggatcgaccacgcgcgcatcggtgctcatgaacggaatgcccaggcactgctgcttggggttgtccgacgggttggtgtgcgatggcgccgctgtttcggtgaggccgtagccctcctggtacttgaggccgtactgctcgaagaggcgctgcgccacggcctgcggcatggcggcgccgccgccgccgatgtgggtgatgctcgacaggtcgtagctcgcgaagttggggctggccatgaggtcgatcaccatggtcggaatgttggtccagctggtgaccttccagcgcgagatgagccgcccggccacgtcgcggtcccagcgcggcatgatgaccagcgtgcccgccgcgaggatggaggtgtgcatcatgctcaccacgccggtgatgtggaacatgggcaccacggccagcaccaccgcttccgacgtggcctggccccagagctggctggccacggcgttgtgcatgaggctcgagtgatggtgcacgcagcccttgggcaagccggtggtgccgctggtgtagggcagcagcgccatgtcgttggcgcccaccacgtgctcgggcgcggcatggcccgcggccagcgcgtcggtccaggccatggccttgccgcccgccagctcgggcaatggatggcgcgtggtgagccagtctttccatgccggcgcgggggcgtcgtcgccgttcgcgtcggcgtcgaaggcatcggtgaactgggtcacgatcatgtgggccagctgctgctccggcggcagcgcattgctggccttggccagctcccccgccaggtcgccggtggtgatggccaccttcgcgtcggggtcgacgatgtagtgcttgagctcttcggcccggttcatcgggttgaccggcaccaccacggcattggcccgcaggatcgcgaaatgcgcgatcacgagctgcgggcagttctgcatgttcagcaccacgcggtcgccgcgcttcacgcccagggcaagcagcgtgccggcgaggcgctcggcctggtcggcgaaatcgcggtagttcaccacgcggccgaagaacaccagagcggccttgtcgggatagcgcgccgccgacgtcgcgaggttgtgccagagcgaggtggcgggcacggtgatcgaatgcgggaggcgcttgggccagaacttgtggtgcgggcgttgttgcatggtcgaaggggcagtcggtcggaggggagaaaaagggacagtccgcagcctaaggcgacccgtccgccgctcccatcggggaagcccccgggggcgtcaccttggcgacgcccttttgtttcaacggcgagaacttcatcgcacgcgccctgcgactacagacaagcccggcgttccgcgcgaaccttcggctccccaacgtcacccgaatgaaggagagtttcatgccagcagacaagcacgcaagcgttcactgggaaggcgccggcaagaccggcaagggccaggtcagcaccgagaccggcgccctcaaggactatccctacggcttcgcgagccgcttcgaggacgacaagcgcggtaccaaccccgaggagatcgtcggcgcggcccatgcggcctgcttgacgatggcctttgccttcgccttggagaaagagggcttcaccgctacccgcatcgacaccaaggccgcggtgcgcctggccaaggacggcgaaggcttcaagatcgaccgcatcgcgctggagctcgacgccgccgtgccgaaactcgacgaagccaagttccaccagatcgcggccgccgccaaggccggatgcccgttgtcgaaggcgctggccagcgtgccggagatcacgctgaaggccacgctggccggctgagcgctgcttatgatcgtctccactacaagaggagacgatccatggcccaccgccacccggtccgcgccgccatcatggcggctttttcaattgcgtcgttcgcatcgttcggcatcggcggccttgcacacgccgcctatcccgacaagccgatcaaggtggtcatcggctttccggccggcggcccgctcgaccagcatgcgcgcctcttgacggacaagctgcaggccgtgctcggccagccgctgatcgtcgactacaagcccggcgcgggcggctcggtgggcgccgacgccgtcgccaagagcccggccgacggctacaccctgctgctggccaacaccggcgtggccgtgatcaacggcgcgctctacagcaagctgccctacaacacacagcgcgatttcgtgccgattgcgcgcaccgccatgcagccgctggcactgctggtcacgccgaagctgccggtgcaagacctgaagcagttcgtcgactacgccaaggcgcggcccggccaggtcaactacggctcggccggcaacggcggcatcagccacctggtgcccgagatgttcaagaccgcgaccggcatcttcatggtgcacataccctaccgcggcagcgcaccggcctttaccgacctgatggccgggcaggtgcagttcatggccgagtcgattccgcaagccgccaactatcacaagcaaggcaaggtgcgcgccctggccgtgaccagccgcgagcgcaaccccgccctgcccgacgtgccgaccgtcatcgaatcgggcatcaagggcttcgaggtggtgggcttctacggctttctcgcgcccaaggacacgcccaaggacgtggtcgccaggctcagcgacgcgttcaggcaggtgctgaccagcgccgaggtgcgcgaccgcatggtgagccagggcgcggacccggccttcctgggcagcgaggatttcgcgcgcttcctggccacggaaacgccacgctgggaaaaggccgtcaaggcttccggcgcccggatggactgaccggccgcccgcattttgggcgacttgcggggcagcccaacccatttcggtgcacataacttgcataccagttggcacagaagctgctgatatgcaggcctatggccatttccgcatccgaaatcagtgcacgcatcgtcgaagcggtgatggcgcagaagctcgcgccgggttcgcgcctgggcgagcagcagctcgccatgctgttcgactgcagccgcaccatcgtgcgggaggcgctcacccgtctggccgcgcgcggcatcgtcaccgtgagcgcacggcgcggctggttcgtgatcgaaccttcgcaggacgaggcgcgcgaagccttcgaagcccggcgcgtcatcgaactgggccttatccgcagtgcgggcagcaccggcaagatcgacaagaccgcactgcgccagttgaaggcgcacctccagcgtgaaaaaacggcgctgaaggaaaacgacgtcggcaaccgcagcttcctgctcggcgactttcacgtgtgcctggccgaatgcctgggcaacaccctcctggccgacacgctgcgcgacttcacggcgcgcaccacgctgatcgccatgctctaccagtcttcgcacgatgccgtgcagtcatgcgaggaccacgtgcagatcgttgccgcactcgaacggggcgaccatgccaccgccgaggcattgatggccgcgcacatcggcacggtgcagtcggcgctgcgcgtgcaggcacccaccgatccgctcgcgcaactgcgcgacgccctggcaccgcttcagaacacctcggccaagccgaagcggcgcaaggccgcgccctcccccgacgacaccgattcaacgacttacctaggagccctgctatgaacttctcttcgtccaaacgccacctcacgctcgcacttgcttccgttgccatgctggctgcagccggtgccgcccaagcccagaacgcactggacaacgtgctgaaggccaagaccatcaagatcgccgtgccgaccgactacccgccgtatggctcggtcgacaagaacatgaagccgcaaggcctcgacgtggaaatggccgagctgatcgccgccaagctgggcgtgaaggtcgagctggtgcccgtgaccagcgccaaccgcattccctacctgcagacccgcaaggccgacctcgtgatctccacgctcggcaagaatgccgagcgcgagaaggtgatcgagttctcttcggcctacgcccccttcttccaggccgtgtacgcggccaagagcatgaagctcaccagctttgccgacatggccggcaagactgtcgccgtgacgcgcggcgccatggaagaccaggaactgaacaaggtggcgccgccgaacgtcgactaccgccgcttcgaagacaacaacgcaaccatcgcagccttcgttgccggccagacgcaaaccgttgccaccagcgcggcggtcgcaggcgacatgctcgccaagaacccgaaggtcagcgccgagttcaagctgctgctgaaagacagcccctgctacgtcggtgtcgcaaagggcgaaaccgcattgaagaccaaggtcaacgagatcatcgcagcggccaagaaggacggcacgctcgacgccatgtcgaagaagtggcttggcaaggcggccggcgacctgcccgtctgacccacgctgaacctttcataaaggcgccgccatggaattcgatttcggtgcagttcttgtcgactggcggctgctcgccaagggcattgcctggacagtcggcctgacggccattgccacggtcatcggcatggccgtgggcgtggcctgcgcctgggcacgcgccaacgggccgttgtggctgcgctgggtggccggcagctatgtggagctgatccgcaacacgccgttcatcgtccagctcttcttcatcttcttcgggctgcccgcggcgggcgtcaagctcacgccggagacggcatcgatcattgcgatggtgatgaacctcggggcctattccaccgagatcatccgcgccggcatcgaggccacgcccaaggggcaaatcgaggcggccgtgagcctggcgctcaacaaggtgcaggtgttcacccgcgtggtgctgccgccggcgctcaagaaggtgtggcccgccatggtgagccagatcatcatcgtgatgctgggctcggccgtctgcggacagatctccacggaagagctgagctatgcggccaacctcatccagagccgcaacttccgcgcattcgaggccttcatcatcgccacgctgctctacctggcgctggcggttgcgctgcgcaaattgctcaactgggccggtccgagattcttcttcggccgctgaacgcaggaagccacaccatggtcgatttttctctctgggacatcctgcgcaacctgctgatggcgctgcgctggaccgtcgtgctgtcgttcatcgccttcgttggcggcgggctggtgggcggcctgcttctgtttttgcgcctgcgcggcggcagcgtcatggaccgcgccgtcggtctctacgtgcagctgtttcagggcacgccgctgctgatgcagctgtttctcgcctacttcggcatcgcgctgttcggcgtcgacgtgtcggcgtggaccgcggccagcgtggcgctcacgctctacaccagcgcctttctcaccgagatctggcgcggctgcgtggcctccattcccaagggccagtgggaggcttcgggcagcctggccttgagcttcgccgaacagatgcgccacgtgatcctgccgcaggccgtgaagatcgccattgcgccgaccgtcggcttcctggtgcaggttatcaagggcactgcgctcgcctcggtcatcggcttcgtcgaactcaccaaggccggcagcatgatttcgaacgccaccttccagcccttcgtggtgttcagctgcgtggcgctgctttacttcgtgctgtgcttcccggtaagcctgtacgccaagaatctcgagaggaaatcccatggccgccgtgcttgaatcccagaccttcgccgcgcccatcgtgcgcgtcaccgcgctacgcaaatcgtacggcaccaacgaggtgctcaagggcatcgatctcgacgtgaagcgcggcgaggtcattgccatcatcggcaagagcggctcgggcaagagcacgctgctgcgctgcatcaacgggctcgaggtgttccaggaaggctcgctcacggtcgacggcaagcccctgctgcacgaaagcgccatggccatgcgcgagctgcgccagcgcgtgggcatgatcttccagagcttcaacctgtttccgcatctcacggtcggcaagaacgtgatgctcgcacccacgctggtgaaaaagcgaggcggcctggaggcggcatcgcaggcgcgcaagctgctcgagcgcgtgggcctggccgagaagttcgacgccatgcccgaccagctctccggcggacagcagcagcgcgtggccattgcccgcgcgctggccatggagcccgccgtgctgctgtgcgacgagatcacctcggcgctcgaccccgaactggtgggcgaggtgctgcgcgtggtggagtcgctggccgacgaaggcatgacgctcctgatggtcacgcacgagatgagctttgcgcgcaaggtgagcgaccgcgtgatcttcatgcaccagggccgcgtgcacgagatggggccgccggccgaactgttcggcaacccgcagacggccgaactgaagcagtttctttcgtcgctgcacgactgaggcagcaagccaccgctcgctcaccgctacttgcgagcctgcgccttcgtgcgcttgcgcacggccatgccgggcgcaggctcgaagttgtcttcaggcccgagcccggtggccacaccgagccgggccgccaggtgcgcggcatcgtagggcgcatgcaccttgacgtcgttgtcgaagtagcaatacacgtcgcgaccctttcgccgggatagccggcgtgagggcgcggccagtttcgcgtccttcacctggcgcccatggcgccaggcgtcgatgcgttcggcccagcggtcgagtgcgccgtcgctgtagccgctggcgtagagctccttgtcgccatgcagccgcatgtagacgaaatcggcgcaaaggtcttcgagcagcggccagcgccctgccgtgtcggccaccaccagcgcgacaccatgccggcgcagcagcgcgatgaactccggattcgcgaaactggcatgccggacttccagtgcatggcggatgcggagtttcgcgggcaccttcaacaacgcacggtcgtcgccgaccttctcgttgtgctctcgcgccagcgcaagagcggaccggccatccctgggcaacagcgccaggaattcttcgaggcgatcggcgctgtaggcaaaggacggcggcaattgccacaggatcggccccagcttggcccccaacgcgaacacgcccgacgcaaagaagttggccagcgcggtacggggttccttgagccgcaggttgtgagtgatgtagcgcggccccttcaccgcaaagacgaagtcgtccggcgttgcgtcgtgccacgcctggtacgacacggggcgctgcagcgaatagaacgagccgttgatctcgatggtcggcagcatgcgcgaggcaaaatcgagctcgaggcgctgcgcaagccctttgggatagaagcggccccgccatggcgcgtagcgccagccagagattccgattcgcgtggcgccctgcatcgttcgtctttttttgccgaagccccgaacgtggcccgcggggcggcggcgtggcgtaggacgtattcccatccgcgtagcggcttgggatacttgcgaaccccgccgccccctgacaggaaccacccggcctgtggcaagctccgataagtatgcaaatccgccccctgcctttcacctcccgccgatggatgctgcgcgcgctgctgggcgccgccgccctgcaatcgcctctctcggcgctggccggtttcaatttcttcctcagcgaatacaccgcgacccgcgacgagctgcaggcgcagatcgccaggcgctttccggtggccgagcgctatgccgagatcttcatggtcgggctgcgcgatccgcagctgggcctggacgcgcgcagcaaccgcgccgccatcacggccacgctgaccattgcgagccccctcctggccgaatcgccggtgcagggcgtggtctcggtgagcagcgcgttgcgctacgacgccgccacgcgtgcgctgcggctcgaccagccgaaagccgagcgcctcgaattgcagggcgtgcaaggcgatgccgaacggctgcaaaagatcggcgcagtggtcgcgcaggaactgctgcaaggccaggtgctgcgcagcttcaccgccgaagaactcaccgtcggccgcaagacctacgaaatcggtgacatcacggtgcaagacgacggcatcaaagtgcagctcaaatgaaataccccctgcttgccgccgcactgctgattgcaggctgtgcggccattctccccaaggcaaagcagcacttcgacctgcaggcccaccgtggcgggcgcggcctcgcacccgagaacacgctggccgccttctccaaggccatcgacctgggcgtgaacacgctcgaactcgacgtcggactcacggccgacggcgtggtcgtcatctcgcacgacaccgcgctcaaccccgaccacacgcgggatgcgaacggcgcatggctcgcaccgaagaacggtgccacggtccgctcgctcactctggcgcaacttcaaagctacgacgtgggccgcctcaatcccgcgagcaactacggcaagcagtttgcattgcaaatcccgcaagacggcgaacgcattcccaccctggccgccctgttcgaccacgtgcgcgcacgcggcgccgcagccgccacggtgcgcttcaatatcgagaccaagatcgatccgaccaagccggaggaaaccgccgcgcccgagccgatggtgcgcgccctgctggccgaaatcgacaagtcgcagatgggcagtcgggtcacggtccagagcttcgactggcgcacgctcgcgctggtcggccaactggcgccgcagttgccgcgggcctacctcagctccgcgcgcacgctcaaggacagccgctggacagccgggctcgacgccgccaatttcacctccacgccgcaactggtcaaggctgcggcaggcaagccggaaggcccggtgacctggtcgccggcctacaacgacctgaccccagcggccatcaaggaggcgcaaggcctcggcttcaaggtgctgccctggaccgtgaaccagcgcgccgacatgctgcggctgatggactggggcgtggacgggatcattaccgactatcccgatgtgctgcgcgacctgattcgcgaacgcggcctgtcgctgccgccgccaggaaaggccgcgccatgaacgccgccgcacggcaactcgagaccctcggcggccgcatcgcggcgctgcaagaaggcggtggcggctcggtcaccgcgctgtcgaacgaggcccgcaccagcatggacttgctcggcgccctgcccccgcgctacggtgaggtgctgctgaacctgctcgaccggctcgaatcgagcgcgctgttcagcgaggagagttgctcgttcagccagaaagacctgctcgacaacctgcaggtgtgggtcgacaaggcccgcgcgcagttggcgtcctgaggagaccccgcatgcaaagacgcacccttcttcagcgcgcagccccggtgctggcgctcgcatccacggcggcatggccgctggccgcatcggccgccgcgccgatggtcgagatctggaaagacccgaactgcgggtgctgccaggattgggtgaagcacctgaacgcgaacggcttcgcaacccgcgtgcacgacgacggcaacgatgcggcgcgcgcccggctcggcgttccggccaagctgggctcgtgccacaccggcatggtcggcggctatgccctcgaaggccacgtgcccgcacgcgaggtgcgccgtctgctgcaggaaaagccgaaagccatcggccttgccgtgccgggcatgccggtcggctcgcccggcatggacggcgccgcctacggaaaccggcgcgacccctacgacgttctgctggtgctggccgacggcggcacccgcgtctaccagagctaccgctgaaccggaaacgaaaccggccggtcgtcagctgaagcgggcgggatcgaacggggcaagcgccgtttctggcacggtgccggcgagcaattgcgccgcgagcttgccggtgcgcgccgagccgcaaaggccgacgtggccatgcccgaaggccagcacgacgtccgtgctggccgccgccgcgccgatgcaaggcagcccatcgggcaggctgggccggtggccgagccagtgcttcacggcgatcgaatccggcgcctgatcaagtagcgctggaaacatcgattgcagatggcggtgcaggatctccgcgcggcgccagtcgggcgcggcctcgagtccgccgatctcgacctgcccggccgcgcgcaggccgccgtccatccagtgcgcgatgagcttgccgtcggccaccatggtcggtgtgcgcggccccacggcagccccttcgaccaccacgtggtagccgcgctccgattcgagcggcaccggcgagccggccgccgcggcaagggggcccgagcgcgcgcccgcgcagatggcggccgcgtcgcaggcgatctcgccggcctccgtttgcaccgcgcgcaaccttccgtcttcgatgcgaaagcccgtggcgcgcgccgccacgcgctctgccccggcctcctgcgcatgtcgcgccagcgcggccacgtaggcgccagggttgcggcagtggccggcctcgggcacgaagatgccgagcgtgtagcgcgcgtcgaggtcgggctcgcgctgccgcagttccggctccggccattcgtcccactgcacgccggtgcgccggcgcacgcgccagccgagcgcgtcgccgtcgaactcttcgcgcgaacggtacgcatgcagcagcccgcgctgctcgatgagttgcggcacgccggcctcggcggcgagccgggcatgcagggccggcgcatcggcaagcagcgtgcgcagtgcgtcggccgtgcgctgcacgcgcgcctcggtccagcccgaggccaggtagcgcagcagccagggcaaggcccgcggcaggtagcgccaacgcagcgcgagcggccccagcggatcggccagccagccgggcaccttgcgccaggcaccgggcagcgcgggcggcaccacggaatgcgacgacaaccaacccgcattgccgtagctcgtggcctgcgggccgccgggctcgccgggttccaccaccgtcacgcgcaggccggcgcgcaaggcctcgatggccgtcgcgctgcccacggcgcccgcgccgatcacgaccgcgtggcgtccggtgccgcccgcggagaaacttcttgcaactgtcatggggacctatcgtagagggcacggtcccataatcggccgccatgcctgttccctcttctcttgcgccgtcttcaggcgccatcaccgacgttgccggcatcgaagtcggccatttttctgacacgcgccggcccaccggctgcaccgtgatccttgcccgcgaaggcgccgtggcgggcgtcgacgtgcgcggcgccgcgcccgggacgcgcgaaaccgacctgctttcccccggcaacctggtgcagcaggtgcacggcatcatgctggcgggcggcagcgcctggggcctggccacggccgagggcgcgatgcgctggctcgaggaacggaacatcggcatggacgtgcgcttcggcatcttgcccatcgtgccggccgccgtgctgttcgacctgcccatgggcgacgcgcgcatccgccccgacgccgcagccggctatgcggcctgcgaagcggcaagccatgaagctccggccgaaggcaacgtgggcgccggcagcggcgcactcgtgggcaagctcttcggcgtgcatcgcgcgatgaagggcggcatcggcacggcgtcggtcaccgtgggcggcgtgacggtgggcgcgctgatcgcggtcaattcgctcggcgacgtgatcgaccccgacaccgcgctgccggtggccggtgcgcgcaccgaagacggcctggcactgctcgacacccgccgcgccctgctgcgcggcgagcagcccaagccgctgcttgcgggcaccaacaccacgctcggcgtgatcgcgaccgacgcggtgctgacgaaggtgcaggccaaccgcctcgccagcgtggcacacgacggcctcgcgcgcgccatcaatccggtgcacacgatgagcgacggcgacacgctgttcgcgctggccaccggccgggtgccgctcgagggcaacgcccccggcatgaccgtgctcggcaccatggcggccgaagcggtggcgcgcgccaccttgcgcgccgtgctggcggcgcgttccgtcaccgtgggcgagttgcacgtgccgtgcgcggccgacatcgccgcaacgaaaggttgagcaccccatggccatgcccaagacgctgaagctgatcctgctctcgatccgcgacctgatcgcctcggcgggcccgatcgtgttcctcgtgatcggcctgctgattgccgcctactggtggctgcagccgcagccgcccaggcatgtgacgctggccaccggccccagcggcagcgcctattcgcaattcggcaagcgctatgccgagctgctcaagagcagcggcatcgaggtggagctcaaggccaccaccgggtcgtccgagaacctggaactgcttcgcagcggcggcgccgacgtgggctttgtgcgcggcggcagcgccgatccggtggccgacgaggaagccggcctcacgtccctcggcagcctgttcttcgagccgatctggctcttctaccgcgccgacagcgcgcagaagatcgaccgcaagacaagcaccctgacctcgctcgcccagctgcgcggcttgcgcgtgaacgtcgacctggcgggcagcggcctgcccgagatcatggagcggctcttcaaggccaaccacctcgaccccgacgcgctgcagctttccaacctcgagcaggcggccgccgccgaagcgctgcaggccggcctgctcgacgccatcgtgctggcctcggcgccacagtcgccgcaggtgcagcgcctgctgcgcgcgcccgacatcaagctcatggacttcggccaggccgatgcctacacgcggcgctttccgttcctctcggcggtcacgctgccgcgcggcgtggtcgacctgtcgagggacctgccgccctccgacgtatcgctgctcgcggccaccacctcgctgctctcgcgcgacgagacccactcggcactgcggcagctctttgcgcaggccgcgcaaggcgtgcacagcgacgccggctggttcaaccgcgcgcgcgacttccccaacacgcgcaccagcgaactgcccgtgagccccgagggcgaccgcgcgatcaacggcacgccgccgttctggcagcgctacctgccgttctgggccagcaacctgatcgagcgcatgtggctggtgctcggcggccttctggtgctgatgctgccgctgagccgcgtggtgccgccgctctaccagttccgcgtgcgacggcgcgtgttccgctggtatgcgcggctgcgcgacatcgaggccaaggtggatgcgcggcaaggcgagcgcaaggagttgctcgacgaactcgacgagctcgaccgcgtggtgaacaaggtggccgttccactgtcgtatgccgacgagctctatgcgctgcgcaacaacatccacacggtgcaaaagcgcgtgcagatccgctggccggaaccgggcgacttcgcgccccgaacgccgctgccgaaggaagccgcagaaagcgcttgacttcgagcgcgctccaacttcgagaattcccgccatggaagccagcttgaccattgcggaagtcgcacagcgcaccggcctcacggcccacacgctgcgctactacgagcgcatcgggctgatcgccgcggtgcctcgggcaccgggcgggcagcgccgttacgcaagcgccgacatggactggctggccttcctgttgcgcctgcgcgagaccggcatgcccatccaggggatgcaggccttcgccaggcttcgaagccagggggacgccagtgtcggggagcggcgcaagatgctcgaacagcaccttgccgaggtccaggccaaggtggcggcgctgcagcaatccatgcgggcgctgtcgctgaagatcgagcactaccgtgccatcgacaagaagcgtccctcgtcaccgggcactgccccggaaaggaagacgagcgatgacgaacgcacacgcaagccagaacggcaaagacaacctgcgctacgagcgcgggctggccaagctccagcaaatcgacggtgaaggcggcatcaaggtcgtcgaaagcctggccggcatcgcgccggatttcgcccgcctgctgatcgagtttccgttcggcgacatctactcgcgccccgggctcgacctgcgttcacgcgagatcgcggtggtggccgccctcacggccatgggcaatgccgcgccgcagctcaaggtgcatatccagggtgcgctcaatgtgggcgtcacgcgcaccgagatcgtcgagaccatcatgcagatggccgtgtacgcgggctttccggcggcactcaacggcctggcggcggcgcgcgaggtgtttgccgcggacgtcccgctgctgggggagcccgcatgaagcagcgcagttttcgcgtccgtatgccgctgctcgggctggcgctgcttgcgactgcgatgaatacgcccgcctcggcgcaaacgcccgacctgccgacctggacgctggagaaacgcgccgtgcatgacgacctctcctcgccggtcggcatggcctacgacgcggcgggccatctctatgtcgccaactggtcggccggcaccgtgctgcgctttgcgccggacggtgcccgctcggtgttcgcatcgggcttgagcggacccagcgggctggcgatcggccctggcccttccggcgacatcttcgtcgcgtcctacagccaggacctggtgtggcgcttcacgccgggcggcaggcagagcgtgttcgtgcgcggcctggcaacgccggcgggcctgagcttcgatcgcaagggccggctgctgattgccaaccgccgaaccaaccagatcctcgcggcgcatcccgacggccggatcgaagtcgctgcggagggattgcaaacaccggtcggcgcggtcgaactgccgggcggcgagctgatggtcagcaacatcgcgggcggtatctcgctggtcgggcaggacgggcgcgcgcgaagcatccacggcgaactgcgcagcccaggcccgggcatcgtcgcggaccgcgacggcgcggccgcctatgtggtcgactacggcggaacgaccgtcagccgcatcgaccgcgagggaggccgcgtcgtggtagccgatggtctctcaagcccggtcgggctcgcccgcatgcccgacggaaacctgctggttgccacctggggtgcgaatgcggcctttcggctggtgcgggcgcgctgagacgccggcttgcccttgcccgccccatgaaaaaagcgcgcggccccttgcggaaccacgcgctcttgtcgaagcaccctgaggtctcttccagaaacaccgaggaaccggctttgccgggcctccggtgttgcccccggtagggggttggcgaagcgacacgaagtgcgcgaagactgggggcgagcctatttcagagccttgtagcgcatgcgcttgggcttggcgccctcttcgcccaggcgcttcttcttgtcggcttcgtactcctggtagttgccgtcgaagaaggtccactggctgtcgccttcggccgcgaggatgtgcgtggcaatgcggtcgaggaaccagcggtcgtggctgatgaccatgaccgtgccggcgaattcgagcagcgcgtcttcgagcgcacgcagcgtttcgacgtcgaggtcgttcgacggttcgtccagcagcagcacgttgccgcctgcaatcagcgtcttggccaggtgcagccggccgcgctcgccgcccgacagcgtgccgaccttcttctgctggtcggcgccattgaagttgaagcggcctgcatacgcacggctggccatctggaacttgccgacattgatgatgtccaggccgttggagatgtcttcccacacggtcttgttgttggccagctcgtcgcggtgctggtcgacgaaggccatcttgaccgtcgagccgatgacgacttcgccggtgtccggcttttccttgcccgcgagcagcttgaagagcgtcgacttgccggcgccgttcgggccgatgatgccgacgatcgcgcccggcggcacggtgaagctcaggttgtcgatcagcatgcggtcgccgaaggacttgctgacaccgtggaactcgaacacctgctggcccagccgctccgccaccggaatgaagatctcctgcgtctcgttgcgcttctggtattccatgtcgctcagctcttcgaagcgggccaggcgggatttgctcttggcctggcgtgccttcgggttctggcgcgaccactccagttccttcttcagcgccttggcgtgggcttcttcgctcttttgctcctgcgccaggcgttcgcccttctgctcgagccaggtgctgtagttgcccttccagggaatgccgcgaccgcggtccatttccaggatccactcggccgcgttgtcgaggaagtagcgatcgtgggtgatggccaccacggtgcccgtgaatcgctgcaggaacacttcgagccactccaccgattcggcgtccaggtggttggtcggctcatcgagcagcagcatgtcgggcttggacagcaagaggcggcacagcgccacgcgccgcttttcgccgcctgacaagaggccgatcttcgcgtcccacggcggaaggcgcagtgcgtcggcggcgatttccagttggtgttcggaatcggtgccggcggtggcgatgatggcttcgagctgggcttgctcggccgccagcgcgtcgaagtcggcgtcttcggcaccataggcgatgtacacctcttcgaggcgcgccttggccgcaaacaccgcgcccatggactcttcgaccgattcgcgcaccgtgtgctcgttgttgagcttgggttcctgctccagatagccgatcgtcatcccgggcatgggcagtgcctcgccctcgaactccttgtccacacccgccatgatcttgagcagcgtggacttgcccgagccgttcaggccgagcacgccgatcttggcgccggggaagaaagagagcgaaatgtctttcaagagctgccgcttgggcggcacggtcttgctgacgcggttcatcgaatagacgtattgagccatctgggggtagttaccttgggtagcggagattcgggacaagcgcgggcgcccgaaagcgggattcgggcgcggcaaaccacacattatcgactcatgcgacaataggcaccgttgccgggtccagttgcccgcaacaccggctctctgccggggacgaagaaagccctttatcacgacgggtttttcggctcccacccctgaccttcatcagccttgactggctcggcgttgccaaaaacgccaagcgggccgatgccactgcgccgtgtatggcgcttattgtttccaatgaattttgacgaactgaagctggctcccgccatcttgaaggctgtgcacgagcacggttacgacacccccacccccatccaggcgcaagccattcccgcggttctcgacgggcacgacctgctcggcggcgcccagaccggcaccggcaagacggccgccttcacgctgccgatgctgcacaagctcagcacgggcgcgagcgccaccaacaagttcggcggcatcggcattcgtgccctggtgctcacgcccacgcgcgaactcgcggcccaggtcgaagagtcggtccgcacctacggcaagtacctggagctcgactccactgtgatcttcggtggcgtgggcatgaatccgcagatcagcaagctcaagaagggtgtcgacatcctcgtggccacccccggccgcctgctcgacctgcagcagcaaggcatgctcgacctgagccaggtccagatgctgatcctggacgaagccgaccgcatgctcgacatgggcttcatccacgacgtgaagaagatcctcgcgctggtgcccagggaaaagcagagcctgctgttctcggccaccttcagcgacgagatccgcgacctggccgccacgctgctcaagaacccgcaaagcatccaggtgacgccgcgcaacaccaccgtgcagcgcatcacccaggtgatccaccccgtgggccgcggcaagaagaaggcgctgctcgcgcacatcatcaacgagaacaagtggagccaggtgctcgtgttcacgcgcaccaagttcggcgccaacagcgtggccgagttcctcaccaagaacggcatcgaggcgatggcgctgcacggcaacaagagccagagcgcgcgtacgcaagcgctggccggcttcaagagcggcgacatccgtgcgctggtggccaccgacatcgcggcccgcggcatcgacatcgacgagctgccgcacgtcgtgaactacgaaatcccgaacgtcagcgaagactacgtgcaccgtatcggccgcaccggccgcgccggttcgagcggcgaggccgtgagcttcgtctgcctggacgaagaaggcttcatgcaggaaatcgaacgcttcacgaagcagacgattccggtgcagttcgtcgaaggcttcggccccgaagacggcgagcgcgccgagccgatcgccatgggtcgccagacgatctggggcggcgccggccgtccgccgagccgcgacgtgatgcaggcggccgccaaggccgcccgcaccgaaatgctgcaacgcattcgcgagaacaaggccggccagggcggcggcgaacgcgctggcggtggtggtggtggcggcaacggcggcggtcaacgccgcggtggcggccagggcggtggcggtcaaggccgcaacgccaatggtggcggccaaggccagggccagggcccgcgtggccagggtgcccgtccggcacaaggccgcggaccgcaaggcccggcacgcacgccgcaccatgcgccccagcatcatcagaatcacctgccgcatgacgagcgccagccgcgccatcacggcaacagccacagcccgacgcaagccaaccaggtcgcgcacctgcgtgctgaagctgtcgcaggcggtgatggccagccggatccgttgcgcacgagcgtcgaccacatgggtggcggtcgcggacgcggccgtccgggcggcggcggtggtggcggctacggcggcaaccgttcgggcggcggtggtggttacggcggcggtggtggcggtggtaatcgctccggcggtggcggtggcggtggcggtggcggccgatcgttcggtcgttaagcggaaccgtgggtagaacacctacccgcaaatgaacaagggcacttcggtgccctttgttttttccgggctttcagcgcggcggcgccgtgctcgccctgatgtgcaccgtgtcgcttcagagcttcccgctgtcggcggggttgtgcacgatctggatcagcacgtcgggcgtataggccctggtgcgcgagatctcggcaatttctccgcctgcggtgccggcgaagaccagcacgccctgccctttgtaggcaaggtagtggcgccaccgatctgtgccgttgtaggtgggaatccaggccttgcctgtgttccggaccgtttcggcgttgggcttacccgcgatcttgatgacttccgcgtagctcatgctgggccgaagctgcgcgaagggggtgccgggcaacggctggccgactgcggtgcgctcttcgtcttcttgcgccgtgaccagcgctcgccggctgggctcgtacaaaggggcagattggcaggcggccagcgcaacgcacgccagcaagacagcagagatcgaccgaatcttcatctttgttttctcccgttgaaatttggcgcggacctgagagcccgccagcacggatgaaaagtccgcagcatcgaattgtcgttttacaagtcccgacacaatcgttgccagggtgcgaatccggcgcatttatcgcgtttttgtcaactgctccacacaaccgcattaacgatggttttgcctattagtaccaaaggcgtctcccagcgtggcacagcgccggacacaatcgcgagccatgcaatacatcccgcccaactacgccacgctcttcgtcgccacctgcaacctgctgaatctcgcgaatcctcatcgcgtgttctacgagaaccaggacccgtacgacgagcgcgaatacgagcgcaagatcgactggatcggcgagcgctttcgtgcgctcaatgccgacgtgctcgcggtgcaggaggtctgggatgaaagcgcgctcagagctgccattgcgcgcagcggcttgcgctacgacttcgtcgcggtgccgggtgccgagaacacgccgccgcacaacggcgcagagggcacgccgcgggtcggcattgccacgcggctgcaggtggaccgcgtgcaatcgttcgtcgactttccgcccggcttcggggtcgaggtgccgggcctcggcccgcacacgcgcttcgagcgcccgccgtttctggtcacgctgcgaatgaagcacggccagcaggtgcacatgctcacggtgcacctcaagtcgaagcggcccaagttcctgcaggacgcgcaaggcaacgcactggaagaccgcgaggaccggaaagtcggcgtgatggcgtctctgcgctcgctcgtcatgcgcggcgccgaggcagccgccctgcgctgcatcgtgctcgatctgctgcagggcacgaacacgccgctggtggtgatgggcgacttcaacgacgacccgcacagcgtcaccacgcaactggtggccgccacctccgaagtggcctacgacaaggccgcgcgcgacgtggcgctcttcaacgcctatgagatgcagggcgagtcggcactgaagaaagacgtcgcctactcgcacatccaccagggctttccggccgtgctcgaccagatcttcgtgagcgaagagttcgtggccacgagccgcaacagcctgggcgacgtgcgccgggtcgactatttcaacgaccacctgcacgaagggcgcgaccgctcgcgctcggaccacggctttgtgcgcgccctgctccggctgcgcacagactgagccgaaagtcgaaaaaagctcagggcatgcgccggccgctctgtcggtcgaacaggtgcacgcggtcggtgtcgatggccaggcccacggtctggtcgggcatcgcatcgacgcggccgtgcaccgccagcaccagcttggcctcgcccacctgcaccaacagttcggtctcggcgcccgtgggctcgaccacgatcacctgtgcattgacgccgctgccgccgcccagcgtgatgtcgccggggcggatgccgtagtgcaccggctggccgtcgggtgccgaggtgcccgctggcacgggccagcgcgcgccatgcgcctcgacccagcagtccgcgcctgagcgccgcacggtgccgtcgatcacgttcatggacggcgagccgatgaattgcgcgacgaacaggttgtcggggcggtcgtacaggtcgagcggcgtgccgatctgctcaacgatgccgtcgtgcatcaccacgatgcggtcggccatggtcatggcctcgatctggtcgtgcgtcacgtagacggtggtggtcttcaggcgctggtgcagcgccttgatctcggcgcgcatcgccacgcgcagcttggcgtcgagattggagagcggctcgtcgaacaagaacaccttcgggtcacgcacgatggcgcgccccatggccacgcgctggcgctggccgcccgacagctcgcgcggatagcgtccgagcagcgcatcgaggttgaggatcttcgcggcccgcgacacgcgctcgtcggtcaccgacttctcggcgttgcgcaaacgcaggctgaagcccatgttctcgcccaccgtcatgtgcggatagagcgcatagctctggaacaccatggcgatgtcgcggtccttcgactcgaggtcgttgaccacgcggctgtcgatcatgatctcgccgccgctgatgtcttcaaggcccgcgagcatgcgcaacaaggtcgacttgccgcagcccgaaggcccgaccagcaccacgaactcgccgtcggtgatgtcgaagctcaggccctggatgatctggaccttgccgaaggatttctggatattgcgaaaggatacggaagccatttttattcccagggttcgctcaactcttgacggcaccggcggtgagtccgcccaccatgtagcgcttgaaggcgtaatagatcgccgcgggcggcaatgcgtagatgaggccggtggccatcagcagctcccacggcgaatcgtcggccgagaggaagttgccgagcgccaccgccagcgtcacgctcctgtcgttggacagcagcaggaaggcgtagaggtactcgttccacgccagcagcagcgaatacgtgcccaccgccaccagcgacggcaccatgagcggcaggtacaccaggcggaacagctgcagcggcgaagcgccgtccatgcgcgcggcctcgtcgagctcgtagggcagcttgtccgacgcctgcttcagcacccagatgcagtacggcgaggcgatggtcaccatcgcgaggatcagcgcccactggctgttgagcaggccatagttgcccatggtcttgtacatcggcaccgcgaggaaggccgccggaatgaagtaggtgaagagcgccaggttcatcaccgtgcgaccaccgcgcacgcgcagccggctgatcgcgaacgcggccgtggtcgcgacgaacagcgtgagcacgccgaccgacagcgcgatcagcagcgaattcaagagctgcagccagaagtggtcgaggtagaagtgcttctgctggaacacgatgcggaagttgtccagcgtcgcgttcttgggccacaggtggcccgaggtcgcggagtccttcgacgagatcgcgaagagcaccatgtggtagacggggatcagcgtccacagcagcaccggaatgccgatcagcagcagcttggcctcggtcgctatggccttgggggtccagcgtttcatttcgagagcctcttcatcatgaagtagacgagtggcaggacgagagggagagccaccacgatcgatgccatcgacaggtcgacctggtcgagccgcagatagcggatgcccagcgttgcgagcacgtgcgtcaggtcggcaggtccgccgccggtcagaaggtagacgctgttgaagtcgcccagcgtccagatcatcgaaagaatgagagacgtgacgtagagcgtcttcagcgcgggccagctcacgaagcggaatttctgccacgacgaggcaccgtcgaccgacgcggcttcatactgctcggtcggaatggccagccgccccgccaccaggatcagcgtccagaacggcagcgacttccatatatgcacgaccatcgccaaggacagtgccagcgaaggatcgttgagccaattgggaccatccgcgccggtcaggcggaagatggtgctgttgatcacgccccactcggggttgagcatgaagcggatcgacaggatggtgggaatcgacggcatcgcccacggcaggatgaagatcgccgaaatgatcttgatccaccagcgcgatgtcacgaagaagcccgagagcacaagggccacgagcatcttgatgttgatggccacgaccaggaagatggccgtgttgatcaccgagcggaagaagatcgggtcgtcgaccagcttcacgtagctttgcggatggcgcgcgagccacagcccgtaccccacagggtagagcacgaaaaccacgaacaccagcaggtagggcacgaccatgaccgcgccccagaactgccagcgcgcgtgccgcgccccaagattgacggtaggcgccgggagcggcgcggcggtggcagtggagctcatgcgagtcagcccggtgaacgtggttttcgaagaatgcggcttactgcgccgcgaccgtcttgatgcgcgcgatcatctcgtcgaccgccttgtccaccggcaccttgtcggtgacgacgcggctcatggccttggcccagacgttctcgttgttgagcacggtgaacttgtagttcttggtgaactcgaaagtcacggtgccggcggcgtactggttgaagaccgagaggcggtgcggatcggccttccagaagtcacgctgctgcgcagccttggtcaccgggaaccagcggcccagcgaaccctcgacgtacggcgtgaggttttcttcctgcagcaggaaggcgacgaactccttggcgcgggccttgttcttggcgtccttgaacaccacgccggtcttcaccgcgctgcggtagaccatcttgctgccgtccggcttgcttgggaaacccgccgtgcggatgcgctcggtgtagttcttgcgcgcttcctcgcgctgctctggcgtgagagtcgcgttgttcgaatcgtcgagccacttggcggcgatggagatggtcgcgttgtgcgtcatcagcgtcgtcttgttgtggaacgcgacgttgttgtccgggtccttccagctggtcgccgacggcggcgtgcagcccttggtgtagggcgtcgtgtagtcggtcagcgcgccgatcaggccggtgcggaccttcggatcatcgaccagcaacttgccgttgtcgtccaccagcttgacgttgtgcgcgtccatgaaggtcaggaacgaatagaacgagtcgctcgaatccacgcccatgggcatgccgatgccgaaggtgcgcttgccgctcttctggcggctggcggtttgcgccttctcgcaccagaaggtccagtagtccttccaggtggtgggaatgtcggtttccttgaggccggcttcggtgagcatgtcgagccagtactcgacgtgcatcgtctgctgcttgatcgggaaggcgtagtacgccttggtcttggtctgctcgttgtgcaggtacgtggtctccagcgtgttgggcgcgaagcggtccttcatgggcgcgagcacgctgctgaggtcttcgagcttgccgtcgtaggcccacttgcccgtgacctggaagtcgtacacgtcggcgtacgccacgtcgggcgggctgcccgagtcgagcgcggacacggtcttggggatcatgtcctggatcgggtactgcgagagttcgatcttcacgttcttgttcttgtcctcgaacttcttgatggctgcgaacaacgcatcgtcctcggccttgtagaagcccttgacccaccagacggtgagcttttcctgcgcggcagcggggcctgccgccgcaagcaaccccagtgcaaatagcgtcggcgctatcagcgatttgacgactttcatggtgtctcctcttcttcggtggaaatgctcgaaacacgagcgtggtgaaaaatccgttgcgacctgggccggccggctagctcgccttgagccgagggggtgggcggctgagccgcggcagccgccggcgcgaaccgagcacgtcctcgatgtcctgccgcgcgccgtcgatgaggcggatgaccgcacgctcggccttggccgggtcgtgcgcaatcaccgcatcgagcaccgcgcggtgcagcggcagcgaaagcgcgggaccgtcgggcttggcggtcgaaatctcgaaactggtgcgcagcagcgcgttgagcgccttgctcatctgcgccagcatgcggttgcgcgcggcgctcaacaggccgttgtgaaagcgcaggtcgaaggtgacgtagtcgccgccgttctccacggcctctttcatgccggcgtaggcgcgctctatctcttcgatgtcctccgggctggcacgttcggccgcgagccgcacggccgccggctcgaccacgcggcgcaaatcctgcagatcgcgcaggaactcgggcgtgagcccggcgcgcgactgccaggtgatgacatcggggtcgaaccaattccacttgtcctgcggcagcacacgcgtccccaccttcggcccggtgacgatcaggcccttggcggcgagcgacttgatggcctctcgcaccaccgtgcggctcacgcccagctcctcgcccaggatgggttcggccgggatcgacgcaccaatcgcataacggccggccacgacagcttcgccgagcagctcgagcgtgcgaccgtggatgttcttgatcatgtgcgtgatgtgaaatttgatatgccgacactcgaaaacactaagggtccggcaggttcttcgcacttatcatatgatgattgaaatggccgatcggcaggacaaaccctgaggtttggagtcgtaagcggtcgtaaacggagacaaccgatgagcacttccccgaagaaaaaagccagcgagctgcgcagccagcaatggttcggccgcaatgaccgagacggtttcatctaccgaagctgggtgaagggcaagggcgtgccgcacgaccagttcgacggtcgcccggtcatcggaatctgcaacaccttcagcgagctcacgccctgcaactcgcacttccgcacgctggccgagcaggtcaagatcggcgtgtacgaagcgggcggtttcccgctcgagttcccggtgatgtcgctcggcgaaacgctgctgcgtcccacggccatgctgtatcgcaacctcgcgagcatggacgtggaagaaagcattcgcggcaatccgctcgacggcgtggtgctgctcatgggctgcgacaagaccacgcccgcgctcatgatgggcgcggccagcgtcgacctgccgaccatcggcgtgtcgggcggccccatgctctcgggcaaatggcgcggccaggagctgggctctggcaccggcgtgtggcagatgagcgagcaggtgcgcgccggcacgctcaagctgcaagacttcttcgaggccgaaagctgcatgcaccgcagccacggccactgcatgacgatgggcaccgcgagcaccatggccagcatggtcgagtcgctgggcatcggcctgcccggcaatgcggcctatccggccgtggacgggcggcgcaacgtgctggcccgcatggccgggcggcgcatcgtcgacatggtgcatgaagacctccacatgtcgaagatcctcacacgcgaggccatcgagaacgccatcaaggtgaacgcggccatcggcggctccaccaacctggtcatccacctgctggccattgcggggcgcatcggcgtcgacctcaagctggacgacttcgaccgcctcgcctccgaactgccctgcctggtcgacctgcagccctcgggccgcttcctgatggaagacttctgctacgcgggcgggctgccggtggtcatcaaggagatcgcgcagttcctgcacaaggacgtcatcacggccaacggccagacgctgtgggacaacgtgaaggacgccgaaaactacaacccccaggtgatccgcccgctggccgagccgttcaaggaaaacgccggcatctgcgtgctgcgcggcaacctcgcgcccaacggcgccatcatcaagcccagcgccgccacgccggaactgctggtgcacaagggccgcgcggtggtgttcgagaacgccgacgacctgcaccagcgcatcgacgacgagaacctcgacatcgacgagcattgcatcatggtgctgaagaactgcggcccgcgcggctaccccggcatgtccgagtcgggcaacatgccgctgccccccaaggtgctgcgcaagggcatcaccgacatggtccgcatcagcgatgcacgcatgagcggcacggcctacggcaccgtggtgctgcacaccgcgcccgaggccgccgccggtggcccgctggcgctggtgcaggacggcgacatcgtcgagctcgacgtgcccaaccgcaggctgcacctgcacgtgagcgacgaagaactcgcgcgccgcctcgagaaatgggtcgcccccaaggcgccgctcgattccggctactggaagctctatgtcgacacggtgctgcaggccgaccagggcgccgacctggctttcctgcgcggccggcgcggtgctttcgttccaagggacaatcactagcactgggcatactccaggctttccccatggagtcgcattgacatgagcagattggtggcggtcgactggggcacgagctccttgcgcggcgcgctgctcgatgcccgcggcaaggtgctcgaggagcgcagcgatgcgcgcggcattctcaaggtgccggcgggcggctttcccgaggtgttcgagtcgctgttcgccgactggatgcagcccgcgggcacgcgctgcctgatctccggcatggccggcagcaagcagggctgggtcgaggcgccctattgcgcctgccctgccgggcgcgtcgaagtgggccgccggatcatcgacatcgacgtgcggccggattcgcgcatttccatcgtgccgggcctgcgcgacgagcacgacggcgttcccgatgtcatgcgcggcgaagaggtccagatcttcggcgccatggcgctcatggacgtcgacgaaggcgtcttcgtgctgccgggcacacacaacaagtgggtcacggtcaagaagggccgcgtcaagggctttcgcaccttcatgaccggggagttctatgcgttgctgagccagcactcgattcttgcgcgcacgctcgatgccgatgcaccgctcgacgaggccgccttcgtggagggcgtcacgcgttcggacaacggccagggcctgctgcacaacgccttcggcacgcgcacgctggcgctgttcgagcgcatgcccacggaggaactcgccagctatctctcgggcctcttgatcggcgaagaactgcgcacgcagtcgctgcatgcctccggcgaagtggtgctgatcggctcacccgcgctcacgcagcgctacacgctggcgctgcgcgccaccggcatcgccacgcgcacgatgggcgccgaagccacctgggccggactgcatgcgctgtccggttttctcgacacagacagaactccttcatgacgactccccaagaaaaattcaaggccgcgatgcgcgagctgccgctggtcgccatcctgcgcgggctcacgccgcccgaggcggccgacgtgggcgacgccatcgtcgagtccggcttccggctgctcgaagtgccgctcaattcgcccaagccctacgccagcatcacgctgatgcgcacgcgctttcccgaggccctggtgggtgccggcacggtgctcgacgtgcagcaggtgcgctatgtgcattcggccggcggcgagctgatcgtgtcgcccaacttcaatgccgaggtggtcgccgaagccgtgcggctgggcatggtctgcctgcccggcgtgatgacgccgaccgaagcctttggtgccctggccgcgggcgcgaccgggctcaagctgtttccggccgaactggcgtcgcccgcggtggtgaaagcattgcttgcggtgctgcccgccggcacgccgctgatgcccgtgggcggcatcacgcccaccaacatggccgaatggcgtgcggctggcgcgtccggcttcggcatcggctcggcgctctacaagcccggcaagcaggcgtccgacgtgcgtgccgatgccgagagattcgtcgccgcctgctcgggcgcaatccacgcctgataccccttcttcaccgttctcttcttttcacatccacgaggccccgtcgatgtccgcagattcagattacgccagccccgccgtgcgcaagttgcgcgaagacctttcgctcgcattgcgcgcggccgcccaccatggcctctcggaaggcgtctgcaaccacttcagcgtgatgctccccggcgcgcaagaccgctacctgatcaacccgcgcggcttgcactggagcgaaatcggccccgacgacatcgtgctgatcgacgtgcacggcgaagtgcttgccggccgccaccgggtggaaccgaccgcgctgttcatccatggcgcggtgcaccggctgaccggccacgcggtcgtgctgcactgccacatgccctacgccaccgcgctcacgctcacggccgatcgcgccctcgatcccacgctgagccagaacgcaatgcgctacatgaaccgcattgcgatcgacgcggtctacaacggcctggcgctcgacgatgccgagggtgaacgcatcgcgcgcgccatggaaggaaaggacgtggctttcctggccaatcacggcgtgatcgtggcgggcggcaccattgcacatgcctacgacgatctctactatctggaacgcgccagcctgcaccaggtgatcgcgcaatcgaccgggcgaccgctggttccggtcgatgcgaagctggccgcacttgccgctgtgcagatccagggcgaacgcgagcaatccgacctgttcttcgaggcgcttcggcgcatgctgccgcccccgccacacggctgacgtccgttcggccggtttcgcgtcggaattggggcgcctaggatggctgtcgtgtcttgcaatggccgcgcaccggcttacaggtcttcacccgatttcgcccaagccttacacagcgttcacatggagccacgacgatagggcttccaaccactccattggagttgccatgaaaaagctcactctcgcattcggcgccgcggccctgctgtcgctggcggcactcagcgcaacggcccaggcacagaccggcggccgcttcatccagacccaggtgtatgtggtgcccgcacccccgccgccgccgcgccatcactactacgcgccgccacccccgccgcaccactactacggcccgcgctacagcgaccatcaccgctacgagcatcggcatcgccactgggaagagcgtcgctacggccgcagggactatgacggggacggcgtacccaaccgctacgaccgccggcccgagaatccgtaccgctactgattttccagcagagcacgaggcccgggcctgtgcggcggcacatgccgccgcacagccgggcgaattgtcggcaggctttgtgtctggttcaggcttgcgccacgcgccgcaatagcccggcggtggtgcgcggccagcccacgcggccgaaccatgcaccgccggcaatcgccgccgcgatgaccacgccgtacaccgccagcgccacgccctgcgccgcaaagacgccggtcagcccgccgccccagcgaaaggcgagccaaccgccaatgcccgccacggaaagacgcgtgaggttgccgatcaccggccacagcaggcgccctgccccttgcgaggcgaaatacagcaccagcccgacaccgaagaagccatagaacggccccaccaggcgcagatagtgcgcgccggtgtcgagcatggcggggtcgctgccgaacagcagcagccagggccgcggaaacagcgcggccgccaggccaatgctttcggtgagcacgaatgcgatggccgcaccggcccaggtggcgcgcagcgcgcgttcacgctggccggcgcccatgcaggtaccgaccatcgcgaccagcggtgcgcccagcccgaacaccagcggcaccagcaggtattcgagcctcgacgcggtgccgtagccggccaatgcgcccgagccgaaatggccggtcaatgcggtggcaatgccgatcgacagattggtggccacggtcgcgaccgcggctaccaggccgacgcgcaggatgtcgcggaacagcggccagcgcagcttcagcgcggcgagcgtgggacgcagcaggctgcgcggcgaccgcaggtagacgatgagcgcgattgaccccagcaggtagtacagcagcagcgccatcgcgccgcccgcaatgcccatgcccggcagcggtccccagccgaagatcaaaagcggcgatgcgggaatgagaaacagcacgcccaccaccgtcacgttcgccggcaccgccatgttgccggtgccgcggatgatggccgagagcgaattgaagagccacaccagcaccgcgcccgcgaacacccagttcgaatacgtcagggccgcgtcgagcgcttcgccggtgccgcccatgatcgcgtagagccatcgcccgccggccagcagcgcgagggaaaagcacaggccaaagccgatcgcgatgaccaccgcatgccacaccagcgcatcggcatcgccgcggcggcgcgcgcccagcgcacgggcgatcgacgaggcaatgccgccgcccatggcgcccgccgaagtcatctgcatcagcatgacgatggggaacaccagtgccatgccggcaagcgcatgggtgcccagcttgccgacgaagtaggtttcgatgagcccgacggaggcctgcgccagcatcacgagcacgttgggcgcggccatgcgcagcagggtcgccacgatcggcgcctccagcagcatgcgcgtgcgcggatcgaggtctcggctcactgggtaacctccgcgctaggcgctgcggtattcgccttgggagcggcctgacggctcatgccgccgccaggttcgcgcgcgccagccgcgcttcgcggatcggcaggtgcaccagcgccgcgcccgcggcgagcgcgatgtcgatgtaccagacgatgtcgtagttgcccgtggcctggaaaacgtagccgcccaggtacgcgcccaggaagccgccgacctggtgcgccagcatcacgatgccgaacagcatcgccatgttggccggcccgaacatcttggcgacgaggccggcggtcggcggcacggtcgacaggaaggtcacgcccatcacggcggcgaacaccagcatgaccacggtcgtcttcggcgccagcaggaagaccagcacggcgatgccgcgcgtggcatagaccagagacagcagcgacttcatgcgccagcgccccaccgcccagcccatcgcaaggctgccgacgatgttgaagagcccgatcatcgcgagcgcccagccgccgacttcggccggcagcccgcaggccgcgacgacaccgggcaggtgcgtggcgaggaaggcgacgtggaagccgcagaccaggaagcccaggctcaggtagcggtagctcggtgtcgcgagcgcctggccgatggcctggcgcgcactcagcggcttcgtgcccgatgcggccgccgaggccgcagccatcgcgttcgaattgcccttgagtacccatgcggccggcaacgccagcagcaccagcacgccgagccactgcatggcgccggcccagcccacggctgccgtcaggccgacggcgatcggcgccatcgcgaactgtccgaaggagccgccggcgttgaccatgccggtggccaggccgcgtttctcggccggcaccaggcgcgtggtcgcggccatcagcaccgacggacccgccatgccagcgccaccggccgccagcacgccgatcgcgaagatcaggccggccgtgctcgtcatcagcggcgtgatcagggtgccgacggcgaccagcagcacgccgaggaacaccacgcggccggtgccgatgcggtcggccacggcgcccgcgaagggctgcgtgaggccccaccagagctgtccgaatgcgaacgccaggctgatgctgccgatgccgagcgcggtcgaggtgttgagtgccgagaggaacaggcccatcgtctgtcgcacccccatcgtgagcgcgaaggcgcccgcggccgccagcagcacgagccagagcgcatggcgccgcagagaggtttcattcatcgcgggctcctgtttggtcttccggctgtccatcgcccagccctgcgcgctgcaggagttccaggctctcgtcgagaagggcatgcagcgccagcacgcgctccgtgccgaggatgtcgttgagcgccagctgcgcgccgtgccagaggcgctgcgcctcggctcgcttctcgcggcctgcatcggtgatcgccagcatgcggctgcgcgcatcggggccctcggtctgcacgaggaagcccgccgccagcagaggcttgagattgcgcgtgagcgtggaggcgtcgacgttcatctcgcgcgccaggtcgaccgggcgcagcggcccgaaatgcagcacatgcgagagcagtgaatactgcgtggtcttgagcccgctgggcgcgacgtgcgtgtcatagaggcgcgacgccagcctggagagccggcgcaggcggaaattggtacatccttggggcctcagcagaggcttcagagcggtgatcatgccattcattgtagctacaataattgtacatacaactatcaaggagttttttccatgatcgagccccatgccatcgacgcctggatcgcccaggaggccgaggtcgtccaacgcctggacgcggggccgggccctggcctggcacgccccgagcagatcgccggcaagaccgggctggaaacgatggaagcgatgctgcgcgccgaaatcccctacgccgccatcgccaagaccctcgacttcgccctgctggaagtcagcccgggccgggccgtattccagggcaggccgcttgcgcagcacctgaatcccctgggcaccatccacggcggctgggttgccaccttgctcgattccgcgctgggctgctcggtccacaccatgatgccggtggggcgcgcctacacgaccgccgagctgagcgtgaactacgtgaagggcctcacgcccaaggtacagcgggttcgcgccgagggcaaggtgatccattgcggccggcagcttgccaccgccgaggcgcggctcttcgggcccgacggcacgctgtacgcgcacgccaccaccacttgcctggtgttcgaggttcccgcaccacgctgagccgccaccgccatgtcttccactccccacgacccctcgctcgcaccggcgttcaaggcccttctcgaccagcgctacagctgccggggctaccttgccgatccggtgccgcgccaaacgatcgatgccatcctgcagctggcgcagcgcaccgcgtcgtggtgcaactcgcagccatggcaggtgatcgtgagcagcgccgcggccaccgagcgcctgcgccaggccttcgactcggacgaagccgcggtcgatgcccagttcgacattgcgccgcccgccgactaccgcggcgtgtaccgcgaacgccgccgcgaatgcgggttccagctgtacgagagcgtcggcatcgcgcgcggcgaccgcgaggcttcggaaaggcaggcgcgggagaacttcaggttcttcggcgcgccgcacctggccctcgtcaccacagaagcgctgctcggcacgtatggcgcggtggactgcggcgcctacgtcaacaacttcgtgctggcggcccgcagcttcggcgtggccagcatcgcccaggcggccgtggcctcccgctcgaaattcctgcatcgctggttcgagattccggacgaccgccaggtggtgtgcggcatcgcattcggctacgaggacccctcgcatccggccaatcgcttccgtacggcgcgcgcgccgctggagcaggtttgccgctgggtggattgagcgtcgatcccgtcgttcggaattccttcaccgtgtaagtgcaaggacgtaaaaaaccacccaaagggcagtgataatgattctcatcgtcagccgcgtggctgcgatgctttttcaaaacacgtctctgcacctggaggatccttcatgaccgaccgcttcggcgtccaaggccgcgccgcccgcgcactgatcggcgtctccgccgcctggctggccgctgccgccctgcccgcctatgccgccaacgacgaactcacgctctacacgacgcgcgagcccgcgttgatccagccgctgatctcggccttcagcacgcagagcaacatcaaggtcaacaccgtgttcgtgaaggacggcctgctggagcgcgtcaaggccgagggcgcgcgctctccagccgacgtgctgatgacggtggacatcggcaacctgatggacctggtcgatggcggcgtgacgcagccggtgaagtcggccgcgctcgaatcggccgtgcccgccaacctgcgcggcaccgacgggcagtggtttgcgctctcgctgcgcgcgcgcgtgctctacgccgacaagaaccagccgctcaccagcttccgctatgaagacctggccaatccgaagtggaagggcaaggtctgcatccgcgccggccagcatccctacaacacggcgctggtcgcggcaatgatcgcgcacgacggcgaggccaagaccgaacaatggctgcgcggcgtcaaggccaacctggcccgcaaggccacgggcggcgaccgcgacgtggcgcgcgacatcctcggtggcatctgcgacgtcggcctggccaattcctactacgtcggccagatgaagagctccaaggaaggcaccgacgcgcgcaagtggggcgatgcgatcaaggtcgttcgcccgaccttcgccagcgccaagagcggcggcacccacgtcaacatcagcggcgcggccgtggccaagaacgcgccgcagcgtgccaatgcggtcaagctgctcgagttcctggtgtcggagccggcgcagtctctctatgcgcaagccaactacgagtacccggtgcgcaagggcgtggcgctcgacccgatcatcggcgagaccatcggcgagctgaaggtcgatccgctgccgctcaccgagattgccaagtaccgcaagcaggccagcgccctggtcgacaaggtcggcttcgatcagtgatcgacatggccgggcacgcgtccccggtgcctgaatgctgatcgcgcggcgccatttgccgggcctgcacgcggcaggcccgctctggcgctcggcctcgttcgcgatcgcggtcggcgtgcttgcgccggtgctcacgctggcgtggctggcgttcggctccggcgtggggcactgggggccgctgttcgcgcacgtgctgccgcgggccgcgctcaacacggccgtgctgctggcgggcgtcggaacgctggtgctggtgatcggcaccggctgcgcctggctggtcacggcctgcgactttccgggccggcgcgtgctgcactgggccctgctgctgccgctcgcaatgccgacctacatcgtcgcttttgcctacctcgatctgctgcacccgatcggcccggtgcagggcgcgatccgctgggcactgggcttcgacagcccgcgacagttccgcctgcccgacctgcgctcgatgccgggcgcgatcttcgtgctcggcttcgtgctctacccctacgtctacatgaccgcgcgcgccatgttcatgacgcagcccgcgcacctgatggaggccgcccgcaccttgggcgaaagccggcgcggcgcgttctttcgcgtggcgctgccgctggcacggccggcgcttgccgtgggcctcagcctcgcgctgctcgagacgctgaacgacatcggcgcctcggaattcctgggcatcaatacgctcacggtcgcggtctacaccacttggatcacacgctccgacctggccggcgcggcgcagatcgcctgcgccatgctgttcgtcgtggtcgcgctggtctggctcgaacgcaatggccgccagcaccagcgcttcggttcggcgcagcgcatgcgcgccatgcagccgcgccgcctgcacggcggtgccgcatggctcgccaccgccatcgccacgctgccggtgctgatcggcttcgtggcgccggccctctacctggtctgggagagcgccaagcggctgcaccagggcggcggcgtatcgcacggcctgctcgcaagcctcggcaacacgctggccctggccgccggcgtgacgctggtggcggtggccgcgggattggtggtcgcatgggcggcgcgcagccagggctcgcgccccaaccgcgcgcgctggcaggcacgcgcggccacgctgggctatgcggtgccgggtacggtgctcgccatcgggctgctcacgccggcgcttgcgttcgacgcggcgctggccaatctgctcggcctgcagggcctgccgctcatgggtgcgggcatcgtgctggtgatcgcctgcgcgatccgtttcctcgccatgccggtcggcggtatcgaagccgggctggcgcgcattccgcccgccatcgaacaggcctcgcggctgctgggcgagaccagcggcggcacgctgcggcgcgtgcatctgccgcttctgcagcccgcgattgcgaccggcgcgctgctggtctttgtcgacgccatgaaggagctgcccgccacgttgctgctgcggcccgccaatttcgacaccctggccacctggctctatgccgaggccgcccgcggcacgtatgaagaaggcgccattgccgcactcgccatcgtcgcggtgggcctgctgccggtgatgctgctggcgcgcaatcaactgggcacgccatcggccctgcccggtccggacaagacatgagttcccctctttccatcgaatcgatccagctcgcctacgaaacaccgcgcggcctgcacaccgtggtgagcgacttctcactctcgctgcccgcgggtgaaatcgcatgcctcttcgggccttcggggtgcggcaagaccacggtgctgcgcgcgattgcgggcttcgagccgctgcgcgccggcaccatccggcttggcgacgtgctgctctcttcgacagacgtgcacctgccgcccgagcaacggcgcgtgggcatgatgttccaggaatacgcgctgtttcctcatctgtcggcgggccagaacgtggccttcggattgcgccattcgagccgtgcgctgcagcgggcgcgcgtggccgaaatgctggcgctggtcggcctggccgatgccggcgagcgctttccgcacgagttgtcgggcggccagcagcagcgcattgcgctggcccgcgcgctggcaccgtcgcccgcgctgctgttgctcgacgagccgttttcgaacctcgacggcggcacgcgcgagcgcctgacggcggaggtacgcggcatcctcaagcgcgccggccagaccgccatcctggtcacccacaacgaggccgaggcccatgccatggccgaccgtgtcggggtgatgcacgggggccggatcacgcactggctggataccgctcaatagcacaaggcgcccatttggcgaatgggcttttcgggaaaaggttgttcgaggccgcaagaatcgcggcgcactcccttcactttttcttcagcaaacgcaatcgccatgtccaagccactcaccctcgtcagtcacctgctgtgcccttatgtacagcgcgcggccatcgccctggccgagaagaacgtgccgttcgaacgcgtcgtgatcgaccttgccaacaagcccgattggttcgtcgcgatctcgccgctcggcaaggtgccgctgctgcggttggcgcggcccgaccgcagcgaagcggtgctgttcgagagcaacgtgatctgcgagtacctcgaagaaacgcagccagggccgcgcctgcatcccgaagatccgctcacccgcgccgagcaccgtgcgtggatggaatttggctcggccatcctcggcgacctgtggggctatgaaaccacgcgcgacgcggaagtgttcgaacagaaacgcctagcgctggccgccaagttcgagcgcatcgaagtcgcgctgggcgcggggcccttcttcgcgggcgtccacttcagcctggtggacgctgtcttcgcaccgatctttcgctacttcgaagtgttcgacgagatccgcaactcgcacatcttcgatgccttgccgaaggtggacgcatggcggcgcgcgctggcggcacggcccagcgtacagagcgccgtggtgccggagtatccgcagcacctgcgcgagtttctgcgcaagcacgaggcgcacttgctcgagctcgcgcaataacgaaaatcggccttctttcccaccacgacagacaccacgagatgcgactcctccacaccatgctgcgcgtcggcaacctccagcgttcgatcgacttctacacccaggtgctgggcatgaacctgctgcgtatctcggagaaccccgagtacaaatacagcctcgccttcctcggctacggcaacggcaaccccgaccaggccgagatcgagctcacctacaactggggcaccgaaagctacgagctcggcaccgcctacggccacatcgcgcttggcgtgcctgacgcctatgcagcctgcgagaagatcaaggccgccggcggcaaggtcacgcgcgaagccgggcccgtgaaaggcggcaccacggtgatcgccttcgtgaccgatcccgatggctacaaggtcgagttgatacaagacaaatcgaaggcccagggcacgcccgggtccggcgccgacgccctgcgcgcctcctagccggccgctgcggcctgcggccgcctcctcgcccggacaaagcggccccagggagggggccgtttaaaatgaaggtgcggcgaattgaagatacaaatgatcaccttttcgcaggcgatcggcatattctttgctggtattttctctgggtacgccggtggcgctaaatgccccacgcgccgttacctcaaatcgcaatcaagcacctttacagttcggcaaggccgtccattcggatgaagcgtccggcggcgtgcctttgaactattttctacatatgcgcttctaccgagcggccagaaattgaccattctcagcattcgcggcaaagccattgatccggcaatatcgctcatcatatttttatttgccgctttgattgtgggagctattccgtttgcgtaccacgacacggcggcacagaatttcccggacgaagaaacgctgctgagtttcttcggagccgactcgtgccagattgcctcgacttcggtggaggaaagaaactcctacgcctgcagcgcgttcctgctggaatcggcggggctgagtgccaagacagccccgatcgcgggtgccctgctgagcgtcacgctcaccctgatcccgatatttcaattcagccggatatcccttggcgtctttctcgtatcgcttggatggggtttcatcagggccattttcctgtcggtcctttcaaaggacatgctctccgcctgcgtcgtgctcctttcgatcatggcggcacaacaaagctggttcggtctcacgtggatcctgtcttcgacgatctacggctgggtggtcagaaaatactggctgctggtcagcgccacctggctcggattgagactgataagaaatcagctcaccgtattccggttgttcgtcttcatcgtcttgatttacatcgcgctctcactgacgttccagatcgcattgggcgcaacactggactttgcccgggccgcggtcaacgagaaccgagaggtaggcgccgaagggtcgcggacggtcatcgatgccgttattgcttccgacaatgccatgctccaggcactcaacgcaacgatcaccttcttcaggctggcgtttcccctcgagctattgcgttttggatcgatcagccagctggcgttcatttcgatcatgcctttcaccttcatatggatggtgaaggccatcgtcaagggcgtgaaatcggacaataagaacttgatccaggccagcaaggtcgcgctggcaccgctgtcttttctcattatcgagggcgtgttcgagcctgatttcggttcatttgcgcggcacttcgccatcgtcagcccgctcgttttttccgccctggcgctggtgcagaaaggcgaactggcccaggacaagctcctgaggcgcaggcagcaagcagccgccccagctgccgcacccaccgcggccccagcggcccttgttggcaccctttctcaggatcgcgcctcgtgaagtcccaatccattgcggtcgatcagccccagtacgtcgaatccatccaggccggacgaggcattgccgctctgctggtcgtcatccatcacgcggcgcaaaaggcacatgcgctgtctggcggcacgattcccctgttcgatttcgggatcatcggggtggacgtgttcttcatgatcagcggcttcatcatctactttgtcaccgccaacaagacgatgacgcacgtggagttcatggaaaagcggatcgtgagagtctttccgctttactgggggctctcgctgctggcgctgctcatttttatcattgcgcccaagctgatcaacagcaatgcgaaagaagcgacggacgtcgccgcgtcgttctttttgtggccgacctccgcgccgtacctggtcaacaacggctggacgctgacctacgaaatcatcttctacgggctgtgggcgctggtcgcgcttccggtggcaaagccaaagaacgcctacatcgcgtgcctggtactggccgccgcatcgttcattggactactctccggaatcgactacaaggtaatgaatttctcattgtttgtagagttcgcgttcggagtcgccattggcgtcgcattcaagaagggactgctccggcagagcattcctttgtcgattgtcttgaccgccgccggggcttttcttgcctacctggcaattgcgcgaggcttcggcagcagcgagctcagagggtttgcactggcgatcccctccgcaatgatattcgtcggaatcatcttgctcggatcgctctggggcaaggcccgcacgatcctggccattggcgacagctcctactccctgtatcttttccacccgttcatcctggtggccattcccatcgcggtgaagtcgctcggcctcgcctcaccgtctcaaattctcgccatttcggccgcggtctgtgtcgcctcgttctgggcttcgcacatggtctacaggttcgtggaattcccgctcactcagatgatgcgcgggatgatcaagtccgcgaagtccctgggcgcggccagagcgcggtgatcctcgcgctcatcagcagcccagcaggtcggccaactggttgatgtcgcgtgcgtgcaggttgttctcgggattgggcgaaacgtctttcggctgggcgcggccgaattcgcggggccgctcgatgtaggcggtcttgaggccgcacacgcgcgccgcggccaggtcgtcgtggtgcgccgcagccagcatgacctgcccgggcgttgcgtcgaacacacccgccacgcccagataggtgcgcgggtcgggcttgtaggccttgaacacctcggccgacagcacgcaatcccagggcaggccggcccgtttggccatttcggtgagcaggccgatgttgccgttggagagcgtgcagatggtgaacttctttttcaggcgcgtgagcccttcgaccgcatcgggccaggccggcagccggtgccaggcgcggctcaggtggcgcttggcggcggtgtcgagccgctcggccatgccgaaatcgtgcagcacctgttcgagcatgctgaggtgcagctcgtcgagcagcgtgaagccgccctcgcctgccgcaatgcgttccatcaccgccttcatggccggctggtagcccgcgcgccaagccagcgcaaaggttgcgccgtccacgcccggcaacgcaagctcggcctcggcggcaatgccgctgtgccagtcgaccaccgtgccgaaaacgtcgaacgcgatgaccttcaggtcgctcgcgtcgaaatccgcgcgcatggtcagcgcggcagctggctcgccgcgcgtgccagttgctcgatcagcgcccagttgccgccctggatcgcgtcggtcggcacgatccaggagccgcccacgcacgccacgttggagagcgcgagaaactcggccgcattgcccgcgtggatgccgccggtggggcagaaggtgacatcgccgaacggcccttgccacgccttgagcatgggcaggccgcccgcctgcagcgccgggaagaacttgagctcggtgtagccgtcttcctgcgccatcatgatctcgctgccggtggccacgcccggcagcagcggcaggccgaggtcatggcaggccttgccgaccgcgcgcgtgtagcccgggctcacgccgaacctggcgccagcgagcgccgaggcctgcgcatcggcggcgctgcggatggtgcccgcgccggccacggcatcgggcacgtcccgcgcaatggcttcgatgcattccagcgcctgcggcgtgcgcagcgtgacttcgagcatgcggatgccgccagccaccagcgcgcgcgccagcggaacggcatgtttcacgtcgtgcagcacgatgaccgggatgaccggtgcatcgcgcatgacgtcgagcgcggtgagtttgttgttttctacagccatgagcaggctccttcttcagcagtcaatgcattgcgccgcatgccggcgaacagttcgcggccgaggccgtggccgtccgcgatgcgctttgcctcggggagcgtggcggtctcgcgctcggcccattcgtcgtcgggcaccagcacggccagcgtacccgccacggcatcgaggcggatcacgtcgccgtcgcgcaccttggcgagcggcccgcccgcggcggcttcgggcgagacatggatggcggccggcaccttgcccgaggcgccgctcatgcggccgtcggtgaccagcgccacgcggaatcccttgccctgcagcaccgagagcggcggcgtgagcttgtgcagctcgggcatgccgttggcctgcgggccctgccagcgcaccacgcacaccacgtcgcgctcgagctcgccggctgtgaaggcctggtgcagcgcggcctgcgaatcgaacacgcgcgcgggcgcctcgatcacgtggcggtcgtccggcaccgaagacaccttgatcacgctgcgccccaggttgccgttgagcagcttgaggccgccggtagcgctgaaggggctctggacgggccgcgcgacggcttcgtccttcgacggagcggcggaattccagaccaggcgcttgttgtcgtccaccagggacggcacattcgaaaattcgcggatgccgccggctcgcacggtcagcacgtcggcatgcatcaggccggcgtcgagcaattcgccgatcacgaagcccggaccgcccgcggcctggaaggcgttcacgtcggcgctgccgttggggtagacgcgcgtcagcagcggaatcacgtcggaaaggcgggagaagtcgtcccagtcgatcacgatgcccgcggaacgcgccacggccacccagtggatcaggtggttggtggaaccgccggtggcgagcaacgccaccatggcgttgacgatgcagcgctcgtcgaccatctcgccgatgggagggcaattgaattttgcctcgctggcgcggctgagcaccgtgcggacggcctcgcgcgtgagcgtttcgcgcatcgcgtcgccgggctggatgaaggcggtgccgggcacgtgcaggcccatggcctcgagcagcatctggttgctgttggcggtgccgtagaaggtgcaggtgccgaccgtgtgataggccgccatctcggcgtcgagcaggccctgccggcccaccaggccttgtgccgcctgctcgcgcaccttggacttttcgccgttcgacaggcccgagggcatggggccggcgggcacgaacaccgtcggcaggtgcccgaagtgcagcgcgccgatcaggaggcccggcacgatcttgtcgcacacgcccaggagcagcgcgccgtcgaacatgtcgtgcgtgagcgccaccgcggtgctcatggcgatcacgtcgcggctgaagaggctcagctccatgccgggcgtgccctgcgtcacgccgtcgcacatggccggcacgccgccggccacctgcgcggtggcgccgaggctgcgcgcctcctgcttgatgatgtccgggtagccctggtacggcgcatgggccgagagcatgtcgttataggcggtgacgatgccgatgttgggcgcgcgctcggtcaccaccttgaacttgtcattggccgggatgccggccacggcgtgcgccacgttggcgcagcccatgcggtcggaaccccggtcgcggttgcggatttcggtcaggcgctcgaggtacgcgctgcgcggcccccggctgcgttcgcgaatgcgatcggtaacgtcaaggacggtgggatgtgtgctcatggggatgtgttcggtcgcgtggccggcatgtcggcactgtcgctttcgcgaccttcgactcggaagtcaatagtaccaagacagcgtgaacgaggccgatggaaatccaccaccgcggcgatacggatttaccgtttgcgccaatcaagcggcacgagggaggctcgtcagtcgaccagcttgacctcgacgcggcgcgcctcggcgttgttgcccgaccccgcggtgaccgcgggcttctgcaggtcgaccttgctggccggcacgcccaggcctaccagcacgtcgcggaccgtgtcggcgcgtttcttggcaagctgctcgttggtggccgcatcgcccgtggtgtcatgaaagccggagaccaccgccttgcggccgctctccacgcccttgatgacggccgccagcgcctcggccgccccgggtgcgagatcggcactgccggtggcgaaatagaagttcaccacgccgttggccacgcggatgctcgcgccatcgggaatcacgaccgtcaccgtctcggtcacttcggccaccgtggtggtgggggcgggcgctgcgggtgcagccgctgcggcagctgccacagcaggcttggcagtggccggcgccgccgcatgccccttgtgccagaccgcgatacccacgacgaagaagatcaccagcgcaatcaatgccaggagaaatccgaggatgaaattttgctggctgtcgtcgtcactcatgagggggcgtactccgtaggaaagaggtcggtaaataatggtgcggtgaaccatgatcacgaaattgtaggcgccgccccctcgggccctgcgccagacccggggccgccagggctggaccccatgcccaggccgttgcgcgacccgcagcccatgctcgaacaggccattgccgattggggtggccgcgaagacttgtggctcttcggctacggctcgctcatctggcgccccgagttcgactttgtcgagcggcggcccgcctgggtgcacggctggcaccgggcgttgaagatgtggagccgcatcaaccgcggcagcgtccagacgccgggcctggtcttcggcctgctgtcgggcggcagctgccgcggcatggtgttccgggtgccttcggcccacggcctcgaaacgcttcgcaggctctggctgcgcgagatgccgaccggcgtgtacgacccgaggtggctgaattgcaacacgcccgagggtccggtgcgcgcactggccttcaccctgtcgaggcgcagccccaacttcaccggcgagctcagcgacgaccgctaccgccacatcttcacccacgcggtcggccgctacggcagctcgctcgactacgcgcgccagaccctgctggagctgcgccggcattcgatccacgacgcggccctggcgcggctggtcgcgctggcgcacgagaagcaggagcaagagcagcaggcgcaagaggcgcagaaggcgcggcaagaaaagctgtccggggcagccgccgattgcggtatgccgccgggtccggtatatgttccggggtctccgaacccatcttccaaaaaggaaaaaccatgaaccatcgccttttcgtcgccaccggcaccgctcttctcgccggcgccctgctctccgcctgcggcggcatgatgggcggcaagccgcgcgcggccgccgagctgatgccgactgcggcgatctcgcccaacccgacgcgcggcacggtgaccttcaccgccctggaccacggcgtgcgcgtggccggcgaagtgcgcggcctggccccgggcagcgagcacggtttccacatccacgaaaagggcgactgcggcgacaacggcaacgcgtctggcggccacttcaaccccaccggcggcacgcacggcaagttcggtgcaccgggcagccatgccggcgaactgccgagcctggtggccgacgccagcggcgtggcacgcttcagcgtcgacgaccacagcatctcgctgaccgagggcgcagccaacaacgtggtgggccgcgcgctcgtggtgcaccgcgaccgcgacgatttcacgacccagccggccggcaactccggcccgcgcaccgcctgcgcggtgatcgcgcggcgctgaacggctagccagcgcccgccgagcgctcccgccacagggcctcggcgagcgccagcgcctcgggcgtgtcgatgtcggtcacgatgccgacgtcgtcgaccatcaggtcggccaccgcatcgatggcgcgcatcgccttcagcaccgatgccgcgccgaagtttccccgcagcgccgcgagctgggcccggcatcccggcccgaagccgaccggatgcccgcgctcgcccctgtattgcggctgcgccgcgcagatacggcctgtgagcgccgcggccaccacgcgcagtgtctcggggcgcaccagcggcaggtcgcccggcaggatcagccagcccgcggcatcgggcgtggcgcgcaccgcagcggcaatcgaatcgcccatgcccggatgcccggcgtcttcgagacgccatggcaggtcgctggcgcgcacggcgtcgagcgtgcgctcgagcagcggcttgccggcgagcggcgcctgcagcttggagccggtgccgccggctgcgatgaaacgctcgccgcggcccgaggccagcacgatcaccaagggggaattcgcctttgccgccatgcgccgagtatgtccgcggaatgaccggaatgccgggcggtggtgcatgcgcaacaatgccgccatgacttcttctcccaccaacgaaacgttggccgcgctgcgcaagagctacgagcgcgccgaactcggcgaaacccacagcgccgacgacccgctgaagcaattcgagcgctggctcggcgaagccatcgacgcccaggtgcccgagcccaacgcgatgaccctgtgcaccgtggccagcgacctgcggccttcgagccgcatcgtgctcatcaagggctgcgacgcgcgcgggatcgtctggtacaccaactatgaaagccgcaagggccgcgagctctcgggcaatccgtatgcggccttgcagttccactgggtcgagctcgagcgcgtggtgcgcatcgagggccgcgtggaaaagaccagcgccgaggaaagcgacgcctactttgcgagccgcccgctcgattcacgcatcggcgcctgggccagtccgcagagcgaagtgatcagcggccgcgacgtgctggtcaagaacgcggccgtggcggccgccaggcacctgctctcgccgccgcgcccgccgcactggggcggctatcgcctcgtgccggatcgctgggagttctggcagggccgcaagagccggctgcacgaccggctgcgctaccggctcgaagacgccgcgtgggtgcgtgaacgcctcgcgccctgaattttcgtcaagcctcgcaacccactactttgaactcgacgcggcggtcgagcgcatcgcttgcgtcgtcggcccccgtgcccacgatgttctcgcggaaccccatgccggattcgcgcagtttcttcgacagcggcggcgcctcgcccaccaaacggctcttcacgctgaccgcgcgctgcagcgacaggcgctcgttgaccgattccgaaccggtgcggctcgtgtggcccgtgaccaccacacatgaatcgatctgcgcggcctggcgcgcgatctgccgcagccacatcgggtaggcggcgctgatcttcgggtcggccaggaagtcggtcgagccgggcttgaacaggaacttcacgctcaggttgttggtttccagccccagtcgcgcgagggtgccgaaggtcttctccgcgtccgcgctgcggccgagttgggcctgcgtgagatacaggccgctgtagatgcgcagctgctggccatcggaccggcgcgaggcggcttcgtagcggctgagcgcttcgctcatgcggccggcctcgtaggccgcggtggcttcctgcagcaccgtcgacgtgggcaggcgttccaggtacagcgcgtcggccgcctggcccggctgtgtttcggcggtgcgaatgtagccttccacgccgcggtccttgccgttcacggggctgtcgcgaaagaacgccgtcggccgcgtgtcgagcgttgcatcgctgatgcgcgccaccgattgcgcaatgaccacgccgctcttgatttcggtcagcgccaggttcaggcgatagcgcccgtcggccgcgtccttgtcgcgcaccagcgtgccgttgagcacgtactgcgcgcgctcgatctcggcattgttgaacggcgtgacggtgaactgcttgaactgcgactgcatgcgctggacgatgcgctgctcggccacgcgcgtgacttcggtctgctggccgctcgagccctcgagcagcgggtcgatcacgatgcggctctgcttgatcgtcgactccaccttggccaggaaggccggcagcttctgggtctgcacgatcagatcgtccaccgcctggttgacggcctgctcgaagggcatggcattgcccggggccggacgatgcgcgcacgcagcggcaagcacggcgatgcacagggccagcacgcgcaacgccgtgcgaaggggtcgggtggtgttcgtcatcatcagcattgactcctcaatatcttcatgtcttcgtccgaaagcggctcgccgatcgccgcgcgcatgttgatttcgctgcagcgcctggagagcggcggccgcttggcggcagcggctttctctacctccggtgcaggcgggggcggcggctgcactgccacggcaacagcctgcggcttcggcctggcattcggccgcgttgccgcggcaggtgcgggcttgggctccgcctccgctggcttcgccgctgcgggcgggactggggccgactcgcgcggcacggcggccgaaaggcagggcgtgcggcacggcttggtatcggtgtcggccgccgccggcaaggcagcactgcacagcgcgatcaccatcgcgatcggcgccatgacggaaaacggcgaagaccgcgcctggtaaatcatcagcgggcaaatgtagagcggcagccgccgctcgccatctcgccaaacggccaccctgccgaacggcataggcgcccgccgcgcacgcggtcggcgcctcggtagcgctaaagacttatgaaaaattcagggaagccactgcaccagggtcatgaccagggtcagcgtggccagcgcgagcaccgtcgacatcgcgacgctggccgtgaccaagtcttcggccgtgcggtagcgctgcgaaaagagaaagacgttggcgccgatgggcagcgccgccgccaccaccatcacggtgagcggaatgccgcgcacgcccagcagccagccgatgccggccaccagcagcggatgcagcaggttcttcaccagcgactgcaccatggcgccgcgccagtgccggccgatgggcgtcagcgcaagcgtgatgcccaccatcacgagcgccaccgggccgaaggcctgcccgagcagcatgatcggcttgtcgatggattcgggcatcgtgagccccgtctgcgcgaacagcagccccgcgatgatcggcagcggcaccgggtggatgatggcgttgcgcagcgcgcgcagcacggtgcgcgccatggggcgcttcgcctggccgctctccgccgcatgctcgcgcgccactgcaagctccagcaccaccgtggcgctggtcagaagcaccagcgagtgcagcgagatcagcgtgagcagcaccaccatgccctgctcgccataggcgaggccgaccagcacgatgccgatcatcacggtgttgctgtaggtgttggccagcgcaatgacggccgccgtgcggttgaagcctcgcagcgccagcgtagccgcgaacagcaggcccgaggcagtgaagtaagccgccaccggcttcaggctcagctcttgcacgtgcaccgtgctcatggcgcgaaacagcagcgcgggcgccagcaagaggaagatcaggttggaaagatccttgacggcgttgccgccgatccagcggcgccggccggccaggtagcccgcggcaatgagaaaaacgacgggcagcagcgaagagatgacgaacgaattcacccgccgaggatagcctcttgcctgccccttcctcccgctcgcgaaggcggaaggaagaagcggtaccggtgacttagaacgtcacgcgcaggcccaccttcagcgaacgccccggcagcggcgcgttcgggtacaccgtcgtcgtcaggatcgaggtcgggctgtaggccagcttgttcgtgatgttgtcgacgcgcgcataccaggtgaggttggcgcgttgcaccttcatgcggtaggaaatcgaggcgttccacagcgtgtaggcatcggtctctcgcgcgccgacgctcggcacgtggcgctgcgccgcgttgtagtcgaagccgaagcgcgcgctccatgggccgttgccatacgccagcgtcgcgcccgcgcggaacggcgcgatgcgcggcagcggctcgccggtgtcgaggttcttcgcacgcaccacgtcgccgcgccattccaggtcgagcgtcgaggcatcggccatgcgtgcgaagccttcggtgcccaggaggcgcaggttgccgctggcctcgatgccggtgaagcgcgcgcgcgcgccgctgtagaggtactcggctagcgtatcggtcgccgcagggtcggtgaccacctggccttcttcatcgagcgtgcggcccgaagccgtcaggccgatgtaattgcgaaagcgcgtgacgtaagcgttgacgcgggccgtgttggcgcccgacttccattgcgcgccgacatcgaagccggtcgacttttctttctgcaggtccggattgccgacctcccaggcggccgttgccacgtgcggcccgttggcgagcagctcgtagtccttcggtgcccgctcggtgtaggcgaggttcgaggtgagctgccactgcggcgtcaggttgaccagcgcgccgatggccgcactgtgcgggttgaacgtgcgctcgccaatggcaaagcgcgtcaccgtcggatcgtcggggtagcccagcgacgtgacgcggactttctcggtgcgcgcgccaaagctcaaccggccccatgacgtgccgagttcttcatacatgaacagcgcgttggagcgcgtgcggctgtgcggcgcaaaggcctcctcgccatcggcggcaaagcggttgctttcgctcgcaaagccgaccaggccttcgaagttgccgatcttgcggtggcgggcttcgatgcgcaggtcgttgctcatgttcgagaacgtggtgccggcctcgccgccttcgaattcggcgtggcggtagttggtgtggctggccttgacgtgaacgctgctgatgatgccgcccggccgccactcgccttcgatcgcatagcggtcggacttcatgccgatggtcacgtcgtcttcggccacggtgccgtagttgctgcggtaggtgctggccgaggcgccgataaagccctggtcgaagaacagcgtgccgcccaccgcgccgccgtgcgcctcgttggccgagttgcagatcttgcgcgccagccagggacgccccggcttgctgcattccaggtcgatgggcaccgagacatccttggcgtcgcggttgaacgcgtcgacgtgcagcgcgaagcggtcgttgccgccctccagcaccacgccgccgttcttctccttgctgccggtcgaaaagcccaggtcggcgcggccgccgaagccgttgatgggctcggtgggaatgcggttgtcgatcacgttgaccacgccgcccaccgcgctgccgccgtactgcagcgccgaaggcccgcgcagcacttcaatgcggtcggtgaccagcgcgtccaccggcacggcatggtcgtagctcagcgccgaagcatcgggcgcgccgccgccgttctgcaggatgcggatgcggtcgccgtcgaggccacggatgatcggccggctcgcgttcgggccgaagtagctgctgctcacgccgggcaggttgttgagcgtttcgcccagcgtcgattcggagcgcatcaacagtttgtcgcccgacagcgtggtggtgggcgcgatcagttcgctggcgcccagcggattgccggtgacggcgatctccggaagagtggctgcggccgcctcggcgggttgcgcctgcggagtcgactgggcctgggccatgctcgcaaaagaagcgagcgaaagaacggcagcgccgatggcgttgcgacggaaattgggaatcatgaatgagcactcgttgaatcaagggacgatctgccgctacccgcaaaggcgggtgcagcaaccggaacacagggaagattcagcgagtggaaggcgggccgcgcgcgtcgaacagcgcaacccagcgggcgatggcttcgccctgcagataggcaaaaatggccgacggcagcagcaccggcagcgccaccgtggggacgcccaacgcgcccgagccgtgcgacagctggtcgtacagccggcattcggcatcggagtggtcgccgaacaggccgacgatgccgccgcgggtcgcatgctcctgcgcgccctccgcatgaacggcctgggcagtggcctgggccgttgcatgggcgtgcgccaggccgggcacgtgcagcgaccggtgcatgagccccagcgtgcccgcgaaccacagcgcaaccaccagcgcgatggcgatcgcccgggtcgacaggatcgaccggttcggcattgggctgagggcgatgtgcacggaaagcagggccttggtgaacgatcaagccttgacgcgggacgcgaaggtcttctggaacttctcgaccttggggccgaccacgaaggcgcagtagccctggttcgggttgttcaggaaataatcctggtggtaggcctcggcggtcgagtagttggcgagcggcgccacctcggtcacgatcggcgagccataggtcttgctcgcctcgatctcgcggatgacctcttgggccacctgcttctgcgcgtcggtcgtcacgtagatgccgctgcggtattgcgtgccggcgtcgttgccctgccggttcagggtcgtggggtcgtgcaccacgaaaaagatctcgagaatttcgcgcaggctgatgacggcggggtcgaattcgaccttcaccacttccgcatgcccggtgcggccggtgcagacctgctcgtagctcgggttcacggtctggccgttgcaatagcccgattcgacgtccaccacgccctgcacgcggtcgaaaacggcctcggtgcaccagaagcagcccccgcccagcacgatggtttcggttggcgacggtgaggaagtcatgggctgctccggcaggtgggaaaaaggcgaacccgatattgtcgcggcttgacggcccggatgccggtcactacattactaacccgtcagtcattaatctcatgcccacgccccgcttccttgccgacaagctctgcccggtgcgctccaaacgcgagcgccgcaaggaggcgcgtcccggcgaactcctggctgctgcgctcgacctgttcgtcgaaaaaggctttgccgccacccgctcggaggaagtcgcggcccgcgcgggggtctccaagggcaccctcttcctttattttccgagcaaggaagagctcttcaaggccgtggtggtcgagaacctcagcggccggttctccgaatggaacgacgagttcgaggccttcgagggcaccacggccgacatgctgcgctattgcatgcgcatctggtgggagcgggtcggcatgaccaaggcttcgggcctgaccaagctcatgatgagcgaaggcgccaattttcccgaattggccgagttctaccgccaggaggtggtccgtcccggccacacgctgctgcggcgcatcctgcagcgcggcatcgaccgcggcgaattcgcgccggtcgacgtcgaccatgccatctacgccgtgcttgcgcccatgatcttcctcatgctgtggaagcactcggccatgatctgcgtcgacggggaagccgcgctcgaccctgaaaaattccttgcgacgcaggccgagacagtgctgtacggcctcacacggcggcccggagcagcagcatgacaagcaaatgcatcgcaggcatcccgcgggccggggccgggcaacctaaaattgaaggtttgtcctgagccccacaaggaaaagcccccaatgaacccgacccccaccctcgagcgcttgcgcttcaacatgatcgagcagcagatccggccctgggatgtgctcgacctggaaattctcgacctcctcgccagcattcggcgcgaagactacgcgccgcccgagcatcgcgcgctgtccttcttcgacatggagcttccgctggccgacggctccgttcccggccaggtgatgctctcgcccaaggtcgaggcgcgcatgctgcaggacctgcacgtgcaaaagcacgagtcggtgctcgagatcggcaccggatcgggcttcatggccgctctgctcgcccatcgcgcagcccaggtgctgtcgctggagatcgatcccgtgctggccgcccgcgcggccgaaacgctgcgccagaacggcgtggccaatgtcgaagtgcgcaatgccgacggcgccgtgccgctgccgagcggcccgagcttcgacgtgatcgtgctcagcggctccgtggcgcgcattccgcagaacctgctcggctcgctcaaggtgggcggccggctcgccgccatcgtgggcgacgaaccgatgatgcgcgcccacttcgtcacccgcagcagcgaaagcaagtgggacaccatccagccgtgggacaccgtggcaccgcggctgctcaatttccccgagccttcgcgcttctcgttctgaacgggaccaccgcatgatcgatcaagtccgccccgccgacctggccgcctggtatgcgcagaaccccggtgcggcgcccgtgctgctcgacgtgcgcgaaccctgggagctgcagaccgcgagcgtcgccccccagggtttcacgctggtcgcgatcccgatgaacgagattccggcgcgcatttcggagctcggcgaaggccagcgcattgcatgcctgtgccatcacggcgcgcgcagccagcgcgtggcggcgttcctgagccagaacggctttgccgaattggccaacgtggccggcggcatcgacgcctggtccgcacagcacgaccccgccgtgccgcgctactgattctttcttcaaggacgttcaatgccttccaggcccaggcttttgcctctctccgcagcgctcgcaagtctctttgccaccctgctcgcactgccggcccaaggccagacactgaacgaactctacgattccgcacgcggcttcgacgcaacctaccagggcgcccgcgcgcagtacgacgcgaccgtggcgcgtgccgcgcaggccaaggccggcatccttccggccgtggggctcacggccggcgcaacgcgcaacaacctggacatcgacaccctcaccggcgccggccgcggaacgacgacgccgcgcgacttcaccacgcagaacgtcggcgtcaacgccacgcagccgctctaccggcccgccaactgggccacctacgagcagggcaagcgccaggccgagatcgccgaggcggtgctcaccacggccgagcaggacctgatcgtccgcgtgagccaggcgtacttcgacgtgctcgcgagccaggacagcctgacgctggtgcgggcgcagaaggtggccgtggccgagcagcttgcatcggccaagcgcaacttcgaggtcggcacttccaccatcaccgacgcgcgcgaagcgcaggcccgctacgacctcgtcattgcgcaggagattgcagccgagaacgacctgcaggtgaagaaggtggtgctcgaccagctggtcggccgccccggcagcgtgccggtgccgctgtcccagcccgtggtgctgcccaccgccatgccggccaacatcgaagcctgggtcgcgcaggccgatgaagtgcatcccgccatccgccaggcgcggctcggcctggacgtggcgggcctggaaatacgcaaggccgaggccggccacaagcccacgctcgatgccaacctgggctacaacatcacgcgcaacccccagggaaccgccaccagcaccgtgggcacgcgcatcaacgccgcctccgtgggcgtggtgttcaacctgccgctgttcgcgggctttgccaccgagaaccgcatcaaggaaacgctcgcgctcgaagaccagtcgcgcagcgtgctcgacggcacccgccgcagcgtggcgcaggccacgcgcgcggcctacctcgggctggtgtcgggcgcgggccaggtgaaggcactcgaagcggccgaggcctcgagccagagcgcgctcgatgccaaccggctcggctaccaggtgggcgtgcgcatcaacatcgacgtgctcaattcgcaaagccagctgttccagaccaagcgcgatctcgcgcaggcgcgctacaacgtgctgctgggcaacctgaagctgcgccaggccaacggcacactcaccgttgaagacatgaacgcgatcaatgcgacgctggcgaagaacgggagcacgcctgcgccagtgccatcggccggcgagcgcccgcaggccgtgccggtcacgccacccagcattccggtcgtgccgccggtgccggtgccgccattcaacccgccggcaccggtcatgccttcggcaccgccgccgcccgtcatcctgaacccgccggttcgctagggatctggctcgccccaggcacaggggcgagattattcgagcgtgggctccgccctcgactcttcttcgaggggcgcggcttcggtcaccacggggtccgcggcctgcgcaatggccagcaccgccgtcgccgtacgttcggccgcgccgcggttggacgacgagaaagccaatgcggcctccgccatgaaggcgcggcgctcggggttctcgaccagcttgagcgccgcggtcacggcctgctccatgttctcgacgcgcagggaggcaccggccgcgagcgacagctgcgccgcctcggcaaagttgaaggtcgatggacccatgaccaccgggcaaccgcatgcggcgggctcgatgaggttctgtccgcccagcggctcgaagcttccgccgagcagcgcgacatcggccaggccgtagtaaagggccatttcgccgagcgaatcgccgagccagatctcggcgtcggccggctcgcccgcggcgctgcggcgtgccaccgcaaagccctgcgattcgatcagcgcggccacttcatcgaagcgctgcggatggcgcggcacgatcatccattgcacgtcgtgcacgcgcttggcaatcgaacgaacggcgccctgctcgggcggcacgggcgaggtggcgccaaagcgcttgagcacgtcgagcagcatgcgctcctcgccgtcgcgcgagctcgcgagcaccaccatcggccgcggcaggcgctcgcgcaacgccacggcggtggagagctggcgcgcatcgggcgaggcgtcgaacttgaggttgccatagatgccggccaccttggcgccgagcgacaccagccggtgcgcatcggcttcggtctgcgcccaaacggcagcgagcgccgagtacgcgggccgtgcgagccagccgaggcgttcggccgcggccagcgatttttcgttgaggcgcgcattggccagcaccagcggaatgcggcgctcggcgcaggccgcggccatctcgggccagacttcggtttccatcagcacgccgatgcgcggctggaagcggtcgagaaaccgcgccacggcacccggcgtgtcccacggctgccagacctgcgtatcgccgggttcgagcagcttggcgccctcttcgcggcccgtggcggtgccatgcgtgagcaggatcgggatgcccggatactgccgccgcaactccgcaatcaagatggcggccgcgcgcgtttcgccgagcgaaaccgcgtgcacccagcactggccttcgccggtgatggcatcgtcgtagtggccgaagcgctcctcgacggccacggcgtagccgggctcggcttccgcgcggcgccgcagcttgcggcgaaccagcggttgcacggcggtggtgaaggcgccgtagaggcgcagcagcagcgaacgcacggggctcagtgcgacgcttcggccagcgtcgcgtcggctttgacggttcgaaggagtgcgagcatttcggcttcgatgcgcttcagggccgcatcggtctggccctcgaagcgcagcaccagcaccggcgtggtgttggaagcgcgaatgagcccgaagccgtccggccagtcgacgcgcaggccatcgatggtcgagaccacggcgggtgccgcaaagctcgcgccggcaaccagcttgtcgaccaccgcgtgcggttcgccttcggcgcacttcacgttgagttcaggtgtcgagaagctcgtgggcagtgcgttgagcgtgtcgctcgcgttcggcgtcttgctcaatatctcgagcaggcggcagcccgcataggtgccgtcgtcgaagccgtaccagcgctccttgaagaagatgtggccgctcatctcgccgccgagcggcgaatcgatttccttcatcttggccttgatgagcgaatggccggtcttgaagatcatcggcttgccacccgcggcctcgatggccggcgccaggcgctgcgagcacttgacgtcgtacacgatggtgccgccgggcacgcgcgagagcacgtcctgcgcaaagagctgcatctgacggtcgggaaagatgttctggccgtctttcgtgacgatgcccaggcggtcgccgtcgccgtcgaaggccaggcccagttcggcatcgcccgtggccagcgcagccatcaggtccttgaggttctcgagcttgctcggatcggggtggtggttgggaaagtcgccgtcgacctcgctgaacagctcggtcacctcgcagccgatggcgcggaagatggccggtgccgtggcgcccgcaatgccgttgcccgaatcgaccacgatcttgagcggacgcgccagcttgatgtcgccgacgatgcgctgcgtgtaggcctcggtcacgtcgaccttgcgcacgctgccgccgggtgcaagcttcgcggtgccttcttccatcaccttgcgcagaccctggatctcgtcgccgtagatggcgcgccccgccagcaccatcttgaagccgttgtagtccttggggttgtggctgcccgtgacctggatgccgctcgagcacagcgtgtgggccgcaaagtagagcatgggcgtggtcaccgcccccacgtcgatcacctcgacgccggtggcgaccaggccgctgatcaatgcctcgacgagcgcggggccggacaggcggccgtcgcggcccacggccacggtcttttcaccggccgcacgggcggcgctgccgaaagcccggccgagcgcttccgcgacctctgcatcgagcgtgacgggcaccacgccccggatgtcataggccttgaaaatcgatgcgctgagttgcatgaagtggcattccctgttggttctggagaccgggccattgtaggcaagcgttccggtgcccacatgtccgaaaacggccagttgaaacgactcgaaaccgtatcatttgcccatgcctacccctcatgcctccaccgaagcgctcgagagcgacgcctgctacctggcgatgaagacgcacgacgcgcgcttcgacggctcattcttcaccgcggtgacctctaccggcatctattgccggccggtctgccgagtgaagctgccgcggcgcgagaactgcaggttctttcgccatgcggcacaggccgaggccgagggctttcgcccttgcctgcgctgccgtcccgaactggcgccccgcgcggcaagctggtcgaccgaagacgcctcgcgcatccttgcattgcaggccgcgcggctcatcgacgaacccgatgcctgggccgaagaaggtcccggcgcagcgcagatcgcggcgcggctcggcgtgagcgaccggcatctgcggcgcatcttcgaagcgcagttcggcgtgtcccccttgcaatatttgcagacgcggcgcctgctggccgccaagcaattgattgccgacacgcggctgccgatgacgcaggtcgcactggccagcggctttgcgagcgtgcgccgcttcaacgcggccttcgtggagcactacggcctcaaccccagtgcgctgcggcgcgccggcggtgcagaaggcggcgaaggcaaggccatcgaagtacgcctgggctttcgcccaccgtatgacgcggacgcgatgctcggcttctttgcacggcgcgcactgcgtggtgtcgaggtggcaagcacggccgacggcaagacgcccaccaagggcagcacgcccaccttcgttcgcctggcccgcacgctgcgcgtgcagcaaggcggacagacgcactccggctggctgcagctgcgcttcgacatggagcgcgagcagatgctgctctcggtgagcgattcgctggccgcggtgctgccgatcgtgatcagccgcgcacgcgccatgctcgacctcgacgccgaaccgatggccatcaacgccgcgctgcacgagtcctttccgcatggcgacgggctgcgcgtgcccggcacggtcgatggcttcgagcttgcggtgcgcgcggtgctgggccagcagatcacggtggccgcggcgcgcacgctgggctcgcggctggtcgaggcattcggcgagcccatggccacgcccatcgacggcctggaccggttgtttcccacgcccgccgtactcgccgcggcaagcggcgatgcgctcgggcagctcggcatcgtgcgacagcggcaggcggcattgcaggcgattgcccgcgaggtcgcctccggcaagctggcattgcatgcgggtgccgacgtgccctcgaccattgccgcgctgcaggagctccccggcatcggtgcctggacggcgcaatacatcgcgatgcgcgcgctgcgctggcccgacgcgtttcccgcgggcgacgtcgcgctgcagaaggcactgggcgtgaccaccgcgcgcgcggccagcgaggcatcgcaggcgtggcggccctggcgcagctatgcggtgctgcgtgcgtggcatgcgccgtcgcccaccgtggccgcggcctcgtccgccgcagagccatctttcaacaacctcacaacggcaggcgcctccgcctgaaatgtcatgaagttcaagagcaaagtcatctacacatcgcacatcgaaacgccgctcggcggcatcacgatggcggccaccgacgaaggcctggcgggcgtctggttcgaccagcaacgccactggcccgacaccacgggctgggagacccgcgacgaccatcccgcgctggtcgaggccggcgcacagctgcgcgattacttcgccggcaagcgcgacaccttcgacgtgaagctcgacctctcgcacggcaccgcgttccagcagagcgtgtggcaggcgctgctcgccataccgtcgggcaagaccatgacctacggagcgctgagcgccaacgtgggcaacccggccgcggtgcgcgcggtgggcgcggccgtggggcgcaacccgatcagcgtgatcgtgccctgccaccgcgtgctgggcgccgacgggtcgctgaccggttacgctggcgggcttcatcgcaagaccgcgctcctggaactggaatcgaagtagagccagcctccaaggcaatgcgcaccatcgagaacgtatgaacacgacaacgaaagacaacactcccgccaccacgccttcgaccaagcccaaagcgtggctcctagacctcgtgctgctgggcgccctctggggcgcatcctttctcttcatgcgcatcggcgcggccgagttcggcgccttgccggcggccgcggtgcgcgtggcggtggccacgctgttcttgctgccgctcctgttcctgcgcgggcacggcgctgctctggggcagcactggaaggcgtcgatggccatcggcgtgctgaattccggcattccgttcgcgctcttctgcttcgcgctcctgaccatcaatagtggcctggcggcggtgatcaacgccacggtgccgatgttcggcgcgctggtggcatgggcctggtttcgcgaccggcccgacggctcgcgcatcgtcggcctcgtcatcggctttgcgggcgtggccatgctggcaagccgcagtgcgggcctgcacgccgatgcgggcggcaacgccgcgctgtgggccgtgctggcctgcctgggcgcatgcgcgagctacggcgtggcggccagcgccacgcggcgctacctgggcggtgtgcccgcattggccaccgccaccggcagccagatcggcgccacgctgttcctcgcgctgcccgcgctgtggttctggcccacgcagatgcccagcgtgcgcgcatggctggcgctgctggcgctgggcgtggcgtgcacgggcctcgcgtacatcctcttcttccggctcattgccaatgcggggccggcgcgcgcactgaccgtgaccttcctggtgccggtgttcgcggtgttctacggcgcggtgttccttggcgagaacatcacgcaatggatgctgatctgcgcggccgtcatcgtctgcggcgtggcgctgtccaccggcctcgtgaagctctggcccggcgcgggctcgccggccgctacatcgcccccgcgaccacgttgacggacagcgcgagcaccagcatgttgaaggcgaaggccagcacgctgtgcaccagcgtgatgcggcgcatctcccgcgaagtggcctgcacgtcggacacctgcgtggtcatgccgaccacgtaggcgtagtagagaaagtcgaaatagtccggctcctgcttgcccggaaaatccagcccgccgtcgggcgagccgtcgcgctggtcgatgtagtagcggtgcgcgtaatgaaaggcgtagatcgtgtgcatcatgagccacgagcccacaagcgccaccagccccagcgcaatatgccccgtgcgtgcggggccgctcatcagcttgacctgctgaagcagcatcgcaatggccaccacgctcgcaccaatgaccaccagcatcgacaccaatatcaccacgttgggttgatcgagcgactgcgcgcgcttgcgggtttgctgtgcatcgaaagtatcggccagccaccacgtgagcacgagaaacaccacgcagttggtgcaccagcccgcaagtccgcgtgccatgccgtcgagcggccacgggatggccgcaaccacgatgcccgccacgccggcatagagaagacgctgcggaccggtggtcgcggaaagatgtttgcgcatcttcaaagcttagcttgaatactttttcaggcttgccaacgcatgcttcaacatcgtcttacacgcgaagcggcaaatcgacgcatgggcgttttaaagctgcgctataacttgtcggtcatcaaaagggagccgccgcctggcgctttgcgcgcataaaaattgcgtgtcgagcccgaggcttttttgtcctctctcttctctcttaaggacctcctcatgctgttgctccgctcccgcccgctcgccagccccgcacggttgacgaagctgggcgcactggccggtgtcgggtttctctttgcgcccgcattggccttcgccgaaccatcgcccgcgctcgatcgtttcagcttttcggtgggagcctatagcgccgatcctaaattcaatgcgacagtcagctcgccgtacggtgcgctgcgcacgcgcgacctcgagcccggccgcgtgaccatgccgcgcgtcacggccgacctgctgatcggcgacagccacggcctctcgttcgactactaccgctacaaacgcgactacttcggccaggccgggggcaacgaatccttcggcggcttcggcacggtcagcgcggtgggcaacgccaacctcaacgtgaagctcgacttcgcgaagctctcgtacaagtggtggctcggttcgggcaacacggtgttcggcctgggtgcgggcgcggcctactacaacatcggcgtcgccaccaacgccaacgtcgcggtgaacggacgcattcgcacattgaacgaagactcgagcgacaacgccgttgcgccactgctcgaggtcggcgtgcggcatgccatcagtcccgacttgcgcctttttgccgatttctccggcgttcgcaagggcggtggccgcttccacggcagcatctacaacgcctccgccggcgtggagtggtttccggtgaagaacgtcggcgtggtgctggcctatggcgccacccacatcgacatggcgcgtgaaaccagtacggcggaaacccgcgtcaaggtcaagttgaacgggccgtcggccttcatcaaggcaaggttctgaatctctggcggcacggcggccctgccatgcgccgggagcggtgcgcataggtgcttgcgatcatcggcggccgcgccatggccccctatgatcttttgatgtacatcccagccccaccccgctccgacaaactcgatgggtgcgccgccagtgcgcgccgcacccggaagccgcacgcgcttggccttgccgcctcggcggcgctgctgctcgccgcgggcgcaccggcccacgcgctggtcatcggtgtgacggaaggcgtgagctaccacgtcaccgaaagccagatcgcgccgcgcttcgagcccattgccgaggtgctgagcaaggcgctgaagcagcccgtgaccatcaaggtgttcataacgtacaacggtgcgcgcgaagccctgaaggagcagcaggtcgacatcgcgttcatccacccggcccacgtggcgctcgaggcagtcaagagcggccgctaccaggcactggcctggaccagcggcttcaccgcatacaaggtgtcgctgctgtgcaaggagccgcagcccatttccgactggaagggcattgccggcaagggcctggtgatgcccgacgcggattcgatcacctcggtgatcacgcgggccatgctgcgcgagcacggcctgcagccggccgcgctcaagctcaccaacacgcgctaccaggacgcggttccgttctatgtgcagaacggctttgcggcctatggcgccaccgcggcatcgggcgtgatcaagacctggaaggacggcggcggcaacgtgtgcgcggagtcgcgcgcggttcccatcaagcaatgggtggcgtcgcgcaagctcgatgccgccacggcaagcgccgcgcgcgaagccctgctggggctggcacaaagcgatgccggcaagcgcgcactcgccacatcgacctacactggcttcgtcgcaccctcgcccgaagccgagacagccttgatgacctggctcggcatctgaagatcggcgggcgcggcgccccaactccgcttttcatgaaccgcccatgaccgacctgtcccgcttccccatcacccagaaatggcccgcactccaccctgaccggctgcagctgtattcgctgcccacgcccaacggggtgaaggtgtcgatcatgctggaagaaaccggcctgccctacgagccgcacctggtgagcttcgagacccacgaccagatgtcgccggagtttctgtcgctcagcccgaacaacaagattcccgccatcctcgatcccgatgggcccggcggcaagccgctcgcgctgttcgagtcgggcgccattcttctctacctggccgacaagaccggccgcttcattccgcaggatgccgcgggccgctacgaaaccatccagtggctgatgttccagatgggcggcatcggcccgatgttcggccagctcggcttcttcaacaagtttgccggcaaggactacgaggacaagcgtccgcgcgaccgctacgtcgccgaagcgaagcggctgctgggcgtgctcgacaagcaactcgaaggccgcaactgggtgacgggcgacagctacaccatcgccgacatcgccatcttcccgtgggtgcgcaacctgatcggcttctacgaagcgggcgacctggtgggcttcaacaacttcaagaacgtggcgcgcacgctcgaagccttcgtggcgcggcccgccgtcgtgaagggcctgggcatccccaagcggggctgatctccggccgaacttcttcggctggaagacgccgccgcccagccgaaaacagaactactcattttccggccgagtgtctttttcagggcacgtgctggtgcttcccgcaccctttcccgcctccttcaggcgcggttaaggttacacttcaataagaataattcttattcaatgttccgagtcatcccgcagattgcgccggtgaccggcccgggaatcaccactgcgaaaacttgcgagaaggcgatcggatgcgcgacctcgtccaggaacttgtggctcactatgcggacttgcgccgccagctgacgcgcgacctgcgggacccccactacgcggcggacatcgcgcagtcgagcttcgagcgggtgtatgcgcacgcgctcaagatgaacgacgacatccgcatcgatgcggcatcggacggaacgccgggcggcggcatcgagtcgccgcgcgctctgctgtttcgcgtggcgcgcaacctgtgcgtggacgacgcccgccggcgcaaggtggcgcaggactgggtcagcacgcatttcagcgtcggctcgcgccagacggtgccgtcctgcgaattcatcgcgtcgcagcagcaggtgctggcacgcgtggtcgagacgctggagacgctgccaccccgccggcgcgaagtgttcctgctgtttcgcgcctacggacacacgcgcgccgagatcgcccagcaactgaacatcaccgagatggccgtggccaagcatttgctgcgcgcggccatcgactgctcgcgcgtgttcgcccggcttcgctcggaattgatcgaacagacgaccgtctccaaccgcacgggcttcgacgcgaagctggccgaagacttcgcctgagcggcgcatcgtggcaagcgcgccggacgaaaagctcatcgaacgcgcgctcgcgctgattgtcgagagcgaaagcgcaccgcacgacgccgcggttgccgcgcgcctggccttggcccggtggcgcagcaggtcggccgaacatgcggccgccgcgctggaagcgcggcggcgctgggatgcccttggcggcatcgcagccgagctgcgcgacttgcggaagtagcgcggcaacccttcactgcaggcgcttctcttcatgccgcgcctcctccagcgcaggcttcatgagtgcggcgccggtcagcgcccagagggtcagcacgtcgtccagcgcgcagatgttccccggatcgacgccgagccagcgcacgagttgctctgcccgctcgggcgacggctcgtcatgcagcgtgcagaagagcgtccacgcaatgttgaaggcagggcgatcgggcggccggctcttgtgggtcttgtcttccattcccctccttcacgcggcgaggctttcgcacgattcacgcaccctgtcttccgcgatcttgcccgcatgcatcgtgatgacgcggtcggccaggtgaaagtagcggtcgtcgtgcgagatcaccaccagcaggtgtcccttggcgcgcagctcgggcaagagctcggtgtagaagaggtggcggaaggtcgggtcctggtcggcggcccactcgtcgaacaccagaaccgggcggccttcgaggtacgcgtgcaccagcgccagccgcttgcgctggccggtcgagaggtcggtggtgctgaacgcgccgttcttcaggctcaccttgtgggcgatctccagccgttcgagataaggcagggccgtttcgggcagcacctccatgcccgcaccgccctcgctctcttcgcccgccaccagatcttcgaacaggtagaagtccgagaacaccgtggtgaagagctggcggtagtcgtcgcggccctcgggcttcacgaccgaatcgtcgatcagcacttcgcccgcctgcggcgcatagaggcccagcagcagcttgatcagcgtggtcttgccggagccgttgtcgcccactacgaacaccatctcgccgcggcgcagcttcaaatcgatcggccccagcgtgaaggcctcgccgccctcgggcgcatcgaaggcatagcgcacgccgcgcatgccgatctcgttcttcaggatcacgccgttggacgcgcgctccaggtgcaggtggggctccggcgtggcaaagcgcgccgacaggtcgccgatgcgctggaacgcgaccttggcgcggcccacgccgggcagcagcagcgcgatctgatccagcggccccttgaggaacagcagcaccagcacgaagccactgagcaccgcgggctcggtcggctggaacgcggcccagcccaggatcagcgcgatcagcaggaagaacagcgccgagccgaaggccgttgcgatcacataggtgttgatcgcacgcccgttgacgacgcggatggtgtcgacgatgcgctcgatctggccggagaacatgcgcgtgcggcgcgtgcggtgcatgcgcagctccttcgcgccttcgctgatggcgcggtaggccttgtgcaactggtcttcctgctcgcgcgccttccagaagccggcttcgccgcggatctgcgccatcaactgcgccgtgatgccgatcaccagcgccaccagcatcagcccgaacagcggcggcgaaagatacgcgaggtagccgaggcaacccagcgccacggcgagcgagatcagcattcccgacagcgcgaaggccacgtcgctgatcatgtccacatcttgcgagagcaccggcatcaggcggtgcgtgcgatagcgctccagcgcatcgatgggtgccgcgagaatcttctgcgccaggctctttcgcacctgggccaccaggcgctggccgacgaagttggtcgacacgtccgacgccatgcgcccgaacagcgccacgccgcacaggccgatgaaggtcagaagcagcccacccgccagaccgcccggctggttcagcacccggttgatggtgccgagcagcgcgaccgtggcggcaccggcgccgacgcccgtgaccgcggacagcacgatccatggaagaaatggtttcagcaggcgcccgatttcggcgccgttgcctgtggtggtagttgtcatgcaaaggctctttccgcccgggggcgacagctggggaacgaccatgcctctgtggcacggctccaatggcttcgtgccacctactgcctagacggcccagacgcggcaatgttcagcgcggcgccggatgaacagcggccgcgcgaatccgtcttgaaaggatgaccccgccgaacgccgacccatgatcccgctgctggagcccttgttccagggcgaactggccgtgcatggcgagaagctgcaatgcgcggacacggtgcccgccggtgcggtgcgcgtggctgaactcgcgcaatcccccgcgctgcttgccgacgtgctgcaacgcaatgcgcgctaccgaggtgtcagcggcgccgattggcgccccgtcgcatccgcgtggagcctcgaatacatcgcgatgctgctgcccccggtgatggccgcggccagcatgctgcggcatgtgtttcccattgcggcggaacacacctgggtgcggctggatgcgcacggcggcccggtcggctttcatatccggcatttgggccggccgcaaccaggggccgatgccgcggagcgctatgaaccgctgctgtggcagcacctcgccccactctttgcggccctttgcggcctcacgcggctcgcgcccaagattctctggagcaacaccgtgcggctcatggaaccggtgttcgacgtggcgctggccgcaacaggcggcgcgccgtcgatcgcagaggatcggcaactgctgctgcacagcgcgatatggccgcgcgatcttcgcaccaacccgctgcacggccgccagcgcaatgcgcccgtcaagctgcaccgggagtgctgcctcaactacctgctgccgcacgagcaccactgcaacgcatgcccgctggcgccggcgcatcgcggcctcgggtgaacagattgcgggccattccgtcttccatctatccatccattccacacctatgtccaaggccaagctcgtctacatcctgtctctgagaaacgccgcggccgacaaggccggccagcacattgcgtacaagggggagcagcgctacatggcgtccccgctcgagtacctggccagggcgctcgacgaaaccccgctgggcgatgcctattcgctcgaaggcatcgtcatcgacgacgacccgcgctcgccgcgcgaccaggccgcgctgcaggattacggcttctcgtgccagcccggcaagaaatggatctttccgggcgggctcaagacgcagggcaagacgctcaccgacatcttccattcggtgccctccgaataccggcgtctgccgctcgatgcggccgaccgcgtggccggcaagaaccgcttcgagcgcacgctgctcgacaagctgctgacgctgcaggccgacatcgtcgtgctcgacgggctgctggtgatcctggacgagctggtgcggcccggcgcaccgttccaccgcaggatcgtcaacatccatccgggcatcacccgcatcgagtctccctacgaacgccgcggcgcctacgccacgctcgatgcgctgcacggcgcgcagggccgcaagatcgtcaactgggcaacgatggaaagcgtggccgtcgcgccgctgttcaaaacgggcgcctcgctgcactacgtcgacaacggcatcgactccggcgaggtgatccacgacgcgctgcgcaccaccatcgaccccgaggacaccatcctcgagctgcgctggaacaacttcaaccacagcctcttccccgccctgcacgagggcctggccctgcttgcagagcagcggcaaccgctcaccgaaagaatcgcatgacgtccaccccccatgtttcctatgcggacggcatgccgcacgcgatcacgcgcgagggcgagatgctcagcgtgcgcaacacgcaggacagcacgcgctcgctctggaaagtcggccagggcagcacgctcgactgggtggacggcagcgatgcctccacgtcccatctgctggcggcgctcgaaggcgcgttcgaataccaaccgacgagcaagagcctcacggtcgccccgagccaaccggccgcggtgctcattcaggccggcgtgctgctgccggccgaaggcggcaaggccctcgcctgccgcgacatgctgtggcagcagccctcgctgtggctgcccaccgtgcatgcgcccatggcgctgcagtacgcgctgagcaacggcaagcgccaccccgtgcgcccgcccaagccgcgcggcgtgctctaccagcgcttcattccgtggctcggcaagaccttttcgtttcgcagcttcgacttcgaggccgacctcgcgatgttcaaccgctggatgaacgaccccgacgtggccgtgatctgggaggaagaaggcgacctcgacaagcaccgccagtacctttcggccatcgaccgcgacccgcacatgtattcgatgatcgcctgcctcgacgacgagcccttcggctacttcgagatgtactgggccaaggagagccgcatcgcgcccttctacgacgtggccgaccacgaccgcggctggcacgtgctgatcggcgagcccgcattccgcggcaaggccttcgccaccgcatggctcacctcgatctcgcactacatctttttgtgcgacccgcgcacccagcgtgccgtgggcgagccgcgcatcgaccacctgcagcagatccgaaacctcgacaagtccggctacgccaaggtgaaggagttcgacctgccgcacaagcgcgcgctgctcgtggtgatgctgcgcgaacgctatttcaccgacgccctgtggctgccccgcagcgacggcgccgccacgcctgcccaacactctgcgtaaaggaaaaaccgccatggtgattcacgacctcatcggcatcggcttcggcccttcgaacatcgcgctggccattgcgctggacgagaaacgccgcgacggccgccgcgtcgatgcgatgttcatcgagaagcaggccggcttcgcctggcacaaggacatgatgctggaccaggcgcacatgcagatctcgttcatgaaggacctggcgacgctgcgcaacccgaccagccgcttcaccttcatcaactacctgcacgagaagaagcgcctgcaggacttcatcaacctgaagaccttcttccccagccgccacgagttcaacgactacctgggctgggccgcggcccagttcgaggatgcctgcgtctacggcgaggaagtcttcgaggtgctgcccgaaaaagaaacgcatggcggcgaagtctcattgctgcgcgtgcgctctcgcgacggcgccggccacgtgaccgagcggctcacacgcaacctggtcgtcagcatcggcggcatgcccaacattccggagggcttcgggccgctcagggacgacccgcgcgtgttccattcgagcagctacctgcgggacatggcccgcctgcccgatgccgcaagaatcgccatcgtcggcgccggccagagcgcggccgagatcttcatggacctgcagggccggccgcacgcgccgcaggtcgacctgatcatgcgggcccgctcgatccgtccgtccgacgacagccccttcgtgaacgaggtgttcaacgtcgagttcaccgactacatctacagccaggccgaggacgagcgcgccgcgctgatcgacgagttcggccacaccaactacgcggtggccgacctcgacctgatccagcagatcttcaagatgttctacgaacagaaggtgcgcggcgagaaccgcatgcgcttcctgcgccggcacgagatccgcggcgtgcatgccacggtcgacggcgtccacctcaccctgtcggaccaggacaccggccgcgacagcacctcgcgctacgacgccgtggtgctggccaccgggtatgcgcgcgaacagcacaaggcgctgctgacgccgctcgctccgtacctgggagatttctcggtcgatcgccactaccgcctgggcagcacgccggacttccatcccgccatcttcctgcagggcgcctgcgagtcctcgcacgggctgagcgacacgctgctgtcggtcacctcggtgcgcacgggcgagatcggcaatgcgctgctcaagacgattccagcgggcacgccgacggcggccaatgccgcaaacagcgccctccgcgagcgccagccggtccgcgcgtaggcaagagctgcccccggggagggtaggcaaaaagaaaggagacagcccgctgtctccttttttttaagtcaaacgtctcatgtatggaagcaccaaggcgccggaatcggccgccttgggcgccgaaacgtgaacacgtcgtattcaagcaccctggagtcatcaaccttatgcgtcccctgccccgtcaacgtctgttgaataccgcgcttgccgcggctttcggcacagccttttcactttgcagcgtgagcgcctcggcgcaagccacgggacagcagccgcgtgccgccgacccgagcctgcccgcgatcaccgtgaacgccaccacggaagaatccgccaccggccacgtcaacggctacctcgccaagcgcagcatggccggcagcaagaccgacacgccgatcgtggagacgccgcagtcgatctcggtcatcacggccgaccgcatggacgccatcggcgccaccaacgtcaaggaggcgctcggctacacgcccggcgtcagcatcgcgcccttcggcgccgattcgcgctacgactggatcacgatccgcggcttcgacggctatgcgccgggcttctacctggacggcatgccgctgcgcaacaacggcacctggggcgtctggaagaccgagaactacggcaccgagcgcatcgaagtactgcgcggaccggcctcggtgctctacggcatggcaagcccgggcggcgtggtcaacatcgcgagcaagctgcccacggcggaacccctgcgcgaaatccagctgcagtacggcaacgatgcccgccgccaggtggccggcgacttctcgggcgcgctcgatgcggaaggcaaggtgctctaccgcatcaccggcgtgctgcgcgatgcccagctgcccggcggcagctcgcgcgacgaccgcacctacatcgcgccttcgatcacctggaagccatcgagcgacaccaccttcacgctgctggcccagtaccagaagaaccgcgcgggcgcctacagccgcatccgccccgtcgagggttcgctgacgccgacgcgcatcggcaccttcattcccagcgacctgaacgtcgccgacccgagcttcgatcacttcaaccaagaccagaagatgatcggctaccagctcgagcatcgcttcaacgacaccttcaccgtgcgtcagaagctgcgctacggcaagctcgaggtcgactaccggaccctgcagtcgccgagcttcgccaccatggacgccgccaatgcggtgaacccgatcaactaccagtacctgaaccgcggcgtcttcggcagccaggaaagcacgacgtccctcaccatggacaaccagttgcaggccgacctgcgttcgggcgactggcagcacaaggtgctgttgggcctggactaccagcgcacccgcatcgaccagtacacctacagcagcgtctccggcgcgccgctgctcgacatctacgcacccgtgtacggcagcgccatcgacacccccagcccctacgtcaacggcgtgagccgcctggcgcagaccggcatctacctgcaggaccagatcaagtggggcgaccgctggtcgctcacgctcggcggccgctacgacacggcccagagcagcgcctacagccggttcgacggcacgacgcaacgcatttccgagaacaagttcaccaagcgcgcgggcctggtctacctggcaccgaacggcctggcaccctacctgagctacgcggaatcgttcgcgccgaccggcgccatcgatccgacgacgaagacgcccttcaagccggaaagcggccgccagtacgaggccggcatccgctaccagccgccgggcggcaagtcgctctacagcgcggccatcttcgacctgcgccgcaagaactacatcacctacgacgcgacgttcatgccgaagcagaccggcgagatctcggtgcgcggcctcgaactcgaggccaccaccgaactcatgccgcgcctgaatctcacggcctcctatgcctacacgccgcgcgccatcgtcacggccagcagcagggtcgcggaaatcggcaagcaggcaacgtcggtgccgcgcaatcgcctgtcggtgtgggcggactaccgcttcagcaacggcctgaaggtgggcgtgggtgcgcgcttcaacggctcgacccatggcgacggggaaatcgtggcgccggccaaggtgccgtcgtacacgctgctcgacgccatgatcggctacgacatcgaccgctggactctggcactgaacctgcgcaacctgaccaacaagacctacatcgccaactgcgcctacggctattgctacctgggcacgcagcgcacggcggtggcgacggccacctatcgctggtaagcccggcgctccagagcaaaggccggatgccctcgcgggcatccggccttttttttgcgtgaggccgcggcgttgccgcgctaggcgggatcgagcgccagcaggcggcgcttcacggtggcgccgaactgcgcgtcgcggatgatgtccaggtgcccggtgcgcgcaaccacctcggtcgagagcacgcgcgcgcggtcgggccagcggcgcagggcacccggcgcctccagcgagcgctcggcatggaacacctgcaccggcaagtccgtcctggcctcctggtagcgcgccgactgcacgcggctgtcgagcgtggcccacagcaggtactcgtaggcctcgtcgcccgcaccgtcgagcggcgacacccaggcgggagccagcagttgctcggccacccaggtctgctcggcctcggtcatgcgggcgaacagctctttccattgcgccgccatgtccgacttggcaagccatgcggccagcacctcgtcggcctgcaggcgctgcgccggcgccaacgtgcccgccggaaccatcggctccgactcgaacacatcgaccgcgccgaagaacacgatctcgatgcgcccctgcagctgccgcgccacctcgaaagccaggtcgccgcccagcgaccagcccagcagtgcgcagcggccgccggtggcggttgcgacgatgaagtccgcatattcggccgcaagctcgcgaatggcaaagccgcgccagcgcttgcgcgtgtagacgtggctcacgaaggcatacaccggccggtcgccctgcaccgcgcgcgccagcggctggaactcgcgcgagttgacgatcaggcccggaaggcagaacagcggcacgcccgcaccgcccgcatgcaggcacaccgcatcgttcgcgctgtcggcccgttgttgcacgcgcgcggccagctcgcgaaggttgccggcctgcatcacatcggccaggctcaggtggctgccgccgggcagctgcttgcggacgagcgcgatcagcttgaggctcaggagggaatcgccgcccagctcgaagaagttgtcgttgcgccccacgcgcgccacgcccagcacctcgcgccagattccggccaatgcctcttcgacatcgccttctggtgcctcgtgggcgcgttcgctgcccagcccttccggctccggcagcgccttgcgatccaccttgccattggcgttcagcggcaggccgtcgagcacggcgaaggcgcgcggcaccatgtagtcgggcagcacctgggcaaggcgctccttgagcaccgcggtgtcgatggcctggcccgcatgcgccgcgatgtaggccaccagccgtgcgcccgccgggccgtccttcgccacgacgacggcttctcgcacctcgggctgcgcgagcagttgcgcctcgatctcgcccagttcgatgcgcaggccgcggatcttcacctggtggtcgatgcggcccaggtactcgatctgcccctcggcattccagcgcaccagatcgccggtgcggtagagccggccgccttggtggtcgaacggatcggccacgaagcgctcggcgctcaggcccggccggttcaggtagccgcgggccaggctcacgccgcccaggtacagctcgcccgcgacccccgggggcacccggttcagctcggcatccagcacatgggcgctggtgtggctgatcggctggccgatgggcacgaggctctggccatcatcccggcaggtccagcgcgtgacgtggatggtggtctcggtcggcccgtagaggttctgcagcgtcgcaccactgaggcgctgcagtgtctctttctgcgtctcggccggcatcgcctcgccgccgcagatgatgtggcgcagccgcgtgctggcctcgatgccttcgtgcgcaaggaaggcctgcagcatcgagggcacgaagttgagggtggtgacctggtggcgctggatgaggtccaccagccgggccgggtcgcggtggtcgccagggttggccaccaccagccgcgcgcccgcggtcatcggccagaacagctcccacaccgacacgtcgaagccgaacggggccttgtgcagcacggtgtcgtcgcgggtgaggccgtaggtgcgctgcatccaggccatgcagctgtgcagggcatggtggcggatggcggcgcccttgggctggccggtggagcccgaggtgtagatcacgtaggcgaggttctcgccgtgcagtgggacttgcggatcggcatcgggctcgttgccgaagtcgaggctgtcgatttccagcgtggtcaggcggctgcggtcgtgcaggcaggcgcgcgtggcgcggtgggccagcagcagctgaaggccgctgtcctgcaccatgtaggccaggcgttcggacgggtattccgggtccagcggcaggtaggcgccgccggccttgagcacgccgaggatggccaccaccagttcgaccgagcgctccatcgcgatgcccaccagcgtgtcgggcttgacgccgagcgcgatcaagcggtgggccaggcggttggcgcggcggttgagttcgctaaagctcagttcctcgtcgccgaagagcagcgcggtggagtccggctgcagtcgggcctgccgctcgatcaggcggtgcacgggctcggcccctggctcgcgctgcgtgttcacgctccatgcagtgagttgcgcctgctcgggcgcgtccatcagctcgacgtcgcccaccgcgtgcccgtcgtcgccggccagcgcaccgagcatcgcgacgtagtgcgcggtcatgcgttcgatggtggcgggctcgaacagctccgaggcatagatgaagcttgtgtgcagccgcccgtccgcatcctcgctggtgctcaacaccagttcgaactgagccaccggcgccgcgagtggatactcttccagttcaaggccgggcaactgcttcagcgtgcgggagtcggtccgctcgtggctgaacatcacctggaacagcgggctcacgctcaggctgcgctcgggctgcagcgcctccaccagttgttcgaacggaagatcctggtgcgcctgcgcgcccatcgcggcctccttcgcctgcgccagcactttggccagactcatgcggctttcgaccgcgctgcgcatgacctgcgtgttgacgaagagcccgatgacgccctccgtctccgcccgatggcggctggccaccgacacgccgacgcggatgtcctgctgcccggtgtatcgatgcagcagcgcctggaacgccgccagcagcaccgtgaagagcgtcgcgccctgggcgcgtgcgcgcttgtggaggccctgcaccagctccagcgcaagatcgacgccgtgcctcgctgccgtgtagtgcccactcggccgccggctgtggtccgttgccagttgcagcaccgggttgccggtgccgaggcgttcggtccagtaggcgagctgcgtatctttctcgcccgcctccagccagttgcgttgccatgccgcgtagtccgcgtagcgaatcggcagcggcggcagctccaacccttcgccgtgcactcgcgcacggtactgcgcgacgaactcgcccaccagaagatgcagcgaggcgccgtcggcaatgatgtgatgcatcaccagcacgagcacgtgcacctgcggcgcgagccggatcacgccgacccgcatcagcggacccgtcgtgagatcgaagggcgtcgcgctcaggcggcgggcttcttcgcgcgcatgcgcttccacatcgccctgcgcaccgaccagatcgatcaccggaatctcgagatcgacatggtcccgcacgatctgttcgcacagcccctgtgcatccggctggaacaccgtgcgcagcgaggcatggcgttcgagcagcgcggcaaaacttgtcttcagcgcctcgacgtccagcgtcccgtgcagcttcagcgcaccggagatgtggtacgccgtgctcttcgggtccagttgccaaagaaaccactggcgcatctgcgcataggaaagctcggcccgggttccggccggcagggccacgatgggcagcttggcaaagtccacgccctgcttttgcagcaggccgagaaacgccttctgcttttccgggggcaggcgcgcaaagcgatccgcaatgctgtgcttgtcgatctccatcaatcctccagaaggtcgagcagcgcggccatctgcgcgaggtcttcggaccctcccgccgccgctgtgcccacctcgtcctgcacgacgccggccatggcggccagcgtcgggttttcaaaatagcgcttgagcggcagctgcaccgcgaactgcttctgcaccttggtctgcacggccaagaggctcagcgagtggccgcccagctcgaagaagttgtcgttgcgcccgacgcgctccacctcgagcacctcggcccagatggcggcgagcgcgccctccacctctccaacgggcggcgcatacgcactgccgctcgccagctccgggtcgggcagcgccttgcggtcgaccttgccgttcgaattcaagggcacggcatcgagcaccatcaaggccgccggcaccatgtagtccggcagcttctgcagcagccgctcgcgcagcaccacggcatccgccgtctgccccgcccgcgcggacacataggccacgagccgcgtaccgcccgcaccctccttcgccagcacgaccgcttcgcgcacctcgggctgcgcaagcagctgcgcctcgatctcgccaagctcgatgcggaagccgcgaatcttcacctggtggtcgatgcgcccgaggtagtcgagctggccgtcgccgcgccagcgcacgaggtcgccggtgcgatagagccgcccacccaccgtgccgaagggggcggcgacgaagcgctccgcgctcaggccggcccggttcaggtagccacgcgccaggcccgcgcccgagacatgaagctcgcccgccacgccaacgggcagcggattgaggtcgctgtcgagcacccacaggccgaggtccggaatgcaggcgcccaccgggctgctctgttcgtcgaggtcggcgcgcacgatcggccggtaggtcacgtgcaccgtcgtttcggtgatgccgtacatgttgaccagctgcggctgctggtcgccgaagcgatcgatccatgggcgcaggctctcgggttcgagcgcctcgccgccgaagatcacgcagcgcagcggcaggcggtcgcccgcggccagcgccgcgctgtgcatcaattgacggaaggccgatggcgtctggttcagcacggtgactcgctgctcgcgcagcagcgccacgaaatcgccgggcgaacggctgacccagaacggcacgaccaccagcttgccgccggtgcacagtgcaccgaagatttcccacaccgagaaatcgaaggcataggagtggaagttcgtccacacgtcctgcgcaccgaagccgaaccagggctgcgtcgagtcgagcagccgcgtcacgttgcggtgggtcagctgcgttcccttggggcggccggtggagcccgaggtgtagatgacgtagaccaggtggtcggcatgcaccgccacctcgggcgcatgcgagggctccgcgctcaggtcggccgtgtcgagcgccagcacgcgcacgtcgtcctgcagcggaagcttcggcgtcacatggctttgcgtcagcagcaggcggatgccgctgtccgcgatcatgtaggccaggcgatcggcggggtactcggggtcgagcggcacgtaggcaccaccggccttcaggatgccgagcaggcccaccaccatctcgatggagcgttccaccgcgatgcccaccttcacctccggccccacgccaaggctgatcagccggtgcgcgagccggttggcgcgcgcgtcgagttcggcgtagctcaggctttcattgccgaagaccaccgccgttgcattcgcatgcagtgcggcctgccgttcgaaccagcgatgcacgggcaactcggtgtcgccggcgtgcaggtctttcactgattcgagttgtgatgaatcgttttcatcctgcaggccgatatcgcccacccgcgcacctggtgcatgcgcaagcgcttcgagcagcgtctccatccggtcggccagcgtccgaaccatcgcttcatcgaactggctgcgtgcatggctgtagctcagcaccagcgtctcgccctggttcaccgacagcgtcatcgggtagttcgtctcttcgcggttccatacctcgccgaagcgcaaccggtccggcgcgccccgcgtcagcgcctggtccagcggatagttctcgaacaccacgatgctgtcgaacaggtcttggccgccctgccccgcccaacgctgaatctcgtagagcggcgtgtgctcgtgcgcctgcgcaccgaggttccgggcctgcagcgcgcgcagccaatcgcccacgcgctgcgccggctgcagcgtggcgatcaccggcagcgtgttgatgaaaaggcccagcatctgctgcgcaccgggcagctcgatcggcctgcccgccacggtggcgccgaagctcaccgtgcgctgccccgtgtggcgcgccagcagcaaggcccatgcggcctgcaccagcgtgttgagggtcacgcgttcgcgcttcgccgcttccatcagcgcgcgcgtgcgctgcgctccaatctcaaagcgctgcatgccgccatgacctgcctgcgcatcgcgcggcttgggcagggtgttggcgagccatgtggggccttcgacgccgcccagctgttcgcgccagtagcgctcgtcggcctcgccgtcgcgctgctgcagccacgcgatgtagtccgcgtagcgtccgccctgggatgcaagagcttcgccggcatagtgccgcagcatctcgcccatcagctgcgaggtgctccagccgtccagcagcaggtggtgcatggtccagacgaagtggtgcttgccgcctggcgtatgcaccagcacgagccgcatcagcggcggctgggccagatcgaagccttgcgcgagctgtgcctgcgccaggtcatcgagcgcgcgggccacgtcgccacggttccgccagtcgtgctcggccatcggcaactcgatcttccgggccacccattggagggcgggctcacccaccaggaaaccggtgcgcagcacctcgtgccgctccagcagcgcgcgccatgcggccttgaagcgcgcgacgtcgagcccgtcgatgtcgacgcgcaactggttcacgtaggcgctgcctccaggcgcatacaggctgtggaacagcatgccggcctgcatcggcgaaagcgggtacaggtccgccaggttcgctgccggaaccggcaaggcatcgagctgctgcgggccgatgcgcgccagcggaaagtccgacggcgtcacgccctctgcgccgctggtgcaatgcgccaccagcgcttcgagctcctgctggaagcgctgcacccagccttccactgcaccgcggtcgtggcgcgcctggctgtagctcacgcgcagttcgagcacgccttcgtggacctggccgttgaccgcgaactcgtgcgtcagcggtgcgcctgcatccaccggcgcaccgctcggttcctgggccagcacccattgcgcacgctcgtcgaaaccggcgtcgaactggccgaggtagttgaagaccacctgtgcacggggcaacgcgcgcagcgcctgttgctgcgcagcgctgacgaggtgcttgagcacaccgtgtcccagccccttgtcgggaatgcggcgcaggctttccttcacgcgcttgatggcttcgctcggttctcccagcggatcgagcgcgaccgggaacaacgtggtgaaccagcccacggtgcgcgacaggtcgatgtggtcgaacaggtcttcgcggccatgcccctccagatcgaccagcaccttggcgtggcccgcccatgcgcacagcgcacggcccagcgcggtcaacagcaggtcgttggcctgcgtgcgataggccgcgggtgcgtccttcagcagcgcctgcgtcgtcgccttgtccagccgaagctcgacggtctgctggtcggcgacggtgttcgatgcgtcggggtgggcacacggcaggctcgcgggcacgtccgccagcgcttgccaatggccgatcccttcggcatggcgctgggcgtagccctgcagtgcgacggtccaatccttgtagctgctgctcttggcgggcagcacgatgggctgccccgcaaggcggtggcggtaggcgtcctgcaggtcttccagcaggatgcgccacgacacgccatcgacaaccatgtggtgaatggccagcagcagccgcgattcgccgcccggcagttcgaccgcgagcgcgcgcagcagcggtccgcgcgcaagatcgagactgcgctgcgcttcgtcgcagagcgcttcaagctgcgccgcatcgcgggccttgcgcacccacagcagttcggcgagttcgctgtccggcatcgcggtgtagtgctggtgccatgtgccttggtcatcctggctgtagcgcaggcccaggctgtcgtggtgccgcaccacggcctgcaatgcctgcccgaaggccggcagctgcaaaggctcgcggcacttcagcagcaccgcctggttccagtggttgcgcaccggcatctgcatttcgaagaaggcatgctggaacggcagcagcggcgcctcgccctcggcatcgccggcagccgtgcgcttcgcatcgcccaccggttcggccgcgcccgcgagctgggccacggtctggcgctcgaagatctgcttggggctcaccttccagcccgcgaggcgcagccgcgccacgatctgcaggctcaggatggaatcgccacccagttcgaagaagttgtcgttccggcctacgcgttccaggccgagcacgccggtccagaccttcgcgatggcctgttcggcctcgccctgcggcgcttcgtacgccttctcgtcctgcaggagttcgggctccggcagggcctgccggtcgaccttgccgttcgggctcagcggtagcgcgccgagcaccacgatggccgaaggcaccatgtagtcgggcagcgcccgagcgagccgatccttcagtgccgccacatcgacggattgccccgccttcagcgacacataggctgcaagccgtgcgccggccggcccgtggcgagcgatcaccacggcttcacgcacttcaggctgggccagcagctgggcctcgatctcgcccagctcgatgcggaacccgcggaccttcacctggtggtcgatgcgacccaggtattcgagctggccgtcgtcgcgccagcgcacccagtcgcccgtccggtacaaccgcccgccgtccgcgtcgaagggatccgccacgaaacgctcggccgtgagcgcggcgcggcgcaggtagccgcgcgccagaccggcgccgccgaggtacagctcgcccgcgacgttgcgcggcacgaggttgaggtcggcatcgagcacgcgcgcgctgcggtcgcccacgggccggccgatgggcgcgtagccttcttcgaaactcgccgcgccatcgaccttccacagcatcggcgtaaccaccgcttcggtagggccgtagccgttgatcagcagctggggcttcagatggcggcgcaccgcgtcgaagccttcgcgcgacatcgcttcgccgccgaacgaatacagctgcaccggcgggcaacggccggtgtcgcgtgcccagtctgcgagctgccgcaggtaggccggaggaaagccggcattggtcacgcggtggcgcgtcatcgcgtccagcgtctgctcggcggtccacagcgatgcatcgcgcagcagcagcgaggcgccgcagcacagggccgtgaagaggcgttcgtgcgcaccgtcgaaggagaacgagagaaagtgcagctcgcaggagtgcggccccatctcgtacagcacggccgtttccacgcaatgtgcggcaaagggtccgtgcgacaccatcacgcccttgggcatgccggtcgagcccgaggtgtagatgatgtaggccaggttgtcgccatgcaccggaacgtggggcgaatgcactggctcggcggacaggtccagcgtgtcgagctgcagcacgcgcacgtggtcgccgcaggggatgcgcgccttcacgtggctttgcgtcacgagcaggtcgatgccgctgtccgcaaccatgtaggccagccggtccgcggggtactccgggtccagcggcacgtaggcgccgccggccttcaggatgccgagcaggccgaccaccacgtcgaaagaccgctccaccgcgatgccgacgcgcgtgtccggcctcacgccgagcgcgatcagccgatgggccaggcggttggcgcggcggtcgagttcggcgtaagtcaacgtctcgtcgccaaacagcagcgccgtggcctcggggcgctcgtgcgcctgccgctccatcaggcgatgcacgggctcgctgccctgctcgtccggggcgttgacgccccattgcgcgagccgttctttctcggcgggcgcaagcaggtcgacgtcgccgaccgcctgcgccggactgtcggccagcgcgcccagcaccgccaggtagtgccccgccatctgcgccatggtctccgcgtcgaacagctcctctgcatagtgaaagctggcctgcacatggccctgggcgtcttcgatgatgctcagcgtgagttcgaactgcgcggcctgcccgcccagctcgtggtcctgcaaggtcaggccgggcaggttctgcagcgcgcgatggtcgcgccgctggtggttgaacatcacctggaacaacggcgccgtgccaaggctgcgctcgggctgcagggcctccaccagctgttcgaaaggcaggtcctggtgcgactgcgcgcccagcgccgcatcgcgcgtggcttccagcgcctgcagcaggctggtgcggctggtcagcacgttgcgcaggacctgggtgttgacgaagaagccgatgaccttttcggcctccacgcgatggcggttggcaaccggcacgccgatgcggatgtcctgctgcgcggtgtggcggtgcagcagcacctgcagccccgtgagcagcaccatgaagagcgtggcgccctgggcctgcgcgcgcttgtgcagtgcatccaccaccttctgcggcagggccacgtcatggcgggcggcgcggtatcggccatcggtgcgccgcgggcggtccgtcggcaattgcagcaccgggtgttcggtgccgaggtgcgccttccagtagccgagttgccgctctttctcgccggcctccagccagtgccgctgccagacggcgtagtcggcgtactgaatgggcaaaggcgcaagccgcgacggctgcccgttggcccgcgcgcggtagtgcgccgtgaactcgtccacgaggatctgcagcgaccagccgtcggacacgatgtgatgcatcacgaccacgagcaggtgcgcgttttcctcaagccggatcagcgccacccggagcagcggatcggccgtcaggtcgaagggcgtctcggcgatgcgccgggcttcttgctgcgcccgcgcatcgcgctctccatccgcgagcgcgccaaggtcgatgagcggaatgtccagccccgcgcgctgctgcaccacctgctcgaccaggccttcggcgttcgcgcggaacaccgtgcgcagcgactcatggcgttcgaccagggcgtcgaaactgacctgcagcgcatcgcggttcagcgcgccctcaagccggagcgcacccgagatgtgatacgccgaactgcccggctccagctgccagaggaaccactggcgcatctgggcatacgagggcgggcaggcgacgcgcgccgcctcgtcgcgttggagaatcggaaactgcccgatcgtcagcccttcggcgcggatcttctggtacaccgcccggcgctgcgccgggttcaggcgcgagaagcgcttgccgatctggtcatgggtggctgccgtgaattccatcaagcgatctccaggctgtccatgaaggcgtcgatgtcggagagagactgggccacgggtttcctttcgccggcacctgcaatgagtcgggccatgtccaagagaaccggctgcctgaaaatgtcgctgacggtcaggtccgcgtgcatcgcgccctgcacccgcgcgaccacctgcacggacatgagcgaatgcccgccgagctcgaagaagttgtcgtggcggcccacgcccggcacgccgagcacctcggcccacaccgcagcaagcgcttcttccacggcgccctgcggcgcctcgtaggcctgggcgttcgcgcgctcgggttcgggcagcgccttgcggtcgaccttgccgttggcgttcagcggcagagtctccagcaccatgaagagactgggcaccatgtagtcgggcagcgcccggccgaggcgttcgcgcaggcgcgcggtgtcgatggcctcaccggcctgcgccgaaacataggccacgagccgcgcgccgcccgcgccctggctcgcaacgacgacggcctcgcgcacttcgggctgcgcgagcagctgcgcctcgatctcgcccagctcgatgcgaaagccgcggatcttcacctggtgatcgatgcggcccaggtagtcgagctggccttcgctgttccagcgcaccaggtcgccggtgcggtacagcctgccaccgccgtcgccgtcgccgtcgaacggatcggccacgaagcgctcggcggtcaacgccgcgcgctgcacgtagccccgcgcgagccccgcaccgcccaggtatagctcgcccgcggcgcccggcggcatcaggttcagctcggcgtcgagcacataggtttgcgtgtcgtcgatcggccgcccgatcggcacctgcgtgcgtccgtcgtcgcggcagctccagtgcgtcacgtcgatggccgcctcggtggggccatacaggttgtagagcgcggcctgcggcagccgcctgaacacctcgttctgcgcttcggccggcagtgcctcgccgctgcagacgatccgccgcaggctggtgcacgcctcgatgcccgggtgcgccagaaaggcctggagcatcgagggcacgaagtgcagcgtgctcacttgatgcgtgcggatcagctgcgcaaggtgcgccggttctcggtggtcgccggggttggccacggccagccgggcgccgaacatcagcggccagaagaactcccacaccgacacgtcgaagctgaacggcgtcttctgcagcacggtgtccgcctcgccgagcttgtaagactgctgcatccacaccaggcggttgtagagcgaaccatgtcggttggctgcgcccttgggcttgccggtcgaacccgaggtgtagatcacgtaggcgaggttctcgctgtcgagcgccaccgccgggttgctttccagatagccgccgaggtccagcgtgtcgagcgtgagcatcggcacgccggtctgcagcggcaggcgttccttgaggcgctcctgcgtcaacaccagcgcgagcccgctgtcttccaccatgtaggcgatgcggtccgcggggtattccgggtcgagcggcacataagcgccgcccgccttcagaatggccaagaggccgaccaccagctcgatgctgcgctccagcgcgacgccgaccttcacctcggggcgcacaccctgctcgatcaggcgatgcgccaattggttggcccggcggtcgagttcgccgtagctcaagacttccgcgtcgaagatcagcgcagtggcattcggacactcggccgcctgttgctcgatcaggcgatgcacgcattgcgcttcgccgcggcgatgggtgttgacgccccattgcgcgagccgggcgcgctccgcatcgcccaacagatccagttcgccgagcttcgaaaccggcagtttcaccagcgcttcgagcacgcgcttgtagtggccggccatgcgttcgacagtctccggctcgaacagctcggccgcatagcggaagttggcccggatgccgccgtcttcgcgttcgatggtttccagcgtcagctcgaagggcgccgcgcgctcctccagatcgatgcgccgcacctgcagaccgggccagccgcgcagcgggcggtcgccctgccccaggtggttgaacatcacctggaacagcggcgcggccgcgtgcccgtgctccgcgcgcagcgtctgcacgaggcgttcgaacggcaggtcctggtgcgcctgggcctcgatggcggtgtcgcggacttgcgcgagcaattcggccaggctcgtctgcgcgtgcaggcgcgcatcgagcacgagcgtgttgatgaagatgccgatgacgcccgcggtttccggacgactgcggcccgcaacaggcacgccgacgcgaatctcgttctggccggtgtagcggaacagcagggcatggaaggccgcgagcagcgtcatgaacaaggtgccgccctgcgcacgcgacagctgcttcagttcctgcgcaagacccatgggaatgtcgagcgaatgctgcgccgcgctgtagtgggcctcggcggaacgcggctggtcggtagtcagggagagcaccggctggctgccaccgagacgctcgcgccagtagccgagctgccgctcgccttcgccgtcggcaagccacttgcgctgccacagcgtgaagtcgacatagccgatctccggccccggctgcgcgctctgtgcgccctgcgttcgcgcggcataagcctgcgcgagctcgtccagcatgagctcgaccgaccatgcatcggaaatgatgtggtgcatcatgagcagcaactggtgctcgccatcggccatcttgagcaaggcgcagcgcagcaaggggccggccgtcaggtcgaaggcggtgcggcagacctggtccaccgcgtcgccgtagcgggattcgcgcgcggccgcatcgagcacgctgagatcgacgaagggaatgtcgatgcggacttccgcctggacgcgctgctccggcaggccttcggggccggggccgaacacggtgcgcaaggcttcatggcgcctggcgagcgactgcatcgcatcctgcagcgccgttacatcgagcggccccgaaaaaccaagtccaccaccaacgtggtaagccgtgttcgcagggttcagctgccacaggaaccactggccctgctgcgcgaaggacacgggcacggggccgtcgatgtggctgcgcacgatggcctcgcgcgcgggcgccgcgttgccgcccggtttcaagcggcgctgcagcaggctcagctgctcgggcgacagcttcgcgcgccgttcggaaagaggggatgtttcgctcatgatgaaaaactcgcagtgatgcgatccgctggcggatgcgggtcgtcggtggccggggcttcgcgctcgatctcctcgatcagccgcagctcgaccaacgcggccagctcggccaccgtcggtgccttgaagaaatcggccggttgcagctctacgccgtaggccttgcgcacacgggacagcaggcggatggccagcagcgaatcgccgcccagctcgaacaggttgtcgtgtgcgcccacgggcgcgatgccgagggcttcggtccacagcgcggccagcccttcttccagttcgccttcgggtgcggcatacggtgtgggcagcgcgggacgtgcatggctggtgcgggcttcggccgacggcgcggtgtcttgggcttccaccgcgtcgagcagattgccgagcgggcgcaggcgcggcgccagcggcgacacggaaaccaccgtctgaggcaggtcggggccgttgacgatgcgctcgaaggcgagcacgccggtgcgctcgtcgaggccgacgccttcgggcaggttcatgtcggccgcggcgccgacgtcgcgccaggcgtcccagttcaccgagaacaccggcagcgccgacgtgcggcggtgggccgttgccagtgcatcgagaaaggcattggcggcggcatagtcgctgcggctcaggccgccgacgagcgtggcgatggaggaacagaagagcacgaagtccaacggctcgccgcgcagtgcgtcgagcaatgcgcgcgtgcccgccaccttgggcgcgaaggctgcctccacctgagcccaggtgcgctgcacgatcatgccgagccccgggtccatcacagcgtggaccacgccgttgaccgcgccgaagcgcgcatgcgccgccgccagggcttcgcgcagctgggcggggtcggtcacgtccgccgtcaccgtgagcacttgcgcgccggcggtttcgagttcgatcagttggcgcagcttgcggcgcaatgccgcgggttcgtcggtcgaggcggcgatgcgctcccagtcgacgcgcgcaggcaatggcgtgcggccgagcagcaccagccgggccttccatgcgcggctcagatgccgcgccagcgccaggccgacgccgcccatgccgccggtgatgaggtacacgccgccctcgcggagccgctgcgtggcgcgttgcatcggcaatggctcgtagttcttggtccagcgatgcggcccgcggtaggcgaccacgaaatcatcgtgtgcggatgcggcctcgtcggcgacccggcgtgccaggtcgctttccgccgcgctttccggcgcgggcagcaccacgtcgacgacgcggcaggcgatcgacggatattcctggcccacgaccttggcgatgccgagcagcgttgccttctcgggtgccagcacctcggtgcctgaaacgtcctcgaggccgtcggtgacgatggtcagcgccattggcgcgcggcccgatccacccaaggcgtcgagcgcatgcacgagcgcgagcaggctgaagtaaccggcttcgaagacgcctgcatgcggcggcggcgcggaccggccgccgtcgaggctccacagatgatgaatccgatggacagcgcccgcttcggcttccacttcccgcagcagggcttcgtggtcggcgcgttcgccttgtcgaatcgtgtattgccgcggcgcagtgcgcgcaaagcgcgagcctcgcagtgccagcaccacctgttcgccgcgatcccgcagcgtgcgggccaagcggtcggtgaagctatcggcgtcgcccaggatcagcgtgcagcccgtgcggtcggcttgctctgcggcgggcggcaacaacggcgtgcttcgctgccagttcggcgcatagaaaagatcggcggccgcagccggcgacgagggccgtacggcggccccggcctcgacccagaagcgctggcgctggaaggcataggtgggcagcggcacgcggcgcctctcgccgccttcgtggcatgcggtccagtcgatgtcgatgccggcggtccacaggcccgcgacggcattcgccaactgctggctgttgcgcgcggtctgctgtgcatgcgcctggctggcccacaggccggcggctgagctgctgcccggatgctgtcgcgccagccctgtcagcatctcgccggggccgacttcgagcaccacgcgcccgggcttgctgaagatgtggcgcagcccatcggcgaagcgcacggtattgcgcaagtgccggccccagtacgcggggctggtcgcctcctgcgcggtgatcggttcaccggtcaggttcgaaatgaaaggaatgcgcggcgcgtgacgcggcaccgaagcgaccagttgctccagcgcggccaccgccggatcgaccagccgcgaatggaaggccacggcgacatgcaggcgacgcggcagatgctggcgcgcgcgcaatgcttcctcggcatgcgcgatggcttcgggcgtgccggccagcacgcagagctgctcgccgttcaccgccgcgaggtcgcagcctgccgcaaggaaaggcgcgagctcggattcaggcagcggcaccgcgagcatcgcgccggccggcagcgcctgcacgaggcgcgcgcgctgcgcgacgatgcgtagcgcgtcttccagcgaaaagacgcccgccacgcaggcggcgacgtattcgccgaggctgtgacccatcatcagcgcgggcttcacactgctgtgcagccaccattgcgccatcgcatactcgacagcaaagagcgccggctgcgcgacctcgatgtggaacaggcgctcgttcgccagcgcctcttcgccggcggctggaaacagcagcgggtgcaggtcgatgccgctttgcgcgcgcagcaaggcgatgcagcgatcgagcgcctcgcggaacacggcgcgttcgcggtagagcgccgcgcccatgaaggcatgctggctgccgctgcccggaaacagaaagaccacctcgggcgctgagagcggtgccttgcgcggtgcggcggcgggagccgacaacatctgtgcggccatctccggatcgttcgccaccacggcgctgcgccatgcaaaggcgcggcgcccggtttgcagcgtgtgggccacgtcttgcagcggctgtgcgggccgtgcctgcagatgcgccgcgagctgtgtgcgcccttgcgccaaggcagcttcgctcttggccgagacgggcaagacctgccatcccggcgccgtcgccgcatttgcaacggccggtgcttcttcgagcacgacgtgcacgttggtgccgccgatgccgaaagagctcacgcccgcacgccgcggcatgcgcccctcggcccacgcgcgcgcttcggtattcacatagaacgggctcgccgcgaaatcgatctgcggattgggctgttcgaaatgcaggcttggcggcagcacgcggtgcttgagcgccatcgtcgccttgatgagccccgccacgccggcggccgcgtcgaggtggccgatgttggtcttcacggagccgatggcgcagaagccgcgccgctcggtatcggcgcgaaaggcctgggtcagcgcggcgatctcgatcgggtcgccgagcgtggtgccggtgccgtgcgcctccacgtagccgatggtgtccgccgccacgcccgcgatgagctgcgccgcgcggatgacttcggcctgcccatccacgctgggcgcggtgaagcccaccttggcggcaccgtcgttgttggcggccgagcccttgatcaccgcatggatggcgtcgccgtcgcgcagcgcatcgtccaggcgcttgagcacgaccacgccggcgccgctgccgatgagcgtgcccgcggccttggcgtcgaaggcgcggcaatgaccgtcgggcgacaggatggcgccggcctggtagcgatagccgccctcttgcagcaggttgagccacacgccgcccgccagggccatgtcgcagtcgtggcccagcagcgcctggcacgcggtgtgcaccgcgaccagcgacgtcgagcatgccgtctgcacggtgaccgcggggccgcgcaggtcgagcttgtaggcgacgcgggtgcacagcgagccgccggagttgccgttcatcagcccgagcaggtcggcaatgccgctctccgcgccgaggccgaaggatggcagcaggttgcggatcaggtacaggttggtgccctcgcccgcatagacgccgaccttgccgggccagcgcgcgacgtcgcagccggcgtgttcgagcgaagcccaggcgcactccaggaagacgcgctgctgcggatcgagggtctcggcctcgcgcggcgtgtagccgaagaagccggcgtcgaactggtcgaagccgtcgaacgtcacgccggccttcacgtactcgggatcgtccagcaagctctgcggcacgccgcgcgcgcgcagttcgtcgtcggtgaagcgcgagaccgactccacgccatcacgcacgttgcgccagaaagcgtccacgtcatcggcgccgggaaagcgcccggccatgccgacgatggcgatctcgatgccggtcggttcggagaactcttgggagttggacatcagttgactctctctgctgtcttgcggcgttgaagcatggcggcgcgctggcgcaatgcccggtcgtcgccagctgcggcagacgacgcggcaccggccggcgcctgctcgatccactgggccagcgattcgatggtggggtacttgaagaggttgaccacggggatcgtggcctgcagccggtcttccagcaggcggtgcgcgcggatcagcagcagcgagtggccgccgagatcgaagaagttgtcgtgctgcccgacctgttcgacctgcagcacctcggcccacaccgcggccaccgtctgcgccacgtggccctgcggtgtttcgtaggcaagctcgctggcgaagacgagctccggcagcgccttgcggtccaccttgccattggcgttcagcggcaggccgtcgagcacggcgaaggcgcgcggcaccatgtagtcgggcagcacctgtgccagacgttccttcagcaccgcagtgtcgatggcctggcccgcatgcgccgcaaggtaggccaccaggcgtgcgccggccggaccgtccttcgccaccactaccgcctcgcgcacttcgggctgcgcgagcagttgcgcctcgatctcgcccaactcgatgcgcaggccgcggatcttcacctggtggtcgatgcggcccaggtactcgatctggccctcggtgttccagcgcaccaggtcgccggtgcgatacagcctgcctcccttgccgtcgaacggatcggccacgaagcgctcggcgctcaggcccggccggttcaggtagccgcgggccaggctcacgccgcccaggtacagctcgcccgcgacccccgggggcacccggttcagctcggcatccagcacatgggcgctggtgtggctgatcggctggccgatgggcacgagactctggccactgtcatcgggatacaggcggcaggtccagcgcgtgacgtggatcgtggtttcggtcgggccgtagaggttctgcagcgtggcaccgcgcaggcgttgcagcgtctccttctgcgtttcggccggcatcgcctcgccgccacagatgatgtggcgcagccgcgtgctggcgtcgatgccttcgtgcgcaagaaaggcctgcagcatggagggcacgaagttgagggtggtgacctggtggcgctggatgaggtcgaccagccgggccgggtcgcggtggtcgccagggttggccaccaccagccgcacgcccgcggtcattggccagaacagctcccacaccgagacgtcgaagccgaacggggccttgtgcagcacggtgtcgtcgcgggtgaggccgtaggtgcgctgcatccaggccatgcagctgtgcagcgcgtcgtgccggatggcggcgcccttgggctggccggtggagcccgaggtgtagatcacgtaggcgaggttctcgccgtgcaacgcgacctggggatcggcgtcgggctcgttgccgaagtcgaggctgtcgatttccagcgtggtcaggcggctgcggtcgtgcaggcaggcgcgcgtggcgcggtgggccagcagcagctgaaggccactgtcctgcaccatgtaggccaggcgctcggcggggtagtccgggtccaacggcaggtaggcgccgccggccttgaggatgccgaggatggccaccaccagttcgaccgagcgctccatcgcgatgcccaccagtgcatcgggcttgacgcccagggcgatcaggcggtgggccaggcggttggcgcggcggttgagttcgctgaagctcagttcctcgtcgccgaagagcagcgcggtggcattcggctgcagccgggcctgccgctcgatcaggcgatgcacgggctcgtgctgcggctcccgctgcgcgttcacgctccatgcagtgagttgcgcctgctcggatgcgccgaggagttcgatgtcgcccaccggctggtcaggacgatcggccagcgcctgcaggatggcgacgtagtggccggccatccgctcgatggtgtcctgctcgaacagctcggccgcatagatcaccgcgagcgacagatggccgtcgggcctctcgcgcgcttcgagcgtgagctcgaactgcgccgcgagatcgggcagtgcgtggtcctgtgccgcgataccgggcagctgcgcgaatgcgcggtagtcctcgaacagatggttgaacatgacctggaacaggggcgtgcggctcaggctgcgttcgggttgcagtgcctgcaccaactgctcgaaaggcaggtcctggttcgcctgcgcgcccagcaccgcctcgcgcgcctgcgccagtacacgcgatgcactcaggcggccgtggatcgggttgcgcagcaccagggtgttgacgaagagcccgaccacgccctcgacctccacgcggttgcggttggcaatcggcgcgccgatgcgtatgtcttcctgccccgtgtggcggtgcagcagcgactggaagcctgcgagcagcgccatgaagagcgtcgcgccctgggtgtccgccatgccgcgcagcttgtcgagcaggttggcaggcagctcgaaggcatggcgcgcggcgctgtagccggcctgtgccttgcgcggatggtcggtgcgcaaatccagcgctgcgtgcgtgtcaccgaggtgcgcgcgccaccaggccagctgccgctcgccctcgccggccgcaagccactcgcgctgccagagcgcgtagtcggcgtactggatgcgcggcgcaggcagtcgcctggcttctccacccagatgtgcggcgtagccggcggccagttcgtcgatcagcaactgcatcgaggcgccgtcggaaatgatgtggtgcatcaccacggcgagcacatgggtctcgtcggcggtgcggatcagcgcggcacgcaacagcggaccctgcgtcagatcgaagggctcggccttgaggcgccgtgttgcttctgtcagttgctcctcgcgctccccgcgcaagtcgatcatcgccagcggcacggagcccgagggcttgacccattgctccgcatggccatcggcggcagcgctgaataccgtgcgcagcgattcgtggcgcgtgacgaggccatcgagcgcggcgcgcaaggcatctgcgttcaacgctcccgtgagtcgaagcgcgccactcatgtgataggccgcactgtgcggatcgacccgccagagaaaccactggcgctcctgcgcgtgggagagcggcatcggcaacagccggcgctctgccgagagcacgggaatcggtgcacgctgcgggcgcacgccttgcgcctgcagttgccggatggccgctgcgcaagcctgcaggcgcggctgctcgaacagcatccgcgccggaaagtcgatctgccaatgcgccgagatgcgcgcggccgcctgcgtggccgtaagggaactgccaccacggttgaagaagtgggcatcgcgagccagcgcgcggtcgtcgtcgccatgtttccagacctcgcgccagatgtcggcgaggacctgctcgacctcgtccagcggcgcctcgggcgctgcctcgctgggcccgccccgcacgaaggcaccgtgctggtagatcgcatacgcgtcggcagtcccgtcgatccagcctgcgcggcaggcgctgcgctgcagcttgccgctggtcgtcttggggaggccgccggggttgagcagcagcacgaccgacagcggctcgccgaacatctcgctcacggcggcgccgagcgcatcgaccagcacctccggcggcaccagcttctgcatgctgcgcgacacctcggccgcgacgccgatgccttcgccgccggcaccctgcaccgcaaagaccgccacacggctcttgcgcaccgcgtcgacctcggcctcgatgagccgctcgatgtcctgcgggtagatgttgtggccgcggacgatgatcaggtccttgatccgccccgtgacgtagagctggccttcgtgcatgaagccgaggtcgccggttcgcagccagcgctggccgtcgcgcaggacgaaggtctcgcgggtctcgcgctccttgccccagtagccgaggcagatgctcgggccgcaggtccagatttcaccgatctttccggatgccgccggcagcagcgactcgacgtcgacgatctcgacccgatgccctggggccgcgacgccgcagccgaccagcatcgtgccctcgtcggccggcgtgccggtgccgcgggccaggccgtcggtggagaaggtgcgcgccgtcatgccgtcgccgcgcatgccgccggtgacgaacagggtgccctcggccaggccgtagcaggggtaggcggctcgcgcgtcgaagcccgcggcagcaaagcgcgcgatgaattcggtttcggtgtcttcgcgcacgggctccgcgcccgtgtaggccacgcgccagctcgacaggtcaagctgcgccagccgcgcatcgttcactcgctcgagacagaggcggaaggaaaaatcgggcccgccgctgtgggtggcacgatggcgcgagatcagctcgagccagcgcaccgggcgctcgagaaagtagcccggcgaagtgagcaccagcggaatgctgttgtagagcggcagcagcagcccgccgatcaggcccatgtcgtgatagagcggcgcccagcagacgaacttgtcttcgggcctcacgcccatgccgtgcgtcatggccgcttcgttggcgaccaggttgccgtgcgtcaccatcacgcccttgggcgcagaggtcgaacccgaggtgtactgcaggaacgcgatgtcgtcgtcggtgggatcgaacggcgtccattcatcggcaagcgccgcatccaccgcatcgacggcgatgatctcggcgcctccgaactggcccgcgcccgcattcatcgcgcgcgaaatggcggcggaggtcagcacgcagtgcgcctctgaatcggtggcaatgccagtgagccgcgccaggtgctgcggccgcatggactcgggcgggaacaccggcaccgcgatcacgccgctgtagaagcaggccagcatgcagaccgcatagtggtcgccgttgtcgagcatgatgagcgcgcgctcccccttggcaaactgctgctgcaaccgggccgcaagggcgcgcacgcggcgctcgaagacgccgtagctgatcgggtcttcgtggtattcaccgttcaccgtgccggccacggtgagccagatgtcgtcagtccgcgtgcgtgccagcgcgcgcagatgggcgacaaaattcttcggctgcaggtttgccttttgcggcatctcggtcatgtcgtttcttcctttgcgcgccaagcgagcgcggctgcgtagccggtgggcgccctgagcgccacggcttgaaaattcgtccattcgggaacggcgcattcgagggcgaagcgcccgttcgtgccgggccggatgccgatcgacttcaggtgcccggccacgccgacgccgatggctttgagcaccgcttccttgcccacccagcgggtgtagagcgcatgcaggcgattggcggcatcgcgcacttcgccgcattcgcgggcggtgaatgccagcgaggagatggcctcgacgtcgacatcggccttgcacgcttcgatgtcgatgccgatctcggtcacgctccgtgcatcgcccagcgcgatgagtgcatgcgacccggagtgcgagacgttgaactgcggcgcgccaccgcctgcacgctcgatgagcggcttgccgtgcgggctcgccacaagcggcacctcggcgggctcgcagcccacgcgcgatgcaagcagattgcgaagcgcggcacgtgtcgcggtgaagcgcacgcggtcggcggttcttgcaaacctgtcggcctttgcaagctcgtcgggcgtcagcacccgccgcgccgccggtgcctcaacggtcaggtcgaagtcgaggcgatacacctcgatgcccgcgggcagcggatcaggccagggcgtgagatgcatggcgatcccgtgcgacgacctttccgaggcgctgcgagagcgccgccagaaatgccgtttcctgctggcggaggaagaagtgcccgccgctgaaccagtcgagcgaaaaggcaccacccgcctcggccgaccacgcgtagatgcgctcggcttcgatctcatcgtcgcgccccgcgaagacgtgcaccggcatcggcagcggcgcctcgcccgcgtgtcgaaagccttcgcaaacgcggtagtcggcgccgagcacgtcgagcgtgatgcgcatcaactcggcgcttgcaaacacttcttccggcgttccaccctgcttgcgcaagtcggcgatcagcgaagcgtcgtcggtcttgtccgcgaagcgatcgggatcacgccgagacggcgcggcgctgcccgaagcaagcagggcaacaggcaatgcacgccccatcgaccgcaatcggcacgtcatgccgtaagcaagcaatgcacccatgctgtggccgaagatcgcgaactcgccgcgcatggcctcggcctgctccacgcagagctgcgccacgaggctgtcgaaatcctgaaccgggctttcggccagccggccgccgcggcccggcagttccacgggcacgacgcgaatccagcgcggcagcaggcggcgccagcgcaggtacatcgtggcgctggcgcccgcgcacggcaggcacagcagcgagacgctcgtctccacgcgcgtcaaccggccgcggcttgcgtgttcgtcggatttttttcctgctgcgccatccactcgcgcagcgagcggggccgcatgtcggtccacgcctcttcgacgtgggcgagcacagtcttcttgtcgcccttcacgccgtcgaccgcggtccaacccttgggcacggccttccagtggggccagatggaatactggtcttcgtggttgaccagaacaatgaaggtctcgtcttcgcgatcgaagcagctcgtcgacatggatacgtccttatgcggttgaacagaaagagcgagccagaggcccggtgggccatctcttcgctcctgctcaacaagacgtttcaggacgggatctgttcactccgcgctggaaggcggcaccaggccggccaacagccacaggcgggctgccttgtcgtaggccttgcgatgcgcgggatcggcaacgagccaggccgtcatctcgtcgcgcgcggccgcatcgaagttctcgcggtcgtactcgcgctgcacccattgccatgcggcgctccagatagggtcgtcctgttcttgtgtcatgcgtgaagggtgtgtggcattgcgcggccgcacgatgcgccagcgctaaggctttcaccttacaccaatcccgcacgcgtgcagccgcgctcaatcatccacaagcaggcggccgcattccttgatggcttgcgccgcttcggcgatgagcccgttcaccaagccgagtgcgcaacccaggcgcagcgcaatctcgcgctgcgtgaggccttcgagccggtagagctcgaacaccagccgcgttcgcgcgggcaacgccgccagcaccttgtcgatcgcatggatcgcctggcgctcgcgcatcaggcggtccggcgccggagggccggccacgtccagtgtctcgacgtcgatatcaaaggtgcggtagctggcctcgaccgtgtggcgacggcagcagtcgagcgccacattgcgcacgacctggcagcaatagccgatgggccggtcggccttgcgcacgcaggggccgtcggcaatcttgaggtacgcgtcctgcatcacatcgtcggcaagctccgcggtgcggacgattcttcgcgccacgcgcagcagctgcggacggttcgcgatgaagacttccgcgagcgtgggttcggacagatgcagcgccacgtcgatgggttctctcatcatgcgaagcggggcagaggccgcccggaagaatgtcggcaaaggtgcagacctgtgaacatgaaggcggtactcctgaagtgctcaatacaaatgagaattattactacttgtggatacaaaaaagccccatttcccaaccccttcatgctccatacccagtagacgtttgagcacgccaaagcgagacagccggcgtgaggaattcaagcaaccaaacgttcgccgatggtggggcggccgcatgacagaaagatgatggcgacgcgcgcgcatctagaattccgcccccttccccgctccctttcccgctccctcccttgcccatgaacatcgtcgtcaacgaagaactcaaagcctatatcgatccattgactccggaggagcatgaggcgctggaacgcagcatcctcaccgaaggctgccgcgacgcgctggtgctgtggggcgacgtgctggtggacggccacaaccgctacggcatctgccagaagcacggcctgccgttccagacggtgcagaacacacgcttcaagacgatcgaggacgtgcacctctggatgatcgaccagcacctgggccggcgcagcatttccgatttcttgcgcggcgtgctcgcgctccgaaagaaggacatcgtcgacgagcgccgcgcacgcgcattggccgacacggcgccatcggacgacaacgacgcgccattcgatgccgacccgcccgcagccggaccatccgcggacaacgcccctgccctgcccccgcccgcgcctctgagcagccgcgaagccattgcccgcgccgcgcgcctgagcagcaaccaggtggtgatgatcgagaagatccagaagcaggccgcgcccgaactggtggcggccgtgaagtccggcgtgatctccatcaacacggccgcggccgtggccagcctgcccgccgaagagcaggtcttcgcggccaacgcgggcaaggatgaactcaagcaggccgccaagcgcgttcgcgaagccaggcgaaagccccgcgaagagtcgtcggccgaatccgctgaatcgaatccggccgatcagcccgcaaagcaggccgacgccgtccagttgctggagcagcgcgtggccgaactgacggccgagaacgacgccctgcgcaggcaggtcgccgagctggaagcgcagctcgtgaactgacccgccggccagttcgattggcggctacagccggatctcgctgatcttcgcgcccgagatcgagacgccggcttcgaggccgacattggtcagcacgaagccgaccacgggctgctggatcgtgttggtgtcgatgctgccgttggcgccaaaggttgcggcggccaccgtggcatcggcgccggccgtccagcccttgctgctgcggaacttgtcgagcgcagcctgcgtggtgaacacgtagatcacagctttcgactgcgcgccagcctggaagccgatcgagcccgcagtggtgctgtagtaggcctgcgtgcgtccacccgcgcgcagcgcgccgcggccgtactcggcgcctatgcccatgctggccccgaccacggcgggaaacaccagcacgcccttcgacgatgcaaccagttcgcgcgagcccctggcggagtcgtacagcttggacaacgcggcatcgacctgggcatcgatcgaagcgcgcgacgatgcgctgctggcctggtcctggggccgagtggtggtgcagcccacgaccgcgatgccaccgactgcgacggcacacgcgagagcaaggctgcggaaatgaatggatcgcatggcgctctctcctttgcaagtaaacgacaaaaagccgagtgctttcactcacgccgctcggcgacctgttcgacccatgctagttccggaaagtcctttgagaaccggcttgcgaaatcggcctacgcgaagtcgcgccctcgaagaactccgcccggccacgggccgacgcagaacggtgcttgcctgagcgctgcagtgccggcagcttcccgagcgactcctcgaagagccgggggagagcctgcgcgcgcgccgtgcggcccctggcgcgtgggcaccaacattcagctgtgcttaacgattgatgcagtttcactaaaccacgcaaaccgctcgaatctctacagtacggcgcatgcacacaccatcgcacctcatggcgctcgacacgccggccgccctcgtcgacctgccgcgcatgcagcacaacatcgatcgcatgcaggcgcgcatgaacgcgctctccaagcgctttcgcccgcacgtgaagaccaccaagtgcacgccggtcgtgcgcgcgcagcttgccgcgggcgcacagggcatcaccgtttccacgctcaaggaagccgagcaattctttgccgacggcatcacggacatcctgtacgccgtcggcatggcgcagcatcgtctgccgcaggcgcttgccttgcggcgcaagggctgcgacctgaagatcatcaccgacagcgcggcctcggccgccgtcatcgccgagttcggccgcgcgcatggagaggcgttcgaagtctggatcgagatcgacaccgacggccaccgctccggcatcaagcccgacgaagcggcgctgctcgaggtcgcacgcaccttgcatgcggccggcatgcggctcggcggcgtgctcacgcacgcgggctccagctatgacctcgatacacccgaagcgctggccgccatggcggagcaggaacgcgcaggctgcgtgcacgcggccgagcgcctgcgcgcggccggcctgccctgccccgtggtcagcgtcggctccacacccaccgcgctgtcggcagagcaactggacggcgtgaccgaggtgcgcgccggcgtctacgtgctgttcgacctggtgatgaagaacatcggcgtctgcgacacgtcggacatcgcgctcagcgtgctgaccacggtcatcggccaccaggccgacaagggatgggccatcgtcgatgcgggctggatggcgatgagccgcgaccgcggcacgcagaaacagaagcgcgattacggctacggccaggtctgcggcatcgacggagcggtgctcgacggctacgtgctgagcggcgccaaccaggagcacggcatcctctcgcgcgaaggcacgcccgaccccgatattgcggcgcgctttccgatcggcacgcagcttcgcatcctgcccaaccacgcctgcgccacgggcgcgcagtttcccgagtaccacgcgctcgcgcaagacggaacgctggccacctggagccggctgcacggctggtaagagaaaccatgagcacaagtattcaacccattgcaccggcgggccttgccaaaccgggcgggcactacagccacgccaccgtggcgaacggcttcgttttcgtctccgggcaattgcccatcacggccgatggcacccggctggccgaggcctccttcgagcagcagacgcgccaggtgctcgacaacgtgaaggcggccctgctggcggcggggagcggcatcgatcggctggtgcaggtgcgcgtctatctcgatgccatcgaaaactggcccgccttcaatgcgatctatgccgagtgggccggcgatgcccggccctcacgcgccatcgtgcccacggggccgctgcacttcggcttcaaggtcgaggtcgaagccgtcgcgctgggctgaacgcggcaggcgacgccgagcgcggcgccgcactgctgacttgcgggcaaaaaccgggcaaaccgaaagttctgcaagatctctctcaattcttaattgataatgattgctatttacttttagagatagcacgtgttgtcgacctcaagactcaagggcacgccccccgccggcgcccgccctgcaccaggaacctcctgcctccctcctttccggaaaacaaccctcagcctcggcaccggcgccacgctgctggtgctgtgcgccgccgcgcaaggcagccgcgcctatgcccaggaagccaccgacaaggcggccgccctgccaacggtcaccgccactgccgcggaagaaacgcctcagcatctcggcgccaaggtgagcagcggcgccctcggcgcacgcagccagctcgagacgcccttctccaccacggtggtcaagagcgaagacctggcggagcgccaggtgtccaagctgggcgacgtgttcgcgctcgacgcgtcggtgtcggacaacagcggcgcctacagcagctgggccagctacatcaccgtgcggggcctgccgctggactggcagaacggctaccggatggacggcaagccctttctgagctacgccatcaccctgccctacgagcacttcgagcagatcgaactgctcaagggatcgaccggcttcatgtacggcttcggatcgccgggtggcatcgtcaactacgtgaccaaaaggccgacggaccagccggtgcgaagcatcgacgtgggctacaagtcgaacagcgtgtggagcgagcatgtcgacctgggcggacgctttggccccgacgaccggttcggctaccggctcaacgccacgcatgaagaaggcaagaccttcaacgacggcggcatccgccgcgattcggtgtcgctggcgctcgacgccaggctggcgcgcgacctgacctggaacttcgacgcgctgtaccagaagcgcaagtccaccgaccagaccccatcgatctccaccagcgcctatacgggcagccgcctgcccaccgccgtgcgcggcgacgatcagcggctcctgggcccggggcagcacctcaccaccgatctgcagctctactcgaccgggctccagtacaagctgacacccgactggacccttagcaccagctacagccacagcacctccaagcgcagccgcaacgaaggcattctttatctgcaggatgccagcggcaactacgacgactaccgctccgacacgcgcgaaggccatcgcttcgaccagtggcaggccatggccgagggcaagctgcgcacggggtcgatcgagcaccagctgacgctcggcgcgtcgtggcaaaagcaggtgaacgactacagcagcaacagcatctaccagtggatcggcaccggcagcatcttcgggcagaacaccaatgcctacgccagcacgaccgacctcacgctctaccgcaacagcgacatcacgcagcgcgcgatcttcgcgagcgacaccttgaagctgtcggaccgctggtcggtgctggcaggcctgcgcagcaccaactacgaacagagcggctacggcaccgacggcatcaagacttcggagtacgccaagaaaggcgtggtgacgccgacgctggcgctgatgttcaagcccgcggccgacaccacgctctacacgagctatgtcgaatcgctcgaacaaggcagctccgtcagcagcctttacgcgaacaacggcgagctgctcaagccgctcaagagcaagcagtacgagttgggcatcaagaccggccgcgagcgctggagcgccacggccgcgctgttccgcatcgagcgcggtgccgaatacgccgacagcgccaacgcgctggtgcaggacggccagtcgatctaccagggcctggaactgggcgcctccacgcgcctgggatcgcagtggcaagtcggcgccaacctgatgttcctcgacgcttcgtacaggcgcggcagcgacaacatcggcaaccgcgtggcgggcgcgcccaatttcgtggccacggcgcaggtgtcttatgcggtgccgcaggtgccgggcctcaagctctcggccgacgccaagtacaccggcagcaccatgctgaatgcgtccaaccagctgaggcttccgggctacgccatcgccaacatcggtgcgagctacgccacgcgcatcaacggccatgacaccacgttccgcgtggcggtgaacaacctcacgaacaggcgctactgggaataccagtacgacaactacatcaagcccggcgacccgcgcaccttcagcctgagcgccaagctggacttctaggcgccgccgcggcgcgcggccctgcaggatggaagaatgagcccctctctctcaactgcctgagcccgcgctctggacgccatgccccattccactgaagccccgatcagcgaagccgccatcgtggaggccgcccatgcgttgcgcgggcgggcggttcgaatgctcgaagagctcgtcgcgcacccttcgctgctggggcatgaacaaggcgcgcaggccttcatggccgaaaccttcgcgagcctgggtctgcgcgtccaccagttcgagatcgacgaacaaaagatccggcagcatccgggctactctccctccatcgttccctaccaggggcgcaccaacgtcgtcggcattcatcagcccgacgggccgcagaagggacgctcgctgatcttcaacggccacatcgacgtggtgccgaccggtgccgaagtgctctggaagcatccgccttttgagccgacgatcgagggagaccggctctacggccgtggctcggccgacatgaaggcgggcattgccgcctacaccatggcctatgcggcgctgcagtcactgggactggcgccggcatcgccggtgtacttccagtcggtggtggaagaagagtgcacaggcaacggcgcgctcgcctgcctggtcgagggttaccgcgccgacgcggccatcattccggagccgctcggtggcgtgatgacctgccagatgggcgtgctgtggttcgcgctcgaagtgctgggcaagccggtgcatgcctcggtagcccagactggtgtgggcgccatcgatttttcgctctatcttttttcggaactcaagaagctcgagcagcgctggaacgagcctgccaaccgctaccgcagctatgcgcaccacgcccatccggtcaacttcaatctgggaaagatccagggcggcgaatgggcatcgtcggtgccctcggcctgccgcagcgacatacgcatcggcttttatcctgacatgaacgtggcccgggccaaggccgaggtcgaagccgcgctggcttcggcctatgccgcgcatccggcccgcgagagcctcagctacaggctgatctacgaaggcttccaggccgacggcttcgatctcgacctcgattcgccgatcgtgaccgagctctctaagtgctaccaggacatcgtcggcgagccgctggagcccggagccttcacgggcaccaccgacgcgaagttcttcaacatctatggacagacccctgccgtttgctacggccccacgggctccagcatccacggcatcgacgagtgggtttccattgacagcctgatgcaggtgaccgccgtgctggcggtgttcatggcacgctggtgcggcgtcaaccgcaccgcgtgacctggctgtgatttatcgcgccactggcttcaagaagatttcgacacgccggttctgcatgcgtccctcttccgtcgcattgcttgccacttgctgggtctggcctcgtccctcggcagagaggcgtgttttggctacgccgcggtctgccagatagcttcccacgctttgtgcccgacgctgcgacagcgtcatgttgtggtccgggttgccagtgctgtcggtatgcccgaccacttgggcgttgatgccaggctcttgggagatggtttgggctacgccgtcgagcacgcttcgaaacgaaggcttgatggtggcgctgtcgctatcgaaagtcacctggctgggaatattgaccttcagcgagccgtccggctgctcggtgatctgcgtgccagtgcctgccgtctggccggacaacttgttgcggatcgctccccagttgtagcccacgcccgcgcccaccgcggcaccgactgccgcaccgatggccgtgctcttcttgttgtggcccatcagattgcccacacccgcaccgacgacagcacctgcgcctgtgcccacagccgtatgggttccttgctcggtcgcgcaacccgcgacgagcaccgcggccattgccagcgaagccagtttgattttcataggtcctccgattgagttgcgcagcgcccgcgctatgcgcgcttgacgaggcgaacgatgatcagcagcacgatggcgcccgcggttgccacgacgaggctgccgaccagaccgccgccactggagacgccgaacgtgctgaacatgaagcctccgaagacagcgccgagcacaccaacgacaagatcgccgatgaggccgaagccgccgcccttgacgagcatgccggccagccagccagcaaccagacccacaacgagaaaccacagcaaactcatttatctactcccttgaataggccgatgcggccatgaagcggcaagcgtagccgccacgcgttcgccaaaaaacaatggtgcaatcagcctgtgatttattgctctctgcagaagaatttcttgtttgccgtgcatcacttcgatggcgcctggccagtgatgtccaccaccacccggcgatccggctgcaggcatgcaatcaattcgggcgtgcggaccgtgcccttgcaattgatggtcacgggctcgcgtgcaccgctcgagccgacctgcatgggcacccgaagacccgctgccttcaggtagtcgcgtaccgtgcttgcacggcgaagcgccagctcctggttgtaggcctgactgccaagccgatctgcgtggccggtgatctgcaggctttgaacttccaccccttgccgatgcagggcccgggcaagctcatcgagttcggcgcgacccttgggcagcatgtcaccggtgttcgaccggtcgaacgcgaaaagggcatccgcgctcaaggtgacgcgctttggcatgacgggagcgggcgcgggtgcgggcgccattgccacaggagcaggcggcttcaacatcgcctcgcagtccgcgcccttccagtggaagtcctggcttttcatgtccttgtcgaaatgcaccatgtactggcaggtgatgaactcgtgtcccttgcccgtgcgaaagttgaagatgtagttccactcgcgcggaccgaacaggccctcgctgaaatgcggatagctgatgagttcgcgaacctggttcttgctcatgccaggaccgatgcggcgcagctgctcgacgtcgacgaacgtgccgttcttgagccaggccctgcccatgtcgggaaagttcaccgaatgctcggccggggcagccggagagccggttgtcgatgcgcagccgacggtgactgccagcacaacagccgacacgaagaattgaattgcttgtttcatgcgattgctcctgactgttcgatcaatcgaacgaaaaaccgaaaccaacgcgaacgatcgccttgcccccgccagagccccagccgatgcctccatgcaaagtggtctgtccattgtcggaacgcttgagcaggttgatgcctatcccggcctggccgttgtagccggcgaccgcgccgctcacgtgatagcggcccggctcgacaggcgtgaccaccgccatggcggccgatgcggcgatgccgcccgacagcatcttggtattgcgttcgatgctgttctgcaggccgttcacccgcgcgtcggtgtacgcggttgccgcggcgatgccgctgttcaactggttcacgttgaccgcatcggtgccggcaactccgggcgccacgttgctgatcgtcaccgggccggtcgagttgttgccgcccatggtcacgctgttgtagttggtcgtgccgtcggcattggtgtcgtacttgaccgtcgactggtcgatcacggccaccgcgccctgcacggccttcagctggctcacgttggcggcgtcgctgtcggccgtgccggctgccacacccgtgatctggcggtactggccgttggccgcgtcgccgaccgacaccgccgcgagcgtgctggtggttgctccgatggctatacgctgcgagtccgtggcgctaggcggaacatagcctgccacgcctgcggctgttgaagcgatcgctccggcgccgagggcgacacccccggcttgtgtgacgctggttcccgcaccgatggccacgccctgaacggcggcggccgaagactgagtgcccaacgcaatggagtccgccatgtgcgacgtggcagcctgtccgatggcaatgccgccggtcgcgctctgctgcaccacggcgccgttgccgatgcccacgccgttattgccattgaccaccgtctgaggacccacagccaccgactccgcgccgatggccagcgaatccgcggcgctggagttcgcgtggaaatacagggtgggggtgacggcaaaggattgcagcgcgctggacaactgccggatcgtgacggcatcctgcgcctccgtcccatcggccacattggtgatctggcggtagctggtggcattgccgacggaaaccgcaccaaggagcgtcctgtcggtggtgttgtaggtgatgacggagttgccggctggaatggtgcccgttgtgggggctatcgcacggtcggaaatggaacccgcgcccaatgccactgcgccggcctggctcgcctggctcaacgcacccagcgccaagctctggtccgcagtggctctcgcacctgacccattggccgtcgccagtacacccgttgcctgtgtgtctacgaagctgtcgggcgcagtcgcaaaggtcgcgtttggggtataggtggtgtccagcggagcaccgttgagcatgtagacccggccgccggttgccgttgaatagttgccggtggccgtagccatcgacccgacggatgttgccgcgatgcccgatgccaccgagttggcgccgagggaagtggctcgtacgttgctcgcattcgcccggcgcccaatgctgacggcgtagtcattcgtggccactgcactctggccaagtgccaccgtggagaacgcactggaagtcgttgcatcgccgatggcgacggcaccgttaccggcagagttggacgcaaagccaatggcgatgcccagccgggcgctcgccgttccgccaatggcgatcgtgttctgggcaagggactgggcgccagcgcctatagccaccatgccaccattgctcgcattggcattgacgcccagggcaacactgcttgtagtagctgctgtggcgcccatgcccaccgccaacgtgttggcggcggaggccaccgcattggggccaacagcgatggagttggcaccagtggcacccgaattcgccaaggtcgaattgccgaccaggttggagttggtgtggaagtacggcgtctcgtccacgctgatccattggccgttcttccacaccgccaagcctgcctgcaggccgttgacgcccgtcgtcgcggtgctgttgtagaccaccatgccttcgactggctggttgccgttcaggccccaggtgttgcgatcggtcagcgcgatgcgggggagtagagcgccgcggttggtactttcgagttccagcagggaacccggattgatggtgatggggttgtcaccgatcttgacctgcgcctgcgcggcggatgcggacagcaacagcagtgcagtacccaccgcgcagcggccgaggggcggcaacttgccgcgggttgtgcgtgaaattgaccaatatgttctctgcatgttcacctcgtctgttggggtctgggttgaccttgtcccggcaataccgccgtagaactttcgtaggcctgacaaacgcgatggtgtcgggcgacaaacgagcgaggtgatctcttgcgaggtttagcgagaattgagacgaattgacgcagggaagtgtgatttagttatcaggtcagagtactttggtttcagatgaccaacccaatggtcgcgcgactgaaaccccgccaggctcaggttcggtcggcgggaaagtggcgcggcaagtccatcacgaaggtggtgcccacgccgggggcgctgtggccgtcgaggcgtccgccgtggcgatcgaccacggcgcgcacgatggccaggcccacgccatgcgaacgcgcggcaaacccgctcgatgccgtggcatccatgtcgccgtccagggccggcatcacgccttccgtgtcctggtgcagcaatgcctccatgacctccggcgacatgcccgcgccttcatcggacacggcaatcaacacccggtgcggcgctgcctcgccgcccgccgacacgcaaagccggatcgacgcgcccgaagggctgtagcggatggcgttgttcagcaggttgaccacggcgcgcgtgagcagcggtgcatccgtccacagctcgacgtcttcttccgtcggcacctcggcagagagcttgacgccgcgctgcgccgcgtgggcccacacctggtcgacagcgtccagcgcaatggcccctgccggcatctccacgaaccgatagctgtgcatgcgggccttcaggagatcgacgaagtcgtcggcgagccgcagcgacctctcggcctcgcggcgcaggctctccgtcaacagcggctgttcgagccagtcggcaccgtgggcgcgcagatcgagcaggctcaggatgttgacctgcggcgtgcgcatgtcgtgcgacatgaagctcagccactgctcgcgctcctgctcggcgcgccgctcggccgtgaggtcgtgcaataccaccagccagcgcgtggagacggagtcctgctggtgcagcgttgcggcccgaacgcgcaataccttcccatcgagcgtcgtgcgctccacgtcgatgccttccgcccactccttggcgccggcgccgagagggtcggtcagcccgtcgcaccgggtatccgcaagcatgtccaccacggcgcggcctcgcagcggatcatccgcttcgtcgctcccggccgcctgcgcgctcagcagcgcacgagcggcggcattgctggtggtgatcgtgccgtcgccgcggcacacgagcagcgccacgggcatctgccacaggctcgtgctgagcagcgtgcggatctgcccgacgcggtcgatggcgtcgtcgagcatgagggcatgggcatgcacgtcgtcccaggcctgcacgggcgcccggcgctccgggtcgaaggcaccgctgggcaccgcgttgagcgccgcggcgcgctggtcgaaaaagcgaaacagcgcgtccagccgccgccagctccacagcatgtagcccacgacgatgcccagcaccggcgccgagggcggcagccacaggtgcgccgccgcgaacatgccaaggctgaaccccacgcacaccgtgatcagcgcaagcgccacggtccacgccttgcgggcaaatcggcgaaagagcgccagcgccagccagatgggaacggcgatccacgccgccagccatgctccgtcggcaaagcgcactgtggttccctggcgcagggcgtcgatcgcattggcatgcagctcgatgcttggaagcgaggtcatcgctccggcgccggtcaccggcaattcgtcttccagccgtgaactgcccaccgctccgatcaggattaccttgtggcgcagaagctccgacggcacatcgcctcgcagcacgctcacaaagggcacagtgcgccagctgcccacaggccccgccagcggaataccgaactcgccttgcatctgccagccgtccgcgcgctgcctggagggcgcgatgacaacatcgcttgccggatggccgctcgccagaatccagcccagatagtcgtgcagatgcccgcgcaggccttcgcgcaagaacatccggcgtgcaacgccatcggcatcgcgtgtgatgttgacgtggccgagcgccttggcgcggcgcgcaaactctggcaagggctcccgaaagccgggtgtatcgtcaagtgccccatcgagctgccccgtatagctcagcggcaaatacaccggaacccgcgtcatggcctgcgccagcaaacggtcttcctccgggtcttccgacggcatgtccaggaacaggtcgagcagcacgcccttgggctccatgggtgcaagccgctccagcagccgcgcatgcacgctgcgcggccagggccaggggcccagcgcgttgatgctgcgttgatcgatccccaccaccagaatgtccggcgacggggtggcccgcgcccggctcatcacatggtcgtaagcagcgaggtcaatttgcgccaggccgggcgagcgctgcagccaccacagcgccggaggcagcagcgccatcatcagcagccattcgacacggaaacggcgccgcacggttcagcggtttgtcggtggcggggcgggaacgtcgaagctgccctcgaagaccgccgcctcggcgccgggcgtcgtgatctcgcggctgcgccagtgatagcgacccggcacgtcgagcgggcccaccagcgcgccgcctccatacagcaccggctcgctcaccagcgcaggcgcaaaggccggcgtgcgcgccagctcgaaggcatagcgctggcccggtcgcgccggccagctgatttcgtagcggccgtcgtccatgcgacgcacaccggccggggcggcacgcacgccgacatagacgatgctgtcgcccggcatgccctcgagctgccgtgcatcgaaagccgtgagccgcaggtggtagaagccggtctgcagatccgcgggcaaggcaaactcgccttgctgcgaacgctcctcgtaggccaactgcagaaagcgctcatcgcgcgccaactgcatgcgatagccgaccgcgcccgccaccggcaccaccgcggcctgcgtgctcccctgcccctggcgcgcgttctctggcggtggcaacaaggtttgcgcctgcagcgcacccgggccctccagcaaggcgccgcgtgccgcagcgagcagcagggccggccgattcgcgctggacacggccacctctccttcgataacttccgccgagatcacgccttcttcgttgcgcgcgcgaaagtgcgtgccgcgcacgcccagtgccgccgtgcggttgcgaatctcgaattcacggccgcgctgcttctcgacatgcgcctcgacgcgcccgtccagcaactgcagctgcgtgacgcggccattggccaccagcacctgaaccgcactgctcgaaggcatcaccagacggctgccatcgcccagccccaggctcaggaaagcgccgcgatcggtcaccaccacgtcgttggcccttaccgcagcgccttgcgccagcgcgcgcggcgcatcgttgcctcttttgagccatgcgctgcctgacagctccaccaccgccgcgacggcagcagtgccgccgctgaggagcagcacctgcccaggtttcagatgctcgggtaccggcacggcattgccgcgttgcagttcgggccagcgcagcggcgtattcatgtgctggcgcgagatgtcccacagcgtttcgccgggccgcaccacgtgcgtgggctgtgcccgcgcagcccctgacagcaccgtgagcgacagcacggcaagcaatgcgagtctgttgtttgccaatgcctgcctagaccggctcgccggccgtgtgctcattgccattcgatgatgcctccaggcgatagccgtgcccataaaccgtgtgcaactgaagcccgtgcgccacgttcaggcgcagcttgattcggagccggtagatctggctgtcgagcgcgcggccgggcgtttcgccctcgcgccccacgcactccagcagatgcacgcgcgacaccggccggccaaggttgcgaaacagcgccagcgccatgcggaactcgctgtcgctcagcaccacgcggcgcgccggctccgcacccgccgcgccaatacgcacggtcgacgagatacggtcgaacacccagctgccaaagcgctccagcgcgcttgccgccgcgagatgcctcgacttcaaaaggcgctggatgcgcgcggccagctccagcgggcgaaagggcttcaccacgtagtcgtcggcgcccgtgccaagggcgcttgccacgtcgcgctcggagtggcgcgaactcagcatcaccaccggaaccgtgctttcccgctgcttgcgcagccaggccagcagctccacaccgttcaggtcgggcacgttccagtccagcaccagcaagtcgaagctttcggtgcgcagcgcatcccgcaaggcttcgccactgctgaaaggcacgcacgacaccggctcctcgatgatgagcaagcgatgctcgagcatgtcgaccagaaggctcatctgggcgggctcgtcttccaggacagcaatacgcatgggggtccggcgtggatgccaagaagatattatttattactaaagttacattgtgcattaaggctggaagtgcgggggcggcattcgatgcctaagtggcattcgatggatgcccccgcactttccgtacctactgcctactgctcgccggccacctcgatgtcgacgcggcgattgggctgcaggcagctcaccagcgccggggtcttcgcggtgcccgggcactgcgccaccggctgccgggcacccatgcccgcggtgcggatggcgttgcgctcgatgccctgttgtgccagcagatcacgcacggtgttggcccgcgccagcgacagcgcttcgttcgagcccgcgctgcccaggcggtcggtatggcccgtcactgcaatggaatgcacgcgcttgaagttgcgcttgatgtcggcggccagccgctcgatcttggcgcggccttcgggcgccaggtcgttcaggctgccgccgccaaagcggaacaggccatcggcgccaagcgttaccttctgcggcggcgtcaccacgggcgcagccacgggaatgggcttgacctgcggcggatcgagcagcattgcgcagttcgggtccttccagtacatgccctgggtcagcctgtcgccgtcgtagcgcaccatgtattggcacgtggtgaactccgggcctttcccggtgcgaaagtggaagatgtagttccactccttgacacccgccaggccctcgctgaaatgcggcgagccgagcaggtcgcgaacctggtccttgcccatgcccgtgcgcatcattcgcagcgcctccaggctcgggaaagcgccctgcttccacttggccgcgtccagcttgggaaagtcctcggcctttggcggtggcggcatctccttggcggcgcttgcctgggcttgcggcgcgatgggataacccgggctggcgcacccgctcagcacgagcacgcacagaagggcaagcaggggcggcaggctgaccagcgtcatcaccagcgccgtggcgcgttgttgcagttgtttttccatgatcgttgttccttgaatcagtcgaagacccactcggcacccaccgtggccgccgcgccggcgcggctcatgcccacgccgcccgtcaggctccaggcgttgttgtcggaggtgcggcggaagctgatacccacggcgctctcgcccttgaagacgccgtagcccacgcgcatcaccgtcttgcccggcaacgactggcccggcatctgcacggccatggcggcggccacgccggcgtaggcattgcggcctatcttgttcacctggtcgcccaaggcgttgatgcggttgttcacgccaccgattgccccgctgagctggttcacgttcacggcatcggtgcccacgaccccaggcgccacgttcgagatgacggttccgttgggtgcctgcccgttgcccagaatgacctggttgtagttggtggtgccgtccgcattggtgctgtagttgatgccgccgtccttcaccgcctgcaactgccgcacgttcaccgcgtcggtcgcctcgataccgccggccacgttggtgatctgccgctcgttgcccgagctgccgaccgacaccgcgccctgcgtggaagacaccgacacgttcgagaaggcttcgcgacgtccgctcatgcccggacggtccgccgtggagccggcgcccagtgccacgccgcccacgctggagaccaccgaggccgcaccgatcgcaacgctgttgcccccggtcgccaccgagttgaggcccaccgccacgccgcccgggccggaggcgctggcccccacgccgcttgccagcgagttcgtacccgtggcaccgtcgttgttgtagttggcctgctgcacgccgccgtcgttcacgctgtagtagtgggttcttgccgcgttgacggttgtgcccaggttcgagatggcggtgttggtggcgtagagctggctgccgttcaccgcatcggtgctggtggcgttcagctgcccggccgccacgttggtgatctggcgctcggcacccgcgctgcccacgctcaccacgcccgtgggcgcagcgcccgcaaaggtgtagctggtgccgccgatcgtcgtgccagtcaccgcggtcgcggtgcccgtggtgctgtcgttgcccagggccacgctgttggccgtggttgcggtggcaccggtgcccactgccacgctgttgatgccgctggccgtggagcccgagcccaccgcggtggcgttggtagccgaggccacgggcgccacgtaggtggccggcgcaccggtgatccacatgttggccgccgtggaggtagccgtgttcaactggctcaggttcaccgcatcggtcagattgacacctgcgcccacgttggtgatggtgttgccgcccatgttcagcgtgttgccggcgttcatcgtgatgccggtgctgttgatggtcggcccgccgctgatcgtcaggctgtcggccaccagatccggcgtggtcgccaccgtgatggtgttgccgctgtgcaccagggcaatgttctgcccgctcacgaactccaccgtgccgccgggtgccacgttggtggccgtgtcgccatcggcctgcaggttccagcccgcattggccacggtgctcaccgcattgagctggttcaggttcaccgcatcggtgcccaaggcgccgggtgccacgttgctgatggtggtgcccgcggcgtcgatgcccgcggtcgtcacgctcggtccgcccgtgatggtcaggccgttggtgttgagcacgctgttgccggtggtcacgctggtggccaccagatccgggttggtggcaatggtcaggttggtgccgttctgcgtgatggcaatgttgtcgcccgccgtcgtcgtcactgtggcgccgggcgccacgttggccacgctggtgccgctcaccgtaccggtgccagtggccgccgtcgtcgtgttccagcccatgttggccacgttgctcaccgtggtcagctggttcacgttcaccgcgtcggtgccggccacgccgggtgcaacgctggtgatgacggtgttgttggcgttgaggcccgcagtcgtcacgctcggcccgcccgtgatggtcaggccgttggtgtccagcaggctgttgcccgtggtcacgctcgtgaacaccggcgtgtcggtcatctgcagctgcacctcgttgcccaccacggcgctcttcaggttggcgccgctgtaggtgccggccgtggtgcccaggccggtgatggcgagcgtctcgcccagcttgcggtccaccgtgccggtgttgcccgtgaaggtcatcggcgtgttggccagcgtggtgatctggctcacgttggccacgtcggtcgggttgacgcccgccgccacgttggtgatggtgttgccgcccatgttcaccgtggtgccaggattcaccgtcaagctgccgccgatggtggtgccgccggtcagcgtggtcgggccggtggccgtcaggttggtggtggtcacgctggtgaaggtgggcgtgtcggaggtcgcgatctgcacttccgccccgttctgcgtgatggcgacgttgttgcccgccgtgtaggtggccgtgccgcccggcgcaatgttctgcaccgtggtgccgctcaccgtgccggtacccgtcgctgccgtggtcacgttccagcccaggttggcggtggtgttcaccgcattgagctggttcacgttcaccccatccgtgccagccacgccgggtgccacgttggtgatgacggtgttgttggcattgatgcccgcagtcgtcacgctcggcccgcccgtgatggtcaggccgttggtgtccagcaggctgttgcccgtggtcacgctcgtgaacaccggcgtgtcggtcatctgcagctgcacctcgttgcccaccacggcgctcttcaggttggcgccgctgtaggtgccggccgtggtgcccaggccggtgacggccagggtctcgcccagcaggcggtccaccgtgccggtgttgccggtgaaggtcatcggcgtgttggccagcgtggtgatctggctcacgttggccacgtcggtcgggttgacgcccgccgccacgttggtgatggtgttgccgcccatgttcaccgtggtgccaggattcaccgtcaagctgccgccgatggtggtgccgccggtcagcgtggtcgggccggtggccgtcaggttggtggtggtcacgctggtgaaggtcggcgttgccgaggtggcaatctgcacttccgcaccgttctgcgtgatggcgatgttgttgcctgccgtgtaggtggccgtgccccctggcgcgatgttctgcaccgtggtgcccgtggccgtgcccgtgccggtggccgccgtcgtcacgttccagcccaggttggcggtggcgttcaccgcgttgagctggttcaggttcaccgcgtcggtaccggccgcgccgggtgccacgttggtgatgacattgccgcccatgtcgaccgtggtggccgggttcagcgtcaggctgccgccgatggtggtgccgccgctgagcaccgtcgggccggtggccgtcaggttggtggtcgtcacgctggtgaacaccggcgcgtcggtcatctgcagctgcacctcgttgcccaccacggcgctcttcaggttggcgccgctgtaggtgccggccgtggtgcccaggccggtgatggcgagcgtctcgcccagcttgcggtccaccgtgccggtgttgcccgtgaaggtcatcggcgtgttggccagcgtggtgatctggctcacgttggccacgtcggtcgggttgacgcccgccgccacgttggtgatggtgttgccgcccatgttcaccgtggtgcctgggctcaccgtcaggctgttgctgatggtcgtgccgccgctgagcaccgtcgggccggtggccgtcaggttggtggtggtcacgctggtgaaggtgggcgtgtcggaggtcgcgatctgcacttccgcaccgttctgcgtgagggcgatgttgtcgcctgccgtgtaggtggccgtggcgcccggtgcgatgttctgcaccgtggtgccgctcaccgtgccggtgcccgtggccgccgtcgtcacgttccagcccaggttggccacgttgctcaccgtggtcagctggttgacgttcaccgcgtccgtaccggccacgccgggtgccacgctggtgatgggcagaccccctgcattgatgcccgtggtggtcacgctcggtccgcccgtgatggtcaggccgttggtgtccagcaggctgttgcccgtggtcacgctggtgaataccggcgtgtcggtcatctgcagctgcacctcgttgcccaccacggcgctcttcaggttggcgccgctgtaggtgccggccgtggtgcccaggccggtgatggcgagcgtctcgcccagcttgcggtccaccgtgccggtgttgcccgtgaaggtcatcggcgtgttggccagcgtggtgagctggctcacgttggctgcgtcggtcgggttgacgcctgccgccacgttggtgatggtgttgccgcccatgttcaccgtggtgcccgggttcaccgtcaagctgcccccgatggtggtggtgcccgtggccgtcaggtcggtggtcgtcacgctggtgaaggtcggcgtcatgctggtggcaacggtcaggtccgtgccgctctgcgtgatggcaatgttgttgcccgccgtcgtcgtcaccgtggcgccgggcgccacggtggccacgctggtgccgctcaccgtgccggtgcccgtggccgccgtcgtcgtgttccagcccaggttggccgtcgcgttcaccgcgtcgatcgccgtgttggtcgcgaacagctggctgccgttgatggcgtcggtgctggtgccgctgatctggcccgctgccacattggtgatggtgcgttcaaagcccggcgagccgaccgacaccgtcgaagccggtgtcgtgcccgcgaagttgtacgtggtgccggcaatgacggcgctgggggtacccaccaccgtagccgtcgtcgagcccgagcccaacgccacgtcgccggcattcacgctcgccgatgcattggagcccagcgcaaggctgtcgctcacgctggccgttgctccctggccaaacgctgccgcattcacactcgatgcgctggccagcgtgccgaccgccaccgaagaagtgccagtggcgctcgccgtctggccgattgcgactgaacccacgcccgtcgcggtgttctggcggcccaaggcgacagcacccgagccggtgaccgtgttgcggtcgccgatgccgacggctccctggcccacgaccgtgttctggtagccgatgccgacagcgccctgcgccgccgtgcccggcgtgctgaccgcctgcccaccgccgcccaccatgttggtgttgccgatggcggtggcgccgttgcccgtggccgtgttgtccaggcccgtggtgaccgcgccagagccggtggaggtgttggggtcgccaatggcgaccgcgcccgcgccggttgcgacgttgccattgccgatggacacggccgagccggtgcccgccacgcccgtggcggttgcgtccaggccgatggcgacgtcacccagctgagccgcgttggcgaatgcaccgatggcgaccgagctttcacccacagccgacgccatgccaaccgctactgcaagttcaccggaggcatttgcataagcgcctgccgccacggcgctgtgtccgctggcgcgcgcactgacacccagcgcagtggaattggtggcagttccttccgcaaaagtcccaaaggcggcggaattgaagccggaggcaatggagagaccgcccaccgcaatcgactgctggccagaagccgttgcatcattcccaatcgcatacgcattgccactcgatgcgatcgcaccatttccaatcgcatacgctagggaggcagatgcgcttgaattggcgccgattgccgtcgaaccttgaccgctggacaccgcgccgccacccattgcgatggcatccacagccgacgccgacgcattctgacccacggcgatggcgcgagcatcagcggctgacgcgccggtgcccacggcaatggcgttgccgccggttgcaccggtgttgtcgaagttggcctgctgcacgccatcgtcattgacgctgtagtaatgcaccggattgccgatggcggcttgtacagcgccgttcagctgggccacgttgaccgcgtcgctgtcctccgtgccggctgccacgttgacgatctggcggtagttgcccacgtcgcccaccgagaccgcgcccagcagggtgctgttcgtagccatgatgcgcgccgtatgtgccgcgcttgcgccaacgggcacgtagcccgccacgccgggcgctgtgttggccaccgagccgctgcccagcgcaacacccttcacccccgcggcggtggagctggcaccggtgccgatggcgacggcgtcgggaccgctggaaacggtgttctcgccaatcgcgatggagcccgaagtacccgaagcctgcgcgttattgccaatgccgatggcaccgttcccggttgcttgggatgcgtaccccagcgccgtgcttccaactccgattgaatacgacccgttccccaaagcgacggccttttcggcctgcgccaaagcaccggcaccgaacgcaatagaattcgcaccgctcgccgtcgaaaaatacccggacgcaatcgcgtgatacccagaggcaatggcaagataacccatcgccgtcgtaccctctgcttgtgcctgcgactggaagccgaaggctgatgacgcatttccggccgcgttggccgccaggccgaccgctgtcccggcggtgtttgcagcggcaccgtagccaactgcgacagacgaacctccataagcgtacgacgaccgcccgactgcgacggagccgctgccgacagcgccggcttgatagcccactgcggtcgcagaatcttgagattgagaacccgcgccgatggacaaggccgcgcctccccacgattgagcaccgttaccaatcgcgatggattggctatatacagccagtgcgcttgccccgatcgcgacagcgccagcgttgaatgactgcgcgccgcaaccgattgaaaccgaggtgtagcctgcataggcgccacattctcctgccccgatggacacggttccgttgccgggaccgacgctgccgccgccacctatctccgtattggcctgcgccggcgctgtgaacgccgcggaaacggccaatgccgcccaggtcgcgcggacaagcagccggcccgctctggacgccccgccctcgccctgctgttgctgatgatcgcggccgcccatcgacgacggttccgcctggacgacgctgccgcccgccttcttgccgcatgcgcgcgccgtttccggagccgcgacgaatgcgcccaaggctgcattccacattgaccggtatgtcttgttcattctctgcccccttgcgttagttggcggtgccgttgatcgaagaagcgccggtgaagcccaaagaggctccccccaggcgttgttgttgctgttgctgttgcagttgcccattcagcgcaaaggccctggcggtgcctgcgctgctcatcagaatctggtgtcttgttgtcatgcggttcctctttcctctccgtgcggatcgatagctgaaagggcttgaggccccacgagcaaacagcagcggcggcggcgggaactttggtgacccggcgtgctcttgtgcgtgcgaaatggatcgtgccgagggggccagggggccgtgagaattgcgcgagattccgtcagaattgagctaaatcgtgttcaaaaaggcggacttaatgcacacatttaggctgttcggcttaagaatctgaccgaccagaacagcttgcgaaaggctttgcgccgcgctgcgagggccttctggatggcgccctgccgaaggcaggcgcgcgctgccgttcgaggggcgacggcggcggctcgatgccgttcgctcaagagggggagagcttggatggcggctgttttgcgtgccgctttgaagtacctgcgaggtcttcagtacctgcggccttttttggcgaccacagggccgcttcggctgagcttgtagccttgtccgcgaatgtgaataagccgccattcgcagccgcgagcgccgccaaggtggagcttttcgcgcagccgcgtaatgcaggcgttgagccatcggcccgacgcgctgggcgcgaggcccgaggccatgccagtcagccactggcgcgtcagcacctggtcgatgttgtgaaagaactcgagcgcaagctcgaattcgagcggggagagtctgatttcgtctccctcgaccaggacggttttgagggacggcatgaagcgatagtcgccccatgtgaggccggggccggtggggggcattgcgtgccgcgtcatgcagtcttcgaggccaacgtagacgtcggagaacgacgaaggcgcggcaaccatcaggtcgcgctcgtcgcagccgagcgactggagcggcttcaagagattctcacgcgtgagaaagagcagcggcacgccggggccgacggcgtttcttgcgccgctgatccacttggtcagatcggcacgccttcgcggcaggccgatgcacatggccgagcagcggagcgaggcggcgggcatgaacagcagttcctgcaggtcttcgaagacaaggggcgcatggccgaacgcgcggatggtgcggcgcatgtgctcccgggtgcgaaacacgggatcgagcactcccacgcgttgatggagcggctgctgctgctgcggctgctgattgctggctgacatggtgtgactcctgtgggctggcaccaagccccgcgcgtgtgcgctttttttgcggcgccacgcggcgatgtaagacttagtgctgaatatgttgcccaccaaggccgcgcggcgaagccgtcttgcgagagttcgcgagaattgaatccgcgggcggggcggttccgcgaatttgttcacgcatggggccggccaaacgcttttcagacaaagcgggcatttcagcaaacgctgaaacaccacgaatcagtgaaaactggcctctcaagccgcctgctggccatacaccccctgcaccctgccccgttcctgttcggccgcaccgtactcacaaaactccagccgatagccctggccatagacggtgtggagccgaagcccgctctcgatgttcaggcgcagcttggtgcgcagccggtagatctggctgtcgagcgcgcggctcgctggttcgccctcgcggccgacgcgctccagcaggtgggcgcgtgagacgggcctgccaaggttgcgaaacagcgcaagcgccatgtgaaactcgctgtcgctcagcgacacccatcgcgcgtgctcgccggccgccagctgaaactgcacgctcgagacgctgcgatcgaacagccagctgccgaatcgctcctgcgcgcccttggccgtggactgcgcgggtgccacgaggcggcgcaggcgcgcggccagctcgagcgggcgaaagggcttgatgatgtagtcgtcggcgccggcatcgagcgcgcgcaccgcgtctcgctcggagttgcgcgcgctcaacatcacgacgggaacggtgctttccctctgcctgcgcagccaggccagcagctgcaggccatcgaggtcgggcacgttccagtcgagcaccagcagatcgaagctttcggtacgcagggcgtcccgcaaggcttcgccgctgtagaacggcacgcatgacacgggctcgtcgaccttgttgagcagatggttctcgagcatgtcgaccagatggctcatctgggccggctcgtcttcaaggacagctatgcgcatgatggtgtgggcctggaggggttgggggagttggctttttttgttctgttcagcgcggggcgcggggcacggcctgcagccacgcctcgaattcgcgcttccagaacctggcccgggcggtggtgccgtggcccacggtgtcggcgctcgcggggatcaagagggcgctgcccttcttgacgcgctggatctcgcgctgcagcacgccaagggccggcgggttgcgctcgtcgtcggccgagttgatggccaggagcgcggcttcgatcttctcgaggccgggcgcggggttgtagtcgcgcgaggcttcccactggtagaggtggtcgttggcgtcgccgcgaaacggcgccttcaggcgctggtcgagcacggcatcggccttttcgcgcgagggcgcgagcttgaacaggccctggtcgcctccgttggtgccaatggcaaagaagacggaggcaaagcgcaggctgggcggctgctcggtgtactggccgttcttccaggcgggatcgccgcggatggaatcgatgacgaggcgccgcatcatccagttgcgaccggacatctcggtgggcagcgacgccatgggggtggcggcatccatgaagccggggtacttctgggcccagatccaggtctgcatgccacccatggagttgcccagcaccagcctcaggtggcggatgccaaggtgctcggtcagcagccgatactgggccgcgaccatgtcgttgtagttgtagcgcggaaacgcggtgcgcagcccatcggagggcttggacgaggcaccggtaccgattgcgtcgggcaggatgatgaagtgctttgcggcgtccagcggctggccggggccgaagagctcgccggcgaaatcaggcgtgagcaggctggcggcggagccggtggtgccgtgcaggatgagcacgggctcgccggccggatcgcccacggtggtgtaggccaggcgcagctcgggcagcgtctcgccgctttcgaagcggaagtcccgcgccacccagtggccctcgcggggcttgggaaaatcggcggcgttggcgcccagggccagcaggcatgggagcagcaagaggcaggcgcaacgcgcgagcccgggcagccaggaggtgatggcttttttcatgacgacgatgcgccaaaacacttttgaatagctgtggccggtttcggccgcgaggacgtcgccctccccggccggcgttgtcaatgagactgacgaggtgttcatgagggctcctggttatctgggtctacatttgttttgtttacgctaacattcagttgtttgcgctaacagtcgctatcttctgttattgttagcgcaaacaacttagggaaaaccctgcatctattgaaatcttttggcttacgtagcgtgcgcgggccggccgctatgcttggcttgcgcgcagccgcaggcgacagaacaagaaagcaaccgacaaatgaacgagcaacccgaaaccacgccctccatcacgctggaggaagtggcgcgcctggcgggcgtcagcgggatgactgtttcgcgggtgctgcacgaccatgccaacgtttccgaccagacccgagccaaggtgcaggccgccattgccacgctgggctacgtacccaaccgcctggcgggcgcgctggccacggcgaagagccggctgatcgcggtgatcgtcccgtcgctgagcaacatcgtttttccggaggttctgcggggtgccaacgagcgccttggagcggcgggctaccaggcggtgatcggcgtctcggactacgacctcgcgaaggaggaagaggtcattgcggccatgcagtcctggcggccctcgggctggatcctggcgggcctcgaacacacgccgcgcgcgcggcagatcctgcgcgaggtgcgcagcccggtggtcgaactgatggacatcgacggcgagtcgatcgacatggcggtgggtttctcgaaccgggaggccggccgcgacacggggcggttctttgccgacatggggcggcgccggatcggctatgtggggggcgacctcagccgcgacttgcgcggcgccaagcgcaaggaaggcttcgagcagggccttgcggaacgcgggctgcaactgcagggtgaattcacggcgccccagtcgtcgtcgctgctgctgggccgcgcgggccttgcgcaactgctccagtcgcatccagacctggatgccgtttatttctcgaacgacgacatggccgtgggcgggctgatgcactgcatggccacgggcatcgatgttcccggccggctggcgctggcaggattcaacggactggaaatcggcgaagccctgccgctgcggctgacgacagtcaagtcaccgcgccatcacatcggcgaactggccgccgaacagatcctcgcaagacttgccggcaagacgccgccgctcaggcaggacgtgggttacgagttcatcgccgggcagacgacgtgacttgaagggcctgcccgcaagagggcgcgctggctcgggggctgaatagctcgaatcggcctccaaccgggtgcgccggcggcaaattacccggctgcagtgtgaagtaatgccactccggccatgtcctttgcactcaattctgacgaactctcgccagattctctcgtcatcgaagacttccaagcaggatcacggttcagcgcgcagtggggtgcccactggtccgctcgacgacccattctgatcggaggtccttgatgaaaaacaatgtgttgaaagcctggtgcgccgagttcgcgggcacgttctggctgacgctgggaggctgcggcagcgcggtgctcgcagccacagcggtcggatccccgaggggcaggtgatgcgaattgccgtactggacgccgatggcgaggagcttgccctcatcaccagcattcttcgatcccttgggcatgactgccaggctttcaccaggggcagcgcactgcagcgcgagctgcagcgagaaaccttcgatctgctggtgctggactggcaattggcggacaccacgggaccggagtttgcgcggtgggcccgcaccacgctgaaagaccgcgtgccgatactcctgatgacccagcggtatgaggaagaggacatcgtggaggggctggccgccggcgcggacgacatcatcgtgagcccgatccgggtgggtgaactcgccgcgcgagtgcgggcgctgatgcggcgcgcctacgcgcaacagccgaccgatgaccagacctggggccgctaccacttcgttccggcgcgccagcgcctggaggtggacggtacgccggtggtgctgacgcagaagcaatacaaccttgcgctcctgctgttccgcaacatggggcgcgtgctctcgcggcggtatctgctggagtcgatctggggcatcagcagcccgatggggtccgatcaggtgtcgcgctctttggacacgcacgtctcgcgcgtgcgcacggcgctccggctgcggccggagagcggctaccggctcgctgccgtctacggccaaggctattgtttcgaggccgtcgaggcggatgcgagcagccttgcctgaaggatggtggccgcaccctcaccccagccctctcccgcaagcgggggagggagtcgaaaccgcgcagacctctagcgggcgtcgttgcgcacggtgtagccgctcgcacgccaggtgttgtcctcatcgaagcggaacgacaccagctcgcgcacggtcttgcttccccccaccaacgactcgaactcgacgctgctgtacatccctgccggaatggacgccgtgcctgctgcctgctgcctgctggcgcgagacggtgacccagtagcgaacacccggggtacccagggattggcgcgagcgcgcgatggcctctgcaaagtccttgcgcgagacgcgctgcttgaccgcggcggacatgccatcccacacggccgcggcacgcccctcgtcgatttgctggacagtggcttgcgcggctttcaccagcgccccggggtccacgtcttgagcggaagccgcagtgcaacaggtggcaagcgtcaataggcaggcggcaatcggtcggattttcatgaggggctcctttgcagcgaatactgccgtcccctccccttgcgcgagagagttttgcgagaatttgtcagattcaaaggcaatcgggccaacaagcgcggactaatgcgcacttgcggcgccgttatttctggatgtcgcccaggcagaggtacttgatctcgacgtagtcgtccatgccgtggtgcgagccctcgcggcccaggcccgactgcttgacgccgccgaagggcacgtgctcggtggcgatcacgccggcattgatgccgaccatgccgtactccagcgcctcggccacgcgaaagatgcggcccacgtcgcgggtgtagaagtagctggccagcccaaactcggtgttgttggccgcatcgatggcgtcctgctcggtcttgaagcggaacacgggtgcaaaggggccgaaggtttcctcgcgcgcgcagagcatgtcgggcgtggcctcggcgatcacggtgggttcgaagaactggccgccgatcttgcgtccgcccgccagcaccttgccgcccttggcgacggcatcgtcgacgtgccgctgcaccttgtcgatggccgcatcctcgatcagcgggccttgcatcacgccttcatcgaaaccgttgccgaccttgagcgccttgaccttggccgcgaatttttcgacgaagctgtcgtagatgccgtcttgcacgtacagccggttcgcgcacacgcaggtctggcccgcgttgcggtatttgctggccatggcgccttcgacggccgaatccacgtcagcatcgtcgaacaccaggaagggcgcgttgccgccgagctcgagcgacagcttcttgaccgttggcgcgcactggctcatcaagatgcggccgacttcggtggagccggtgaagctcaggtggcgcacgacgtcgctctcgcacagctccttgccgatcgcgatgctgttctggctgtcggccgtgagcacgttgagcacgccgggcggaatgcccgcgcgcaccgccagctcggccgcggccagtgcggtgagcggcgtgagctctgccggcttgatgacgaccgtgcagcccgcagccaatgccggcgcaaccttgcgcgtgatcatggccagcggaaaattccacggcgtgatggcggcgcacacgccgatggcctgcttcatcaccagcaggcgccggttgttgtcgaactgcggcagcacctcgccgttcacgcgcttggcttcttcggcaaaccattcgatgaagcttgcgccgtaggccacctcgcccttggcctcggcaaagggcttgccttgctccgcggtcatcaggcggcccaggtcttcggtgttggcgatcagcaggtcgaaccacttgcgcaagacgatgctgcgctccttgccggtcttgccgcgccaggccgcgagcgccttgttggcggcagcaatcgccagggccgcgtccgcgcgcacgaggttggcgacgtcggccagcttctgacccgtggccgggtcgttcacatcgaatcggctcgcgcccttgacccattcgccggcgatcagcgcatcggtcttgagcagggtcgggtcgttcagcaatgcgaggggggatgtcttcatggtcatggcgttctgttgtctcgggaaaatcaggctggccgacagccagccgcatgcatcagcggtagggcacgccgggcagcacgcaaagcatctcgtagagaagattggcgccgagcagcgcggtgtttccgctggggtcgtagggtgggctgacttccaccaggtcggcgcccaccacgttcaggccgcggcagccgcgcacgatctccagtgcctgtggcacggtgaggccgccgatctcgggcgtgcccgtgccaccggcgaacgaggggtcaatgccgtcgatgtcgaagctgatgtagaccggatgtgtcgggccgatgcgctcgcgcacctctgccatcagcggggccagcgactggtaccagacctcgtgggcctgcaccacggtgaagccctgttcgcgcggccagtcgaaatcatcggccgcatagccggtgccgcgcaggccgatctgccagaccttgtcgcaggccagcaggccctcttcaacggcgcggcggaatggcgtgccatgagcgatgcgctcgccgaacatgtcgtcgttcacgtccgcatgcgcgtcgacatgcaccagcgcgaccggcccatgccggcgcgccagagcgcgcaggatgggcagcgcaatggtgtggtcgccgcccagtgtgagcggtgcacagccggcggccagcacggtgtcgtagaaggccgagatgatgtcgaccgacttttcgagcgaataggtgttgatgggcacgtcgcccaggtcggccacgttgagccgatcgaacggcgccgcgccggtcgccatgttgtagggcctgagcaatgccgattcggcgcgtatctggcgcggcccgaaacgcgcgcccgggcggttggaggtgccgatgtccagcggcacgccgatgaatgccgcatccagcccctctgcggacgttgcaacgggcagccgcatcatcgtgccggggccggcgaagcgcggcatcgcgttgccgccgagcggctggttgggtctggtggcgggcatggcgtgctggtggttcagcgccgacggccgcgcagccattcgagcacgagcagcagcgtggtggtgaagatgatgagcagggtcgccaccgcggcgatggtgggagagatgttctcgcgaatgccggtgaacatctggcgcggcaaggtcacctggtcgggccctgcgaggaacagcgtgaccaccacttcgtcgaacgacgtggcaaaggcaaacagcgcacccgagatcacgcccggcgcaatgaccggcagcgtgatgcgcatgaaggtcctgaacggtgtctcgcccaggctcagcgacgcgcgcaccaggttgtggttgaagccggccagggtggcgagcaccgtggtcagcacaaaaggtgcgcccagtgccgcatgcaccacgatcaggccgaagtaggtgtcggccagcccgacgggcgcgaagtagaggtacgtggcaacacccaccaccacgatgggcaccaccatcggcgaaatcagcacgctcatgagcaagcccttgaacgcgaagttcgtgcgcgacaggcccaccgcggccagcgtgcccagcacggtggccagcaccgtggcggccggcgcgactatgaagctgttgcgcgccgcgcgtgcccactcgggcgattcgaacaggtggcgataccacttgagcgaccagcccgggatcgggtaggccaaaaaggaactgtcggaaaacgacagcggaatcaccaccaggatgggtgccagcaagaaggccagcaccgcgacacagccggcgcgcaccagccaccagccgagcttgtcggcaaaggtggcataggcagggaattggggaagcttcagcatgcttttctttcttccttgccgttcagccgaggctcagctcggccttgccgatgcggcggtacacggcatacagcaccagcgtggcgacgagcagcacggcgcccagcgcacaggccatgccccagttgatttccacgttggtgtagcgcgcgatgtagtagctcagcatctggtcgtccgcgccgccgagcagcgcgggcgtcacgtaatagccgatggccaggatgaacaccagcagcgcaccggcgccgatgccgggataggtctgcggcacgtacacccggaagaaggccgccagcggcgagctgcccagcgagactgcggcgcgcaggtaggtgggcggcacgctcttcatgacgctgtagagcggcaggatcatgaagggcagcaggatgtgcaccatggcgatgatcacgccggtgcggttgaacagcagcgccagcggatgatcgatgaggccgatgcccatgaggccgcggttgaccaggccttcggactgcagcaacacgatccacgccgccacgcgcaccaggatggaagtccagaacggcacgagcaccaggatcatcagcacgttggccttgcgcgccggcagcgtcgacagccaccaggccagcggataggccagcagcaggcagaagaaggtgaccacggcgctgatgttgaaggtgcgcagcaggatgccggcaaaggcgcgctggtcggcgggcatgcgctccacctcgcccgcgacgtcgcgccgcaggtcgaccgaggcgagcaggtagtcgggcgtccagcgcgaaccgttcttggcgatggcctgccagaacggcgcctcgccccagcgcggatcgagctccagcatgcgcgtcttgatttcttccggcgtgccagcaatcggcagcgccctgaaggcgcccatcacaagcgagcgggcgcccgcgatctcagtgttgaggcggcgcgccagggcgcccgcatcggagctgtcgggcagttggccaaggtcggccgcgatggcggcataggccgcgggcgcgggcgcctccttgcggtcccagccatcgagcgcacgcacggtgcgcggcagcgcgttggccacctcgggattctcgaccgcgcgctgcaacagggccacgatgggcaccagcagcgtcagcagcaggaagaccagcagcggcaccgtgagcgcaaaggcgcgccacttgcggcgcgactcggcgcgcgccagtgcacgccggagctcgccgggcggcgccgcttctgccaagacgggggggacagacattgccgcttgcatggcctcttgcctgcttactgcgtggcccaggatgcgaagcgcttctcgagcgcctcgccctggtcagcccagaaaccgacgttgaactgcagcgcatccttggcattggccgccgaggtcggcaggtcggccagcaccttggggctgagcgcagccagggccttggtgttggtggggccgtaggcgatgttctgggcgtagaccgtctggttggccggctgcatcgcgaactggatgtacttcagcgaagcctccttgttcggtgcgcccttcgggatcaccaggtagtcgaggtcgtagatgccgcccggccagtagatcttgaggtcgcggccttcgcggttggccgcgtcgatgcggccgttgtacacggtggtcagcaccacgtcgccggccacgaggaactgcggcggctgtgcgcctgcttcccaccactggatgttgggcttgagttcggtgagcttcttgaacgcgcggtcggcgccttccttggtggcaagcaccttgtagacatcggccggcttcacgccatcggccatgagcgcgaactcgaggttgtagcgcgcgcccttgcgcatgccgcgcttgcccgggatcttcttcacgtcccagaagtcggcccagctggtgggcgcggtcttgagcttttcgccgttgtaggccatgacggtcgaccacacgaacaggcccacgccgcaatcggtgaccgcggccggcaggaagtcggccttgttgccgatcttcgaatagtcgagcttctcgaacaggccttcgtcgcagccgcgcgcggcgtccggcgattcgacctcgaccacgtcccaggtgaccttcttggtctcgaccatggccttgatcttggcctgctcaccgttgtattcgaccggaatgatcttggtgccggtcttctcgtagggctcgtagtaggccttcttctgcgcgttggcgttggcgccaccgaagttgaccacggtgagctgctgctgcgcgaaggcaggcagtgcgaagctggccgcaacggtgcaggcaaggagagtctttttcatggcgggtatcttcctgggtgatgaacggaaacgagaaacgggactgggttcagagggcatacatgcgcgcatgcgcaacgggaaattcgagcgccaccgagtcgccggcctgcggcgtggcgatgccgcccgcgccggtcagcggcagcttcacggtggcctcggcctggccgccgcccacgctgcacagcagccgcaggtggtcgccgaaatagatgacgcgcgccaccacggcggcgagcatgttggcgccctgcgcttccggccggtggtgcagcaccacgcgctcggggcggatgcaggcctcgacggcagcgcccgcggccgcgccgctgacgttgagcccgtgcagcacgcggccatcgggcagcgtcatttcggcatgcttgccgccccggctcagttgccccttgagcacggtgttgtcgccgacgaaaccggccacgaaacggttggacggtgtctcgtagagccggccgacggtgtccagctgctggatcacgccttcgttgaacacagccacccggtcgctcatggtgagcgcctcgccctggtcgtgcgtcacgtagacgaaggtcacgccgagctggcgatgcaggtccttgagctcgatctgcatgtgctcgcgcagttgcttgtcgagcgcgccgagcggctcgtccatgagcaccagttgcggctcgaacaccagcgcgcgcgccagcgccacgcgctgctgttggccgcccgagagctggccgggcaggcggtcggtcatgccgcgcagctgcaccatgtcgagcgcgcgctgcacgcggcgctgctgctcgtccttggacaccttgcgcacggtgagcggataggccacgttctggcccacgctcaggtgcggaaacagcgcatagttctggaacaccatgccgaagtggcgcttgtgcggcggggtgccggtgatcggcttgccttcgagcaatatctcgccggaggtgggcgactcgaagccggccagcatcatcagcgtggtggtcttgcccgaccccgagggcccgagcaggctgagaaactcgccgcggtggatgtccaggtcgagctggcgcaccaccaggtgttcaccgtcgtaggttttctggacgcgctggaagcgcaccaagggttctgctgtcgtcatggaggggctcaagaaaagggaccgttcagcgcagcgcggcgaagctgtccgcgagaagcgccaggccttcgtccacaagcaagtcggatgccgtcagcggcaccagcacgcgaattacattgccgtaggtgccgcatgacagcaggattaacccgcgccgcgcggcttccgccaccacctttcgggtcagcgcggcatcgggccgggcggtgtcgccctcttcgaacagctcgatggccaccatggcgccgagcccgcgcacgtcgccaatggcgggctcgctggccgcgatgcggcgcaggccacccgtgagccgctcgcccagcgcccggctgcgcgccagcaattgctcgtcgtcgaacaccttgagcaccgcgagcgcggcggcgcagccgatggggctgccggcataggtgccgcccagtccgccgggcgcgggagcgtccatcacctcggcgcgacccaccacgccggagatcgggaaaccgcccgccatcgacttggcggtggtgatcaggtcgggcgccacgggccattgctcgctggcaaaccaggtgccggtgcggccggcgccggtctgcacttcgtcggcaatgatgaggatgccgtggcggtccgccagcgcgcgcaggccttcgacgaagtcgtggggcgccacgtagaagccaccctccccctgcaccggctccaggatgaaggccgccacgcgctcgggctcgatgtcgttcttgaacagcagctcgaccgagtgcaaggcgtcgtccacgctcacgccgtgcagcgcattcggatacaacgcatggaacacctcgcccgggaacgggccgaagccgactttgtagggtgcgaccttgccggtcaggcccagcgtcatcatcgttcggccgtggtaaccgcccgtaaaggcaatgacgcccggccggcgcgtgtaggcgcgggcaatcttcaccgcgttttcgaccgcctcggcgccggtgctcaggaagatcgatttctttgcgaattcgcctggcgccagcgcgttcaggcgctcggcaagttccacgtagggttcgtacgccatcacctggaagcaggtgtgcgaatagagatcgacctgcgccttgacggcggcgctgatctccgggtggcagtggccagtgttcaggaccgcgatgccgccggcaaagtcgatgtagcggcggccctcgacgtcccacatctcggcgttggcggcgcggctgacaaaaatttcgtgggcctggcctacaccgcgtgccactgccgcgctgcggcgggccatgagggcggcgttgctgagatggggttcgcgctgcatggattcgacctgtgcctgaatgaagaagcaggcactttaggtttcagctccagcgccgaccatgtacaacgaatgcgatgattttgcggactgtgctggtcttgtatcctgtacatactttcctcaatatggtgcagatcggcctgccgggatactcgcgatgctcattcttcaccccgaacagccgactccgctcgtgagtcagatcgtggagggactccgcgggctgatcggcgcccaaaaactgaggcccgacagcaagctgccctccatccgggcctttgccgcggcccatggcgtcagcgtcttcaccgtggtcgaggcctacgaccggctggtggcgcaaggccttttggtgtcgcgggccaacgccggcttcttcgtcaagcggcgaagcgacgacaactcccccggcagcggctcgacggcgccgcaacccgacccgcgcttcgatgcgcgctggtatctgcggcagatcttcgagaaccgcaacctgccgctcaagccgggctgcggatggctgccgcacgactggctgttcgaggacggcatgcgccgcagcctgcgcagccttgccgcgggcggcaccgacatcggcggctacggtctgcccttcgggcacatggcgctgcgcatggcggtggccgattcgctctgcgagcggcagatcgcggtcgaggccggccaggtgctgctcacccagggctcgagccaggcgctcgacctggtggcgcgccagttgctgaagcccggcgacgaggtgctggtggacgatcccggctatcccaacctgatgttcatgctgcgctttctgggcgtgcacatcatcggcgtgccgcgcacgcccaccggctacgacctgcccgcgctggaggcgctgctagcgctgcaccggcccaaggccttcttcacgcaaccgcggctgcagagccccacgtgctcgctggcgtcgatgccgcagctcgtgcgcctgctccagcttgcgcaggagcatcagttcgcgttggtcgagaacgacatctacgccgacatggacgcctcgtcgcgaccctcgctcgcgagcctcagccagttgcgccaggtggtctacgtcggcagtttttccaagaccatctcaccgaacctgcgggtcggctatgtggtggcgcagcccgggctgatggaagacctggcccagctgaagatggtctcggggctcacctcgtcggacatcaccgagcggctggtctttggcgcggtgaccgacgggcgctggcgcaagcacctgaagtcgctgcgggaacggctcgcgcaggcgcattcgaacgtggcaaggcgcttggaagcccagggcttcgagatttttcatgagcccgcagcgggcttgtacctgtgggcgcggcatccggacatcaccgatgccgcggacctgtcgcggattgccgccatggagggcatcatgctcggcccggggcagttgtttctggtgattccgcgccccacggggtggctgcgcttcaacgtggcgttcagcgaggacgagcggctttggcagtttctcgcgcgcagcatcgaagagcgcaaaggggagtgagtgagtgcggcagggctcgaatgcgagccccgaaaagacaaaagggttagcagacgttaatctgctaacccttgtcggaactggcggagtggacgggactcgaacccgcgacccccggcgtgacaggccggtattctaaccaactgaactaccactcctggtagacaacgttcactccttgcggagccaagtgctgacgacttgtgcctgcttcacttgcgcgaaactggcgaccctacggggattcgaaccccggtagccaccgtgaaagggtggtgtcctaggcctctagacgatagggtcaaaaccttaggaaccgtgctgcgatcagcacttcttctcttctcgacactttgatggtggaggtaaacgggatcgaaccgatgacctcttgcatgccatgcaagcgctctcccagctgagctatacccccgtgtgggtgtcgagcctcaaattatagcctgaaaaatcaggctcttttcaaacgctcgatgactttttcgcgagaaaaaattgcgagcactgaatcgagggatggtgtctgcgcagttcccatcacgaggacgcgaaccggcatggccaacacaggcattttcacagaatgtgcggccaaaacttccttgatgccggcagcaatcgaagttttttcccagttcacgctcgcgagcttttcggccagcgtggcgatgacgggcttcaccgcgtcggtgatgtgctgcgcgcgatcggcttcgctcacggtcacgtcggcatagaacgctgcggcccagtcggccaatgcaaccgtggtctcgcaacggtccttgaacagcgcgcagatcgcggggaggcgatcgtcggcgtcgataccgcgcttcttcaactgcgcggccacgagcggtgcgagctcatcatcaggcttggccttgatgtattgcgcattgacccacgacagcttggcggcgtcccactgggcggggctcttcgacaggtgcgaaccgtcgaaccagctcaccatctgctcgcgcgtgaagagctcgtcgtcgccatggctccagccgaggcgcgcaagatagttgagcatggcttcgggcaggtagccgttctcttcataggcggtgacgctcacggcgccgcggcgcttggagagcttctgcccgtcgtcgcccaggatcaccggcacatggccgaacgcaggcagcggcgcgcccagcgcgcgaaagatgttgatctgccacggcgtgttgttgatgtgctcgtcgccgcggaacacatgcgtgatggccatgtcccagtcgtcgaccaccacggcgaagttgtaggtgggcacaccgtcgggccgcaggatgatgaggtcgtcgatctcgcggttgttgatggtgatctcgcccttgacgaggtcgttccacgtcacgtcgccttcgggcgggttgcagaaacgcaccacgggcggcacgccttcgggcacgggcggcagcaccttgccgggctcggggcgccagcggcggtcatacaaggtcttttcgccgcgggcgcgctgggcttcgcgcatttcgtcgagctcggccggcgtgcagtagcagtagtaggccgtgccggccgcgagcatttgcgcaatgacttcgcggtagcgctcgaggcgctgcatttgatagatcgggccttcgtcgtagtcgaggccgagccagtgcatcgacgcaaggatctggtcggtcgagtcctgcgtggagcgggccacgtcggtgtcctcgatgcgcagcacgaactctccgccatggtggcgtgcgtaggcccacgagtagagcgcggtgcgggccgtgcccaggtgaagaaagccggtgggagacggagcgatgcgggtgcgaactttgccggtcatggaatcgatcagaatttcagggtgccaaggccgcgaagcaagtcggccttgatgtcgtcgatgtactcgaggccgactgcgacgcgaatgagcccctggccgatgccggcggcctggcgctgcacttcggtcaggcggccgtgcgacgtggtgccggggtgggtgatgatggtcttggtgtcgcccaggttggtggcaatgctcaccacgcgcgtgctgttgatcacgtggaaggcattggcgcgcgccgtctcgggatcgttgccgaccacgtcgaacgacaccaccgccccgccctgccccgactgctggcgcatggccaggtcgtgctgcgcgtgcgaggcaaggcccgggtagtagacgcgcgcaatgccgggctgcgtttcaagccactgggccacggccagcgcattggcgcactgcgcctgcatgcggatgccgagcgtttcgaggcccttgagcacgacccatgcattgaacggcgacagcgccatgccggcggtgcgcaccaccgggccaaacacatcgacgatgagcttcgacggaccgcagatcgcgccggccatcacgcggccctggccgtcgaggtacttggtaccggaatgaatgatgaggtcggcgcccagttcggccgggcgctgcagcgcgggcgtgcaaaagcagttgtccaccgcgagcagcgcgccgccgccgtgcgccaggtcggccagcgcgcggatgtcgcacacctcggtgagcggattggtgggcgtttcggcgaacagcagcttggtgttgggcttcatggccgcgcgccattcagccacgtcggtctgcgagacgaatgtggtctcgacgccgaacttggcgaactccttgccgaacaggttgagcgtggagccgaacaccgagcgcgagcagatcacatggtcgcccgccttcagcaggcccatgcacatcatgaggatcgcgcccatgccggtggaagcgccgatcgcggcctcggtgccttccattgccgcaaggcgctgctcgaagctggtgaccgtgggattggaagtgcgcgaataggtaaagcccgcttcggtaccggcaaagcggcgtgccgacgtttcggcgtcgggctgcacgaagccgctggtcaggaacagcgcttcggagtgctcgccatgctggctcggcgccaggccggtgcgcagcgcgagcgtgtcgcgatgcagtccgggcggcagggttcgttcgtcggcagtcaattcagctctcactcgctgtgattgggaagcgcgaggcgcgaagaatcttcttcggtctcttcgatgcggggacggttgccgttcatgcgcgagatcgcttcggtgtcgatgtcgccggtcacgtacacgccgtcgaagcaggaggcatcgaaaccgttgagcttggggttgagcgagccgatggcgcgcttcatggcatcgacgtcttgatagatgagtgcatcacaaccgatcagctcgcggatctgctcgacggtgcggtcgtgtgccaccagttcgtccttggtgggcatgtcgatgccgtagacgttgggatagcgcaccggcggcgcggcgctggcgaggtagaccttgcgtgcgccggcatcgcgtgccatctgcacgatttcacggctggtggtgccacgcacgatcgagtcgtcgaccaggagcacgttgcggcccttgaactcgctggcaatcacgttgagcttctggcgcaccgacttcttgcgcacgccctgccccggcatgatgaaggtccggcccacgtagcggttcttcacgaagccctcgcggtagggcacgccgagcaggtgcgcgagctgcgtggcgctcgggcggctcgattcgggaatcgggatgatcacgtcgatctggttcggcggcacggtggacaccacgcgcttggccagcgtctcgcccaggttgagccgcgcctggtacaccgagatgccgtcgagcaccgagtccggacgcgccaggtacacgaattcgaagatgcaggggttgagcgtgggcgcctcggcgcactgcatggagtgcacgttgccctgcaggtcgatgaacacggcttcgcccggatcgatgttgcgctcgaacacatggcccgagccttcgagcgcgaccgattcgctggccaccatgacggtgccgtcggcgctgcggcccatcgacagcggacggatgccgtacggatcgcggaaggcaagcaggccgtggccggcgatcagcgccaccacggcatacgagccgcgcaggcgcttgtgcatgctcttgaccgcggcaaacacctcggccgggttcagtggcacgccgcgcgatgcgcgctcgagctcgtgcgcaagcacgttgagcagcacttcggagtcgctctcggtgttggtgtggcggtggtcggtggagaacagctccgaacgcagcgcatgcgcgttggtcaggttgccgttgtgcaccagcacgatgccgaagggcgcgttgacgtagaagggctgcgcctcttcttcgctgtaggcgttgcccgccgtcggatagcgcacctggcccagacccacgctgccaggcagcgcgcgcatgttgcgcgtgcggaacacgtcgcgcaccatgcccttggccttgtgcatgaagaacttgcgttcaagcagggtgacgatgccggccgcgtcctggccgcggtgctgcagcagcagcaaggcgtcatagagcagctgattgacgggtgcgttgctgacaacgccgacgattccacacatgaacgattcctctcagggcaggtagcttgccaacttttcaggcaacgcgggtttcaggccctgcaatgccgcatcgagaacaatggcgctgcgcgattcgtgccaccaggcactgtcgctcaacgccagcaaatgaacaatgaccgccagaacgagcagtgcaaccgcaccccgcgccgctccgaaggccccacccaatatccggtccaccggcctgaggccgacagccgcaatcagctttcgcgtcagcgccgccaccaggcccacgccgaacgccaccgccacgaacaccagcacaaaggccagcggatagcgccaggtggcctgcgggtcgccgaagggcagccatgcggccacgctcgacgccagccactgggcggcaatgaatgcagccacccaacccgccagcgaaatcacttcgaacaccaggccccgccagaggccgaacagcatcgacacgacgatgagcgcgacggcgatccaatcgagcagggccacggcaacgggcgatggctactacaacgtgaggatggcggccgacaaagacaagcccttgaccttctccgcggccttgtccgcctcggcgcgcgagctgaacgggccgacacgcacacgcgtgcgctgctcgccgtcggacgtcttggccacgttcacataggtcttgaggcccgccttctcgagcttctgccgcacttcgcgcgccttgtcggcatcggcaaaggcaccgacctgcacaacgaagcggccgccgtcttcggtggcgggcttggtggtgctggtgttggagggcttgccttcgagcagggcgcgcgcgcggttgccgtcctcggccgcagccggcttgggcgccgcgggcttgggttcgggtttggcttccggcttggcctcgggctttggcttcggttcgggcttgggttctggtttgtgttccggctttggctcgggcttgcgttccggcttggcttcggccgtgggccgggtttcggccggaggcgtgctggcggctggcttgccgggtggaatctcggtgccgtcggcggtctcggtgatcatgccgccgctcgacgcggacgggggcgccgccgccacgcgggcgccgctgtcggccgcgccggtggtgggcgcggcgggcgcgggcgttgcaggcaccggcaatggcttgaccttgttgcggtcgggaatctcgatgggaatgtcgaccgagaccggacgcggctgggtgtcgaacagcaacggaaatccgatgacgccaagcagcaccagaacggccgcgcccaccaaccggtgccgcgcgcggcggcgcatggtttcgacactttccgcagggacggcagccggtgcgccgcgtccttcgttgccttgcgggccgcgcgtgcggaacttgaaaaacgccatgaagttcgatccctgaaggagtgcagcgaggtggtgccagatggtgcggacgggccggcgatcagccgccgggcagcaggtgtttggcttgcagccggggagtgccgtgctccagcacgccacccacggtgaagaacgatccgaagaccacgattctatcagcggggtctgcgtgctcgatggctgcgcggagcgcttccatcggcccggaatgcacgcttgcggaggcgtcggcgcgcttgttttgcgcctgccagctcgcaagcagatcgccggccttggcggcgcgcggcgtcggcagatcggtgaagtaccagcggtcgatcatcgggccgatgcgcgcgaggatcggggccaggtccttgtcggccatgacgccgaacacgccgtgcgtggtgggatagaagcccatcgcgtcgaggttctcggccagcgccgcgaccgcatgggcgttgtgcgccacgtcgagcaccagcgcgggctcgcccggaacgatctggaagcggccgggcagctcgaccatggcgagccccgtgcgcacggcctgcgcggtgatgggcagttgcggccgcagcgcttcgagcgccgcaagcacgcccgcggcattgagcagctggttggcgccgcgcagggccggataggccagcccgctgtagcgccggccgcggcccgaccaaccccactgctgcttgtcgcccgagacgttgaagtcgtgcccgaagcgccagaggtcggcgccaatggccgccgcgtggtcgatcacgctttgcggcggcatcgggtcgctcacgatggcgggcttgcccgggcgcaggatgccggccttctcgaagccgatgctctcgcggtcggacccgaggtagtccatgtggtcgaggtcgatgctggtgatgaccgcgcaatcggtgtcgatgatgttgaccgcgtcgagccggccgccgagcccgacctcgagaatggccacgtcaggcttctcttcgatcatgcagcgcaggatgccgagggtggtgaactcgaagtacgtcaggggcatgtcgccccgggccacttctaccgcctcgaagtttgctattaatttcgaagcatcgaccgcttcgcccgagagccgcagccgctcctcgaagcgcaccaggtgcggcgacgtgaaaaccgccgtgcggtagcccgcatgcgtgaggatcgattcgagcatggcgcaggtcgagcccttgccattggtgccggccacggtgatgaccgggcagtcgaagcgcaggcccatgcgggccgccatctctctggcgcgctcgaggccgagctcgatgttcttcggatggagttgctcggcgcgcgcgagccagtcgttaagggtttccatggaggccggcattgtcgccgacccggaaagcgcggggcgccccacgttttatcggcatcattggcatccatgacaaccctctacggcattccgaactgcgacaccgtcaagcgcgcccgcacctggctcgacgaccatggcgtcgcctacaccttccatgacttcaagaagcagggcgtgcccgaagccgagctcgaccagtggctcaagaagccgggctgggaggccttggtcaaccgccgcggcaccacctggcgcaagttgggcgaagccgaacgcaacgcggtggtcgatgccgtttccgcccgcgccgcattgctggccaaccccagcctcatcaagcggccggtggtcaactggggggccaaaaccggcgttacgacagggttcgacgccgaagcctgggctgctgtgaatgccgtgtaaaccccggaacccgtctcgccggccggcctccaaccccgatctgcaggagagaacaccatgaaccgacaagtctttcgcgccctctcgggcctttccgtggccggcctgctgacggcaggcgccgccggcgtggcccaggcccaggaagcatgggcgagggtgatttccgccacccccgtctacgagaccaccggcagcagccccagttacaacgtgacctacgagtacggcggccgccaatacaccacgcgcatgaacagccggccgggcgccaccatcccgatccaggccggcgcctacggcgtgacgacggcaccggtcgcgccccagccccagttgcagccttacccggtcgaagccgacagcggccagcagcagtaccagtaccagcagcccccgcaatacgcacaaccgggcggatcggcctgggacaacgtggtgcccgagcccggcgtggtggtttccaacgcgccgccggcaccggtctatgcgcagccggcgccgatctacgcacagccggcgccggtgtacccggcccccatctacgcgcagccgacctacgtctacccgcagccctacgtctatccgccggtcggcatttcgctgaacctggggtactccaggggctggggcggctatcgtggatacggctatcgccactggcgctgaaccgcgcgatacggcggccgggctggcaataccggccaagccctaaaatcgaggacttttccaacccccaaggggtgcgccgccgcggtggcgcgtcctcgacaagccgaccgcgcatgcgccggcgccttccaatgacgacgactaccgacactctcaacagcgccgcagtggcgaccaaggccaatgtgtatttcgacggcaagtgcgtgagccacagcctcacgttggccgacggcacgaaaaaatcggtcggcgtgatcctgccgtccaccctgactttcaagaccggcgcgcctgaaatcatggaaggcaccgccggcagctgcgaataccaactgtcgggaaccaccgagtggattgcctcgggcgcaggacagaagttcaacgtgccgggcaattcgagcttccagatccgggtgaccggcgagccctacagctacatctgccacttcggctgacccctgaaccgccaaccggacacccgcatgtcgaccattctccaaaacgttcccgccggccagaaggtcggcattgccttttcgggcggcctggacaccagtgcggcactgcactggatgaagctgaagggcgcgattccctacgcctacaccgccaacctcggccagcccgacgagcccgactacgacgagatcccgcgcaaggcgatgctctacggcgccgagaacgcccgcctgatcgactgccgcgcgcagctcgccaatgaaggcattgccgcgctgcaggccggcgccttccacgtcacgaccgccggcgtcacctacttcaacaccacgccgctcggccgcgcggtgacgggcaccatgctggtgtcggccatgaaggaagacgacgtccacatctggggcgacggcagcacctacaagggcaacgacatcgagcgcttctaccgctacggcttgctcaccaaccctgctctcaagatttacaagccctggctcgaccagctgttcatcgacgagctcggcggccgcgccgagatgtcggcattcatgaccaaagccggcttcggctacaagatgtcggccgagaaggcctacagcaccgactccaacatgcttggcgccacgcacgaggccaaggacctggagaacctcgacagcggcatgcaaatcgtgcagccgatcatgggcgttgcgttctggaaagacgaagtcgaggtcaagcgcgagaccgtcagcgtgcgcttcgaggaaggccgcccggtggccctcaacggcgtcgagcacgccaacctcgtcgacctgatcctggaagccaaccgcatcggcggccgccacggcctgggcatgagcgaccagatcgagaaccgcatcatcgaggccaagagccgcggcatctacgaggcgcccggcctcgcgctgctgttcatcgcctacgagcgcctggtgaccggcatccacaacgaggacaccatcgagcagtaccgcgacaacggccgcaagctcggccgactgctctaccagggccgctggttcgacccgcaggccatcatgctgcgcgagacggctcagcgctgggtggcgcgcgccatcaccggcgaagtgaccgtcgagctgcgccgcggcaacgactactcgattctcaacaccgtctcgcccaacctcacctaccagcccgagcgcctgagcatggaaaaggtggccggcgcgttcacgccgctggaccgcatcggccagctgaccatgcgcaatctcgacatcgtcgacacgcgcgagaagctcgcgatctacacccgtaccgggctgctgtcgccgggccagggcacctcggtgccgcggctctcgaacgacgacgagagcaagtaagccgacgcgcttcttgcaatgacaaacgggccctcgcgggcccgttttcatttgtgcgtcgtgcgtgcctgtctatcgatcagtcgccgccgcctcctccgcacccgccaccgcaaccgccggaggaatcccctcccccgctgccgccgtcaccgctgccgctcgattcgctgccgccgaagccggtggcatcgccggagctgccgccatccgatgacgacgaatcgccaaagctggtgccgcaatgggcgccggagccgttgtgccgatcgacggccttgcagtcgggcacgtagtcgaagccgcccggaatgccgaacttcacgtcgagcgcaaacaaaagcggcaggcgcgccggcttgcgcggatcgatgctttcttccttgcaggcccaataccagctgcggcgcaggccgtcgttgcgcttcgggtccttgcccagcacttcggccgggctgtggtgaagcatgccgccaaaggccgccttgcaccagttctggtaggaacggcggcatccgggcctcgcggatgaactggcggcgcaggctggtttccatgaagcccagcgtggccgccagggcccacgcgccaagaatcaatggcaccagcaccagccagccgccatggcggaagatgaagaacaccgagaccaacgctccgaccaccaccgcgcggcgaacccagatcagcgcggcaatgcgccgccggtagttcaggtgcaggaagtcgaggtccatcagacgaccaccggctccggctccagccggatgccgaagcgctcgtacacgctcgtctggatggccttggccagcgtcatcacctcgccgcccgtcaccgggttttcgagcccgccccggttcaccagcaccagcgcctgcttttcgtagacgccggcattgccgaccgacttgcccttccagccgcaggcgtcgatgagccagccggccgccagcttgatgctgccgtccgccatggggtaatgcacgatcttcgggtcgcgcgcgatgatgtcggcgcactgctccggcgtgacggtcgggttcttgaagaagctgccggcattgccgagcacccgccagtcgggcagcttggcgcggcgaatggcgacgacccagtcgaacacgtcggtggcgctgggcgtgaagttgccggcctcctccatcttgcgttcgaggtcgaggtagccgaccaccgccttccacggcttgggcaggcgaaagcgcacgcgggtgatcagcgcccggcccgagagcccgaaatcgttcggcccgctgcgcacgtgcttgaacaccgagtcgcggtagccgaaggcgcattgcgcggcgtccagcgtgaagctgcgcccggagtccaggtcgatggcgtcgagcgaatcgaaacggtcttgcagctcgaccccgtaggcgccgatgttctgcaccggcgcgccgcccaccgtgcccggaatgagcgccaggttctcgagccccgggtagccgtttgcgagcatccattggatggcgtcgtgccagacttcacccgcgccggcctccacgatccaggcgcgcggggtttcttcgaccagccgcaggcccttgatctcgaccttcagcaccagcggcttcacgtcgcccgtgagcacgatgttgctgcccccgcccagtacgaaacggggcgcgtcgcgccagcgggggtccgcccgcagttcggccacgtccccctcgctggcgatgcgcaccaggttctgcgcgcgcgcgacgatgccgaagctgttgtacggctgcagcgggacgttgttctccacgatcatgggagaattgtcgcatccagcacccgcgaatccaggaggagcccaatgccgtctttcgataccgtctgcgaaccgaatctgcccgaagtgaagaacgcggtcgaaaacaccgccaaggaaatcgcgacgcgtttcgatttcaagggcacggccgccgccgtcgagctcaaggacaaggaaatcaccatgatcggcgatgccgagttccagctcgtccaggtggaagacattcttcgcgccaagctcaccaagcgcagcgtcgacgtgcgctttctcgacaagggcgacgttcagaaaatcggcggggacaaggtcaagcaggtcatcaaggtcaagagcggcatcgaatccgagcaggccaagaagatcacccgcatcatcaaggacagcaagctcaaggtgcaggccgccatccagggcgacgcggtgcgcatcaccggcgccaagcgcgacgacctgcaggccgccatggcactcatcaagaaagacgtgcccgacatgccgctgtcgttcaacaacttccgcgactgagccgcggatgaaatccctcgtcgtcgcggtgcagctgctggctgccgctgcgggcgcgcatgcagcgagctcggtcatgctgaccggcaccatcggcagccgggccatcctgatcgtggacggcgcgccgcccaagaccgtggccgtcggggagaccttccagggcgtcaaactcgtgtctttgcaggccgaactggcagtggtcgagctcgaaggcaagcgcctcaacctgcgcatggacacgccggtaagcattggcggcggagggggcacgggcggcggcagccggatcgtgctgccggccgacagccgcggccacttcatgacgcaaggcgccatcaacggccgccccgtcaccttcatgctcgacaccggcgccacgtcggtcgcgatgtcggccgccgatgcgcagcgcatcgggctggactacagcaagggccagcgcgtgcagatgagcaccgccaacggcgtggccagcggctacaagctccggctccagtcggtgcgcgtgggcgacgtcgaggtgtacgacatcgacgccatcgtctcgccccagcccatgcccttcgtgctcttgggcaacagcttcatcaatcgcttttcgatgcgccgcgacgcggaccagatggtccttgaaaaacgctactgagcgccggcgtcaggcctgcgctgccgtgaccacgatctcgatcttgtaggccgcattggccatcttggcctgcaccgtcgcgcgcggcggcgtgttgccggcgggaatccacgcatcccagacctcgttcatggccgtgatgtcgttgatgtcggccagaaagatctgcgtcatgaggatgcgcgacttgtcgctgcccgcttcggccagcaggcggtcgaccatgtccagcacctgcgtggtctggccgcggatgtcctgcgtggtgtcgtcgggcacctggcccgcgaggtagatggtgccgttgtgcacggccgtttcagagaggcgcgggccgacgtggtagcgggtgatggatgccatggtcttcaagcctttttcttcgagccgagtttcgactccgtgccggccgcgagccggcggatgttttcgcggtgccgccagatcagcagcaggctcatgatgatgatcgcaatcagcaccgtgcggtcgagcggccatgcaatgttgccgcccagaaggtaataagccggcgcaaagaaggccgccaccagcgacgacagcgacgaatagcggaagaacaccgcaatgatcagccaggtagcgccggtggccagccccagccagggcgcaatgcccaccagcacgcccgccgcggtggccacgcccttgccgccctggaagccgaagaacaccgggtacagatggcccaggaaggccgcgaggcccgccagcgcggccacgccctcgcccagcccccattgcgcgccaaagtggcggatcaggaacaccggcagccagcccttgagcgcatcgagcagcaaggtggccagcgccgcgcccttgttgcccgagcgcagcacgttggtcgcacccgggttgccgctgccgtagctgcgcgggtcggccatgccgagcgacttgctcacgatgaccgcgaaggacagcgagccgatcaggtacgaggccacgatggccaggagggaaggcagatgaaagctcaaggcggcgctccacgaaggatggatgttcttattcgctgattcggacagagaggcttgccgccggtctcacgccggcgggccggctattctgccagcgcgcactgcactggcttggccgccagcaaggtgacgcacacctgcgggtcgatgcccaccaggtagccgcgccgcccgccgttgatcgcgatcctgggcagctcgaggatggtcgactcgatgtagaccggcatctggcgccgcgtgccgaagggcgaggtgccgcccaccatgtagccgctgtggcgctgcgccacctcgggcttgcagggctccaccgatttggcgccgatctgccgcgccagattcttggtcgacacggtgcgattgccgtgcatcagcacgatgagcggcctggcgtcctggtcctgcatcaccagcgtcttcacgacggtgaaagggtcgaagcccaacacctcggcactgtgctgcgcgccgccgtgctccaggtattcgtaaggatgctcggtgaacgcgaccttgctcgcgcgcagcagctgcgtggcgggggtttctgaaacgtgagcttttttgatcacgccgccggatcccggatctcccaccggatcctgtcgatctcggccagcacctcgggagtgagcgtgatgccgaaggcgtcgatgtcttcgtcgagctgcgccagcgtggtcacgccgatgatcgtgcttgccacctgccacttggtgtagcagaagcctagagcgagctgcaccggcgtcaggccgttgtcgcgcgcgagctggttgtaaaggcgcgcggccttcagcgcgtcggggcggccccagcgttgcttgcgcaccgactcgtagctcgaaatgcgcgcacccttcggcgcctccggcccctcgatgccgctctggtcgtacttgccggtcaagaggccgaaggccagcggcgaatacgccagcagcgacacgcccagccgatgcatggtctcatcgagcccgttctccaggccgcggctcgccaggttgtagacgttctgcaccgtggccacccgcggcaggccatgctgctcggccagccgcacgaactcgtgcacgccgtagggcgtctcgttcgagaggccgatggcgcgcaccttgccggccttcaccagcttgccgagtgcctcgagctggtcgtggatgggcgtcttcgagctttccttggcggggtcgtaatagatgctgccgaaggccggcacgtggcgctcgggccagtggatctggtacagatcgatgacgtcggtcttcaggcgcctcaggctcgcattgcacgaggcctcgatgtcctcgggcgtcatgccgctgcctgcgcgcacccagggcatgccgcgcgacgggccggccaccttggtggcgagcgtgatcttctggcgcgctccggggttggccgcaaaccagttgccgatgatggtttcggtgacgctgaaggtctcctgccgcgtgggcaccgagtacatctcggccgtgtcgatgaaatcgacgccgcgctcgagcgagcggctcaggatggcatgggaagtgggttcgtccacctgttcgccgaaggtcatggtgcccaggcagatcggggtgacgtgcaggtcgctctggccgagttggatttttttcatgcgcgggatgctaccgccctccccggcaatgcgctggccacgggccaaaaagccgggcgccagctgtcctgtgccggactgcgcgccggcgccgggctccttatcatcgacgcccatgtaccaagctcttcgtccctcgcgcagcgaattcgtgcccgtgcgcaacctcagctaccacgtgcgcctctggggcgagccctcggccgcgcggccgccgctggtgctggtgcacggctggatggacgtggccgcctcctggcagttcgtggtcgatgcgctggccgaagagcgcttcatcgtcgcgcccgactggcgcggcttcggcctcaccgagggcggcggggtcgacaactactggctgcccgactaccttgccgatctcgaatggctgttcgaccactacgcgggcgaaggcgatgcggcgcggccggtcgacctggtcggccacagcatgggcggcaacgtcgccatgcactacgcgggtgcaaggcccgagcgcatccgccgtctcgtcaacctcgaaggcttcggcatgccggcgcgcaaacccgaggaagcgcccgcgcgctacggccaatggatcgacgagctcaagcgcctgcaccgcggcgagatggcgctggccggctactccgccgtggacggcgtggcgcgccggctcatgaagaccaacccgcgcctcacgcccgacaaggccaattggctcgccagccactggtcggcaccgcacgcgcaggccgacggcagcgagcgctggcagatcctgggcgaccccgcgcacaagatcatcaacgccaacatcttccgcgtcgatgaaaccctcgcgctctatgcgcggatctcggcgcccacgctgatgatcgaggcctcggacgacagcctgcacggctggtggaagaaccgctacacgctggacgagttccaccagcgcctccagtccgtgccttcggtgcgcatcgagcggctcgacgacgcgggccacatgctgcaccacgaccagccgcagcgtgtggccgggctgatcgagcagttcctggcgggctgagcctcaggggccttcagccccggcgcggccctgcaccgtgcgctgcagcgccgcgcgtgccaggagccgcgtcgaatcgagtgtcggcagcggcgagttcacgtcgttcatgatgagcggaatctcggtgcagccgagcacgaccgcatcgcagccgtcctcgtccttcatgcgctggatgacgcggcggaacgcggtgacggcaccaggcgtgaagacaccgcagaccagctcgtccatgatgatgcggttgatctcttcgcgttcttccacggtgggccgaacgtattcgagccccttggccgaaagcttttcgggatagacctcgctctcgaccagccatcgcgtgccggtgatggccaggcgccggaaaccgcgctgcacggcctcgtcggccacgcactgcgcgatgtgcagccacggcagcggcgagcgtgcctcgatgaagggcagcgcctggtgaatggtgttgtcggggcagaccagaaagctcgcgccgatcttcgcgagcttgttggccgacgcgagcatcacctcgcccacgccgcgccagtcgttgcggtagatgtgcgccatgtagtccgcgagcgagggcgtgtgcatcgagacttcggggtgcgcatgcgggcccagcagttgggcgccctccacgcagatggtctggtagcagagcgccgcgccttcggcggagcatccgacgattccgatgtgctgggtcatggcgcatcctacaaaaaagaatgccgccatgcccggctgaccgatcaggcgtggctcgcctcgctgtccagatgcgccatctgcgcggcggcgtagcgctcaccggccgcggcgcccttcggcactgcacgttcgatggctgcgagatcgtccgcgctcaaggcaacgccgagcgagcccagcgcttcgtccagccgcgtgcgctgccgcgcgcccaccagcggcacgatgtcctcgccctgcgccgccacccatgcaatggcaatctgcgcgaccgtcacgcccttggcgtccgcgatcttgcgcagcgcatcgaccaacgccaggttgcgctcgacgttctcgccctggaagcgcgggctgtgcgtacggaagtccgcagcacctgcgccctctttcttccaatgcccgctgatcagcccacgcgacagcacgccgtaggccgtgatgccgatgcccagctcgcggcaggtcgcaagaatgtcgtcctcgatgccgcgcgagatcagcgaatactcgatctgcaggtcggcaatcgggtgcacggccgccgccttgcgaatagtgtgcgagcccacttccgagagcccgatgtgccgcacgtagccggccttcaccatgtcggcaatggcgcccacggtgtcttcgatcggcacgttcgggtcgagccgcgccgggcggtaaatatcgatgtggtccacacccagccgctgcagcgaatagaccaggaagttcttcattgcctcgggccgcgcgtcgtagccgctccaaccaccagccggatcgcgcagggcaccgaacttcacgctgaccagggccgcgtcgcgctgcgagcccttgaggcccctgagcgcttcgccgatcagcatttcgttgtggccgctgccgtagaagtcgccggtgtcgagcagcgtgatgcccgcgtccatggcggcatgaatggtggcgatgctttcggcacggtccgaggggccgtacagcgccgacatgcccatgcagccgaggccgatggcggagactttcgggcccgcggccccgagttgacgtgtgttcatttcagcttcctttcgttgaggtccgcatgcggttgcgagcggcatggctgtagtctggaagaaagcacctcgttcgataatccacccatcaccgcacgagctgtgcaaaaaaccgcacaatccgctttcatgaccgaccctgacctttcggacctcggcgccttcatggcagtgacgcgggcacgcagctttcgcggcgccgccgcgctgcgcggcgtgtcgccctcctcgctcagcgaggccatgcgccggctcgaggcgcagctgggcgtgcggctcctgaaccgcaccacgcgcagcgtgacgcccaccgaggccggccagcggctgctggagcgcattgcgcccgcgctcgacgacatctcgggcgcgctcgacacactcaacagctttcgcgacagccccaccggcacgctgcggctcaacgtgccgacgatcgtgacgcagcgcgtgctgccgccgctggccgcccgcttcctggcggcgcaccccggcatcacgctggaggtgacgaccaacgacaccttcatcgacgtgctcgcggccggtttcgatgccggcattcgctacgacgagagcattgcaagggacatgatcgcagtgccgctcggcccccgcgtgcagcgcttcgtggccgccgcgtcgccgggctacctggcggcgcacggcacgcccaggcacccgaccgacctgctgcagcacgcctgcatcggccatcgctttgcgagcggcgtgctcgcggcctggggcttcgtgcgcaagggaaagaccgtccgcatcacgccgagcgggccgctggtggcgtcgatgatcgatctcgaattgcatgcggccgaatcgggccttgggctcatctacaccttcgacgagtacctgcgcccgtcgctcgacaggggcacgctggtaccggtgctcgaagactggtggcagagcttctcaggcccgtttctctattacccgagccgcacgcacatgccggcgccgctgcgggcttttgtcgactttctcaagaacgaggcgaaacactgaggcgcaggcacctcaaccagcccacgggagggagaggagaaagtcagaaggcctcggtattgctccttccccttctgggggaaggctgggatgggggcggctcccgtattcagcgacggccctgttttgaacgccgtcgtgcccccacccctcccctcccccgggaggggagggagaaagtcagaaggctctgggtattgctttcacgcgtcgtcgtcggcgtcgttgcccgtgagggacagcacttgttcgacgaaggcctcgaacagcggcagcgcggcgggcaatccatcgaacgactccgcctcgccggcatcgaagaaatgcggcttgccggccggcagcgccacccattccccggcttcgaacagcagacccagatagccgtcttgcgtgggcaggtagacaagcgccgcgcggtcgagcacctgttgcccttgcggcgcggcttcgcggccccaggccacgccctgccgagccaggtgctcgttgatccagccgtcgcacacatgcgtgtctcgccaatttccttcggcgtcgaaaacagcgagcacgggcatgggcgtccttttgcttgagagttattgcaggaaactgggcttggcatagccctggaacttggtgtcgaccacggccttgaagtccttcgaatggtaggcctccacaatgtccttggcccaggcagtgttcttgtcggcgctcttcacggccaccacattgaggtagtggtcgggcgtcttctcgagcgccacggcctcgttgagcttcaggcctgacgagatcgcgaagttgccgttgacgatggcgtattcggtgtcgcccagcgagcgcggcagctgcgcggcttcaagtggaatgaacttgagcttcttcgggttctcggccacgtctttttcagaagcgcgcagcggatcgacgccgggcttgatggtgatgagcttgttctgctccagcagcaccagcgcgcgggccaggttgctcgggtcattgggcagcgtgaagcggtcgccctctttcacttcggccagcgtcttgcgcttggtcgagtacacgcccagcggcgcgatggggccttgcaccaattcggccaggtcgagcttctggtcggccgagaacttcttcaggtagacctgatgctggaaaaagttggcgtcgagcgagccctgcgcgagcgcgaggttgggctgcacgtagtcgttgaattcgaccagcttcaccttgtagcccttcttctccaggatgggcacgatgccggccttgagctggtcgatgttggagccggcggtgccgccgatgacgaggttcttcttggcttcttgcgcctgtgccagcgaaagcccgccgaacgacagggcaaccagagacagggcgaggacggagcggcgcagcagtgcggttttcatgagatcaaaaaaagaaagggaacaaaaattcaacgcttgtccagcctgcgcgccgtggtgttgcccacgaattgcaggatctgtaccagcaccacgagcagcgccacggtgagcaccatcacgtcggtctggaagcggtagtagccgtagcggatggccaggtcgccgatgccgccgccgcccaccacgccggcaatggccgagtaggagagaaagctcaccgccagcaccgtgagcgccagcaccaagcccgagcgcgcctcgaccaccagcacgcgccagacgatctgcagctccgacgcgcccatggcgtgcgccgcctcgatcacgccgcgcggcacttcgcgcaggcactggtcgaccagccgcgcaaagtacggaatggccgcgaacgacagcggcaccgcggccgccagcggcccgatggaggtgcccgcaatcacacgcgtgaacggcaccagcgccaccagcaggatgatgaaaggaaacgagcgcacggtgttcacgatccagttgagcaccaggaacgccggcttgttttcgagcgactggcccggccccaagaggaacagcagaatgcccagcggcccgccgatgagcaccgcggccgagaggccgatggccagcatcaggaaggtctggccggtggcggtccagagctcggggaggatgggcgcgatgttctcaaacataggccacctcctctgggctgcgctgcaacgacggcgggcgcggctcgatgggttcgcgcgcctcgcgttcgcggcgccgcaccagctcgtcgatctcgcggcccaatgccgtctttcgatcttcactcggcgcatcgaccgcgaactgctctaccagccggcccttctccaaaatggccacgttgcggcacagcacctcgaccaccgagagctcgtgcgtcacgatgacgatcgtcacgccgatcttctggttgatgtcgcgcagcgtttcgagcagcgcgcgcgtggtttcggtgtcgagcgccgaggtgggctcgtcgcacagcagcacctgcggccgcggcgccagcgcgcgcgcaatggccacgcgctgcttctggccgcccgagagctgcgccgggtaggtgtcgatcttctcggccaggcccaccagggcgaggcattcgcgcacccgcgcatcgatctcggcgcgggaatggcggccgtggatcttcagcgggaaagccacgttgtcgaacaccgtggcgttctgcagcaagttgaactgctggaagatcatgccgatgttctgccgcgtgtcgcgcagctcgcggcgcgagagcgtggtgaggtcgcgcccgccgacgaagaccttgcccgcatcgggccgctccagcaggttgatgaggcgcagcagcgtcgacttgcccgcgccgctcttgccgatcaggccgaacacgtcgccctggtggatgtcgagcgagagcgactgcacggcgtcgaacacctcgccgttgggcagggcaaatgatttctgcaccgattgaagacggatcacgggctctgcgttgccgcggcggcccgcgccggaggaaggattgctcataaaaaaggcagcggcgggcgtggagccgaccgcgaaggttcgcaaaaaggggccgagtatgaaaacaaaggcgccgaaaaggaacgaacaaatcgtcgcgtgcttattcgataaatcacataagaccgcgaacgcatggtcgagcgatgccatatcgatatgcgcattcgttcgttcccaagtgcgccgggcaatgccacattcgcgccttcatttttttgatttcgcgccacaacatgcacaccaatttccgccgccgcaccctcgcccttgcaacgctggccgctgccctttttgccggcagcggcgccgcgctcgcgcaagacaagaacaccgtcaaggtcggcgtctccgtcggcagcgccgagcaggtgttcgaagtggtgaagaaggtagccgcgaaagacggcctgaacatccagctggtggtgttcaacgactaccagctgcccaacgcggcgctggcctcgggcgacctggacgccaatgccttccagcaccagccctttctcgacaaccagaacaaggcgcgcggcttcgacatcgtgcccgtgggcctgaccatcaccgcgccgctgggcttctactcgcacaagatcaaggcgatcgagcagttgcccgacggcgcctcggtcggtatccagaacgacccgtcgaacggcaaccgcgcgctgctgctgctgcagtcggccggcctcatcaccttgaaacccgaggccgtgaagaacaacaccgccacgccgctcgacgtggtgagcaaccccaagaagctcaagctcgtgccgctcgacgccgcgcaactgccgcgctcgctcgacgacctggtcattgccgccatcaacaacgactacgccgagaaggccgggctttcgctcaacaaggacgcggtcatcaaggaatcggccaagagcccttatgccaacctgattgccgtgcgccgcgccgacaaggacaagccctgggccaagcgcctggtggcggcgtaccagtcggcggaggtgaagagcttcatcgagacgcagttcaagggctcgctggttccggcgttctgatcgcgcgacgttgacccttgccccctgcgcgcccgcgccgcgcgcaagggggcatttttcttttggtgccctgacgcagctacggtctcgcggcaaggaaccagaatccaaaccggaatctaggaccccatctaattcctataacccattgattaataatgattattccaataagctgagcagaatttcaaccggaattcatgcccctagagtccaagcctttgctggtctacgaccagcctcatcagttcgaaccgttgctgccaacgcaaaagctcggcgaactgagcgaagtcacgcgccggatattcgagaagtcagcacaactgaaaggctccgcgagtccgcaagcccgggcagcgctgcgtgagattgttcggtcgatgaactcgtactactcgaaccgcatcgagggacaaagcacgcatcccatgaacatcgagcgcgcgctcaggcaagacttttccgaccagccggatgttgccaagcgtcagcgtgtcgcgctggcgcacatcgaggccgagcggcaattggaagagattgtcggcaccgaagcgggtacgttgagcagcagcttcctcaaaaaggcgcatgaaagcctctacagccgactccccgaaccagatcgccgcaccgacgacggccggatcatcactccgggagcccttcgcacgcatgacgttgcggtgggccggcaccagccgccggcgtggcaatcgatcccgcaattcctgaagagaatggacgaggtctacagcagcctcaagggtgtcgatgcggtgttgtacaccgtcgcagccgcacatcaccgaatggcctggacgcatccatttgaagacggcaacgggcgcgcggtccggcttcagacccattgcgccttgcacttgatcagtggcggcctctggtctgtcaaccgcggcttggctcgccatcgagatcgttactacgaaatgctggacaacgcagacagcgcaaggcaaggagccctcgacggccgcggaaacctcagcgaaaaaatgctctgggagtggtgccgctactttctggaattgtgcgaagacaaggtcaatttcatggcctcgatgcttgacctgtcaaagctcaaagaccgtattcgcgcctatttgctggtacgcggttccacaagcggcatgacggaataccgcgaggaggcgctgctccccctgcatacgattgccgcggtcggcgcagtctcgcgcggcgaattcattcggatgacggggctggaagagcgcacggcccgaaaagtgatctcgcgattcatcaaggatggacttctgaagagcgacagccatcgctcggacctgaacatcggttttccgctcgagtcgctgagcatcctcttccccaacctgtaccccgaggcggcaacagcggttctggagtgagccacgccaaatacgggagccgcccccatcccagccttcccccaaagggggaaggagcaatacaggggccttcccaggcgggtcatcggtccatgagaaaatgtccggtttcccccgaacacagtcaggacaccccatggacgcagaacaaatcaaccaaatcggcgcaaccctcgcggacctgagcgcccggacggccgatttacggaggtatctttgactacgatgccaaatccgaacgtctgaggacggtcaacgcatcgctcgaagatcccaacgtctggaacgacccgaagaaggcccaggagctgggccgcgagaagaaatcgctcgacgacgtggtcgtgacgctcgaccgcctcaccagcggcctgtcagacaactccgagctgtacgagatgtcgaaggaagaaggcgacatggacggcttgcagtccattgccgatgacgccgccgcgctcgaagccgacatcaagcagctcgaattccgccggatgttcaacaacccggccgacccgctcaacgcctttgtcgacatccaggccggcgcgggcggcaccgaggcctgcgactgggccagcatgctgctgcgccagtacctgaagtacgccgagcgcaagggcttcaagacgcagatcgaagacgaaacaccgggcgacaccgccggcatcaagggcgcaaccatcaaggtggaaggcgactacgcctttggcctcttgcgcaccgaaaccggcgtgcaccgcctggtgcgcaagtcaccgttcgactcgtcgggcggccgccacaccagctttgcttcgatcttcgtgtatccggaaatcgacgactccatcgagatcgagatcaacccgtccgacgtgcgcaccgacaccttccgcgcatcgggcgcaggcggccagcacatcaacaagaccgactcggccgtgcgtttgacgcacatccccaccggcatcgtggtgcagtgccaggacggccgcagccagcacagcaaccgcgacgtggcgtggaagcgcctgcgttcgcgcctgtacgaccacgagatgcgcaagcgccaggaagagcagcaaaagctcgaagacagcaagaccgacgtgggctggggccaccagattcgaagctacgtgctggacaacagccgcatcaaggacctgcgcaccaacgtcgaagtctcggccacgcaaaaggtgctcgacggcgacctggacgtgttcatcgaagcctcgctgaagcaaggcgtgtaatcgatgagcctgacccacgacaaggtcgaagccttcatcttcgacatggacggcaccatgatcgattccatgccctggcatgcgcgctcgtgggtggaatttgtggcgcgccacgggctgaagctcgatgtgaccgacattcttgcgcgcaccacgggccgcaccggcaccgagtgcatgcgcgagctgttcgagcgcgagctttccgacgccgagtgccaaaccctggtgcacgagaaagaagaaatctaccgtgccctctttcacgacaacttcaccgaagtggccggcttcacagcctttgccaaggccgccgtggtgcgcggcctgaaggtggccgtgggcacggcgggcgacaagcacaacatcgagtttgcgatgtcgcgcctgaagatggacccattgccgctggccattgtgggcggggacgaaggctttgccggcaagcccacgcccgagatttttctggaggctgcgcgccgcattggcgtggcgcccgagcgctgcatcgtgtttgaagatgcgcccttcggtatcgaggccgcacgccgcggcggcatgcgtgccgtggccgtgtgcagcacccattccgccgccgagcttgccggcccccatgtgattgccgcggttcgcgactacgacgaactcgcccattcgaactttctggagacactcgatgctgctgcagcgtgacgcccaagggcaaccgattgccattcgccgcgaagactatgccgctccggccttctggatcgacaccgtcgacctgaccttcgacctggaccccgccaagacccgcgtgctcaaccgcatgcaactgcgccgcaaccccgacgcgccggcccagcccctgcgcctggacggcgacgagctgaacctggcgcgcgtgctggtcaacggccagggcgcatccttccgcatggaaggcgaccagctcgtgatcgacgggttgcccgatgccttcgagctggagatcttcaccacctgctgccccatcaagaacaccaagctgatgggcctgttcgtgagcgaagacaccttcttcacgcagtgcgaggccgaaggcttccgccgcatcacgtattttctcgaccgtccggacgtgatggcgatgtacaccgtgaccctgcgcgccaacaaggccgcctacccggtgctgctgtcgaacggcaacctggtcgagcaaggcgagctgcccgaaggccgccactttgccaagtgggtcgaccccttcaggaagccctgctacctgttcgcgctggtggccggcaagctggtggcgcgcgagcagcgcattaccgcgcgcaacggcaaggagcatttgctgcaggtgtacgtgcgcgcgggcgacctcgacaagaccgagcatgcgatgaactcgctggtcaactccgtgctgtgggacgaagtgcgctttggcctgccgctggacctggaccgcttcatgattgttgccaccagcgacttcaacatgggcgccatggagaacaagggcctgaacatcttcaacacgaagtacgttctggccaaccaggccaccgccaccgacgccgactacagcaacatcgaaagcgtggtcggccatgaatactttcacaactggagcggcgaccgcgtgacctgccgcgactggttccagctctcgctgaaagaaggcctcaccgtcttccgcgaccaggagttcagccaggacctttgcgccgatgcctcggcccgcgccgtgaagcgcatcgaagacgtgcgcgtgctgcgcaccgcccagttccctgaagacgcgggccccatggcccacccggtgcggcccgacagctacatcgagatcagcaacttctacaccgtcaccatctatgaaaagggtgccgaggtagtgcgcatgatgcagacgctggtcggccgcaagggctttgaaaagggcattaccctttacttcgaacgccacgacggccaggccgtgacctgcgacgattttgcgcaggccattgcagacgccaaccccgattcggaactggcccgcctgctgccgcagttcaagcgctggtacagccaggccggcacgccgcgccttgccgcccacggcgtgtacgacgcgcagaaccgcagctacaccctgagcattgtgcaaagctgcccgcccacccccggccagccgaccaaggaacccttcgtcattccgctgaacatgggcctgctcgacgccagcgggcgcgaactgccgatgcagatcgagggcgaagagcagatcacgcacggcacccgcacgctggtgctctcgcgcgccggcgagcagatcacctttgtgggcctggacgccgagcccgtgccttccatcttgcgcggcttcagcgcgccggtgattcttgactttgaatacaccgacgcccagctgctcaccctgctggccaacgaccccgacccgttcaaccgctgggaagccggccagcgcctgggcctgcgcgccgcgctgcagggcattgcggcgcttgcaaccgacaccaccccggtgctgaacgacgcctaccttgacgccatgcgcagcgtgctgcgcaaccccaagctcgacgccgccttcaaggagctggtgctcacgctgccttcggaaacctacattgccgagcagctcgacgtggtggacccgcagcgcgtgcacctggtgcgcgatgccatgcgcgcccagctggccaccgccctcttctccgactggcaacaggtctacgaagaaaaccacgacaccggcgcctacacgcccgaccccacctcgtcgggccgccgcgcgctggcgggcatggcgctcaacttcttgtgcctggcggggcgctcatcgggcgacaccgtgtggcccggcaagacgctgcagcgcttcaaggacgccggcaacatgaccgaccgcttcaacgcgctcaacgcgctggtgtcgtcgggccacaccctggccgcacaggcgctcgcgcgcttccacgccatcttcaaggatgaagcgctggtcatcgacaagtggttctcgctgcaggcgggcgcgcccgaccgcggcggcgacatcttgccgctggtgaagcagctgatgaagcaccccgacttctccatcaagaaccccaaccgcgcccgcagcgtgatcttcagctattgcagcgcgaaccccggcgcgtttcaccgccccgacgccgccggctacgtgttctggagcgagcgcgtcatagagctggacgccatcaacccccaggtggccgcccgccttgcccgcgcgctcgaccgctggagcaagctggccgagccctaccgcagcgccgcgcgcgaagccattgcccgcgtggccgccaagcccgacctgagcaaggacacccacgaagtcgttacccgcgccctggccggtaactaaccaaggaacatacaaagcacatggctcaacaacaaaagatctccctcacccgctacctcgtcgaacagcagcgcgccgacggcctcattcccggccagctgcgcctcttgctcgaggtcgtggcccgcgcctgcaagagcatcagccaggccgtcaacaagggcgcgctgggcggcgtgctcggcaccgccgaaagcgagaacgtgcagggcgagatccagaagaagctggacatcatcgccaacgaagtgctgattgaggccaacgaatggggcggccacctcgcggccatggccagcgaggaaatggacagcatctacgtggtgcccaaccgctacccgcagggcgaatacctgctcatgttcgacccgctagacggcagcagcaacatcgacgtgaacgtgagcattggcaccatcttcagcgtgctgaagaagcccgacgacacccccggcgtgcaggaagccgactttctgcagcccggcacccagcaagtggccgccggctactgcatctacggcccgcagaccaccctggtgctcaccgtgggcaacggcgtggccatgttcacgctcgaccgcgagcaaggcagctttgtgctcacgcaggaagacatccagattccggccgacaccaaagaatttgccatcaacatgagcaacatgcgccactgggacgagcccatgacgcgctacatcgaagaatgcctggccggcaaggacggcccgcgcggcaaggacttcaacatgcgctggattgccagcatggtggccgacgtgcaccgcatcctgatgcgcggcggcgtcttcatgtacccgtgggacaagcgcgagcccgaaaaggccggcaagctgcgcctgatgtacgaggccaaccccatgagctggctcgtcgagcaggccggcggcgccgccaccaacggcaagcagcgcatcctcgacctgcagcccaccaaactgcatgagcgagtgagcgtgatgttgggttcgcgtaacgaagtcgagcgtttgacccagtaccacgccgaaaaggcctgaaggtcttgctataatcgcgggcttagccggtgtagctcagtcggtagagcagctcattcgtaatgagaaggtcgggtgttcgattcatctctccggcaccagaattaagcggtaaaacgcgatagcgatcactaacctctagcgaggtactagcaagatcaccagagagcgaattttcgctttcttcaaagcctcccttgcggaggctttttctttgcagttgaagaagtcgtacttctgaatcgcctcggctttcgtagaggccgatggattcaagtcaagccgctgccgtggcggtctgatcggcgaattgccatggttacactccgccgatggacgctctcaccttcatcgccgagcttgttaaagctcttgcttggcccgctgttgtggtgttcatcgtcatcttcttcaaggaaagactgaccgccctcgtcgacaagctcgaagaatggaagggtcttggcatggaggcgaagttcaaccgcaagctcgaaacagtcgctgctgagacgaaagagattgcagttgaagaactgatcgcacctactcctgaacttcccgtgctccccaacgttgaacaagcagacgatccgttcaccacgttggacgagcagccgatagtgaacgccctcctgctttatgggaacccaagcgcaggattcagcctcggtcgttcatacctcgaacgcatcttgaacgaacagttcgtcaaagccactgggcaagtcccgggcctaatcatgccgttggacgcggtgatcgagcggctggagaaggagcgctacatcactgcacgcatgaggcgaaccattaaggagttgttggcgcttggcaatgaagctgtgcacgagaagttcaagccgagtgttgagagcgcccgcgcgtacgtcacctcagtccaatcgatagccgacttgatgaggctcagagcgaagcgcttctgatccgttcactactaccggttgccgatgctcaggccttgacctgcttggtcttcgttcggccatgcactggtcgcggcaccttgtaatccggatcaaccgccctaagtgcctcaggcatcttctcggcaatagcaatcaacgtcttcgctgcgccggtcggttcgcggcggccttgctcccactgctgcagcgtacgcactgacacgccgagcagttcggcaaagcctgcttgcgacagacccgcattctcccgcgcggcaacaaccggcgtgtagaccttgcgcgtctttccggcgcccatttcgcgtgccgactgcacaagcaaagcctcgaagtcctggctcgcttcgaaggcggccagttcggcatcactcattggctttttctgcggcattacgcaactccttcagggtttcgccagagatcgaatcgaggttcgctttggcgtagatcaacaacaagacgagctcaccgggcttcttgcggttgaagtacacaactcgcacgccgccactcttgcccgaaccggcccggctccagcgcacctttcgcaccccgcccgacttctggaccggatctccggcatcagggttcgcggagatgtaggccgcaaactcgcctcgctcttcctctgtccaatagttcggccatagcttttggaagattggggtttcagcgacggtgagcatgctcgacagagtacgccattggcgtacattctacgcctacgacatcgtgatcatcgtcacggattcggcttaagaatttgcaacggccggccggttgctgatcgtccccaatgctggccaaggccggtcgcgaacgcctcatcaaggcgttgggccgagaaagcccgcccgttgcgcatctgaaacaaaagaactacaccttgtatgccaatgtggcggtaatccaccataggtagttctccgaaacagaagaccacaaagcgcacgcgccaagtcgccgcggaaagcgcatcatctccatggacgaacccccgtttcaagactgtgcgaggcagcatgacaaggttcaaaaaggtcttctggattggcggcgggctcgccgtgctgggtgcgcttgccgcgtacgcggtgatccacgagctgaagacttcccgatggcaatcggcgctgtggcgcgactttgccaagggtgcgggctacaccgtcgaggcgggtgccagcgatgccgtccgctttccccagaccgggccgtatgacgagcggatgggctaccacgatctgcccgccttcatccagcgcctgcagcccgagggctacgtcatcacccgccaggcgcgcatgtcgccgcggctgctcgagcttcaggagcacgggctttttatcccgtaccgcgagaaaaaccaggccggcctgacggtgcgcgactgccgcaatacgacgctgctgcacacgcgggtgcccagccgtgcgtacgagcgcttcgaagaggtgccgccgctgctggtcagcgccttgctgttcgtggaagaccgccacctgctcgacgcggagccggcgcagcgcaaccccgccatcgacccggaacgctttgccaaggccgcggccgagcaggcgctgcgggtgctcagccccagccggtcggcgacgggtggcagcacgctggccacccagatcgagaagtaccgccattcgccgcacggccgcaccgtgtcggtccgcgaaaagctgcgccagatggcgtcggcctcggtgcgtgcctaccaggacggcgaggacacgctggcccggcgccgccagatcgtggtcgactacctcgacaccgtgccgctggccgcgcgcccgggcatgggcgaggtgcacggcctgggcgacgggctgtggacctggtacggacgcgatttcagcgaggtgaaccgcctgctggtcgacaacgccgaaggggccgcgcccacgcccgaggcgctccagcgccaggccgaggccttcaagcaggccctgtcgctgatgattgcgcagcgccgcccgtcgcagcatctgctgggcgacggcacgggcctgtcgcggctgaccgacagctaccttcgtctgatggccgaggcgggcttgatttctccggtgctgcgcgatgcggcgctggccgtgcccttgcacctgcggcctccactgccggccacgccccggcccgactttgtgcagcgcaaggccgcgaccgcgctgcgcacccacatctccaccctgctcaacgtgccgcgcgcgtatgacctggagcgcctcgacatggaggccgaaaccagcctcgacagccaggcgcaggcactcgcggcgcgggtgctcaccagcctgcaggcgcccgccgcggccaagtcggcggggttgtacgggcaccacctgctcgacccgggtgccgaccctgctccgctgatctacagcttcacgctgttcgagcgcggcgcgcaggccaacctgctgcgcgttcaggccgacaacatcgaccagccctttgacgtgaaccagggcgcgcggctggaccttggctccaccgccaagctgcgcacgctggtgagctacctggagctggttgccgagttgcacggccgctggggcgagctgagcccggcccaactgtcggctctgaaaaccagcccgcgcgacccgctgggcgcatgggcgcggcaatacctgcagcgcaccaaggatcgccgtctcacgcccatgctcgaggcggccatggagcgcaagtattcggccaacccgggcgaggccttcttcaccggcggcggcctgcaccagttcgagaatttcgagcgctcgcgcaacaacgaattcatgacggtgcgcgaaggtttcaagcactcgatcaacctggtgttcattcgcttgatgcgcgacctggtgcggcaccgcatgttcggcggcgcgtcggatgccgagagcatgctgcaagacccttccgatccgcgccggcgcgagctgctggcgcgctttgccgaccgcgaaggctcggcctacctgatccgcttctatcgcaagtaccagcgcctgcagcctgccgacgccgaggcgcggctgctgcgcagtctccggccgtcggcgccgcgcatcgccagcgcgctgttcaccatcgaccccgatgccagcgatgcacggctcgaagagctgctcgtgcagcgcacgggccgcggcgccgcatcgcctcgcgcattgcgggcaatgcgcaccacttactccggcttgtcgcttgccgatcgcggctacgtggcgcgtgtgcatccgctcgaactgtggctcgtcggctatttgaagagccaccccggagccacgttgaccgacgtgctggacgccagcgcgagcgaacgccaggaggtgtacgcctggctcttcaagacgcgccacaagagcgcgcaggacaagcgcttgcgcgagctggtcgagatcgacgccttcgccgaaatccatcgctcgtggcagcggctgggctacccgttcgaatcgctgacgccttcgtacgccagcgccatcggcgcctcgggtgaccggccgcgcgccctggccgagctgatgggcatcatcgccaacgacggcgtacggcggccgacgcaacgtgtcggcgccctgcactttgcgcgcgaaacgccttatgaaacgcgccttgagcaacgcaacgcgagcgcagaaagggtgctgccgagcgaggtggccgcatcggtgcggcgcgcgctcttcgaggtggtgcaggacggcacggcgcggcgcctgaagggctctctggtggatgcgaacggccgcatcatcgaaattggcggcaagaccggcacgggcgaccaccgcaacggccacggcagcggtcgggcggagcgcaagatcagccgctcggccactttcgtcttcatgatcggcgatcgctacttcggcaccgtcatggcctacgtcaacgaaccctatgccgcgcgctaccgcttcaccagcgcgctgccgactcagctgctcaaatcgcttggcccacagctgttgccggtgctcgagcgcagcggttgcagtggcgattgattgattgatcgattgattggttgatgcaaatccgcgaactcgccaccggcctgcagtttcccgaagggcccgttgccatggacgacggctccgtgctgctggtcgagattgcccgcggcacgctcacgcgcgtgcggcacgacagcctggtgcaggtggtggccgacctgggcggcgggccgaacggcgcggccctggggcccgatggcgcggtctacgtgtgcaacaacggcggctttcgctggcacaccgaggccgacggctgccaccggccggtgggccaggccgatgactattcgggcgggcgcatcgagcgcgtgaacctggccacgggcggcgccgagcggctctacgacgcagccgacggcggcgcgctgtgcgggcccaacgacatcgtgttcgacgcgcaaggcggcttctacttcaccgacctgggcaagacgcgcgaacgcgacatggaccgcggcggcgtgttctatggccacagcgacggcagcggcgcgcatgccattgcgcggccggtgacgacgcccaacggcatcgcgctgtcgcccgacggctgcacgctctactacgcagaaaccgaaggcgcgcggctctgggccttcgacatcacggcaccggggcgcgtgcgcaaggagggctggccttcaccgcacggcggccgcatgctgtgcgcatcgccgggcgggcactaccagcgcttcgactcgatggcggccgatgcgctgggcaacctgtgcgtggccacgctgctgcacggcggcatcaccatcgtcgcgcccgacggcagcacctgcgagcacgtgccgctgcccgaccgctacaccaccaacatctgctttggcgggcgcgacatgcgcacggcctacatcacgctgtcgggcagcggacggctgattgccatcgacgattggcctacaccggggcttcggttgaacttccaggcctgaagccgcacgcgggctcacaccacacccttcttcgcactccccgtcagcgacgcgaccgaaggcacgatccattgccggtcattgagcacctgccggatgcgctcgcgcaaccattgatgcgccggatcggcgcggtggcgcgggtgccaggccatgcgcaggggttcggactgcaccgcaaccggcaactcgaaaaccgccaggccgagcgaagcggccatgccccgtgcggtgcgttcgggaacactggccaccagatcggtacgcgaggcggcgatcagcgccgagaaggtgctcggcacaagcaacgccacctggcgctgcaagcccaactgggccagggccgtgtccaccggcgaaggctcgccttggcgcggcgtgacgccgacgtggcgcgcggctgcataccgctctgccgtcatgggcgttttcttcaagcccttctgcagcggatgcccggcgtgtaccgcgcccaccagtgtttgctccgacagcacctgggtttcggtttcgggatcggtgcctcgaaagctccccacatccaggtcgatacgcccttcgcgcaatgcgccggggtccgcatgggtttcggggagaaactggagcgaggccagcggcatctcggcctccagcgcctgcgacaggctggccccgaacaccaccgcaatgccttcgggcgcccgcacgacgaagcgacgtcgcaggccaaccaggctttccgcgcctgcaggtgcgcgcaatgcctgcgcctgtgcgagcaaggcgcgcacaggctcggccaacgccagggcgcgcggcgtcggcacgagcttgcggccggcccgcacgaggatcgggtcgccaaacgactcgcggatgcgcgccagggtgtggctcatggcgggcgtgctcaggttcattcgcgcggcagccgccgtcacgctgccggtggacagcaacgcatcgagcgcggtcaacaggttgaggtcgtatgtgttcgccatacgaaatcatatgttcaatacattgcactgtacaaaatcattgccgcttccgacactggcgccccttgccttgatcgaaacggttccatgaaagcttcacgtacgtcttcgccccttctgccattcgccatgctcgtgctgacgctgatcctcgcggcgctcgaccagaccatcctgtccaccgcgctgcccgtcatttctcgcgagctcaagggaggctggccgctggcatgggtgttctcggcctatctgctggccgcgacggtggtcattgcgctgtacgggcgcctggcggatgtgctgggcaagaagccgatgctgctgttggccatcggcttgttcctggccggttcactggcttgcggggcgagccaggatgtacagcaactggtgcttgcgcgcgccctgcaaggcgcaggcggcggaggcctcatgacgctcaccatgctgatggttcccgacctgttcgggcccgaccagcgcggtcgctaccaggcgctgctcggcgcggcatacggggtctcgaccatgttcggcccgctgctgggtggcgcgctggtggagcacctgtcgtggcattgggctttctggatgaacgtgccgccggccgcgctggcctggggcgtgctggcatcgaccctgccatcgaagccgatggcggcccaagcaccggctgcggagggacaacagcgcatgcgcatcgactggctcggcgcggtgcttctcacggctgctcttgtcttgttgttgctcgccacccagcatggcaatctgaacctgcccgagcgcgtttcgctttggcttctgttggggctgggggccaagttcacgctggctttcatctggcggcaacatcgcgccgcgcaccccttgctgccgctgtcgctgttcgcccgcccggcctatgcggcggtcagcttcatcgggatggccagcggcgttgcgctctacgccgccgtggtgttcctgccgcagtatctgcagatcggcctgcacctgtcgcccaccggttctgcctggcacttgctgcccttgatggcaggcatcaccgtggcggccgtgaccagcggcaagctgctgcgtgcgcagaggcccgccgtctcggtggcgcgtgtggcctgcgtgctgatgttgctgtccttcggcctgatggtgggcgcgctgcgctggcttcccggtgaagccctggcgctgtcggccgcgctgctgcccctgggactcgggctcgggctgctctttcccatcgtcacggtggtggcgcagcgcgtgtcgccggcgcagcacatgggcattgccacggcggcacccatcatgctgcgcagccttggcggcgcggcgggcgtggcactgctggccgcgctgctcacgcacctggtcaagcaggagcttgccacggtgggcgccctggcacagggtggagcggcggacgccgtcacgacggcgctggggcacggcctgcaatccgtgttcggctgcgctgcggcggccgcgcttcttgcgctggtcgcttcgaactggctggtgcagacacggcctcacgaagggcttgcgaagaacgtcgttctcgaacctacatcgtgaagcgcgtgtgccgcgcaatcaccgcctcttcatcagtcttgaacacccaggcgctgacacggctctgcggcgtggtcagccgcagggcgcccgcagaattggcccgcgcatcgacatcgataccgagccagccgcactcttcgagaatgcgcttgcgaagcgcggcggcgttctcgccgatgccgccggtgaacacgatggcatcgacaccgcgcagcgccgcagcaaggctgcccatgtgctgcaccgcctgctcaacaaaatgcgtgatggcttccgcggcagcgggcagcttcgaggcttcgagttcgcgcatgtcgctggacacgcctgaaagccccagcagccctgattcgcggaacagcagcttctcgaccgcgtcggccgacatgcctcgcgagcgcatcaggtacagcacgacggccgcgtcgagccggccgcagcgcgtgcccatggtgaggccgtcgagcggagaaaagctcatcgtcgtcgcgaccgaacggccctgcgccatggcgcacatcgaagccccgttgcccaggtgcgcgacgatcacgcgttgccgcgcgagctgcggcgcgagttgcgcgaactgcgccacgatcgattcgtaggacaggccatgaaagccgtagcgccgcacgcccgcgtcgtgcagcgcgcgcggcagcgcaaagcggcggttcacgtcgggctgcgccgcatgaaaggcagtgtcgaagcaaagcacctgcggcacgccgccaaaggcgtgcatcgccgcgcgcacgcctgcaaggttgtgcggctggtgcaagggcgcgaggggctcgagcgttgccagttcgttcaataccgcttcatcgacgcgcacgggctcgacgaagttcacgccgccatgcacgatgcggtgcccgaccgcggcaatgcgcgccccgtcgccctgccgcacatgccagtcgagcagcgcggccagggcgccctggtgcgaccgctggtcaccttccagcgcggcgtcgtgcagcgtgcggccttctgcgtcgcgcacgcgcaaccgtgccttgagccccgcgcccagaccatcggcctcgcccgaccatcgggcggcgggcagcgcgccgccgttgtcgccgctgctcgcatcgaacagcgccaccttgatcgacgacgacccggcgttcagcgtgagcagcagcagcgaatcggccatggcctactttaatccgcaccggcgcggacgcggtctttatagccccagggcagcggtcctttccgggaaactggaacaatgcagacaccatggacggcctcgatctcatcaaaacattccgcgaagtggcgttccggcgcagcttctcccgcgcagccatctcgctcggcatgtcgaaagccaccgtcagccgctacgtggccgagctggaagagcgcagcggcgtgcgcctgctcaaccgctccacgcgttcgctgagcctgacggatgccggccaggtgctgctcgaccgcagcgccgagctggtaaacatggcggaggccacgctgaacgacctgcaggcccatgcctcgcacccgcgcgggcggctgcgcatgagcgcgccgcacgggctcattgccggctggctgtccgacgtgatcgccgaattcatcaagctctatcccgacgtgtacgtgagcctggtgttcaccaacagcgagatcgacctgatcgaggaaggcatcgacattcacctgacgggcgggcgcatcgacgacatgaacctgatcgtgcgccggctggtgccgttcgacatggtggtctgcgcaagccccacctactgggcccggcgcggcattccccgggtgcccgaagacctggcccgccacgacgtgctgagctattcggccaagcccaccacccacctgcccttcgagaccgacggcaaggccgtcgacgtgccggtgcacagccgcatggaggccaacgacgcggttgcgctcatcgagctggcgctgcgcggcgcgggcgtggcttatgtgccggagccgctggcgcagtcgcacctggagcgcggcgcgctggtgccggtgctgcgcgagcacatgccgcacgaccactggctgtatgcggcctactcgcagcgccgccacaacagcgcggccatgcgcacgatgctcgactttctcgagcagtcgatgggcccggccaacgagccgccggtgttcccgccgatgccacgcgtggaagcggcggcatgcgccctgtccagggcaccaacaagcgccgctccggcggccaccccaccggccaccgcaccagccaccgcgccgacagatcgaacggacaggctggtgcgccagtcatgacgattgcccatggcggggccgtgtcgtgttgcaattgcacgctttccaacgtgcacgcaaccgacgcatgacgacctcttcttctgcttctctcctgattcgccctccgacgcgagacgactacgcggcatggaagccgctgtgggacggctacaacgccttctacaagcgcgaaggtcccaccgcgctgcccgacgagatcacccaggtcacctggcagcgcttcttcgatccctacgaaccggtgcatgcgctggtggccgagcgcgacggccagctggtgggcctgacgcactacctctttcatcgaagcacgacgcgcatcgagccgaactgctacctgcaggatctgttcacgctgccttcggagcggggccagggcgtggggcgccagttgatcgagggtgtgtgcgcgcacgtgaagggcgtgggcgcgcaccgcctgtactggcagacgcacgtgaccaacgcggccgggcgcaggctctacgacaaggttgccagccacgacggattcatcgtgtacggcaccttcgtctgagcggcgcggctctcagtacttgatggtcacaccggccttcacgccgttgttgttcttgccatctgacagcacgccgcccgtgagcgacacgttgccgcccgtgctcgcgcccagcgagtaggtgggccggggcgtggtggtgtcggtgcctatataggtgccgctgccgtcgggccgctgcacgccgactgtggcgcccttggtgtaggccgaggtttcggtggagttgacgttgggcgccacgtagatggtgcccttctcgtcgctgtcgaggggcaccttcacgggttcggccattgcagcggcggcggcccaccacgcggccacgccgaggcaggcaaggatcagtttgctcatcccccaatcctaggggctgcgcgcgccggagccagtaggacacaggcgatttgtcacgcctcgttgcaatagcggcggggcgcttgtctcgcccgggaaggggcgcaccgctcatgtgcgcgggctgcgcaatttctacagtgactccatcggcgaagtgcctgggcccaatgcagggaccgagcggcgccggtcggccaccgtcactgggagacacgcatggaaccgctcaacctgcagccacgaaacctgacgaacctgctgcatgacgaggcgggcatgtcgttcatggagttcgctctgcttgcttcgcttgtggtggtcgtttgtttgctcctgctgcttgcagcacggcgcgcggcctgaaggcgtaacagatcggcaaaggtgaaaccatgaacagaatcttccggacgctctggaatccctcacgtggcgcctgggtggctgcacccgaaatttcgcgcggccacgcacgctcggccagcaccggcaccggccagcgcacggccgcgctggtcagcctgcatgccattgccatcgcggtgctctacctgagtgcctcggcggcactggccgccggcggcgcgggcggccagcccgtcagcaccgcactgcatggcggggccggcggcagcgacggcggtggcggcgccggcgccctcaacgacgtcaatctgggcgcgcgcgggggcaacggcggatcgtcgaccgacgccggcgtggcggcgggttccgccgccgacatcggctccttcgctggggccaccgcgggcgcgggtggtgcggcgggagcctcgccgggcgccgacggcgccgcgggcgcatcgcataccggcggcttcggcgccggcaacggatatggcggcggaggcggcggcgggtactacggcctggcgatgagttccagcaccaccgccaccttcgggagcttcacgggaggccgcggcggcgcgggcggcaatgggttctgggcagccggcggcggcggcgccggaggctatggttccatgctggtcggccctctgggcgactaccacgccttcggcaactccacgggcggcgcgggcggcaagggtggcgacgcgtattcgcaaggcggtggcggcggcagcggaggcagcgggttcttcatgcggtcgacgacgccgggattcaccttcggcaacagcggcaacatcaccggtggcgtcggcggagccggcggctccgagctgctgccggcacgcttcaacgccgcgggcggcggcggcggtgccggcgggcacggggtcacgctggctggcagcaccgtgaccgtcgacaactccggccagatcaccggcggcgccggtggcgcgggcggtgccggcggcggaggtgcgggcggcaccggcgcgcccggcggcggcggagacggtggcatcgggctccggtccaccggggccggcgcaacgctcatcaacggcggcaccattgccggtggaaccggcggcatcggcggggccaacagcaacggcggcgccagcggtgccaacggcgccggtggtgagggcgtgatgggtgccaacctggccatcaccaacaacggcaccattgcgggcggcctgggcggcaacggcgtcacgcgtgcttcggccgtgaagttcaccggcggcagcagcagcctgaccgtgaacgcgagctcgacgctcgtgggcgccatcaccatcgacagtggggccaccgccagcatcatcgctggagccgatggcctgagcctggccaatgccttgcggctggacggcacgggcactatcgacaccaacggccacggcatgggctggtcgggcccgatctcgggccgcggtggcctggtgaaagacggcacgggcaccctgaccctcagcggagccaacacgtacaggggcgccaccaacgtcgccgagggcaccttgcgcgccggcgtggccaataccttcagccgcgccagcgcctacacggtcgccccgggcgccacgctcgacctggccggccacaaccagaccatcgcatcgatggccaacggcggcaccgtctcgctgctgagcagcgcgcccggcgccaccctcacggtgcaaggcccctgggtgggcaacggcggcacgctgcgtctgggcacggcccttggcacgagcagcagcttgagcgaccggttgatcctcagcggctgcacggccattgccagcggctcgaccttcattcaggtcaccaacctgggcggcctgggtgcgctgaccaccggcagcggcatcgaggtggtgactgcgatcaacggggcgacgaccaccgctcagaccacccgcagcgccttcaccctcacgggcggccatgtggacgccggtgcctacgagtaccgcctgcacgccgccaacgccgctggcgcgggcgagaactggtatctgcgctccggcatcatcgtcgcgcctcctccgccgccaccaccgccacctcccccaccaccggccccgccggcgcccccagcgccacctgccccacctgcacctccggcaccacccgcgccccccgcgccaccgccgacggaaggcgacccgctgagcgacgacggcggctcgccatcgaccgcaggaggcgtgacagtgcccacctaccgcgtcgaagtgccgctgtatgccgcactgcccgagcagttccgccaggccaacctggccatggtgggcaacctgcatcagcgagtcggcgacgatacggccggcgccatcaccgcaacaaacggccaaggctaccggcaggcctgggcccgcatcatccgcatggaccgcaccatcggccaagccggcaccgtgagcccgcgcagcgaagggcgtctcacgggcttccaggccggcgccgacctgtgggccaaccccagttggcacgtgggcctctacgtgggtgagctcgaaggccacatggacgtgaacggcttcgcgcgcggcctgccgaactacgcggtcggctccaacgagctgcgaagccagtacctcggcgcctacgccacctggaagaacgacagcggcctgtacctggacggcgtgctgcaggccgggcgccaccgctacaccgcatcgaccgcgctgggctccgccggttcgggcaagggcgacagcctgctggcctccatcgaggtaggccagggcttccgcatcacgccggactggatcgtcgagccccagctgcagctggtgcaccagcgcgtgagcctggacgatgccagcatcgtcggcgccctggtgcagcaggacagccacagcggctggctggtgcgcgccggcgtccgcatcaagggcgagatgaccaccggcgccggcccgctccaaccctatgcgcggctgaacctctatcgcagcagcagcggcacggacgtcacccgcttcatcggtccggcgggcttcaccgacattgccacacgcaccggtggcaccagcaccgagctggccgcgggcgccacgctgcggctgacgccgggcatgagcctctacggggaggtgggcaagctgtgggcttcgggcggcggggcgcgcgtgaagagcgggctgaatgccagcgtgggcctgaaggtgcgctggtgaggcgcgcctccggctctggctctactaccttggctgcgaaatcacggctgccggcgcatcgggcatcgccagggggttgagccccggcgccccgacacgcgtcagcgtgttgcggtcggtgtgatggaacggctcggcctgtccctggatctgcatcaccgtgtcctggtcgtacgaccaggtgccgtcggcattgatggtcacggtgatgttccacgccagcgtggtgaaggcgtgctcgatgaaggggttggacacgatgccgttcaccaggctgccgcgctcggcgctgaggctaaagcgcgtgtccccggccttggcatggccgctggccatggccacctgtccgcgcggaatggccagcgtgtgcagcacggtctcggtggcgggctcccagagccagtagcccacctggtcgtggtacatcttggtgaggccgggcttgtggatgtaggtgtggtagcgcaagccatacagcagctgggggccgttggtctgcggatcgatcggctgcagctcgtagcgctcgacgtagacctgcgtcttcgggccttcgcgcttgggcttgacgtccaccccgcggctgccctcccagataccggccatggcgcgcagcgggccgaggttggcgagcgtgtcgggatcggcgttgggctcggtgtagatgtcttcggtcgggttcatgtgggctgtcgatcgtggtgatggtttttgattctgcttgagggtggttgcaaggaccgcaccgcgccgcgcgcaggcccgaatgcgccgtagcgcacgcgctggccgctcaaggcttcgactctttcgatccatgcctcgggggtggcgatgccgccaggctcgtaaagcggctgcgcgccttgcagcaactgcgtcaaccggtgctgctgctcgaggtccgtcgcgtcgtcggccaatggcagcgacgcgaggctggcgccgtcggcagtgcgatagctcgcgcaccagcgcaggcccgcgccctccaccgcatcgagatggcttgccaccagcccatgcagcggaccggccgccgcgagcgcatagcgcagcagcatcgcatcgggatggccgcggcgaaacgcgccttgccagccttcgtcggcgttgtgcggttcggccagccgcgcgtcgagcgcgcggtcgtgcgtgggcagcggcccggggccgtggcgcgtgatgtagctgcgcagcacgcccaggtgctgcacgggcgcatcgatgccgacatcgcgcagcacggcttcgacggcggcggtggagatggtgctccaggtggtgtgcggatgaaagccgcgccactcgtcgagcagcacgccctgcgcgccttcgaacagcacggtgccggggcgcgccaggcgctggccgatggcgtcgacactcgcgggtggcgacaggcgcaagcacggcgccgccgcgtcgagccagcgctgcgcaagcgtcgcgtcgccgagcagggccagttcctgcgcggcctcggcatggggaggtgccgcttctgcaaactcgcgctgcagcgcgatgcgcagggcttcgagcttttcgagtgcccgtacggggtgccgcatgtcgccgtagtgcagggccgtgccgggcgcggccagcgcctgccgcaccgtttcgccgacgcccacgccgcagctgccatgcgccgccgctcccctcgcccattcgcgcaggcggcccgcggcctggtggaacggcgtggtgacgcggcagcgcgcatcgatcagcagccgcgcgaacgcgtcgttcacccccacgcggcgcagcgcttcttcctcgacgcgcagcgcggtcgggtgcaccaccatcgggctcgcgagcacggtcgccaccccggcgtgaaagctgccggcgccgaactgcgaaaaggtgtggtggcggccatcggacagcaccacgttgtggccggcctgcgcgccgccgttgaagcgcaccacggtgtgggcctgcagctcgccgcagaggtggtcggtgaagcggcccttgccgcagtcgccaaagcccaggccgagcagcgagacgtagcgcgtcggatgtgccggcgagctcacacgggcgtcaaccgaagagccgcttccaccacgaggaacgcggtgcagaggccacggtggcgggcggcgcgcgccgcggtgcctggggatcgagcagcgcggcatagccgtcgagcgcatgcagcacaccggcgacgcgctgcttctccatgccggtggcggccatcaccttggcaagcccgtcgagatgaggcacggccttctcggtgagcgccacgatgccggcagccaccgcgcaggcgtcgtcgggcgagtccatgcagatcacgtgatcgccgagcagttcgcgccagcgcggctcgcagcggcggcggcgctgcgcgtcgggaataaggaagaacaggtggcaggtttcggccgcggcagcaatgacttcctcgatcggaatgtcctcgtcgagcttttcgccgatgagtccctcgacctgtcggcgcgagacggcgggatacggcagctcgtcgccggtcacgaacaggtagccgcgcttcttgcgcttcacccagcagtccatgtcggtgtgctgcgccatcacgtagaaggccagctcgtagctttcttcgccgctgcccccgcccccgccttcgagataactccaggtcagccactggtccatgagcggcgcggtcgattcgaactggcccacctgcagcgaagcctggtcggaattcgcgtcgccgatggccatgaacatgagctgcggatcggccacgccgcaatcggtcaggagcttcatgaaggtgggcagctcgcggcgggcgaggatctgcgggatgtcgcccatcgagcccgtgacgtcgagcgcgaatgcaatgcccagcgagttggggtggtcggcgttgtcgcgcgactcgcgcaccttgagcccgtgcggattcatcagcgggtgcgtggcggtctgggtgaacacctcggagccgggcttggcggcgcggtcggcaatgagtgccgtgtgagcggcgtgcgagtagtttccgtagcccatgggtgcgtgctcctctgttttccgatggttgttttcaggcgccgggcgccgggtcgaaatgaacgaactgcggcgtgccgaaggcttcgcgcgatgcggcggacaacgcctgctcgatgccgcgcgcgcccagccgctggcattcggcggcgtcttcgctgcaccggcgcagcaaggcggcgaacggcgcgggcgtgcggtcgccaaaaccggggctgtcatcgggcttgccgccgtgcagcacggcgcgcacggtccaggcgctttgcatcaggtcgcgtgccgcggcggcggcatgggccggcccggatgcctgctgcgcccgcgaccagccgacgatcagcacgccatggtcgcgcggatgcacgagtgagtgcgcgggcgacaggtcgcgatgggtccagcccgcgtcgtgcacgaaggccagcacttcgagcatgcgacgccagagccacacggcatgccgcgcatcgatgccccgcgggttggcctgttgcacgttgtgcaggctgccccagaaaccgggcgggtggcgcagcaccagcgcctggcgggcaccgtctgcaagcccttcggccaggcccgtgcccaccggctgcggcaggcggcgcgtgaaatacgaagcgcccggcatggcgagcgactgcaagccctgcagcaccgcggcttcgcgcagcagcacggcgccgtccgcggattcgcgtgccagcttgaccgtgacgcgctccggcagcgcaccgagccgctcggccagcagcacttcgctgtgctcgccgatggccagcggtgccagcacgcggtagcgcgcgccgcgccattgcagcgtgcgcccggtgtcgccgtggtcggcattcgcccggcgcagcgctgcgcgaaaactctcgcgctcgaccgtttcctcgccacgcgtgatggtggcgccgcaatagttgcagttgacggtgcgccagcgcgcggcgcgcggcaacggcgccgagcattgcgggcagctgagggcgagcagtgagagcatggcgggcctagtcgttcctggacgccgtcttgtcgggcgcggccagcacccggtcgatgcggcgtccctcgagtgcggcgatctcgaaatgccagccggcgcagtcgatgacctcgccggtcccgggcaggtggcccgacacagccatcagcaagcccgcaacggtgttgtagcgcccgcgctcttcatcgggcagctcgcgaatgccgagccgcgcgcgcaattcggagacgggcatcagcccgtcgagctcccacacgccgtcgggccgctcgcgcgcccaggcgtcggtcagggtaccggcctgcagttcgccggtgatggcctcgagcatgtcgcgcggggtcatgaggccctgcaccacgccgtactcgtcgaccacgaacacgaggcggccgccacgctcgcggaactgctcgagcagctccatgccggtgagcgtctcgggcacgaacacggccggcgcggcctcctggccgagcacgccgtcatggccggtgcccaggcgcagcaggtgcgccacgctgatgacgcccaccacgtcgtccagcgaattgcggcacacggggtaccacgaatgcacgatgttgagcgcacccgcatccgccactttctgcagcgcctctgccacggtgtccgaggcgtcgagccattcgatgtcggcgcgcgggaccatcagcgacgacagccggcggtcgtccaggtggaacacgttgcgcaccatctggtgttcgtgctgctcgatcacgccggcatccacgccctcttcgaggctggccgaaatttcttcctcggtcatggagcgcgcggcattggcgtcgatgcgcagcagcttcagcaccgcggccgtggcgctcgcgagcagccacacgaagggcttggcgcctttggcgagcccccgcatcgggcgcgacacccagcgcgccaccggctccggatagagctggccgatgcgcttgggcaccagctcgccgaagatgatggtgaagaaggtgatgccggtcaccaccacggcggtggaagccacgctggccgtgccgcggcccatgcccaggtgctccatccacacggcgagcggcgccgcgaaggcggcctctcccacgataccgctgagcatgccgatcgaggtgatgccgatctgcacggtcgagaggaaatgggtgggctcctccatcagcttgagcgcggcttccgcgcccaagtctcctgtctcggccagcgctgccaggcgcgcgcgccggctggttgaaagggccatttcggacatcgcgaacaacgcgttgagcgtggtcagcaaggccagcaggagaacatccatgaacggggggtgaaaatgaggacatggcactttacttgatcggcgacatccagggctgcgacgccgccctccagcaactgctcgacaagatcggtttctcccccagccgcgacaccatcgtcctgctcggcgacctggtcaaccgcgggcccgactcggccgccgtgctgcgacgcgtgcagggcttcggcgcctcggcgctgagcctgctcggcaaccacgacctgcatcttctgggcgtggcgcacggtgcgcgcaagtccggccgcaaggacacgctggccggcctgctggaggcgcccgacagcgaagccatgctcgaatgggtgcgccagcagcacatggcgctgcacatgcagattggcggcggcgacctgctcatggtgcacgccggcgtgctgccgcagtggacggtgggcgacacgctggtgctggcggccgaggtcgaatcggtgctgcgcggcccggcgctgggcgagttcttgctcggcatgtacggcaacgagccggcgcagtggagcgacacgctcaccggcagcgcgcggctgcgcgccatcgtgaacgcgctgacgcgcatgcgcttctgcacggccgaaggggtgatggagttcgagagcaaggacggcatgcggcccggccccgaaggcttcatgccctggttcgacgtgcccggccgaaagaccgcgaaggccaccgtggccttcggccactggtccacgctgggctggctttcgcggcccgacctgctttccaccgatacgggctgcgtctggggcggctgcctcagcgcggtgcgcatcggcgccacgctggacgatcgcgaactgatccaggtgaagtgcgagcaggcgcaaaagcccggccagccgggctgaacggcttcaggtgcgcggcaggcggaagcggtccagccgaaggccgcgcgtgatcaatcaaccctgcgccacgacgccaaagcccgtatcgaaggtgcccttcacgtcgagcggttgcttgatgaggccgacctggcggtagaagtccgccgtgccctgctggtcggcaacgacctgcgcgtcgatgggcacccacttctgctggcggcgctcgaactgcagcttggccgcctcgggcggaatgccgatgatgcgcgcgagcgcggccgagtaggcgtcgacgttgcggtacgaccagagctgcgccttcaccacgcgctgcagaaaatcctgcagcaccggccgcttggcggcaatggccgcatcggtggccgcaaggtagctgagcccgggcagcagcccgcgcccgctgacgagcacgcgcgcgtggtggctgacctcggccagcgcggtgtacggctcccaggtggcccacgcgtcgaccgagccttgcgtgagcgcgagcttggcgtcggccggcgcaagaaagcggatgttcacctcctcgggcttgaggccggccgcggtgatggccttgagcgtgacgtaatggccgatggagccgcggttggtcgcgatgctcttgcccttgagatcggcggcggtcttgagcggtgagtcgggccgcaccagcactgccgtgccgtaggaatctgaacggttcgcgccgatggccttgacgcgcgtgccggcggccagcgcaaagatcagcggcgcatcgccgatgggaccggaatcgaccgccgctgcgttgagcgcctcggccagcggtgcggccgccggaaattcagaccactggatgtcgtagcccaggccttcgagtccgcctgccgcttcgagcagcgcgcgcagcccgcccttctggtcgccggccttgagcaccgggcggccctgtgcgcgggcctgcaatgagaaagcgggcaaggccaccgccgtggcggcggcaaggccgtgcgcgaggagctgccggcgcgagcggccgggttgcaatgggttcatgggttctccgtgttcggtcgaggaaagaaagaaaaaagaaagtcagtggatgaaaccgcccttgacgaagcgcacgggctcggcgtccatgcgcgcgatcagcgcgcccaggccgtcggccggtagagctgcgccgccctgctccgccgcgcgttcgctgctgcggcacagcaggtcgtcgtcggaccagccggccttgccaggctccgcgcgcgcgcgcagccagccgtcgcggtcggcaatcagctgcgtgccggccagcggatcggtgccggcgatcagcgccagcgcttcccatgcggcggccgaatcggccacgcaatctgcgcttgttgcaacagcgcccgaaggcggcagcaaccgcacggtcacgagcctcgggtcttcggttggcattgcatcgcccgccacgatgcgcacgcgctgtccgtgccaactcgcgagccggcgcggcggctgcgaaccgcagcgcaccgccatgtcgggcaggccgatgggctgcggccagctgccgagcgcgcgcaggctctggcccgcgcccagcgccttcatgtagtcgatcaaggcccaggcgtcggtctcgccgagcttttcgccgaagccgggcatggtgggttggccgccctgccgcgcatcgcgcgtgccatgaagaatgcgccagagcaagtcgccgtcggcacgtcgccagagcaaggggccattgaggttcggcggccacaccgccagcgaggccgcgagcggcccttcgcccttgccgtccgcgccgtggcaggccacgcagttctgttcgtagagcgcgcggcccctggcgatggaggcggccgtgaagccgctcggcgaggactggaaactcgtgggcgtcgcaggcaccagcaccacgtgcgactcgggccagggcgctgcgatcagcagcatcggcaccagcgcgagaaagtagaagcgcggacgccgccagaacagcgcgagcagcaacacgagcaccgccacggcgacgaacaccagcgtccacgccaggctgcgcgcctgccccaggtcgatcagcaggttctcgcccgacagccggcgcgcccacggccaggccggctggccatgcacgtgcgccgcgagcccgagcgcatcgagcacgcgcagcagctgcagttgggcgccctgaagcaggccgatcagcaggttgagccaatcggcctgcggcgtgctgttcatgtcaccacgtggcgtcgagccccaggtgccgcaacgcctcgtggcgaagctcggcgagccgcgcatggccgcgatgccgcgggtacggcaggtcaaccacgatctccgccgcgatgcgcgccggccggtcgctcagcacgatcacgcggttggcgaggaacagcgcctcttccacgtcgtgcgtgaccagcagtgccgagaagcccgcgcgctgccacaggttgaccagttcgctctgcatcgcgatgcgcgtgagcgaatcgagcttgccgagcggctcgtcgagcaccagcaactgcggatcgttgaccagtgcgcgcgccaatgccacgcgctgcgccatgccgccggagagctggtgcggaaaggcttttgcaaagtcggtgaggcccacgagcttgagggcctcgtcgacacgcccgcgctgcgccttgagcacgccgcgcgcctgcaggcccagcgccacgttgtcccacacgctgcgccacgggtagagcgtcgggtcctggaacacgacgatgcgcgacggatcgggccgcgtaatcggcgcatcgtcctgcgtgatgcggccggccgtggcgggctcgagcccggccaccaggcgcagcaaggtcgacttgccgcagccgctcggccccagcagcgcgacgaactcgcccggcttcaccgtgaggtcgatgtcgtcgagcacctgcagcggccccgccggcacatcgaaccagtggctcacgccgcggatgtcgatgtgcgcgccagcctggcgcacgcccgtttcggcaacaacggcggcggctaccatttgacggttcctttctgccacgacagcacgcggtcgcgcaccttgaagagcagcgtgatcaggcccgagcacagcacggccatcacgatcagtgcggcgtacatgttcgagtacgaagcccatccctgcgcccacgaaagatagaagccgagcccggccttcacgcccatcatctcggccgtgaccagcaccgagaacgccgcacccagacccatgaagaggcccacgaacacctgcggcaaggcggccggaatggccacccgcagcaccaggaaacgctcgctcgcgcccatggtgcgcgccacgtcgtagtagttgcggttgacgcctgccacgccggaccaggtgagcaccgcgaccgggaagcccgtggccagcgcaatcaggaacaccgcggccgcatagctcgacggaaagaagaagaacgccagcggcagcagcgccgaagccggcaccggccccaggaagcgcagcaccggatgcacccagtagcccgcgatgcgcgaccagccgatggtcacgcccgtgagaaagcccgcgagcgcgcccagcacgaagccgtgtgcgagcaaccgcgccgagtgcagcaggctctcgccaaggcggcgccaatcgtcgacgtaggtttcgacgaggctttgcggcggcgcgaagaaaggcgtggggagccatgcgagcttggcggtcgcaacctcccaggcggcgaagagcagcggcagcgcgacgagccagggtccggcgggccgcagcgcccgtgcgacgcggccggcacgcggcccgagcaatgcgacggccagcagcagcgcacccgccacgattgcggcgatgccgaactcgtcggtgtaggcccagtcgctgaagcccacggcctggttcggccagtagatcgtcaggaggccgagtgcgagccatgcaacggtggcggcaaagccgctgcgccatgggggaacggctgggtgctttcgaaacggtgacgcagcggtggccggtgcgcgtgcgggcgccacggcccccaccctggccctcccccggaaggggagggaatcgaagcccaatgcggggtcgggcgtgctcatgccagcggatcgaaagagacgtgctcggcaaagcgcaccggatcggtggtcttcttgagcacgccgacgccgcggaaatcgcgcgcatagaactccacctcgtcgcgcaggttcttgccgagcggatggtggctgtgcgtgagcgtgccgagcagcgcgcgcaggtcttccacgggcaccttgggcgaatacttggcaaagagcttcgccgactcgttcgggttctcggccacgtagtcggaggcttgcgcaatggcgcgcaccagcgccgccacggtcggcttgtccttgcgcacgagctcgccgcgcgcgccgacgatgcagcagaccttgtccttgtattcgcccgagaggttgctcgcaatctccacgaaggcgcccttgttgcgcttctcgatcaggtagacgttcgggtcgccatcggcaatggcgtggatctcgcccttctgcacggcgatgtcgagcaggtcagccgggtactggcgccaggtcacgtccttgtcggcatcgacgccgttcttggccagcaggatcgagaagaagttcttgcccgggctcgcgatgtccgatacgccgatgatcttgcccttgaggctcgcgatgctggtggcacccgccgccttggcgcccaccagccgcacgcagccgccgtgcgagctgccgacgatcttcacgtcgaagcccgactccagcggcttgagccagcggtggatcatgcccaccgccgcatcggccttggctgtggccagcgactccagcagctggtcggtggagccggtgtagttgatcaggtccacctggagtccgttgcgctcgaagtagccgcgctcctgcgcaacgacgacgggcgagaggcagaacgcggcggcgttccatgcgaaggtgagcttgcgggcctgctgcgaaaacgcctgcgaggcgatcaggccgcccgaggcgaccacggcggcggcgccgcccgcgcgcaggacaccgcggcgtgaaagagatacggtcatcgagaactccggtagtttttctttagagcagcagttcgggctccgcttcgaccaagccttcatagaggctgtcgaaagaatggatggccccctccgggccgccgatctggctgtgcgtgtggcgtgccgtcgcctcgtcgatgggctgcggcttgccggcggcctcggccagcaactgcgtgtggcaggcgttgtccagcgcgatataccaccaggcggcagcttccaccgtcgggcccgcggtcaggatgccgtggttcttgagaatcgcgcccttcctgtcgcccagtgcgcgcgcgatgcggtcgccctcgctggtgtcgaccaccatgccggtgaagtcgtcgaagagcgccacgtcttcgtggaacacgcagctgtcctgcgtaagggcgtcgagcttgcggcccagcgtggaccaggccttgccgtaggtcgagtgcgtgtgcgcggcggcaacgatcttcgggttgtgctcgtggattgccgcgtggatggcgaaggccgccttgttgagcggccggtcgccaatcacagtttcgcccttcgaattgaccagcagcagatcggagaccttgatgcgtgagaaatggatgcccagcggattgacccagaagtgatcggccagctccgggtcgcgcgcggtgatgtggcccgcgaggccctgggcaaaaccgaagcgtgcgaacaggcggaaggcgcccgcgaggcgctcctgccgatggcggcgttcggcctgcacgctggtgcgtggcgggatcggatcgaaccagtatttctgctgcgggttcgggttgagcttgagcggttgggctgcgttgcggtcgatggaaaggacggcactcatgaaaaatttcctgggtattggttattgctccttccccctccgggggaaggctgggatgggggcaggcggcgctcgaacggccgcggcgtcgcgaaggccgtcagcccccacccctgccctcccccagagggggagggagaaagacctaactcaggcggccttgcggaccgaggccacgcgctgcgccaccagttcgcgcgtgcgcggaatcaactcgcgcccatagtccgtcgcgtcctccagcggatcgaagccgcgaatcaggaacgtggtcacgcccaggtcgtagtagtcgagcagcgcatcggccacctgctcgggcgtgccgaccaatgcggtgctgttggaccgcccgccgatttcctgcgcaatggccgtccacagccgcttgtcgagccgtgagcccttctccgccgcggccagcaggcgcttggcgccttcgctctgctgcgggccgccgcggttgtagccctgcaccacgcgcaggcgcttggtctcggccaggatgcgttcggcgcgcgcccatgcggcgtcttcggtctccgcgaggatcgggcggaacgacaccgagaagcgcacgctgcgcccatgcttggcggcttcggcgcgcacgcgggtcgtgagctcgcgcgcctggtcgagcgattcgccccacagcgcatacacgtcggcgtacttgccggccacgggaatcgccgcttccgacgcaccgccaaaatacaccggcacatgcggcttgccgttgcgcgtctgcaccggcttcacttccgagaacgcattctggaagcggtagtgcgcgccttcgtggtcgaagggcttctcgccggtccacaccttgtgcagcacctccaggtattcgtcggtgcgggcatagcgctggtcatggtcgagccagtcgccatcgcgccgctgttcatcgtcggagccgcctgagatgtagtgcacaccgagccggccgccactgaactggtcgagcgaggcgaactgccgcgcggccagcgtgggcgcaacgaagccggggcggtgcgcaagcatgtagtggatacgctcggtgaccgaggccgcgtaggccaccgtcagcgtggcgtcgggcccggtggaatggtgcggcaccagcacgcggtcgaagcccgcgttctcgtgcgcctgggcaaaggcacgcacatagtcgcggtcgatggccgggcccctgggggcatggatttccgagaccttctggccctggatcatgccgatgaattcaacgtcgttctggctcatggtgtcctcgtgttttttcaggattgaatgcggggttgttcaggcggcgggcagacgcagtacgttttcgaagctgcggtcccacaagggcttgacgtcggccgggccgtcgagcacgccgatcttcagaaaggtgtcggccacctcctggtggctgcgcaccacggcgtcggtgacagggcccaggctgtagtcgccgctgcggccgttgaagagctcgaccaggtcgcctacaggtacgcgcgtctcgcccgattgcgcgcgcgcatacgccaggaagttgccgttgatccatgcaaaggcgcgctgcaggcgctgcagcaggtcgctcaatgccgcgcggcgcagcgcgtcgtccagcgcgcgcgggttggcgtagatggggaagttgcccgagagataacccacgccggtcttgatggtgcgcgcgccgtactgcgtgcgcgcaagctggccgttgtagccatagatggcccaggcgtcgaggtcgccgcgcgcaaacgccgaaaggccgtccgagggcgtaaggctcacggcctggatgtcgctgaacgagagccccgcctcggccagttgcttggccaggtagtagtgcgaggtggtggcgcgcacatagcccacgcgcttgcccttgaagtcggcaatgctgcggatcggcgaatccttgcgcgccagcgtggcctggttgttcaggtcttcgtgcgtcacggccaccagcttcacgctcgacttctggcgcgccgcaaacaccggcggtatctcgctgcccgaacccaggtcgagcgcgtcgccgttgatggcttcgatatgcagcacgccgttgttgagctcgcgccagtcgatcttgtagggcgtgttggcctggccggaagcctgcagcagcggccgccagagccccttgtaggtgcccacgcgcagggtcacgcccgaaagatcgcgtgcgggcgttgcggcctgcgttccgcctgccgcagcgatcgtgctccacgctgcggcggcctggagcaggcggcgccggtccattgataaatcagatttcatggcccggaccgtaccgaggccggcgctgaaagcgaacgcagaaaaacgagtttgcatatgcgggatgcgtcgttttcgtcgcggccggtcgccgctaacgtgccggaccatgagtgcactccccttgcgccgcccgccggccacgcccgaagatcccgcccctgccacggtggacgccgcattgctggcgcggctgtcggcacagttcgccgccaccgcgggcgaccacgaccgcagcggcgcctttccgcgcccgaacttcgaggcgctgcagtcgcacggcctcatcggcctggtggcgcccgcggcgtacggcggcgggggcgcctcgctggcgacggcgcggcgcgtgattgcggccgtggcgcgcggcgaaccggccaccgcgctgatcctgacgatgacctatctgcagcaccacgcgctcgcacgcagcgacagccgctggccgccgcatctgcgcgagcgcgtgttgcgagacgcggtggatcgcggcgcactcatcaacgcgctgcgcgtggagcccgcgctcggctcgcccgcgcgcggcgggctgcccgcgacggtcgcacgccgcgaaggcggcggctggaagatcgacggccacaagctctacacgaccggcatcgaaggcctctcgtggctcgccgtgtggggccgcacggacgaacccgcgccgcgcaccggcgtgttcctggtgccacgcaatgcacccggcgtgcgcgtgatcgcaagctgggaccacctgggcctgcgcgcctcgggcagccacgaggtggtgttcgagaacgtggcgatcgagctcgaccatgcggtcgacctgcgtgccccgaccgactgggcgcccgatgccggcagccagaccgacatcgacgcccatgccacgcagcaggcctggatgacggtgctgctcggcagcctctacgacgcggtggcgcaggccgcgcgcgactggctcgcgggcttcttgaaccagcgcgcgcccggcagcctgggcgcgccgctcgcaagcctgccgcgcgtgcaggagcacgtgggagaaatcgccgccctgctgcgcaccaaccgcgtgctgctcgacgatgccacccatgccgtggacgaaggccgcgcgcagccggccactgaaagcggcctgctcaagtacaccgtgacgagcaacgcgatccgcgcggtcgagctggctctgcaactgagcggcaaccacggcctcacgcggcagaacccgctggagcggcactaccgcgacgtgctgtgcagccgcatccacacgcctcagaacgacgcgatcctggtcgcagcgggcgcgcgtgcattgctgccctcgggagccaccgcatgaccgacctgctcttctccaaggcctccaaggcctcgcgccgcagctggctcaagcaagccgcggcactctcgctcacggccgccggcccgctgcgcgcatgggcgcagccgcagacgacgctggtgctcggcgaccaggccggcggcctgcgcgcgctgttcgaagcctcgaaggcgctcgaaggcgcgcctttcgcctaccgctgggccaacttccagggcgcggcaccgctgttcgaagcgcaacgcagcgcggcggtcgacacggcggtggccggtgacctgccggtgctggccgcggccgtcggccggacgccactcaagatcgtcgccacgcgcgtgggcaaggccgatgcactcggcatcgtggtgcagcccgattcgccgctgcagaaggtggccgacctgcgcggcaagacggtgatcgtgtcgtccgcgcgcggcagcatctcgcagtaccagctgtatggcgcactcgaagaagccggcgtgcggcgcgacgaggtcacggtgaagttcgtgctgccgaccgatgcggccgcggccttcgcttcgaagcagatcgatgcctgggccgtcttcgacccctactacacgattgcgctgcagcagggcgggcgcatcttgcgcgacgggcgcggcatcaacacggcgctgggcttcatcaccgcgagcgagccctcgctggccgacccggccaagcgcgcggccatcgtgcagtttctcgaccggctggcgcgtgccggcgaatgggcgctggccaatcccgaggcctatgcgcaagcctacagccagctcacgcgcctgccgatcgaatcggcccggatcatcaccgcgcgggcctcggtcaccggccgtccggtgtccgaagccgacatcgtcgccttgcaggccgtggccgaccggtcggcgcgcgacggcatcctgccggtgcgcgtggacgtgcgcgccatcaccgacgcgcaggtctggaaacgtccggcgtgagcggagtctctggcattgcgccgctgcgcgagttcgtcggcgcattcggccgcctgctcgacggcggcccggacgagccgcgcattctttccgaaggcggcacactgcttcgcgcgctggtggcgcaggacgactggctgcccgacgcctttgcccaacccgacccggcgcgctaccagcagtttctgctgcacgccgacagcaccgagcgtttttcggtcgtgagctttgtctggggaccggggcaagcgacgccggtgcacgaccacacggtgtgggggctgatcggcatgctgcgcggcgcggagtacagccagggctacgccctcgggcccgatggcctggcacggccgcaaggtgccgcggtgcggctcgacgccggcgacgtggaagccgtgtcgccgaccttgggcgacctgcaccgcgtgcacaacgcgcatgccgatcgcgtgtcgatcagcatccacgtgtacggcgccaacatcggcgccgtgcggcggcatacttacccggccgagggcggacgcaagccctttgtctcgggttactccaacacgcttcctcccaacctgtgggaccgctccgccgaactgagatcgacgacctccgcatgacgacccctgcctctgcctccgcctttccccttgcgccctttgccgccgtgcgcgcgcgcctgctcgcgcgcgaagaaaccgcgctgctcgacgtgcgcgaggaagaccccttcgcgcaggagcatccgctgtgggccgcgaacctgccgctctcgcgcatcgagatcgaagcctggcgacgcattccgcggctggacaccttcatcgtgctgtacggcgcgcatggcgccgccgacctggcgccgctggccgcgcgcacgctggcgtcactgggctacacgaacctgcacctgctcgaaggcggcctcgaaggctggcgcgcggccgggggcgagttgttccgcgacgtgaacgtgccaagcaagtccttcggcgaactggtcgagcacgagcgccacacgccatcgctttccgcacccgaggtgaaggcgctgatcgatggcaaggccaacgtggtggtgctggacgcacggcgcttcgacgaataccgcacgatgagcattccatcggccaccagcgtgcccggcgcggaactggtgctgcgcgtacgagagctggcacccgatcccgccacgcaggtgatcgtcaattgcgcgggccgaacgcgcagcatcatcggcacgcaatcgctagtgaatgcgggcattccgaatccggtggcggcgctgcgcaacggcaccatcggctggaagctcgcgggacaggtgctcgaccatggcgcggaccggaaggcaccggccagcatgtccgatgcgcaccgcgcagaggcgcaggccgacgcgcggcgcgtggcagacaaggccggcgtgcgccgcatcgcgctcgatgcgctgcatacgctcgaagcaccgggacgcacggtgtaccgcttcgacgtgcgcacgcccgaggaatacgaggcaggccacctgcccggcttcgcgagcgcgccgggcggccagctggtgcaggaaaccgatcaccaggtgccggtgcgcggcgcgcgcatcgtgttggctgacgacgatggcgtgcgtgcttcgatgagtgcgtcgtggctcgcgcagatggggtgggaagtctatgtgccggacgcagtgccaggcgcttcggccttcacggaaaaaggggcgccgccgcccgcctatccgctggccgcggtggccattcgcgagatctcgcccaatgacctcgcggccttgctgaagcagccggcagcaacggccgtgatcgacgtgaccaccagcgccaactatgtgaagcggcacattcccggcgcctggtatgccattcgcgcgcagctggcagaggccgtcggcacggccattccgccggcgcggcgctatgtgctgacctgcggcagcagcctgctcgcacgctatgccgcggcagacctgcgccaactgctcgacgcgcgcggccagagcgacgtggaagtgctggtgctggctggcggcaacgcggcgtggtttgcggcgggcctcgaagccgaatcgggcgagactcggctcgcgacgccgcgcaccgaccgctaccgccggccctacgaaggcaccgatgcgccgccggaagccatgcaggcctacctcgactgggagtacggcctcgtcgcgcaactgggacgcgacggcacgcaccatttcaacgtgatctgagagcgcggcagcgggctgcgccaccgtcggactgcgcggcctgcagcggccggtcaccggcccggcaaagctggttccgcggtgttccacgaaaatgacaaagccccaaaaaaggggctttcgatcaattcgtttcagcgctcttgaagagggccgcgaccttgcgcttggtcttgatgttgcttgagatgccgcgcgcgggtgctgccttggcggcggcttcccaggcgggggtggcgtcggcctggcccggttcgtagggcttgtcgaaaaacggatcgcgcggtgctgacggcgcgcggtgcggtcgcccgccgccgcggcgcgcatcggcgccgatgctgctgcgttcgcgcggctggtcgagcacgtcgcgtgcgtcgccggcctcgccttcttcgcgccaatggcggcggccgtcgttgatgcggccgcgaggattgtcttcctcgaactcgacgggttcgagctcgatcttcttcttgatcagcttctcgatgtcggccaccaggcgcgcatcgttgccgccgctggcaaagctcacggccaggcccgacgcgcctgcgcggccggtgcggccgatgcggtgcacgtagtcttcggcgttgaacggaatgtcgaagttgaagaccgccggcacgtccttgatgtcgaggccgcgggccgcaacgtcggtacacaccagcaggtcgacttcgccggccttgaacgaggcgagcgccttcaggcgttcgtcctggctcttgtcgccatgcagtgcggtggtacgcagaccgtcgcgctccagcgagcgtgcgaggcgcgcgcaaccgagcttgctgttgacgaacacgaaggcctgcgtgatgccgcgctgcttgacgatctgcttgagcgcacggcgcttgtcgtcgtcggccacgctgtagaagtgctgctcgacggtggacgccgtttcattcggccgcgccacctcgatggtgacggggttctgcaggtagctgccagccagccgcttgatctcgggcgagaaggtggccgagaacaacagcgtggtgcgctgcttgggcaagtagctcaggatgcgctgcaggtcgggcagaaagccgatgtccagcatgcggtcggcctcgtcgagcaccacgtactccacctggttgagcaccgcgttcttggcttcgatgtggtcgagcagccggcccggcgtggccaccagcacttcgacgcccttcttgagctcgagggtctgcggcttcatgtcgatgccgccgaacaccacggtgctgcgcaggttggtgtacttggcgtacagcttgacctgctgggccacctggtcggccagttcgcgcgtgggcagcaacaccagtgcacgcaccgggtgccgcgcgggcgacgtggacgagttctcgtgcttgagcatgcgctgcagcaagggcagcgaaaaagccgcggtcttgccggtgccggtctgcgctgcgcccatcacgtcctgccccgaaagcacgaccggaatggcctgctcctggatgggagtcatggtctcgtagcccatttcggccacggcgcgcgccagcggttccgccagcgatagattggagaaggagcttgtcattaagccctctattgtcgcactgccgcaaaaaatggcagtgacggcggcgtgacaacgtccgcgccgccggcattgctatttaattaatagcaagccagccagcaaacatcagccttccagaaccagatgctcaaagattgcgggcattgaaagtgtcgcacgacttgacgtcgccgctctgatagccggcgccgaaccaccgttggcgctgcgcgctggacccgtgggtgaagctgtcgggcaccacggcgcggcccgcggaacgctgcaatgcgtcgtcgccgatcttctgcgcggcgttcatcgcggcctcgatgtcgcccgggtcgagccacttcttcgactcttgcgaatggtgcgcccagatgccggcaaagcagtcggcctgcagctcgacgcgaacgctcagcgcgttgttctgcgactggctcaggcggccgcgcatgccgtccaccttggcggtgacgccgagctcgtcctgcacgtggtggccgacctcgtgcgcaatcacgtaggcctgcgcgaattcgccgggcgcaccgagctggttcttcagcgtgtcgtagaagccgaggtcgatgtagaccttcttgtcgccggggcagtagaacggccccatcgccgcctggccagtgccgcaggccgtgggtgtggcgccgcggaacagcaccagccggggtggttggtaggcgccgccgttctgccggaagatattcgtccagaccacttcggtgttcttgagcacggtcgagacgaaggccgcctcgcggtcgctcgacggaggcttgggtgcgggcccctgttgctgctgcacctggacctgttcgccaccgccgccgctcaacaggctgagcacggtcagcggattgatgccgaagatccagcccgcgaccagcgcgacggcgatggtgccgatgccgatgcttcgcccgccgatgaaaccgccaccgccgccactgctgcggcggtcttcgacgttgtcggattgttcgttgccttcccatctcatcgcggtctccttgccggccttgcagaagtgtgccggagcgtcgctggatggtactttgtccgtgccgatgccttgtaagcaaaacaggcatttgcatgcctgcggggacgccgtcggcaaccggctccctgaggggtacctcaggtcttgggaagcgtgacgccgcgttggccctggtacttgccgccgcggtccttgtagctggtctcgcagacctcgtcgctctcgaagaacagcacctgcgcgcagccctcgcccgcatagatcttggcgggcagcggcgtggtgttgctgaattcgagcgtcacgtagccttcccattcgggctcgaacggggttacgttgacgatgatgccgcagcgcgcataggtgctcttgccaaggcagatggtgagcacgttgcgcgggatgcgaaagtactcgaccgtgcgggccagcgcaaagctgttgggcggaatgatgcagtagtcgccgtgcatgtcgacgaagctcttctcgtcgaagttcttcgggtcgaccacggtgctgtggatgttggtgaaaaccttgaattcaggcgcgcaacggatgtcgtagccgtagctcgaggtgccgtagctgatgatcttgtggccggcggcctcgcgcacctggccgggctcgaagggctcgatcatgccggtctcttcggccatgcgccgaatccatttgtcgctcttgatagacattaaaaacaccccagtcttcgcgcacttcgtgtcgcttcgccaacccctcaaggggcaacaccagcggcccggcaaagccggttccgcggtgtttcccgaaggggcagcgcggcgccgctaggtcggcgattgtggcatgagcgaacggcgcgtctagcgctcagcccgcctgcgaaatcaccgtgcgctcgaccagccggtcgtcgccaagcacgatcatcgagaagagcagttcctcgaggttgcttgccagcgcggtcttgcgcgccagcagcggcgtggccgccggatcgagcaccagaaagtcggcctcgcagccgggctgcaggttgccgaccacgccttcgagccccagcgcgcgcgccgcgccgccggtgtggcgccaccagagttgcgaaggggcgatgctcaggccggtcttggtctggccctcccggccgacgtagtaggccgccatcatcgtgtggaaggggctgaagctggtgccgccgcccacgtcgctggccaggccgtacgggtagccgacgcggtcggccgcgtcgaagtcgaagaagccactgcccaaaaacaggttgctggtcgggctcacggcggcggcggtcttcgtgtcgcgcagcagcgcgcggtcggtgtcgtccaggtagatgcaatgcgcgtacacggcgcgttcgcgcatgaggccgaagccggcatacacgtcgaggtaagaacgcgcttttggatagagctcgcgcacccacgccacctcgtcacggttctccgccacatgcgactggatccacgtgtcggcgtacttcgcggccagctcgcctgcgccgcgcatctgggcatcggtgctcgcgggcgcgaagcgcggggtgatggcgtagcccaggcgatcgacgttgtgccacttgcggatcagcgcctcggagtcgatgaggctctgctcggtctggtcgcgcacgccgtcgggcgagttgcggtcctgcagcaccttgccgctgatcatgcgcaggccccggcgctgcgcgccctcgaaaaaggcatcgaccgacgcgacgtgcgaagtcgcgaaggtgagcgaggtggtcacgccattgcgcagcaactcgtcgaagaacacgtcggccacttcgttcgaatgcgccgggtcggcaaactttgcttccgcggggaaggtgtagttctcgagccagggcaggagcccgggcgacggcgcgccgatgatgtcggtctgcggaaagtggatgtgcatgtccacgaagcccggcgcgaggatgcgcccgggcagatgcgtcacatcggcatcggggtggcgcggcgacacggcggcatggctgccggcatcgagcacgcgctggcggccggcattgtcggggccgacgaccaacaggccgtcttcatcgaaaaccggcaggccggcgtcgtcgaatcgcaggagggaggcgcggtaggcttttttcatcgttgctgcggagggtaaaccagccccggggcgccgcaatttccatgcgcgtatgagtgctatatgccgtccccacttcaatccggcggcaaggcgcgcgactggatgtcgaagggcacgcgagcggcacggccgcagtcctcgggcagcacctgtacggcgggaggtgcggcgcttgccaccgccgtggcgagcgcgagcagcgcgcccgccagtcgcgtgcgcctgctcattgccacacgcgaaacacgcggcccgtcaatgggccttcgacgctgcgcacataggccagcgccacgcgcgcggccggtacggtttcgacgcccggaaagagcgcgccatacgcttccaacgattcggtcagcagcgtcgggctgaccgcgttgatgcgcaggccccgcgtcagctcgactgctgcgcctttcacgaaaccctcgaccgccgcattcacggccgccgcattggctcccccgcgaaccggatcgtcggccgctacgcccgtggtcagcgtgatcgagccgccatctgccagaacgcgctggcccagcagcgcgaggcgcacctggccgagcagcttgtcctgcaggccgatgttgaaatcggccggccgcatttcgaccagcggcccgaagaacaggcccccagccgccgacacgatcgcatcgacacgccccaccgcggcatacagcgcttcgacgctcgcatcgctcgtgatgtcgacctgccggtcgccgcgcgtgcggcccgcgcggaccacctcatgcccgcgctcggccagcgcctgcgccaccgcgctgcctacggcgccggtcgcgcccacaacaagaaccttcatgcaaacctcgctaaaaatgaatgagaaggctcattgttttgcgaatcgatagtttgataaattgccatctggttcggcaattcgaaactatgggttctcaatatggacaagctgcgcgccatggaggtgttcgtcgcaacggtggacgcggggagctttgccgccgctgccgaggcgctcgatctttcggccgtgatggtgggaaagcacatccgcgcgctcgaagagcagcttggcgcccgcctgctcgaacgcaccacgcggcgccacgcgctgaccgagatcggcgccgcctacctggagcgctgccgcgacgtgctcgcgagcgtgcacacggccgacggcgtggcggaatcgctgcgggccatgccgcagggcgtgctgcgcgtgacggcgcccgtggcctatggcgcgcatcggctcacacccgtcattgccgagtacatcgccgcctatccgcaggtgaaggtggatctgagtctcaacgaccgcgtggtcgatcttgccgaagagggcttcgactgcggcgtgcgatcgggcgcggcggtcgacgaacggcttattgcccggccgctcgcattggcgcgcatgttcgcggttgcaagcccggcgtgggtcgcgcgccatggccggccccggcatccgtcggaactcgaagcctttccgctgctgggctttgccgcctggggcccgaaccattcatggcgcttcacgcagggcggcgagacggtgcatgtggcggtccgcggcccgtactccaccaacaacgggcaggcgttgctggcagctgcgatggcgggcgtgggtgtgatcgtgcaggccgatgcgttgctcggccccgcgctggcttcgggccaggtggttcaactgctgcccgactgggagctgccgacgcgccaggtgcacatcatgcgactgcccgaagcccgtcccagcgccaagctgcgcacctttgtcgacctggtcgtcgaaagactgggctagctatcgcccgacgcgcccctgcacgccttcggcgagccagttcatcttcaggatctgctcgtcgtccagctgcgcgcccttggcaatgacgacacggccttcgttgtcgcgcacgtcgccggccaccgcgcggaacggctgcagcttgcccgacgcaatgtcctgctgtcgcgccagcacctcttgctgcacggccttgggcaccttgctgccgaagtcgccgacgcggatcattccgtccttcacgccgccccagacattgccgctcttccagcttccgtcgagcagggcctgcgcgcgctgcgtgtagtagccaccccactggtgcgtgacggcgacgatctgcgcgtcgggcgcgaccttgcgcatgtcggagtggtaggcgacggccatctttccgcgctcctgcgccgcggccatcacggcggtggagccggtgtggaaggcgaccacgtcggcgttctggttgaacagcgccatggcggcatcgcgttccttcggcggatcgaaccactcgttgagccacaccacgatcaccttggcattcggattcaccgagcgcatgccgagcgtgaacgcgttgatgccctgcagcacctcgggaatcggaaagcccgccacatagcccgcaatgttcgtcttcgtcatgcggcccgccgcaatgcccgcgagatagcggccctcgtagtagcgcgcgttcgcggttgccacattggccgcggccttgtagccggtgaccgattcgaacttcacatcgggaaagtcgcgcgccaccttgagcgtcggctccatgtagccgaagctcggcgtgaagatcaggcggttgccctgctgcgcaagatcgcgaatcacgcgctcggcgtcggcgccttcgggcacgttctcgacgaaggtggtcttcaccttgccggccagcgccgcttccacggccttgcggccttcttcgtgctggcgcacccagccggcgtcggtcaccggcgcgacgtagacgaagccgatcttcagcggctctttcggcgcctgcgtttgcgaaaaggcgggagataaaaagcaagcggccatccacgccagaacggcgcggcccgcgaggtttttgtacatggtggtcctctacatggccccggaaaagcaaaaaacccgcagccggccgggacgcccggctgcggggtgcggattttagtgcgccgggtccgcctgcacatgcacatgctgtcgcaccgcctcgagcagcagcgtggccagccgggccaccggcgcctcggccgccgcctgtgcgcgatagagcatgagcgacatctgcggcagcgccggaaggccgaccgccgtgcggtcaatggcgcgcacgtgcgcgggcaggccgaagggcgtgcgcaccgagagcccgaggccggccgatgtggcggcccatagcgcggcaaggctggcgctggtgaacgcatggcgccacggcgtgccggcacggtcgagcgcagcggtgacgatttcgcgcagcgggcacggtgcatcgagcaacaccagcggcaggggctccttgctcttgcgcgcgccgggccggcgctcgcgctccttccaccacgccgcgtcgagcgcatcgggcgcccgtgggccgatccattgcaacggcaggcgcgccacgcgctcgccgtgcggcgtcatctgctcgccggtgtcccacaccagggcaaggtcgagttgccggagttcgagccgctcgcgcagttcggcgctgcgcgccacgcaggcctcgatgcgcaccttgggatgcgcgcgcgaaaagcggccgagcacggcaggcagcagcgtctcgccgaagtcttcctgcaggccgaggcgaacccagccttgcaggtcggcaccgcgcatcgcggcgccggcttcctcgttgagttcgagcatgcggtgcgcataggcgagcagcgtctcgcccgcatcggtgagctccagcccgcggccggccttgcggaacagcacggtgccggcctgtgcctcgagtttcttgagctgcgcactcacggccgacgtcgagcggcccagcttgtcggccgcccgcgcatagctgccaagcgcgatgccggtggaaaaactgcgcagcacgtcgagatcgaacatcacctgggacatggatttcttccttcctcgatcgtcctgttttatcgaacgatcagctcattattttctgattttcaaaacctttgcaacggcggagactgcgcctcgacatgacgcattcgatcccctccccttcgtatccacgccgccaccgctggaaagtgctggccgcgggtgtcgccgccaatgcggccttctccgtggccttcagcggcattccaatgaccgcggtgctgatgcgcaccggctaccagctcgacaacgccacgctgggcctggtgctcggcctcatgggcctgggcatcgcggtgagcgagctgccatggggcctcttgaccgaccgctggggagacaggccggtactgctcacaggcctcggcaccaccgcggccgcgctggtggcgatggcgctctgggcggcgccgagcgcacagcacattccgggtctgggctggctttgcggcgggctgctgctcgtcgggttgctcggcggcagtgtcaacggcgcgagcggccgcgcggtcatgacgtggttcgaagcgggcgagcgcgggcttgcgatgagcatccggcagacggccgtgccattgggcggcggcatcggcgcgctggtgctgcccttcgtggcgctgcatttcggctttgccgcgctctacggcttgctggcgctgctgtgcgcactgagcgcggcaatgagctgggcctgggtgcatgagccgccggttgcgccgcgcgccaaggccgcggagacatcaggcgcgccgaagggcagcggcccgctgcgcgatgcgcgcgtctggcgcatcgtggccggcatcggcattctttgcgcgccgcagttcgcggtgctgtccttcggcacggtgttcctgcatgacttcggccatgcgggcctcgcaaccatcacggccacgatggtgttcgtgcaggtcggcgccatggtgatgcgcgtctggagcggccgctggaccgaccgtcggcgcaaccgccctgcctacctgcgcgcctgcagcgcactcagcgtgctgctgttcgctgggctcgcgctgctggtgctggcactgggcgcaggcacgcacaccgtcgactcatcgacactgcgcattgcgctggtggcgctgctggcggccagcggtgtctgcgtgtcggcatggcacggcgtggcctacaccgaactcgccacgctggccggtgcggcccgcgcgggcacggcactgggcatggcgaacaccagcgtgttcctggtgtgctttgtcacgcccttctccatcccgcacctgctcgcgctgcagggctggccgctggtgtggctcgcagccagcgcatgcgcgctggtggcaatgccgttgctggtgcccaggcccggcgctgccgatcagaagcttgcgaagacggcgttgagccggtcgacgtaggcgcgcttggcggccgcgtcgatgaagctgccttcgaagctgttggccgcaagctgccacgcctgctgcacgccgagcccggtggccgcgaaggtctgcgtgaagttctggttcatgtagccgccgaagtaggccgggtcgtccgaattaacggtggccaccagccccgcgtccagcagcgcgccgaggttgtgctgcgccaggtcgggaaacacgcagagcttgaggttcgacagcgggcacacggtgagcggaatgcggtcttgcgcgagccgcttcatcagcgccggatctttcgcgctctgcacgccgtggtcaacgcgctcgaccttgagcacgtcgagcgcgctccacacgtaagccggcgggccctcttcgcccgcgtgcgcgacgaggtgaaagccaagctcgcggcagcgcgcgaacacgcgcgcaaacttctcgggcggatggccgacctcgctcgagtcgagccccacgccgatgaatttgtcgcggaagggcagcgcctgctccagcgtttcgaaggcttcttcttcactcaggtggcgcaggaagcacaggatgagcgccgcgctcacgccgagcttcggctctgcatcggcgcacgcacggtgcaggccgttgaccacgacctccatcggcacgccgcgcgccgtgtgcgtctgcgggtcgaagaacatctcggtgcgcaccacgttgtcggccgcggcgcgctccaggtaggcccaggccatgtcgtagaagtcctgctccttcagcagcacgctggcgccggcgtagtagatgtccaggaagctctgcaggttggtgaaggcgtaggccttgcgcaggtcttcgacgctcgcatacggaatggccacgccgttgcgctgcgcgagcgcgaagatcagctcgggctccagcgagccttcgatgtgcatgtgcagctcggccttgggcatggcgcgcagcagctcgggcaggcggtcggcggagatcttgccgaagctcttgtcgaagagggggcgggaatcggtcatggtgggaagtcgacgttgtgattgcgcacagcataagcgcacccgccccgtgcgggatgcgccaaaccgtatacgttcaatcgatcccgcgcgccgaactggtgagcgagcgagcgcacagcagcagcgttggcgccagcttgcgcacggcctcctccatggtccagcggctggtcggcgccacgacgtgcaccgacgcgacgggccggccctggctgcccaccacgggcgccgcaatcgtcatgtcgccgaggaacagttcctcggcgttggtggcaaacccctgcagcctcgcctggcgcaaggcctcgaggatctggtcgacaccggtgcgggtgtgggcggtatgcgccacgcggtcggaggcctcgatcagcgcccgcgcctcatcctcgggcagcgcgctcaggtaggcgcgcccggaagcggtgcaatacatgggaatgcggctgccgatcggcatgtggaccggcacgaactgcgcactgacaaagcgcgcgacatagaccatgtcgaggccgtcgggctcggtcaggcaggaggtttccgtggtgaccttggtcagttccgacaggaacggattggcaacgtcgatcagcgggttggccgccaggtagttgaagccgatttccatcacccgcggcgtgagctggtaacgccgcgtctgcgggtgcttgcgcacgtagcccagcttttccagcgtgaagaccatgcgctgcgccgaactcttggtgatgtcggtggccgcagccacgtcggccagcgtcatggtgcgccggcgggcgctgaaggcctgcagcacggccaggcccttctccagcgactggttgaaaagcaggctggggctttcgccgggggcggcttcgggtgtggcgtccatggctgcggagtatacccatatcggcctgaaatatcgaatatcgatacgatcaactcgcctaatggtttctatttattgatatgagattcaaaagaatcgattattggcatgcatgttgcatcgtccgccgagccatttcttccttttctcctttcgctctttccaccttcttcgaggagtgcttccatgaatcgcatcgttcgccaccttcaccgctttgccctgggcctctgtgtcgcgggcgccgcctcgctggccggcgcgcagggcgccgcgcccgccacttacaacgtgggcgccacggccacgggcgtaccgttcaccttcctggatgtgaagaccaacaccatccaggggatgatggtcgacaccgtcactgccgtcggcaaggctggcggcttcggcgtcaacgtgcagcagacggtgttctcggcactcatcccctcgctcaccgcccgcaagatcgacatcgtctcggccgccatgctgaagacggcggcgcgccaggaggtggtcgacttcagcgacccggtctactcctatggcgagggcctgatcgtgaagagcgacgacacgcgcgcgtacgtctcgctcgacgagctcaagggcgaggtggtcggcgcgcaggtcggcaccgtgttcctggacatgctcaccaagaaaggcatcttcaaggaggtgcgcagctacgactcggtggccgacatgacgcgcgacctctcgctgggtcgcatcaaggccggcctgggcgaccagcccatcattgcctaccagctgcggcagaacaattttcccggcgtgaagctggtcgagagctacaagcccgtgaacgtgggcgacgtgtgcctggtggtgcgcaagggggatgccgagacgctggcccgcctcaacaagtccatcgccgcgatcaaggccgacggcacgctcgccaggatcgtgcagaagtggggcatctgacgcatcgcacccatggccgcttctttcctccagaacgcgcaggatttcctgccgatcctcctgcagggcgccgtcgtcacggtgcaggtcaccgtgctctcgttcctgctcagcagcgtgctcggcctcgggctcgcattgatgaagctctcgccggtgcgcgcgctctcgtggacgggcacggtgatcatcaacctgatccggggcctgcccatcatcgtgcagctcttctacatctactttgtgctgccggagttcggggtgcagctcacggccttccaggccggcgtcatcggccttggcattgcctactcggcctaccaggccgagaacttccgcggcggcatcgaggccgtggacgcgggccagcgcgaggccgcccaggccatgggcatgcgctcggcgctgatcatgcggcgcgtgatcctgccccaggcctttcgcatcgcgctgccgccgtacggcaacacgctggtgatgatgctcaaggactcctcgctcgtctcgaccatcacggtggccgagatgacgcgcgccggccagctcattgcttcgtcgacgttccagaacatgacggtctacacactggtcgccctgctctacctgctgatgagcctgccgctggtctacgggctgcggcggctcgaaaagcgcttcggcgccggaaggaaacacccatgatccgcgtcgacggactggagaagcgcttcggtacgcatcgcgtgctgcagggcgtgagcctgcatgtcgatgccggcgaggtggtgtgcctgatcggcccctcgggttcgggcaagtccacggtgcttcgctgcatcaacgggctggaatcgtacgaaggcggagaggtgcgcgcatttgacgaacgcgtcgaccgcaacgacaagagcattcaccggctgcgcagccgcatgggcatggtgttccagcgcttcaacctgttcccgcatcgcaccgtactggagaacgtgatggagggcccggtctacgtgctgggccacaagcccgcgcaggcgcgcgaggaagcgcttgcgctgcttgccaaggtggggcttgccgaaaaggcgcaggcctatccagcccagctctcgggcggccagcagcagcgcgtggccattgcgcgcgcgctggccatgaagcccgaagccatgctgttcgacgaacccacatcggcgctcgatcccgaactggtcggcgacgtactcggcgtgatgcgcgccctggccgacgaaggcatgaccatgatcgtggtcacgcacgagatgggcttcgcgcgcgaagtggccgaccgcgtgtgcttcctgcacagcggcagcatcgtggaagaaggcccggccgcgcaagtgctgggcgcgccgcgccagccgcgcacacaggatttcctgcgtcgcgtgctgcatccctcggcggcacctgtcgaggtccggccatgagcgccgcgccgggccgccccaagcaagctcgcaccgcagtgcgtagcacggaggttacccaatgagcgcagcgcacgcgctgcccgcgtcgctgtgggcagccaccgcgccgcccgcgccgccaacgccgcccttgaccgaatcgcgcagggtcgacgtactggtcgtcggtggcggcttcaccggcctgtcgaccgcgttgcacctggccgaggcgggtgtgcaggtttgcgtgctcgaggcgcacgagcccggctggggcgcctccgggcgcaacggcgggcaggtcaaccccacgctgaagcatgaccccgaggacctggcccgcatctacggcgtcgagcgggcggcgccgttgatcgacgccgtctcccgctcggccgacgtggtgttcgacctgatcgcgaggcacggcatcgactgccagccggtgcgcaacggctggctgcaggtcgcctactcgccaaagcacgtggcgggcctgcacgcacgcgccgcccaatgggccacgcgcggcgtgaacaccgagatgctcgaccacgcggccgtcagcgcacgcctgggcaccgaggccttcgcaggcggctggctcgacccccgggccggcggcatccagcccctggcctacacccacggcctggtgcgggccgcgcaaggcttcggggccgcggtgcacggcggcacacaggtgaccgcgctggagcgccggggcacgcaatggcacgccagcacctcgaccggcgccaccgtcatcgccgaccaggtggtgctcgccaccaatggctacacggggccgttgtggccggggctgtcgcgcaccgtgctcgccgccaacagcttcatcgtggccacgacaccgctcgaaggcactgccgccgacgcgatcctgccgcacggcgaaaccgcctcgacctcgcaacgcctgctgctgtacttccgcaaggacgcagagggccgcctgctgatgggcggccgcggccactttgccgatccgtccggcccggcggacttcgcgcacctggaacgctcgctcgaattgctttttccccaactagggccgctgcgctacgagtaccgctgggccggccgcatcgcggtcacccgcgacttcatgccccacgtgcacacgccggcgccgggagtgactattgcgctcggctacaacgggcgcggcatcgcactggccaccagcatgggcaagcacctggccgcgcggctcgtcgatgcgggggcggattttccatatccggtgacgcccatccagccgataccgctgcatggcctgcagcggttttatgtagctggaggagtggcctggtacagcctgctggatcggatggcctgaggcgattttcggaatttttcctgaccgtcaccaggccgccgcagtgcccagcagcgcacgccgggccagcagaaaggtcgcggcattccagctctggcccgccatgcccatcggcgccagcgtgcggccatgaaaccactcggtgaaacgccagccgccgagttcgttcacgtgcgcaaggcgcgcgagttcgggccaggccatgtcatgcaggcccaggcgggcgagcgccatgacccagaagccgccgacgaaaggccagatgccgccgttgtggtactggtgcacgacgttctgctggtggcgtgccatgtagggacgccacagctcatgctcgcgcgtcagcggatgcagcaccacgcgcaccgggtacggatcgcacgcgcgtgccgcggcaatggtcttgacgatgcggttggccatcgcggaatcggccaggccgctctgtatggccagcacgttgccgaacacgtccccctcgttgccgacaaaggaaagattgacgaagctgagatacaggcccggatccgttcgcccgcggcgcgcatagtgccgcagcagccgcgcgcggtggtactcgggcaggtcctgctggtaagggtgaaagagatggttgaagtgatgctcggtagcttcggcgtgggctagctcgaagcggcgcttcacctcataccagagcgcgttggtgtacagcacgtagcccgagcgcggcatgatgtcggcccagtcgctggcttcgttctgctgcaagagccggaagtgctggtgctcctgcgccagcagccagccgatggcgcgctccacctcgccactccaatgcgaggcgccgaccttgccatggcgccgcacgtggtccaccgcaatcagccaccacagcgtggcgtcgatgcagcccaggtaccagaagtcggcgtcctgcccttcggggtcgacgtatttgggaatctgcccgttgggcgcttgctgcgccgcgagcgcatcgaggctggccacggcgccctgctccagcgcggccacaccgctgccgcacatcgccatcacgcagatggcggcatcgcgcccgaagatgcgcgtgtagcgtcgcgccacggccgcctcggtccggctggcggccagaatgccatgcggcgtgaggttgcgttccaggagttggatcgaggcttgggtgcagtcgtcgatcagcgcgagattggatgcgtcgagatgggtcattcaaaaaaaagggtcgcccgcgggcgacccattatttacacgtgcgcaatgcgcgcagcgattacttcttgtcgcccggcaccttgccttccacgcccttgacgtagaagttcacgcccgacaggaacttgtcgtcggccacggcatccttggcgaccacttccttgccgtcctggcccaggatcgggcccttccagatcacgaagctaccgtccttcaagccctttttcacttcctcgaccttggctttggtttcggccggcacatcttcggcgaccgagacgatgtcgatggcaccttccttcacgccccaccagctctggccggtggcccacttgccttcgagcgcgtccttggtggccttgatgtagtacggcgcccagttgatggtggccgaggccaggtgagccttggggccgtaggccgtcatgtcggaatcccagccgaaggcgcgcttgcctttttcctgtgcggtcttgagcacggcgggcgagtcggtgttctggaacagcacgtcggcgccgccgttgatgagcgcggtggcggcttcggtttccttcggcgggctgaaccattcattcacccacaccaccttggtggtgatcttcgggttgaccgactgcgcgccgagcgtgaagctgttgatgttgcgcagcacctcggggatgggcaccgagcccaccacgccgagcgtgttggtcttggtcatggcaccggcgatgacgccggccatgtaggcgccttcataggtgcggctgtcgtaggtgcgcatgttctcggccgtcttgtagccggtggcatgctcgaacttcacgtccttgctgtcggtggccaccttgagcatcggctccatgtagccgaaggtggtaccgaagatcagcttgttgccttggccgaccatgtcgcggaacacgcgctcggcgtcggcgccctcgggcacgctctcgacgaaggtggtcttgatcttgtcgccgaattccttctcgagcgccttgcggccgttgtcgtgcgcgaaggtccagccgccgtctccgaccgggccgatgtaggcgaatgcgatgttgagcggcgcagccggtgccggtgcggcggccgtgggtgccggcgccggtgcgggggtcgcggccggtgcagcggcttcctctttcttgccgcagccgatcagggccgccgaagcgaccgccgtgagggcggccagcttgagcagggagcgcttgttcagatcattcattgtcgaaaatcctcaaaaaggacaggttggcggaaatcgagaagcaagattatgagccggggtagaacggctttcctatcgaggccggcatgttgatgcgaatgaaggcaggattccgcgaaatcagcgccaacacgacgatgggcgcgatgtactgcagcatgctgagaaactgcggcggcacgtcgacgccgctgctctgcagatgaaaaccgagcatcgagacgccgccgaacaggtaggcgcccagcaacacgcggatcggccgccaggtggcaaaggtggtgagcgccagcgcgatccagccgcggcccgccaccatgccctcgacccacagcggcgtatagacggtcgacaggtacgcgcccgccagcccgcacagcgcgccgccgacgatcaccgcgaggaagcggatgcgccgcaccgggtagccgagcgcatgcgccgactcaggcgattcgccgaccgaacgcagcaccagcccggcgcgtgtgcggtagagaaaccagatgaggccgacggtcagcaccacagcaaaatagaccatcgggtgatggcgaaagagcgccggcccgatgagcggaatgtcgctgagcaccggcactgcgtaagacacgctctcgggcagcttggcctgcacgaagttgatgcccaggaacgccgagaagccgacgccgaaaaggctgagcgccaggccagtggcgtattggttggtattgagccagatcaccagcacgccgaagaaggccgcaagcaacgcgcccgccgccatgccggccaggaagccgagccaggggttgcgcgtggtgaccaccgtcgcaaagcctgcgatggcggcgcagagcatcatgccctcggccccgaggttgacgatgccggccttctcgttgatcaacaggcccagtgccgcaatcgcgagcacggtgccggcgctcagggtggagccgagcaggagtgcgtagctgtccatgtcagtggctccgttgcgggttgattgtttgatgctcttgttcagggcgcgtgcacaggccaccgggtactcccctccgcgaatgtcccccggcttcgcctcctcctttatttcgctgcggggagcacccggcgccctgcgcacactgggcgctgcgattgttccgttcgatcaaccactgctctgaacaacgaccacgtcgatggggtgctctgcgcagcgaaataaaggaggaggccgaaggccgggggacattcgcggagcagagcacgccgtcggcgtggtcgtgccctgaacaaggccccgaacgcgcaacgcatcgaattgaagaacgggttttcatcctagagcgctccttcggtcgaacgcgcagcagcaggcgctgtgatcggcgtgctggcctgcagcgaagacgtcgcccctccggccgtgggtgccttgagggccgccttgccccggatgcgataggcgatgagcgtgtcgcaggccagcagcgtgaagagcagcagcccctggaacacccctgtgagcgacttgggcaggccgaggcgcgactgcgcaagctcgccgccgatgtagaacatgctcatgaggatggccgagaacaccatgcccaccggatgcaaccggccgacgaaggccacgatgatggccgcaaagccgtagcccgccggcacgtacggcgtgagttggcccagcgggcccgccacttcgagcgcgccggccaggcctgccgcgccgcccgaagtgagcaacgcgatccagatggcgcgccgcgccgagaagcccgcatagcgcgcggccgcgggtgcgagcccgccgacctgctgcgcgaaacccgcccgcgtgcggaacaaaaacacccagagcgcgccgacgcccaacagcgcgatgatcagcccgatgctcacgcgcgaacccttgaagagccgcgggatctgcgtcaccgcctcgaaggtcttggactgcggaaagttgtagccgtgcggatccttccaggggccgaagaccatgtagccgagcagcagcgtggccacgtacaccagcatcaggctcaccagaatttcgttggcattgaacctgtcgcgcaggaaggccacgatgccggcccacaccatgccgccgaccgtgcccgcgaccaggatggccaccacgatccacgagccggtggtcttgtcggccagcaacgcgacaccgcccgcggcgatggcgccgaacacgaactggccctcggcgccgatgttccagacgttggagcggaagcacaccgccagcccgagcgcgatgatgagcagcggcgtcgccttgatcgtcagctcgccgatcgcgtagccgctcttgatgggctcgtagaagaacaccagcaggcccttgaccgggtccttgccgagcgcggcgaacagcgccacgccgatcagcaccgtgatgagcagcgcaagaatcggcgaggcaaaggtccagaagcgcgaaagctccggacggggttcgagcttaagcatgggccgcctccttcttgttcttctgtccttcccaaagaccgctcatccattcgccgatctgcggcagcgtggcggccgcacggtcgatcgagggcgacaggcggcccttggcaatcacgtgcaggcggtcgctgatgtcgaacagctcgtcgagctcctcgctgaccaccagcaccgcgcagccggcgtcgcgcagcgcgaggatctcgccgcgaatcagtgcggccgcgcccacgtccacgccccaggtgggctgcgagacgatgaagagcttggggttggcgtcgatctcgcggccgacgatgtacttttgcaggttgccgcccgagagcgaacgcgccgccgcgccgggcccgccggccttgacgttgaagcgcgtgatgatcgccttggcatgcttctcgagcatcgccgtgcggatccacccgcccttgcccacggcgttgctgcgcgtgagcagcaggttgtgcgcgagccccagcgtgggcaccgcgccgcggcccagccgctcctcgggcacgaagtgcaggcccatggcgcgccgcgcgcgcggccgcagccggccaaccggcttgtcgaacacctgcaccatggccgcttcggcccgcacgtcctcgcccgagagcgtgtagagcagttccttctggccattgcccgacacgcccgcaatgccgaccacctcgccggcacgcacctcgaacgagatgccgtcgaggtcgacgccgaactggtcttcgcgcgccagcgtgagagcgttgacgcgcagcgccactgcgcccgcatgcaccggccggtgctgcaagggcggcggctcgctgccgatcatcaggcgcgagagcgattcgttgctttcgttctgcggattgcacacgcccgtgaccttgccgccgcgcagcaccgtgcaggccgtgcacagctcgcgaatctcgtgcagcttgtggctgatgtagaggatgctgcagccttccgaagccagcttgttgagcacgctgaagagcttgatcaccgcctgcggcgtgagcaccgaggtcggttcgtcgaggatcagcagcttggggttggtgagcagcgcgcggatgatctcgacccgctgcatctcgcccaccgacagcgtgtgcaccggccgcgagggatcgatgtccaggccgtattcgctcgccttggccgtgatgctgcgcgccacttcggccagctgcagcgacttgtccaggcccagccacacgttctcggccacggtgagcgtgtcgaacaggctgaagtgctggaacaccatgctgatgcccagtgccctcgcctgctgcgggttgcgcagcgccaccgcctggccatcgaaagtgaccgtgccttcatcgggcttgaccgagccgtagatgatcttcatcagggtcgatttgccggcgccgttctcgccgagcacggcgtgaatctcgccgggcgcgacggccagcgaaatgtcgctgttcgccaccaccgcggggtagcgcttggtgatgttcgcaagctggagtctgggagttgtcatgccgggttcagtggggttttctcgttcaacagcaacaagcggaaaacatggctacaagtctaatagcgtgcccgcgacgatcggcgctcgcggccgtgctcaatgtcctcctacataggcaaacttgaacaggaagatcgccgcgatcacccagaccattgcatgcacttcccgtgcccgcccggtgaagagcttgagcaccgcgtaggtgatgaagccgaaggccaggccgttggcgatcgaataggtgaaaggcatggccaacgcggtcacgacggccgggatcacttcggtcgtgtcttcccattcgagatcgaccagatcgcgcagcatcaggcagcctacgaagagcagcgccggtgcggtggcataggccggcaccgagcccgccagcggcgagatcatgaggcacgcgaggaagagcgccgccaccaccacggccgtgaggccggtgcgcccgccggcctgcacgccggccgcgctttccacgtaggcggtggtgctcgaggtaccgagcagcgagcccgcgaagatggcgccgctgtcggccaagagcgccttgttcatgcgctccatcttgccgggcacgagcaggccggcgcgcttggccacgcccatcagcgtgccggtcgcgtcgaacatctcgaccaggaagaacaccagcaccacgttcaggatgccgcccttgagtgcgcccaggatgtcaagctgcatgaaggtgggcgcgatggatggcggcgcgtcgaacacgccttgaaacttgttgccgccgaagaagaacgacagcacggtcaccagcatgatgccgatcaggatggcgccgcgcaccttgagccggtcgagcaccacaatgacgaggaagcccagcgtcgccagcaccaccggcgccgaatgcaaatcgcccagcgtgacaaaggtggccggcgatgccgccaccacgcccgcgctcttgagcgcgatgagcgcgaggaacatgccgatgcccacggtgatcgccgttcgcagcgactgcggtatgccttgtatgaaaagctcccgcaaccccgtgaccgtgacgatgaggaacaggcagcccgagatgaacaccgcgcccagcgccacctgccatgtgtagcccatgcccagcaccaccacgtaggcgaagtaggcgttgagccccatgcccggcgccatggcgatcgggtagttggcatacaggcccatgatcagcgtgcccaccgcggcgatcaggcaggtggccacgaagaccgagcccttcggcatgcccgcgtcgccgaggatcgacgggttcacgaagatgatgtaggccatcgtcaggaaggtggtgagccccgcgatgacttcggtgcgcaccgtggtgttgtgctctgtcagcttgaacatgcgttcaagccagttcgcgctctgcggcgcggtgcgcgggcgcgcggcctcggtgctccccgaggcacggggatcggtgaccttgggcacctcttcaaacctgttcatgtcgcttgtctccagctgttttatgcggcggttcttcatcgttgcttcggccacgccgccagcgcggccgaaggcttcagggcggatcgggaaattcagtcagcgaagcccgcgcaacgtgcgtcgaaggcgcgggccgcagcgatgccgccacgcccttgatgcattcgcgcagccagcgtgcggagctcgacgaatgggtgcgctcgtgccagagctggtagtacatgaggcgcggcagcgccaccgggcaatcgagaatcttcaccggcagccgcgccgcgaagcgctcgcagtactggcgcccggtggtcagcaccaggaggctcgaggccaccatgtcgggaatgaggctgaagtgcgcgcagcgcgccgtgatgttgcgctgccgcccgagctcgtcgagcatctggtcgatgatgccgcgccccccggggtgcatgggcgtgggcgcaatgtgctcggccgcgagccaggtttccaggtcccagccgcggcgcaccgccggatggtcctggttcaccagcgacaccacctcgtcgccaaagagccgcgccatgtgcaggtcttccgggggcttctgccagttgccgatcaccaggtcgacctgcccgagcgccagatggccgtggtagtccgagtcgggagagagcgcgtggatctcgatctggcacagcggtgcctcgcgcttcacgtgcgccaccagcatcggcaggaagagcgggtccaggtagtcgctcgcggcaatgcgaaaggtggtggccgccgactgcggctcgaagccgcgcgcatcggagaacagcatctcggccgcgcgcaggatgctggcggcgggctcgatcatccgcagccccgcatcggtcggcaccatgccggagcccgagcgcaccagcagagggtcgcccgacagctcgcgcaggcgcttcagtgcggccgaaacggccggctggtacatgcccaggcgaatggcggcgcgcgagacgctgcggtcggtcagcacggtgtgaagcacccggatgagatgaagatcgatcttgtcgaaaagggcctggtcacgcatggcgctcccccacggcagtggtccgcaaccccggcgcggcaaagccggttccgcggtgtttcgcgaaggggatcaggacgtagggcattgggaggactttggacatgcgccaaagtctacgagtggctatgcagactggacggcggtgatcgcgcgaagaatcgactcgctcgtggccggcgcctgaagcggcggatcgaccctgtggccgccgaccgccgacaccgcgtcgcggatcgcgaagaacaccgagaacggcagcaggagcggcggctcgccgacggccttgctgcggtggatcgagtcctcgaagttctggccttcgaacaggcgcacgttgaacaccggcgggcagtcgttggcggtcggaatcttgtaggtgctgggcgcgtgcgtggtgagcatgccgcttttcggatgccacaccagctcttcggtggtgagccagcccatgccctggatgaaggcgccttcgacctggccgatgtccacggccgggttcagcgacttgcccgcgtcgtgcaggatgtcggcgcgcaagagcttccattcgccggtgagcgtgtcgacgatcacctcgctcaccgccgcgccataggcgtagtagtagaacgggcggccctgcatcttgtccttgtcccagctgaggccaggcgtggcgtagaagccgtcggaccacagctgcttgcggtcgagatacgcctcacccaccacggtgctgaaggccagcgagcggccgttgacatcgaccttgtcgttggcaaagcgcacctcgctcgccttgccgccgtggcgttctgctgcgctctcggccaggcgctcgcggatctggcgtgcggcatcctgcgcggccttgccgttcaggtcggcgccggtcgatgcggccgtggccgaggtgttggccaccttggtggtgtcggtggcagtgacgcgcacgcgctcgaagctcacgcccagttcatgcgccaccacctgcgccaccttggtgttgaggccctgacccatttcggtaccgccgtggttcacgaggatcgaaccgtcggtgtacacgtgcaccagcgcgccggcctggttgaagtgcttcacgttgaacgagatgccgaacttgagcggcgccagcgccaggccgcgtttgagcaccgtgctcttcgtgttgaaggcggcgatctcttcgcgccgcgcgcggtagtcgctgctggcttcgaggtcggccaccagttcgtgcacgatgttgtcggtcacggtctggcggtacggcgtgacgttgttctcggccttgccgtagaagttgatgcgccgcacgtcgagcggatcgcggcccagtgtgcgcgcgaccgagtccatgatgttctcgatggcgatggcgccctgcgggccgccaaagccgcggaaggccgtgttgctctgcgtgttggtcttgcccgagtagccgtgcatggccacgttgggcagccagtaggtgttgtcgaagtggcacagcgcccgggtcatcaccgggcccgacaggtcggccgagtggccggcacgcgagaccatgacgatctcggcaccgaggatgcggccctcgtcgtcgtagcccacttcgtactcgtaccagaagcagtggcgccggccggtgatcatgaagtcgtcgtcgcggtcgagcctgagcttcaccggacggcgcagcttgctggccgccaccgcggccacgcaggcaaagagcgccgactgcgattccttgccgccgaagccgccgcccatgcgccggcattcgacgtgcacctcgttcgactgcaggtgcagagcgtgcgccaccaggtgctgcatctcgctcgggtgctgcgtggagcaatggatgtgcagcgcgccgccctccttcggaatggcgtagctgatctggccttcgagatagaactgctcctgcccgccgacgtcgagcgtggcggtgtggcggtgcggcgccgcggcgatggcggcgcgcacggcggcctcgtcgccttcgttggccgcgccgccgctgcgcacgatgtgcatcggcggcaccacgtactggccgcgcgcatgcgcgtcctgcggcgtgagcacgggcggctgcgcctcgacggcgatgacgtccttggccttggcggccgcacggcgcgcggcctcgcgcgtttctgcgatcacggcgaacaccggctggcccaggtagcggatctggccgccgtccttcagcgaaagcaggatcgggtcgtcatgcacgatcgagccgcaatcgttgctgcccggaatgtcgtcggcggtaagcaccgagactacgcccggcatcgcgcggatggcatcgagcgacagcgccgtcacgcgcccgttggccgcgggcgacaggcccagcgcgcaatgcagcgtgccggcaatttcgggaatgtcgtcgatgtaggtggcttcgccggccacgtgcaggtgcgccgactcgtgcggccggctgatgccgacgcgcgcgccctggtcgtgcgccagggtttcggcgccctggtcgatgcgggcggcggtgttcttgaggtagtcggcaaaggcctcggagggctgcagcaggcgggcgtcgatgggtttgttcatgatcagaccccttccgcggccttgtcggccttgatcgtcgttgaatgaggcatcgcgctccacacgctggtctcttcaagcgacagcgcgccttcggtgcgggtttcgagccagagccgctggatcaggttctgcgccacttgcaggcggtagccggccgaggcgcgcatatccgacagcggctggaagtcttgcgcgagcgccagcctggcggcgttcacgctggcctgggtccatggcttgccgacgagcgcggcctcggcgttggcggcgcgcttcacgatggcggccatgccaccgaaggcgaggcgcacggccttgacggtgtcgctgccgggctccagttcgaccgcaaagccggcgcacagtgccgagatgtcgcagtcgaagcgtttgctgatcttgtaggcgcgcacctggcgctgcatggccgcgagcggaaccgccagcccctgcacgaactcgccgggctgcagctggttcttcatgtagtcgatgtagaaatcgggcaacggcatgcggcgcacggcattgccgcggcgcagttcgatctcggcgtcgagcgacatcagcaccggtggcgaatcgccgatgggcgaaccgttggccacgttgccgcccatggtgccggcatggcggatgggaggagaggcaaagcgcagccacacgtcttccaggctgggcacgcgctgcaccagggcttcgaaggccgattcgagcgaggcgcccgcgccgatgtagagctcgccgcctgtgtcgttctggcggacttcgatggtcttcatttcagccacgtcgcccacgtagatgatgtcgcccagatcgcgaaactgcttgttgacccacaggccgacgtcggtcgagcccgagagcagttgggcaccgggtttctgctcgcgcagcgccgcaagctgtgccagtgtcttgggggcatggaaatggtcgacgcgggcgccgagcggcgcggcgtagtcgaagccgtcgttgccgcgcaatgccgtgagcgcggccaccacgggctctgtatcgagccgcaccgccggcaggtcgaacatgcgctggcccgcatccagaatcggccggtagccggtgcagcggcacaggttgccggaaagctcgtcggccagctgctgccgcgtaggctgggtgccctcggcctggtggtgctcgtacgcggaccacagcgacatcacgaatccgggagtgcagaagccgcactgcgagccatggcagtcgaccatggcttgctgcaccgggtgcagccggtgcacgggatgcggacgcttgtcctgcccctgcacttcggtggcggcgggcgcgttggcggggcactggtccttgaggtcttcgaccgtgaagagcgccttgccatgcagggtcggcaagaactggatgcaggcgttgaccgtctgcaactgcaggccgccgatgacgccgggggcattggcatcggtagccagctctccgatcacgaccgtgcaggcgccgcagtcaccctcgttgcagccttccttggtgccggtgcagtgcgcgtcctcgcgcagccagtcgagcaccgatcgggtcggatggacaccgctgacgtcgacgatcttgccgcgatggaagaagcggatcggttggatgttgttgcgctctgtactcatgctttttggctcgtgggtgaccggttttcccggccatgcccggacgttagccggttgcgccccggcccacataccgcgtgaaccatattgcgtatgtcggcgcgggtatgcgacctagggagaaaccctgaagagcgagagcaagtcccgggccatggttaggactggcagcgtggaatatgggcactttcgaaacgaatctcgcgcgctgatatttgttgacattcctgatcgcctttcgctcccactttcgcttccagaatccggccacatagcccgccgacctccgtggccttcggatcgcgaaggccgtaatgctcggacttggatagacgtggtcgatctgcggggcgagcaggtcgacttcacgggccgccagttcgacgttccgagaacagcgccgtgatcacctggcgcagccagtggttggccggatcggcctcgaagcgcttgctccagtgcagcgatacggtgaagtcgcgcagcggaaacgacggctcgacgatggcgtagccgccctcttcggcaaagccgcgcgcaatgttgcgcggcatcaccacggcaagatcggtggcacgcacgatggccggcaacaccatgaagtgctcggtcgtgaggcgcactcggtcttcgaggttcagcagctgcaggatgcgcagcgtgtcggcatgcgtgcgcaccgccacgtagtcgagctcctgcaatgcctcgagcagcgcctgcccgctgcgccgccgcttggcgaagggatggcccttgcgcagcagcacgatgtagcggtctttcagcaactgggcgcgctgcgtgtccttcaccttgggcaggaaaccgaaggcgaagtcgacccggccgctgtcgagcgccgcggcaatgtcgccggtggccagtggcatggtctccacccgcacgctcggcgccagctcgcgcagccgcgccatcagcgccggcaggaagcggccctcgccgatgtcgctcatgtggatgcgaaacagcttgcgcgacgtcgccgggtcgaagcgctcgggctccgccagcgcctgctgcagcatggccagcgccgcctgcaccggcaccgccagccgctcggcccgcggcgtgggcgccacgccgccgggggtgcgcgtgaagagcgcatcgcccagcaagaggcgcagccgcgtgaggccgtggctggccgccggctgcgtgagccccagggcatcggccgcacggctcacgctgcgggcccggaagaccgcatcgaagagccgcagcaggttgaggtccagcttttcaatatgcatggcgtttatgtcgcatagcttgcttattttattgatgtatggcggcgcggcgaccacactgcgcaacccccaaaagaaaagagacacgatggaagtttcattcagcaaggaagtcgagttgctgcgcctcggcgccggcgacaccttccacggcgagggcatcctcgccatcaccaagggcctgttgcaatccggcgtggcctatgtgggcggctaccagggcgcgccggtgtcgcacctgctcgacgtgatggtccagggcaaggcctacatggacgaactcggcgtgcacgtggaagcctgctccaacgaggcctcggccgcggcgatgctcggcgcgtccattcactatccgctgcgcggcgcggtcacctggaagtcaatcgtcggcaccaacgtagcggccgatgcgctctccaacctgtcgtcgcccggtgtcaccggcggcgtgctggtggtggtgggcgaggactacggcgaaggcgccagcgtgatccaggagcgcacgcatgcctatgcgctcaagtcgagcatgtgcctgctcgatccgcggcccgacctgggcgtgatggtgcgcatggtcgaacacggctttcggctctcggaggcttcgaacatgccctgcctcatggagctgcgcatccgcacctgtcacgtgcgcggcagcttcgagtgcaaggacaacatcgcgcccgcggtgtcgacccgcgccttgatgagcgagcccgcgggcttcgactacatgcggctcgcgcatccgcccgtcacctttcgccacgaaaaactcaagggcgacgaacgcattccggcggcgcggcgctacatcgtcgaacacgggctcaacgagttgatcccgggcggcagccatgccgacctcggcatcgtggtgcagggcgggctctacaacgcgctcgtccgcagcctgcagcagcagggcctcgccgatgcgttcggcgaaacggacattccgatcctggtgctgaacgtgacctacccgctggtgcccgaacaggtggccgccttctgcgtgggcaagcgcgcggtgctggtggtggaagaaggccagcccgaatacatcgagcaggacattgccaccctgctgcgccggcgcgacatccagacgccgctgcacggcaaggacatgctgcctgcagccggcgaatacggcgtcgaggttctctcgggcggcatcggcacgttcgcggcaaagtacatcgaggccggcgaagccttgtcgtccgcgaaggcctggctggccggcaaccgcgaacgccgcgaggcggtggcgcgccagctctccgtgcccttgcccaaccggccgccgagcttctgcatcggttgccccgaacggccggtgttctcggcgctgaagctcgcgcagcaggagaccgggtcggtgcacatcgcggccgacatcggctgccatgccttcggcaccttcgagcccttttcgatgggccactcgatcctcggctacggcatgagcctggcaagccgcgcgggcgtggcgccgatgatgaaccgccgcacgctgtcgatcatgggcgacggcggcttctggcacaacggcctgctcacgggcgtgcagagcgcgctcttcaacgacgacgacgcggtgctgctgatcttcaagaacggctacacctcggccaccggcacgcaggacatcatctcgacgcccgacgacgaaacgaaggagcgcgccgtcgacaagcagcagagcctggtcgacaagaaccagaccatcgaggccacgctcaccggcctgggcgtgaaatggatgcgcaccgtgaccacctacgacgtggagcgcatgcgcaagaccctgaccgaagcgctcaccagcgacttcaacggcctgaaggtggtgattgccgaaggcgaatgccagctcgagcgccagcgccgcatcaagccctggattgcaagcctcttgaagaaaggcgagcgcgtggtgcgcgtgaagtacggagtggacgaagacgtgtgcaacggcgaccacgcctgcatccgcctctcgggctgccccacgctcacgctcaaggacaaccccgatccgctcaaggtcgatcccgtggccacggtgatcgacggctgcgtgggctgcggcctgtgcggcgagaacgcgcacgcggccacgctgtgcccgagcttctatcgcgccgaggtggtgcagaacccgaagtggcacgagcgcctgctgcattcgttgcgcggcgcgttcgtgcgagccctgcaacccgcatgaagggcgacgacatggaacgcaaccgtcccctcaccctcctcgtctgcgcccttggcggcgaaggcggcggcgtgctcaccgaatggctggtcgacatcgcccgccatgccggctatgccgcgcagagcacgtcgattcccggcgtggcgcagcgcaccggcgccaccacctactacatcgaagtgttcccggtgccgctcgcccagctcgacggcaggcgtccggtattcagcctgagcccggtgcctggcgcgctggacgccatcgtgtcgtcggagctgctcgagaccgcgcggcagatcggcaacggcatgagcgcgccgatgcgcacgctggtcatcagctcgtcggcgcgcatcttcaccacggccgagcgcatgcagcccggcgacggccgcgccgatgcgcagcaactgctcgacgtggtcaaggccttcagccgcgaacaccatgtgttcgacatgaacgccgtagcgcgcgaggccggcacggtggtcagcgccgtgatgctcggcgccattgcgggcagcggcctgtttccgttcccgcgcgccgcctacgagcacgtggtgcgcggcggcgacgcgagcgcgccgcaaaagctgggcaagatagcggccgcgagcctgcgcggatttgccgccgccttcgatgcggtgaacgcgccgcgcgcacaggccgccttcgtgagcagcgtgatggccggcgacaccagcgatgcgccgccaccgccgcgcgccctgcccgatgacctggcgcggcgctttccgcccgccgtgcacgacatgctcgcgctcggccatgcgcgcgtgctcgactaccaggacgccgcttacgccgagctttatgccgtgcggctggccaaggtgctcgatgccgagcgcgccgccgatcccgcaggcgcacaaggctttgccgtcacccgcgagaccgcgcgctggctcgcgctgtggatggccttcgacgacatcgtgcgcgtggccgcgctcaagggccgcgccagtcgtgcgcaacgcgtgcggcacgaggtgcgcgcggccgacgaagacatcgtgaaggtctacgaccacttcaagcccggcaccgccgagttcgccgcgctgctgccgccagccttggcacgccgcgtgcaggcctgggaccggcggcgccaggcaggaggcagggagccctgggcgctgccgctcaaggtgggcagccactcggtgttcggcatggcgtcgctgcggctcctgtcttcattcaaatggctgcgccgccgcggccagcgctttgccgaggagcaggcgttgatcgaacgctggctcgcggctgtggagagcggcacgcgcgaagcctggacgctgggccgcgagttggcgctgtgcgggcggctcatcaagggctacggcagcaccaacgaacgcggcaagcacaacctgctgcacatgatcgacgagctcgcgggcggcgcggccctgccggcgcccacgcgcgccgacgcgattgccgcggcgcgcgaagcggccctggcggacgaaggcggcaaggcgctcgatgccgcgctggtgagtcacggcgccgcgccgcggccggtgcaggctcagccgatacgctggatgaagcggccgcccaccaccaccctatcctgaattcataacaaccaaggagacacgaccccatgccccaccacgcccttccctggcgacgacgcctgctgttcaccgccgcctgcgcgctgctggcctgcacgcacgcacagacccatgccgacacctggccctccaagccgatcaaggtgatcgtcaacttcccgcccggcggcgccgcggaccagatcgcgcgcgcagtctcgcagccgctgcaggaggcgctcaagcaaccggtggtgatcgaaaaccgcgccggcgccaacggcaacgtcggcggcgaggcggccgcgcgcgcgccggccgacggctacacgctgctcatgagttcgggcggcatggtgtcggtgaatccgcacctgtatgcgcgcatgagcttcgacccgtcgaaggatctggtgcccgtggcggcggccgcgcgcgtgctggtgttcctggtgaccaagccctcgctgccgcccaccaacgtgcgcgagttcatcgcctacctcaaggccaatccgggcaagctctcgtacggctcgccgggcaacggcagctcgccgcacctggcaggcgaaatgttcaagagccaggctggcgtcttcgcgctgcacgtgccctaccgcggcgccgcgcccgcgcttcaagaccttctggcgggccagatcgactacgccttcgatcccggcatcggcctgcagcaggtgcgtgccggcaagctccggctgctggcggtgggaagtccgcgtcgctcgcctcagttcccggacgtgcccacgctcgacgaagcgggtttgcgcggcttcgatgccgacaccgtgttcggcttctacgcgcccgcgggcacgccgccggaagtcgtggcgcagctgaatgcgcagatcaaccgcgcgcttgcgctgccggccgtgaaggagcgcatcgcctcgctcggcggcgaagcggtgccgggctcgccggccgagttccaccagcgcgccgcggccgattcgcagcgcttcggtgcggtgatccgcgaccgcaagatcagtgcggactgagcgcgcgcttcgcgcaccgattgccgacgaaaatgagcccatgagcagcagcaaggaaatcatctacaccgcacgcgtcgagttcggcgactgcgaccccgccggcatcgtctggtttcccaacttctttcgctggatcgatgcggcctcgcgccacttcttcgcagaatgcggcgtgccgcgctgggaagaaacggcgcagatgctgggcgtcatcggcacgccgctggtcgacacgcacacgcgcttcgtcaaggccgcgagctacggcgacacgctgcagattgcggtgcgcatcaccgagtggcgcgacaagagcttcgtgcagacctaccgcgtggcgcgcggcgaggatctgatcctcgaatgcgaagaggtgcgcatctttgccgcgaagcgcgagggcggcggcatccgcgcggtgccgattccgccatccattcgtgcgctctgcgaataggccccggtcttagaatgaaccgatgaactggcgcactcttcttccccttgccctgcttgccaccggctgctcgtcaccccccaacgaggtggtgccgttccgcgatggggccttgcgtgcccccagctacacccaggccgccgactattgcagcgccaagcgcgcaacgccgcgctggctcggcaaggcacctgcggaatctggcgttctgttccagtgctactgagcttcgcggcccatcgcgaggtgtcttgttgagcaccgcgccaaagccctgcgcaatgccgagccaaagggttgacggccctcatgacgcagtgcaacaatcctgcatctttacttcggagccccgtgcgtggacagtgccagttggatcagtgacaagacgcgtgcctcggcaggcgtgacacacccggccctctagcgcaggctcttttgcgctgcggccgccgtgcacgcagcgtgacccgttcgccattcaggcaaagcggttctcccctcccgaatcccgtcgttctccgtcactgacttattcagtcagcttgcgtgtgtccgtgcacgaggcccttcatcgcgaaggagccttgccatgcgtcaaatccaatctcgtcagcagcagcaacagcagcagccggtgcaggaatccgttcgcccgtcggcgcacgtgcccgcgcgcgccgcggccaccaagcaagacgtcgagaacgagatgctggaccgcgcggccgcgctctggaccacgcggcgcatccgcagcttcttcctgctgctcgagcaaccctcccgcaccacgcaacgctgacgcgtcgccccaccccgcaccgctaggcaaccaagaaacaaggaggcctcatggaacccgcttctcattggcgcccctgcgcgccgcccatgttccgaccgatcgataacaacgaaatgcagcgcactgcgccgcaaggggattcccacgcctgattgatggaggcgggaggttcttcccttcgcggcccgcgccgcgaaggaaaaaaagtgaagaacgtcctgaagtcctttttcgagagctttctgcgcagccgccgcatgctgcatcatttcgagcgctggcagacgctgctgggctccaagccggtgggcgtggcctcggccgccatgccggccgatatcgccaaggcactggccgccgcatcccacaccaatgccggcgagctgctctcaaggctcgacagttcgccgcagggccttggcgaaacccaggcacaggtgctgcgcaagcgcctcggcagcaacgaggtgcgccacgagcagccgctgccgtggtggacgcatctgtggcagtgctaccgcaatccgttcaacctgctgctgaccgtgctggcgctgacctcgtacgtgaccgaggacatgaaggccacactcgtgatcggcagcatggtggtgctgtcgaccgtgctgcgctttcttcaggagtcgcgctccaacaaggcagccgagcggctcaaggcgatggtgagcaacaccgctaccgtgctgcggcccgagcccgacgcagccgcgggcgcgcggcgtgtcgaagtaccgatgcgcgacctggtgccgggcgacgtgatcgcgctctcggccggcgacatgatcccggccgactgccgcctgctgggtgccaaggatctgttcatcagccagtccgccctcaccggcgaagccatgcccgtggagaagttctccatcgaccgcggcggccctgaagccggtgtcctcgagcgcgagaacctgcttttcatgggcaccaacgtgatcagcggcaccgccaccgcgctcatcgtgcacaccggagaccgcaccttcttcggtgctctcgcgcagcgcgtgacggccgccgacaacggcaccagcgcgttccaggccggcatcaaccgcgtgagctgggtgctgatccgcttcatgctggtgatggcgccgctggtgctggtgatcaacggcgtggccaagggcgactggtgggaggcggcgctgttcgcgctgtcgatcgcggtcggcctcacgcccgagatgctgccgatgatcgtgaccgcgacgctcgccaagggcgcagtggtgatgtcgcgccggaaggtgatcgtgaagcggctcgaggccattcacaacttcggcgccatggacgtgctgtgcaccgacaagaccggcacgctgacgcaggaccgcatcgtgctggagcgccacaccaacgcgtggggtgaagtgtcggaccacgtgctgcagctcgcctacctgaacagctttcaccagacgggcctgaagaatcttctggacaaggccgtgctgaatcacgccgagatgcagcccgggacgccgctgcagacggcctggcgcaagatcgatgaagtgcccttcgacttttctcgccgccgcatgtcggtggtggtggagaacggcggcagcgagcacctgctgatctgcaagggtgcgctggaagagatcctgtcggtatgcactttcgtcgagcgaggcgccgaggtgctggcgctcgatgccgagctgctcgcgcgcatccatcgcgtggcgtcggagctgaacgcgcaggggctgcgcgtggtggcggtggccagccaggcgctgaaggcggaagcgcgcaagcccgcctacggcgtggccgacgaatcagggctcacgctgctggggtacgtggcgtttctcgatccgccgaaggaatccaccgcccccgcgttgcgcgcgctggctgaccacggcgtggcggtgaaggtgctgacgggcgacaacgaactggtcacgcgcaaggtctgcggcgacgtgggcatcgaagccggccatatcgtgctcggccgcgagatcgaggacctgcgcgatgacgaactgcgcgcgctggtcgagcgacaccaggtgttcgccaagctcacgcccgcgcacaaggaacgcatcgtgcacgcgctgcatgccaacgggcacgtggtgggcttcatgggcgacggcatcaacgatgcaccggcgctgcgcgccgcggacatcggcatctcggtggacggcgcggtggacgtggccaaggagtcggccgacatcatcctgctggagaagagcctgatggtgctggagcaaggcgtggtcgagggccgtcgcacgttcgccaacatgctgaagtacatcaagctcacggcgagctcgaacttcggcaacgtgttctcggtgctggtggcgagcgcgttcctgccctttcttccgatgttgccgctgcacctgctggtgcagaacctgctgtacgacgtgtcgcagatcgcgattccgttcgacaacgtcgacccggagttcctgcgcaagccgcagagctggaacccggccgacctgggccgcttcatggtgttcttcgggccgctgagttcggtgttcgacatcatgacctacgccgtgatgtggttcgcgttctcagccaacacggtggcgaaccagaccttgttccagtcgggctggttcatcgaaggcctgctgtcgcagacgctgatcgtgcacctgatccgcacgcgaaagatcccgttcctgcagagccgcgcggcctggcctctgctggcgatgggcgctgccattgccgtggccggtatctggctgccgatggggcggctcgcgcactacttccggctgcaggcgcttccgctggcctactttccgtggctggcggcgatgctggccggttatgccgctctgacgcaaacggtcaagggctggtatgcgcggcggtatgggtggcagtgacgagcgagtgttcttgttccttttgttcaggggtcttttgttcagggcgcgtgcacaggccaccgggtactcccctccgcgaatgtcccccgccttcggctcctcctttatttcgctgcggggagcacccggcgccctgtgcccactgggcgctgtgcttattccgctcgatcaaacaccgccccgagcaacgatcccgtcgatggggtgccttgcgcagcgaaataaaggaggaggccgcaggccgggggacattcgcggagaaaggtaccccgtcggcgggagcgccgccctgaacaacggcataaaaaaagcggcaccgccgaagcgatgccgcctttccagaaaccaagcggactgaacgagccgctcagacgctcatgatcgaaacagccttggtgttcaggtaagcctcgagcgcctcggggccgccttcggagccgtagcccgaatccttcacgccgccgaacggcatttccggcgagggtgcggcgggctggttgatccacagcatgccgagttcgagtttctggctcaacaggtgcgcgttcttgatcgacttggtgaaagcgtagcctgccaggccgaacggcaggcggttggcttcggcgatggcttcttcgagcgtgtcgaagccgcggatcgccgcgatggggccgaagggctcgttgttgaacacgtcggcatcgagcggcacgtcggtcagcaccgtgggcgcgaagaaattgcccgtgtcgccgatacgctcgccgccggcggccacggtggcgcccttcttgcgcgcatcgtccagcacgtgggccatggccgtgaggcggcgcgcattggcgagcgggccgagggtcgtgccttcggccaggccgtcgccgagcttcaggccttcggtgtacttgaccagcgtgcgcgcgaactcctcgcgcaggctgttgtgcaccaggaagcgggtgggcgagatgcagacctggcccgcgttgcggaacttggcggcgcccgcagccttcacggccagcgccacgtcggcgtcttcggccacgatgaccggtgcgtggccgcccagctccatggtgacgcgcttcatgtgcgagccggccagcgcagccagttgcttgccgaccggtgtggagcccgtgaaggtgaccttgcggatgatcgggtgcgagatcaggtagttcgaaatctcggccgggttgccgaacaccaggcccacggtgccgggcggaatgccggcatcgacgaaagcctgcagcagcgcggcgggggatgccggggtttcttcgggcgccttcaccaggaacgagcagccggtggccagcgccgcgccgagcttgcgcacgatctggttgatggggaagttccacggcgtgaacgcggcgacggggcccagcggctccttgatcaccagttgctgcgcggccaggttgcgcgaggggacgatgcggccgtagacgcggcggccttcgtcggcgaaccattcgatgatgtcggccgcggccagcgtttcgcccttggcttcggccagcggcttgccttgttcctgcgtgagcagcttggcgatttccggggcgcgttcgcggatcaggccggcggcgcggcgcatcacggcggcgcgctcgttggcgggggtgttgcgccacttttcaaagccgcgctgggcggcggccagggcgcgatcgaggtcggcgatgctggcatgcgccaccttgccgatggccttgccggtggccgggttcacgacgtccagcgtcttgccgccggtggcgtcgacccattcgttgtcgatcagcaggcgggtgtcggtgtaggtggcggtcatggcgaacttttccttcgaggactggatgatggtgaaaaagggggaaatctggatgcgcggcgcggcaccccgaaaggtgcgccttgcgacagcggcggcaatttgccgccgccgggtgcataggttaacccgacttcacaaagcccgccggagccggggaaccggcccccctcccgtcgctacaggatcaggagcgcgcgaaagtcgttgacgttggtgttcgtgggcccggtcacgaacaggtcgccgatggcgtcgaaatagccatacgcgtcgttgcggtcgaggtggtccgacagcttcctgccggccgcggcagcgcgcgccagcgtgtcgggcgttacgaaggcgccagcgttgtcttccacgccgtcgatgccgtcggtgtcggcggccagcgcccacacctgcggctggcccatcagtgcgccggccagccccatgcaaagctcgccggcccggccgccgcggcccttggcctggccgggctggcgcgggcggatggtgacggtggtttcgccgcccgaaagaatgacgcagggccgcgcaaatggctggccgcggtgcgacacggcgcgtgccaatgcggcatgcaccttgccgacttcgcgcgattcgccttcgatctcgtcgctgaggatgtgcgcttcgatgccggcctcgcgtgccacccttgccgctgcttctagtgattgctgcggcgtggcgatcatgtggacttcatggcccttgaacacggcgtcgcccggcttcggggtttcgagcgcgccgctttcgagttgcgcgcgcaccggcgccggcacctcgatgccgtagcggtcaagaatggcgagtgcatcggcgcaggtggtcgcatccggcaccgtggggccgctcgcaataacggccgcgtcgtcgcccggcacgtcgctgatggtgagcgtcaccacgcgcgccggcgcgcaggccgcggccagcctgccccccttgatacgcgacaggtgcttgcgcacgcagttcatctcgccgatgccggcaccgctgtcgagcagctgcttgttgatgcgctgcttgtcggccagcgtgaggccttcggcgggcaagaccagcagcgacgagccgccgcccgagatcaggcacagcacgaggtcgtcggccgtcagcccctgggccaacgcgaggatgcgctcggcggcctgctgcccagccgcatcgggcaccggatgcgcggcttcgacgagttcgatgcgctgcggcacgccttcgggccgagccggaatgtggtcgtagcgcgtgacgaccaggcccgacagcggcgcgtcggccggccagagggcttcgagcgcctgcaccattgagccgccggccttgccggcgccgagcaccagcgtgcggcccttgggcggcggcggcaggtgggcgcccagcgtggacagcggcagcgcgcggtccaccgccacgcggtagaggtgctcgagaaaggcgcgcggtgcttcgcgcggatcgggcacgggcccgatggacgaggtcgatgcggtcatggcttgcgttgtctccatccggcgattgtgcggcgaacggcggcccgctctcttgatcgcggtctattcctgcgtctagttcgtcttggcgccggcctggaaccaccggccgatcagtgcgcgctcttcttcggtgatgccggtcgagttgttcatcggcatgatcctgctcaccaccacctgctggtagatggcctgcgcatgcgccgccacctggtcgggcgtgtcgacgcgcacgttcttcatctgcacggccgcaccatggcacatgaagcagcgctgctcgagcaccttctgcacgtccttgaacgccaccgccggtgcggccgccgaggcggcgggcgcggccaccggtccgggtttcatccagacgatggtgagccccaggaccacgatgccgatcagcgcatagggcagcgggttgcccgcgttgccgagcttgaagcggtgccgcaccacgaagaactgacggatggccgcgccgccgagcatgatcagcagcagcacgatccagttgtactggtgcgtgtaggtaaagctgtagtggttgctgagcatcgcgaacagcaccggcagcgtgaagtaggtgttgtgcacgctgcgctgcttgccgcgctgcccgtgcaccggatcgaccgaccggccttcgcgcagggcctgcacgttcttgcgctggcccggaatgatccagaagaacacgttgccgctcatcgtcgtggccatcatggcgcccaccagcagaaaggccgcgcggcccgcgaaccactggcaggcaagccaggtcgcgaacacgatgaagacggcgatcagcacgccgacgatggtgtcgccgttcttgcggcggccgaagatctggcagatgccgtcgtacaccatccagaacacgacgaagaaagccagcgccacgccgatggcggcgccgggctgccagtccatcttggtcttgtcgatcaggtacgtgctggcgttccacaggtacgacatggtgaagagcgcaaagcccgtgagccaggtgctgtagctctcccaatatgaccagtgcaggtggtccggcagcttcttgggcgccagcgcgtacttctgcatgttgtagaagccgccgccgtgcacggcccactgctcgccgcccacgcccttgtcgagcgattcggggtcctgcggcttttcgagactgttgtccagcatcacgaagtagaaggaggcgccgatccaggcaatggcggtgatgacgtggacccagcgcagcagcaggttggcccagtcgaggtaatagctttccatgtgtggtgctctttctcaaccccgtcggcgcgtgggggcgccgccaaggggtttcttcagcctgctcaccactgcgggcgctgtaagcagagaaagtgccgcgaacgcaggctccatggaatgggcctcgctccgctgcggcttgttgtggaccgaaagtgtatacagttttggcaaggggcggaatgcttttttggggcgttgccgccgggaaaaccctgttcagcccagggattgcaacaactgtgccgccaccgcgacggcgatcacttcaggctccttgcccgtgatgcccggcacgccgatggggcaggtgatgcgcgccagctcttcgggcgtgaagccgcgcgcctcgagccggtggctgaacgtggcccatttggtcttgctgccgatcaggccgatgtacggcaggtcgtcgtgcgtgcgcaagcgcttcaggcaggcgatgacgatgtccaggtcttcggcgtggctgaagctcatgatcagcacccggctgcccggtgcgagtgcggccacggcatcctgtacgggctccgaatgctcggtgtcgatctgcgccggcagggcatctggaaacacgccgtcgcggctgtcgatccagcgcacggtgaacggcaggctggccagaagccgcgccagcgccgcgcccacatggccgccgccgaacagcgccaccggcttgagctgcgcgaccaattcgcgctgcaacgccggtgcatcggcggacgtgatgcggcgataagagagaaacaccacgccgccgcagcactggcccaggctcgggccgagcggatagcgccggatgccgtcgatggcgcgctggccggcaagcagctcgcgcgcttcctgcgtggcctggaactcgagctggccgccgccgatggtgcccgtgagcccttcggcccacacggccatccaggtgcccgcctcgcgcggcgccgagccctgcgtcgattcgacgcgcaccagcaccgcgtcttcctgcgcgagacgggccaccagctgatcgacaaagccgttcatttccgataccttagtttgcacaagactcacgtataacccgatgatgaaacgtcagcctacgccgcgccgccttgcatgggcgataaccgcactttcttccgccctctggctcgccggctgcggcggccccaaggccgttcccggccagttgagcgaggtcaagaccgaaccggccgggccggcagccattctcggcgccgtgccgcgcgcatcgaacgcggccaccgcgcgcgagtaccgccgcgacgccgcgcgccacatctacgaggccaacaagtcccgcatctacagcggccagctgccgcccatgctctatgccgtcggcacgctgcaagtccatctcgatgccagcggcaaggtgctgtcgctgcattggatgcgcgcgcccaagcacgcgcccgaggtcatcgccgagatcgagcgcttcgtgctgaaggcctcgcccttccccgccgccacacgccttggtgcggtcacgtggaccgacacttggctgtgggacaagagcgggcgtttccagctcgacacgctcaccgaaggccagttgcaaggcgactgacctcaggagccgcggtaggtggagtagctccacggactcacgagcagcggcacgtggtaatgctggtcggtgtgcgccacgccgaagtccagcgacaccttgttcaggaaattgggctcgggcagcttcacgccgcgcgccttgaaataacccgccacgtcgaacaccagccgataggtgccgaccttgagcgagtcgttgtcgtagagcggcccgtcgctgcggccgtctgaattcagcgtgaagcgtttcaccagcgtggcggcgtcgccctcggtggtgtaaagcgccacctccatgccggccgcggggccgccgtgcatcgtgtcgagtacgtgggtgctcaggcccatggggcgctccttcatcaaaacaaaatcgtgcgggaaattccggtggacaaaagtgtatacagttaccggctttgggtctatcatgaaaaacatggagtcctccaccacacgttcgatcgtcgacgcgctgaccaaggccatcgtcgagcaccggctgcagcccggcaccaagctggctgagcaaaagctggccgaccacttcggtgtgtcgcgcacgctggtgcgccaggcgctgttccagctgtcgcagaacaagctcatccgcctcgagcccgcgcgcggcgccttcgtggccgcgcccgcggtcgacgaggccaggcaggtgttcaaagtgcggcgcatgctcgaggccgagatgacgcgcgagttcgtgcgcaccgtcacgcccgcgaagatcaaggcgctcaaggagcatgtggcgctcgaaaaatcggccgtgtcgggcgaagacatctcgggccgcacagagctgctcggcgacttccacgtgcgcatggccgaactcatgggcaaccaggtgctggcgcaaattctcggcgagttgatctcgcgctgcgccctcatcacgctcatgtaccagagcaccagcgcggccgagcactccaacgacgagcacgccgacatcgtgaaggcgctggccgcccgcgacgaagagcgcgccgtgcgcctcatgaccgaacacctggaacacgtcgaggccaacctcacgttcgaccgcaaggttccgaccaacgacatctcgctcgccttgtcctgatccacgccatgaccgtctacgacaccacccagccctacccgcgcgacctcgtcggctacggccgcaatccgccgcacgcccaatggcccggcggcgcgcgcatcgcggtgcagttcgtcctcaactacgaagagggcggcgagaacgccacgctgcacggcgacgcgggttccgaacaattcctctccgagatgttcaacccggccagctttccggaccggcacatcagcatggaaggcatctacgaatacggctcgcgcgccggtgtgtggcgcatcctgcgcgagttcgaaaagcgcggcctgccgctcaccgtgttcggcgtgggcatggccctgcagcgctaccctgagctgaccgccgccttcaaggagctgggccacgagatcgcctgccatggctggcgctggattcattaccagaacctggacgaagccaccgagcgcgagcacatgcgcctgggcatggaagccatcgaaaggctcaccggcgaacgcgccctgggctggtacaccggccgcgacagcccgcgcacgcgccgcctcgtggccgactacggcggcttcgagtacgacagcgactactacggcgacgacctgcccttctggatgaaggtgcagaagaccgacggcacggtggtgccccagctcatcgtgccctacacgctcgactgcaacgacatgcgctttgcactgccgcaaggctattcgcacgccgacccgttcttccagtacatgaaagacaccttcgacgcgctctatgccgaaggcgatccgcaaggcgacaacagccccaagatgatgagcatcggcatgcactgccggctgctcgggcggcccggccgcattaccgcgctgcagcgctttctcgatcacatcggccagcacgacggcgtgtgggtctgccggcgcctggacatcgcgcgccactggaagcagatgcatccgttcgaagcggccaccaaaggaagctgaccatgagcctcaccatcgaacaactgaacgcagccgcgcccgacgaagccgtcgcgctgctcgacggcatctacgagcactcgccctggatcgcccagcgcgcgctggccgcacgccccttccgctcgctcgcgcacctcaagcatgcgttggtgcaggcgctggccgcgtcgtcggccaacgagcagatcggcctgattcgcgcccaccccgagctcgcgggcaaggccatggtcagcaagacgctcacggccgaatcgaccaacgagcaaagcaaggccggcctgaccgactgcacgcccgaggagtttgcgaagatccagcaactcaacgccgactacaacgcgaagttcggcttcccgttcatcctcgcggtgcgcggcccgcgcggcaccggcctttccaagcgcgagatcatcgacaccttcgagcgccggctgttcaaccaccccgccttcgaactcggcgaggcgctgcgcaacatccatcgcattgccgagatccggctcgacgacaagttcggtgccaacgtctcgctcggcaacgacgtgtgggactggcaggaagcactctccgttcacaccgatcccggctatgccgaaaagggccagctcaccgtcacctacctgaccgatgcgcaccgcgcctgcgccgcgcagatctccggcctgatgcgccaatgcggcttcgactcggtgcacatcgatgcggtcggcaacgtcgtcgggcgctacgagggcgccacgcccggcgcaaaggcactgctcaccggctcccactacgacaccgtgcgcaacggcggcaagtacgacggccgcctgggcatcttcgtgccgatggcctgcgtgcgcgagctcaagcgccaaggcaagcgcctgcccttcgctttcgaggtggtgggttttgccgaagaagaaggccagcgctacaaggccacctttctcgggtcgggcgcgctcatcggccacttcgatccgcgctggctcgaccagaaggacgccgacggcatcaccatgcgcgaagccatgcagcaagcgggcctgaagcaggaagacattccgaagatccagcgcgatccggcgcgctacctcggctttgtcgaagtgcacatcgagcagggcccggtgctcaccgagctcgacctgccgctgggcatcgtcacctccatcaacggcagcgtgcgctacgtgggcgaagtgatcggcatggccagccacgccggcaccacgcccatggaccgccgccgcgacgcggccgctgcggtggccgaactcattctgtacaccgaacagcgggcggcgaaggacggcgactcggtcggcaccgtaggcatgctcgaagtgcccagcggctcgatcaacgtggtgccgggccgctgcaagttcagcctcgacctgcgcgcacccaacaacgcgcagcgcgacgcgctggccaccgacgtggtcgaagaactcaaggccatctgcgagcgccgcggcgtgcgctacgaactcgaggagaccatgcgcgctgccgctgcgcccagtgcgcccgcctggcagcagcgctgggaaaaggctgtcgatgcgctgggcattccgctcttccgcatgcccagcggcgccggccacgatgcgatgaagctgcacgaagtgatgccgcaggccatgctcttcgtgcgcggcatcaactcgggcatcagccacaacccgctcgaagcgagtaccaacgacgacattcagctcgcggtggaggccttccgccacctgctggacaacctcgccgccgaacaagctcactgaaaagaaaaatcatgaccgactacgccaagctcgacgcctggatcgacgcccacttcgacgaagaagtgcagtttctgcagcagctggtgcgcgtgcccaccgacacgccgcccggcaacaacgcgccgcatgccgagcgcacggccgagctgctgaaagacttcggcatggaagccgagaagcacgcggtgccggagcaggaagtaaaggactacggcctcgaatcgatcaccaacctgatcgtgcgccgccagtatgggagcggtggccgaaccgtggcgctcaacgcgcacggcgacgtggtgccgccgggcgacggctggacgcacgacccctacggcggcgaaattgccgacggcagcctctacggccgcgccgccgccgtgagcaagagcgacttcgcgagcttcaccttcgcgctgcgcgcgctcgaagccgccgccaggcccaccaagggcagcgtcgagctgcacttcacctacgacgaggaattcggcggcatcctcggcccgggctggctgctcaagcagggcctgaccaagcccgacctgatgatcgcggccggtttcagctacgaggtggtcacggcccacaacggctgcctgcagatggaagtcacggtgcacggcaagatggcgcatgcggccattcccaccacgggcgtcgatgccctgcagggctcggtcaagattctcaacgcgctctacgcgcagaacacgctctaccagcaggttacgtcgaaggtcgaaggcatcacgcacccgtacctcaacgtgggccgcatcgaaggcggcaccaacaccaacgtggtgcccggcaaggtggtgttcaagctcgaccgccgcatgatccccgaagagaatccggtcgaggtcgaggcgacgatccgcaaggtgatcgccgatgccgcggccgaaagcgccggcatcacggtggagatcaagcgcctgctgctcgccaattcgatgcagccgctggccggcaacaagccgctggtcgatgccatccagaagcacggccaggcggtgttcggcgaaccgatcaaggccatgggcacgccgctttacaccgacgttcggctctatggagaagccggcattcctggcgtgatctacggcgcggggccgcgcaccgtgctcgagtcgcacgccaagcgcagcgacgagcgcgtggtgctcgaagacctgcgccgcgccaccaaggtgattgcgcgcacgctgagcgacctgctggcctgagcttttattacgcggcggtgcgtctccgaaagcccgaccttgaacaccccctccaccgttccctacaccggcatctggcccgccctgctgaccccgctcgacgagaagctcggcatcgacaccccccgcttcgccgcacacgccttgcgcctgctcgacgccggctgcaccggcgtgacgcctttcggcacgaccggcgaaggcccctccttcagcgtgagcgagcggatgaacgcactggccggcctggtcgcccacggcgtgcctgccgggcgcatcctggcctctaccagctgcgccgcgctgcccgatgcgttcgcgctgacccggcatgcggtcgagctgggcgcctacggctgcctgctgctgccgcccttcttcctcaagggcgttcccgaccagggagtgatcgacgcctaccgatggatcatcgatggtgttgccgattcgaggctgcgcatcgtgctgtatcacatccctcaagtggcaggcgtcgggctgagccaccacgtcatccgcacgctgaagacgctctacccggacacgatcgtgggcctcaaggacagcagctgcaagcgcgaggattcgctggcctacgccgaggcgttcatgccgccgatgcaggtgtgggtgggcaacgagccggatctgcaaacgatggccgcgcgcggcagcctcggcgcggtgagcggcatcgccaacgtcatgccgcgcctcgtgcagcgcctggttgcgggctccacgcagcccgaggtcgatcagcagcgcgtgctggacctgctcaagattctcggcggctacggtttgacggccgccttcaagggcctgatggccatgctcgacgacgcaccgggctggatgcgggtgcggccgccgctggtggcgctggatgcggccgagtacgaccggctcgcggcgcagctgcgcgccttcggcatcgatcgcgaccgcgactgagtttggcccttgcgctgggggcgtccgacgcggcgcatcagtcgtcgcctacaaaggcgcgggggcatggacgtgcagcatggttgcatgaccgaacgcagttcaacaccccccaacgccacgatcccgctgaccgccgatgcccagtcggttgcgcatcgcttcgccgatgtgggcgggatgcagatcttctatcgtgaagccggcccgcgcgacgcccctgtgctgctgcttccacacggctatccctgctcgtcgttccagtaccgccggctcatgccggcgctggcggaccaatggcgcctcgtggcgccggactatcccggctttggcctgagcgacacgccgtccgctgatactttcggcttcgacttcgatgcctatgcggcctttctcgaagccttctgcgacaagctgagacttgatcggtacgcgctttatctgcacgactacggatcgcagatcggcttgcgcctggcgatccgccggcctgagcgcgtggccgcggtgatcatccagaacggcgacatctacgaagacacgctcggccccaagtaccgggccattcaagaatactggcgcgatccatcggccaggcatcgcgcggtgctcgaagaggccgtgagcgaagacggctttcgcgccgagttcgtcggcgaggtttccgccggacaggccacgcagattccgcccgacttgtggaagctgcactggcccttgatggacacgccgccgcgccgcaagctctcgctcaagctgatggaggggctgaagaagaacctcgaatggtttccgcgctaccaggcctatctgcgcgagcaccaaccgccggcgctcatcgtctggggacccaacgatggctacatgcccgaggcctccgcccgcgcttacctgcgcgaccttccaaaggccgagctggtgctgacggacggcggccactggctgctcgagacgcatctcgagcaggtggttccggtcatccgccggttcctgtccgcaggcccttcacgctgacggcaatctcccgcgtcacctggagaaacttctccacgtcggcggccgagtggcagtgcagtggcgaaacccgcaccgtgccttcgagcccgaaggaatcgagcatgcgcttcgagtagatgctgcttgccgcgcgctcgtacacggtgacgccgcgcttgccgtactcgaccaccgcctgcgtgcagtcgaggtgctcgaagccgatgccgatgatcaggtcgcgcctggtgaggtctggatgatcgaggaagactttcacgccttcgatattgcgcaggcccgtggccttgccgctcccgtcgagcagcgccgcgagcagggcccgctcgtgcagttcgatgtgcgcaatgcccgcctcgaacagcgctcggcgctcggtggcatccgaaaaatggccgccgagccagcacacgtagtcgacgatttcggtgagcacggcaaactgccagggcgccgaactgcccaggtcccagaagtcgggcttcttgcccgcgagcttgtggtgcggcagcagcgccgcgcgcaccgatacccatgagagtcccgagccacggcagccgaagaacttgtagggcgccatgttgatgccgtccacgggcgtcttctgcaggtcgatcaggccgtgcggcgcatgctgcacggcgtccaccacgatgtagagatcgggcttgatctcgcgcgcgcgccggacgatctgttccatgtcgagcttggcacccgagatgttcgatgcatagatcacgttgagcaggcaggtgttttcgtccaccagccgcacgatctcgtcggcatcgacgccgccggtctcggggttgctccttgccacccgcagctcgcggccggtcttgcccgcataaaggctcatggcgtcgaacgacgagggatgctcgagcacggtggtgaccatgttcgtgcccggcacgttctcggccaccgcgcgcaccatgtcgaacatcgcgcccgatgccgtcagcgatgcatagacgctgccgccccgcgcgttgaggatggtgcgcacgtcggccgcggccctggcctggatctgctgcagctcgacggccgtggcgtgaatgcgctccgcgttgtcgggaatggcatcgacctgcatgaagcgctcggccgcagccttcagccggaacgagccgcccgcgttgtcgaagtagagacgctcacgcccgtggtggtcgtggtcgacgtggagaaagcgctctttcacctcgcgcatcagcgcgtcggaaaacgccagcccgttggcatggtgtgtagttgccgacatcctcaaacgcccttgttgttggggttcttgtagacctcgcgcacggcgtcggacatcgggaagttgaggttcacgttgcgcggcggaatgggcgccatgaaccacttggcgtagagcttgtcgatggcgccggacttcatcatctcggtcacggtctggtcgacgatggccttgaactcggggtcgtccttgcgcatcatgatgccgtagggttcttgccgcagcacgtctttcagcagcttgtagtcggaagcgttgggctggttggcgatcaggccggccagctgcacgtcgtcgagcacataggccacggcgcggtcgctcgcgagcagcaggaaggcgtcggccgtgtccttgcccgcaatttcctgcacctcgatgttctcggtcttgcggaagccgcgcagcagctgcatcgaagtgctgccggccaccgtggcgacggtcttgccctgcaggtcggcgatcgagttgatgcccgagttcttcttcaccgcggcggtgatgttggtgacgaaatggctcggcgcaaagtcgacctgctgctggcgctgcaccgtgttggtggtggtcgcgcagtcgaggtcgaccgtgccgttctgcaccagcggaatgcggttggtcgaattgagcagcgtgtagcgcacctcgatcttctgaaggccgagcttggccttgatggcatcgaccaccttcaggcagatctcgttggtgaagccgatgggcgcgctttcggcgccggtcttgtaggagaacggaatctgcgtgtcgcggctgccgatctgcaccgtgccggtttccttgatcttgcgcagcgtggggctctcttgcgcggcggcagcaccgcagagcagcgcaatgctggcgccgagcgcgagggactgtttgaggttcatcgaatgttcctttgaggatgaggcaagaagtacacggggggcaggaccggagcgaatcttctgcgcaccttcaaatttctaaaagcgattttttgtgatcgaataacatgaataaaaggattcaatacaagggcgcgcaccatgatgaccttcaagcagctcgaagccctgtactggatcgccaagctcggcggcttcgcccaggcggccaaccagcttcacacctcgcagtcggccgtgtccaaacgggtgcatgaactcgagctgctgttcgacaccgagcttttcgaccgcagccagcgcaccgcgcgcctgactgaaaaaggcgaggagatgttcgtgctcgcggccaggctgctcgagcaacgcgacgccgccgtcgagcagttcggcaagccgggcgtggtggagcgccggctgcgcatcggcgtgaccgaactgaccgcgatgacatggctgccgcggctggtcggcctgatccagcagcactatcccaaggtcattctcgaacccgacgtcgacgacagcctccagttgcgcgacaagctgctggccgacgagctcgacctggtgatcgtgcccgacacctttgccgattcgcgcatgcagagcaaggccatcggccaggtgaagagcgcctggatgtgcaagcccggcgtggtgccggccaccggccgcatgcggctgcacgaactcgcgcggcaccgcatgctggtgcagggcaagaactccggcaccggccgcgcctacgacgcctggatgaaggaccagggcgtgcagccgtccgacaccatcgtggtgagcaacctcgtggcgctgaccgggctcacggtgtccgggctgggcgtgagctaccttccgcgccagtgcctggacccgctcgtttcggccggcatgctcgccgtgatcgacgtggtgcccgccctgccggtggtgcgctatgtggccatgcacaagggcgagcatcgcagcgcgctcacctcgtccatcgtgatgctggcgcaggaatgctgcgacttcacgcgcatgttccaggcccaggccgacgaagatcccgacgaatgagcaagcggctggtgcacacttgccactcgccttgtctctcaaccccctgccgcctctttcgcacatgaaaccccgcaagcaaacctcgtccacgcccaacatccgggtcgcgcccagcggggtgcacgggctcggtgcatttgcggcgcgcgacctgccggccgaggcattcctcggcctctacgaaggccggcgctacacgcagcaggagatcgcggccaagtcgtggaacgaccagctcacctacctgttcacgctctccaaccacgagacgatcgacggcgccaagggcggcaacggcacccgccacctgaaccacgcctgcgaccccaactgcgaggcggtcgaggaatacgacgacgcgggcgagctgatgctcaagttccagaccctcgtgccggtggacgcgggcgacgagctgttcatcgactattccctgaccgcggacgatggttcgccagccgaaaattatccctgccattgcggctcgccgaactgccgcgggaccatgctggcgccggttgacgcggaggaatgaccgcccgctgattcgaccgcggtcgaagtcgaaggcgccatggctgcgggccattggcgcctttttttgtgtcctccgagcgcctcagggaatgtacggatatatgaattgccggatgggcttgattgcacacgttttttgtatacaaataacgcacccgatacccggcgcggaattttgcgttggaaagcggtccctcaacccaccattcgcacgaggaaagacccatgagcacagtcgtcagccaggcccccgcgggggcgagcgaagccggccacgcgccgcatgccgaatccaacgcgctgatcaagcccggctacgacccgcggctgaccaacgaagacctggccccgctcaagaagcagacctggggccaatacaacatctttgcgttctggatgtccgacgtgcacagcgtgggcggctacatcacggcgggcagcctgttcgcgctgggcctgtcgagctggcaggtgctggtgtcgctgctcgtgggcatcgtcatcgtgcagttcttctgcaacctggtggccaagccgagccaggtgacgggcgtgccctaccccgtggtgtgccgcgcctcgttcggcgtgctgggcgccaacatcccggccatcatccgcgggctgatcgcagtcgcctggtacggcgtgcagacgtatctcgcatcggccgccttcatggtgctggcgctgcacatgttccccaacctcgcgccgtatgccgacgtggcccagcacggcttcgcgggcctctcgacgctgggctgggtggcgttcatgatcatgtgggtgctgcaggccttcgtgttctggcacggcatggaagccatccgcaagttcatcgactgggccggtccggccgtgtacgtggtgatggccgtgctctgcggctggctggtgtggaaggccggctggagcaagatcgacctgaacctgggcggcatcaagttccagggctgggacgcgctgccggtgatgctctcggccattgcgctggtggtgagctatttcagcggcccgatgctcaactttggcgacttctcgcgctacggcaagagcttcgacgcggtgaagaagggcaacttctggggcctgccgatcaacttcgttttcttttcgctgctgacggtgatcaccacggccgccacgctgccggtgttcggcgagttgatcaccgatccagtgcacaccgtgggcaagatcgacagcaccaccgcggtggtgctgggcgcgctgaccttcatgatcgcgaccatcggcatcaacatcgtcgccaacttcgtctcgccggccttcgacttctcgaacgtggcgccgcagcacatcagctggcgcacgggcggcatgatcgccgcggtgggttcggtgtttctgacgccgtggaacctttacaacagccccgaggtcattcactacacgctcgacgtgctgggctcgttcatcggcccgctgttcggcattctgattgccgactactacattgtgcgcaagcagcgcatcgacgtggacgcgctctacaccatgagcaagcagggcaagtactggtacagcggcggctacaacccgaaggcgatccaggcgctgatcccctccgcgctggtgccgattctgtgcgtgatggtgccggcgctgcgcggtggcgcgaactatgcatggttcatcggcatgggtctgggcttcgtgctgtacgtgctcgtgaaccgcaacaacaagacttgaaatactgaaagagaaaggccgcgccgtgcgcatcaagatcatcaatcccaacaccacctggagcatgaccgagaagatcggcgcctgcgcccgcgcggtggcgcacgccagcaccgaaatcgtcgcggtcagcccggccatgggcccggtctccatcgagagccactacgacgaggcgctggccgtacccggcctgctgcaggagattgcggccggcgagcgcgacggcttcgacggctacgtgatcgcctgcttcggcgatccgggcctccaggccgcccgcgaactggcgcgcggcccggtggtgggcattgccgaggcggcgatgcacctggccagcatgctgggcagccgcttcagcgtggtgacgacgctgggccgcacgatggggcaggcttggcacctggccgagatctacggcatggagcgcttctgcgccaacgtgcgcgcctgcgagttgccggtgctcgaactggaagagcccggttcgcgtgcgcgcgaacgcatcgtcgacgagtgccggcgcgcgctcgaagaagacggctccgactgcatcgtgctcggctgtgccggcatgaccgacctgtgcgagcacatcggcggcctgctcggcgtgccggtgatcgacggcgtggccgcgggcaccaagctcgtcgaatcgctggtgacgctgaagctttcgaccagcaagcgcggcgaactggcccacccgctgcccaagcgcatgacgggcgcgctcgaaggcttcaccctggtcggcccataagaagaacaagaacaagaagaatggcacgggcgtgccggcaatcccgctgagccacaatcccgacatgccccgcgccagctccaaatctcccgtctcccctgccaccgccgctcctgccgacaacggcgcggctgccgccgacaagggcagctccatcgaaagcattgcgcaggacattgccaccgccatcgtcgaaaagcgcctgccgcccggcacctggctgcgcgaggaagcgctgggccgcgtctattcggtgagccgcaccaagatccgcgcggccttgctcatgctgtcgaaggacaagctcatcgagatgattcccgacaagggcgcgttcgtctgccagccgacggtgcaggaggcgcgcgaggtgttcgcggtgcgccgcatcctcgaaagcgaagtggtgcgcctgttcatcgccaatgcacggccgcgcgactaccaggtgctggagcagcacatccgcttcgagcgcaccgcactgcgccagaccaccaccacgggcaccgtgcgcgagaaggtgctgggcgattttcacgtggcgctggccgaggccacgggcaacaagacgctggccgagctggtgcgcgagctggtggcgcgcagctcgctgatcgccatgctctaccactcgtcgaacgacccgcactgctcgtcggacgagcactccgatttcctgcgcatctgccgcaagggcgacgtggaaggcgccgtggcctgcatgaccgagcacctggagcgcatcgaggccagcctggagctcggcaccgagaagcccgaccgccagctcgacctggtgaaggccctgctcgcctgaaaaaggtctgcaaagcggccccaaggggccccggggagcctggggcgattcagtgcctggctttcggagagtgcttccttggcttgcgcgcaggagagccagccggtgcgacagcggccgttcccaggcgttccgcacctgcgatcagtccgtgcaggaacaccatgatcagccgtcccgagggatccgaacgagtggtcgtcctctgcaatgccagcccatgcgacagtgccatgaaggcagcggccagttcgtccggtgcggcagaaggcgtgcgcccgagcttgttgaacaactggccgatcacggcgccaatctcggaccggtgcttgtcccacaccttctggtactccgcagcgaacgtttgactgcggttggcatgcagctgcagctcgatggaaagcatgcaccaatcggcatcgtgattgagcgtggaagcccaggcttccagttcggcaagcatctgctcgggcttttgccgctcgttgcccatgaccttggaaagctgcgccgcttccccttccatatgccgtcgcagcagctccagcaggacgtcttccttgcttgaaaagttcgaatagaaggcgccttgggagtagcccgccttgtccgcaatgtcgcggatcgacgcacctccatacccgttcgacacaaacaagtgctgcgcggtttcgatcagacgctcgcgagtctgcgcccggctttcctcgcgggtcaggcgccttcctgctgtcgttgggctcatgcctcaaaagatatcacatgaactttggatatcgactggcgggcacctgcgtccgggggccaaggccggaaaccaaaggttcaaatatcacttgatatttcaaaatggcgacggtacattcaaaactcgtttgatttttgaaattcaattgatatggaaaaaaccaaggccttgaggtccgcgtttgtcaccggcgctaccggccttctcggcaacaaccttgtgcgcgagctggtcgcgcgaggcgtctccgtcaaggcccttgttcgctcgaaggccaagggccagcaacagtttgcaggggtgaaaggcgtcgagttggtgttgggcgacatggcggacgtacgcgctttctccaacgcactgcgtggatgcgacgtggtgttccacaccgctgcgttctttcgggacaacttcaagggcggcagccattgggaagaactcaagcgcatcaatgtggacggcacgcagcagctcatcgagcgggcatacgacgccggcatccggcgcttcgttcagacctcatccattgcggtgctgaacggcgagccgggcatgcccatcgacgagacctgtctgcgtgacctggcagatgccgacgacgactactaccgaagcaagatattggccgatcaggtcgtatcggcctttcttgcggcgcaccaggacatgcacgcgagctttgtcttgccaggatggatgtgggggccggctgatatcggccccacctcgtcaggacaattcgtcaatgacgtggtgcttggaaaactacctgggctgctgcctggcagcttttccgtggtcgatgcccgcgacgtggcgagggcgcaaatttcggccgcagaggacggacagcgcggcgaacgctacctggctgccggccgccacatgacgatgcaggaattggtgcccttggtagggaagatcgcgggcatcaagacgccgacacgcaatttgccctttccgctcttgtatctcttggcggcggtacaggaactctacgcgcggatcagcggcaagcccatcttgctcagcctggccactgtgcggctgatgcgcaaggaggcggggcgcagccacttcaaccacacgaagagcgagcaaaaacttcagctgaagtttcgtccgattgagcaaaccgttgccgatacggtcgcctggtatcgcggcaatggctggctgccaagtgcgtcgacccgatagcgccaagcagaccgcttcttcgccccggcaacgggcgtgagccaccaaacccaaccaaaggaaagaccgtgacgaacagattgattttgaaactcttgacggccttcggcgctgtttttcttgtcgcggcagcgccgcgcgaatccgcagcacagggggttccttcggccagggccgcggacagcatggccgagttctgcagaaaaggacaggcagagtacccgggaggcatcgctcgcatgcatccttcgttcaaattcaacatctgctggtggctcgaggatgccggaatcgaagcgagcacgttcgacgaaatcgttgcaacgctgccagaacacgccgggccgtcgcagccggtctggcaagcgactttcagcaagcccgctcaggcgcatctggaacgagcccgcgcggccgaagagcgcggtcgcaacacggccgcatcggccgaatacaagaaggccgccttctatctgcggatgaaccggctccccaagcgtgtcccggtcgcggatttgcaggcgaccgaacgagcccacgcggtgctggggaagccgctccaacggatcacgttcaagaccggagagaaagaattcatcggctacttccgggcgccgtcgacacgacgcagcggcaacgaaaagctgccggtcctggtgattctcggcggcctcgacaacctgaagacggagatgatccggcatagcgactatttcgtcggtcgcgggttcgccaccctcattgtcgaaaatccggacactggggagaaccagcttggattccgtccggagtcctccgtgatgtttgacgccgttgcccactacatcaagacccgcagcgacctggacccagaccgagtggccatctacggctggagtatgggaggctatctgggaacgcttggcgggctgaggaacgacttctacaaagcgatcgtgaacataggcggacctagcgattcgagctttgggcaagcgcattgccagattgctcccgcatggatcgtcgcgccctacaccgtgtttgcgaacatgaatccgcagacgacaccccgtcaagcgatgtgcgaatactacgaagcattccaactctcacgtcaactgaagatgcctactgcggtgcagttgcgcaaacccattcttatggtgaacggcgctcgcgaagacctcgtctccagagatgaacccgcatctcttttggctcttggcttcaacgtgacgcaactggtaattggagatgatggccacacggcggaatcgaacatgcgagagcacttcgagttcaccgcgaactggctcatacggcggctgaaaatggaaaattgatctgacagctggaaggcaccgcggcgatgcgggttttcctgcatccagtttgcgacataaattgtatacagtttggcgtacacacactgtggacgcctcggacaaccgcgccgtccacgcacgttccccttgccgcgccaggagacacacgatgacggccgagacctcttcccctgttcagacagtccatccggtggaccagcgcctgccttcgggcaagcttgcggccctcggcctgcagcatgtgctggtgatgtatgcgggcgccgtggcggtgccgctgatcgtcggccgcgcgctcaagctctcgcccgacgaggtggcgctgctgatctcggccgacctgttctgctgcggcattgccacgctgatccaggcgctgggcgccacgcagtggttcggcatcaagctgccggtgatgatgggcgtgaccttcgcctcggtcgcacccatggtggccatcgccaacgccaaccccgggcagaacggcgcgcagctgctgttcggcgccatcatcggcgcgggcgtggtgtcgatactgatcgcgccgctggtgagccgcatgctgcgcttcttcccgccggtagtcacgggcaccatcatcgcggtgatcggcatcagcctgatgcgcgtgggcatcaactggatcttcggcaaccctgtgggcccgacggcgccggcgctggtcgatccggtctacgccaagtggctggccgaggtgacctcgccgggcagctcgattcccgcggtgcccaagggctttgccatcatgcccacggtgcccaaccccaagtacgcagacctctcgggtttcggcgtggcggcgctggtgctcgtatccatcttgctgatcgtcaagtacgcgaagggcttcatcgccaacatctcggtgctgctgggcatcgtgatcggcgcggtggtggcctcggccacgggcctcatgacctacgagaaggtcggcaaggcggcctgggtggacgtggtgctgcccttccacttcggcatgccgcagttcgacccgatcctgatcttgacgatgacgctcatcatgatcgtggtgatgatcgaatcgaccggcatgtttctcgcgctcggcgagatgaccgaccgcaagattggccagaaggccctggcgcgcgggctgcgcaccgacggcctgggcacgctgatcggcggcatcttcaacacctttccgtacaccagcttttcgcagaacgtgggcctggtggccgtcacgggcatcaagagccgctatgtctgcgtggccggcggcgtgatcctggtcgtgctcggcctgctgcccaagatggccgcgctgatcgagtcgctgcccaccgtggtgctcggcggcgcgggcctggtgatgttcggcatggtggccgccacgggcatccgcattctttcgggcgtggacttcaagggcaaccggcacaacgcgatgatcgtcgcggtgtcgatcggcatcggcatgattccgctcatcgcacccaacttcaagcagtggatgccgcatgcgattcactcgctggtcgagtcgggcattctgctggcgtcgatcagcgcggtgctgctcaacctgttcctcaacggtgcgaagcacgacaaagaggccgtgatcgccgcggccaagcaggccgaagcccactgagctgttgctagatcatcgccagcggccccttgcgccgcggcggtggatgcagccggtccaggtccgccagggtcgctgcatcgagcttcagctccgcggccgtcaggttctccttcaggtgcgcgctgcgcaccgccttcgggatcgccgccacgccgggccgggcgatcaccgcggccagtgccagctgcgcggccgtcacgccaagccgttcggccagttcagccagcccatcatcttcagccagcgcaccctggtcgatcgggctgtaggccatcagcggcatgccgcgttcgcgctgccacggcagcaggctgaactccgggccgcgctcacccagcgacaggtacacctggttcgccgcgcacccagggccgtcgccgatggcctgcaccagttcttccatgtcgtcggtgtcgaagttgctcacaccccagcgagcgatgcgcccgtcggccaccagcgaatgcatcgccccaaccgtctcgcgcagcggatggctgccgcgccagtgcagcaggtacaagtcgatcgtctcgatcccgagtcgcttcaagctgcgctcgcaagcctcgggcgtgccgcgccggctggcgttgtgcggatagaccttgctgacgatgaagagctcatcgcgccgcacgtcacctgcgcgcaaggcttcgccgatggcctggcccaggacggtttcggcgccaccctcgccgtacatctcggcggtgtcgatgagccggtatccgagcacgatggcctcgcgcaccgccttcacttcggccgcgcgatggccggcgttttcgcccatgcgccaggtgccgagaccgagaaccggcatctcgccgccggtggggagttggagtgttcgcatcgggccatggtacgggggacacatgaaccggttgcgagagccggcaggcagatggccgtagatgcctcgagccttctaattatttgaagtcaaagtcaatttcatgacagggaatttttgatctctccagtgaaggcattccgcgtggccttcttattttgtcaaggcaatctgggtgccaaccccctcttctggcctggttctcgcttctagaatttttcgaaagcagcccgcgtcacgagcgctggcgcaccgaacgaaacgaacttggaacaggttgagtcaatgcagagaaagcacaggattgccgtcattcccggagacggcatcggcgtcgaggtcatgcccgaagggttgcgcgtgctcgacgcggtcggccgccgcttcggcatcgatttttcgtacgaccacttcgactggggctccgaccactatgtgcgcatcggcctgatgatgccggccgactgggccgacaagatccaaggccacgacgcgatctacttcggtgcggtgggcgcacccgacaaggtgcccgaccacattgccgtgtggggcctgctcatcaagatccgccgcgacttcgaccagtacgtcaacctgcgccccgtgcgcctgatgcccggcgtgcccggcccgctggcgcaccgcaaacccggcgacatcgactttctggtggtgcgcgagaacaccgagggcgagtacacctcggtgggtggccgcctgttcgaaggcacgccgcgcgagatggcaatccaggaagcggtgttcacgcgcatcggcgtggaccgcatcatcgaatacgccttcgagcttgccagccggcgcaagcgcaagaacctcgtggccgcgaccaagtcgaacggcatctcggtgaccatgccctactgggacgaacgcctcgccgaaatcgccaagcgccacccggacatcgcgaccagcaagtaccacatcgacattttgtgcgcgcacttcgtgcagcaccccgactggttcgacgtggtggtggcctccaacctcttcggcgacatcctctccgacctgggcccggcctgcaccggcaccatcggcatcgcgccctcggccaacctgaaccccgagcgcaaattcccctctctattcgagccggtgcacggctcggcgcccgacatcgcaggcaagggcatcgccaacccgatcggccagatctggtcggccgcgctgatgctggaccatctgggcaacaacgacccggtgtacgcagaggcttcggctgcggtgatctcggccatcgagactgtgctgagcgagggtccgcgtactcgcgacatgggtgggaacgcttcgaccgtggatgttggtcgcgcgattgctagctgcatttcggcatgacgcgctgctcttgttcagggcgcgatcacgccgacggtgtgcggagcgaagcgaatgtcccccggcctgcggcctcctcctttatttcgctgcgcagagcacaccatcgacgtgatcgttcagagcacttgttgatcggttggcacaggcgctgcgtccatgtgcgaatggcaccgggtgctccccgcagcgaaataaaggaggagccgaaggcgggggacattcgcggaggggagtacccggtgtcattcgcacgcgccctgaacaagagcatcccacgacacaacgccgagcggagtcactgaaatgggcctgttcctgctgaaacgcacgctgacgttgatcggcaccctggtgggcgcatcgatcatcgtgttcctggtactggagattcttccaggcaatgcagcgcagatgctgatgggccccgatgccgcacccgaggccgtggccgccctcgccaccaagctcggcctcgaccagcccgcctggacccgctactggcactggattgccggcctcctgacgggcaacctgggcgacagctacgcctacagctcgccggtgctcgacctgatcctggaacgcctcgcgcttaccgttcctctggccatgctggcgatggccctcaccgtcgtgattgcgctgctggtgggcgtgaccgccgccgcgcgccacaacaagctcggcgacgtcggcctgatgagcatggcccaggtcggcatcgccattcccaatttctggttcgccatcctgctgatcctggtgttctcggtccagctgcagtggttctcggccggcggcttcgagggatggagcgagggcatcttctcgggcatcaagtcgctgctgctgccggccctgtcgctggcggtggtgcaggccgcgatcctcgcgcgcatcacgcgctcggcggtgctcgaggtgatgcgcgaagacttcgtgcgcaccgcgcgcgccaagggcgtttcgcagcgcgccgtgctctggacccacgtgctgcgcaacgcgatgatccccgtcatcacggtcatgggcatgcagttttccgaactgctggccggcaccatcgtggtggagaacgtgttctacctgccgggcctgggccgcctgatcttccaggccatcagcaaccgcgacctgatcgtggtgcgcaactgcgtgatgctgctcgcggccatggtggtcatcgtgaacttcgtggtcgacgtgctttatgccgtgatcgatccgcgcatcaaggccagcgacatatgaacacccttgctattccaagcccgagcgctgcggcgctcaaggtccccggcttctggcagcgcgcgctgaagcaccgcagcttcgtcatcggcggcgtgctggccgcattgctgctcgtggcggctctcgtgtccttcgtgtggacgccctggtcgccctatgccatggacatggcgagcaagatgcaggccccttcggcttcgcactggctcggcaccgatgcattcggccgcgacgtggcgtcgctgctgctggtgggtgcgcgtgcatcgatcctcgtcggcgtgatcgcggtcggcatcggcctcgtggtcggcaccgcactgggcctgctcgccgcagccaagcgcggctgggtcgaagaagcagtgatgcgcctgtcggacttcacgctggccttccccgcgatcctttcggccatcatgatgacggcggtgttcggcgccggcatcgtcaacgcaatcgtcgccatcggcatctacaacatcccgacgtttgcacgcatcacgcgggcctcggccaacgcgatctggtcacgcgagtacgtggccgccgcgcgcgcctgcggcaagggttcgttcgccatcacgatgcagcacgtgctgcccaacatctcggcggtgctgatcgtgcagatcacgatccgcttcgcgattgccatcctggccgaggccgccctctcctacctcggcctgggcacgcagccgccgcagccctcgtggggccgcatgctcagcgaagcgcagaccctcatgttccagcagccgctgctggccgtctttcccggcatggcgatcgcgctcgcggtgctgggcctgaacctgctcggcgacggcttgcgcgacctgctcgatccacgcctcgcacgcgccaggtaagcaatatgcctctcctcgaagtcaacaacctccagatcggcctgcagacccagcgcgggccggcgcaggccgtgcgcggcatttcgttctcgctggagcgcggcgaaacgctcggcatcgtcggcgaatcgggctgcggcaagtcgatcaccgtgatgtcgctcatgggcctcttgccatcgagcgccaaggtcacgggcagcatcaagctcgacgggcaggagctcgtcggcctgccggaaaagcagatgtgtcagatccgcggcaaccgcatcggcatgatcttccaggagccgatgaccgcgctgaacccggtgcacaccatcgcgcgccaggtcggtgagccgctccaactgcatcgcgggctgacgaaggcgcaggcacgcaaggaagcactgagcctgctcgaccgcgtgggcattcccgacgcggcctcgcgcctcgacgcctacccgcaccagttctccggcggccagcgccaacgcatcggcatcgcgatggcgctcgcctgcgggcccgacctgctgattgccgacgagcccaccaccgccctcgacgtgacgatccagaagcaggtgctcgacctgatccagggcctggtcaaggaaatgggcatggcgctgatcctgatctcgcacgatctcggcgtgatcgccaacagcgtgcagcgcatgctcgtgatgtacggcggcagcgccgtggaaagcggcccgaccgacacggtcttcgccggtcgcgcccacccctacacgcgcggcctgttcgcggcgcggcccgccatcggggccgtgcgtgccggccgcttgccgaccattcgcggcagcgtgcccgaactggtcgacatgccgcgcggctgcgctttcgcgggccgctgcgcccacaccatcgacctgtgccagagcacgcggccccaagccacgatgctgcccaacgaccacacggtgcgctgcctgcggctgggcgaaatcgccgcgtcgaatgccaaggcggccaccgcatgagcaagtccaccaccgccggccagcccctgcttgccgtgaacaacctctaccgccactacgcgctgccgcgcgaaaagctcttcggcccgccaccgaccgtgaaggcgctcaacggcgtgagcttcgaggtgcgggccggcaagagcgtgggcatcgtcggcgaatcgggctcgggcaagtcgaccatcgcgcgcctggtgatggcgctcgacacgccgacctcgggcagcgtatcgctcgaaggccgcgacctgcatgcgctgccgaaggccgagcttcgcaccgcgcggcgagatttccagatggtgttccaggacccttacggctcgctggacccgcgccagaccgtggcgcgcatcgtggccgagccgctcgaggcgctggccgaaaccagccgcgccgtgcagcgcgagcgcgcctcggaagccctggccgccgtgggcctgcgcaccaccgacatggacaagtacccgcacgagttctcgggcggccagcgccagcgcatcgccatcgctcgcgccctcatcacacgccccaagctcatcgtggccgacgaacccgtgagcgcgctcgacgtatcggtgcaggcccaggtgctcaacctgatgcaggacctgcagcagcagttcggcatcagctacctgctcatcagccacgacctcgcggtggtgaaccacctgtgcgacgaagtgtgcgtggtcttcaagggccgcatcgtcgaacggggtcgcccggccgacctgttccagcacgcccagcacgaatacacgcgcaccttgctttccgccgttctgcacacaccgtcccgctagccgaaacgggctctcttttcctccaccctcacatctccaggatctatcgaatgttgaagcgacgcacactcatgacttccgccatggccgcggcaatcccgggtgtattcctgccccaggcccgcgcgcaggccggcaagaacacgctgacgatcggcatgccgctcgagccgccaggcctggacccgacgagcggcgccgcgtctgccatcgcggagatcacgcagtacaacatcttcgagacgctcaccaaggtgaatgccgacggctcggtcacgccgatgctggccgaaagctggacgtcgtcgcccgacatgaagaccttcgtcttcaagctgcgcaagggcgtgcgcttcgagaatggccagcctttcaacgcgtcggtggtgaagttctcgttcgaccgcgcgggcgacgccaagagcaccaacaaggacaagcgcttcttcagcgagatcagcaccgtggcgctcgacgagtacatggtgggcgtcaacagcacgctgcccaaccccgacctgcccttcatgctgggccagtcgaccgcctgtatcgtcgagcccaagagtgccgagaccaacgtcaccgcgccggtcggcaccggcccgtacaagctgagcgcatggcagcgcggcgcttcgtgcacgctggtgaagtcgccgacctaccgcgacccgaaccttgcgaagaccgcgaagttcgtgttccgtttcatgtcggacacggccgcgcagaccgccgcactgctgtcgaacgacatcgacatcttcccgcgcgcgggcacgcgctcggtgagccagttcaagggcaacccgcgcttccaggtgatcgaggtcggcacgcgcggcaaggtgatcctgaccatcaacaaccgcaagaagccgctggacgacgtgcgcgtgcgccgcgccatcctcgcggccatcgaccgcaacgccatcgtccagggcgcggcggacggcttcggcaggcccatcggcagccactacgccctgggcgcaccgggcttcatcgacaccacggcgatgaaccccttcgacatcgagaaggcgaagaagctgctggccgaggccggcgtgaagacgccgctcgaactgcgcctgcagctgcccccgccctcgtatgcacgccagggcggcgagatgatcgcggcgcaactcgcgcagatcggcatcaacgtgaagatccagaacgtggagtgggcccaatggctcagcggcaccttcggtggcgcgcacgacttcgacctgacgatggtcgcgcacgtggagcccttcgacctcgtgaagtacaccgagcccgactactactggggctacgactcgaagaagttccgcgacctgttcgtcaccatccagaacgaagagaacaagaagcgacgcgccgacctgctggccgaggcgcagcgccagcttgcgaccgacgcggtcaacggcttcctgtaccaggcggtgttcccgaccatcgcgcgcaaggaagtgaagggcctgtggccgagcatgccgatcgtggtgaacgacctggccgcaatctcgtggagctgatgcgatggccaagcccctgtactccctgagcgtgcaggagttgcacgcggcctatcgcagcaaggaactctcgccggtggaagtgacgcgctcggtcaacgaacgcatcgcggcctgcgagcccgaactgcacgcgacgtggctgttccgccccgagcttgcgctcgaacaggcccgcgcctccgaagcgcgctggctggccggctcgcctcgcggcacgctcgacggcgtgcccgtgaccatcaaggacaacctcgcgaccgagggcgatccgatgccgctgggcaccgccgcctacgacctcgtgccgatggcgcaagactcgccgcccgccgcacgcctgaagaaagacggcacggtgctggtcgccaagaccaccatgcccgacctgggcatgctgtcgtcgggcctgtcgagctttcatgaactctcgcgcaacccgtgggacctgtctcgcacgccgggcggctccagcgcgggtgccggtgcggcggctgccgcgggctacggcccgctgcacgtgggcacggacatcggcggctcgctgcgcctgccggccagctggtgcggcatctacacgctcaagcccagcttcggccgcattccgttgagcacgccctacatgggccgctgcgcgggaccgatgacgcgcacggtggccgactcggcgctgatgatggcctcggtcgcgcaacccgacgaccgcgactattcggaactgcccgcgccagccatcgactggaccgccttcgaggtcgacccgtcgttcctcaagggcaagcgcgtggcgctgcacatggacgcgggctgcggcctgccgctcgatgcgcagatcgccgatgcggtgcgccgcgcggcgaaccgcatcgaggcggccggcgcgctggtggaggaaatcaagcccttcatgacgccgaagatgctgcagggcatggaccacttctggcgcatgcgctcgtgcctcgacatgcaggccatgccggccgaaaagcgcgcgaagatcctgccgtacatccgcgactgggccgagagcgccgccgggttctccggcgcgcacatcttcgacgcctacagccagttcgtcgccacgcgagcggccacggtcgcagccaccaaggcctacgacttcgtgatctcgccggtgtcgcccaacatgcccgcgcccgcggaccatgcctcgccgaccaacgacccgatgctgccgctggagcacatcggtttcaccgtgccctacaacatgtcggaacagcccgctgcttcgatcaattgcggctactcagccgagggcctgcccatcggcctgcagattgccggacgacgcttcgacgacctgggcgtgctgcagttcagccgcgccttcgagcagatccgcgaagcacaacacccctggccggagcctaggtgaccggccgcaaggagacaaatcaaatggacgcaacccactacatcgacggccgccgcgtgccgtccgaaggcaacgccaccatcgatgtgatcgacccgagcgacggccagaaattcggccagatcgcgcgcggcacggccgccgacgtggacacggccgtgcgcgccgcacgccaggccatgggcgagaacttcgacggcccctggggcgcgatgaccgcactggagcgcggccggctgctcgccaagctgggggccgccgtgatgcagcaccatgaagaactcgcgcagctcgaagcccgcgacaccggcaaggcactgcgcgtggcgcgcaacgacgccaccgcgctggcccgctacatggagtactacgccggcgcctgcgacaagctgcacggcgacaccctgccctacgagcgcggctacaccgtgctgacggtgcgcattccgcatggcgtgacgggccacatcattccctggaactacccgatgcagatcgcgggccgcagcgtgggcgcatcgctcgccgcgggcaacgcctgcgtggtgaagccggcggaagacgcgagcctgtcgctgctgcgcctggccgagattgcgaccgaggtgggctttccggctggcgcgctcaacgtggtgacgggctacggcaaggaagccggcgccgcgctgtgcgcgcacccgggcatcgaccacatctcgttcaccggctcgaccatgacgggccgcagcgtgggcctggccgcggccgagcgccattgccctgtgacgctggagctgggcggcaagtcgccgcagatcgtgttcgccgacgccgacctggacgcagccgagccggtgctgttgaacgccatcatccagaacgccggccagacctgctcggcgggcagccgcgtgctggtcgagcagtcggtctacgaagaggtggtgcagcggctcgcgaagcgcttcacggccgtgcgcgcgggcacgcccgccgaagacctggacatggggccgctgatcaacgagaagcagtttcgccaggtgcgcgacatggtctcgacggccgaggccaacggcctgaaggtggcggcgcgcggcacggtgtcgccgaatgcatcggccaccggctactaccaggaggccgtgctgttccgcgacgtgccgcacgacagcgacctggcgcagcgcgagatcttcggcccggtgctggtcgtgatgcccttcgccgacgaagccgaggcggttcgcctggccaacggcacggacttcggcctggtggccggcgtgtggacccgcgacggcgcgcgccagctgcgcatggcgcacaagctgcactgcggccaggtcttcgtcaacaattacggtgcggcgggtggtgtagaactgcctttcggcggcgtgaaatcgagcggcttcggccgcgagaagggcttcgaggccctgctcggattcacgaccctcaagaccatcgccatcaagcacggatgaattcatgacaagcactgaacagcaacaagccccccgccgcgtgggcctcgtcggcgtcggcctgatgggccacggcatcgccagcaacatcgtcaagcacggccaccagctcaccgtgctggagcacgcgggcaaccagcccatcgacggcctgctgaaggccggcgccacttcggtgaaagacgtggccgcgctggccgcgcaggtcgacgtgttgatcctgtgcgttacgggcacgccgcaggtcgaggcggtgatgctgggcgacaagggtgcattgactgcgctgcgccccggcacggtggtgatcgactgctcgacggccgtgcccgcctccactgccaaggtggcggaagcggtgagcgccaagggcggcaagttcatcgatgcaccgatgacccgcaccgcaaaggaagccgcagaaggccggctgaatctgctggtgggcggcgacgccgaggtgctggcctcgtgcctgccgctgctgcgttgctttgccgagaacgtcacgcacgtgggcggcatcggcgcgggccatgcgatgaagctgctgcacaacttcgtgtcgctgggcaccgtggcgctgctgtgcgaagctgctgcctgtgcggagcgcgccggcgtgaagcccgacgtgttcgtcgacgtgctcgccaagggcggcggcaatggcgtggcgctggagcgcgtcaagcccaagctgctgacgggcagcaccgattcgctgaagttctcgatggccaatgccaagaaggacctggggtactacaacgacatggcggagcagtcgtcttccagccatggcattgcgcaggctgtggatgcgctgctgacgcatggcgtcgagaagttcgggccggatcgcatggtgctcgatctggtcgaagcgatgcgctgattttttattgtgttctgtgcgctgttgttcagggcgcgtgcacaggacaccgggtactcccctccgcgaatgtcccccgccttcggctcctcctttatttcgctgcggggagtacccggcgccctgtgcacctgggcacctgggcacgctgctggtgtaccgccgatcaacaaccgctccgaataacgctcccgtcgatggggtgccttgcgcagcgaaataaagggggaggccgcaggccggaggacattcgcggagcaaggtaccccgtcggcgggagcgtcgccgcgaatgaacccgagcccgagccctaaggcatcccccgcgccagcaaatgatcgacaagccgacgctgcggaaaactcaacgcctcctgccgcgtgcacagatacatccgtcgtgaagcccaagcgtcggtgaggttgatgaaccgcagcttcatctccttgcgataggtcaccgcagccccctcgggcaggatgcccacgcccatgcccgcctcgatcatccggcacacggcctcgaagctcttcacccgcacgcgcagcttcagcaccttgcgcgcgctcatggcggcgtcttccatcgtgcgggagatggcggagtcgtcttccagccccacgaaatcgaagtcgagcagttcctcgaacgacacctcgcgcccgcgccacggatgcttctgccgcacgatggccaccagcctgtcggtgcggtagggaatgaagttgagcgcggggtcggccgcctcgctggtgatgacaccgacatcggcctgccggtcgcgaatggcctgcacgatgtagacgctgcggtgctcttccacgctcacgcggatctccgggtagcgctggcggaagctcgccacgtcgtcgggcaagaactggcccatggccgatgcattggcatgcagccgcacgcggccggtagcgccctgggcgtagtcggagaggtcggcacgcatgcggtcgacgtcgcgcaggatctggcgcgcatgcatggcgagcgattcgccagcgccggtgggcgtcacgcccttcgaggtgcggttgagcagcgcgacgcccaggtggccttcgagaatggccaggcggcggctcgcggccgacagcaccatgtggctctcggcggcggccttcgacaggctgccgtgctcaatggcgcgcaggaaaagcgccagcgaatcgaggtcgggtctcatcggattctcgtcgtgctgcgggggccgccattgtcgggccagcgggatgcttcgagtcggccgaagcattggagcggtcattggtccacgccgatcggttgacgccggcacgcacccctggctacattctcgagcactgggtcaccgcagtgatattcggcgtaccgctttggcggatcgtcgcacgcacgggcaacccggcgccatggcagtcctgttcttcatccccctggtggacatcggcgtgctctggcggcttgcgtacggcaagtggcccggcatgcccgctcgtccctgaaagcctgcacggatggccgcgaggtcgcaccctcttcgccaggaggcctgtgcctctgagaaaaattcaaactcattttcgaaatcgaagtccatgttcggtcgaatcaagctccatccattcatcaaggcgaaccctccgcatgccgactgcgcgccggcgacgaaggcactgctgcacatgtacgaggggcagttgcccgccgcgctgctcgagttgtggcgcaagcacggacttgggttctatggccgccggcagatctgcctgatcgatccgcaggcgtggcaatccatgctcgaccgatggatcgtttcgccacccagcgccaccgtgcgcgtgcccattgcgctgacgccattcggcacgcttcttttttacagaaagctcactgctgcagacgaggacgttgcggcactgaaccccgtgacccgcagcatcagcatcctgagctgggacctcgtggatctgttcaacaacgttctgagcgacccgagccagatcgatgaattcatccaaccggccatgctcgaaaccgcgcagcaacaagccggcacgctggctcccggcgaggcgtaccacgtcgacccgatgctgttgtccatgcagatgctgaagatcgcgaggacggatgcgctcgcgcttcaccagaagcttcgcgcgcaggtcgaccacgagcagacgccgcccgcgccgcccccggacagcgtccgcgcggccctgcccgacaaatatcgcgcggccttcaaggacctggaaagaaaagacggccacccgagcgggctttatctatcgacttacatcgattggcgccggctggtcgcgctcgacgcggatggcagctaccaactgctcttctggaagaacgatcacaagacgggcgaagcatcggacatacggcgctacagcgggcagtatcgggtgctcgaaaccgaagaaggcgactgcctgctgcagctcgacctggtgttcaccagcaagtcgctgggcagcgatgccaacgatgacggcctgtatctgatgcgcagcggcggacagccgctgctgttgcaggccgcccgcctcgaggacatggcgacggccatcggcggccgcgcagcaacgatgggcagctccgagcactatttccggcccgtgcgtctggacgatccttttcccgtcgaggactccgacgggatggacactccgcccttcgaggacctgccggttgcgctgcaggccctggtgcaccgcgagccgctgagggcgacgatcgtcgaggtcgccgccaacagcgacccggaagacgacaccgtgatggtctgggtggatctgggaagcaacgacgggctgcggaagaacatgccgctcatgtcgccccaaggcagcccgcgcgcactttacggctgggtgtggcggatggaccgggagcggtgcggagtcggcatcaaggtacggcgggacgcggcaggcgccatcgtcaacgggcccgagaccggcgacgtccttgtcagccgggcggattgaagcgcgatatcgggtgggtgggtgctgaagagcgagcccgggaataccctctgacccctccgaagtcttcttgcctacatttgcccaaggggaacaaactgatggaccagaagacggttaagtcattgatccgccatggccgcaagaagtggtcaaaacaacaaagctatggactcgctccttcagccccgaccccatggggcaactgtgcaagtaatagtgttctggactggcttacctggagggcctagggcagttctctgaagggtgcatcgctccttcgcgccagcgatcatcactggcatactggtcgtctatacagtttcgacatgatgaaacgcacatggacgacgttgtcaacacgatgatccctgccgcctatgacgggcgcgaacaagcgctcgttaagcatcgaatgctcgaggactacctcgagaagctttttctaatcatcggtctgacgtccagaagcggtggtaccgccgaactttgctatgtcgactgcttcgccggtccctggggagactcgtcagaggaaatgcagacgacatcgatagcgatctcgctcaagactcttgacggctgccgtcaaaagcttgccagcctcggggtctacgtaaaaatcagggctctctacgtcgaagagaaactcgcgtcgtttcagcggctacagacctacttggctgctagcacgcctcggagcgtccgatcgcattgcatgcaaggtgactttgtctcgcttcggcaggacatcctggattgggtcggttcggaatccttcgcgttcttcttcatcgaccccatgggctacaccgagattgctgtcccaacgctttgcccgctgctccgccgcccgcgctcggagttcctcatcaacttgatgtacgaccacgctaaccgtgcgatgtcgatgcacggcatgaagagtgccatgacgacgttgcttggcgagaaactcgaggtggccgatctagcgccgcggcagcgtgaacgcgccatcgttcgcacctatcgtgaaaacctcaagcgttgcgttcccgcgtcgacgacccacccggcacgagcggcacatgcgcgcgtgatgaacccacagcgtgatcgcacgaaataccacttggtatacgtgacgtcgcacccgctgggtatcgtgaagtttatgcagatatcggaagccgccgatcgcattcaatcccaggtgcgtgcggtcaagcgcgataagaagaaggcggtcgacaagggaatggacgagctctggcccgtcggatcgatggtggatttcgacgccactcatgccgccccaaaggatgtcgacgagttttggcaggcctacctcgccgacggtgatcgtcttatcgataccgccgccttcgccaacatcctcgaaaagacagactggtttgaaggcgatcttcaatcttcacttgtaaggctgatcaaggcaggtcgtatcgtcaaccgatcggccgacgcgtcgcgtcgctataagcgccccctgcattttgaagcaggcatcggcgagcgccttgcttgggtggcgtagagcgcgatcgaggcgctgttaacgacgttgacgtgtcccctgccgatcacaggcgcggggcaccacagatcgtccaagcgcggtcaaaggaagatcatgggccgctgcggagcagcggtcagaacatcgccaggtcgcagagtggagccgcgcaatcgccggctgccgtcggcggctgctgacgcgccgatatcgccgctgcgaatcgccgcatcgagggacatacggatcatgtcggcagtcgccggcgtcgagcttccgaatcgctccaaaagttcgccgaagaggatgggcttgccgtgatcgtaaattgtcgggaccaacttcgcagccagccctgacaggcaccgctccgaagcaaccttatcgaagtgatgggcttctcctaggtcgagtgagtcttgccccgtgaccgaaccgtcaacatttgtgctgtagccgagcgtgaaaatgtctggctcgaggtagtgcgagaaatgattggagagtttccagtgcaactccatcatcacgtcgcgcgccttgaagctgttggagagatgcacaagccaatacgtccaggccgtgctgcccttcggggtgatgtagaagatcgtgtagtgtttggccccgctgacctcgaccaggctcttggccaggttgcgttggatggccgatcgccagacattgccgccagcgagcttgagaccatcaatggtctcccaattgatgtaccggtctagccccaattccttgagtttctttcggctctgcgcggtgttgctgaggaacgcgatcaacgagtcgacgttgaacgtgaggaggacctccgcgcctttgacctgcgagaagatcgttcgaagcagcggtgccgaaacctgatcatacgcatactggtcgagcaaaaagatggcacgctcaccgcgctctcgtgcgcggatgtccgcaatgatcgaagaaacgcgttcttggaacgtgcctcgaagcatttcgatgtcgctccccagtctgctctgctctacccgcgcgcaaaccagctgccgcaggtagtcgaaattgcctttgtctttttcgacgaagtaatacttcgcggcgatgtgccgcggcttcagtcggccaacgttgagtgcgacttgttgctccgcgactgtattcaaagcaatgagtggcgagccttcgtggaagttgatgccgtcttcggccatgtactccccgccgccggcaaagccatccacgattgacagcgtcaacttctcgatgagcacgttgctcatgagcacctggatgtatcgctcaagataacttcgaacaatttggtgcttgaccaagctgtgtggatctatgggcggagggcggctgcctaggtgccaagcgtacttttcgtctcgtttgaccatcgtgggtggcgcagtgggaataggccgatcctaaccgcgctctccaacacggccaattcatctcctgcgttaaattgccgctgcggcaggcatttcgtcccaggtacggccatttagcaagcggccatttgcttgcttggcccgacgcttgccgtcagcgccccatccgccccactgcttgaagaaaaatgcaacctcttgctcttggcactgggtccgcacagcctctgcccactcggtcttcattggacgtgccttcggcccagactctccgccaacgatcacccaatggatatcggtaaggtcgagctctcccacatcagccagtaggggttcgaccgacaggaagcggatcgtggcgggtacctttcgaagatagtcgatacgcggcacaccgtacttccgatcctcgaccgaaacgcccagccaggcgttggccgggacagggcgagtacggaaatagcgcgccatccgggccgctcgcttggtcagaatctggtaggtgtggtggggcgtctgcgcgatcacctcgaacaccttggcgatgtactcgtccggcacgcgttcgtggaacaggtccgacatggagttcacgaagtagaccgtcgacttctttcgcttgagcggatcgttcagccgatcaggcagcaaggtaagcgcgaatccattctcatagcctgccgttcccatggccttcagccgcttggccatggcctccgcatagcaatgcttgcagccaggcgagatcttggtgcacccgacagtcgggttccaagtctgctcagtccattcgatcttgctgatggttgtcattgtgatttccaatgcttagttagcttagcgctccttggcgcgagcggtcggtaactacgaacaattcctctgacgacgccgatgatgttcagcgtttcccgagggtctacagcctgtgtatcaacgccatgtggcatcaggtgaggccgcccgtggtctgtcctgaattccttgatggtgtgcatgccatcgatctcagccaccacgatgtcaccgtgtgtggcttgcacactcgcctccaccaccgccacatcaccgctcagaatgcctgtgtccaccattgagtcgccgcgcactttcacgagcacggtcttggaaggccgagccaccaagagttggtccagcgcctgagcctgcacaagaccagtggcgtctccgcccgcgccgaaacccgcacgcacttcgtcgtcactgaggtccagcgtgaagaagcttggcccaggcgccagtcgtccaccgacggacttggccaggtggccggtagcaatcaaccgctgggtgaacttgaacgcagcgttcttcgccttgaatcccagagcctcggccattcggctgtacgacggaaagcaacccatgcgggcatatgtgtcgcgcaaacggcgcagatgcgcgtggtcgttgttcggtcgggccatcgcggcattttagtgaacaatcgtccactaatcaaagaaaagttgcggatgcagccgaggccgcactcttcaggcaatgtcagatgaggttggagttgctggtcagaacagattgaagttgcggctgcgcgcaatgtcgccccagatgcgatcgggcaatgaatgtcgtgagaaaaacacgagacggtagatagagcggcccttgccatcggtgatgagaggcatctggccgctgaccgtgaagcctagcgcctcgaccgcctgacaccaggcagtgaagaaccaaccaggcaagctggacttggacagcgcatcggcgggcaccgaggcgcgccagcccggcaatgcgtggtcgaaccgatcccgcttggggttcaattccatatcgatattgcgcgtcaggtccatcaggctgaagtgaacggcaaagtccacgtattgcagcttggctaggcgctcgatgattgagaaggagaggtattcgaggttgtacgggtcgatgtaagccaaaaccaatgagccgaatggcacggctttgatcattgcatcaacagtctgaagcgccggccctgtaaagctctgcactgacgcaccaactgcggcgagccgcaactcgttggcttgtgctcgttttccttcgatatcgccaatcagcattcgggtgtccacccggacaaacttcgtgggcacaggatatggcggatgaaccatccagtagtacacgttgcgactcacgtagagctccaggtgcctggcgggtttcccttccggaatcggccatcgcaatagctcaagcagttttgagcgattcttttcaagaaactgcctgcgccccaggattcgactgaactgccccgccctgtcgctctccgacttgccgaatatccggtcgcggagtcgacgtccatccttggccgtatatgtcggctggttgtacttgcactccccagtcacgagaaggttctcttccggccaataggcgaaaacgtcaaagtcgccaacgtcatcgaagcgctcgctgcgaaacctcctgtagaaatcgacgccccgctcgacgaatggagtgtgacggtcaaatatatctttggtgcgaatctccaggcgcttttcgattccctctttgacttcgcggataagcggctcgacgttgggccaatcgaaatctgcgggaaggtagccatcacgcaccggtgacatccagttgtacatggaccggctcgtcgcctccgcgccccaacgtagttgggcgccatctacaaccagtggcctgatcgcgtagcgatgggttcgcttgctgtgctcccagtagggaacttccgcttcgtcgacatctcttccgaaaagcctgagaacgcccttttctgagagcgtcaggaacgacacgatgtttttcgcctcctcaggctcgagccgatcgatgctttcaacaagaacttgcacgatccgctcgggggccgccgcgtacgagagtgagagctcgtcgtcgaacccggacctttgagcctgggacagtaccgccagagctgtgatcaggttttgcaactcaaatccaacatcggctttgaatgcggtttttagcttctccgactcaagtaactcttttgctgcgccctccacgacgtcttcgctgttcgcgtcaatgtccaaccgtgacttcgcgtaccagcagtcactcacgggatacgcgaaggcactcgcggagaatctgaactccaaagctgaacggtccgccgtaggcgaactcattgccaatcgaaacaaggcgatggaccgccgggacaaggtggaggtccagttgcaggatgagcttcggcgggctgccaaggctgccaatactgccgaactcttgggggggatcagccaagctctccagttcacgcaagtgatgaccatggccagcggcatgatgggtggagaggcgatttcgaagtcgaccactgcgccgttgaagacttcggcagatgttgtgagggccgtgcaaggcgctggggctcgggcggcggccgccgccgccgaactcgagttggagcgcggccaactcattaacgcgattcagggtatcaacggaaagatcctcgacgccggagtgaagaacgggatcgaccagccgggcattttcaaggtctacttgcactgaatcagcacgctgctcgcggggtgggaagactgccttgacgagtaaatcgcacgctgcgcccacggtgcggatcagctggcacgccccttgcgcttacatcagaggcgaattgcagcgactgcctacgcggctcgacagccggatcgaagtacttctgcccccctctggaagtcgccccctgcctgaccgggtccggaattcaacatgggtcgtttgagcgctcgtcgcataccggcaactggcgggcgtagccaccgcgtactgccgagcctttccgaaggtgttgtccaggcttccgcccgatattgcgaaccgggcgcgcagcgccgcaagctcttctccggggcagcaatggagcggcaacgagttgttcgacgtccgcacccatttcgtttgagtaccgagccgcggcaaatcctctatccagcgctgccggaccgttcgacggacgggatgttttcatgcgtgcatcaacgcctgagcagatgcctcaaggaaggaagcagaaccgagacgaactcgtcgtatcggttgtcgaaaaccgcccctggcaccagatgcttgtccctgaggcctctgatggtctggtcttgcttgggcgttgcaggcggccgatggccttgccacgcgagcaggaacaggcgccgtagcgtgggctcgtttcgacgaccgcgctggagggcagcagcgagcacctcggaagggctgttcgagcggctaccgatgacacggccgtgcttgaaagtgagaagtaccggcaagatgcccttcgtgttccagaagtgccagctgagtcccggagcgaactcttcgcgccaatagcggtacctggtgagccgatagcacgccgtgaaaacggcatcgcgctgatctgtgggcgcacctgcctcgtagtaggcgagcgcgaccctcaggaagtcgtccaatgcctcactccagcttgcctgcgattcgaatgtctgccggtcaaggtcccttcgcttgaacctgtgccagtgtccgtgcgacctgagcgccgtatcgaccagctcctgggacgcgaagatgtattgaccgccccggaccttgtcggcgccatgctgcagcatgagctccagcgtgacctcgtcctccatcctggcagcctggctcctgtcactcgttcccgtgcacacgcaatgcaagcgccggactggccggtgcaaggtcgtccagtccgaagcaatccccgcacagtgctgccgaaatcgacgctcgaagttgtcggtcattccgacatagaaaaacccatcctccaaggcgagcgcgtaaatatagagaacgcgcgagttggcgccgggccggccaccttggtcgacggcggcaggctcctggtgaacgctattcaacgggctcgctgcggaggaaacccgcttggcgagccgtacgaattcagcaaacacctcgtccgggacctcactccccatcagtgccttttgccatccgcgtactctgggccagctgacaccgaggatgtccgtttgcctgcgcgaaaatccccctctgtcgctggcgccttgggccagcgtctcttttgtcaatcgcatgcttgctcgtgagtagtcgatcagggccggcggatgcgctctatggatgaaaggtccgccagaaactcagaatggtgcgaatcgagcttacacgtcgcgctcgtcggatcacctcaagattgcgccgactgtgtgcgaagttccttcttgtaccgcttcatcagagattgcatcagctccgacggctcgacggtcagtcctgcacaaagcgaaaccaggctggtcagggacggactggtcgtcgctgtctccagtttggccacgaaggtgcggttgagtccggctgcgaatgccagctcctcctgattgaagccaagcgctgcccgccgagctttcagctcggccgcaaaggctctcagcagcgcaggatcttgagtcgaccgcatgcaacgaatctcgttgcacggcctactttatgcacccgcttgtatggtacaaattgatgcatcagaagattgaaggaaaactggatgctcagtgttttcggaatggatgcagaaacgccgtcaaataaatggcggttttcgacccaagtgcgcagagggtgtgcatgactcttccgctcctgctcgcgctggctgtcgccgttgtcctgttctactgggtctgggtcgtggccccgcgcgggatccaggtgcaacgcgaggcactcctccagacggaaggtcgagcgacgggggcggcattctttccgctcgatccgcgccgcatgctgggatcctgggagggaacgtgcatcgtctttgacccggatgccagaaaggcatgcatcgtcgtcaaaggcaagacagcccataccgtcgatttcgactacttccggatgtggcatctcaagtggatcgagcagtttcaagggccgctgagcccgtacctgcacgtgcacttcctctttgagacgagtgacttcgatcgcccgaccatccgggtcaatgtgtcttccaaggcagagggtgaccaatggaacgcgaagctggcgatcctgctgcagtagcggctggccggtcgaatccggcaagcatcgctctgatgagcccgcccccgctcagccgttgcatgttgacaatctcggttgcccgatgcagtagccaccgctaagataagcccgacgaaaacgctccttcaagacccacttcaaacgccatgttgaacttctcagccgcaaccacacaacgcgtcgcattcgacgcgggcgcagctgtgcacatggtcatatgttcgcggacgtcgacccgaacctcgaaccggatagcggcggcgatatcgcctcgcctcatcctcgttccccagtccaggagctgacagattcggctccctccaggagcccagaatggtcagcccgaagcagttttcctctctcccgccaacaagcgccagccccaagctcctgttcgtcggcgaccctcatagcgacttcgcccccgtgatcgccgcggtcgagcgcttgcggcccagggcgatcgtgctgctgggcgacatccaggcgcgccagcctgtgcacctcgagcttcagccgatcctggctctcaccgaggtctggttcattcacgggaaccatgacacggactccgataccgactatgacaacctgtggggatcggagctcgtggaccgcaacctgcatggacggatcgtcgatatcgccgggtacagggtcgcgggcctgggcggcatcttccgcagcaagatctgggatccgcgccggccgatcgaagaggccgcattcgcctcgaccgacgcgctgcgccgctccatgcgccccgaagagcggtggagggacggcattgcccgccggcaccgctccaccatcttcccggatgactaccttcagctactccggagcccgcccgccgacattctggtgacgcacgaggcgccggcagcacatccgcacggctggcaggcgatcgacgagctcgccgagacgctcggcgtccagctcgtagtccatggtcaccatcaccagagcatcgactatctcgcggaagggatgcagagtgctgcagcaccgttccgtgccctcggcgtcgacatgggctcgcacctgacgtggccgcgggatccaaaaaaggaggctggatcggaagttcttccacaagacttgctggaccttgccatgcaggtattcggcgcagaggctccagcttggctggacaagccacacaagctgctcgacggccagacgccagcagctttcgcagccgggggtgggtcggaaaaggtccgatcgatgctcaacgccatccaatacggtggtgtcgtatgaggcccgatgagagtggattcggaggtccagagtgatcctcttcctcgacttcgacggcgtgcttcatcccgaaggggaggatcacatccacaacggcggcgtcgacttctgcttcctgccacgcctggaggcgttgttgcgcgagttcccgttcgtgaagatcgtgatcagttcgtcctggcgtgagcacctgctcaacaagacgctgctgaagccgttctccagcgacatccgggcccgcatcgttggagctacccctccttcggggtttggccttcagccgccgtacaggaagcgtgaaggagaaatcctcgcttggctacagatccacgatgcggtcgacgagccatgggtcgcgctcgacgatgcctattggcagttcgatcgctgcaaggaccacctggtggtgtgtggctcattcaccggcttcgacgacaaggccagtgccgagcttcgcacgcgctttgaaggggtgtcccgatgaaagtgctgattctttccgacctccacctcgagttcgctccgttcgagccggtgcctgatctcgaattcgatgtcgtcatcctcgccggcgacattcattcgccggccaagcgcgccctccagtgggcgatggatcgcttccgcggcaagcccgtgatctacctgcttggcaaccacgagtactacgatggacggctggatacaacactggcagaagcgcgccgcgaagctgaaggcagcaatgtccatctgctcgacggtgacgagctggtgatcggcggcgtgcggttcctcggcgcgacgctgtggaccgacttcgcgctcgccatcgagacacctgaaggtccgatcagcgatgtcgggcgtgccatgaagatggcgaccaatctgctgaacgactacgcgctgatccgcacggccgacgagtcggcggagcccgacacttggcgtgacaagcagggcagaaagcttcaagcggccgacacgcttcggattcatcaggcgcagcgcgcttggttgcgcaacgaactttcggaaccgttcgacggaccgacagtggttgtgacacaccatgcacctcatcgcggctcgctggcgcagcgctacgccgatgactgggcctcgggcgcctttgtcaccgagcttccggataccttctttgatgtgcccgtgctctgggtgcatgggcacacgcatcagcagttcgactatcgggtccgctcctgccgagtcgtgagtaacccgcgcggctatgtgaactggagcggcaggatcgagaacaaggcgttcgatcctggtctggtcatcgatgtgcaaaatgttactggaggtgaggactcgtgaagctgctcatcctttcggacctgcatctcgagttcggcgtcttcaacgtcccgaagatcgactacgacgtcgtgatccttgccggggacgtcttcgtgccaggctccaaggccatgcgctgggcccggcgggcagacactttcggggacacggtctcgatcgtcttcgtgccgggcaaccacgagttctacagcggcgtgctgcagaccacgcagaaggaaatggcgctgtctgcggccgcgtgcaaggttcatttgctggcgcctggcgaggccgtgatcgagggcgtccgatttctgggctgcacgctgtggaccgatttcgagttgcccatccaggccaaggccggccccaccgtcgacatcgagcgcgccatgaagatcgccaagctccaactcaacgactactcatcgatccggtgggccgagacaccagagcctgccgatcagtccatggtgcacgtcaagccgaggaagcgccgcctgacgcccgaggacacgcgagcgctgcaccagcgtgaccgagcctggctggcccagaagttggccgagcccttcgacggaccgacggtggtcgtgacccaccatgcaccgcaccgcggatcgctcgcaccacactaccaggccaattggctgtccggcgccttcgtgagcgagcttccgggctctttcttcgacgttccctcgctctgggtacacggccacatccacgagagcttcgattaccaggtcggcaactgccgcgtggtgtgcaacccccggggatacatgcggcatggccgtgaccaggagaacaagcagttcaaccccgagttcatggtcgagctatgagtgacatccagtcatctatccgcacgatccagcaagtgctggctgccgcgactgcggtctcgggcggggacctcgaggcggccatcctctggtacaggaaagagccactcgcgccattcgactacaagacagctgagtcgctggtggccgaggggcgagccgccgatgtgctcgatctcctggagtccttccaagccggtttcgtcggatgacaactccgcgcaccacccacgttggtgactccagcgacctgctgttcctggatatcgatggcgttcttcatcccgtcgagaccggccactcgttcagcagcaggttcttcagccatttgccgctgctggaagagctgcttcgagagttcaagtctgtagaggtcgtcatctcgtcggattggcggcgagccgaaagcatcgaacagctgcagcggtatttcagtgccgacatccgacaccggatcatcggcgcgacgccgcagattgacccccatgtcgctgtccaccatcggcggcagctggagatccatgcctggctcgacggaaacggccgcagcgacgctgaatgggtcgcacttgacgattggccctcgcactttgaagcgggcttcgaacggctcgtgctcatcgaccccaagcgtgcgttcgatcaagatagctttcaggaactgcgctcgcacttcttgcggttcgcggccggccgttgaaccgccataggatcagttggcgaactgtgcttggttcaagaaagctgcggcactcaagcttcatcgccacttcgacgcacatatgaaatgaacccctcatcccgtcggacctccacgcgcgatccgcccgctgtaaagcggtatatcaatgctgatgagccgcgtactgtggctccattcgacctctctacgcgggcgagacatcacggaacgcgagaccgtttcaacggggtggtcgcagccggccccagtgctgcgtccaattggtccagaagggactggagcaactcaacataggtgtcatagccctcgctgggatgctcccacgggatggcgaagatgctcatcagcacttcgacgcaaagtccgtggaagtagacctgaagtcgttcctcggaaaaatcgaagcgcagaagcaagtgctggatgcgatggtgtagctcagggtggtgaaactgcttgacgggcgtgtcggtcgacaaaagatagaacgaactcaacaccgcgctcattaccgcccaggccaggtgcattttggctttgtcgtcgcggtctcccacaaggatgtcccaggcgccgttgtcggcttccttttcgcgctcgagcttgtcttccgcggataactcgcgccagccgtgtgcgtggttgctgatgccatgcatccactcgtgcaacagcaagaacgatatggcctcctgaaaaattaggttggttttctccgtgaagtagcgctcttggtcgctcgccgatgtgattggggagggcaggcccttcggccacggcgtgtagacatccgccaccgtctgcgcccagttgcgcagtttctcggctcgagcaagcagttgagggtcaacgacggaggtaggctccagtttcggtctctgcaccacctcttcgtagcgaatcaaccatgcgtagatgaagcaccagagcacctccaagtgcgtgacatgcagatcaatttccgcgggctctccagacaccttgggcccgacgggcgagaccaagtctgcacgcagagaaatcaccggaagaaccgtgccggaatcgacaaccttctgcagccggtcgacggtaagccgtcaattaacctttcaattacccacaagtctggcgtctcggcggtccacggaatgatcgagattcccgttattcctcgcaagaggactctgccaacgggaacggatgacaaagtttgtgcggattgatggagccagcaagccatccgacaatgggtcatggataaccggcgaggtcgccggttgcgagtttcgcgactcacgattgggcaagagattgagcagcttgcttcaaaaactcggcggcaacatcggaggcacgatcccgttcgcatgccaggactgggctaacaccaaggctgcctaccgattcctgtccaacgtcgatgtcgacgaacatgccattcttgctgggcacttccaggccacgcgtgatcgggcccaggcgagttgcggcccattgctcatccttcaggacaccacggagttctcgtacaagagggacaagccggaattgatcggcttcaagggggtgactcacagccgacgtgacgaagcgggccgtccccaaccgcacactacctgcggcatcttgatgcactcgagcctcgtcgtgacggcacaggggctgccgctaggcctgtgcgcgatcaagttctggagccgtcagaagttcaaaggcaccagcgcgctgaaacgcaagatcaacccgacgcgtgttccgattgaagagaaggaaagcgtcaagtggctgctgaacctgcgccagtcgagcgccttgatcgacgagcccgagcgctgcgtgcatattggtgatcgcgagagcgacatctacgagttgttctgcctggccgatgagctcggaactcgcttcctggtgcgaacctgcgtcgatcggctggctggcgatggcggtcacacgatcgctgacgaaatggccgaggttcgcgtgcggggtctgcatcgcgtcgagttccgcgacgagcggggccagccttgccaagccaccctcgagatccgataccgccgtattggagtgctgccgcccatcggcaagcagaagctgtacccggcgctcgagttaacggtactccatgcgcaagagcgtgaagcgccagccagtcgcgccccgctgcagtggaagctcatcacaaacctgccggtgcattccaaggccgaggccatcgagaaaatcgactggtacgccatgcgctggaagatcgagaccttccacaaaatcctgaagtcgggttgccgagccgaggactcccggctgcgaacagccgaccgcctgaccaatctgatcgcgatctactgcatcctgagttggcgcatcttctggttgacgatgctcaaccgcgcccaccctgacaccggcccaggcgaggcgttcaccgataccgagatcacggtgctggatcagctgtcaccgaccacggctgttcccgagttcttgcctcggacgctgtcgcactacaccatcaagttggccaagctcggtggctacctcgcgcgcaaaggcgaccctccacccggcaacatcgtcatgtggcgcggcctcacacgcctaaccgacatcgtcctcggtatgcaactcgcggcgaaagttgtgggtaattgaaagcttgaggccacgcttaccgtagtcttgggagaattgggcatctagcgccggtgcacagctccaaggtcctggggcgtaacatttcctatggccagtcgtgcctacgagatagagcgaaggattttccctgggttcatcagattccatgggtcgaatgccgacttcaccatcagcatcatctgcaggtcgatggccggcttgaatcgcaccaggcgctctacgtgcatcctgccgatgccatgctcggcgctgatgctgccaccgagttccacgcttgccgcgtgcacgatgaggttaacgctcgcggccgccctttcgcattgctccggcgtgccgtagaccgagcgtggcagcaccgcaacgacgtggatgttaccgtcgccgatgtgtccggcgtggcacaccgcagctcccgccacctgctgctcgatgcgctcggtcacgaggtcgatgaagcgcgagagcttcgagaccggcaccgacgtatcgttcgagacggtaaagcccgctcgtttgttggcttcggaaatgttgtgccgcagctcccagatgcggttcgccttggccaaatcggtcgcgactactgcgttggttaccaagtcgcgctcgaaggcttgttcgagcgtgttctgcaattccgcgacagcatcccagtgcagcgaactgtccgcgatctccatcagcacgaaccaagggctatccagctccattggcaactgaaggccatggccatgctgcaggaccatctcgacctgccggcgcgacatgatctcgaaagcttcgatgcgattacccaccagttcctgcatgaagcgcagcaggtccaccgcaggctggacgcccggcagcgccaccatggccgtggcggagacattgagacggggaaagagctttagcactgcggctgtcaccacgccgagcgtgccctcggcgccgatgaacagctgcttcaagtcgtagccggcgttgtctttgcgcagcgcccgcaggccgtcccacacgcggccgctcggtagcacgacctcaagacccagcaccagttcacgcatgttgccgtagcgcaagacgcccgtcccaccggcattggtcgaaaccagcccgccgatctcgcagctgccgacgctgcccagcgccaatgggaactggcgctggctctgttcggcggcctctcgcacatgggccaggatgcatccggcttcggccgtcagcgagttgttgccggcatcgatctcccggatgcggttcatgcgcgacagattgaggatcacggccgagcgcccgggttccgcgaccgcgccgcccgtcaacccggtattgccgccttgcgggacgatcgccacttgctggctcgcgcaggccttcacgatctcggccacttcgttcgtgctgcccggcagcaggaccgcgattgccgcaccccggtatcgcccgcgccagtcctgctggtacggctgcgtgatgcccgtatcggtcagcacccgcgtagcgccgacgatcttggcgaactggtcgagcaaagcagcggtgtcgagactcatgctttctcctgggcaatgacacacacgactcactccctcttgagtccgccgatggatttgatgaccgcgccccacttggcgagttcggacttgaccagtgcatccagcacttcgggcatcgatcccacgggcaccgcgctgaggtccttcagcttcgcctgtacctccggcagcgcgaccactgcctgcagctcacggctcagcagttcgaccaatggccggggcagctttgcgggcccgaacacgccgttccaggtgtaggtttcgtaaccagggatcccagcttcggcgagcgtcggaatgtctggaaaagaaggcgaacgcttgctggttgtcactgccagtgcacgtgccgacccagcccgaatgtgcgaggccgcaccggtgagaacgtcgaacaggatgggaatgtggcggccgaccaggtcggtcatggcggggccgccacccttgtacggaacatgaccgatgtccacgccggccatggatttgaacagctcgcccgagaggtgcggcggcgtcccgacaccggacgatccgtagctgaatgtgcccggttgcgacttaagtagcgcgatcagctcctgcacgttttgcgctttcacggacgagttgaccagaaggacgttcgggaccgtcgcgacaagtgagatggccgtgaagtcgcgctgggcgtcgtagggagcaggcggtgtcgatagcaggttgatcgcgtgcgtcgcaaccgtgcccatcagcagcatgctgccgtccgcggctgccttcgcaaccttcacggcgccgatggccccgccgctcccggcaacgttttccactaccacgctgtgcgcgatgcgttccgacagcttctgcgcgatcaggcgggaaacgatatccgtcgctcctccggccgaaaaagggaccaccaacgagatcgatcccttcggcaagaccgattgcgcgaagacgtgcgacaacggcgcgcccagcgtggctgcaacaccccacttcatcatattgcgccgagatagcttggtggcggtcatgctcatgtctccgtttatttatgggcaggatcaacaagaatcataggttttgatcaaagacagataacaatagaatattggcatacctgccatcagcgttcttgatggccacgggtgatcggcggcgagcaccaagagacaacgtctacagcggctggcttctctcacgggcttttgggcgcacttgcagcggcctggcacacgcattcacccgcagagatcggaaggaagaaaacgaaaggcgtggctccccgtcttccagactggttcccgagctgttgccacagggatgcgatggccttgttttttggagcaacatcggaacagttgtcgatgccgtccaagaatcggaatcaccaccacaggcgtgccgcgaccgagggcctccccctgaacgcagcccttacttccgagccgggcatcacgcgtggccttcactcgccacaaagaattcgaaccacccacagcgttccgcgaactggctttcagccggcacgccggctcgtcctccgggcgccctccggctcacccaggttgatcggctcacacacccgctgcgcaagccgggcgccattgaatttgatgggattggacaagagcttcatttcggcgtcgcacgggtgcggaacattcgcgaccatgtcgatctcttggagaaatggattctcaagcgcctgctttacgttgaggaccggcgagatcggaagcaccccagtcagcacttccagccagtgcgccgttggatactcgctgaacgccagatcgagtgccttcgtcagttcggcacggtactgggcgcggactttctgggaagtgaagcgtgcatcctccgtgagcgccggtttgccaatgaccgccagcagcgcattccagaacttgtcggtcatgcacatgacatagatccaaccatcacccgtcttgaaagtctgcaccggggtgacagagaggtgagcacctcgaggcagccgtcgggacgcatgaccttcgttcagataccaggtgcctgcgtatcccagctgatggagcgcgacgtcgaagagactgacatccacatcgcagccgacccccgtcatttgcgcgcgccgcactgcgccgagcaggcccaacatgccggtaatgcccgtcatgtagtcaatcaccgatgcgccaaaacgcgcaggttcaccttcgggatcgcctgtgagatccatgaggccggactccgcctgcatcaagaaatcgtacccgggccaggccgcgcgtgagttgttgcggccataggcggaaatgtgcaggcagacgacctccggcttgaccgcctggagatgctggtattccaacctgagtttctccggctgatctccgcgcaggttgttgacgacggcatcggcgcctgccacgagtgactcgaaggcagcgcgtccctccggggttttcaagtcaagcgagacggacttcttgttggtgttccatccctggaacaccaagctgtcgtcagtcccaaggaaatagggccccatgaagcgggctggatcgccgccgatttccttgttctcgatcttgatcacttcggctcccatgtcggcgaggaacatcgagccgtacggaccggccgcgaattgctcaatggagaggatgcgcagtccttcgagtggcttcattggtcttccttattcgacggacaacttggcctgctttgccaatgcgccgaactcggtcagctccttggcgatccgggctttcagctcagcgggcgaactggtgagtggctcgatgccttggttgagcatctgctttcgaacttcggggtcgttgacgattgcgacgacctcggcattcaacttgtcgacgatcgcctgcggcgtccccgcaggtgccagcaggccgaaccaggtaccgacatcgaattcggcaacgccagcctcggcgagcgtgggcacgtccggcagtgcgctggagcgcttggcggtagtgaccgccagagccctggtcttctgggccttgatatgcgggagcgccgaagtgaccgtgtcgaacatgaccgaaacctggccgcccagcagatccgcgaccgccggcgcgctcccgcgatacggaatgtgcatcagcttcgcgccggtgcgcagcttgaacatttccccaatcaaatgatgcgcagacccaggacccgccgagccatagttgtacttgtccggctcggctttgctgagggctataaggtcctgcaccgatttggcgggaaccgacgcattcaccaccaccacgttgggcaccagggcgatcaggccgatcggggcgagatctctctcaaagcggtacggcaatttggcaaagactgcctgcgcgatcgtgtgatgcgccgcgccgaccaacagcgtgtagccatccgacgcggcttttgccacgaagtccgcaccgaccgtggccgatgcaccggatttgttttcaatgacgacagcctggcccaagctcttgctcaaacggggcccgatgattctcatcaacgtatcggtagtgcctcccgcgggaaatggcacgatgaccttgagaggcttcgtcgggtaggcggaccctggctctgtggccaaggacgaaaagatggtcgacgcggcgagggccccggcgacgccgacgatggtgcgacgctgcattctgaatttcacggttgtctcctgttcagttttaggcaatggatgaaagcccgtagctctacgccgcggcggaaaacgttggatcgagttcgctgcttgcaacgatgccgctgtcgtggagcctgccaatctcggacgcggacaggcgcagaacttcggccagcactgcgtccgtgtcctggccaagaagtcctgccggtctgacagcgctcctgggagtgccgatctgacgcacaggtgtgcctgctgcccaatgctcacctacccctggggtcacgacacgctcgtagataggattgcggcttccgacgcgcgagtcttcgttgagcaactgggtaacggtccgatagggcccccagcacacattccgcgcatccagggcagcaccgacttcaatgaaagtacgcgccgcgaaccacggtgcgagcgcgtcggcgatctcctcacgcgactcgtgtctgctcgcttccttggaaagatcacgcccggtcacccgttcgatcgaagcgatgctcaactccgcatcgcaagcggccacaagcgcgcgccactgaccagccgaaatgcccgccaccatgacgcgccgaccgtctgccgtgacaaagtcacggccgaaggcaccgtagatgttgtttccaatggccgggcggtctcgaccgtagagttcggcttccgtcatcacacccaggtgcgacagcgaagaaaacgcacatctgatagtgcaatctgcagctccgccccctgcccgttcagcttccgatgccgaagtgccgcagtcagggcgaaggccgcctggtatgcgcaacatgcatcccaggccggaaacacactgttgatcggttccccgcggaggcccgaagcctgggggtagcctgtcgaacaattcaccgtgtagtcaacggccgtggacccgttggcattcccttggatggtgcagctgatgacgtcgcttcgcagtgcggccagggtctcgtgagagagccagggcgttgcaatgttggtcagcaatacaccaccttcttcgtccggggcgcagacgaggcgctgcaccagttcccggccttctgcccggcgaatgtcgactgcgatggatcgcttgtccttgttgagaccggtccagtagaggcttctgccgctctccgcggtcggcatcctgccgtaatcaatgccgcccccgatcatgtcgatacgaatgacgtcggcgccaaattgggcaagggtcaagccagcgagtggcgccgcgataaatgcggagctctcgatcacgcgtacgccgcgcaagtgctgatagttcattggacccgccggccgccttaagcgaagttggcggagcgcttttcgagaaaggccgagatgccttccttcgcgtccgccgaagagaacacacggtcgctggctttgagcgactcgcccacggcttccgcatcggacctctcgaaggccaactggatggttgcctttgcggcttgcagcgcgagcgctggaccacgactgagtttttgcgcgatctctctggcagaagcgagcgccgtgccctgatccacgacgcgatttaccaagccccatgccaaggcttgcgccgcagtgatcggctcgcccagaaagaccatctcttttgcgcgcgcctccccaatccggcgcgcgacccgataagttcccccgctgcttgggaatacccccagcttgatctccggcaggcacagcttgacttgggcttcggcgacgatcaggtcgcagcagacggcgatttcaagcccgcctccgtagacgtagccgttcaaggccgcgatcgtgggcttgggaaacgaacgcagctgttcgaagaccttgttttggaaaatgagctttttttccaacgctgccccaggctcgaacatctgggtcagttctgtgatatcggagcccgcgcagaatgcgcgggctccagcaccggtcagaatgagtgcgcggacgctgtcggccctttccagggctttgagcgtctcgtacagctgccgtgtgagcggcgccgacacgacgttcatcggaggattgttcagaacgatgactgcatagccatcgctgatctcgagttcgattactttggcgtccatggtcttgccttcactgtgcagccggcaagactatggcgcaccgcgccagcgggtgcgtggctaggtcatgccgctggtggcccggaagcgagccgattgggtgtagcgatcgctggggtagtaactgatcgacgactggatcagcgtgccattgacgtcgtaatagaagcgcttgatcagcagcgcggcgacccccgcctcggcgtgcagaatctcggccagtttccggtccaggttgaccgcagagacgtcttgcctgacttcgtggacacgcacgccgaacatccgttcgatgttcttgtagatcggcgtattggagaccggtggagtcacctgcgcctgggcgtaccgcggttgcacatagatcaacacgtagctcatcggcaagtccgagcccggtacttttcgcaagaatccagcctcggaaagcaggagcccttccttgcaatcgagctcgcgtgcgagttccggggtcgtcgtcacctcgccgagcgacaccgcgtgcatctgcgtgttgcccacgaagctcaacaggtcttcgatcgagttgaccgcgctgaacatggcgcgtggaccgggcccgcgcacggtcgtgccgatgcccgggtgcgaagagatcagcccctcttcccgaacaatgcgcaacgcctgtctgaccgtctgccgactcacaccatagcgctcggtcaattctttttctgagggcaatatgctgccggcctggtatttgccctcttggatgtcccgagtcagcacgcctgccagtgcggagtacaacggctgccgcccaggccctgtcgcaccgagctgctctttgggcgctacttcttctgccatgaaatgaatgtccttgcttccgttcgctcgcaatgaggcattgctcgtcgagcctcctcgcgataagcaagcattgtgcgatggacaggtagggtcgggaaaaggagatcgtcgcattcggcagtagcgtctggacgcgcgcagccggtgagctatcaccaaggactggcggtttggcatcactgagcgagaaggttttgagattcatttgtacggatatcctaatgtacgtacattttaaactgccggccgggctcaagaaacattggtaaaccctaagacagctttggcccgtccttggagccgcgaactccagtcgtgggcccttgatgaaggcggcttgatcgaccgccgtcgatcccgctcgccgcttttatgacggctgcatcaaatacgagacgaacagcgagcgcagaaccggcagatggcccgcaaagaagtggtccgccccggggacgacaacgacgggcaacgtctgcggacgagcccattgcaagatcgagccgagaggtacgctctcatccatctcaccgtgaactacaagcgtgccaggtgggacggactctgtcgggtagctgcgtttcccatcaacctcccccacaggcaggctgaacagcacaatgcgaccggcagccgctcctgagtccgacaggcgcttggccacgcgggacatgacgaatgatccgaaggaaaagccgatcagggccaatgggagcgtaggatagctgtctcgcacctgggcgatcaccgccagcagatcttcggtttccgcatatccgtggtcgtgctgcccgtcgctttttcccacgccccggaagttcggccgcaatgacagccacccgaggtcgcgcgcggcgcgcgccagcaggtgcggaatcttgtggcgcgcgcttccgccgagcaggggctgtggatgggcgacaagcgccaagccgcacggcgcgtcggcaggcgaatcgacgagcaactcgatgcgccctgccggagcctcgagcatcagccgtaccgagtcgaactgttcgcctgtctgaagttccagcaacaagcgggacacggtactttctcttccgatccgcagcttcagcgcggagccagagcgcgaatgaagacttcggggtccacgttgccgccagaggctacaacggccacgttcttgccagcgagatcgatcttcttcgcgagcactgcggcgagagaggcggcacccgctggctcgaccgccagcttgagaaagcgaaaggctgcagccatcgcagcaagcgcgtcctcatcggacacgctcagccctcttgcgccatggcgctggagcaccgtcaggggcaacgcccccgccagcggaccgttgatgccgtcgagcaatgtgagccgccccggcggattgctctcgggctttccgctctgtagcgagcgcgccattttctccaaccccgcgggttcgacgacgtagatctgcgcctgcgggaaggcgctcttgaccgcttccgcaacaccggacgccaagccgccaccgcttgtgttcaagaggaccgcatcgggctgtacgccaagctcgtcaagttgctcgcacatctcgaggccgcaggtcccctgcccggccatgatgtccaggtcgtcgaagggtggcacgaacgtcatgccgcgctgctgggcgatgcggcccgcgatctcggcccgatcctgcgtgagcgggtcgtagacgacgatctccgcgccccaccatcggcagttgtcgaccttgatggcggccgcattgttcggaaggacgatcaaggcggggcaacccacggcatgggccgcggctgccaacgcatgcccgtggttgccagccgagaaggtgaccacgccccctcccctggacgcatcgtccatggcaaggagcttgttcaaagcccctctgaacttgaacgcgcccgtgcgttgcaacgattccgccttgacatgaatcttgcaccccgcgagctggtccagcatgggcgaatccaacaacggcgtccgcaccacgcgccccctcaggcgttctgcggctctgcgaatatcagagattgagaagccgggcatgggcgtgcggcgcgtcaatcgcgcaccaccaggatggcttcgatctcgacaaccatcccgtgcggcagggaacccatgcccacagccgaacgcgcatggacaccggcctcgccgaacagcgccgtcaggaggtcggagcatccgtcgatcacacgaggatggaatgcgaagtccgcggatgcattcaccattccaagcagcttcacgatggactgcacctttgaaagatcccccacggccagcttgaccgtcgagagcagattgagggcggtctgacgggccgcgtcgtagccgcgcggaatatcgtccgctgtctccagtcgtccccgcaggtacgaaccgtcgggaaacttcggtccgtgccccgacaggtagagcagatttccgaccttgcgaaacggcacatagttggcgctcggcgccatcgggtccggaagcaccagcccagcgagcgaaagccgtgcttccggatgcatcgggttgtcgaaattgtgaggctcgccgtgcacgattaaattcccttgttcgacggattgctgtacgcctcgcgcaccgcattcgacatcgggaactcgagattcacgttgttcggcgggaccggacgcgtgaaccacttggcatagagctcgttgacctcgccgctcttcatcaggcttgtcagagtctggtcgaccagttccttgaagcgtgcatcttccttgcggaacatgaatccatagggttcgtcccgcaggcgctccggcagaattttgtaggtgcccggggcacgcgcgttggcgatgagtccggcgagctgcacatcctcgagaaccattgcaacggcgcggtcgctggacagcaggagaaaggcctcggacgtgtctttgccggagatctcggcaatgtccaccttctcggtcttgcgatacgcgcgcagcagttgaatcgctgtgctcccagacaccgtcgcgaccgtcttgccaccgaaatccgagaaggtattgatcccagagtctttcttgaccgccgcggcgatgctgccgacaaagatcgtgggggcgaaatcgacctgctgagcgcgtgccaccgtattggtcgtggtgctgcactcgaggtcgacggtgccgttctgaaccaggggaacgcggttggttggcgtcacgatcgtgtactgcaccttgaggttgggcatgttcagcttggccttgaccgcatcgacgaccttcatgcaaaggtcggccgaatagccgatcgggtcggcggccgcggataccttgtacgagaacgggaatgacgcgtcccgccccccgagatgaatgaccccgctgtccttgatcttctgcagcgtatccactggttgggcggtggccactccgtggccttgtgcggccagcatgacgaatgcggaaatcagcgcgtgtttcagatccatgaacatctccagaaaagtacgagaaagtggaatcgctggcgatcggccggcgcgttacgcgccgcgtgcctcatcgcatgacgaagggattgccggcgaccgcgccgctgttgatccagacggtcttgacctggagaaactcccggatggcgtcgatgccgttctcgcgccccagaccggaatccttgtagccgccgaaaggcgccatgaagctcacggcgcggtaggtgttgacccagacggtgccggcctgcagtcgctccgacatgcggaccgcgcgaccgatgtcgcgggtccagacggcggcggcaagtccgaagcgcacgtcgttggcgatggctaccgcctcagcctcgtccttgaaccggaggaccgacagcaccggcccgaagacctcttcctgggcgatgcgcatgctgttcttcacttcgccgaaaatggtcggctcgacgaaccagccattcccgcactcgggcttgtcggctgcacgcccgcccagaagaagcttggcgccgtccttgcgggcgatctcgaggtattcgagcaccttgctgtattgggccggcgtcgtgacaggaccaacctgcgtcccggcctccatcggatcgcccatctttgcgctgcgcgcgatatcgacgagtttttcgacaaaggcgtcgtagatgctgtcctgcaccagcaggcgcgagccggcgatgcaggtctggcccgtggccgcgaagatgcccgagatcgcgccgaacacggcctgctcgaggtcggcgtcttcgaacacgatattgggcgacttgccgcccagctccatcgccgtgtgcttgaagtgccgcgcggcctgttcgttgatcgtgcggcctgtcgtgtcggaccccgtgaagctgatcttccgcacaaggggatgctcgaccagtggcgcccctacgtccttgccgaagcccgtgacaacgttgatcacgcccggagggaaaccggcttcgtcaaagagctcagcgaactccagcgtcgatgccgaggtgaactccgatggcttgatcaccaccgtgcagcctgctgccagtgccggtgcgatcttccagctggcgagcatcagcggcgagttccagggggtgatcgccgccaccacaccgagaggctcattgcgcgtgtaggcgagatagcctttcttgtccagaggcagcacgctgccttggaccttgtcggccaacccgccgtagtagcggtaccactgggggatgtagttgagttgccccagcatctccgcaagcagcttgccgttgtcccgcacctcgatctcagcgagcctttgcgcgtcgcgtgcaatcaagtccgcgaggcggtgcagcaaaagcccgcgctgcgtggcgctcatctcggcccatgggccttccgtcagcgcggcatgtgccgcatgcaccgcgcgctcgacgtctgcgaccgttcccttcgggatttcagcccaggtttctccggtgtaggggttctgggtctcgaaccactgcccgtcggcggggtcgacggactgccctccaatgcgaagctgatagcgtttcatctcaaaacgacctcggcagcccgagcagatgctcggccacatagctcaggatcagattggtggagatcggtgcgacctgatagagccgcgtctcgcggaacttgcgctcgacgtcgtattcgttggcaaagccgaagccgccgtggaactggatgcatgcattggctgcttcccaacttgccttggccgccaggtacttggacatgttggcctgggccccgcatggctgtttcgcatcgaacagctcgcaggccttgaagcgcatgaggttcgcagcctcgacctcgatgtagctttccgcgatggggaactggaccccctggttctggccgatcggccggccgaacacgacccggtccttcacatagcggctcacccggtcgatgaaccaatagccgtcgccgatgcattccgcggcgatcaacgtgcgttcggcattgagcccgtcgaggatgtacttgaagccctggccttcctccccgatcaggttctctgccggaatctcgaggttctcgaagaacagctcgttggtttcatggttgaccatgttcggaatcggccgcacggtcagtccgctcttctcggcctggcgcagatcgaccatgaagattgacatgccctcggtcttctttttcacctcggccagtggcgtcgtgcgcgccagcaggatcatccagtcgctgtgctgcacgcggctgatccacaccttctggccgttgatgacgtagcggtctcctttcctcaccgccgtggtcttgatcttcgtggtgtccgtgccggtggtcggctcggtcacgcccatggattgcaggcgccactctccgcttgcgatcttgggcaggtacagatccttttgcgctttggagccgtgacgcagcaacgtactcatgttgtacatctggccatggcacgcgccggagttgcctcccgagcgattgatctcttccatgatgaccgacgcctcggtgaggccgaggcccgagccgccgtattccgccgggatcatggcggccagccagccggccttggtcagcgcgtccacgaacgcttcggggtaggtgcgctgctcgtccaccttgcggtggtactcgtccgggaactctgcgcacagcgcgcgcaccgcgtcgcggatttcctggtagctcgtgtccggttgactcattgcttcaccacctcagaacggagggaaaccgagttcagcgcgaaaccggttcttcacgaagacaccatcgcgcggcggcaaggcacgggggggctcgtctgcatggatcgcaatctgcgcgaaggccacgccctggcacgcgttggcgcgctccgcaacttcatcggcaccctcaaggcggtcgatgcggaacgagtcttcgatgccgaaacccttggcgacggccacgaggtcggtgcccaggctcgcatggctgcgctgcatgccggtttcaccgaagtgcccgttgtccagcacgacgatcgtgaggttcttcggttgacgtgcgccgatggtgccgaggctgccgatgcccatcaattgctcaccgtcccccgtgatcacgacgaccggcctcgaaggctgggcgagcgccagtcccaaggccagcgaggtggcaccacccatggccccccaaagatagaagttccggtcgcgatctccggcggcaaaaacatcgtacgagggcgagccgaggccggagacaaccagggccgagggtgtggctgcaagcagccgcgcgacgaaagcgcggcggtccaccgccgtctgtgtggaggtcgtcatcagttgcgctcccatttctttcgcccgatcaggctttgcgacagcagtacggcaaccttctcgcccgcgaggaaggcagcatccaggcccgcgctgacgatttctcccacttcgtcggggtcggaagctctcagcacggtgatgcccatcagctcgagcgcgccttgggtgttctttcccatcggggcctgccacgggttgaactccgcgtactcgccgcgcatcgtcacgagggtgaggaaggggaagttgcaactgttcagcagcgagaacatgttgacgcagttgccgacgccgctgctttgcatgagcaacgcggcgcgctggccgccgagccacgcgccgctgacgagggccacgccctcttcctcggtcgtcagcacggtgtcgatgatctcggggtcggcctgcgcggcacgaatggcgtaggaatggcctgcgtcaggcacataggcgatctgctgaatgccgccttccttgagtgcgtcgaacacggccttctgccagttcggcggctccttgattgcttccatctggtattccaattggttccgatgcagcaatcttattttgtgattacatctgttgaacaatagaattaggtgattgccgccatttcatttcagcatcggaagcaccgtggatttcaaacagttgcgcgcactcgtcacggtggctgaaaccgggaacgtgacccgcgcttcggcattgctcaacatcgtgcagccggcagtctctcgccagctccgaatgctggaggaggacgtcggcgcggaactgttcgatcgcaagcggcatggcatggaactgacagaagccggtaagacgcttgtggaatatgcgcggcgagtcctgggggagcttgatcgggcacgcgccgagattcgccccaccaagggagccatcgggggcatcgtttgcgtcggcttgctgccaagcacctgcgacctgctctccagcgcgctgatcacggccgtggcgcagagctacccgggaatccgcgttcgaatcgccatgggctacgccggtacgctgcagacctggctcgaagcgggagagatcgatgcggccctgttgtacgaccccatgcccacgccaacgatccgggtcaagccgctgctcgaagaaggactgtgggtgatcggcttgccttcgagccggctgcgcaagaacaagcccatgccgctctcacaactggccgggcggccgctggtcttgcccagcgcgccgcatggtttgcgcacgctggtcgaccatgctgccacgctgattggtcttcagttgaatgtcgtggctgagaccaacgccatgagcgttcagaagagtctggtgctcgggggacatgggctgaccattctgcccaccatcgcggtagcagatgacttgtcacgcggtcagcttgcgggtgccccgctgatcgagcctgctctgcagcgcaaaatcgttcttgccacgtcgtccacccgccacacgaggacgcctgtacgttgtgtcgtcgcagaactcgtgagatgcatgcacgaggccgtgcttcatggcgattggcgcgcagttcgatggctgggcgaataagcgtagtcgagccaatttcaattcggaactggtcggtgagcgatccgttcctcgaatgaatgcatcctgcgatcagtgaacgacttccgttggaagcggtgcttctaggtcgttccctgtgggccatgcaggtgcttcagggcagcgagccgtggatctggtgtgcgacgacttacgccggatacaaggccagcttcacacagggcgtcaccgagatcggctgcgctgcgtgggtattccggggcatcgtgaccgcccattccgggccatcgtgaccgagcattccgatcgaacgtgaccgttgattccgggctcaacgtgaccgatttccgggtagtccggaatcgccggtcacgatggcggaatcgatggtcacagcagcggaacgctgccgtacgtcagcgtgttggtgttgcgcatttcatccaccccatgcggggtagcctgcccggttttgccggagacaggcgtgcccgcaccaaggatcaacatgcgcaagatcagagacgtcttacgtctcaaactcgaagcccgcctctcccacgaacgaatcgccgcctctctgggcatctccaagggcgttgtggccaagtacgtcggccttgccagcgtcgcgggcctggactggcccaccattcaaacgctcagcgacacggcgctggagcgtcgtgtcgtgcaaggcaggctggaccgtccctcgcactacgtgctgcctgactacggccgcgtgcaccaggagctgcggcgcaagggcatgacactcatgctgctgtgggaagagcacgtcgcggcccaccccgggcagccgacctaccgctacagccagttctgcgagcggtatcggcgctacgcgctgcgcctgaagcgctcgatgcgccagatccaccgcgccggcgagaagctcttcgtcgactacgccggcccgacgatcgagctcaccgatggcaatcgggcccacatctttgtggccgcgctcggcgcgtccagctacaccttcgcctgggccacgccacgcgagaccatggtcgactggctgcagggctgcgcacgcgccctgagcttcatcggtggcgtgccgcagcttatcgtccccgacaacccgcgcgcgatgatcgcgagcccgaaccgctacgagcctcgggccaacgacacggtggaggacttcgcgcgtcactacggcacctcggtgctgccggcacggccccgccatccgcaggacaaggccaaggtcgagtcggccgtccaggtcgtggagcgttggatcctcatgcgcttgcgccatcagcgcttcgccaacgtggacgatgtcaatgaggcgatcgagccgttgctgcagagactcaacagcaagccattccagaagttgcccggcagccgcgcgagcgccttcgccgatctggatgcacctgccttgcagtcgctgccgctgcagccctgggagtgggcggccttcaagagcgtgcgcgtccatatcgatcaccacatcgagatcgacggtcatcgctacagcgtcccgcagaacctcgtggggctgctcctggaggcgcgcatcacggagcacgcggtcgaactgctgcaccgcggccagcgtgtcgccgcgcatcagcgcagcgcccacaagggtggcttggacggcgacactcatcttggccggctgaacgacaagcatgatggccggtggtgaggagtcgaaggcggcgtagccgccgtagacgacgagccaccggcggcgccggtttggtgggggttcacgatggcgggttcaggtctcaagaagaggtcggcccagtgccaggttcccgaatcaccgatcagcaggtacgcctctacatgaacacccgcaagaagaagtcccaggagttggccgcggccaaggccggcatcagcgagcgcagcgcgcggcgcatcgagagcgcggtgacgctgccctcccagaaccctcggcgctattggcgctcgaggcccgatccgtttgctgacgtctgggaggcgcagatcgttccgctgctcaaggccgcgcccaagctgatggccgtcacgctgctgcgcaagctccaggacgaccatcccgatcgcttccccgacggcatggtgcgcacgctgcagcgtcacattcgccagtggcgcgccgtgcaaggcccgcccaaggaagtgttcttcccccaggcccatgctccgggccatcaaggtctttcggacttcaccgcgatgggcgatttgcgcgtcacgatctcaaacgcgccgttcgtccacatcctgtaccacttcgtgctggcgttctctcgctgggagcatgttgaagtggttgagggtggcgagagcttcgaggcgctgtccaagggcttgcagaacgccctgtggcaagccggcggcgctccgcacgagcatcgcagcgacagcctgtcggcagcgttcaagaacctggccgaagaagaggacttcaccgtgcgctacacagcgctgctggatcactacggcatgctgggcacgcgcaacaaccgaggcgtgagccacgagaacggcagcgtcgagtcctcgcatcggtacctcaaggaggcgatcgaccaggcgctgctgcttcgcgggcaccgcgacttcgaggatcgggtgacctacgaggggttcgttcgtgacgccgtgatgcggcgcaaccggcgcaacgcggctgcgtttcgtatcgagcgcgagcagttgctggatctgccgcacaggcgcaccaccgacttcgtcgaggaggaggcgcgcgtcacgcgctgcggcaccttcaccgtacgcgccatcctctacagcgcgccatcgcgcctgatcggccaccgcctgaaggtgcggctgtacagcgaccgactggattgctacctctcgggagcgctcgtgctgacgcttgcgcgcggggcgcgatcgcccggcaccacccgcgggcgggtgatcgactaccggcacttcatcgacgagctcaagcgcaagccccaggcgttcaagggcttattgttccgtgatgcattgttcccgcgcgaggcgtaccgcctcacctgggagcaactcgacctgaagctgacacgtcgccaggcctgccaggccatcgtcgcgctgctggagatggctgctcgcgacggtgtggaaggcgtgctggccgaacgtctcgacgcgctgcgcctggccggcgagttgcccgatgtgaagcgtttgcgcgaggagttcgccccacgcaagaccgaggtgccgcagatcacgatcgagattccgccggcgagccgctacgacgcgctgctgccaagcgagcacgaagacgagctggaagaggtcgcagcatgaccgccgcagcattcgagcccggtcgcaacgccttgatgctcaacgagttgcgcctgccgacgatcggcaggctgtggcccgacttcgctgagcgctcggacagggaaggctggccagcaagccgcttcctgggtgggctgctggagcacaaagtggccgagcgggagaagcgccgcatcgagcgccaccgggtggagtcgcgcctggatgtgaccaagacgctggccagcttcgagttcgctgaggtgccgatgctgtccaaggcccatgtcatggcgctggccagcggggattcgtggctcgagaagggagccaacattttgatttttggtccgccaggcgtgggcaagagccatgtcggttgcggcatcggccatgcactgatcgaggccggccggcgcgtgctctacatgcgcaccagcgagctggtgcagcgcctgcaggctgctcgccagaccctccagttgccccaggctctggccaagctcgaccgctacgacctgctcattcttgacgacatctcgtacgtgcggaaggaccaggccgagaccagcgtgctgttcgagttgatcgccgagcgctatgagcggcgcagcatcctcatcacggccaaccagcccttctcgggctgggacaccgtgttccccgatgccggcatgacggtggccgccatcgaccgcctggtccatcactcgacgatcttcgagttgaacaacgtggagagctaccgcggcaagcaggccgcccgggaacagaaggtccagcgcgacaacgacaaggcgaatcgccggcgtcaatcatccagcgacaacgacaaccagtccaaggagccacaaccctagtcccataaaaaacgacattcacccctgcccaaccggccaagatgaatgtcgtttaaccggccatgctgcttgacgctatccagtggcttcacgaccgtcgtcgcccacctgccggcggcgcaccgcgcgcatctcgaatggacacccgagcgcctggtgcattgggggcagagcatcggtgtggccacgggccgcctggtggcgcgcttgatcgaggagcggcgccacccggagcacggctaccgcgcgtgcctcgggttgctgtcgctggcacgccgctatggcaaggaccgactggaggcggccagcctgatcgccctggagctggggacagcgaagtacgcgcatgtgaaggccattctggtcaacgagcgagacaaggctgccccgagcacggcgccgagctggatcagccctccccatgagcatgtgcgcggcccaggctattaccagtgacggtcgagcgcacccgctgaacatcccggacaacaaggaatccaatgatgatgaacacgactctggaccagctgcgcagcctgaagttgctgggcatggcagcaggaccagctcacgagcgccggcatgacgaccatgagcttcgaggagcgcacggcgttgctggtcgagcgcgagatccactggcgcggcgacaagcgtcgtgaacggctcttgaaggaagcgcggctgaagtatccccaggcggccatcgaagacatggatgcgcgcgccggtcgcggtgtcgatcgcaaggccgtcatgagcctggcactgggcgactggatcgattcgggccacagcgtgctgatcactggcccgacgggtgcgggcaagtcgtggcttgcttgtgcgctggcgcagtacgcctgccggcgaggccgctctgcgtactaccagcgcatgccccggctcggcgaggagctgcgcatccggcacggcaacggcaccttcggcaagtggctgatccagctggccaagaccgacgtgctgttgctcgacgactggggcatggcggcgctggatgtccaggccagatccgacctgctggagatcatcgacgaccgggcggccagcaaggccaccatcatcaccagccaactgcccatcgagcactggcatgcatgggttggagacgccaccattgccgacgcgatcctcgatcgcctgatgcagcaaaaccaccgactcaccctcacgggtgagtccttgcggcagaccgcgaaaacgtcccaaaaggagaagaacaaagacccatcgtgaccgccacttctacaatctgatcgcgcaactcagtacgcatgatgaccggtcacgatcaagcggaatcgtcggtcacgttcgccggaatacgcactgcgcacgcgaggcgcaagttcttcgaggctccaggcgagcaccaagagtgccgtggccgagcaggcgatggagttcttcggtgagctctaaggccaggcccgtggccgatgcgctacacgcatggatgatcgcgcaccgccttcgcgcgaccgatggcacggcgctggcccgggtgctggactacagcctgaagcgatggaccgcgctcacgcgctacatcgacgatgggcaattgccgatcgacaacaactgggtggcgaaccagatccgtccgatcccgctcgggcgttcgaactggctgttcgctggctcgctgcgggcggggtcgccgccgcactcgcagcccatgagcagaacgattgctaactaaatctcatcgcccggcgcattctgcgcccgatcggctctggatcttcgtcctcgccaatcagcctcggcccgatggtgcgatcggcgaccaagctcttcagggttgcgaccccgccgtcgagcgcgtcctcccaactgtcgaatacccccgcgctgccaaagagcaccgcaaaaccggtgggatcgtcaatgctctcgatgatgagccagtggaagacgccgcactccgattcctccacggtcacggcaatcgttctgagatggtcgatcacgggctgcgttctacgcgttggcttgccgcgtgcacgatcaggttgacgctcgcagccgccgcgtccgaaacactggggtcaggggtatccagtccgtcgaagagatcgacgagttccttgtctttcgcgttcatctgccggctccttggttgatggcttcgaattccttgtcgtgtatggcctcgctcgcgcaggaggcgttcgtgatgttctcccggcaggtcagcccggtctactccggcagcctcgtcgcggcctgcctggcgaacggcttctcgctgcgcgtgatccacgggattcgctcgatctcgtcccagcttgctttcgtcggatgcggacagggcatcgcgctggtgcattcatcctcaagcacctggcgccggagaacgtcgttttccggcgcctcaaggagcgccggaacgtcgtcaccacggctgttgcatggagcaacgcgcgcgccaatccagctgtcgatacagtcattgccaagctgggcgccggggagcggaaaaactcctgtgctcgctcagtccaagctgccgattcagacgccccgcctccttgacggcgttcggcatcggaaggttgatgttcgctcccgtcggaggcacgggataggtgaaccacttcacgtggatctcaatgatctctccaacggcacttgcacagagcgagagagggccccatggagccgagggctctatgctgtgagtcatgggcttaggcttacgcgcctgcaaaggcggtcactgcatccaattgccaatgtctgcgttgtagccttccccaccagtttcaccgtcgccccccagactgaacacatcgatttcaccgtgcaagcccggggcacggtattgcatgtcattaccccatgcatccttgggtaatttgtccatgtaagggcgccagttgggcggaatcttgccgctgctgggcttctggaccaaggaagtgaggccctggctggaggtgggatagcccccggcatcgagtttgtacaggttcagggcttgcacgatatctgcaatctgctgcctggttgcggcaacccgcgcatcgttggggcgatccatgatcttggggatcaccagcgcagcaaggatcccgaggatcgtgatgacaaccagaacttcgatcagcgtgaagccgctgcttctttgacgacgtggcatatgcaaatgtccttgctcaaaaattcaattgggaaatttgaagggtgtagtgattgggagctccagcgggccggagataagcgctgagaaatcccggggattggctgatcaaaccggcagcgtcggcaagctctccgttgaactgaagcccttgctgcgcagaatgcttgccctcgccagaaatcatcagaggaccgtcctgactggtgaccgagaagctcatcccgacactttcggcatggcccttcagcacaaatgaacccaactgccctttgggaatcaagctggttgcggcgttaagccactgcacttccacctgggatatcttggtggactgccagtttccttgcgccgaaatctggcggaagttcacaagaccgtgccattcgcctttgttcaggatgccaggcaagagcggcgtgagttccctggcctcgatgtccagtccatggagattggcctgccatccgctcgagccgatctgcaggtgccccacgggctgcccgttggcgctgacctggaaaagcaggcgtccattctgaaagccaagcagcttccaactcagtggtggcagggagacctggcgcgggctcttgtccggcttgccggtgatcacgccacgcccgttccaaagcgtgccgtcgacatcggccagactccacaagcgatgggatgcctgttgaagcacgatgccgatgagactggccggggccagccatacgatgaagaccaaggtcagcaggccagtgacagcgatctgatggaagcgcttcaccgtctagtcctttccaagtgcaagggtggcctggatttcgacaatgcctggtcgatccgtccgagtgacttttgctttctgcacgaccaggcgcatgtctttctgcacaaaggcgacccattccaaccattgatcgaatggaaccaagccttgcaatccaacctggtcttgggcgtccagagtctggatgatttcggtgggcaagccgaatctggaaagtgaatcgatcaccgaaggcgtatgcacctttttgacattgctgccagctgcaggaagctgcttgatttgccgcagttcgtcggcctggacgcgcatgacgcccagcgccttcagttcagccgcccattgggcccgcgcctgctcctgggccgaggccagtgcaaaccagaaccagaccaatgccgccacggccatgccgacgaaccatgccgctagcaggcgttggtctcttctggacaggcccttccaccagaattgcaggtgcttcatgtgccttcctttgacaccagcgccgtggtgacgacgccgttgttggctgattgggtgacggcggtgtatccgcgctgccgcatgccggcttccagtgcgcgggcattctgccccgtgccgttccagacgacgatcattcgcccctgctcatagtccaggctcgtcagcctggcttgcgcaagttgctgcgccaaggcggccagcaccggcacgaactcctccgaccgcgattcgccgacgtgcgcacgcgctgcctgccacatctggtgcaagtggcgggcgggcttgtcggtcttttcggcgctgccgcccacctcctgccagagagccgactgctcagccttgacctggcgtgtggaccaccaggtcttgcccagatcggtcagggccatcagcgtctgaatggccatgcaggcggcaatcgcgaccagcgcggtcctgaacgcgggttcggcgaggagtttgcgccggggcatccagtcgcccaccagcaggttggggctgggttgcgacaaggtggtgtgccaatccagcgcagccgtccgctggacaggaatgccccattggcgttcctgtccaaggaagagcgtggacgcaaggccgtgcaagaccatgcgggccggtgactggccagggttctgtgcccagcgcaaggtcagcgccacgggaggctcgccgcagtcggcgggcatgtccaaggccatggccgccacgccgtcgtgcagccacagatggccgtcctcgttctggaaaatccgccattcgtccggcgcagcggggagtttgtcggccaacgactccacgcgcaccaaaggccgacccagttcccggaagctggcgagcagctgctccagccgttggcgttgcaatgtgcagcaaaccacgtcatccccgtgcaggcgcaaggggatgacgaccagacggcccaggtcgtcgatcagcgcgtcttccagcgccatggcgaccgcggcggtgtctttccagttcacgccggggggcagtttcacgcggtggtagaccagctgctcctgggacaggatcaccacgtgctcggtggcctggggccaccgctgtggcgcatcctgcccggtggcgatggagcgctccccgtcgagcaggctccacgcgcagtccaggtggcgatgcggccagcccgcatcgaggtagagatacaaggttcggctcatgggcgtttcatccaaacaacgtcgggccaggtgccgggctttcgtctcaacagggcaaccgcagaagcgcgcccttgcccgaaggtggcatgcacttcaaccctgaagaaatcactgcggaccgagatcgactcggtgcggaatccgtctctcacatcaccggtcagcaaggtatagaaatcgggggtgtagtcgaacggcgaggccgcgcgcctgtcgaaaatctccttggcctgctggaagctgagtcccggaacaatggcgtagatcagttccaccggcgcggtgttcacgttcagcttggaactggtgtcgggcagcagggtgatgtatttgcccagcttttcaatcacctcagacgtgtacccaggtatggcctccaagctggcggtgcccatgtaacgaacccgttcagaggctttgccagacagcttcgatctcagggatacggccagcgcttgaggcagttccagcgcccccaacaggcgttcgtactgttcccacgcgtagggatcgcccgacagcagccacgccatgttgaatttggattgctcgtcaaacatctggccactgatttcgccaccagccaccgggatcgggggaacccgggtggcccaggcctctcccaagtggtccttgcggatgcgctgacgctgccgttcgtacacgaccgaacgggcccagtcaacgccgcccatcaccagccggtgggcctggcgtgcgtctcggagcatcttcacttgagtgacccagacatcgacgcgccagaggatggccgatgccagcacggtgactaccgccaccagcagcagcgccatcaccagggcaacgccttgctgatgacgcatggaggccgttgcgcgggtgctcatggcagggcatagacccgtgtgacgtcgcgcccgtcgtccagcaccagggtgacgcgcaaggcgcggggcctggcatagggagtgccttcgagtggccagctgccgtgccattcgccctggtcatccaggaaggacagggtcatggcccgcacgccgccgagcagtggcgtctccaggccttggacagtgacctccgttcgtccggtaccaggccctgtatcctgcgggcgggacaagtctgcttccagcatgcgtaccaaagtgccattgcgcaacgcgtactggacgggccgcacgcttcccgcagtgccccagatggtccagtgggccgcggcgccatggccccgccaacggacctggggaacatccgcgggcaagccatcgacagcgcaagtgacgtcgtcccccatgcgtgcccaggccatggcgatgctgcgccagcgcgcttgttcgtcatacaccacgtcgcgggctctgatgacttgcgccaggcctttgctcgccatggcccccagcactgccagcaaggcaatggcgaccatgacttccaagagggtcatgccctttgtcgtgcgccgagaagtcaaaagggctcccctggtcttggattggactgatggatcaaatacccttgaaccactacctttgccgtcggatcgtctttcagggacacatgcacgtccaccttgcgtgccaacgggctaggggtgtcactcacttcttcgacaacgacaaaatcaagcccgcactggcgctcggcctgtgcgggctgtatgcctgcgtccagccagtcggcgcgtgcatggtgcagttcgagccggttctgccccacccagtcggcacacatctgggtgcgaaggcgcagtgcattggcggctgtcaggcccgtggacctgacggccgcgatgagaccgatgctgagcaccagcagcgccaccagcacctccagcaggctgatgccctgaacgccatggggcccggcacgatgcaagcgtgtgcagcgcattcagcttccttgctccaccgtttgcaccacgctgccggaagctgtggtgtcgaggcggatggtccgcggcccatcgcgcagccggaggcgcagcagtggcggtgtggccccgatgaattcgatgcgcaacggcggttgcatggccttgttgtcttgccaagcctgctcgatgcggacgtcgtcgctcaattcgcccgccttcagcccctcggtgtcggaggtgcggatccaggtgccgtcgttttggcgcttctcgaagtgatagtgacggccattggtccccaggcgcaggtgctgccccccgatcacgctggcgaacatggccgcctccagtgtggcgacgaacttttccagcgaaacctgccgctggaccgccgcggcgttgcgggcgctgggcatggccatgaccagcatcacccccaggatgaccatcaccaccaggatctcgatcagcgtgaatcctcggccacgaagcgtcctggcaaccatcacatgagcacctggttgatgttgaagatgggttgcatgatggccagcacgattaacaggaccatgccccccatcaccagaatcatcagaggctccagcagccgcaccagaatggtcacatcatgttccagcgacatttgctccaaccgggcggcctgggcgagcatctcggccagctgaccgctttgctcgccactggcgatgaggttgatcagcaggggcgggaagccctctttgcgcctgagcgcccggctcaggctcttgccggcattgacctcctgcagcgcctcgcccacgatctccttcaggggaaggcgctccagcagccccttgccggcctccagggcgagaagcagcgggacgccgctgcgtaccaggatggccaaggtgctggcgaacctggccgtgtctgcagagcgcatcagttttccgagcacgggaaattgcagaagcctggtatccactgcacgccggaatccgtatttcttcatggcattgcgccaccacacggcggccagcatcgccgcgcccagggcatagcctccgccttcgcgcacacctgcactcacgctcagcaaggcgcgggtgagcagcggcaaggtctggcgctgattctcgaacaccgtcaccacctggggaaccacgtaggccagcagcacgcccaccacggccagggccaccaccagcatgaccagggggtagatcatggcttccagcgtcttgctgcgcagcgattggctttctgccaggtagtcggccaggcgcgacatgacttcgctcagttcgcccgccgtctcgccggcccggatcaaggcgatgtacagcggcggaaaagtgcgcggatgcatggccaacgcatgagccaggctgtggccggcgcggacttcattgcgcaccgcgttgatgatgagcgcatgcgcgggtttgtctacctggccggccaaggtgaccagtgacgcatccacattcaggcctgcccgcagcagcgacgcccattgctgcgtcagcagaaacagggcccgcgccggaatgcggccccggtgcccacccgccgccgatgcaggggcgccggcctcgtccacggacaccggcagcagtcctttttcccgcagggcggtgcgcaactggggggcgctgtcggcctcctgggtgcctgcgacccgggttccggatgcatcgatggcctgatagcggaaggctttcatcgatctccagccacacgcatcaactcatcgacggaagtcacccccgcccggacccagcgctggccgtcctcttgcagcagccgaagtccgccgtgctcgcgtgcggtgtcgcgcaggacatgctcgccggcgccgtcatggaccaggcggcgcagccgatcgtctatggccagccattcgtagataccgagccgtcctgcatagccggttcctctgcactccgggcagccacgcgggcgaaatgcatggccccgaccagcggcctcgtccgcatagacagggtctggctctttgcagtgcgggcacaactggcgcaccagacgctgggccaacacgccgatcagactggatgcaagcaagaacggctctacccccatatccaccagacgggtgatggcactgacggagtcgttggtgtgcacggtggccagcaccagatggcccgtcaggctggcttggatggcgatctgcgccgtctccagatcccggatttcgccgatcatcaccacatccggatcctgtcgcagcaacgcgcgcagagcgcgcgcaaaagtcatgtcgatgcgtgagtggatctgcacctgaccaatgcctgccagatcgtattcaaccggatcctccaccgtcatgatgttgcggttgcgcgaattcatccgcatcagcgccccatagagcgtggtcgtcttgccggatcccgtggggccggtcaccagcacaatgccatgcggcgcgtggatggcagcgtcaaagcttgccagcgtatcgggcgccatgcccagcacggccaggtccatgcgcttggggtctttgtccagcaggcgcatcaccacgcgttcgccgtgcgacgtgggcaccgtggacacccgcacgtccactgtcttgcccgccagccggatggcaatgcgtccgtcctgcggcaggcgcttttcggcaatgtccagttgcgccaggatcttgatgcgtgaagacatggccgcatgcagcgcccggtgcggtgccagcacttccagcaactcgccgtcgcggcgcatgcggaccacggtgcggtgttcttcgggttctatgtggatgtccgatgccccctcgcgcacggcttgggcgatcagcgcattgatcaggcggatcaccggcgcatcgccgtcgctggccagcaggtcttcgaccggcggcaaatcattgaccaactggttcaggttcacctcctgcccggcggtgtccacaatcgatgcggcgctatccccgccatccgcataaatggacgtcagcgcttgcaagaattcctcgtctgggaccacgctgacgggaacctgcgcacccacggcgcggcggacttccgacagggcggccacgggcgtgcctttgcacacccacaggaccggatcgcccgcggcagaatgcagtagcacgctgtggcgacgggcaaacaggtacgggatccggcccgaggccaaagcattcagggcctccatctgctacctcggctcatccatcactgtcgcggtctctgccgcaggggctgttcgcgcggacgacgggttgagcgatgtgctggtcttcaggtccacaggggtcagcaaagggccagcttcctgcttggccttttcgttggtcgctttttgcaagccctggatgtagttgtatcgatccatggacagcgtggcatcgtcctgcgccgatcgcaacgtcttgggccggatgaacaccagcaaattggttttggagcgcgtcttgctggagtgacggaacagtgcaccggccagcggcacatcgcccagcgcgggcaccttgttttcgccgtcgctcaggctgtcctgcaacaggccgcccagcacgatcaggccgccgtcttgcacctgcacggccgtttcgatggtgcgggtgttgatggtggggccggaggcgttggtcacggagctcggcaccacggacgaagcctcctgaatgatcttcatgcggaccatgccgccctcggacacctggggcagaatccgcaaagacagccccaccttgcgcctgtcgaacgtctgaaatggcgtgaccgtggacgatgagttggtcgaggagtaactgcccgtgatgatcgggacgtcctgcccgatcatgatctgcgcttcctggttatccagtgtcatcaaattgggcgtggacagaatattcccgccgttggtagtttccaggaacgatgccaatgccatcaagttgttgatgacggccccactgggcaaggtgatggtcccgttggcgatgcccaggttcaggcccactccggtccccgtcgggttctgagccatgttcaggatgccggtggccgcacccggaaaattcgagcccccaaccacacgggtacccgtgctgcttttgtcaaggccgctaaatgcctgccactggaatccgaactgtgcagcagtgtcactgttcacttcggcaatcagggcctcgacatagacctgcgcacggcgcaaatccatctgtttgatcaccttgcgcagccgctcaatcacgatgttcggcgcactgatcaggatggcgttgttggccacatccgcctggacgtaactcccctgcactagtccacctgccgtctgccagccgccgctgctggcgccgccactccccgaagccccggccccggccacggctgtctgggtgctgccccccatgccgctgttgggcgccagattggactgccggttcgggttgagcgaggacgttgtgttgttctcccccgatagcgcgccggccgccttggcagtggtctggtcggcagacaggatggcccgcagcatctgggctacttcgctggcgaccgcgttcttcaggtaaatcacctcgatgttgcccccggcttccgggcgatccacctgcttgatgagttgctgtgcccgcaacagcttgcccggtgagctgctacggatcagcaggctgttactgtgcggttctgcatatacggcaaacccgtcacccgcaacagccatggcattggctccggaagccccgcttgctgcagttccggtggggcctacgacagccccctgttgggcagggccgtcggtcatcaggttctggatgatgggggccagttcggtggctgtggcatggctcagcggcaccatcaccggaagacccatgcctggcacatcaatagctccgaggatcacctccagccgcttcagattttgcgaatagtcggtaaccaccagggtgttgttcgcggggtaagcgatcacggtggcggcgttgtgaagcaagggcttgatggccggcccaacggcctgggctgcttcgtacttcaaggaaaacatccgtgtcgtgatggtgtcgcccgccataggggtgccactaaggcccacggccacagactgctggcgggcatcggcctcgggcaggatgcgtaccactttaccttcgtccaccacggcaatgccctgcaggcgcaaggccgcaaccagggtcggatagaccagcgagcgcggcatgggcgctgccgacaccacattcacattgcctttgaccttggggtccaggacaaacatcttgccggtcaattccgatgccagcttcaggaccatcgacacttctgcgttggccagattgagggtcacgggttcgtcggcggccagcgccgtcaacacccataaccccaagcctgcaccccacagcaacttgcgaaaactcatcggaaatccttgataaaggggggagggcctgcgggcctggattggtcttgcgggggttctcgatctggcccacctggggctgacgatctcaatggcagttcaccgcgcagcgcgtctttggacagcacgacgctgtcgggccgcacttcgactacctcgtgacccgaggacaatcggtctcccactttggccacgaccacgtcgaagccaccgtccgttgcaagcactgcgcggctgtgggcaccgggcacgacgtaggtgcccatcaatcgccaacgggcatcgatagtgtttggagggggggattcaccaacttcgctggacggtggtcgctcagttgcaacttcaaagaaatggcgggctgtcacgcgattgacctgctccgacagcgttgaagaagccttggcaatcaccgccgggctatctggtgcggcccgccaccagaagctttgagcaacgatccatgccactgccaagcaggccagactttggacgctcaacgggatggctttttctttacaccaagacactaggccaggcatcaaggggcttggcatattccagcgcatttatgtcctacttttctgattcctgcataccgccccacataaacaaaagccccggcctgagccggggcgggaacaggcgctatgtgtcaaagtaggttgcggttgttcaccacgtgaatcattttgtaaccccattgttgctcgttgccttcccagctaccgtaatccctccattcccacgaatacaaatatctataattaaatttggtctgcggatccctgcggaaatgggctccatgaaaatggccctttttccagcggcggaccgctacgatgaccggttgagcccattgccctggcctcagttcggtacgcatgtcaaaattctccgactgcgtttgagtccaagtcttctggcgttgaaattcgcctgacacactgacacccaaagcctgaattggaaagccgaagccaccgccgaccttccagccaatggtgtgagcataggacgtggacttaccttgcccccaagtaaagtggcagccgctggaattggagctgcaatactggacggtaccatctgatttcccgcgccagacccagtcatcccaagtactgctagcttgttgaatgacgcgcgcctgtgtgccgccatcggcatgggcctcacccaagtaggagttggtaccaaaccacgccaaggcatgcccggcagttaccagcagccctgcagcgacagccgcttgttttattcgcttcataagacctctcgatttttaaggacggtttaagaaaattggctgctatttatgcagcaaggtgggtttctgaaatcatgatttcatgaggagacccttcacgagaactcacgaactcacgaactcagggggatatttttttttgaggctcaaagaaaaaattctcaaccgagttattcaaatcctcgggtttgttgatttttccttgcgcgatttgctcgaccacatcggctttgctgtaaatgggaatgagccccaagcctccaccgtgctcttcaggcgcttttcgaatcaccactgcagtgatatccggtagtgatgcaccaatggcttcgtaggcaatttgggcggccttggcgcgcgattccggcgttccatcgctgtcgatcaacacccgccgatcccgatccaggctggcctggatgctttgtttgagtgttttgagatccgcggaggagtcggtgtcaaagacgtcgtatttggcgtcgggctcgcgcaactggccaccgtggtttttcagctcggccatcacagcgccgttgccgccgctgccggataccaagttgaaggcggccatcacactgaccgggcgggcaggttcagacttggcgggcgcggcattgggtacggcaagagtggtgatggcggtgccggcactctcggtgttggctccgcagcctgccagcacagacaagacagtgcacaggatcaaggatctcaaggctgacggtggggacaggatggcgctcatggattgctaacaactggtgtgtcagaaaagtaaagttctgttgccctggacaggggcaggatggtgcattgcgttcgcggcacaaacaaacgggtcactaagcaggtcaaggtcttcatggagtccgcgtcagggcatcgaataatatagtcataactatcatgtaactataactaccatttgtgtcaaaaattgctcggaagattcctgatgccacacgcgtccctcccataccgtccatccaccctcccccaaccctcgctggtcacgaagaaacagcccgcgcagcagcgcgccacagagacttgtgagcgcatcctggaagtgacggcgcagacgctggtcgacgtcggcatcgagcggctgtcacccaacctggtgagcgagcgcgccggactcacgccgccggcaccctatcgctattccccaacaagtacgcgctgctgtccgaactgaggccgcgcctgatgcaggcccagaacgcgcgcgttggccgctggatcacgccggaggtgttgaactggggcgtcgacagtctggagcgggcgatcgaggaactggtcatcgacacctatgacgcgacagtgcagaccgtgggcggggtatggatcatgcggggcctgcgcgctgtgcctgccttgcagctaggtgcgactggcctcccgcgctgccgttacacaagagcaggcccgacccgagatctcggccaggcctcggattccgcgatcaggcggccctccgatttagctcggcgacacgccttctgttcaagacggtaaccgtcaaagcggatcgggttggcgagcagcttcatctctgggtctgctggatgcggtacatccctcaccatgtcgatttcctgaaggaagggattgtccagcgcctgacggacattcagtacgatgcacaggcgcaagagaccatggccgaatacgagaaggcgatgctgggcgcgctggccgcgatgtggaggtcgcattcgcgcagatgcgcgcggcggatgccggcgtagtggagctcgaacaggcgatgaaggccagcacgggagcgggcccgtaagagtgagcgcctgttcgaggcaggtctcgccgatctgaacaccgtactggacgtgcggcgcggtcgactgcgtgcacaagacgcgctgctgcaagctcgcggaacccgctggatcgctgtcagccagcatcccgcaacgccaccgaagagcggagtgcggtcgtcgcggccttcttacttcgccactccgcttcgcactcgtcccttgcgccgtgccgtctcgccgaggcggccgacatcgggccggattcgaggcaggtggctagccaccatgccggcaacaacgcgggccacagccttcacgtcgaggggctcatcgaagagcatctccacggtcgcgtacatcaggtccaccacgacgcggctgaccagcctcaactgggccagatcgacctctggcaaggcctgcgccagcacttgggcctgagcctgcgtgacctgggcgtgtgactccagtcgaacttgttgcagcgcggggacggcccgcatcgcccgcatgatccacacgcctccgaccgtttgaacggttgcttcgtaggtgtcgaggatcaacccctcgagcgcctcctcgaggtcctccacggtaccgcggaacacatcgaccgaaatccattcggcgatgcgctcgttttggcgctgcatcaagcgctggccgagttcgctcaggagcgcgtacttgttcggaaagtagcggtacagcgccggcggcgtcagcccggcgcgctcgcatacgagattggttgacaaccgctcgatgcccacatcggccagcgtctgcgccgtcaccacgaggatacgctcgaaagtgtcggtcgcgcgctgctgcgccggttgcactttggtggccagcgagggttgttgctcccgcggcttgggcgtggtgttgatcatggacgacatcgggattctcccaggtcttttgcctcgtcacatgctagtaatgactatatactagttattactatctaatctgtgagtggcagttcgctcggcggtcgcagtcggtgcggcggttgacgactatgagagccatccctaccttggcacctcgtcctggctcggcgcgcacgtgccgctcatgaagaccgacgtgttccacaagattgccaccatcccttcctgcgcatcggtaccaccgccgcccgtctggcgatgaacaccgagctgttcgagaaatgtgccgaggcctatgttctggccgccgcgaccggtgggcaggtggaccctctgccgtgggtggtgcgccacgtcgcgaaccggcgactgatctgggatgaacgccgcgccgctgagcgtttcgcccacgggctgctgccagaagaaacgaaggggtattgatgcaacccgatcgacacgagacgcttggtgcgccgcaggtgggcgcggcgctggccatcggtacggtcgccttgctgatggtcggagtgcagcccattgcactcggcgaactggtggaggctcgcaaggtcagcctcgagggcgtgggagtggtagcgatgggtgagatcgtcgcactcggggtaggctcgctgatcggcgatgcgatgcttccggtcgcacggttgcgcctggtgacaatcgtcgctgctctgctcaccgttgtgatcaatctgctctccgcgttggccgatggagacgttcagatgctggcggcgcgcgtcgcagccggcgtgcccgagggggtgctcgtctggtgcacgacggccgtgctcgtgcgcaccgcacagcccgctcgggtggcaggcattttcgtcgtcgtgatggcgctgggccaagccgccttcggcatgctgctggcacacctgatcatccccggccaaggttggcgcggcgtcttcacggcgctagcgctggcttcgctcctgccgctcgcgctggctttcatgcaacggccgcgtctggcgccgttggtgccacccgccgtctcgggctttcgttggtcacctcacacactgcggccgctggctgtcgtgttcctgcagctggcggcattgggagcgttcgcggcctacctggaaccgctgggcaaggcagccgggctcgactcgcgctcggcacagaccctcgtcgccggcatgctcgggatgcaggtggtcggaggcatcgccggcactgccgccgtgcgccgttggccaaccgtggcatcccttgtaggcgcgtcactcgggttggccgcggttacggccatgacgtttcgactgccaaccggcggtgcgcagcacctcatgctcgcgaccgcggcgttcggcttcgtctggctgttcatgcagccgttccagttcgccctgacgtttctcactgatggcagcgggcgcctgggcacgctgatccctgcggcgcaattgctgggcagtgcattcgggccgctgatggcctcattcgttgtcgttggcgacgatgcctccgcagtgcctctggtgagcgctggattcgccgtcgcggcggcgttgctcgtgctcggcgcagcgcggcgccgggccatggggaccgcatgacgatactgcccgccgacaccgacaccatttcgcgcatcttcgaacaacaattgcagacatcgttcgcgctgcgcgacgcgacagctgcggagcgcgtgcgcaagctcgcgcggctgagcgacgcactgctgcagcggcgcgaagcactccatgtagccttccaggccgatctgtgcacacagccgtcgaggtcgacctgaccgacctgctgtcagtgatcgaagaggctcgtcaagctatgcgccggctcccgaggtggatgcgggcccagagcgttggaagcaccctgacgacagtcagcacctcggctcgcatcgccttacagccgcggggccgttgcctcatcatcggaccgtggaactacccggtgaacaccttgctcggtccgctggtctctcagccgtcgctgccggcaacacggtggtcttgaaaccctcggagttgactccgacggtcactgccgtcatcgatgaactcgtgcgcaaggtcttcgatccgtccgaggttgcgctggtgcacggcggtgtcgcgactgcacagcgactgctcgcgctgccgtgtgaccacatgttcttcaccggctcgcccgctgtcggcaagctcgtgatggccgccgccgcgcaacacctcagctcgataacgctggaactgggtgggaagtcgccggtcatcgtggctgctggcacggacttgttgcatgctgccgagttggcggtgtggggcaagatgacgaacgccggccagacctgcgtcgcgccggaccatgttttcgtgcatcgttcattgaaggatcgcttcgcgcagctgtgctcggacgcgattgcgcggcgctacggtgcagatgacgcagcgattgaggccagtgccgatctcgctcgagcgtctgatgacactcaatgtcgccacgtctatcactcctaggatcccctgccttaaaaatgagcaggtagggttttgcgtgggtcagtcttagacggaattagtgcgttggtggactgaaccccatcgactggaccactggggtcatcagaactaagcgcctgctcagcgaattgggattcgaattcgttgggtggacgatagccgagcaccgccttcgccttgggataaagaaagcggccgagcggcgtcagcttcatggggcgcgtagctttgtcaaagagtttcccgccaagcagatcctcgagctacgcgatttgcatgctgactgcggcggacaccacgtgcagcctggtagccgcgaggttcgcgctttctgtctcgacgacctcgcagaaatagcgtagcgatttcaagttcatattttttgatcttatggtcaaaattctttggttgtgcatctactttacttaactgagtatcagggcctgttccaacttcttctggagacaaccttgatttctgaagtgaacgagccgttgtggctctctcaagcccgctcgctctcgagcgcggaggtgtctgacgccctcgacttcttcaatcttcctggcagcgcactgggcattcgcccggttgcaggcccggccaagctcttcggccaggctttcacgatccgctttgcgccgatcgatcgatttcagcctggaacagtcggggatttcatcgatcgtttgttgcccggcagtgtcgtggtgctagacaacggcggacggctcgattgcacggtctggggcggcatcctgagccagttggccgcccagaagcggatcggcggaactgtgatcaacggcgtgtgccgtgacaccgccgaggcggacgaggccggctatcccctgtacgcgtgcggcaaattcatgcgcactggcaaggaccgggttcaggtcgaggcttacgagcagcccgtgaccttgggcgacgttcgcgtctgcaatggagacctcgtgatcggcgatgcggacgggatcgtggtggtgccacacctgcgcatgcaggaagtgctcacgaaggcgctggagacgcgcgtcatcgaggcccagattctcgaggccgcactggccggcatgccgttgtcggaatcgcgaaagaagtatggctaccacacgctgcagcgttcacccacggcgctgcaaggtcaaggcagctgacagcaaagcgccacagagctacctcgtcggagacaaatcatgaaaccagttcccaatctgttccgtgctgcagcgttcggcctcttggcggtcgcagtcggaggcggagcgtccgccgagtcggcgtatccgtgtcaggtcgtaaggctcgtctcgccgtatccgcccggcggcacaaccgacatcctcgcgcgcctggtggcgccgggcctcgcgaaagagcttggcaccaacgtgatcgtggacaacaagggcggtgccagcagcaacatcggcaccgagttcgtgtcggccgccgcgccggacggctgtaccttgctgctggggaacaacacgggggtggtcatcaatcgcaacctctacaagcttcgactcgaccccatcaagtcgctcgcaccggtcgtggaggtcgcctctgtgccgttggtgctgtacgtcaactcggccgaatcggcgaggacgcttgacgaattggtcgcggccatcaaggccaagcccggcaagtacagcttcgcttccgggggcagcggcagcccgcaacacctgatgggcgagatgctgaagctcgagatgaagctcgatatgacgcacatcccctatcgcgggcaaggacctgcgctggccgatgtgatcgccgggcaggtgccggtcgccttcgaaacgaccacggccatcgcttcgcagctcgggtcggggcgcatccgcgcgcttgcaaccactggcagcacacgttcaaagaatttgcctgatgtacccaccatgaaggaactcggccacgcgaacttcgtggtcgagaactggtatggcgtcttcgttcctgcgaagacgcccccggcacttgtcgagcgtcttaaccgcgatctgatcaaggtactcaagagtgcaaacgcgtcgaagagcctggctgacatgggttcgcgggacgtcactgggagcgccgagcagttcgcccagttcgtgaacaaggagcttccttactgggaatccatcgtgaagcgctcgggcgccaaggtggactgaaccgtcgctatcgcgcctcgtcaatttttcatgtcggagatacccgtggccacttctgatcagatcacgcaacttcgcgcccttggcgcagccaccatttatgaagcgcagggcgccaagggcgcattggacagcggcatgaagccgatcgatcccaccgtgcgccttgcaggacccgccctgaccgtcgactgccgtccagcggacaacctgatgctgcactacgcggtgcagaaggcgaagcccggcgacgtgctcgtggtcgatgccaagggcttcatggaggcgggcccctggggcgacgtgctgaccatccaggcacagaaggtgggcattgccggactggtgatcgatggctgcgtgcgcgacgccaacctgatcatcgagcttggctttcccgtgttctgccgcgggctgtcgatcaagggcacgggcaagaaccagcccggcaaggtcaacgtacccatcaccatgggcggcgtgacgatccaacccggcgacatcgtcgtgggggaccgcgacggcctggtggtcgtacccgaggccgacgtcgaagccaccatcgcgagcagcctggcgcgagaagaaaaagaagcggggcagcgcgaggccatcgagcgcggcgcgttcacggccgacctgctcggcctggcggacacgctgcggcgcctgggcctgacctgagcgctggcgccgtgcccgcgacgaccccggggcgcggttcagacacccatggagacaacaagatgaccagaactcttcctcgcaggcacgtcgttgccggcattgcgctggccgcattggccaccacggctttcgggcaggcctatccgagcaagccgatccggctcatcgtgccctggccggccggcggtgccgctgattcagtagggcgcgcggtggccgaagggcttcgcatgcaactgggccagagcgtgatcgtcgacaacatcggcggggccggagggaacatcggcacccagcagttcatccgccagccggcggacggctacacgctgctgttggccaccagctcgaccaactcggccaatccttacctctacaagaagaccggcttcgatccgatgaaggacttcgtgccggtggcagcgctcggcctcattcccagcgtgatggtggtcgccgcagggtcgccccacaagtccccggcggacatcgtcaaggccgcgaaggccgcgcccggcaagctctcgtacggttccggcggcgtgggcaattcggcgcacctggcgggcgaactgttcaagtcgatcgcaaagatcgacgtgatccatgtgccctacaagggcagctctcccgcactgaccgacgtgatggccggccaactcgacttcatgctcgacacgggcgcctacgggcaaataaagggcggaaagatccatgcgattgcggtggcttcggacaaacgccatcccatgctgcctttggtccctacgttcgacgaactcggcatcaagggaatgaccatgaacgcctggtatgggcttgcctctccggccggcaccccggcggccgtggtcgacaaggtgaatggcgcggtccaggcggccttcaagtcgggcgagctcggcaagcgcctgacggacatcggcgtcgagttacggccgggcgatgcaggcagcttcgcgactttctggaagtcggaactcgaccgctacgcgggcctggtgaagctgacgggggccactctggactgagaagtgacgcgcgcaaaacctccgcctgtcgcattgttcgccgacccgccagcgccccgcagacgccggttcggcgctccagtctgctcgtcagcctcaaggcgcctcgctttgaatctctactcgagaaccgccccactcctctgttgacgtatgcactactcaaaaaacaacgccccaccatccgattcgccagacctactgccggttgaccagcctcagacccaggtgcccggaagcaaggtctcgccaacttcgcatgcctgcgaatgggacgaatggcggcccatccgggatgtgggtgacctgccgcgagacgctacgccagcagctttcaacaggctcgcccgaatgactgcatccaacaaaaactgacctgaggcggtgagatcctcgccgagtgagcaggcaacttcgaagaaaaccaaatgagttcgcaattgattcgttccgtcctcatcgcgagccggtccgagatcgccattcgcgtcatgcgcgcggcatccgagatgaacatgcgcacggtcactcgcgaagcagattgcaccggcgctcgcggagtagttcgtcgaacaattcgcccgcgacacgttctctttggtgaccgcgtacgagggttttccgctacccctagcggccgatgaagtcactccgttggccgatatagacccattcaagtcagagcgcagatcttagatttcaccgctaccttatctccgagtaactgtgatgacctcattcacgcgtctccttcgcactgcagtcttgctggtgctatttgttcggcccgccttggcagctggccctgacgacgccaagggcctgtggttggccgcggaaaaggatgcggtcctggagttcaagccctgtgctgataccccgacggcactatgcggacacatcgtgtgggacaaggatgcaggccagcccaatgacacctgcggtgtgcagattgcgcggctcgaacgctacgaaagcgaagcttggcgcgatgggtgggtctatgaccctcgcgatggaaagaaatacaagggcgcgctgcgagtgaagtcgggagagctgcacattcgtgcgtttctcggcgccgagatcctgggtcagaccgagcggctgcaacgcatcgccgctcccccagaaacccccgtgtgcaagccctgatcccgtcacgttcaacccaaccagcgaaaggaactcgcatgaacaatggccccctggtctttctggtgtccatcagcgcgctgctcagcagcatcgccgctcccgcccgagccgacgaaatagcgagctattccatcgagaccgaggtcaaagtggtcagcgaccaacgcacccgcggcatttccgattcgctgaaccggccgggaatgcaattgggcgtgcagttcgcacacgaaagcggcgtgattgcgctggtgcagttgtccaccatcagcaacaagtcatacaccggcagcgcgggttacgacgtgctgctggccaccggctggcgtttcggcgatccagatggctggcatttcggcgtggggcttgctactgagttctttccgggcgcgaagttcgatgcgccctatgccttcgatttgaatacaggcgagcctgccgacgtccgaaggaccaggtacgacacgtcctatgctgtgctcgaacttggatggggtgcgctcgatgcgcgcattctgaacgtcctgtccaagaactttcgaggcgccagcactggcggcgtctgcgggcagatgctggcgttgtcggtcgatcccgccagggcccttgattgctatgcgcgcggcgaccacaactcgcgaggcagctggcttgtcgacctggactacaagatccccttgagcgacaagaccacgctgaagctgcacgcaggcacacagcgcatcaagaatttcagagaggccaactacagcgactattcgatcggcgtactgcacaagcaatggggcttcgaatggagcgccgaatacgtgatgccgaaaacaaaaacgcgcgagttgttccaagtggttgacggcaacaggatccgctcggtagatggccgtcgcctggtcttggccgtctcgcgaaagttctgaggcattgatgagtcttgcccaacgtctggtccttgccatcgacctcggcacgtccggctgcaaatgtgccttggtcgcgctggacggcgctatgaggtagctgtcactcttttctcaacggattcaggcggttagctttgcagcatgactgtccgcagaatcccttcttccctcaagtggctccttgacaagagatcccgccttgaaggcgagctattgaaagtagagaaagagggctgcgccatgcagcagctctgtaatagtccgcttgaggccgttgttgacggctaggggtttaaggcgtgatgtcggtgacgtgttgaagtagagcgaacgccacacgccatgcgcggccatcacaatgaaccgtggctgtgcgctggttgatccgaacgatttctccgacgtggcgcttgaggctttggtcggagaagctcacacgctggccgacgcggaagtcctgtttgtgatggatctccggcggtggcctcaatggtgcggcatgcgccggtgagggcgacttgtctgcctgctgctcatcgacaggcacgacggccgcgtacagcacgctgaagcgctgtttgctttgctcgtcgatcagcgtgacctgccggtccttcatcgccgcgatgcgagcctcgcgcagcttgccggtcccccagtcccagtacttcaccagttggcccatgtgcagctgcgagcgcgcctgcacgatgcgcctggggtcggccatgagttgctcgatgacccagctgagctggtacagctcagcgctggtggccatggggagatcttcgatctgcttgacacgcatgctggcgattttgccagcggcgatgcgctcaggccgcgagcttgtcggtcggctgtgagctcgtcggcgccgccttggcaagctcactggcgaccgcccacggcagcaactcgtcgatgcggttgctcggatggtcggcgatgcgctcgagcacgtggcgcaaataggcctgcggatcgaggccaacgagcttggccgagccgatcaaggtgtaaatcaccgccgcgctgtgcccgccgttgtcggagccgagatgcaggtagttcttgcggttatgcggagcttcacataagcgcaataaggcgaagtgcgcttttatgcgaagtgttcctcggtcgcctgtctccttgccctcgactgcgggcgcgacgcgcagccggggtacttcgcatagtcacagtgatcgtaggaactccagcaacgccttcggcggccggtatcgcgcctgcttgacaccgggttgcttcaagcgcgcgagtgcacgctccttcatggcgaggtccgcctcaacatacatatgcgtcgttgacggattctcgtgaccgagccacagcgcgatctcacaagggtcggagccggactgtagaaggctcatcgcggtcgagtggcgcacgacgtgcggcgatacccgtatggacttcagcccagggtgcgtggtcgccgctgcatcgacggccagtgccagccgctgcgccacgttggcgcgtgtcatcgttcgaccgtcgcgcgttggtagccggacgatcacatcgtcgtcatcgacagtgatcagggcgagtcgggcgcgtcagcggcctggcgtgaaggcttccagcgtctggtcagcgatgtgggcctgggcagagccggcatcgtcatggggctggaggtctcccgcttggccaggaacaatgccgactggcatcggctgctggagatctgcgcgctcgccgacacgctgatcctcgacgaggacggcgtgtacgatcccgcaaacttcaatgatcggctgttgctgggcctcaagggaacgatgagcgaggccgagcttcacgtgctcaaggccagattgcgcgggggtatcctcaacaaggttcggcgaggcgagtatcgctgcgtactgcccaccggattcgtctacgacggggccggcaatgtggtcctcgaccccgactctcaaatacgggagacgatcgcctacttcttcgacaccttctcgcgcgtgggctcagcatgccagacggtgaaggtattccgagacgagggcctgcgcttcccatctcgactgcgcaatcgcgacgtcgtggtcttccgacctctgaccgcgtccacggcaatccgcacgctgcacaacccgcgctacgctggcgcgtacgcatatggtcgacgacgctatcgccgcgctgccgacggcatgaaggtgcagcaagcccgcgactgcaacgactggcttgcgtgtatcccggatgctcaccccggctacatcacttgggaacgattccaagagaacctcaaactccttgaggcaaacggtcgtgcgtacgagatggcgcgcgcctcgccgccgagagaaggtgcagcgctcctgcaggggcgcgtggtctgcggccggtgcggtcaacacatgcgcgtgcggtatgccgcaaggcgcggagggttggaggcatggtacgtctgcgaccgcgcccatggcaagagcgccgcgcccaattgccagtcaattgcgggagggcccatcgacgccgcgatcgcagcggtggtcgtcgaggagatgacaccggcggcggtcgagttggcgctcgagatccggtcagagattgaatctcgacaggaggaggccgaccaattgcggcgtcgcgcgatcgagagggcccaggtcgacgcggatcttgcacagcgtcgcttcatgctggtcgatcctggcaaccgtctcgtcgctgacacgctcgaatccgagtggaacgacaagctgagaacgttggcccgggcgcgagaggaccgcgagcgaggaaggcaggaagacgagcgcctccttggcgagacggttcgcgaaagactcctcacgatgacgacggacttccagcgactgccttgcgcgttgcctatctcgcccgcagctacggcctgcgctcgcgctacgatcgacttcgagaccggggcatgctaaccaaggcagaggcggcgacacgcttgaacatccacgagtgcacgctcgtgcgctgggcgacgaacgggctcatcgcaaggcacgcctataacgcccacgcctacttgtacgaggacccaggagcgaccccgccgagcaagcattgcagtcgatgggatcggctcgttgatcggacggtggccatcaagaaaacgggggcgtcaatgccctcgccttcatcgggaagaggtgcagtatgaagatagttggttggccagcaggcacatcccatcgccgtcactccacagcagcttgaccagatcgccgcgccgcccgcggaagacgaagacgtggccggagtacgggtcctcggtgagcgccgtctgcaccttcgtcgccagcgtgtccatgccgcagcgcatgtccgtcacgccagcggccaaccagacgcgggtgcccgcgcgcgggccgatcatgcactctggcgcagcgcacgcaggacgctgcacagactgtcttcgtcgatagcgccacgcagtcgcagttgcgcgccggcgaactccagctcgatgacgccggtccgcagtgtcggtctcgatgacgatggggcaggcgcagcggaagtcggaatggacatgacctcgctcgccggtgctacctctatcggcaacagcaccgccggcggcgcgtcgcctgcggctcgaacatgctccctgcgccacttgaacagcatgttggcgttgatgccactgcgcagcgtgatcgccgatacggacgcgcctggctccaggctttgtcgcaccagctcttgcttgaacgaccggtcgtgatttcgccggctcgccttcgctgagtcttgcgcaatcttcatggtgtgcaccatctcctttagcgcacacctccatgcgggtctgcgattcgggtcagatgcttcccgcagcctgcgcatcaggcaagggcggccttcgtcggactattacgttgcgccagcgtcttcacgccaacgaatttggtgcccggctgctggatcgccagccagatggcgcgtgcgtctgtagcgtcggtcttgttgccgttcacgaatgggcgcacggctttggcatgaatcagccgcacggcatggccctgcgccgtcaactcacgggcccagtggtgcgctccgccgcaggcttcgatgccgatcaggcaaggtgcatggttggcgaagtgccctaaaaccttggagcgcttgagctgcacgttgacgatctcgccagtgcccatgtccacggtgtgaagctggaacacattcttggcaatgtccatcccaatgacctgcaggccacccatccagccgatggtttgccccgcgctttgtgtagtactacgatgcatgacggatcctcgctggtgtttgtgaagaccttggtctatcacgccacgggcactttgatgccgtatccagtcgagggtccagcttgtccagaagacaagccacattcccacaacggtcacgctgttcatctctgtactcccgcggcatttgtgctgcccgcaggcagggaggcatccattacatctcctggtagtccaagttttcgtccgcacccctagggtcagagatcggcggaatcaaacaccaagattggactagtgggatggacgcccccttgtacaaaaaggggggcgtccatcccattagtccacgcgtggctcgaaatgaatctatcttgtgctcaaccagacaggggaagatggacgtgagcacaaagtccgccacccgtcctgttgaccaattccaagagcccgccatgagcctgacagatcgcggcggcaatcgatagccccagtccgctaccgcccaagtggcggtcacgcgagtgctcggctctccagaagcgctcggtcattctcggcagtgcatctgggtcgacccctgggccgcgatcgcacacggaaatgagcagctcggaattcgatggaatcacatcgatagataggtgctttccagagcccgcgtatctgattgcgttgtcgatgaggatgagcaggacttgaccgatgcggtcgcggtcgccggtcacccttgcattccttgaaatggacacccgagggaccaacccgacttcgttcaagcgcggcgctgcccacgccaatcgctcctgaacaagatcgtcaagcaggaactcttctcgctccagcgagagctgacccgcgcgagcaagcgagagaagatggaggtcgccgaccaggaagttgagctgctcgagttggcgatacaccatgctcaactgagtctcatcgcatgaaaatacctgatcgagcatgccttgaacccggcccatcgcagcgttcagcggggtacgcaattcatgcgcaaccatggcgctcgattccctgacctctctctcgtactgctgcagcttggcggtcatgccattgaagtccaccgcgagaccgatcagctcgtccggggcgccggcaaccacgctggctcgcgccgagaagtcaccctcgctcacgagtcgagcagcatctgcgacgttggtgaactgcctggacagcggacgcgaggcatacagtccgcataacacgatgacagggatcgcacagctcaccatccccgcgagcaaccaccagtcacggctcgcaacgccaggaagaaagtcaaccacgtcataatgctgctcgaacagctgccacaaccgcgatgcgttgctgtgcggatcggcccgcagttgctgcatttcctgtctcgcatccggcggcaaccgactgagcaccctggcatctgaaatggcgaagcgcagccacattgcaagagcaatcgcaatgaccgtaatcacggccagcatgctcatgcgaaatcccacccatcgccagagcggggtgtgtcgggaatccgcggaaaaaagcctcctcattggaagcggtagcccactgcacgtaccgtcaccagcacgcccgtgattccatgcaattccagcttgcgacgcaggttgtggatatgggcatcgacaacgcgttccaaggcgtcgctctcgggcaggcatgcttccaacaattcgcttcgagtaaacgccttgaacggcgtcctaagcaatgaggccagcaggttgaactcggtgggggtgaggtctagcggaattcgctggccctcggcatcgtcgactgatgcgacaaaggcaccggtgtctaccgtgaggcgaccatgcttcagtggcccccctgaagacttggttgagttgacgcggcgcagtacggcatacacgcgcgcgaccacctctttcggactgtatggcttgacgatgtagtcgtctgccccgtagcgcaaggcgccgagcttttccggctcgtcgccgatggcggtcaccatgatcaccggggtgtcgccggcgcgccggatcgcagacagcacctcggtgccaccgagcttgggcagcatgacatccagcagcaccagatccggcttccactgcgcatgcaaggtcactgcctgagcgccgtcgctggccacggcgaccacaaatccatctctcttcagataggcctcgaggatgctggcactgtcggcatcgtcctcgaccaccagcactcttttttcattcatggtctgcgcgtcttaatgaaatcttgaaatttcccgaaagcaaccttgaacttggagcaagacactctcagtcgaaattgaccttcccgactgacaccatgattctattgcccgcaggtctcagatccagttgccttccgttggcactggccgtcgccaccctgctgatgggcggctgttcattgactcccgactaccagcgccccgcagcagagctccctccgaccctgggggctcaccataccgagcaggagagcgctcgaacggcggcaccggctgagctttccgagcaggaacgagcgttccttcgagcgttctcgcccgcaagggatctcgcaccgatggtggctcgcgccctggcgcataacgccgacttccgtctggcagcgctgaaggtcgagcaggcacgtgcgcagtatcgcgtcgaggaatcggcacgcctgcctcaggttggcctcaatgctcaacgcacacggcagcgcttcgacagcgccacgctgcaggcccgctacggccaagacctggtgtacggcagcgtgggcatcagcgacttcgaaatcgacttcttcggcaagatgaaagcattgtcggagtcggcgcggcaacgatacctggcctccacgcatgggcagcaggcagcgcgaggtgcgttgattgcagaggtgcttcgcgcttacagcctgaagcttgctgccgctcaggcacgtgtgcagatggaggccatcgatgccgacagcgcagctttgctggccatcgctgtgcgccagcacgaagtggggctgagctcggtcgacgaactcaacaatcaacggcgccaggctgatcaggcacatgtgcgtacgctacaggccgccgacgatgacagtgcggcgatgcgcgccttgcaattgctcactggctacgatctcgccacagccgagggcgatctcgatggcttgcgcgcgtccgacatatccgtggcggcgctgcgcagtctggactctcaggtgctgttgcagcggcccgacattcggcaagccgaggccgaactgcgcgctggcgacgcagacatcggcgccgcgcgggcagcttttttcccctccatacgcctcagcacctcattgggaacggcgagcgacaggctgaacggtctcttcgaggccggcagtcggatgtggagcttcacgccacagctggtgctgcccatcctcgaccatggccgcaacagcgccaatttgaccctggccgaggtgcgcaagcaggccagcgtcgccgactacgagaaggcaatccagtctgcgtttcgcgaagtcgccgacgcgctcgatgcgcgcgccaccctgtccgttagcgagtcgagatcgcgcgagcaagccgaccgcgaacgcttgcgaatcaagcgcatggccgcacgcaccgcacagggcctgcaggatcgaaacacgctcctgattgagcaggtccgggcgacccagtccgaactcgaccacgtgggcatcgctcgcgacctggtgctgaaccgcatcgcactgttccgtgcgttctatggcgtgcaactgccgtcctccctttgaactgacctccttggaaattcacatgaaaaaacacatgcttcgccgcgctcccaacttgctgggaccgctggtcattgcgctggtccccttggctgcgcgtgccgaggaaacccagacctggagtgaccgcttgctgggcgacaagacccaagtcagcgttggcgccgcgacgatcgtggcgccgcgctaccttggctccgacagctaccgcgtgcagttgctcccggtgtttgccatcgagcgcggcatcttctttgccgataccagccgtggcgccggtgttcagttccagaccgacagcggcttctatgcatcgcaatcggtctactacgacttcggccgtctccagcgcaacagcgtgttgcgcccgggctccacaaggctggcaggcatgggcgatgtgccgggctcggtgaccacccggacattgctcatgcagcagatcacgcccagtttctcggtcaacgccgaagccgagttttccctgaaggacggagctcgccgcaaccactatcgccttggcgccgagtacaaccttctgaagaactccaccgacaccgttgcgctcgatgtagacgtgcatgccggcgaccgacgctacaaccaggcctacttcggtgtcaccgacgcgcagagtgcgcgcacgcctttcagcgcgttcaaggccggttcgggaatgtacgcgtactccatcggtgccagctggagtcacacgttgagtccccactggacgaccacgctgcacgtcgcggtcatgcagtacgtcgacaacgccaaggccagcccgctcgttgcaaaacggacctccgtcaccggcgatgctgcagtgacctacaccttctgacgagcgctcgatgagggaggggcataccgtgaaatttttttctcattcttccgttcggctgtgcggattgatcgccatcctggtgttggccggttgcggcggaaatgtcgcgtctgtcgctgcgccacctcgtgccgtcaaactggaaacggtcgggatgagcgcgctggccgaaacacggtttgcggccgtcgttcgtcaggagcaacgtgccgacctcgccttcgaggggggcggacgcatcgccgcgatcggcgtcgacgtcggtgatcgggtgcgcaaggggcaggtcctcgcacgcctggatccggagccggctcgcctgaggatgcagcaagccgacgccaatgccagttccaccatggcggagttcgaggagcgcaagacccaactgcgccagcagcaggccatgttcgacgacggggcaatctcttcggcgacgttgaccaccagccgggttgccttcgaggcagcgcagtccaggtcccgtgttgcggattcggaccgggatctggccaggcgtgcccttcgccaggtcgatatccgcgctcccttcgacggcagcgtggtcgcacgtttgctccagccacagacggacgccggggcaggacaggccgtgctccagctcgaaggacaaggtcatgcgcaggtggttgccctgctgccggccaatgttgcatccaccctggctgctggtgcgtcagcgacgggctaccgcagcaacgcgccagacaagccgctcgcattgcagcttcgcagcgtatcgacgcggttggagggcgccgcgactgtgcaggcgatcttcgatttgccagcgcaggaggaggctctgcgcagcggcgagagcttgctgcttgcattgcccgccgctccgaccgagttgactgtcccgctgacggcggttgtcccgacgtcggaaaaggacgccgcggtggtctttgtctacgaaccacaaattggtcatgtgcagcgccgcgccgtcgtctcgggctccatcgagggtgcccgcatgcatgtacgccaggggctggcgcctggagaaaaggtcgtcagcgctggcgcctcgttcctcaccaacggtcaggcggtcacggtcttccgcccggaaacccgtcttagcggaggtaccgcacaatgaatttcacacgcgcggctctttcctccagccggctgacactgttcgctgcgctgttcatcctcgtcgccggcatcgttgcctttctcggcttcccctcgcaggaagagccatcggtcacggtgcgcgatgcgcttgtctcggtggcatttcccggcatgcccagcgagcaagtcgagaacctgctggctcgccccacagaggagcgcctgcgcgagatcgccggtctcaaaaagatcgtgacgacggtgcgaccgggcagcgcgatcattcagctgaccgcctacgacgacgtcaaggagctcggcgcattgtggcagcgcgtacgtgcaaagagcgccgaggtcggcgccacgttgccggccgggacgctgggccccttcgtcgatgacgatttcggccgcgtctccgtcgcctcgatcgccatcgtcgcgccgagtttcagcatgagcgaaatgcgcggcccactgcggaggatgcgcgagcagctctacaccttgcctggtgtggagcaggtgaccacgtacggattgcaggaggagcgcgtctatgcgacgttcgatcgcgcccgcctgctcgaggccggcctgaccccggccagcgtggtcgaacagttgcgcgcccagaacattgtcacgcccggcggtcaagtctctgcatccgggttgacgatgaccgtcaccacctctggcgaggtgcgcacggtcgacgagctgcgtcagttcctcgtgacggtgcccggggcctcgggcacacgagagacgccactttcccagctcgcacagatccaggtgatgccggccgacccgcccgagagcgctgcgatctaccaaggacagaccgcggtcgtggtctcggtatcgatggcccccggaagaaacatcgctgagttcggccaggcattgcgccacaaacttgacgagactgctgccctgttgccggcgggcttcgagcaacacatcgtgaccttccaagccgatgtggtcgagcgggaaatgggcaagatgcaccacgtcatgggggagacggtggtcatcgtcatggcggtggtcatgctgttcctcggctggcgcaccggcctgatcgtgggcgcgatcgtgcccctgaccatcctgggcgcactgatcgtgatgcgcgccctcggtgtggaactgcaaaccgtctccattgcagcgatcatcctcgcgctcggcctgctggtcgacaacgggatcgtcatcgccgaggacatcgagcgccggctcggcattggcgaagaccgccgtgccgcctgcatcgacgccgggcgcacgctggcattgccgctgttgacgtcctcgctggtgatcgttctggcgttctcccccttcttccttggtcagaccagtaccaacgagtacctgcgttcgctggccatcgtgctggcgatcacgttgctgggatcctggctgctcagcatcacggtcacaccattgctttgcctgcatttcgcgcgtgcccatgcatccccgaccgagggagaagggcactacgaatcagcgttttacaggggctatcgcaagatcatcgaaagtcttctgcggcacaagctgatattcgtaggaacgatggtgctgttgctggcgggagcgatcacggtcatcgcgtccattccctacgacttcctgccgaaatcagatcgactgcaattccagatgccagtcactctgcagccgggcagcgactcccggcagacgctgcagacggtccaatcgatcagccgatggctcgctgacgaaaaggcgaatccggaggtggttgacagcattggctacgtcgccgacggcggaccgcgcatcgtgcttggcctcaatccgccgctgccagcggcaaacatcgcctatttcacggtcagcgtccgcgcgggcaccgacatcgatgacgtcatcgcgcgcgcgcgccagtacacccgtgcccactatcctgaagtgcgagccgagcctaagcgcttctcgatgggatcgaccgaggcgggggtagcgatctatcgcgttgtcggtcctgacgaggccgtgttgcgtgccgccgccgaaaagatcgcacaagccctgcgcgccctgccagggacggaggatgtctacgacgactgggatgcgcggattccgcgctacgtggtgcacatcgaccagttgaaggcgcgccgtgccggcgtcaccagccaggacatcgcacaggcgctgcagatgcgctacagcggcgcagatgcatcagtgattcgcgacgacggggtcaatgtcccggtcgttctgcgcggcgatgcaggcgagcgcgccgccaacagcaatccgggagacaccgttgtgtaccctcagggccgcggaacatcagtgtcactgacggccatcgcgacgattcaaagcaacaccgagccatccacgatcatgcggcgcaatctgagtcgtgcgatcaccgtgacgggtcacaatcccgctctcaccgccacccagatcgtcgatcgactttccggtcaggtggcagcgctgaaattgccgccaggctaccggatcgaactggggggcgagatcgaggactctgagcaagcgaaccaggcgttgttgcagtacttcccgcatgcgctgggtgcgatcctgctgttgttcatctggcagttcaactcgtttcgcaagctcttcatcgtgatggcgagtgtgccgttcgtcctgatcggtgcggcgttggcgttgctgatcaccgggtacccgttcgggttcatggccacgttcggtctcctcgcgttggccggaatcatcgtcaacaacgcagtgctgctgcttgagcgcattgaagaagagttgcgcgaaggattggagcgccgagaggcggttgtcgctgcagctgtgaagcgactgcgcccgatcgtgatgaccaaactcacttgcattgttggattggtcccgctgatgctgtttgccgggccgctgtggaccggcatggccattaccatgatcggtggcttggcgctcggtacccttgtgactctgggcctcattccggtgctctacgacttgctgttctcgtctcgcatgcaagcacgcgagatgttggctcgcccatgaggcgcatccggcggcgtggcccaagagcgacggacaacgatcgaggcccacggtgcgtttcttcaggcgactgctgaacgagcgtggcgctttcacggcatgcctcgggctggttgcgctatggctgtggttgtggttttgtcggtgatgctccaggcgatagcagaagcgccagtcaggaaaggcagtgcgatggaaggtccaaataaaaatttaggcatttcttccatatgaaatcggcatgcgacagaccgtgccgcggcatgatcagagatcgtcgcaaatttgacagttttcgaggcggccgagacatagcatccggcaccacatgaatacccaactcgcgaacgtccacccggtctcacgcccacgacgcgccctgctggttggcagcgcgctactggcgggctccgctgtcgcaggtatcggatacgtcgccactcataccaatcagccggttgccatggacagcttttccgaccttgtccgcgcgatgcacacgctcgagcgcctgcgcgaagcgccgctgcatacccgctcgggctgggacctggcccacgtgctgcaccacgcggcgcaaagcatcgaatactccctggacggctttccgcagttgaaacctgcgtggttccgcgcctcgttgggcagcatggcgtttgcagtgttctcggcgcgcggcaagatgagccatggtttggaggagccgatacccggcgcgccggcgattgcgtcgggccagccgctgaactctgccgtggagcatctgatcgatgcattgaatcgattcgaacgacacaatgcggcgctcgcgccgcacttcgcctatggcgcgctgagcaaatccgagtacgcgcgcgcccatctcatgcacctggcgaatcactgggatctggtggacgccggctgacgcgcgctgccgagcagcgccacgacttcctgcacgagcggcgtgctccttgtccggctccaggccacggccgtggttacgacatgcaggttttccttcagcggacgaagcatcacgttttccggggcaagctttttcatcgatgcgggcacaagcgcgatcccctggccacagccgacgaatgcgacctgcgaggcgacgctgcaagtctgatggagcactctgggcgaaaagccgtgagccaggcaagcggccgtcagtccatcgaagtagaccggactgacctgcctggagaacatcacgaaatcctcgtccaccagtgtcgcgagcccgatgcgtgccatctgcgcaaagcgatgccctttgggcagggcgacggccagtttgtcctgcttcaggggaatgctgccaatggactcgcccatgtcgccttcgagccgggcaaacgccagatcgacatcgcccgactccagggatggaatggcctccgcactgtcgatctccttgaccgacaccgtgagatggggatagcgctccctcagcttctccagcaagggcggaagcacatcgagcattgcggaactgatggccccgatcgtcagcacgccagtctgtcccgccgcggcttccctgatcgcgagctccagccgctcgacttgctgcgcgaactttcgcaccgccggcaggatcgctgcgccaactggcgtgagttgggcgccccggcgcgaacgctcgaacaacttaagcttcagcgattgctcaagtacctggatctgctcggtcaagggcggttgcgacatcccgaggcgcttcgccgccctgctgaagttctgctcttcggccaccgcgaggaacagccagagatgacggatgagacggaagttgatcgtattcatttcataggcttggcgtatggatgccatccagattccggaatttacatatcaaaggcttcgacggaaagtatgtcttcttcaatctgcccattgcagcgaatgaccgcttccctacttgaccgcctcgcagccctggacaccaacacggtttccgatgcactcgacttcctcgaccttccaggcgccacgttcggcctgcggccgctctgggattgccccaagatcgtcggtcgcgccagcaccatccagctcggccccaagaccgatgcgaagcctacagcccacctgatctcgcccgtgatttccgagatcacaacgggcgaccgcatcctcgtgatcgcgggcggcctggacggcatctcctgctggggtgacatccttgcgaacgcagcacaggtccggggcattcgaggctcggtcatcgacggactcagccgagacatcgatggcagtgaatcgatcagttaccccgtctatggacgcggcgtcacgatgatcagcgcacgcaatcgagtgatccagatcgcctcgggtacgcgcatcaaagtggcaggcgtcgatgtcgacgaagacgactacctgatcgcggatcgttgcggaacagtcttcgttcccaccgcgcgaattgaagaggttctggcgctcggcgagaagatcgcgcgccgacaggacggcatggtcagcgccgtgcgccgcggcaagtcggtcgccgacgtcatgcacgacaaggaattcgaagccatcaatcaaggtactgtgaaatgaacgccgaagacaaggaactggtcgcggtctttcacgggctcgaagtaacgggcgtctccgatgcaagaaagattgcgcgcacagtgatcgatggtgcatgccgcgacttcctccagcagcgggacccgtcatgaccttgagcgacgaacagtactttcagcggctgaacgttcatctggccagcgtccagccctccgcaacctacaagatgatggatcgcgtcgctgccaggcgggcatccggcgcgaaggtgatctccctgtccgccggagagcccgacttcgacacgccggcgcatattcgcgctgcagccatcgacgccatcaacgcaggacacacccgctacacccaggtcgccggtatgcgcgcgctgcgcgaagccattgccagcaagttccagatcgagaacggcctggactgcacgtggcagaacaccatcgtgtgctccggcggcaaacaggtgatctacaacgcattggccgcgacgctgaacgtcggcgatgaagtgatcgttccagctccctattgggtcagctatcccgagatggtccaactctgcggcggtcgggccgtcgtcgtgacgtgcgacaacacctcggggttcaagctgacgccgggcaggctggctcaagccatcagtgccaggacccgatggctgatactcaactcaccgtccaatcccacgggagcggtctactcgcgcgaagagcttcgcgcgctgaccgacgtgctgttgaaacacccgggcgtcctgattctttccgacgacatctacgagcatctgatcttcgatgatgccgagttctgcacaatcgcagaggtcgagcctcgcctggcgcagcggaccgtcaccatgaacggcgtatcgaaagcctacgcgatgaccggctggcgaatcggcttctgcaccgcaccgcgctggctgctcgatgccatggaaaagctgcaaggccaacagacatccggcgcaagctcgatttcacagcacgccgccctcgccgcgctcaccggaccactggagttcatcgaggccagccgccaggtttttcagacgcggagaaacctgatggtgaaggccttgaacgccacgccgagccttcgctgcgacactcccgccggcgcgttctacgcattcgcatcctgcgaaggattgatcggcaagagatcgcccgcaggaacaccactcgtcaccgacgaggatgttgcgctcgcgctcctggaggaagcggatgtggctgtcgttcatggcagtgcgtttggcctgggcccatacattcgtattgcctacgcactggacgaccacgcactgcagcaagcgtgcgatgccatttcccgattcgcctcggcctgcagctgagttgtctcagggggccggtgctagagtgaatctatggcacatgaaactcccggtcgactgcgagtcgccgagctcagaaaactggcagctgaggcggagggcttcagcgccaacgaaaactgcgtttgccggatgcggcatgccggtggatgggaaagcatttccgacgaacgttggcccgtcgatctcatggagttgcaaggtacattgcgtgacgaggaactccaggagccgactttcgaagagttccatcccgccggcacgcgctacgactcacccgatgcaccagtcgcggtcgatttctttccattcaaccggtgcaacgtctatcgctgtgtcgtctgcaagctagtggtcctgcggtacacagagtacggcggctactacgtggatcaccgggcacgttgtgtgaaggcgtcgttgatcgtcgattgatgccaatcgacggatgaaccgcttcgtcagcgggcgagcgactgtgccaacgcgatgtcgagaaatgaatcgaccaactggtgtggaatgccgttgcggcggatcgcaaagacgttggctgtggtcttgactcccctcacgggcaggaaccggatatcgctgcggtggctgtccgcgaccgacttgccgaccagcgtgaagcccagtcctgccgcgaccaggcccaacgcggtatggatctccttggcctcatagccgactcgcggcttgacccccgcggcttcgagtgcctgcatcgtgtgccgggcgaagctgctgttggggtctttcggatagctgatgaaggaagcgtcggccaggtcctgcggattgaggaccttgcggcgggccaggggatcggtggacggcaaagcgaccagcagcggctcgctgaagagcggaatgcactccagatcgtcctccaggacatagggtccgatggtccgggccagcccgacgtggatcagcccgttgcgtaacgcttcaccctggtgctccgtgaggatctccgtcaagtcgatgcgcaccttcggcgcgcttcctttcatcgtgcgcacggcatccggcagcacggagaagatggtcgagcgtgtgaatccgatgctcaaccacccgaagcggccaagcgacaagtctttcgcttcttccagcatccgctgcgtatcggacagcaacgccttcgccttcggatagagaaaccgcccgagcggcgtcaatttcatcggtcgtgtggcccggtcgaagagcttcccgccgagttgttcttccaactgggcgatctgcatgctgactgcggcgggaacgacatgcaacctgctggccgcaaggttggcgctctccgtttcgaccacctcgcagaaatagcgcaatgctctcagattcatatcttctgatcttagagccaaaactcgccgattgcattcgctcttttcttaactgagcattgagggcctgtttcaactccccaggagacaaccttgacttccgatgtgaatgagccggaatggctctcgcaagcccgctcgctctcgacggccgaagtgtccgacgcactggacttcttcaacctgccgggaagcgcattgggcgtccgcccgatcgcgggcccggccaagctcttcgggcaggcgttcaccatccgcttcgcgccgatcgaacgcggccagccgggcaccgtggggcgactacatcgaccgcctgcggcccggcagcgtggtggtgctggacaacgccggccggctcgactgcacggtctggggcggcatcctgagccggcttgccgcgcacaagcggatcggcggaacggtgatcaacggcgtgtgccgcgacacggcagaagccgatgaggccggctaccccctgtacgcgctcggcaggttcatgcggaccggcaaggaccgcgtccaggtcgaggcctacgagcaaccggtgagcctgggcgacgtacgcgtgtgcaatggcgacctactgatcggcgacgacgacggtgtggtggtggtgccccaactgccaaggcgggccgaacaaatagcaccagtaagacggcagtgcgaaggaggcgcgcggatgagttcatcgcaactactcggagatgaagtagtcatgactaatgtatagtcatgactaccatattggcttatgcgacacccactcgcaaaccctaatgaagcggggcgaattggttgaactggctcgggcttggtgcagtgaactagggcgtaccccagtccagcgcttgagcgcgcatatggcgtggcaaaggaatttacgtgcttgtgtgcgttgatggattgaaagccaaccggtgcctagctgaaagtccccagtgctcgatctcaatgatgtggcggtgtttgtggaagttgcgtgctgtgacggcttcgccgaagcggcttggcgcttgaccgcgccacctggtgcctgcacggccccgatgacgcagagattgacgtcaaggtgagtgggtgttttaccagcaacacccaggatgcgcagcatttggctgcccgcgctggactcaggagcgccgcgctgccatcggtcttgaccgtgtccggcatggcgtcgggcacgctcgtccccgtcgtaccgcagtacctggacatcaccacgcatcgcgccgcaggtaagcacattcatcgaatggcctcgcgcgcatttcctcacgctgcaaacgacgtggcccgattcggtcaaggccctgcccgggcacccgaagagatccgacttcccacggaggcggcatggctgagcgtcgcctccgctcgacaaccaaccgcacacttgagcaccaacctaccccaatgaagaacgacaaaccttccctgctccctgccccagacgactgtaccgagagcctcctgcgccgcgaacttctgctggggctggggatggtggcgatggcggcctggctccccggctgtggcggaggcggtggcagcaacgaatcggccggtccggctgacagtttgccgccgctcgcccaggaggcactcgatgacgccgccgcggaaccggtgccggccgtcgacaagagcgtcccccgtaccttcgcacaccctgggctgctgcacacggaatccgacttccagcgcatgcgcgacaagctggccgtgagggcccagccctggacggatggctggaatgcgctgctgcgcagcggccgcgcgcagctgtccgcaagcgcggcgccgaatcccgtggcgaccgtcatcagggggggcgacggagagaatttccgcatgctggtcgaggacctgcgccgcgcctaccagttcgccctgcgctggaaggtatccggcgacacggcctacgccgacctggccgtgaagtacctcgatgcctggtccgccacgctgaagacgatcaacggcaacaatgacaagtacatcgcggcgggcctgtacggttaccagttcgccaacgccgccgagatcatgcgcacctaccgcggctggagcgccacaggcgtcgcacgctgccagcagatgatgctgaacgtcttctatccggtgtgcagcgagttccgcagccgttggacctcgttcagcgcagagtacgcgatcggagcgtgggcatcctggacgctactgaccgcctgcggcctggcggccatcggcgtgttctgcgatcgctcagacatctacgacgaggcgatgacgtactacaagagcggccgggccagcggctcggccctgcacaacgtgcacgccatgcaccccggctatttgggccagtggcaggaatccggccgcgacgccggccactgcacgctcagcatcggcctggcaggcgcgctgtgcgaaatggcctggaaccagggcgatgacttgtatggcaacctgaacaatcgcgtgctggccgccgccgaatacgtggccaagtccaacctgtccgacgccaacggcaggccctatgacatgccgttcgtgccgtttaccaacttcagcggcagcgcgcaggcggtggccgagcaggacaagccatcgctgcgcccgatctgggaagttctctacaaccactacgtgaaccgcaagggtattgctgcgccgtgggtcagcgcgatgtcggcgaagctaaggccggaaaccgaccagtggatgggcgacgaccccaacgtgggcacgctgaccttctcgcgtgacccggtagctccggccaagccatcccaactgacggcgatgatcgcaggaggccgcgtccagctctcctggtggggcagcgcgggtgctacgggctacatcgtcaaacgcgccacatcgctggacggtgcctaccagaccattgccaccgtttccggtctgtgcacctacacagacactcccggcaacggcaactggttctatgcgatcacttcggtgatcaaggggaacgaggtcggcccatccaatcgcaaaggcgtcacgatgcccggcagcctgcgcatgcgcattgccttcggtgaaggcagcggcagcacagccgccgacatggtggttcgccggaatgccacattggcctcgggtgccggttggggcgaaggccgcacatctggcagcaaggcgctgttgctcgatggcaggggtgcgcacgtcgcgctgccagccgacttggcttccggcctgtcggatttcacgctagcggcctgggtgtacgtcaacagccacgcgaccgacgcgcggctggtcgacatcggatccgacgacatctcctacatggcgctcgtgccgcgcgatgcgaacagcaggctgcagttcacgatcagcggtacttcttttcgcggggagcagagcgttgcagccccccaactgccgaccgggcgctgggtgcacgtggcctttacgctggccggcatcaccggaacgctgttcgtggatggtgcgcgggtggccagtagcaacacgctgacttatgcgccgtacaacattgtcaactccagccaggcctgggtcgggcgctcgcagttcagccacccgggtttcaacggcagggtgcaggacttgcggctctacgtcggcgccctcggcagcatcgatatcgctgccatggcaaggtagttgcaaacccagcgagcgtgccccgggtcatcggcagttccaccggatagaccttcacgggcgtactaccggcacctcagcgaaataccgcggcggcgcatggtgccgcgatcacagcccatccccgtgggtctactggactgatgaagccaaaaccaccagctgcctgcgcggcttcgccttcggccgcaacgacatcgaatacatgcaattcaccacacgcacgacgcctgcatggtgtctgcccgacgcatgctgcctccgcccgcagcgacattgctcaagcagcgcgccaggaagatccgcactacagcgccggtggccatggtgaatatcgagcaagccttgaaacgcctgggccttgacggcctggtccgtcgaaatgatctcagtggcgcctttgtcgtggaggccacagccgagcagattcgagagctggcggcgacgcccggggttcaggccattcggccgaatcggcggcatctcaatatcgcttcctaggcccgtcgaaggaaagccatggaccaggctccaactcaacgatcactgtccgatccggcgggccaaggcacagcagaccaccgacgtctgacccaacggctttcggatgtggtggacgggcgtcagattctgtcgccggcgaagttcatcgagatgatgggcctggatagcttcgcgcggctcgtgctcaccgatccccaacgcgcgttcgatcaggacagcttccaggagctgcgctcgcacttcattcggttcgcggctggccgatgcaccgtcgtcacttcgacgcacatgagatgaaaactcatatcgcgtcggacctccacgcgcaatccgggcgcgagccgtcggcgcccaagctgatgttctttggagacccccacggcgatctcgaacccatgatcgccgccgtcgagcgcttccggcccgaggcgatcatcctgctgggcgacattcagccacgtcggcctctgcacatcgcgctgggcccgatcctggttctcaccgaggtctggtttatccatgggaaccaccacgacacggactccgatgccgactacgacaacctgtggggatcggagctcgccgaccgcaacctgcatggacgcatcgtcgagatcgccggtttcaaggttgcaggtctgggcggcatctttcgcagcaagatctgggaccctcgacaaccgctcaaggaagccgcattcgcctcggctgacgcgttgcgccggtccatgcgtcccgaggagcggtggaggggcggcgttggccgtcgacaccgctccaccatcttcccggacgtctatctgcaactgctgcgcagcccgcccgccgacattctggtgacgcacgaggcgcctgtagcacatccgcacggctggcaggcgatcgacgagctcgccgagacgctcggcgtccagctcgtagtccacggtcaccatcaccagagcatcgactatctcgcggaagggatgcagagtgctgcagcaccgttccgcgccttcggcgtcgacttgggctcgcatctggcgtggccgcgggatccacaaaaggagactggatcggaagttcttcctccagggtgatcctcttccttgacttcgacggcgtgctgcatccggagggagaagatcacatcctcaacggcggcgtcgacttctgcttcctaccccgcctggaggctttgctgcgcgagttcccgttcgtgaagatcgtgatgttgtggaccgacttcgagctcacgatcgaaacgcctgaagggctgatcagcgatgccgggcgtgccatgaagatggcgaccaatctgctgaacgactacgcgctgatccgcacggtcgacgagtcggccgaacccgatacatggcgggacaagcagggaagaaagctccaggcggccgacacgcttcggattcatcaggcgcagcgagcctggctgcgcgacaagctcggcgaaccgttcgccggaccgacggtggtcgtgacgcaccatgcacctcatcgcggttcgctggcgcagcgctacgccgatgactgggcgtcgggcgcattcgtgaacgagcttcctgacatctttttcgatgttcccgtgctctgggtccacggtcacacgcatcagcagttcgactatcgagtccgttcttgccgggtcgtgtgcaacccgcgcggctacgtgaactggagaggcaggatcgagaacaaggtattcgatccgggtctggtcatcgatgtgcaacctctcgctggaggtggtgacttgtgaagctgctttgcggagttcgagaccttcgaagttccgaaggacctgaactacgacgtagccgtgctggcgggtgtcgtcggtgaagacctcagtgctgggccatggcattgctctgggctggtttctcgatggcacgcaaccgtttcaccagtcttcgccgccctaagcgcgagcaacaccgcacggcgtgcgccttcctgagccggggcgctcggctgcaacgtgctcgccggcgacggccaggtgatggcggccgaggttgacgctgcggctcgaaggcgcggtgcgcgacacgggcggcctgcacctgatggacgacaactgcgccacctccgtgcccggcctctacgccgcgggggatgcgacaacgcgaggcgatctccggcggcttcaaaggcggcagccacaacgcggcctgggccttgttgtctggcttctgggccggcgcggcggtctttatagggttaaaccattatgaacaaccggttgttctaggattaaccttcataccaatcccgaattcagcagtgccatcccacggtacttcgaaccacacaaccacgagatgcatatgaaccgcagagaaaccatcttttccattgccgccctagccgtcgtgaggtccgggagcgcgtttgccgcgggagagccgaagatcggtgtggtcgtgaagatcggtggcatcccgtacttcaacgcgatggaagtcgggatcaaggaacgcggaaaggtgttgggctacgacgccttcatggtcgcgcccaccggcacggaccccgctctgcaggtcaaggcgatcgaggatctcattgcccaaggtgtgaaggccatcggggtcgtgcccaacgatttgaaggcattgggacccgtcctggccaaagcgaagcaggccggcatcttcgtcgtcacccatgaatcgccgaacaatcccaacgccgactgggactttgaactcgcgacggtcgtaggctacggcgaggcccacgcgaagctgctcgccgaaaaaatggatggcaaggggcagtacgccgtctacgtcggctcactcaccgtacccttgcacaacctgtgggccgacgccgcagtcgcctacctcgccaagaaccatcccaacatcaagctggccggcgagcgctacggcgtttcggaggatgccgacaagagccgggccacgacgctcgacctgatggcggcgaaccccgaactgaaggccgtgctttgcttcggcgggcaggggccgatcggcgccgggcgcgcggtggaggaacgtcgccgggtcggaaagttcatcgtggtcggctccgtctcgccgcgccagggaatctccttgatcaagaacgacgtgatcgccggtgggtttcgctggaatccccggacatcgggccaagtcttcgtcactctggccgatcgcctcatcaaaggcgtccccgtcaaggacggcgacgtcatcgaagggctcggcgtcgtcaggccggatttcaagaaccacacgatcaccgtggacgggctcatcaagctcgataagacgaccgtcgacgagatggcggcccagggcctttgagggcttcgacttcgaccactagcgaaacggagagcccgatgccctcaatcgattcggacgaatcgccatttctctcgctcagcaacgtcagcataaggttcggcggcgtcgtggcgttgcgcaatgtcgccttcgaggtccgccgcggcgaggtgcactgcctcgccggagagaacggcagcggcaagagcaccctgatcaagatcgttgcaggggtctaccagcctctcgatggtgcctcggtccgagtcgatggtcaacggcatccgcagatcagcccgagactggcgcagcaactaggcattcgagtcatctggcaagacctcgcgctctttccggagatgacggtcgccgagaacattgcgatcggagagttcgttggcaagaggccgggcttcgtgagccacgctcgaatgcgggacgtcgcccgcgatgcgctcggcaggcttggtgtcgaactggacctggacaggtcactgcgcaaccacccgattgcgcagcgccagatcgtcgcgatcgcgcgcgccctcatcggagaggcaaagctgatcttcatggacgagccaacggcctcgttgacccaatccgagaccgactacctccttggcatcatccgtggacttgcagcgtccggcgtggcggtcgtgtttgtgagtcaccgcctggctgaacttctcgagatcgcggaccgcatgacggtcctgaaggacggagaacttgtcggcgtgttccctacgaagggaatgacccagtccgatgtcagccgcctaatgaccgggcatcccctgcagcagttgcgtacggctcggcgcgtgccgggtggccgcgcggtcctcgaggtttccgggctcacgcggcgcggggagtttgaagacatttccttcacgctggccaagggcgagacactggggatcactgggctcctgggcgcagggcgcacggaactcgcgctagcgctcttcggtatggcccggcctgacaagggggcgatccgcctcgacggagtcgaactcaacctgcgatccaatcgcgatgccattcgcagtggcatcgcctacctctccgaggaccggctctcgctcggactcatccaggtccaggcgatagaggacaacctggtgcttgcgtcgctgaagaaaactgtcaggggcctgtttctgtccatattgcgcaagcgcagtgccgtctcatactggatctcccgcctgcacatcaaatccggcgcattcggcaacgcaatctccagcctgtcgggaggaaaccaacagcgcgtggcaatcgccaagtggctggccaccgatccaaggatcctgatcctcgactcgcccactgcgggcgtggatgtcggtgcgcgtgccggcatcttcgagattgtggaggaacttgcccagtcgggactggcgatcatcctgatctcagacgaggtatctgagatccatgcgcattccgaccgggtgctccacatggcgcacgggcggctcgtaggcacctacgacccgtcgacggtttcactcaaggaacttgaagagtcaatctatgcgtaggatcttcgccaaccactcaaacgaactggccctcgttgccttcattgccgtcatcagcctttttctgtcggcgacaacgaagaccttcttttcgctcggcaatgcgctcgacctgctcaacatcagcgcggtgaacatcatcttcgccgtcgggctcctggtagtcctcgcgtccggaggcgtcgacatatctttcagcgtcgcggcatcggtcgcccagtacctgacggtcctcgccgtcgtgtcgctcggccgactgaactggctgtgcggcctgctcttcgcgatcggcttcggcatcaccttgatgtcgatcaacgcgttcctaatacgacagtttcgcgtcatctcgatcatcatcactatctctacgttcaacgtgtacttcggccttctgatgttctttaccaagggccactccctcttcgatctgcccggttggctcgccaagacggtcgtggtcttcgaacgcgaagtcgagggcggcgactggctagagatcaagcttccggtgctggcaatggttgcatgcgtcgccgccacttggatactgttgactcgcacgacaatcgggcgccagatcttcgcattcggcgacaacgccgaggcggcgaataggcttggcatcaacatccgcgccatccaatacttttcctatggatggttgggaatgatggccgggattgctggactgatgcagatccactacaccaaggaggtcgtgccccaagccctggtggggcgtgaactcgacgtactggccgcggtcgtcttgggcggcgcccggctcggcggcggaaaaggcagcgtctcgggttgcgtactgggcgtgctgctgatcgcaatcacgcagaacggattaaacctcatgggcgtctcccctttcgcgtttcagatggttgccggactcatcatcattattgccatcacactttccagtctcaagctcacggcccggaagccgctcaaaggattgccatcgtgaccgcgcgccaacacaagcccgtttgggcggtctcgacggaaaccaagacgctgtcggcggcgctcgccgtagcgatagtgaccttcgcgctaatcgagccgcagttcttgtctctccgcgtggtgcaatccgccgcgttccagctgcccgaattgggaatcctcactctcgcgatgctactgcccaccctcacgggcggtttgaatctcgccattacctacaccgccaacattgcggccttgttcgtcgcctggatcgttctaatcaacggcggcacagacgcaggcgtcggtgtcttcgccgtcgcctgcgttctggcactgctcgttggaggcgcgtgtggtgcaatcatgggcagttccatttcgctcaccggcgcgcatccgatcctggtctcgctcgcgatgatgatcttcctgaggggcgtaggagagttcttgaccaagggcggggacatgtccgtccttccccaatttgtcagtcacctgggacaaggcagcctctggggcataccgatcccggcgatgctcctgctcgcatgcctggtcggcacccacgtcttcttgggccgcactcgccttggcttctatacctacatggccggctccaacatcgaggcgacgcgttatgcgggcgtgaatacgcgcttcgtcatcgtcgccgcctacgcgctttcgggagtgttgtccgccatcgccggcatcgtgatgatgacccgcttcaactcggtgcgggtgggccacggggaatcctatctgctgatcaccatcctcgcgtgcttcctaggaaacgtggatccgcacggcggattcggaagagtgctgccggtggcaatcgctttgttgctgctccaggtcctgacgtccggagccaatgctatcggcgcgaatcagcatctcgcgacggctttctggggcatgctgctcatcgtcgtgatgggggtgcgctggctggcttccgcgttctccgagcgccgcgctaagcggtcgttcaagcgggcgcaatcgttggcggtcgggccagcgcggatcgtgccaccggcgtagcggcctgcaacccccgaggaggggcgcattcggccgtcgcgtatcattcagcgcgcctggcgggcctcgccgctaccgcggggatcgccctcgttttccaatgccgaccggagggtccagcatcctatgactgaagcgaagccgcgtcgcaccaccatctacgacctctccaagcgcctgggaatttctgcgccgactattagcgtggtgctcaacggtacttggcagaagcgccgtatctcacgggaaaccgccgagatcgtgttgaggcacgcaagcaagatcgattacatgccgaaccgccaggcgcagtcgctgagaggcagcgccgggacaatggtgggactgctgatcccgacgcacgacagccggttcttcgccactgttgcgcgcgccttcgaggagcgggtgcgtcagagcggacgttgtcctgtcgtggtcagcgccgcgcgcgacccggtgcgggaaagggagacgaccaagaccctcatctcctactcgattggcgcgttggtcgtctgcggcgcgaccgatcctgacggggtccacgacatatgcgagaagttcggcgtcccgcacgtcaacatcgatctgcccggcaagcgcgcaatgtccatcgtgagtgacaacgtcctcgcgggaaccagcctcacggacgctgtcctcgagcgcctgctcgcgaagggggaattgcaggctgccgatatccatttcgtcggcggcttgagcaatttggcaacgagagaccgaatcaagggcttcaagcagtccatggtcagccgccgcatgaagccgaaagccgacgcgatccagaccattggctatgacgcggccatcgccgaagcgaacttcgcagcgctgtacggccagggcaagaacgtaccgaaaggactgttgattgacggccttcctgtcttcgaggggttttgccgattcgcccgtgctcattcggttgccgccgaaagcgtggttgtcggctgcttcgactacgaccccttcgcgtctttctgctcgttcgagactttcatgatccgtcaggatgcccggcgcatggtcgacatggccatggatgccctcgaatccgaaaacgtccaggcgggcatccactatgtgacgccagaactggtctgctaggccccgtacttgttcctgttgatctgcgcgaagaaagcttcccagtcggccttggtcagaatgcgcggctcgcccagcgagcgcgagagaatgtactgccgacagacgatctcgagccggtgcgtcagcttgatcgcctcgttcatgtcctggccgcgtgccgtcatgccgtggttgctcatcaagcaggcggacgtcgtgcgcagcgcccccgcaacgtcttcagccaactgcgagctgccgaacgtcgaataagggacgcaggggacttcctcgccgccgaacagtcccaccaagtaatggaacccaggcaacggcttgcaatgacaggccacagctacgcaattgtccgagtgcgtatggaccaccgcatttgtctctgggttgtcgcggtaaatcgctgcatgtagctgccactcgctcgatggacgcagctgcgcgcgccattcaccagcggtgcttacgtagacgacgttctccacggagatatcagacccgttggcgccggcgggcgagatcaacatcccgtcgccgaaacggacactgagattgccggaagagagctccgtcagacctagatcgaccactctcttgtacgaagccacgaggtcggctctcgcggctttttctgtctcttccattcattttccttggtggaaccagatatttgaacaatcggttgttctagtttattcccgcctcatcttctttgtcaaattaccaaattacttccacgattgatctttcaaaagcaatccgttagagttgaacaatcggttgttcaatttctcatcgtaatcgcaaggatgacaatcggggagcgaaggaatggcggcgatagcagtgctggacatagggaagaccacgctcaagcttgggatctatgcgtcgactggagcgaagctcgctagcttcgaagccccgaatcgaccaatacccggcgtcttctatctggagcccgatcaccgggaaacctgggagtttttccttgcgtccctcgcaagatcgcaggcttcacaaccgatatccgacatcatcgtcagcacccacggctcgtcaggctacctcgtgaatgaggatgggacctggacgcctcttcctgactatgaaagcgccatgccacacgctgtgcaggaggcatacattgcagaatcggacggactcgaggagcgcggcagtggaataagtcccggatcggggcatcttgcaagacagctgttctgggtcgagcggatcacgccaaacgcgctgctcaaagcgattgcgatccttcccgccgcgcaattctgggcgtggcgcctgtcgggcgtcatggcgacggagctgacagccctgtctgcacaaactcatctgtggaatgctcacgaggatcgcttcacatccctggtgtaccggcgtgggtggcagcgcctgatgcccgcggtcaggcacgctggagacgtgctcggcaagatcgaagcgcggcttgccacgttgatcggcgttggcctcgacacgcgtgtccattgcggcgttcacgacagcaccgccaatttcttccgataccagagttccggctacgaggatttcaccttgctctctagcgggacgtggctcgtgtccatgagcgacatggtcccagtcctggcccaagtccgtcgcgactacacagttcacgtatccgcgagccgtactcccttctggagcgtccggatcatggctggaagagacttcgacacgttgagccaccatgctcgcgattgcatcgacctcgaccgagtaaacggagtgctcaactccggagtcttcgcgcttccgagctttggtcccgtggaggggttcttgaagggttcgggtggacgcggggaaatggtgggagcgcctcgcgaaggcgcgatcgaccgtgccgcactcgcactcgtctactacgccctgctcgctgacctgtcgctcgacacgtatccggatcgtggcgacatcgtcgtcgacggcaacatcactgcgcaggaaagccttggctccttgatcgccgcgatgcgcgaggggcgccgcgtgctcttctcttcggcgaaggacgggacgctcatcggcgctgcatacctggcgggcgctcgaccttcgtcgcctccgttgatgcacgagcaccggcatgacggtatcgacctacgagccctgcagtcctaccgaacagcgtggcgtgctcaagtgctcgagcgatatccggacgcgacgccatttgtaacagccaaacggcttgacggcggagatcaatgtgacgagtggctcaggttgacgtcccgccaacacgagatctgaccctgtcgttgggtaagaaggcaagtgccgccaccgcaaatcctgcgctgatcaatgggactgagccaacgttgtcaccatgcacggacagggaggcgacgagcggcccgaatgcgcttcctagcaattgcaacgcaggaacgaccatggccacccgtccagtcggatccacgcgaaaagcgaggctgatctggaatggcagcaagaagatagctgcgaatccgaaggtgccgcatgccaacacgaactgaacactgctccctggcacaaggcagtagacaacaaacccagctgccccgatcacaagcgtaccgctgagcagcatcagcacgtcacgcacgaaacgcactgcccacgtcgctgcacagcagccaagcaactgcatgaacagcgacatggaaaccactgactgtgcgtccttcgacgcgaacccgattgcgtggccaagggcttcgaggtatgcccagaatgacccgatcgccgccagctggaggaagacaacgatcaaagccgaggcttctagcctcgaccagaagaaactcgatgcgggatcgcgttccaagggaaacatgtgagtcggcaacatccggaccaatgcgcagggaatcaaggacaggcaagccagaagtatgaatccgcccctccaacctgcgagtggaatcacggctgacgccagcacggcagctacggtcgcctgtgctgccgtttgggcgataaaatacaggccgccgatgcggcttgggttttcggaccggacgatcacgttggtgattccccagatcagaaggccctccgacaggcctgccgccgcgcgcaccgtcgtcaggccggaatcccccatacagaagatcgtagcagcgtccagcgatgcggtcataaccgatgccacgacaatactgcgtctgaggtgctgcaatggaagtagcgcatttccaatgactacgccgatgccaatcgcgatgatctcggccattgccacgaggcccaccccctccattgagacattgcctgagttggcaagctctcccaaaagtatgggctgcaagccggcgatcagaacagcaatcgaaccgatgattaccgcggcgactatctgcagtgtgttgatcttcccgacattgaggtcttgatgcgtttgcatagcggtttcaaagttagttttggctgtcggaagtgacatacgcgcgcaggcagtgctgcagatggttagtcagaagctacgtgagacggaaagaacgactgcgcttctgtctagacggcgggtgcgatcaccgtcctgcaccaggtacagctcgactgccttggttcttgttgtgacccagtcgacgttccactcataaccccaccgcttgtgcgtcaggccgatgcgatagtcggtgaaattgccctcagagaaatttgccatgcgctgatgaccggcatgcaggttgagaacggtcgtcgaggtgagctcgtacttgtagtcaagatcaagcagcaaggtccccctggtgccatggttgcctcgaccataacaggaggccgcggcttgcggatctgcggaaaattgcagaatgcttccgcacacaccacctgtatcggccccccgataggtgcgcgacagcacgttgaaaacgcgggcttcgaacgcgccgtaacctacctccaggagtgcgaagttcgtgttgtagttgctcgttcggaagtcgccgggcgtggagcttccagcgtcgtacgactgcggcgcactgaacttcgctccgggaaagacttccgccgccaacccaactccgaagtgccagccgtcggggttgccaaatcggtacccgccggcgaatgttgcgctaacgccgttgccttcggggaactgcttcttgttgaccgttgcaaagtcggcgaagacgacaaagcctgatgcatgcgccgcttgcacgctgagccgtgcagcggggcccttcagtgaatctgaaatcccccgattgcgggaatcggaggtgaatgtcaccttcgtgtcgatcgcaaagctggctacaccgtcgtcttccgactcagccgcaaatgatgcagttgcatagacaagaagaattacgcccaatgcggggggcgaggtaaagttggtcgtcatcatggttatgtctgggtaccttgatgaacacctacgacttgcacgcgggtgctgagggcattgccagcacctttgaaagtcgctccgtttggcccagtatttcggtcccgacaaacgcgcgaatcctcatctcgtcagtcttgacgcgcactgtccctttgtactttttctcgtcccgggggtcgtagatccaaccgtctcgccatgcttcgttctcataccgactgagctgtgcaatgcgaacaccgcaggtgtccttttctttgccggcatcgacgtcccagacaatttttccgcagagcgctccgggcttgtcgggacaatccctgaactcgacgatggcatctttctgctcggtcagccaaagcccttgggcgtcttctgggcttgcggccgcgttgccgagtgaggctgccgaaatgagtgccagggccagtgagaagtgatagcgatgattcatgacatctattcctcggaaactcgattgagtaggtgttattcggcttgtcacacgccgaagatcgctggtgcaagcctgaaaattcagatgccgcacgagggcgagcgggcatggattgaactggcagacgagcccgacgggctcgcttgccatcaaacagaaaccaggatgcgacgttcttcggtggctcgcgctcaggccggttgaacggccccggggtagttgtgagctgccgcgagctgcattagcggggcgaggcgcgaggccggcggtatggcgttgcgatcacgcgcgatcgcagcgaatgcctcgtccgtgacggcgagcgtctgtgtgatgacgctttggtcgtgcgccaccgagaagtacatgttgtgccatgggtgcaaatagaccccgcgctgtacgcaggccgttacccaggcatagccgacgcggaagtcagggtcgtcttcaaacaagacttgagggatttgcgccgggccggtttggcgcaggccgaacccgtgtgagactgcctgctgacgaagaccctcacgaagcgcctctgcggaggctttgagtttttcgaggtagtccgtgtctcggatctgcttgagcgttgcaaccgctgcggccatcggcaccgacgaaaaccagaaggatccagtgacgaagatgctggcggcggcggcgcggatgcgctctgatccgagcagcgcggagatgggatgcccgttcgcaaagcactttccccagcagctgaggtcgggttgaatgccgatgagcgaccagctgcagtcgcgcgccaagcgaaaacctgcgcgtacgtcgtcgaccacaagcaatgcgccggtctcgtcgcagagcttgcgtgcggtagtcgcgtattcaagatctgggctttcttgatcgcgaaaactgtcgtgccggaagggcgtggcgtataccgccgccacctggccttcgttggccttgaatgcgtccaccaaactctgagcgttgttgtactcgtagtagacgatgctggctcgatcttccggcaacgtgccgatcttgaacagctcaggcacacaccaaggcgctgcaccgtggtaggcgccccgcgcagcaagaatgacgcgcttgcccgtgtgtgcacgggccacgaccatggccatgcttgttgcgtccgttccgttcttgcaaaacatggcccaagccgagtgcgagaccatcgacacgaacagttcggccagctcgatcattacttcacttggaccggtcgtcgtgtctccgagcttgcgctgcgcgtccgcggcggcctcgaccactgggtggttgtagcccagcaggttcggtccccaggcacacatgtagtcgatgtactcgttgccgtcgtagtcccaaattctcgcgccttgcgcgcgatggatgaactgagggaactcctcgggaagtagcgccgtcgagagatggccgtacatgccgccgggaatcacttgatgagcgcgctcgcgtagcgcgagttcgcgcttgttgttgccaaccatatcgaatccttctgtggtttagaaatctgctcagccggatcgccaagcgccaaataaccaatatttatctggttatgagaggtgcaatgcatgttccgtgccgggatttttcaaccattcggaggcattggaagtggcttttttggtgcaacaacctcaacatttctgcggttctcgcccaaaacggtgccgcagatcggtgcgcaagagctgcatccgcatcagctgcataatttgtatatttatcggggtagcgcggatggctcgttgagagcgggaagatgtgttgccgtgcatgtagcgccgcagcgttggcgtcaaggtgacccgctgctctaaggtcagaggccatgaaaatcaaggattcgacaaaaaccaatgtgagtgccgcgcgaggcacgctcagcgcaccgaagcgccccaagcaagagcgcggcatcgcgaggttcaacaaactgcttgacgctgcagacacgctgttggcgacgcacgaactggatgaagtggggctttaccagatcgcacaggaagctggcgcgcctcccgcatcggtctaccatttcttcccgtcccctcaggccgttctcattgccctggctgagcggtatcaccaaaaggttgccgacgtgagcctctatgtcgagccgggcagcagcccgacgtggcaggagcttttgagacagcgcttgtcgtcaacagtaaagatattcaaccaccatccgacgatgcagaagctgttcctgggcagccacgcgaaccacgaaatggcgtcttccgaggttggcttcaacgagatgctcgctcagcgctttgtttcgttctacgaccagttcttccacatgccggtcatcacaggtatcgagcagaagtttttggtgatgttgacactgctggatgcagtcatgaggttgtcctatgccaagcaccgcaccatcactgcggagtttgaagctgaagcagcactggctgccatcgcctactgccgtacctttttgccggaagtaatcgagttgcgcgcggcgaagcgggcagttgatcctcgttgaagtggcgctcctagggtcctattcgtggggaggcggatagagctgggctacggcccgaatcagagaaaaagccaggccgcaaccaatgtcagcgaccccgcatagaggccgcccttgtcgtgcagccatctgaagaatggcgtgggcattgattgaccgattttcattcggcccgcgcccgctcatcagccaaccgacaactccgagcgcccgcacgcgaggcgaacagcaggtcatagagcactggaatcagcccaagcgtgactagggtgccgaccgccaggccgccgatcatcgtgatcgctatgcccgtccacaatggcccgccgaacagcatcagcggcaccaagccgacgatgcaggtcagcttggtcatcacgatcggccgcaggcgcttcacagccgcggcgacgacggcctccctgcgctccaggctcttatgcaactctacttcgatgcgctccagcagcaccgcgttgttgacgatgatcccggccagcgcaagaaggccgaatgtggccatgaagccgaatgggtagcccgtgagcaagagcgccagcgccgcgccgatcagcacgaatggcacgctggccatcacgatgaacagcttgcgaaatgagttgaactgccagatgaacagcagcaggatcgctcccagcgcgtgcggaaagtactgcagcagcggcctgattggcctgctcggcgtcctcgatttcgccgcccagttcgatgcgatagccggcaggcagcttgagcgccgcgaccgtgccggacaacttcgccacgatgtcgttggcggtcaggccggggttgtgtctgttgatttccatctggaagtgaccccctagggtcagagatcggcggaatccaacacaccaaattccggcgcattgggctcaacacccgtgcgatgtgcatcagcatcaatagtagatattaatcgatttccctaatgcgaaaacgcgccttgctggctacgatttccatggaacacgataaatatcgcatttaagaagccaggccctcaaaaattcggcgcaggaacgatcaacttcagcatggaaaaaggagtccggatggtttggaacaacccgcgcaacaacgccctgcagaagcgcgcgcagcgcttgatcccgggtggcatgtatagccgcatgccgaccgggccgctgccacacgaattcccgcagtttttccagcgcggcaagggttgccgcatctgggacgtcgacggcaacgagtacatcgatttcatgtgcgccttcgcgcctgaacctgctgggctacaacgatccgcaggtcgatgccgccgctgcccagcagaagctgggcggatgcgctcaacggccccagcaacgaagcacaagaggagacacgaatgacgatccgttggatgttttccgcggcatggccgcgacgccgaagtaccagaccgcgcgtcgctctgctggccatgctgctggcggtctcggcctgcggcgagggacccgtacctgcactctctgcgctggacatccggcaggcggaatcgctgcgacccgcgtcggccgatctgcgtgcgcgctacgagcgatcgtgcatggcctgccacacgtccatcgacgcgaaggcgccgctgaccggtgccgtcgcgcaatggaagccccgcttggacaagggcatagacctgctggtgaagcatgcaatggaaggcttcaatgccatgccgccccggggactgtgcgcggattgcgatgaggcccatatgcgcgcgctgatcgtattcatgagccagggaaaggaggcactgccatgaatcccgtgtcccgacgagatcgaggaagccgccgcacggtgctgaaagccggcgccggcatcgcggtggccaccgcgctggccggccggggcgttgaagcccgggcggccgagacagcagccgcggcaacgacaaccgagcccccgatgccgacgccaaaggtaggctggacgaactggtccggcatccagcgctgcacgcccaaggccttcgaaaccccgagcgacgaggctgaactggccgaggtgctgcgcaaggccggctcggccggagtgcgctgcgtcggcgccggccattcgttcaccgcactggtgcccaccggcgccacactggtttcgctcgaccgcatgtctgagatcgcgaccgtcgacgtgcaggcgcagaccgtgacgctgcaggctggcgcacgcctggcgctgctgtcgcgccagctcgacacacagggcttcggtctgcgcaacctgccggacatcgacacgcagtctttcgcgggcgccatcgcaaccgccacgcacggcaccggcaagacgcttcccgcactgcacgccgacgtcctcgcgctgcggctcatgacgcccaacggcgaggtgctcgaatgcagcgggcagcgcaaccccgaactgcttgccgccgcacgcgtgtcgctcggcagcctgggcgtcatcacgcaggccacggtgcgcgtggtgccggccttcaatctgcatcgccgggtgttcctgcgaccgctgcagacgatgctggatgaagcgcccgcgctggcgcagaagcaccgcaacttcgagttctactacctgccccacaccggctatgccgccggcatcgtcaacgatttgtatgccggcaccgacaccgtgcagtcgccttcggccgacgaggacatgctgcgcgatctgcgccgcctgcgcgactggctcggctggtttccgcagctgcgccgctgggtggccgccaagctaatcgacgccgaccagaccgaggaggcaaagaaccgctcgtggaagctgctctcgacccagcgagccaccaagttcaacgagaccgaatgccatgtgccccaggccgatgggctcgcctgtgtgcgcgaggtgatcgccgcgctggaacggcgcaacgacgtgttttttccgctcgaattccgcttcgtacaggccgacgacgcatggctgagccccttccaccggcgcgacagctgctcgatcggagtgcatgcggcccaaggcgagccctacgactacctgctgtcggaaatcggtccaatcttccgcaggtaccagggtcgcccgcactggggcaagctgcacgacctcggccccgcgcaactggccgcgctatacccgaattggaacgatttcctggcgctgcgtgcgcaactcgatcccgatgggcgcatgctcaacccctatctgcgtcaactgttcggagtgaatgcatgagccgccgaaagatcgtgctgggcaccctgggtgtggccgccgtgggggccttcgcactgcgccccggcgacaacggagcgccgtatgacgactacttcggcgcgctcaacgaagagttgaagaagaacggcccgatgcgcccctgcatggtcgtcgacctcgatcgcatggaccgcaacctcgaccttgtgatgcgcagcctcaggcaaggcggcaagcactaccgcatcgtcgagaagtcgctgccttcgcacgcgctgatcgactacgtcgcgaagcgctcgggcacgaagcggctgatgtcgtttcaccagccctttctgaacatcgatgcgcagatttttccgagcttcgacattctcatgggcaagccgttgcccgtggcatcggcggccctgttttacaggcagcacacgggccccttcgatccgtcgcggcagctgcagtggctgctcgacacgcccgaacggctgcggcagtacctctcgctcgccaaggggttgggcacgaagatgcgcatcaacatcgagatcgacgtgggcctgcaccgcggtggcatcgccgacaacgccacgctgggccgcatgctcgacctcgtcgtggccaacccgcagcaactggagttctcgggcttcatgggctacgacgcgcacgtgggtttcggtgtgccgaagcagttgggctcgccccaggaactgctggccaaggcgatggcgatctaccagggctttgtcgaccatgtgcgcaggtattacccgtcgctgtggaacgacggtctcacgctcaacactggcggcagcccaagctacaagcttcacgagactgagaagctgagcaccgaagtcagcaccggcacggccctgctcaagcccacacactacgatatcgacacgctggccgcgcatgtgccggccgccttcatcgccacgccagtcatcaaggccggggggccggtgatgatcccggcactcgacggcaagtcgaaaatcttctcgtggtgggacgtgaaccagcgcgagaccttctatgtctatggcggctactggctggccaaatacgagtcgccgaaggggctgcagttcaacggcatcctgggacacagcgcgaaccaggagaacgtcaccggctcgtcggcggtgggcctgaaggtggacgaccaagtgtttctgcgtccggttattgtcgagggcgtactgctgcagttcggcgacctcgtcacgctacgcggcggcaagatccaggatcactggccggtgtatcaacaaacgggatgaaagtcatcgaaggcccccttgaaacaagacatgcgacggatctggacggtgcagtcgcgctcgaacaggtgcacgatgttgccatgcgtgtcgccgaggatctgcaattcgacgtggcgtgctcgctgcaccagcttctcgaagtacacctcgtcgttgccgaaggccgctagtgcttcgcggcgggcggcagccaatgcgtcttcaagctcgctctcgtggtgaatggctcgcatgccgcggccgccgccgccccaactggccctgagcattaccgggtagccgacttcgtccgcaaggctcttgcattccgcgatgtagcagtagcggttcggtggcgggcatcactggcaccccggccgccactgcggcgttgcgcgcagccaccttgttgcccagggtgcgtatcacctcggggctggggccgacccagtggatgtcggcgtcaatcacggcttgcgcgaactcggggttctcggacaggaagccataccctgggtggatggcatctaccttggcggcgcgcgccacgcgcaggatatcgtcgatgccaaggtatgccgccagtgccttcttaccctcaccgaccaggtagctctcgtcggctttgaatcgatgcagtgccaaccggtcctcgcgtgagtagatcgcgagcgtcgcaagcgcgaaccttgaacgacgcggaacacaggagaattcgaagtcgccctcgggcgacgttcctgacattaagggggcatgcgctcagcacgagtcacagcgattgatcagtcccaatgtgctgtggtcagttttgatgcagaggccggcgattcggctagcagtgataaaagccgcgcaaggccatgggctacctggcttggcgtcattggaatgctccgggaacgatcatgtcacgcactgcagcattggcgagaccggcaatgcactcgttcgcaggctgctgaccgattcggcgtgccgcttcaaggcttgcatcgggtaggcccagcggcgccaggaggcgctgagtgagtagatctgtgctgagaggcaaaactgcgcttggcgcggcgactttccacatggttccgaagcagttacaccggtgttcttgcgggcgtgaagcaaatgctgaccacaggtcaactcgcaccagccgtctcccgcagcttcgcaatggatgtgatctcgatgcggccgtattgctggtggatcgaaccagttgccgcgagccaccgaagctctttggccacggtctgcctcgtgataccgagcattgcagcgagcgtttcatgagatacctgcacggctgaccgcgcctgcgtcggggctatcgatgagacatcgccctgcgccaagtgcaacagccggcgagcgacctgtgcacgcatagatctcagcatcgcatcctcgaccgcgctgtagagtcggtgcacgcgtccggccagcaacaacgcgatggctgtggagaaggcggcatgctgcatcaggcctgcgaacgcgatggatggcactgtcaataccagcgaagagtccactgccatgacgtcgtgggatcgtcgggagccatcgagcagcgacgcctcgccgaaccagtttccggcgtcgaggaatgagagaaccgcttcccgcccgtcctcgcacagggtcgagaccttaagcgtccctcccatcactccgtagaaggcacgcggtggatcgccgcgccggcataggatctctcccggccgcagacgcagtacctgcccagcctgcagcagttcgttgcgatcctcgatgggcagcgaactgaaccaacggttgcccgccatctgcttcatcagagccgggtcggtcagcatccccactcccaccttgttgtcaaaggcagcgaaagcccgtgaattgtcgatttcttgactgtgttgcatcgaccgcgcctgtaccgtgtatgtctattccatgactgcaggaaattccaatgaacatcccatcgcttaaagagactgtgagcaccgaggaatggcagctgcgctgcgatctggcggcttgctaccgattggtcgctcactatggctggtccgatctcgtctttacgcacatcagcgcgcgcctcccagggccagagcatcacttcctgatcaacccttatggcttgttgttcgacgaagtcaccgcttcgtcgctcgtcctcgtggaccaggaaggcaacaaggtccgcgagtcgcccttcccggtcaatcgcgccggtttcgtgatccacagcgcgattcattcggtgcgcgaagacgtccaatgtgtcttgcatacgcatacgcgcgcaggcgtggccgtcagcgcccagcgtggcggagttcttcccgtctcgcagcagtcgacgttcgtccttgctgcgctcggctatcacgactatgagggcgtggccctgcacgacgaagagaagccccgcctgcaggatgacctcggtgggggtagcttccttatgctgcgcaatcacggcctgctcacagtgggggccaccattgcggacgcctttctcgctatgtatgtgttcgaaatcacttgccaaatccagttgtccgcgcaggccggtggagaactcatcacagtggacccgaagatcatcgctggcgtggctcatgcgtcgcgcgtgcagaccggcggcatggggggcggctttgtttggccggcactgctgcgccgcctcgaacgcaccgacccgacctacaacacttgaccacacgatccagctcccgctaccaaccacaatcatctttcatcaaatcatcatcatgaaatacctcgaagaagtgacatcgaagttcaggtcagccattgcggctggccccacgcccgacaagagcctcaggatcaacctgaaggacaccggcgtcgtcgtggtcaacggctcgtccgtgacgaatgatgacgtacaggcggacaccaccatcacaatctcccgcaaggacttcgaaggcctggtggccggcaagttgaaagctccggtcgcattcatgcagggcaagatcaagatccaaggcgatccaacggctgcgctgcagtggctacccgtcatccagcgcacagccacctgaacagaacgtgggcgcatccgtacggatcgcgccactcacgttcacgtcagaaggccccggcgccgatgcgtcaggggcctctcagcatcgcctcaagccgaggtcgcttgacgcgccgccaactgagcatcgcggccgatcatctccatctggtcgatcaggccgcgcagcttcttggcgtcagtaccgagcaagcgcaccgcacgagcctgctccggcggcatgaagacctcgagcgccttgcgcttgacggcacgcatgatggtctcggcaacgaactccggtgtgactggttcgctcgcaaacgctagtgcggtcgcgtcgtcgttcttctcctgctccagcatcggcgtttgtgttgacgtggggtgaacgatagtgaagtcgatgggtccgcggcgctcttcgagggcgagggcgtgatggaatgcacgcagcgcatgcttcgacgccccgtagctcgcgatgccggggaacgggaggaacgccgtcatgctgcacacagtgaccatgtgaccgtggccctgctcacggaagcgtcgcatcgtggccagcatgcctgtcactggacccatgaaattggtgtccatggtgtgctggtgcaattcaatcgacacgtcgcgcgcattgcctgtgtgcacgatggctgcgttgttcaccaacacgtcgaggggaccaaagcgctgctcggtggcgtccagcgcctgctcccaagcctgcggagagcggatgtccagcgcgacagagcaagcgcggtcacccaacggtgccgccatcgccttggccccgcgcaggttgatgtcggccagcatcacttggtgaccctgctcgatggccaaccttgcgaaggcagcaccaatgccgctagctgcgccggtcaccaaaaaaatcctcggctttttgactttcatgcttcgatctttcagtacaagtgaactgatgtggggagttggacgacggcgctcaagcctggcctgcgccaggcacttccacacgcgtcgccaggatgcgcgccgtgcggttgctgcggcacactgccggatcggtgctgtctgcggtgcagatgtagagcgtcttgcggtcttcgccgccgagcatgcaggcagcggccaactgcccggtaggaatgcgttcgaccacctcgccgccctcacgcatgcgcagcacttcggacgtgtacggcgatgcggcccagataaggccctccgcgtcgaggcagatgccatccggtaccgcgccgctgggcagttcagcccattcgcgccggttggacaaggtcccatccgccgcgaggtcgaacgcggtgaggcaggctgctccgctctctccgacgatgagggtcttgccgtcggcggtaatcaccatgccgttaggaaagtacgtctcttcttcggcgatgtgcacggtcccgtccggatcgacgcgcgccaacaccgccgggcagggatcctcgggcggatatagcgagaagccaaagttgccgacgaacgccacgccgtcctcacggacgagcatgtcgtttgcgaggcctgtggcaatggcagacagatcggcgtgcaccacgaagtttccgtccccttcgcaccgcagcactctcttgtcttccatcgagacgacgagcatgcggccgtcgggcagccatccaatgcctgacaccgggccggggaacgtcgcgatcgtctcgcgacgaccgtctggcatcagccgtgccacttcgtttgcatggatgtcagagaaatagagtgcaccgtcatgccagcgcgggctctcgccgaaggcgaggttctcaaggatcgtttcgagtttgcgggtcatggcattacctttggtttcatcgtgtgttgaagccgcgatcaggcggcgtagtagttggcatagagacggccggtttgcttgatcatctcggtgtcgcacaagttggcggcgaagcgggcagggttcatgctcgagaggtccatcggtgcctgcccagtcacgatccaatgggctagcaactcgcccagcacaggtgagatcgagaatccatcgatatcgcgtccgccgagcacgtacaagcccttcacactcggtgccgggccgaaaatgtgatcgcagtcgactgtcgtggtcgtcaggtcgctgcggcattcccgcagcgcgatgtcgcgcaggacagggaactggccgtggatgcggccaaccagtgcacgcgctgcagagaggtcggcctgcaggtgctcgccgctcagattgcgcagcgcctctcccggcccaagttgccggggcaggtcctcgtagccgccaaacatcaggccgccttgatccgaacgcacgtaggcgttggcatccagaatgtgcacgaccggttgcggtgataccgcctggggcagcgacacgctgatcatcatgtggtgcagcctggctacttccggtacgcacgcgcctgccaagccagccaccaaccgcaaccagccacccgctgcatcgacaacggcagtggtgcggatctcgccgcggcctgtcactacgcgagagacgacgccgctctccacgacgagctcatgtacctcagtgttcggcaacaacatcgcgccgcgccgcgccgcagcccgggcataggccggcgccagttgcgccggctctgtatatatgtccttgcgcgcaaagccgaccgcgaggatgccctgcgtctcgagcagcggcatcattgcgcgggcttcctgaggtgagatttccttgacgtcgaggccaaggtattgggctctctctgtggcaccgcgcatcagcgaagcatgctcaggcgtacgagccagggtgaggctccccgcctggatgaactccagcggctcgccggtttcctcggtgaaccgttcgaacttctcgatggcgcgcccacccagtaccgtcatcatctccgtactgcgaacctgcctagtgagcccggcggcgcgtgatgacatctgcgagccgatctcggccttgtccacgagcgcaacattgcgcccttcgcttgccaggtagaaagcggtgctggaaccgagcggacccgatccgatgaccaccacatcgacgttatcggtcattcgattcactcatgattgagacacgatcggcaagcccactttcaacagctcgcaagacagagggatggacagatcgacgccatcgcctcaccgcggggccacaggagtgtcgagctcgtgcggacgggggcggcacgcttcacccgtctcatgagcggtggcgcttcgaagtgctagccagacaaatggcgcggcggccatgacggcggcacacatggcataggcgaacttcatgccgcccagttcgctgaacgcggagcctgccagcaccgtgccgccccctgcccccaggaacgtgatcacgacgcttcgggacacgagggaaccgtccgtatcgacctcggaaagcatgccagtgaggaacgggatcacgacgaacagtgacgcgttgatcacgacctgactcacgagataccacagcgggcctgccgagctgaagaaggctaccaatgacgcaaccatcacgagctgcgaggtccagatgatcgacaggcgatgcgggcgactggccgattgcgacggaacgacggccccaatgaatccgagcagcgacgacaacgacaacaggatgccgatcattgagcccgacaggccgacgcgtgcacccacgatgccagcgaccgcccattgcgaggcctggatgccgtagagcagaacgatgacgatccagacggccagcaccagcttcaacggtgccttagcaccggacccggtcgcgtgagccgggcgctgatggagggcgaactctccaatgtgcctgagcgcgagcaccgcggccaccatcaggccagccagcagtaggaagatccatcgtgacagtacggcctcgggcaagaaggagatgcccaccaggatggctccgtccaggatgccggcggccaagttgatctgcccccacaagcggtcggtggacgcgcggtgcgcgacgctggcagcaacgacaacaaacagcatgccctcgaacaggccggccagtccgcgtgcaatgctaagcacttccacgttgggcgccaaagcactggccgcctgcgccagcaccgctccgatcaggccgagtcgtgagaaggtgtgagctccccgggcaatccaccgcgggaacaacgcgcagctgacagcgatgccgaatatctcgattcccgcgatctgcgtggcggcactgtcggtcaggccgaaacgcgtcgttaccgcagagacgatgaatggcgtgaggatcatgccgttgatggccaccgcgtaggcgagcgcaagcctcagtacagcggctgtcgagaggtcggaacgatgtgcagtggtgttgtccataggggtggtttgcgtagcgggccgccgcgaagatcttgctggagacttagttgccgaggaacaatcgggcgacaaaccgggacagcttcccgtagggcgcagcgacaaggtcggacttgttgaatgggctgagcgtcatcacaccgcgggcgtgcgagaggcgaatgaagccgtcgcggccgtgatacgcgccggtgccactctcgccgacaccaccgaacggcaggtcctcctgggtggcatgcagcagcgtgccgttgacggtcacgccacctgagcgcgtgttgtcgagcacggcgtcaatggcacgatggtcgttcgagaagcagtacagcgccaacggcttggggcgggcattgatgagctcgatggcttgctggatgtcgcggtatccgatcacgggcaggatggggccaaagatttcctcgcgcatcgccatggcgttggtcggcacaccaagcaggaccgtgggcggcaccttgcgctcaccggcagcgcgggtgtcatcatgctgcagcacgcgcgcacctgcgcttcgggcgtcttcgatcatgtcgaccagccgacggtggtgccgatccgagatgaccgaggtgtaatccgcatttccggcaacgcgggggtacatctctgcagccgcttcgaggaatgccttggcgaaggcgtcgacctggtcctctggcgcgagaacgtagtctggcgcgacgcagctctgcccgccgttgaacagcttgccgatcgcgatcaggcgggctgccttcttcagagggtagtcgcggcacactaccaccggcgatttgccgcccagttccagcgtcacgggcgtaaggttcgcggaggcggcagtcatcacgctgcgtccgaccgaggtcgaacccgtgaagaacaggtgatcgaaggggagagtcgaaaagcgaccggccacatcggacccgccgaggatcacggcgactcggtcttccgggaaaattttcgacaggagcgcagccagaagcttcgaggtgctgggtgtcagctcagagggcttgatcatgacccggttgccggcggccagcgcttcgacgagtggcacgagcgtcagggtcagcggatagttccagggcgcgagcactcccaccacgcccaacggctggtagacaatgcgcgcgctggctgggcggaacgccatgcctacgctgcggcgcaccggcttcatccatcccttcaggtgcttgcgcgcatgcttgatcgagttgagcaccggcatgatttcgccgaaatctgtctcggcggaggagcggttgccgaagtcggcgcagatgcttgccgccaactcatggcgatgctgtttcaccgacccgaacagggcctccagagcggccattcgctcctggtaggtgggggcaccttgctgctggacggccgcacgctgcagcgcaaagatgcggcaagcctcgtcctgagcctcggcggtgtgatggagggacatcatggcagacatggggttgttccgttctgttgtggttgagccgtgcgggagttcagaagaagcactgcccgtcgccgcgataggtgggcactcggcctacgatggctccgtcttcaatgagcacgagttcattgaagcgctcgcagagttcacctgccttcgcatggcggaacagcaccggatcgccgatctccagtcgtactccggggggcagcaccaccggcgtctgcacctcaccggcgccctcgttgtcgagcagactgcagccggcgggcagccaaggctgcggcaaccgattcctacccgccggccccgaagcgcaataaccgccgcccgaacatgtcaccattcccggtttcggcatgcgcgtaaccgctagcgcgaagccggccgccggctgcgcacggaacgcggcgtagtggtcgaatagcgtgggcacgtaaagccctgagccggccgccagctcggtcacgctcgtgtcctggagcgtgctctcgaagctgccggtgccgccgccgttgacgaagcgcaaacggtgccctgcctggccaagcgccgccacggtgtcgcgccgacgcgcattcacctcggccatcgagcggcgcttcaggtaccgaacgatgcggttcttcaagccctggccgggctcgtcgtccatcaagccggcaatctggccttcgtagcccatcaggccgtcaagccgcacgcccggacgccgggcgatctccccggccagggccaccgcggatgccggaccattcaccggcgagcgaaacgggccgaagtggataccagggtagtcggacgacatgtccaaatcgatggacagcgggagcgtcacctgttcggtctgcgcaatcgcggcaagcttctctacctgctcaacgccgtcgaccatcagcgtgatgctgcgcccggctcgcacctgggcggccacggcgtgcacgtccgccggctccaccgagggataggccacgaccaagtcgtcgaagccctggctggccagccaggccgcttcgccggccgaatagcaaagcagcccctggaacaggggatccgtagccagcactcggcggatgatgcccacggagcggatcgacttggtgaccaggcggatgggcacaccaccggcacgctgacgtagcagcgtcaggttggcgccgaaggcatccaggtcgacaaaggccaccggcagcctctcaccggctagcgcgctgcgaaagtaggcatggtcccgcacgggggggcggccggccaatggtctgccgttgatgcgggatgctgcgcatggctggaccgcgggggatctcgccacaggcgctttgaaggattgcattgaatggcctttggtatcgcggagtcacgacagattagtgactgaccagctttctctggggtccgaatcggccaggcatcggggtacattcggccactcacatctacgggttatccctgttcgatgaaacgcgcaagcgggtcggaaagcggctgtatcaatggcagtcggccgcgatcggcggtgagaccgaccgcggtcaagcgggccttggaagagacgggagaggtcgagagagggctcagcccaggtcgcgcgagacgacccaggccgagatcttgccggtgatcgtcttggacaccgagacgcgtgccgcccacgtcaccaacttgttgctgaggcctggcaatacgccacgcttgccccggtgcatggcttcgtagccgattttcgccatggccccggggctgctgaatcccagccgcgccatgcggcgctcgtcgactagtccagcggcctggaagaagttggtctttgtcgggccaggggccagatgcgtgcaggtaacaccggtgccgcgcagatcgaaagccgtggcctcggagaagctgatcacgtacgccttcgaggccgaatatcctccttcgaggccatgcggcactacgtagcccgcggacgaactgatgttgaggatgcgaccccgtcggcgctgcaccatgggccgcacgaaatgaactgagagttcagacagcgtcacaacgttcaactcgagcatcgccacgaactggcctatttcgtattcctgcaccggcagccctacgatacccgcgccggcgttgttcacgaggtagtcgatctcaacgccgagcgcctccacctgctcgatcaaacgcccggcccctccgggcaccgagaggtcctccgtaagtggatgcacgcggatgccgtactgctgttccagttcagcggcaaacaccgcaagctcggcgcggctcctcgggctcgaacagaccacgaggtcagtgccgtcgcgggcaaacagtcgtgcgaattcggccccgatgcctttggaggcgccggtgatcaatgcatagctcatgggtgggtgcttctgccgttagatgtacgagatgtgacggcgccagcgacgaacgcgagcgcaggatccccccaccgtacaagtcgctgcaggagggagggggggtaaaatcggtcaccgctgtgtctcaaccggactctgcgaagcctctactcaaagtagcgcaatcgagcacgccgatgaccatcaagctcactgcagatccccgatattcgaaggcggatgtgccgccggccgtgattcgttcgaccctggaactcgcgaaactgcgcggtcactcggccgagcgcctttgccgaggcctgggcctctcacccgacgatctccagaacgccgacatgcgtgtgtcgtatcggcagaccagcctcctcattcgtagggtccagcaggctgtcggtgacccggcgcttggcctgtcagcggggtcgcgccaaaccatcatctcgttgggcttgccgggtctgggaatgctcacctgtcgcacgttgggcgaggcgatcgcctacgcgacagaacatcaacaggacgctggagcattgcttcaccacaggcattttgtcgagggtcaagcgttcatcgtggaagccacccctcgcctgtacgatcctgaactcgagccctatttcgtggaagaggccttctcctgcgatgtggcggtagtgcgaagtctcatcggtccgcagtacaacccgcttcggttggaactgagctaccccaagcctgcctacgcagcggcatattcggcgttcttcaaatgcccgttgcggttcggcgcgtcggcgaaccggcttgtgagtgacgcgcgctggttggagtactccctccccgggtatgaggaattcacctgcccgtatttgcgcgctcaactcgagagcctgatgccacgacgccaggaacgcaacgacctgctggagtcgatatcgacgcacctgcgcgcccatctggacgagccgcgcgcccttgaggagacggcgagcgacctgaacatcagtgtgcgcacgttgcgccgtcggctggccgacctaaacctgtcgtatcgcagcctcgttgaccaagcgcgccacgaacgcgccttggatctgctgaagcgaacgtcactgacccatggccagatcgcactggccacggggttcagcgacgcgaggaacttccgccgtgcgttcaagcgctggacaggtcagctgccgggtgacgcccgaggcgctcccaattctgttgtgtgacacgcaacatctcggacccaatgtcgattcgatggccgcttaccgagcaggcattgaagcggtcgcaacgctcctcgcgcacggtgagcgatctcaagccgctgttgaagggcgactggtcgcgcaggattaacagtcaacgaaacgttaactgtccacccagttcgcctgaagcgaggtccctgtctgcgttcgcagtcatggccacgctatgcaacaggttggtggtcatgtgtgcatctccttgaaatgatcgagcggcgctccgtgtcgcgcgtgagtgctgtagttaccccacctcgattcgttcctaccggtcgatcttcgcttgaagttccaaggttccgattcgtcccaggttatcgactatttcgccgagatcatcgaaacgaacaccccacgccggtccgatgcccagcgagtacaaagaagcgttgtatcgatcgggcctcgcatgacagaccgtgacttcactacgcaccgccaaggccaaagccatcccgacggcttgcatttttgagcccatgtgaacgaccgatatgttcttatgatcttgcccccgtatttcaggacacgggctattcgcaatgtagcgcctgctcgatgtgagccagacgctgttgggcagcgcgatgctgcctgaactccctgggtgatttcatcttcaatgccgagtgcggatgcacctcattgaagtgctcgaaggctgcggccatctgcgccattgccgttctcgcatcggcaaggtccatgcggctgacgtaatcgcgcttgaacgtgttcacgaagctctcggccatgccgttgctctggggactgcacacgggcgtgttgaccgggctcgggcccagttgtcgagcacgcgctgtagcttggcgatctcggcacgagcggctgccagttccgaagccggcaccacagcctcgcccgccgatacagccgtcagcgccccttgccgctccagcttgcgccactggaacagcaggctggcggcaacgccttcctgacgtgcgacgagcgacacgctcatgccaggttcgtagcttcgacgaaccagtgcggccttctctgcaagggaccagcgcctgcggcgctggtccctcatgatcacttcgacggtatccgtattcctagtcgtactcacagatggtatgggcgcctccctcccaggctacttccgcaccggcctatacggtgccagagttgtcccccctaaacgaatcggagaccgtcatggaacgtacgatcattgccgtcgacatcgccaagaaaatttttcagttgcactgggttgaccaagagaccggcagcatcgagcgtctcaaattgaagcgcaaccaaatgatcgaatggttcgccaaccgtgagccgatgctggtcgtcatggaggcatgcggcggagctcatgaatggggtcgccaaatgctgaatttgggccacgatgtccgattgttagcgccaaggaaggcccgaccgtttgtgcaacgaaacaagacggatgccgcagacgcgcaggcgatctggaccgcctgccgccagcccgggatgcgcttcgtcgccgtgaaatccactgcgcagcaagtagttctagcgctgcatcggattcgcagccaactgatgaagacacggatcatgcagaccaacgaacttcgtgggctgctctatgagtttggcgttgtcctgccggaaggccacaaggctttgctcaaagaactgccgaccgcacttcaccaggcggaggagcggctgccgtccatgctcatcgaaagtttgcacgagcagattcgtcgcatcaaccagcttcagtctgatattgtcctcatcgagcgccgcttggcacagcagctaaaagagagttcggcatgcaaggcagtcgccgagatccccggggtgggcttgatgaccgcaacagcagtcgtcgccgccatgggctcaccaacttccttcaccgatgctcgcgagttcgcagcctggatcggcttggtaccgaggcagaccggcaccggcggacgcatagtgagcgtccagtccgaccatcttgaaagcctgctcggagcataggagcctagtccccatcaacaactcttggtggacacgtgagcactatccccgatcaacaagccggcacacgccggcgacgtcgcattcacagcgacgaattcaaggcaaacgcagtggccagctgcatgcagccgggcatgtcgatggcggccgtggcgatggcccaaggcgtcaacgcgaatctgctgcgccgatgggttcgcgacgcagagatgaactcgggaaccaccgtcgtcagcgcgaccaccgccgaggccccgaaggcgcaagaagccaagacagtgttcgtcccggtcagcttgccgccaccagggcagccggctcatgtcccggacgttcgcatcgagctgcgacgtgggccgatagcggttaccgtgacctggccggcgagtgccgccagcgagtgcgcggcctggatgcgcgagctgcttcgatgatccgcatcgacgcgatgtggctggccgcagaccctatcgacatgcgcgccggcgccgagcgcctgttggcgcgcgttgtgcaagtcttcggcgcagcgcaggcgcaccatggctacctgttcgcgaatgcccgcggcacgcgcgtcaagctgctggtgcacgacggcttcggcgtgtggtgcgcggcgcgccggctcaacgcggggcgcttcgtctggccgggcacgacccacacgacgcccttgctgtcgctcacacctgcgcagttcgacgccttggtcctgggcctgccgtggcagcgccttcctgagctgagcatcatcacgcgggcctgaggcccagacacaaccgcccttgcatgcgtgacagtggatgtgccgatggcgtcatcgtcgtggtctggcaccatgcaacgcatgcttggcgtgcgtgatcttcctgcagcgaatccttcgggactgtccgccgagacagctacgctggttgctcagctgctccagcgggtgcaagaccaggagcaacagctggccgagcgcgacgcgctgctgcagcgcaaggaccgcgagatcgcactgcgcgaggccaagatcgagaagatcaccttcgagctggccaggctcaagcgctggaagttcggcgccaagtccgaggccatgaacgccgagcagcgccgcctgttcgaggagacgctggccgaggacgaggcgggcctgcgcgagcagctggagcggcttcggcgtgaagccgccgcggccgcggccggcgcagctgcctcggacacaacgaccaaggcgcccccgcgccggccgcgccgcaacccgttccccgatcacttgcgccgtgtggaacaccaccatgagcccgagcgcaccgactgcctggagcccggttgcgggcgcccgatgacgcgcatcggccaggaggtcagcgagcgcctggacatcgtgccggccgagttcttcgtgcaccgtcacatctacggcaagtgggcctgccgctgctgccaggtgctgcgccaggcgcccagcgtggcggaagtcatcgaaggcggtatcgctgccagtggcttcgtcgcgcacacgctgatcagccgcttcgtggaccacatgccgtactaccggcaagcgaccatcaacgcccgcagcggcgtgcacacaccgcgctcgacgctggcgtccatcaccggccaggcaggtgcagcgctggagccgctgcacgaggcgcacaggcgcttcatcctcagctgcgcggtgctgcacgccgatgagaccccagtggccctgctggacccgggcgcgggcaagacgcgccgagcctacgtctgggcctacgccagaagctggcacgacaaggtgcctggtgtgatctacgagttctgcccgggacgcggggcgcagtacccgctggcattcctgggaggccgagggagacacggccgacgatggtcgggcacgttgctgaccgaccgctacggcgcctacgagaccgtggtcgatccccggctgtatccggaccgcctgggcgcagcctgcgccgcgcacgcgcgccgcaacttcgaagagttgacgcacgacggcaccagcgtggtgggcctggaggcggtgcgtcgcttcgcgcgcatctacggggtcgaggcacagttcaaagagctcagcgatgacgagcgccgggcgcaacgccagcagctcgccaggccgctgtgggaagagctcaagcactggctacaactggagcgccggctggtagccgacggcggcccgacggccaaggccatcgactacacgctggggcactgggccgcgctgacgcgtcacttggacgacggcgcggtcgccatcgacaacaaccacctcgagcgccaaatcaagccgtgggcgatgggccgcaaggcatggatgttcgtgggcagtgaactcgctggccaacgcgccgccatcgtgatgagcctggtgcagtcggcgcgcctgaacggccatgacccctgggcctacctgcgcgacgtgttgcagcgcctgccgacgcagcgcgccagccagatcgaggacttgctgccgcaccgatggcagccagcgtccgacgcgcgaccatgaccttgctcacgcaggccgtgatggtccgggcgaacatcgacgtcgaccgcatgagcgcgcaacaaaaggttgagctggctgacgaaatctacgtccagcagcccaacctgctggcctccatcctcgtgttgccgcgctacggtgtcgacatgctgcagcttgaggtgccgatccacgttctgctggtcgccttccaggccatgaagcactgcgggcacgccgtgccgacgatctctgaagacgtccaggaaacctgcttgcagcggctgacggcgacgatgcagttcaccgagggcgtgccgccagacctcgttgcgcagatgatcacgaagttctgcgtcgaccaccccgagcgctacttgttggcgttcgtgtacggccaccttggccagcacgacctgctgcgcgtgagaactgacgccgagaagttcttgctgctggccgccctcaacctcgtggagtgcattgcctacgtcggagcgcagttgcagtccaagtgacccgcgtggggccggtcaagatgggatgactggacgctcacgacgcatacggcaattgggcatcagcaagcgaggcgacggacatttgcgaacgctgttgatgcatggcgctcgagccatcgtcagatctgaacgggcgacaacctggggctggttagcggggctactcgcacggaggccttattgcgtcgtggtcgctgcggtggcaaacaagatcgcgcgaactatctgggccgtcctggccaaggggcagccctggcggcaaacggcttggcagacgtcgtgatgccaagttgagctgacgaaccaaaggttaggagagcaagtgacgcgacatgcgtgatgggtcatacaggtaagaccgggacgggaccattccggtaggagtagtgagcttcgagctcgactcacagatgggaagctccgtcagcgaatgccatcagggcccgcaggcaattcagcctgcaatgcaggccgaatataagactgcagcctgctcatcgaccacgcgcgagtccgttcttgcaatccgggaggcgcccatataagtcctactcctatctttaaagataagcgatagaccgtgtcctgtcattcaaggggccagctcacttacccgcctgggcatccaccttctcgatcacgatccgcagtatctgctggtaatgcaacgtcgaggcctccaccgaattggcgtcgtcgagtacctccacctttgcgccgacgccttgctcgtggcccgacatttcatcgagcagactggagattaccttccgctgcatttcaagacgaaagcttcgccgaggctcagggggactgccaagaatccagaaaatgaagttatcggggtctgccagtggctggtccgtcaatcgctgaaggcatctactcagacgctcagtcctgtacggaggaacagcaatgatgaattcctcgcgattctcattgctctttccggggtaaagctcgttggtctcgacttccgctacgccgtactcatgaaccgagctctcatcgccaggacggcatgccgtgagcaccaaactttcgctgtcatttgcgtattgcgcgctcgtcggcaaggtcagtagctggtgggcttgaggtctggtgcgagcagaaatgcggccgccatcacgacgcgctccgctgcggcgagcaaacttcttcagtgcgatgccatgacgttgacctgataggacacgtccagcagttttcctttttgcgcgtagtagcgatcgagtcgccattccttcaggatgtccatcgcaagggagaaagtcccaagtttcagcacatagagactcgtgagaggaaaatcgacttcggattccagggccaggaccaggcgggcgagggtccgggactcttcgctgctggggtcggcggtgatgatccggcgggcttctttgattgcgttcatgctattcctcttgaagaacagataaagggcggctgtcacagcctcgaaacgcagtgctggcctactcggcgccatgtaggtagtttttcttgctttttcaggcgaggagtgccaaggttctccggtcagcgccgcagtctagcaccggccactttgtcaaggcacgtgttttgcaggcttgaaggctcatgcgccattcgttcgtataccgtggggttcgggttgacgtgtcgctccagaagcagggcgatgcgtgtcgctggagttgcgaactgggcgatgggtcaaggcttcgagctgcaggcggtggctcaagctcgtcgatcatcgaagagttgcacttggcatgcgtagcggcgcgtcgggagatcgatcggcgcagccgtattttggcgccccaccatgagtgattccgttctgagccttcaggtccagcgagtgactttcagcaacagatttgtctggatgattctggagcgcggggccgaagatgaggccgtcgagattgcggcctccttgtggacctatgacaagccctccgaggcatatgaagcgggcgcgaccgtcttgcaaaagtcggaacggtgcaatccgcagcgtacgtagtcggccgtccaacctggacaatccgacgcgggctgagtgagaaagatcagcacggggggcgccagttgtgggaaagcagttcgtcgatgcggctgttcgggcgggctttgcgacgctcgcgcactgcgcgaccaaggattcccagaatgggtggtcggacgcgctacgcgccctcgagccaggccttccactcgaacggttggaatccttcctcaggactcacctcgtccgcggtgcgcagttcgctattgcgccagtgccggcggctcagcggttccgccacgttctcccagtcatgcacgaacaagcctgtgaagtactgtgccagcggctcgtcgtcgaacagcaagctggcatctcgattggttgtcgcgcccatgttggtcaagttgtggctgcccagcatgacccgcttgccgtcgatgatcagtcctttggtatgacagcccctctggatcctgatgcgcttggcgtcgaagccgtagtccttcagcgcctcgaacatcacccgaccgcctgtcggatcccggtcttgcagtcggaagatgaggcgcacgtctaggccgcggcgttgtttgctgagcagcgtgttccagaactcgatgtagcgcccgtcggcctgctgtggcggcaccgacaggctttggttctgcacgagaatcgatttgcgcgccgccttgatcgccgggatggcgatgtcgaggtagttgtcgggcgtgaggattggctgcaccgtgaactggcgcgtctcgtcgaacggggcgaaataagtcactgcggccaaaccctcttccgcacgcggcaccgtgcctccgacgaaccagagttccggcagccccgcgaactcttccgggcgtgtgtcgcgattcgcgtcgaaatcgccgcgcaccgctgtctggtaggtctgcgcgaggccgggatgctcgatgacggcgtgccattcccggttgttttcatcgagcagttcacgcagtgcggcaatgtcgttaaccgggtccgcatcgggctggctggagcctttccagttgccactcgagagccatagcgcctcgtcatctcggatcagtaccttgatgtgatagtcgtgattaacccatccgcgcaccgaaccgagcttgacccaggccacacgaagcttgtccccgagcgcgttgcgcaggtcgcgcaccatcgcgtcggagtcgcgcacggtcggcgcgttacggatgcttccccgtgctgaatcgagcaccagggtcagttcctcgaactgcggagcctgggcagtctccgtgagagccagccgaatatggtcggcagtgaattcgtacattgccccgaccaatcgcgtccgggcagcctggatgaactcccgcagcacgggccagcccgcgtcggggctcacatgagccttgacacgcatggtgtcggtgaccgatgccaggtccaaatccggcggtggcacgtaggtaatctcttctggcgtgacccgggccgccagcagggcttccgtacgcgctggcccgacactcatgcgcaggaagtcttcgacgctgggccccatgacttccactgggtacccctcgaaggtgcgaggcagctctgtcacgccagcggccatcagttccgccgtcgtgcgtttgcgccgcacggttgcgaccagtgcacgctggtcggtgatgccgctttcgtcgaacacccagcccgcacggaccccgatcacgtcgttgcgacctgccatcagggcctccttggcgcgcgccaggaccgaggccaagtcggttgctgcgggcgctacaggaagcgccgacgagggagcgggcacgacagcaagtcccgctggcccatcaggaactgcggctctggcgttcgccgcgatgtcgccgagtgcgacagacacccgcagcggaatggtccaggtggcggtgccatccgatgcgacctcggcgcgcaaaccgagcgggtctgttgatggatctgccaaacgtctgtagaccggtgcggctgccggcgttgcgaacaaggcagccgcaggcggggtcgtgacgggtgcggccagcgcctcacgcctgtcgaggacggagggaacgtccggtgccacgagctcatcgaggtagtcgccggccccttgcgccggcccgggattgcgccaccatgcgagcagacgcggcacacgcgtgccctcattggccagccagcgaatgcggtcttcgggcatgccgttgcgccacacggagccatcgacagcgagaatctggcccgcatcattggtggcccacacgccggcccgatgcagcgccacgacctgccactgatcgttgtagacgggagcaccggacgaacctggcgcggtgtcggtccgatagtgcaggaagtcacccggtttttcgatgacctcgttctgccgaaacgcgatctgtttgggctgacccgaaggatgctgaatgatgttggagaactgccccttggcgatcaacgtttcgtcgtcatcgaccaggcggttgtagccgatcgatgccagcttgtggtcatccgtggccgtctccgacactgcgaccagcgcgaagtccagggtctggtcggacaggaagaatcgctgcggctccagcctgaacacgtgcccaggccgtggcgcaccatcgcccagttgagtctggtagccaaactcggcgatcgacacgcgggcgatgtccgccgtcttcagcacgtgccaattcgtcagcaatagacgcggtgagaccaggaagccggtgccgtagccgagcagtgcgccgcttgaaccgttgacacgcacgcgcgccaccgtgcccgccacgcgcagcgctgcctcgagaaacactatctccatcagatcactcgagccgaggatgcgctcggcgcgagtatcgggcggcagggaaaggccatccgccactgaaggcaccgctgcggccatggcgctgaaggccttgccatcggcgctcggctgcagtccgcgcgcagcccagaacggcgaggacgcctcggcgccgaccggcgatcgcgtggcatctcccttcgcgctgtggtcgcgcgccggcagcttgtccccgccgtaggtcttccagcgccgctcgatatcggcaacgatgtcgcggtcgatcagcatgcgttcctccgtcattcgggtttccggccaagctggccgtagttcgtagcatggcgcaaagttcatgacatcgtcatgaaaccctcggcgtatgactgagcgccggtgacgatcgcagggtcgaggccaccgaagaacatccgcacctacctgtctaagttgccggtagcggttccagttccttggcaacgggcgcatggaacagaagcagggtcggttttccggtggtccccgtggcctcatcaaaggaacgcgtgtaactgtagccacaatcacaggtgaaaacagccatgcgccgagcattgcgcaactggtgccaggtgaacgtcgtgatcggcaagcgctcctcgacgggacagacctcgctaccgcacacccagggcccaggtccgaacggcgatcggtgctgatctcgttgctcaaggaaatcctgcagcagcacgtgatagagcggatgaacagagcgccgatcgtttcgcaccatgtgagtcagccagtttccgcgaagcgtctctccgtccatgacgtccggcaatagttccagcgcacgaccatagaactggcgcaaactggcgttcagcaacttctggtcgatcatcaacgcggaccttgaaagatccgtttcatgcagcagttggaagtaatgagcgcgccactccttcaacgtgcgtgccggtggcggctcgtccagcagacgcttgctcagcaacgccagccgctccaagtgcggcatcacatcccagtggccaggaggcacgatcggctccgcctcgaccgggcatgtgctccatgaagccggctgaaagaaatgggactggcgcctttgcgcactcaggcagagacttgtgcgatgccgatggcacatgagcacaccgggaagttggtgctcccgcagccagtagagctccccatagttctcatacatctctgcggcacagttcggacagtaacgtagctccccgacgcgacccacggcgtacgcttgcaatcccgagagggcttgaatcgtattgaggcgtcccgttttcatccccttcctcagcgcttcgcgcatctttggcggctcgaaggccgtgaagtaggggaacagggtcagttcgtcgatcacccggtctgcttccacggcgtgaaagggcacgtgcatcgcgagttgatcgaggtgccccggcagatcgagcaccgccctggcgctcttccgaccaaaaaccatctccatgaagagtctgggttttggttgtcccaggtgaacccacgagcgagccagcacgctgtagaggatctcgccaggatagggtttcggaaaatacgccagcacgatcaacgcgcctgctgctgctgcagatcgagcacaggggacacgacgaccctcgactcgcacagggcttggtagggagagagggctcgagtcgccccttgcgcgacgatgtagcgcagatcggtgggctgcagttcctgcggttgaggggactcgtgatccttttcggagaccttctccttgttgctaaccgacttcaatttggtactcttcaccttggcggtcgccttggctgcccgggtgctttggccccccgcttccgtcttcgccttttctggtgtgcccacctcgatctgctgggcgacccgcttcagcagatccaacggattggccccctcgacctctgcgcccaggctctcgaccagaacctttgcaatgtcttcggagactccgaacgcctgaagcgcgctcaccatcttctgagccggcgtctcgggtccagtcgctgcgggcttgacctggtctgatgccggttgcacccccacgaccagcgatgacgaagcggccgattgcaataccccgcccacgtatatctgaaacgtttgaagatcgtcgtacttcaccagtgccttgctgtccttcagacgaagcgcctggatcatcggtgcgaccaaccagaaatcctccctggcaacacgccggatgagattgggcgtaatgatctccttcgagtcggggcgcgtctcgccgatcgagatcagacgcatttgcgcaagcatgaacatcttgaccaccaggtcggtcacgccttgcgattcatcgtggagcacgttgctgaggtcctgcgtcagcggcgtcgcattgcgcgtccactggaacgtccacatcttctgcagaaagtactcccacacctcatccttgggcatcggatcccaatgcaaggcgccaaggccgctggagcggcgcccctgcctgaaattgccctgcagaacctggacggcactgggcgtgccgatcaactcgacgggaatgccgatcgtgttgaccagcttcaccaggaagctgagcacctcttcgccggcaccggagcgcgcgtgcttcagatgctggatttcatcgatcaccagaaggccgatcccgtgaagcgtggcaacctgcgccatgtgcacgaccatctcgtcctcaccacccttgccgtagagcttgaagtatttcgtgccgagcaactggtccacggcggtgaagaaatcgatgcacagttgcttaggcccccctttctgaggactttccagcttgagccataccaactggaccatgttcagttcgggatgaacaatgatctgcgggtactgcaggagaacctgctcttccgcgcgcgtctttcccacgcccgaacaccccgtcaacgcaaagctcagcgcggtcgggtggaagaaaggaatgacgttgcttgcctcgatgtcttcgatggcactgcgaacccctccggccagacgagcagcgtagccctgtgctgccggattgcgccccatgtacccctgccggatcatcatgtccagccgctctgccagccggatctgccggtccatgggttcgaagtaccgcagcaaccgcatgacgcagtgctttctcagtttcgcggggtagttacgctcccttggatcaaagatcacattgccgcgcaggaccgcggcccattcctgcatggagaggatcggcggcagctttgcgatgaacggattcccctcgtactcggggagattggcggcttcaaaattgaactgggtcatttggcaactccgatttgcatgatttcaagaatgctcggctcggcgtcttcctgttgcgccggggtggggaattggaggacttcgcctccgttggatgggggccgcttggcaggtgatgcaactgcgtgcgccgtcccgtcggaaggggtgaacacttcgtcgcttcgacgctcctgcttttcttcggcacgattcgtacgaatctgggccacccgggcgcgattgctctccgtcgaaggtgctcccgcctgtgcctgcgcatcggcaatggtctcgtcgatcagagtcacgagcgccgagtctgcgagttgctgattcgcgcgatggttggccgaagcgttcttcgcggactcgccctgctcgccgatttcccattcggagagccccaggaacgctcggctgcgcggtgtgaaggtgcacacatcgaacttcttttcgtcgttgcgatgcagatagatgcgctccatgcagcgcgagtcgtaggacaccttggccgaccaacgcccctcctgccgggcccggtcgaaccaatgttcggccatcgcccgttcgcaggtgtagtgctgcccgcgaaaaagaaccccttccttcgtgacgctcgcggaaccggtcggcatgagggcgaacttgacgaggtcctcggggtactgacgcaactgcccgctgcggttcgcgatgccccattcccacagatcgcagggcaccggcaagacctcatcctcgacgaccccgcgatcggcgtcgtagtccttcagttcgtgatggttgttgaagtagaggacgcagccgatgatgatcttggtgaactgatccagatcgagcgtcgcgtccaaccggtagtcgctgccgccgcgggcacggaagtctttcttcacgtaccccggggtatatggcttgaacttcgcgggcaataaccgaaagcgggtttcgacgacgcccttccagtcggcccggtagggcgccgtgttttccacgatcactccgaacatggcctggagcatttccaccttctcgctctccaactcgccacgatctccgagaaggaatgtgcaaaggtgtcggcacggccagtcttcggggttgatttccagaccgtattgggcacagaaggcgaccttgtccgtagcggtgttcgccaaggccatcatcgcgcccacccaggatggcccctccagaccgatgtaaatacccactatcatgcgtgagaagacatcgatcaccacgtagacgacgggtcgacctacgatcttcttgcggttgagccgcgacacgatgtagacgtcggcgatggtggcatcgatcgcatagcgcgcgccaggcccccacacgccctgcgttgccgtcccgatgtagccgcgcatgtccttgtcgtagatcttggcgcctacgcgccgccgccttatgtcgaagcggtcgagctccttgtagaaccagaacttgaactgatcgagcgtggggcgcagccattcgccggactttgcgtcgagtgttcggccgacgctttcctcgcgctgtgtctcctcattcctgacgcggcgcgtgaagaacctcgccaccatgtcgtcataaacgcccttgatggtgaatccgttctcactggtatagacgcccacggccaccgcaaatattttgcgcattgccttcgagacgttggtgccaacctcggtgccgtacttgcgcggccgcccccgcttcaccccttccgtgtagttacgctccttccccttggccccgcagttggggaagtccggcagcaaggcattcttgacttgaccgcgctgccagtagcggcgaaggttgtcgtagatcgcctgcttgctgcctcccttgctctcgatgtgcagcgtgatctcccgagaacgccgctgcggatggaatatctccggcagcatgaccaccatcgtcgctatggagttccaggccgcgtcgcgcacgcgaacttgcgaatcgctcggcgaggctgtcgacgtgacaggcaagaatgggtcctcttctggcttcagaagaagcgcccggcctgccagtacgtcatcggagagctcttccgattcgcggatcgtaggaaatgcatgtcgatcatcgatgtcgaccacgaaccagaccctgttggacggatgcagccagagcaatcgcagccgctgtggcttatctgggtccgcgcctgaatacaccaggaccgtgttgacgaatagcatcaggcggccctccgcagattcatcgaagccgcaactttgtcatccgccaaccagaagacgcccgcggactccttgatatcgaacgggcgatcaaggtcatagaccaggcgcttgttcgacgcaaggtgacgcagcgcggtcagcgcctcgcccacctcaaatccgcagtcgttctgaagctgctggcacaaccactgcatgcttgcgccctgcgtacgcgccagagcgtgaatgaactgctggcacctgtcgcgccaatagtccggatgaggcgtgaccaggtgctccaggcttcgcatctccgcgagccactcaaggttgcctacgcgcacggcgggaatttcacgctcggtgatcagggcccacggcgctccttgcatttcccagtaacgtgactcgatctcgagcttctcgatcacgcgcgcactgtcgttgagctctttcgtggtcttggccgcccgcggcaagagccgctttgccgcatccttgccgtaggtcacgacaacgtcggtggtcatgacgatgtcaacgccggtttttgggtcctggggatgcttgacccccatgctcgcggcgatctgccgcgtcacttcgcgatcgagcggaaattgctcgcgcaagtcgctcacgttatcgtcccagtcgtagatcaagatcagcgctcgctcgatcttggacagcgtgtgatgcagccgcccggtcttgcggccgggaactcgcgacgacaagccgttggaaggcacatcgtggatggtgaggaagggtttgtagtcagccccttcgccttgacctcgcccctcttcgatgaacctggcgatcttgtcttcgtccatcgcgtatcggtgcttagccaagatgcacctccattgcggctggccaacggcgactgcgttgggatgaggtcgcaactgaagagcctgccgagcttggcgaggcacatgacttccactgggacgacagtggatcggatatggaatggttcattaacttcctctttgcaaaacgccctttcgggcccatttgcacgggaagcccctcggcgactgtccgtccggcgcgcggacgcgcacaccgctgctgttgcagcggcgatacgcattgcgcgaccaggaacgacagatcgcgaccaaattgaagacgtgcgtctccccagcgcgaaaggtcttgaaacctcgcgccagcggcagtaaagtcagctttcggttaggagtgcagacttcaaagggcccgtacgcagttctgaacctgcgtgcgggctttctgccatcagtggcctgttagtgcttgggggtcttctcgtgctcctttccggccaagtgccccaccgtcgcgggcggctcaccgggctgcggttctgtgggtgactctgcaaactgcgccactaggtaggcggcaacatctgcggtcaggaaatatttgcctcgccggtgcggtgtgtccatgcagcggatgggcacatgccctcgctccatgcttttttccagcgcagcgacggtcttgaatcgcagcacttcggcgagcactggcgaatccatcaccggtccgtagcgcgacatgaggaacgattcgatgcgctgctgcgcaggtgcggcggcacagccgttctgcgtcggatccggcatcaaaacatcggtctggttcgaggtcatcccccatgatcgtgcagggccaagaaccagcgcaagtaggcctcgaaggcctgatttccttcgtgcagtagtactgcgcgaaaccaagaattccacagcagatcgtcaaaaaacaaggtgctttccaccttgctccgaggcccgtctgtgcaaatctcccccgtgcgcaacttcatccgaagcagagcgccgaagccgctcgaagaccaagttcgacggccttctgacatggcgaaatctggacgctctgattcatttttgaatttcttttcggcgtcaaagcaaagatcggtcatttttcttggtgttgtaattgcgcctaatacaagtgggtcacgccgcgtcggtccacgtcgatctcttgctgaccgttttcatccgtgcgcccctctcacagccctttgctattgccgcgcctagcggcgataggcgagcttgcaacccgcttcatcacggaggtcgccggcaagtcgaaactgaacgcgacacagtggctcatcgcgtttcatctcgacaaggacgcatccgaagctgagcgcatcccaatgagcccgaagcgactcgcatcgctcatgatgtgtccccaaacgcgcatcgtcacgcagctctcgacaatgcgacgcaaaggattgatcgagcctgtgaatctcaagcccacgcaaccacgccggccgcttcgcgaaggtcgcaggttctacgcgctcacatctgccgggctgaggttgatcagaaagagtgttgccaactcggctgcggccgatgaactctttgctacgctggttcattccaaggtaggcttggagatcaaggccttgcacaagaggctcgaggacgcatcggtgcgggactgtctcgattcgatttcagtcctggagatcgccctgagggaacagcggatcaagaaggctcgccggtaaatcctgccaggtcatggatgctgcggcacttcccggcgcagaacgcctgcggatcgcgccgggggcgggtgtggcacagccctcggttggaggcctcctgcgcctgcagtccaccggtttgttccccggtccagcactttattccccagtccacgacttaattccccgtaggcaacattgcttgtatgcaagacaaggcctgacttgcatgcatgcaaacccagacaagacagacagacagacaggagactccatgcctcgctttgccaaatccctcttcggccaggtcgtcatcgcgctggtgctcggcgtgttggccggcctcttcgtgccggaattcgccgtcaagctcaagccgctcggcgacggcttcatcaagctgatcaagatgatcatcccggtgctggtgttctgcgtggtggtgcacggcatcgcgggcgcgggcgacctgaagcgcgtgggccgggtcggcgtgaaggcgctgatctacttcgaggtgctgaccaccatcgcgctggcgatgggcctggtgctggccttcgtgttccagcctggcgtgggcatgaacgtggatccgggcaagctcgacgccaacgccatgagcgcctatgcctcgaacgccgacaagctcacgagcggcggcacggtcgagttcctgatgaagctgatccccaccacggtggtcaacgcctttgccaccggcgacgtgctgcaggtgctgctgttcgcggtgctgttcggctgcgcgctggcgctgctgggcgatcgcggcaagccggtgggcgtggtggtggacgcgctgtcgctggtgctgttcaagatcatgggcatcatcatcaagctggcgccgctcggcgtgctgggcgccattgccttcaccgtgggcaaatacggcatcggctcgctcaagcagctcggcatgctggtcgccctcttctacggcgcggtgctggtcttcgtgttcgtggtgctcgggctggtcatgcgcatgtcgggcttcagcctgtggaagctgctgcgctacctgcgcgaagagctggccatcgtgttcgccaccacctcgtcggacagcgtgctgccgcagatcatggccaagctgcgccgcatgggcatccgcgattcaaccgtgggcctggtgattcccaccggctactcgttcaacctcgacgcgttctcgatctacatcacgctggcggccgtgttcatcgcgcaggccaccaacacgccgatctcgatggccgacctgctgaccatcctggccattgcgctggtcacttccaagggcgcgcacggggtgccgggctcggccatcgtggtgctggcggccacgctgcacgccattccggcgattcccgccatcgggctggtgctggtgctttcggtcgactggttcatgggcatcgcccgcgcgctgggcaacctgatcggcaattgcgtggccactgtggccatcgccgcctgggaaggcgacatcgaccgcgagcgcgcgcatgcggtgctcaacggtaccgactcgcccgacgacgagccgctggccgagcccgagcttccggcggcgcccttgggcgcgggcatcggcggccactgaagccgatgagcaccgacgtcactcccacctccatcgcggagcgcgtggtcgaggccatcctggcgcaaaagctcgcacccggcgagcggcttggcgaacaggcgctggccgagaacttcgcggtcagccggaccatggtgcgcgaagcgctcatgcagctgcaggcgcgcggcttcgtcgaggtgcagtcgcgccgcggctggtacgtggtggagccctcggccgaagaagcgcgcgatgccttctcggcgcggcgcatcgtcgaggcgggcatcctggccgaaagcgaaggccgcccgctgcaaaaggtgatccgcaagctgcgcgaccacattgccgacgagcggcgcgccatcgaggccgccgacgccgccacccgcgccttcctgctggcggactttcatgtctgcctggccgagcagatggggcaccagttgctggtcgacgtgctgcgcgacctgacggcccgcaccacgctggccgccacgctctaccagtcgaagcacgaagccgggcaatcgtgtgccgagcatggcgccatcgtcgccgcgctggaggccggcgacacggccagggcgcgcacgctgatgatcgagcacatcggcaatgtcgaacgctcgctcgaggtggaaaccgcggccgagcccgacgctccggcccggctgcgcgccaccctggcgccggtggcgctgccgcgcgcccggcgctgaagccgccgcggcgggcagcgggcggcggcgcccggcccgccagcggggcgacaaggacaaggacaaggacaagtgcatgccggccgacacgggcgtgtgttccggctcggctacagtccgaatcacctatgaactcaccccaactccagcgcggcgtgttcctcgccctgctcgccgtcgtcaccgtggcctttctctgggtgctgatgccgttcttcggcgcagtgctgtggggcgttgcgctggcgatcctgttcacgccgctctacaagcggctgctcaagaaaatgcccggctggcacaacgccgcggcgctttccacgctgactatctgcctcttcatcgtgattcttccgctggccatggtcggggtgtcgctggtgcaggaaatcgtgcaggtcacgcagaacatccggtccgggcagatcaatttcgcggcctacttccagcagatcctcaatgccttgccgcaatggctggtgagcatcttcgaccgcttaaacctcggcgacatgcaggcctggcaggaccgcatttccgcgggcgccgcgcaaggcagccagctcatcgcaggccaggcgctcaccatcggccagaacactttcgacttcgtcatcagcttcttcgtgatgctgtacctgctgtatttcctggtgcgcgacggcacggcgctgtccaagatgatgcgcgaagcagtgccgctggccaagccgcacacgcactacctgctcaacaagttcacgaccgtgatccgcgccaccatcaagggcaacgtggcggtggccatcgcgcagggcgccatcggcggaattgcgttctggctgctgggcgtgcagggcgcgctgctgtgggccgtgctgatggcctttctctcgctgctgccggccgtgggcgcggcgctcatctggggcccggtggccatctactacctggccaccggccatttctggcagggcggcatcctgatcttcatcggtgtgttcgtgatcgggctggtcgataacgtccttcgcccggtgctggtgggcaaggacacgcagatgcccgactacatcgtgctgatgtcgaccatcgggggcatggcgatcttcggcatcaacggcttcgtggtcgggccggtgatcgcggcgctgttcatggcggcgtggagcctgttcgtggagtcgggccagctcgaaaccagcgccggcgacgacaagaacaacaacagctgaagcaagcccttgaaggccgcccaggcgaggcggccgcgggcaccgaggcgggtgcgccccgcgcctgccgcgtgcatttcgcgcgcgcgttttcgcattccgtcgcatggcgctggcgagcgcgtgccggctgcgagatcgtcgaggcctccaacttccagaagaggtctgcccgtgaactttccactgccccgaccggatgcgcgcgccctgtgcgccgccgcactcctctccccgctggccgcgctggcggccgacctgagcctgaacgtggccgacggcccggccgccgaagccacgctctacgtggcactgtacaacgacgccgccagctacgccgacagcaaggccgtggcctcgcagaccgcgccgatgctgggcggcaacgcccgcctcgtgttcacgggactggcgccggggcgctacgcgctgcgggcgttcgccgacgagaacggcaacggcaagctcgacgccaacctcatgggcatgccgaccgagcgctacggcttctcgaacgacgcgaagggcaaccgcgccgcgcccgccttcgaagccgcggcgatcagcgtcgaggccgacctgcagaccgtcattcacctgcgctgaggagacgccgccatggaacgacgcgaactcctgcgcctgctggcttcggccggcgccctgcccctcttggcaccgctgactccgctggcccgcgcggccggtacggccgacgactggcaagcccgtttcgaagccgccgccacgccctggaagaccggcttcgccacgcccccggacgacctgccgctgacccgcgccacggtgcgcgggcgcttccccgatgcggtggccggcacgctgtttcgcatcggcccggccggccacgacctgggcggcgagcgctaccaccactggttcgacggcgacggcatggtgcaccgcttcgtgatcgacggggccgacgtgcggcaccaggggcgctatgtcgccacgcccaagcgcgtggccgaggtgcgggccggccgccgcctgttcgaggccttcggcaccatgccgccgggcgtcgagccgccgacctcggccgacagcatcaacgtcgccaacaccagcgtgctaccgatgcagggcgaggtgctggcgctgtgggaaggcggctcggccacacgcgtcgacgcgcgcacgctggacacgctgggcgtgaagacctggcgcgccgacctcgcgggcatgccgttctcggcccatcccaaggtcgacccggacggcacggtgtggaattttggcgtgagttccggccagggcctgctggcgctgtacgagattgcgcccgaaggcacgctgcggcgcgcaaccgtggtgccggtggccgacatgccgatgatccatgacttcgccgtgaccgagcggcacatggtgttcctgatgccgccgctggtctacgacggcaagcgcaaggaggccggcgcgagctttctcgatgcccacgtctggcggccggaactcggcatgcgcgcgctggtagtcgacaagcagaactgggaacggcgccagatgctcgcgctgccggcgggcttcctgttccacgtcggcaatgcctgggaagaagacacgccgcgcggcacgctcgtccacatcgactacgtgcgatcggacaacgccgattcggtgttcaggaccaaccgcgaagtgatgcgcgcgcgccgcgtgaagagcacggacccgcggctgaccgtcgccacgctgaacctcggcaccggccaggccacgcagcaggcgctgccgctggaggccgagtttccgcgcatcgatccgcgccgcgtcggcctgcgccatcgccaggtggtgcatgccacacagacgcgcctcgacgtgccgggcttcggcgcgatcgcgcgaaccgatgtcgaaaccggccgcagccagcgcttcagctacggcacccgggccatggtggaagagcatgtcttcgtgccggacggcaccaggccgggctgggtgctgggcacggtgctcgatttcggccggcagaagacggtgctgtcgtgcttcgcggccgaccacctggcggcgggtccggtggcgcaggccacgctgccctacgcactgccgctgggcctgcacggcgccttcgtgccggcctgaagcgcatcgcgagcgcgttcaggccgcccaccacccttcggcaaaccgcccctgcaggaaggccacgaaacccgacaccttgcccggcaccagcttgggcgagggaaagacggcgtggatttcctgctcgggcagcttatggtcgccgagcacttcgaccaccttgcccgaagccagcgactcgctcgccacgtagcgcggcatgagcgcaatgcccaggccgtcgcgcgccgcggccaacacggcggaaaggttgttggagcgaaagcggcccgagacgggcaccgtcaccgcatcgcccttgggcgtgtgcatgcgccagaactcgtcgcccaccacgctgctgtagatgagcgccacgtgcgcgctcaggtcctgcgcgcgtttgggcgtgccgtgcttcttcaggtagccgggcgccgcgaccatggcccaggggttggtgccgagatagcgcgcgcccagcgatgaatcggccagcttgcccatgcggatggccacgtcgatgccctgcgcgatgaggtcgacatagcggtcctcgaagctcaggtcgagctgcacttgcggatgccggcgcatgtactcgagcgccagcggcaccaccacgcggcggccaaaggccaccgaggtgccgatgcgcagcagcccctgcgcctggttctggcgcagctgcacgatgctctcggcctcctcggcctcgcgcacgatgttcttgcacttctcgtagtagagcgcacccggctcggtgaggctcacgccgcgcgtgttgcggttgagcagccgcaccttcaggcgcgcctcggtggccgcgacctgcttggtcacggtgggctgcgtggtgtggaactcgagcgccgccttcgagaagctgccggtctcgaccacgcgcacgaacatttccattgccaacaatctgtccatggccggatcgtaatcacttattccaatccggaataggctttatggtccgcagccgtcttcttcgaatggcctccgcttcctacagtggacctcactcaaggagacagtcccatggcaaaaatgaaagcggtccaggccgccgtgctggtgatggaaaaagaaggcgtgacgcaggccttcggcgtgcccggtgccgccatcaacccgatgtattcggctctgcgccagcgcggcagcatcggccacatcctcgcgcgccacgtcgagggcgcctcgcacatggccgagggctacacgcgtgcggtggccggcaacatcggcgtgtgcatcggcacctcggggcccgcgggcaccgacatgatcacggggctctattcggcctgggccgattcgattcccatcctctgcatcacgggccaggcgccgcgcgcacggctctacaaggaagacttccaggcggtcgacatcgagtcgatctccaagccggtcaccaagtggtcggtcacggtgcgggaacccggccaggtgccgcaggtgttccagcaggctttccacctgatgcgctcgggccgcccgggcccggtgctgatcgaccttcccttcgacgtgcagatggccgagatcgaattcgacatcgacagctacgagccgctcaccccctacaagccggccgccacgcgggcccagatcgagaaggcgattgccatgctcaacgcggccgagcgcccgctgatcgtggccggcggcggcgtcatcaacgccgatgcgtccgacctgctcgtgcgctttgccgaagccaccggcgtgccggtgatccccacgctgatgggctggggttcgatccccgacgaccatccgctgatggccggcatgtgcggcctgcagaccagccaccgctacggcaacgcgacgatgctggcgagcgacttcgtgctcggcatcggcaaccgctgggccaaccggcacacgggctcggtggacgtctacaccaagggccgcaccttcgtgcacgtggacatcgagcccacgcagatcggccgcgtgttcacgcccgacttcggcatcgtgtcggacgccaaggtcgcgctcacgctcttcgtccagatcgccgaggagatgaaggccgcgggcaagctcaccgaccgccgcacctgggccaagtcgtgcatcgagcgcaagaagaccatgctgcgcaagaccaacttcgacagcgtgccgatgaagccgcagcgcgtgtaccagtgcatgaacaacaacttcagcaacgacacctgctacgtgagcaccatcgggctctcgcagatcgcggccgcgcagttcctgcacgtgtacaacccgcgccactggatcaactgcggccaggccggcccgctgggctggaccattccggccgcactgggcgtgcgggccgccgatccgtcgcgcaagatcgtcgcgctctcgggcgactacgacttccagttcatgatcgaagagctggccgtgggcgcgcagttcaagctgccgtacatccacatcgtggtcaacaactcctacctcgggctcatccgccaggcgcagcgcggtttcgagatggactattgcgtgcagctcgcgttcgacaacatcaatgcggggcccgacgccggcatcgagagcagctacggcgtggaccacctcaaggtggtggaaggcctgggctgcaaggcgatccgggtgaacaagcaggaagagattgcgccggccatccagcgcgccgaggcattgatggccgagttcagcgtgccggtggtgatcgaggtgatgctggagcgcgtgaccaacatcgcgatgggcaccgagatcgacaacatcaccgagttcgagcccctggccgagcacccggccgatgcgccgaccgcggtggcggccgagatgctggactgagcacggagacacgcaccatgcccaagtttgcagccaacctcacgatgctcttcaccgagctgccgttcatgcaacgcttcgaggccgccgccaaggccggtttcgaggcggtggaatacctgttcccctaccccttcgagaagaaggaactcgccgcggccctgcgcgccaacggcctgcagcaggtgctgcacaacctgccggccggcgactgggacaagggcgagcgcggcatcgcctgccatccggaccgcaccggcgagttccacgaaggcatcgcgatggccatcgactacgccaccgcgctgggctgcccgcagctcaactgcctggtcggcaaggtgccggccggcgtgggcaccgaggccgcgcacaagacggtggtcgagaacctgcgcctggccgccagtgaactcgaagcggccggcctgcggctcttgatcgagccgatcaacaccttcgacattccgggcttcttcctcacgcgtaccgaccaggcactggcgctgatcgacgaggtggggtcttccaacctgcgggtgcagtacgacatctatcacgcgcagcgcatggaaggcgagctcggcaacacgctgtcgaagaacctcgcgcgcatcggccacatccaactggccgacaaccccgggcgcggggaaccgggcacgggcgagatcaactacccgtggctcttcaggcacatcgattcgatcggctacgacggctggatcggctgcgaatacaagccgcgcagcgacaccgtcgacggtctgggttggcggcaggccctgacgcagcagaagtgaacgaagaagacaacagcatccaaggaaactgaagacatgtcgcaatcgcaaaaaatcggattcatcggcctcggcatcatgggcgcgcccatggcgggccacctgctcgacgcggggcaccagcttttcgtgaatacccagggcaacacgcccgagcccttcatctcgaaggcgaccatctgcgcctcggcggccgaggtggcacgccaggccgacatcatcttcatcatggtgccggacacgcccgacgtggaaaaggtgctgttcggcgagccgggcacgcagggcgtggccgaaggcctgaaggactcgcgcggcaagatcgtggtcgactgcagctccatcgatccgattgccaccaagggttttgccaagcgcatcatcgcgctcggctgcggctacatcgacgcgccggtctcgggcggcgaagtgggcgccaaggccgcgagcctcaccatcatgtgcggcggcgacgaaggaaccttcggccaggtgcggccgctgctcgagaggatgggcaagaatgtcacgctggtcggcaacgtgggcgacggccaggtctgcaaggtggccaaccagatcatcgtggcgctgaacatcgcggcggtgggcgaggcgctgctgttcgcctccaaggcgggcgccgatccggccaaggtgcgccaggcgctgatgggcggtttcgcgagttcgcgcatcctcgaggtgcacggcgagcgcatgatcaagcgcaccttcgcgccgggcttccgcatctcgctgcaccagaaggacctgaacctggcgctgcagagcgcccgggcgctgggcgtggccctgccgcagacggccggcgcggcgcagctcatgaacgcctgcgcggcgctgggccatggccagcaggaccattccgcgctggtgcgcgcgctcgaagcgctcgcccagcacaccgtcgcgccagactgagcctccggctcaggtctttgccgcctccagggactctttgaggttgcgtcggcgccacgcccaggtcttcacggcctgcggcaggatgccgaggcacgaggcgtagtaggtcaccttgaagccccagaagcgcgggccgatgggcgtgttgcggaacaggtcgccggccaggatggacaagagcgcctcctgcatgcgccagatgttgcgcggcgccatgaacagccggcggatggccggcgaggtgatgcggtagatgaaccacgagaacatcttcggtccgtgcttcatcaccttctcgtagtggcggaaggcgcgctcggcctccttcgcctcgcccttgagccagtggtcggccgccgtggccgcctcgaagccgctgttcatcgccaggtacacgcccgacgaaaacatcgggtcgacgaaggcataggcgtcgcccaccatcatgaagcggtcgccgcggcagaacttgctgtcgtaggcgtagttgccggtggaggtggcgccttccatcagcgtggcgttcttcaggcgttcggccagcttgggcgcgagcgcaatggtttccatcaagaactcttcgagcgagcccttgcggcgcttgaagtaggccggcgaggccaccgcgccgacgctcacggtgccgtccttcagcgggatgtaccagaaccagccgtggtcgaaccagaacagcgtgatgttgccctcgaagcggccgggcctgcgctcggcattggcaaagtggccatagagcgccgcgctcgcatgcttgcggttgcgctgcttggcatcgaactggttcgacagcagcgtgtcgcgcccgctcgcgtcgatcacgaagcgcgggcgccagctggtttcggtgccgtcgtcggccttcaccttcaccagcgggcggttgtgggggctgcccttgccggcgtccatgtcgacgccggtgacgcgctgtccctcgaaagtgcgcgcgccgcgcttgccggcatggcggaacagcagttcgtcgaattccgagcggcgcacgtgcacggcgtacggaaagctcttgtccatcgcctcggcgaagtgaaagtggctgctgtggtcgtgccagggcgagacaaactccgcaccgtgcttgcgcaggccgatggcctcgacctcggtgcggacgcccagccggtcgaacagcggcatgttcatgggcaagagcgactcgccgatgtgaaagcgcgggtgctgcgccttctcgatcagcaccacgtcgtgccccttgtccgccagcagcgcggccacggtggagcccgaaggcccgccgccgatgaccacgacgtcggggtcggtggtggtgaaagctccgggtgtcatgcgctacccctccgttgtctttgtgtgtttgggttgacgatggccggcccgctggctgcggagccttgcattgccttgtttaaccttggttcaccttggttaacactttcggagtttagcgaaccggcgtggcgttccatccaagctatggattcaggcgctttcggcattccccctctctgagcaggccccgcttttgcggtagcctcattgcccgtcagaaacaaggagacttttcatggctgcacctctctcgcccgcagaagaagctcttcgcgaagcagcgcgcgaataccaccgctcgcccgtcaagggcaagatctcgatcacgccgaccaagcccttgctgaaccagcgcgacctgtcgctggcctattcgccgggcgtggcctacccctgcctggacatcgcggccgatccgtcgctggccgccgacttcaccgcccgcggcaacctggtgggcgtggtcaccaacggcacggcggtgctgggcctgggcaacatcggcccgctggccgccaagccggtgatggaaggcaagggctgcctgttcaagaaatttgccggcatcgacgtgttcgacatcgaactggccgaaaacgaccccgacaagctggtcgacatcatcgcggcgctggagcccacgctgggcggcatcaacctcgaggacatcaaggcgcccgagtgcttctacatcgagaagaagctgcgcgagcgcatgaacatcccggtgttccacgacgaccagcacggcacggccatcatctcggccgcggcgctcatcaacggcctggaactggtcggcaagaagatcgatgaggtgaaagtcgccgtctcgggcgccggcgcggccgccattgcctgcctggacgtgatggtgggcctgggcgtcaagcccgccaacatctacgcctgcgactccaagggcctgatctacatgggccgcgcgggcggcttcgacgaatccaaggcgcgctacgcccagaaagacaccggcgcccgcaccctggccgacgtggtcaaggacgccgatgtgttcctgggctgctccgcgcccggcgtgatgagcgccgacatggtgaaaaccatggccggccagccgatcatcctggcgctggccaaccccgagcctgaaatccgccccgagctcgccaaggccgtgcggcccgactgcatcattgccaccggccgttcggactacccgaaccaggtcaacaacgtgctgtgcttcccgtacatcttccgcggggcgctcgactgcggcgccagcaagatcacggaagaaatgaagctggcctgcgtgcgcgagatcgccgagctcaccaaggccgacatcagcgaagaggtggccacggcctatgcgggccaggagctgtccttcgggcccgactacatcattcccaagcccttcgattcgcggctcatcctgcgcatcgcgccggccgtggccaaggccgccgccgcctccggcgtggccgcacggcccatcgaggacatggatgcctaccgccagcacctgacgcgcttcgtctaccagaccagcatgttcatgcggccggtgttcggcgccgccaagatcgccgcctccaagcgcgtggcctacgccgagggcgaggacgagcgcgtgctgcgcgccgcgcaatgggccatcgacgagggcctggcccagcccatcctggtgggacgccccgccgtgatcgaggcacgcatccagaaggcggggctgcacatccgcgcgggcaccgacttcgagatcgtcaaccccgaggacgatccgcgctttcgcatctactgggagagcttccacaagatcatgggccgccgcggcgtgacgccggaggccgccaagaccatggtgcgccgctccaacaccaccatcgcggcgctgatgatgcacctgggcgatgccgacgccatgatctgcggcctggtcgggcgcttcgacgtgcacctggagcacatccgcaacctcatcggcctgaagcgcggcgcgccgggctttgccacgctgaacgcgctcacgctcgaaaagcgcacggtcttcatcaccgacaccaacgtgaacgaagacccgagcgccgagctgctggcgagcattgcgctgatggcggccgaagaggtgcgccgcttcggcctgccgccgaaggtggcttttctctcgcactcgaactacggcacctcgagccgcggctcggcgcgcaagatgcggatggcgcgcgacctgttcgcgcagatggcgcccgacatcgaatgcgacggcgaaatgcacggcgatgcggcgctgtcggaagaagtgcgccgcaccgcgctgcccgaaagcaccctcacgggcgaggccaacctgctggtgtgcccgaacctcgactcggcccacatcctctacaacgtgctgaagatgaccggtgccaacggcatcacggtcggccccatcctgctgggcgccgcgggctcggcgcacgtgctcacgccgtcgtcgacggtgcggcgcgtggtcaacatgacggcgctggctgtggcaaatgcgaccacggcgctgaagtaggcgctccccgctttcttctcttcgcccgaacgccccgctgcgcaacgcagcggggcgtttttcattgcgggccgatcaggtgcacgccgtgcctcgatgcggcgcccgcacgcgccagaagggcgcgccgggagcgccgcagccgccgctgaagccgttttccgcctgtccatcattttttgggctggcatgcaatctgctaataccctgagcagatattttaaatatcttattaatatatttacagaagcaacgaccccctttgggctctccatccaccctctccgattccggaagcaacccatgacccatccccgctggcaaggcatcttccccgccatcaccaccaagttccacgccgacgaaagcatcgatgccgagggcaccgcgcgccacatcgacttccagatccgcaacggcatccacggcctggtgacctgcggctcgctgggcgaggcgagcacgctgacgctggaggaaaagctccaggtggcccagatcgcgctggaagcggccgacggccgcatcccggtgctggcgaatgtgtcggaaaccagcacccgcgaagcgctgcgctatgtggacggggccaacaagctgggggtggcgggcttcatggtgatgccctcggtgatctacgtggccgatgcgcgcgaggctatgctgaatgtgcgcaccatcgcccatgcggcccagaagccggtcatggtctacaacaacccggtggcctaccgggtggacctgaagcccgagcacatgctggagctggcggactgcgaatggatcgcggcgatcaaggagagcacgggcgacatccgccgcatcacggacctgcgcaacacggtggggacccgctaccagctgttcctgggggtggacgacctggcgtacgaagggctggcgctgggcgcggatggcctgttggccggggtgggctgcgcgttcccgcgggaaaccgtggcgctgtacgacctgatgaaggcgggccagttcgccgaggcgctggcgctgtaccagtggatgacgccgatgctgcacctggatgtatcgaacaagctggtgcagaacctgaagctgatcgacgtgctggtgggcgtgggcagcgagcacatgcgccgcccgcggctgccgctggtgggcgaggagcgcgcggccgtgcaggcgatcgtgaagaaggcgctggccacgcggcctgtgcagtaccagtcggttgcctgaaggcgcgattctcttctcaccatggaagaacacaccttggaacgcgggggcttctcccgccgcgtgctcgacgcgtcggacttcgtccttggctgcgagcgccgccttctctcgggcctgatgggcctgctcatcgtgctggtgctgctgaacgtggtcacgcgctacggcggcgtgccgctctactgggtcgacgaggcctcggtgtactgcgtggtgtggctcaccttcatcggcgcctctgcgatgacacggctgcggctcgactttgcggtgacgctgctcaccgacaagctgggcgaaaaagccgcgcgcatcgccaaggccggcgcctccggcggcgtgctgctgctgggccttgcgctgctggcgatgtgctggctctacatggacccggtgggcatcgtgcgctggggcttcgatgccaaggaatacgccgccgagtcattcaactttctctataccgagcgcacgcagacgctgaactggccgacctgggccatccagctcatcctgccgattttttcggccacgctcagcctgcatgcgctggccaatctcgtcgaagacctgggcctgcagccccggcgcacgcacaccgagttccacgtgaccaacgcagacgcggtgaactgacatgctgacttccgcattctttctattgatcatgctggtgggcgtgccgatcggcgcctgcctgtgccttgcgggcatcgtctacatcctcgagtcgggcgacacggtgctgttccagtcgtttccggtgcagatgttcggcggcgtcgacagctacagcctcatcgcgattccgctgtttatcctgatcggcgaagtcatgaacggaggcggcatcacgaagcggctggtcgacctcgcgctggccttcatcggctcggtgaagggcggcctcgcctacgtgaacatcctggccaacatgctggtgtcgtcgatcatcggatcggccaccgcgcaggtggcgatcatgagccagatcatggtgcccgagatggagaagcagggctacgacaagaccttcgcggccggcatcacggtgtacggcggcatgctggggccgatcattccgccctcggtgatgttcgtggtgtacagcgtgctggcgcaggtggcggtgggcgacatgctcattgccggcatcattccgggcgtgattctcacggtgctgttcttcatcgtgatcgcgtgcatggggttcatctacgactacccgcgcaccgcgaagcggaccatcaggcagcggctctacacgatgctcacgacctgccccacgctgctgattcccatcgtcatcgtcggctcgattctgggcggctttgccaaccccaccgaagccgccgccgtgggcgcggtggccgcggtgctggtgggccgctacgtcaccaaggaattccgcttcgggatgattccgcagatcctgctgaagtcggcgatctactcggccgtggtgctgttcctggtggcggccgccgcggtgttctcgtggctcctgatctacggcaaggtgccgcaggccacggccgcatggatccagaccgtggcgaaggacccgatcgcattcctgctgctggtgaacctgatcctgctggtgatcggaacggtgatcgacggcattccggggctgatcatgacggtgcccatcctgctgcccattgccaccgagatctacggcatcgacccgcgccacttcggcgtggtggtggtgatcaacctcgtgctggggctgatgacgccgcccgtgggcctgagcttcttcgtggcttccgccgtgaccggcgccaagcccggaaagatgttcatcgtcaccttgccgttcttcctgatctgctgcgcggcgctggtgctgctgtcgctgtacccgagcctgtcgctcgcgctcatcaagtaagtccccgcctctcgtccttccccttcactcaaccggagcctcgcatgtccctttcccgccgcaaattcgtcgtccaggccgccgccggaaccgccgccgcgtcgtccgccctcttcaccaccgtgtcgcgcgcagcggccgccaaggaattccggctcggcctcatcacgccggccggccactcgtggaaccgcgccgcactgggctttggcgaggcgctgaagaaggcgaccgacggccgcctgagcgccaccgtgttccattcgggtcagctgggcaacgagtcggccatgatgcagcagctgcagtccggcgctctggacatgggctggatccaggcggccgaactcggctcgcgcgtgtccagcgtggcggccatcaacgcgccgtatctcgtgcgctcgaccaccaacgtggcctcgctggtccgcacacccgccgcgctgaagctgctcgacgtgctgccgcgcgaaaccggcaccatcgggctgggctggggcatcacgggcatgcgcgtggtgtttgcgaccaagcccatctcgacgcccaccgacctcaagggcatgaagctgcgcatcaacccgacgccggtgtaccgcgacttctaccagctgctgggcgccgcacccacgccgattccgacccccggcgttttcgacgccatgtccaacggccaggtcgacgggctcgaggcggacatcgagttctcgtggaaccagcgcttcgaccgcgtggccaagacgatgctgccgatgaacgcgctgttcatgcccttcgcgccgctggtgtcgggccgcatctggcagacgctcgacgccaaggacaagtcgctcgtcaccgacctggtgaagcagtcactcgacgcgcagatcagggacatcgtgaccaccgaactcggcttggtcgacaagttcaaggccagcggcatcaccatcaagagcgacgccggctacaaccctgcgccgatcattgcggaattcgacaagatctggctgcccaaggcgccgcagatcgccgaactgcgaaagatcggcgcggcgctctgagccagggtcccccgggggccggcatgcgcgcttgcgccccatgctggttcaagccccgggccggttccggctgaaatccgcaagaactcccaaggagggtgcgccattgccccggttgcgcaccgcgacagttccgcggaagggttcgcaccaatcgcgtgcgggcaccgtttttgcttgaatgctgaagcattcacctctacggatcccgcatgaacaagcgccaacttctccagtccttcctcgccgcctcggccctcagcttcggcctttccccggcctttgcccagaccacgacgccgatcaagttccagctcgactggcgcttcgaaggaccggccgcgctgttcctgcaccccgccgccaagggctacttcaaggccgcgggcctcgacgtcaccatcgacgcgggcaatggctcgggcggcacggtcacgcgcgtggcctcgggcgcctacgacatgggctttgccgacctggcggcgctgatggaattccacgccaacaaccccgacagcccgaacaagccggtcgcggtgatgatggtctacaacaacacgccggcctcggtcatggcgctcaagaagagcggcatcgccaagccggccgacctggccggcaaaaagctcggcgccccggtgttcgacgcgggccgccgcgcgttcccgatcttcgccaaggccaacaacatcggcgccgtcaactggaccgccatggacccgacgctgcgcgaaaccatgctgatccgcggcgacatcgacgcgatcaccggcttcaccttcacctcgctcctgaacctggaggcgcgcggcgccaaggcggccgacatcgtcgtgctgccctaccccgactacggcgtgaagctctacggcaacgtgatcatcgcgtcgcccaagctcatcaaggagaaccccgaggcggtgaagaaattcctctcggcctttgccaagggcgcgaaggaagtcatcgccaacccggcggtggccatcgaatcggtgaaggcgcgcgacggcatcatcgacagcaagctcgaaacccgccgcctgcagctggccatcgacaccgtgatcaacagcccagacgcgcgcagcgaaggcttcggtgcggtgaacgcgggccgcatgtcgctgatggcctcgcaggtatcggacgcgttcaacaccaagacgcgcgtgagccccgacgccgtgtggaccgctgcgctgctgccgccggcggccgaactcaacggcgtgctgcgcaagtgatggcggacgcatcgagcgcggacgctgctcctttcgtcgatttccaggacgtctggctcgcctacaacgaagagctgctgcgcgccaaccacttcgcggtcgaggccatcgacctgaaggtcaagcgcggcgagttcattgccatcgtcggtccctcgggctgcggcaagtcgaccttcatgaagctcaccacgggcctcaagatgccttctatgggcaagatccgcatcgacggccagcccgtgaccgggccgctcaagatctcgggcatggccttccaggcgccttcgctgctgccgtggcgcaccacggtcgacaacgtgctgctgcctcttgaaatcgtcgagccctaccgctcgaacttcaaggccaaacgcaaggaatacgtcgagcgcgcgcgcaagctgctgcagaaagtcggcctcgcgggctacgaagacaagtttccgtggcagctctcgggcggcatgcagcagcgcgcaagcatttgccgcgcgctcatccacgaacccaagatgctgctgctcgacgagcccttcggcgcgctcgacgccttcacgcgcgaggaactctggtgcatcctgcgcgacctctggaccgagcagcagttcaacgtgatcctggtgacgcacgacctgcgcgaatcggtgttcctggccgacacggtgtacgtgatgagcaagagcccgggccgcttcgtggtcaagcgcgagattgagctgccgcgtccgcgcgagctggaactgacctacaccaaggagttcaccgacatcgtgctggagctgcgcggtcacatcggcgccatccgcaacacgggcatcagcgcggcgcaaaccgccgctgccgccgtgtctcactgaaggcgcgccatgaagaacaccaagcaactcgaacgctggtcgccctggctgctgctcatcgcagtcatcctgctgtggcaggtgatctgcgcgggcttcggcgtgtcggacttcatctttccgagcccgctgcgcatctggaaccagttctgggagttcaaggaaatcatcgcaggccatgcgtggcgcaccttctgggtcacgatggcgggcttcggcctcgcgatcgtggtgggcgtactgctgggcttcgtgatcggcagttcgcgcatcgcgtatgcggcgatctatccgctgatgactgcgttcaatgcactgcccaaggcggccttcgtgcccatcctcgtggtgtggttcggcatcggcgtgggcccggcgattctcacggccttcctgatcagcttcttcccgatcatggtcaacatcgcgaccggccttgccaccctggagcccgagctggaagacgtgctgcgcgtgctcggcgccaagcgctgggacgtgctcatgaagatcggcctgccgcgctccatgccctacttcttcggctcgctgaaggtcgcgatcacgctggcgttcgtcggcaccacggtgagcgagatgaccgctgccaacgaaggcatcggctacctgctgatctcggccggttcggccatgcagatgggcctggccttcgcgggcctgatggtggtcggcgccatggccatgctgatgtacgaactcttcagcgtgatcgaaaagcacacgaccggctgggcgcaccgcggctcgcaaaaccagtgatgcgctgcgaatgacacgcgaccagatcatccgcgcgctgcggcgcgccgacgaggtcgcccgccgcgccatggcaatgggccggcaccccttcggcgccgtgctcgttgcgcccgacggcgaaaccatactcgccgagcagggaaacatcgacacggtgaatcacgccgaagccacgctggcgcgccatgccgcgcagaactggccggccgactacctgtggcaatgcacgctggtcacgactttcgagccttgcgcgatgtgtgcgggaaccagctactgggcccacatcggccgcatcgtctacggcgccgaggaaagcgcgctgctcgcgctcacgggcgaccaccccgagaaccccacgctcagcctgccctgccgcgaggtgttcgcgcgcgggcagaagaagatcgaagtgatcggccctgtagccgaagtggcggaagaaatgatcgccacgcaccgcggcttctgggaagcgcgttagataacgctaggccagcagcagcgtggcctcgtcgcgccagtaggccacggccgccagccagccttcccacacgcagccgttgcagccgcgcccgcagcaggtggtgggctcgggcggcggcacgcgcaaggcaaggcctcgggcccggagaagcgactggacgctctcgatcagcgcctgggcgctggcgagatcggtcggagaagcaaggtcttgttcagaaagaagcatggcaggcacctgccgattgtcggcgcttcagcaggcctgtcgggatcaagccctggccggtgccgatgcggcaaccgcggcgaaagcctccagggcaagatcgacctcatgctcgccgatgtggcgatgggtgacgcagcgcaatcgatgcctgctccacggacggaccaagacgcccaggctcttgagcgcggcctcccattgaacggcatcgagccccgtggccttcacgtcgacctgcacgatattggtctggggcgtattggcggtgaggcctggaatccgggctgtcccgccggcgagccggcttgcgttggcgtggtcctgtgcaagccgttccgccatggtggtaacggccaccagccctgccgccgcggcaatgcccacttgccgctggctgcccccgagcaatttcctgagccaccgggcacgttcgatggtttcggcaggccccgcgagcacggcgcccatgggcgcactcaggcctttggacaggcagagcgaaacggtgtcggcgaaagcggcaatacgttccgccggcacgtccagggccacggccgcattcatcagccgcgcaccgtcgaggtggacggcggcccccgcttgcctggacgcctcgaacacggcctgcatgtgcgcaagcggcagcaccgcgccgccggcgttgttgtgggaagtctccaggcacaccacgccggttcgcagcttgttgcggcccggcgcgagggcctcctggagcagctccaggtccatggcgccatcgacgcccgcaatgtcctggtagaacgccccggtcagcgccgcggcgccccgctcggccacgtagatgtgcgatgcggcttcggcaagcacgagttcctggcgttggacttgcgcgaggatggccaggaggttggccatcgtggcgcttggcgcatacagcgcggcttcctttccgagcatggccgcggccgttgcctccagctcttgcgcggtcgggtcgccgtcgagtccgtcgtcgcccagcggtgccgaggccatgcgctcgtacatctgcggcgtgggccgcgtcaccgtgtcgctgcgaaggtccaccggcggttgttccgccccgtccgccatcgttgttgcggcctgcgtcattcggcggtcgctccggtggccttcacgagcgctgcccacttttttctctcgctgttcaggaacgcatcgaaactttcgggcgtgccggtacgcacatagatgccgcgcgccgccaggttggcccggacttccgccgtgtcgagcacgcgattgatttccttgttcatggtccgcacgatgtgcgccggcgtcttcgcaggcaccacgacgccgtagagggtgtagtactcgaatcccttgaagccgctctcgacgaaggtgggaacatcgggcagcgacacgtcccgggtgcccgaggtcaccgcgagcgcccgcagcttgccgctcttgatcagcggcagtgccgaaaccagcgacgagacgtagaagtcgacctgtccccccagcatgtccgccatggcggggccgccgcccttgtagggcacgtgcaaaagatctgcgcccacggtaacgcgcaggttctcggacaccaggtgcccgacggttccattgccggacgaggcataggcgagcggcttcttcttcgagcccgccagcaacgaggccaggttgtcgaacgggctgtcggcccgcacgaccagcaccgacacgccagtgcccaccagcgctaccggcgcgagatccttgaccggatcgaagctgagcttcttgtagagaaactgattgaccgtcaggttgctggtttctcccagtacggcggtgtagccgtcgggcggcgatttcgcgccgaaatccaggccgatgttgttgcccgcgcctggcttcgtatcgacgacgacctgccatccggcctgctcgccgagcttggccgcaagcaggcggcagacggcatcggtgccgccgcccggcgggctcggcgagaccaggtggatggtgcgctcgggtacccacgcatcggccgcgtgcgcctgccacgcggcgagcgcgagccccagcatgcatgccagccacctggcgcgtgcgaaagagtggtgtcgggtgtcgttcatggtgagggtgtcggtcgtgcaggttaaaggatcgggacgaagccggagcagaagccatcgatcctaggcgcgccatagaatgagtaaagcgatatgtacaaatatcaactgtgaggttttctcatgaatctcgcgatgctcgtcacattgaaaaccatcctcgaacaaggcagcttcaccgcggcggccggcgtggtgggctgcagtccgagcgcggtgagcctgcaggtcaagcaactggagcagtatttcggcaagccgctgttcgatcgctccacccgcgtggtggtacccacggcctttgcccgcgaggtggtggacgccgtgggcgatttttcccacaggctccagatgctgcgcttccgtccggtcgtggaagtggcgggccgcatcaaggtgggtgtgatcaccagcatgcagagcgacgtgctgccgcaggcactccatgcgcttcgccagcggcatccgtcgctggagatcgtggtgccgccgctgaacgacagcggcgagctgatttcagaactgaaggcggcgcggctcgaccttgcattgcttgtccggccggaatccggcggttcgcgccggctcgtctggcgcgagttgcaccgccagccctatgtgctgctggcgccgccgaatgcctccggcaagacggccacgcaactgctggaggcctatgactggatcggctacgacctgtctcttgcgggaggccgcgtggccgcgcgctacgtgcgcagccagatccctaatgcacgctgcgccatggaactgcgctcgatggacgcgatcgtggcgatggtcgcccagggcctgggggtttccgtcgttccccaacccaggcggccgctgatcgaggcctatgcggtgcgagaggtgagcctcggaagccgcgccccggtccgcaagctctccctggtctggcgcagctcggacgccggcaaccgcaatgtcgaggctgtggctgaagctttcactgcggcctttggcatgcggccgcatcggtgaggcgcgttcgcgcagcaggcttgcgccttaccagaagatccagagcgcaaggccgccgaagatcgaccacttcacgaggtagtaggcccgcttgtcccaggccttgaggcgcttgccgatgacgcggatctggtagatgtacttgaacgcgcggttgatgccgcccgtcttgtcgccggcctcgttgggcgaactggcggcggcgagcaggttcttggcgaaccagcggttcacggcgctggcccagcggtacttcagcgggcgctcgatgtcgcagaacaggatcacgcggtcgtggtcggtcgtgttctcggcatagtggatgtaggtctcgtcgaacaccacggcctcgccgtcgcgccagtgatagcgctggccgtccacgtcgatgtagcagccctcgacgcccggcgtccacaggcccaggtggtagcgcagcgaaccggcgaacgggtcgcggtggcgcacgaggcggctgcccggcggcagctcggcgaacatggccgccttgatggtgccgatgcccttgagcagctcggtggtgcgcgggcacagcacggccgccgagggatgcgcctcgtcgtaccacttcaggtagaagcgcttccagccgctcttgaagaaggagttgaagcccacgtcgttgaactggctcgaggccttgatgctgccgccgttgcgcatggcgagcgcctcttcgcggatgacctgccagttttcctcgagcacgcgcatctcgggaaactgcgcgggcgacaggtacggcgtgctcggcaccttcgagaagatgtacatgaaggcgttcaacggcgccaggaaggtcgagtgatcagacagctgcctgaagaaacgatgccggacctggccgcgaaaatgaacgtagagcgcgctgagcgcgaagatagcaagaatgacccacttcattgttgaaagtgtcctgtagacggcgccggggctaaccgggtagtgtaaatcgtcgccccaaattggacctgaccacgccttttggccgtgccccgacggaggtttcaggttgcgccgcatgggccggggcgggtcgcccgccgtgtcagcgcagcagcttgatcagcgccgcgatctcctcgccgccgagccccgccgcatcggcgcgcttgaaaaggcccgcggcgaaagccgggaactcggtgttgatgcccgcctcctgcgccgtctgcaggatgcgttgcgtcgcctcgaccgagatgcgcatcgggctctgcgagaccgcgaagtcgccggactggatcacggcgccctcgtgctgaaggaacgcggcgaaggtcggcatgatcccggccacgatgcggccgtactccgcgacggcgaatccttcgtgctcggcaatgcgcgcgccatgcatgaacccgagcaacgtgccgtagatagtggagagcgtcgccaggtccatggccgccgcggcgctggccttctcgcccaggtacacgataccgccggccagcgccctcaggagcggctctgcttcgcggaaaacggcttgcgcgcccgacacgaggatcggcgtgtcgggctgtcccatctggtccggcgcggcctggatcgcgccttcgaggtaggcggcgccatgccgatgggcccaggcctcggccgcgagtgcgtcacgggggctgccggtggtcagctggatcagcaggcggccgtccatcgccgccgcgacgccgtccaatgcaaagatcgtatcggcggcccggtagtcgtagacgcacatcaccgccgtccgggcggcgcgcaccgcttcggctgcgctgcgcgccagcaccgcacccttcgcgagcagcgcatcggctttctccgccgtgcggttccacaccgtgaccttgtagccctggtcgagatagagccgcgcgatggcgatgcccatcgagcccaggcccagaacggaaacttccttgttgctcatggcgattccaatgcagatcttgcaggttgtgacgaggcctgcatcgtaggaattgcacttgccaatggtcaagtacctaccataaagtgtggtacttaccaaaacgcatgtattggaacggcggatgaaggcaaaaaagccctacaactgcggcatagggcccgcattcgaagtgatcggcgggaagtggaaggcggtgatcctgtgggagctgcacgcgcagccgcaccgcttcggcgagctgaaacggcttttgcccgacatcagcgagaagatgctgatccagcagctgcgcgagctggaggccgacggcatcgtcaaccgcgaggcgttccacgaagtgccgccgcgagtcgtttactcggagacgaaactgggcgcaacgctcaatgcagcgctcgggccgctggccgattggggcgaccgctacgccaggcgcgtggaaaccgcgcgcaagcaggtcgaggcatcgaagtagcggtgcaaacagaaagaaccgaatgtcgttgctgaaaatcccggcggccgccctgttggccgcctcgctctctctttctcttggccttgcacacgcccagatggcgtgcacaccgtcgtccgtctacgcaggtccgccgatgcgctcggttcccgaggtcgtctggaagaaggacttccggcgccccatcgacggcgaactgcctcccgacctgcaggctgcattcagcggcgctctggacaagatgctcgcccatgttcccgccgcgagcgccgcgatcgccattcctggcgaaggctcctggtccgccacgcgcggactggcgcgcaaggagccgcccacgcgggccgtcgcggaccagcccttccaggtggggagcacgacgaagaccttcgtggccgcgatggtgcttcagctcgtcgaagagaaacgattgaagctggaggacaccatcgagacctggtttcccgatgcacccaacgcgcggctcatcaccatcgagcagttgctgcggcataccaacggactggtgagcttcaacgcattgccgtcgctggggacgaaataccgcccgccggccgacgtcatcgcactcggcacagaccagccgccgcagttctgccccggaacgaactggagctacaccaacaccggctacgcgatgctgggcacgatcatcgagaaggtggaacgcatgccgctggccgacgtgctggccaggcgcctgctgcggcccctgtcgctcacgcacaccgcgatgcgccagcccggtgtcgaactgccggtggctaccggccacgcgagcggccgggcggtcgatgtgcaggaccagtacgccacgccctacgcggccggcgcactggcatcgaccgcagacgacctcgtgcgcttctggcatgcattgctcggaggccaggtgctgcccgacgatgcggtgcaccgcatgttcacccgcatgcccgcgatgctcggcccctacaccgggggcaattcgtcctacggcatgggcgtgcagttctacgacgtgcccgatggtccgggcctgatgctcggacacagcggcggcatcgatggcttcaccactgtggttgcctacgtgccggcggacgatctgtacgtggccgtgtcgttcaacgagaagaacgtgcccgctgaagccggactgtgggcgctggttcgcgccctgcgcgcctaccgcaccttgcgctgaagccggcgccgtttcaggcgttcaggcccagcccgtctcgatctcggtcttcacctcggtcatgagccggtgcaccgggcatttgcccgccacgcgcagcagttcatcgcgctgtgcctcggtcaattcgccggttacgcgcaggctcgacttcaggcggtagacgcccttgcgttcctcgctgtcgtcgcggtcgacgaccacctcgatgtcttccaccggcatgcccttgcggcgggcgtagagcagcacggtgagcgccttgcaggcggccagcgaggcatcgtacaggtcgtggggctccgggccagcgtcgctgccgccgcctgccggcgaggcgtcgatggcgatttcatggttgcggatcttgaggatgtgacgcgtacccgtgatgccgtcgcgccggaccgtgatgctcatgccgatgtccttgtggggtgttgaatgcggcgccatcgtagcccgcaagccactcgctcagcggtccaccgcgagcatcagcgtttccttgatctcctccatcaccacgtagctgtgcgattcggccgccacgggcagcttcttgaggatgtcgcccaagaggtgccggtactcgctcatgccgcgcaggcgcgccttcacgagatagtcgaagctgcccgacaccaggtggcactcgagcacctcgggcatgtgcagcagctccttgcgcaccttgtcgaacacgtcgcccgacttggccgacagcttgatttccacgaacaccagaagcgtcttgcccagcgcctcgggcgacacgtgcgcgtggtagccgctgatgacgccttcgcgctccatgcgcttcacgcgctcggcgcaaggcgatgccgacaggccgatgcgctccgcgagttcggtcattgaaatgcggccctggcgctgcagcaggtcgaggatcttgcggtcgatgcggtcgagttcgggcatttcacttcgcacggggcatgaaggcgattcttcgcagtggatttcactgcagaacaaataaaaacgatgaaatccactgcattgtgcactttagattccatccattcaccttcattcgcgtaaatacccatgaaagtcatcgttctcggcggcggcgtgatcggcaccacgacggcctactacctcgcgcgctccggcgccgacgtgacgctgctcgaccggcaggccggccccgcggaagaaaccagcttcggcaacgccgggcaggtgtcgccgggctactcgacgccatgggccgcgcccggtattccgctcaaggccatcaagtggatgttccagaagcacgcgccgctgtccatccggccagacggcacgctgttccagctgcgatggatggcggccatgctgcgcaactgctcgcccgagcgctacgcggtcaacaaggaacgcatgatgcgcgtggccgaatacagccgcggctgcctgcagcagctgcgcgcggaaaccggcctcgactacgagcatcgcaccggcggcacgctgcagctgttccgcacagaggcgcagctcgatgcggtgcagcgcgacatcgcggtgctcgaggaatgcggcgtaccctacgaactgctcgaccgcgatgcgcttgcgcgcgtcgaacccgcgctggccggcgcgcgcgaccggctcacgggcggcctgcgcctgccgaacgacgagaccggcgactgccacctgttcacccgcggcctcgcggacatcgcacgcggcatgggcgtggacttccgcttcggccaggcggtcgaaggcctggagatggcgggcgaccgcatcacgggcgtgcgcaccagcgccggcaagatcctcacggccgaccgctacgtgatggccttcggcagctattcgcgcgccgccatcgcatcgctgggcctcgacattccggtgtaccccgtcaaaggctactcgctcaccgtgccgctcgtcgacgaatcgctggcgccgcaatcgaccgtgctcgacgaaacctacaaggtggccgtcacgcgcttcgacaaccgcattcgcgtgggcggcatggccgaactcggcggcttcgacctgcggctgaacccgcaccgccgcgccacgctcgaaaaagtggtgagcgacctgttccccggcggcgacctgccgcgcgccaccttctggaccggcctgcgcccgatgacgcccgacagcacgcccatcgtcggcgccacgcgctatgcgaacctgttcctcaacaccggccacggcacgctgggctggaccatggcctgcggctcaggcaagctcatctccgacctcgtgaccggccagcgtccggaaatccgcaccgacggattggcgatggaccgctacgcgcagggctcgccgcgcgcagcgcgcccgaacccggcaacggcgcacgcttgatgcggcggccgctcaggcggcttttgcaatcggaatcgccccgctgttcatgccgcggtagacctccgcctcgccgtgcttcgcaagtagctgcatcaggtgcttgcggatcagcatgccgggccggtccgattccatcgaatactcgacaccccgccggcgcgtgtcgaccagcgcatcggggtcggtcgattcgaggatgtccttgtcctcgcgcgtcaccgcttcgtcgaagtcgatcagcatctgcgcggtgcagtcggcctcggtgtcgttgcggaacagccattggcacagctgcatgcggccgtcgtcgatgggcgtgaagcagttgatgatgatgtggcgcacgccgctcggatattcgatgtcgagccggcgcgagaacggcaggaagtaggcgttgcgcatgtggcgcgtggtgatcggttcggtcacgccgctgatggcgtgaaacttgggcggattgaccgcctcgatcaccgtctcggcgtagaagccgctctcgttttccaccagttcgtacttgctcggcttcgggctcgcggccacgccgaaggtggcgcggtgcacaaagctgaagtgcgaattgtcgaaagagttctcgagcgcgcgcatcgggctggtctgccactcttcataaaactggaagatggtgcggtagcccggatcgtcgaactccggaatggcgggaatgtcggcaatgggttcttcgagtgccacccacgcgtagccgtagcgcgccgtgcagcggtaggcggtggtgcggtactccggcgagatcttgcggtcggcctcgtactgcggaatgcggatcacctgcccgctgcggtcgtaggtccagccgtgatagccgcactggatggcgccctgcccgcaggcctggccttcggcatcgacgcaccagcctttcgaaagcttggcggtgcgatggcagcagcggtcgcgcaaggcggccggctggccggcggcgtcgatgaagagaacgatgtcttcgcccagcagcctgaaaggcttcgggccgttggcgagttcggtgagtggcatgacggcatgccagaacttgcggaagacgggttgttgggtgacgagcatgcgtggactccttctgttgcgcgtgggtacgaacgaacttgaaagagcaatttcctgccgctggggctgaacgcttctactctgcgccacttgccttgcaaattgcgcgcccgcattgtggcgcgggccggcccatcttccaagccctctccacgtcctgatcgcaatgcccgggcaaaagaccgtggcatgcagcttggcatgggtcgtgcatgaactcgcgcaagagtagaagcgttcagcagcgcacgcaccaccgttgtgcgctcgcccggaaattgctcttgaagtgcctccgccttgtgcgggggattcaagactcacaatgattccgaggctccacatgcaacgtcgactttttcttggcggcagcgccgccaccctgctccctctcgccgcccctgccgtgttcgcccaggggggaggcaagctgaccccgctcaagttcacgctcgacttccgcatcaacgggcagaccgcgccgttctttctggcgcaaagcaagggctactacagggacgaggggctcgacgtgaccatcgacaccggcgccggctcggtcgcgtcgatcacgcgcattgcgagcggcgtctaccagatgggcctgggcgacatcagctcgctggtggagttcaatgcgcagaaccccggcaccccgatggtccaggccgtgtaccagtactacaaccgcgcgcccttcgtgatcatcggccgcaaggaccgcggcgtgacgaacgatttcaagagcctggcgggcaagaaggtggcggccgcggccgtcgaatcgacccgccgcgcctggccgatggtggcgcgcaagcagggcatgcgcagcgacgccttccagtggcagaccaccgacttcagcgcgcgcgacaacgtgatggtgcgcggcgacgtggatgccgccacttactttcacgactccgcggtttcgctctttgcgcgcatgaagcccgaggagctgtcggtgctcaagtatgcggatgccggcgtcaacctgtatggcaacgccattctcgcgagcagcaacctgatcgcgcagaaccccaggctggttgcggcctttctgcgcgccaccaaccgcgccatcgtcgagacctttgccaaccccgcgcccagcattgcggccatgcgccagcgcgaacccatcctcgacgaaaagatggagcttgaacgctggggcgtcacggcgcaatatgtgggcgccgtcgacacgcgcagccacggtctgggcgacatcaagaagctcacgctcgagcagcaggtcgacgaggtcgtcgacgtattcggcctcaaggtcaagcccgcgtccgacgccatcttcaatacgtcgatgctgccattgcgcagcgaaagaaccctccccaagacatgattcaagacatgagtcccgctggcagccacaccgaactccccgaagaaaccacgctcgacgaacgcgacgagcgctacctgcgcaaggccatcgtctggtcgcatgcggcgcgccgccgcggcaaccggcccttcggatcggtcatcgtctcggccgacggtgaagtgctggccgaagcgggcaacagcaacgccgagaccggcgactgcaccgcgcacgcggaagtgaacgccctgcgcgcgctcgcggggcgcggcctcacgcgcgaggagctcgccggcgccaccatttatgcatcgggcgagccctgcgtgatgtgcgcgggcgccatcttctggtcgaacatcggccgcgtggtgtacggcatcgatgccgaacggctgcgcgtattccgcggcgagcggcaggaccagcgcgatgcggaactgtcgtgccgcgacgtgttccgcgcctctccgcatccgatcgaatgcatcgggcccgcattgttggacgaagccagcgccgcccaccacggagcgtggagtagctaggtccacaggaaagagagcgcgcgggggcgaatagactcgttggatgtcctggcacgcacgtctccatctcgattaccggcacgaaaccgggcgcagcgttgcgcgctttcggcacgacgggccgttgcgcattctgcaaagcctgtatccggagggcgatgcgatctgccacaacgtgctggtgcatccaccgggcggactggtgggcggcgacacgctggacatcgacatcgaggcggcggacggaagccacggcctcatcaccacgcccggcgcgtcgcgcttctaccgctccgaaggcgaactggcgctgcagcgcacgcgcatccggctcgccaggggcgcgcggctcgaatggctgccgctggaggccatctgctacagcggatgccaggccgagaatcggctcaccatcgaggccgaacccggtgccgagatgatcggctgggacgtgaccgccctcggcttgccgaatgccaaccagcccttcgagcgcggcacctatctgcagcacatcgaagtgcccggcgtctggctcgagcgcggccgcatcgatgcggcggaccaccggctgctgcaaagcccgctgggcttcggcgggcaccgctgcatcgcctcgctgttcttcgtggcgggcacgccgtccaccaaggcgcggcgcgaggcgctgcttgccctcgcacgcacggccatcgatgcgcatggcctgcaagagaacgcgggcgcaacgagcccacatgccgagatcgtcgtgctgcgcgtgctcgcgccggtggtcgagcccgcgatgcagctgctgcggcaggtgtggcaggcatggcgcgccgagctgtggcagctgcccgcgagttctccgcgcatctgggccacctgagcccttcgcaggttcaggccggcatgtcggtacgcggcaaccgcaggtgcttcttcaaggtttcgaacacctgccgcgtgaccgggttcaccacgtggctgcgcacgtacaggtagtaggccaggtcgggcaggcgcggcatgccgtcgcccgcgccgagcacgcgcaggcctgcgtcgagctgttccacgccgcgggcggtcacgcccaggcccgcgcgcaatgccgccttgatgccgatcaggctcgacgacgtgtagcgcggcgtccacgccacgcccgcggcatcaagcgcctcatggccgatgcggcgaaagatgctgggcccgtccgccatgatcagcggcaccggcttggccggatcgtgcacgtagcctgccgcgcagagccacacggtcggcgaattgcgcagcaccacgccatcgaactgaggatcggcgcggttcgagatgatcatgtcgacctcgccgctcttcaatgaggtcatgaggtaggggctgcggccgatgtggatgtcgagctgcagcagcggcgatgtgcgcgctatctcggacagcagcagcggcaacatggtctcggccacgtcgtgcggcgcgccgatgcgcaggttgccttcgagctcgccctgccggaggctgcgcagcgcctcgtcgttgagcgcgagcagatggtgggcataggtcaggagccgctcgccatgttcggtgagccgcttctgccggccctgccgggcgaacagcgggtggcctgcctgctcttcgagccgctgcatctgctgcgtgatggccgactgcgtgcgccccaggtgcacggccgccgccgcaaagctgtggtggctgacaaccgccacaaaagagcgcaacaagtcgagatcgagcgtgggcatacattaattttattgatgtatttcgtgcgccggctggattgtcgagtcacgcccgcgtcactaaagtgaatgcacaccaagacaagcatccccactggagaaacctgcatgagcaccctgtccgaccagcgccgcgaggcggttgccgcgtccatcgcccagatgaagaaagccattggcggcgctgaacccacccgcgaaaacctcgatgcggtgctcggcgcgctgcaaggcctggccgcgcgcaccgactattggggtgccaccgactttccggcgcccgaggccggcgagcatcaggcccgctacctgatcgccgaagacccggaccagagctatgcgctctacctcaacgtgatgcggccaggcaagaagatcgtgccgcacaaccacaccacctgggcctgcattgccgcggtggaaggcaccgaacacaaccgcgtgtacgagcgccgcgacgacggctcggtgccgggcgtcggcaagctcgatgaaaccgcgctcgtcgttgtggaaccgggcaagggcatcgcgctcatgcccgaagacatccactcggtcgagatccagggcgagcaggtcattcgccacctgcacatgtacggccgagcgctcgaaacactgaaccagcgcactgcgtacgacctcgcggcgggcacgtaccagacgatgggcatcggcgtgcagacgcgccgctaggcattcccttttccaattttccgatgcgggccgcgatgcggcgtcgcacggagctgctcgccctgccgcttccgcttcatcgatttttctcctgccccatgacgacttctcatatcgatccgaagaccctcaaatcctggttgcacgacggcggcgagatcgcgctgctcgacgtgcgcgagcacggccagtacggcgaggcgcatctgttctacggcattccgctgcccttcagccggctcgaactcgatgcaccgcgcctcgtgccgcgccgcggcgtacgggtggttgcgtatgacgatggcgattccgacgtggccgagcgcgccgcccggcgactcgcggtgctgggctacaccgacgtgcatgtgctgcaaggcggcacccgcgcctggaaggcctcggggcaggcgctctttgcgggtgtcaacctgccgtcgaagaccttcggcgagctggccgaagaggtctatcacacgccccgcgtcagtgccgatcaactggccggcatgctggcgcgcaacgaaaaagtggtggtgctcgacggccggcccgtgagcgagttccacaagatgaacatccccacggccacctgctgccccaacggcgaactcgcctaccgcgtgcgccggctggtgcccgacaccaccacgcccatcgtcatcaactgcgcgggccgcacgcgcagcatcatcggcgcgcagacgctcatcaacctcggcctgcccaacccggtctatgcactggagaacggcacgcagggctggtacctgaacgaccacacgctggagcacggcggcacgcgccgctacccggtggagagcggcagcgccgatcttcggcccgccgcgcaagccttggccgaacgcttcgacgtgcccacggtcagcgcgcagaccgtgcagcaatgggccggcgatacggaccgcaccctgtttctctgcgacgtgcgcacgcccgaagaattcgcggccggcagcctgccgggcgcacagcacacgcccggtggccagctgatgcaggccggagaccagtacgtcggcgtgcgcggcgcgcggctcgtgctgttcgacaacgacggcgtacgcgcgccgacgattgcgagctggctgcggcagatggggcacgacgcgagcgtgctcgaaggcgggcttgcgagcgggcttgctctttcgcctgcggccgttcccgcggcccccacgctggcgaccatcgatgcgcaagcactgtccgcccgcctggcccgaggcgacgtggcgctgatcgacctgcgcccgagcatgcagtttcgcgccggccatattccgcaggcacgctggtccattcgcccgcgcctcgccgacgatgtgaaaagcgaaacgcggcaactggtgctgctggccgacgacgccgcactcgcggcctgggccgcggcctccgagttcgccggccgctcgcccgccccgctgctgctcgaaggcggcatggccgcgtggcgcggtgccggactgccggtggaagccacgcccgagctgcccgccgatgcggagtgcatcgactacctgttcttcgtgcacgaccgccacgacggcaacaaggaagcggcgcgccgctacctggcctgggaaaccgggctggtcgcgcagctcgacgcacaggagcgggcggctttcaggctgcccgccgtgccgcacgcctgatccggtttcgcatcgttccttccactcgtttgccgttgtccgttcctattccaggagtcctgccatgtcgtctgccgatcgccttccgggccttgcccgtctctccgtcgtcgtcgccgcatggctggcggccatgaccctgcagcctgccgcggccgagccgctgcccgcgcgcaacggcttcccttcgcagacggtgaagttcgtctcgccctttccacccggtggcggcaacgacgccacggctcggctggtgaccacgcgcctgccggaaatcatgggccaggccgcggtggtggacaaccgcggcggcgcgggcggcaacatcggcgccaggtcggtggccgaggccaagcccgacggctacacggtgctcacctcgcaggtgtcgatcatggccgtgaacccgtcgctctactcggcgccgggcttcgatccgctgaagaacttcatgcccatcacgcaggtcaacgcggcgccgctcgcgctggtggtggaagccggttcgccctacaagacctttgccgatctcgccacgcgcgccaaggcgaaccccggcaaggtcacctatgccacgccgggcaatggcacgctctcgcacctggtcggcgtggtgctgcaaaaagacagcggcgtggacatgacccatgtgccctacaaaggcgccggccccgcgctcaccgacctgctcggcggccaggtcgacgtgctggtgacctccaccgcctcggtcgcgggcatggtgcaaagcggcaagctgcgcgtgctggccgtcaccagcccgcgccgcatcggcgtgttcgccaaggtacccacgctcgaggagctgggctacgccaatgcccgcttcgaagactggtacggcttcttcgcgcccgccggcacgccgcccgagcgcgtggcctatctgcacgaagccatcgtgcgcacgctgcgcctgcccgaagtgagcaagctcgtgaccgacggcggcagcgaggtggtggccaacacgcccgaagcctttgccgcgcagttgcgcctggacatcgatcgctggtcgcgcgtcgtcaagctttccggcgcgaaagccgattgacgcaccatagaggcctcgcgaacaacgccattcgttcaccaccatgcccgcttcttcgcacaccgatcccgccgcgcaggcgctggaaacgcgcctcgcccacaccggcaagcagtccctccacgccggcggcaagcccgtcaacccgccgctggtgcgcgcgagcaccgtggtgttcgacagcgtggccgccatgcgcgatgcccgcgcacggcgcggcgacgagcgggttttcagctacggcgcacgcggcacgcccaccaccttcgcgctcgaagatgcggtgagcgaactcgaaggcggctatcgcacgcgcctctttcccaccggcctcgcggccatcggcatggtgctgctgtcgtacctgaagcccggcgaccacgtgctgatgtcggacagcgtgtacgagccggcgcgcaacctcgtgcattcctttctcgacccctacggcatccgctgcaccttctttgccgcggacggcagcggcgtggaggaacgcttcgagccgaacacgcggctcgtgtatgccgaatgcccgggctcgctggtgtacgagatgtgcgacctgccccgcctggccgagctggcccatgcacgcggcgcgctcctggccgcggacaacacatggggctcgggcgttcaataccggccgcttgcgctgggcgccgacatctcgctgatggccgccaccaaatacctctcgggccattccgacgtgatgatgggcacggtcgccaccacgcgcgaggcctggcagccgctcaacgagcgctgcgacgccttcggcatgacggtgagccctgacgacgcatggctggtgctgcgcggcatccgtaccctgtcagcccggctgcagatgcacgagcggcatgcgctagcagtggcaggctggctcgaagcgcgacctgaagtggcggccgtgttctgccccgcgctgccgcagcaccccggccacgaactctggcagcgcgattgccgcggcaccaacgggctggtctcgttcgagctgcaaccgggcatcggaaacgccgcggtcgaacggatggtcgatgccctctcgctgttcggccggggttcatcgtggggcggctacgaaagcctcgtggcctgggccaacatgcgcgcggcgcgcagcgtgaccgactggaccgcgcgcggcgccgtggtgcggctgcacgtgggcctcgaagcgccttcggacctgctggccgacctggcgcgcgggtttgccgccttgagcgcaggctgagcggtcttccttgccggctcaggcggccaccggctcgaccggttctggctcgggctccggaagaatcgccgtcagcgcaaagtcgaccaggtgaagccaggtcgattcgagtcccatgatgctgtggtgatcggagccgggaacggtctgcacgctgatgggcgtcggccaggccgcgatgagcttttgcgagcgctcgggcagcaccacgtcgtcgcgctcggccagcagcacctgtgtttttgcggccacctccttgcagtgcatgagcgaatcgaaccggtgccgcagcagcagcgacagcggaaccagcggaaagcgccgctttgccacttccagcatcgagtcgtagggcgtgaccagttgcaggctggagaaatgctgctgcgccaccagctggatggccacgcccgttcccaggctgcgcccgaccacgtgcaggcgtaccttgggaaaagccttgcgcaagtggctggcaaactggatcgcgtccgccaccgaggcgatctcggaaggatggccctgcgaatcggccacgccccgatagttgattgccgcgaatccgaagccatcgggcagccagtgcagcgcctgcgctgtggcgcgtacgtcctcgccgcggcccgcgaaatagatgaacaggtcttgcagcgagtcttcgccctgcgggtgatagacgtagccgcggaccatgccgcccggcaccgtgtgcgagtaggtggaaaagtggtcggacagatgaacgaccggatgctttctgacgttgaacaggatgtgcccctggcgtgcggccaggatggtccagtacgccgcgatgctgccaatggcggcggccgaaaccgagagtgcgatgcgagagactttgcgggacaaggtgagctccggaaaaaagtgcgatgccagggccgcggcttactgcttgcagctgccgccgacggtcaccgtgccgtccttgcattccgtcaggatgcgttcgttcgcaggtgctggcgcggggcgcgccaaggcgccgtcggctgcgggagcgccttcgcgctgatagacgatctttttgctgccaagatcgcagctgcccaccacctggccattggcctgtgcgttggcatcgatggtggtgacgctgaaacgcgtcacacccgacgcggcgatcttcgattcgatctgggcgcgcagggcttcgcagttttcagcgccgtgggcggcgccggcaaaagcaagcgccatggaaatcgaccagagtttcattgatgagagtcggcctcatgccgaggatttcgtgaaccaggagtctagccccgcattcaccgatgagacatcctcgcgcacactgaggtaaccgcacgtcacaggccccggaatgcaggcttactcgcaggcgtttctcccggccggagaatggcgcagcctgttcaggaaggtgagctgcaccctggccgtgtcgctgccctgcgacgcggcccgcagcatccacctgcgggcctcgcagcggtcggccttcaccgctgcgccgtatagcgtagggccggccagcagcaccatgccgagcatctcctgcgcctcggcgttttcctcgaacgccgcctgcctgagctgctcgagcatcgcgcggtagtcgcgcgcggtctgcgcttccagcgccagctgaaagcgctgctcggcatgcagcacgacgttcgcgtcgggcggctgcgccgcggaaagcgccgccccgaggcacagcgcgcccgcaagaaagatgcgccagcgcagcgaccagctcgtgatctgattcagttcggatgccatcgatgttctccaccattgagttgtgtgaagggcatcgtggcagcaagcgcttgcaaaaagaaactggaattcgcgcaggcaggctcagtgcgcgcctgagcctgcgcccgctttctgcgctcttccaaacgatcagaacttcgcggtcaaggccacctgcagttcgcgtccggggccgggcatgatgaggttgtcaacgctgccgtgtgccgacacgtagtactttcggcccgtgatgttcttcaagttcaccgagagttcgtatttcgcggtccggtagctcgcggccaggtcggccgtcacatacgaaggcagcgtcaccaggttgctgagcgaggcgtagcgcgccgccacgtagttgacgccaccgcccgcactcagcccatggcccaggtccttcatgagccacacgaaggccgaatgccgcggcgtgagcgacgccaccttgccctgcaccggcatggccgcaccaatgggcagctgcagcgaactcacggtcgccagcgacttgaccatgcggccgtccaggtaggcgtagcctgcgctgacgtcccagcggcccggcagcttgccggccagcgccagctccatgccgttggtgcgctgcgtgcccacgttgatctggcgcgccgggttggcaggatcggtgttcttgatgcccgagcgctccaggttgaacagcgccgccgtgaggttgagcgcgccgtccaggaagtcgagcttggcgccgatctccttgttgaccgtgatctcggggtcgttggccgcgttgttggccgacagtgcaaaggtctcggccgaaggctggaacgagcggctgtaagacacgtagtaagactgcgcttcggtcggctgccagaccacgcccgcgcgcgggctgaacttgcggtcggtgcgcgacatgggcgccagcgtgcgctcgaaggaggtttcctggtcgaacacgtcgtagcgcccgccgatcagcgccttccactgcggcgccagcgtgatctggttctgcgcgtagagcgccgtcgtcttgaaggtggagttgctcggaatcgcgctgttggccaggtagcttgcaagcggaatgggcggcggcgcggacaccgggttgaggatgctcacgcgctcgaagccggtgggggaagacaccgaatacaggcgcttgtcctgcttgcccaactcggcaccgaccagccattcctgcttgaagccgccgagctcgttgcgccaggtcaggtcggtctggttgaaccagccgctctcgtcgcgatcgacgaagccgcgcgtgcggcccacggtcatccgcaccgggtcggtggtgccgctgggcaaggtgttgaagcggtcgagcttgtagctgtagtagcgggtggtgttgcgaaggcggagcgtatcgctgaagcgatggttgagcgtggctgtgaaagactgcacgcgcgtggtcgtggtgtcgtcgcgcttcgcgaaggcggagccgtagtaggtgccgatgggcacgttgaccgggcggccgttgagcgccggaatgccgaagtccgtcagccgctggtcgtaggcgctggtgtactgcagcagcaggtcggtctgcgggctgaacttcatcgccagagagggggcgatgttgtagcggtcgatgaactgctggtcgcggtagctgcccgatttttcgcgcgccacgttaaggcgaaaggccatgttctcgccgatgggctggttcaggtcggctgtgagccgcttgaagtcgtgggtgcccaggccgagcgacacctcgccgaagggacgctcgaatatcggcttcttggtcacgcggttgaccaggccgcccgacgatccgcgaccgtagagcaccgcggccgggcccttgagcacttcgatgcgatcggtgtccgagaggtcgcgaaagtacagcgcgtcgtcgcgcacgccgtccacgaaccagtcggcaatggccgtgaatccgcggatgaccacctggtcgcgctggccgtcgccggcattgaacgaaacgccgggcgcattgcgcagcgcgtcttgcatcgacgtggcgccctggtcgcgcagcagctgcgccggcagtacgttgaccgcctgcggaatgtcgcgcagcggcgcactgcccttggtggccgtgctgctcaccgatggcgcatagccggtctcctgctcggaggtgacggtgatctccttgagcgtgtcggtgccctgcgcgtgggcggcagcgcccagaacggccagcacggcaagacacaggggacggtggcgcaggcgcggcgcacgcgatcgaacggacatgaaaaatttccttcagggcaacaacaagatcgcgaagcgacatgccgcctcgccatccatcggatggagaaacgcatgtgccctgcctcgaaaatctgggttgggtgccctcgccgacccatgctggcgcggtggccagggagtgcagcagaaggggatcgcatcgcgcgaaccggcggattctaaacgtcggttcgcccaggggcgccaggcagttgcccggcgcaacgctcagttggcgctcaggtccatcagcatgcgcgacagcagatagagccgcggcaccacgctctcgacctcggcgtattcgtccggcgtgtggatgccgccgcccacgatgccgaagccgtcgagcaccggcacgcccacacccgccaccaggctggcgtcggccgcgccgccgctgctctcgatggtgagcttcttgccaatctcgccgtagatgccctcggccatcgcgaccagcttgtccgacgcaggcgagcgcggcatcggcggcaggccgcggatgaggcgcacgcgcacctcggtgtcggggatcagcttgtcctgcgatatgcggaccaggtccttctcgacacggtcgagctcttcgggcgtggcggcgcgcacgtcgcccttggcgctggcgctcgcgggaatcacgttggtcgggccgttggccgcgagcaccgtgaagttcactgtggtcttctttgcggcatcccccgtctttgaaagctgcagcacctggtgcgccacttccatggcggcgttgcggcccgcgtcgggcgccacgcctgcatgcgaggccaggcccttcacttcgatgagggccgtggccgagcccttgcgctccaccacgaggccgtcggccgggcggcccggctccagattcagagccacgtcgtgctgcctggccacgcgctcgatgagcgcgctggtgccgaccgagcccacctcttcgttggtgtcgatgaggaaggtgatctgcccatagtccttgaagccgatcttctgcaggatcttcagcgcctgcagcccggcgaccacgccgcccttgttgtccatcaccccggggccgtaggcgcgcccgtccttgatgtagaacggcttggccgcggccgtgccttccttgaacacggtgtcgatgtgggcgaggatcaggatcttcttcttcccctggccggtgagcgtggcaaccacgttggtgccgggatgcggctccgccggaaaggtctcgatgcgcgcgccgagcttgcgcagctcttcaacggccatcgcgcgcaccttgtccaggccctcggtgttggccgagccggagtcgatgttgaccatgcgttccagcagcttgagcgcctcgtccttctgctgcgtcgccgcgtccagcgcaccctggtgcggcttctgggccatggcggtgccggacagcagtgcgcaggccagcaccatgccgtggcaggcggtgcgcaacggcgcgggtttcatgaagaaggggtggcgcttgtgaaaggtcataggtccgttctgttgtttgttcgttcgagcttgggcgaaagaaagcccgcttctcgcgggcgatcgcaggctatcacccgcgttccgcgcgggtcaagcgaacaagcaacaaacgggccctgcgccctagcagcagcggcccttgccggcgccgtagcgcgcctcgagccgctcccgaaaaaacgcctcgtagctcatcggcggctggtccgggtgggtggccgccatgtgggtcaggtaggcgtcgtagtcgggcatgccgaccatgagccgcagcgactgcttgagcgagcgggcgaagtagcgcccggcctccggcaatgcgagacccatggcttcgctcagcgcgccgccgacgcggcgagcggttcgaacggcgtctcttgcgcggtggggcggttggccgcgcgcgccgccaggcatgccttcacggcatacaccagcacgctcagcaccacgaacatgaagagcgcgcagagcgcagcgtcgagccggtcgttgaagacgatgcgcgacatggcctcgggcgtcttggccggcgccaccagcacgccgttggcaaggccttcggtgtacctggccgcatgcgagaggaagccgatcttcgggtcgggcgagaagatcttctgccagcccgcggtgagtgtgcaggccaagagccacgtggccggcgcaatggccacccacgcgtagcgctcgcgcttcatgcggaacagcaccaccacgccgagcagcagcgccaccgcggccagcatctggttggagatgccgaagagcggccacagcgtgttgatgccgcccagcggatcgaccacgccctggtagagaaagtagccccacgccgccacgcagagcgccgtggcaatcaggttggccggcagcgaatcggtgcgcttgagcgcgggcacgaagctgcccagcagatcttgcagcatgaagcggcccgcgcgggtgccggcgtccacggccgtgagaatgaagagcgcctcgaacaagatcgcgaagtggtaccagaaggccatcatggcctgcccgccgatcacctggtgaaggatgtgggccatgcccaccgcgagcgttggcgcaccgcccgcgcgtccgaggatggtgctttcgcccacgtccttggcggtttgcaccagcatctcgggcgtgaccacgaagccccagctcgagatggtttgcgcggcctgctgcgcggtgctgcccaccagcgcggccgggctgttcattgcaaagtagatgccgggctcgatgcacgaggccgccaccagcgccatcaccgccacgaacgattcggccagcatgccgccgtagccgatgaagcgcgcatggcgctcgttgtcgagcatcttgggcgtggtgcccgaggagatcagcgcatgaaaacccgacaccgcgccgcaggcaatggtgatgaacagaaacgggaacatgctgcccgcccacaccggcccgccgccttgcgcaaactgcgtgagcgcgggcatttgcagcgtgggcatgacgaacacgatgcccagggccagcgcgatgatggtgccgattttcaggaaggtcgacaggtagtcgcgcggggccagcagcagccacacaggcaggctggcggcgatgaagccgtagcccaccagcatccacgtgagcgccttgccgtcgaaggtgaagagcggcgcccacgcggggttctggctcacggcctggccgccgaagatggcgagcatgagcagcacgaagccgatcagcgacacctcgccgatgcggcccggtcgaatgaagcgcaggtacacgcccatgaagagcgccaccggaatggtggccgccaccgtgaaggtgccccacggcgattcggccagcgccttcaccacgatcagcgccagcaccgcgaggatgatgatcatgatcatgaaggtgccgaacagcgcgatcatgccgggcaccgtgcccatctcctgcttgacgaggtcgccaagcgagcggccgtcgcgccgcgtggagatgaagagaatgatgaagtcctgcacggcacctgcgaacacgacgcccgccagcacccacaagagccccggcaggtagcccatctgcgcggcgagcaccgggcccaccagcggaccggcaccggcaatggccgcgaagtggtggccgaacagcacgttcttgtcggtgggcacgtagtcgagcccgtcgttgtggcggtgcgccggcgtcttgcggttgccgtcgagcctcagcaccttctcggcgatgaagaggctgtagtagcggtaggcgatcaggtaggtgcagatcgcggcggtcaccacccagagggcgttgacgctttcaccacgcgtgagggcgacggtgcccagcgcgaatgcgccgaccacggccacaacgagccacaccaggtggcggcggatgctgtgcattgggaatgtctcctcggtattggaaccgggagtgttccccgccagcctcgaacccgcatccgtcggaccgcgtgggcgctatgcgtgggaattcttaatggaaaaccctagcgccggccatgcgcccgcggcgctcctcatgcaagcaatggcgtcaacggacggtcgacatcaccgttgcgcggcagcggggctggtcgcgcggggccagcaggttgcagttgtccagcgcacgctgctgcatgtcgctcagccgcggctgttcgccgggaggcggggcgtcccactggcgatagaccggcggcgggggtggctgctcggcccagcgctcgcggcgctcgtattcgcggcgctgctctctttcgtaggcgcgctgttcgcggcgctcgtagcgctcctcgcggtcgcgctggatgcgccacatgcaggtgttgaagtcgacgccggagcggccgctcgcgcagtagaggcggtcgtgctcgtaggtgtcgggatcgcgctgcgcaaaggccgggagcgcggtggcaaggcccaggatggccaggacgatgagtttcttcatagggacctctccgaggttcggtgatatcggcacagcatgccacaccggtcggaccgccccaaggcaggcatccctgtagaccgatgactacgctgaaccgttgagttggattgagtcgcgcttttcaagcgcttaaagccggcgcgcctgcatcggttggcgcgaccagtagatgccgtccagccggtcgagccgcacctccccgccggtcgatggcgcatgcacgaactgccctgcccccacgtagatgcccgcgtgcgtgggcgtggacgcgccgaagagcaccaaatctcccgaacggatgtccgacgcggacaccggccggccgaacgccgccatgcgcgccaccgtgcgcggcgtggcctggcccgcgctgttcttgtacacgtagccgatgagcccgctgcaatcgaacccgccttcgggcgtattgccgccatagcggtatggcgtgcccaccaggccgagggcatggatcgcgacgctgttcgattcctcggacgtgagcggcgaggtgccgtagccggccgacggcggaggtgcccgcgggctcgcgcaacccagtgccaggaggcaggcgccaatggaaagcagacggagcagcagcagtggcatgcggggacgtggcgcgggtactacgagtgcgtcgggcatgtgggattggctgtcttgtggacgtggccagactctaacgcgagcagcctatccggccaaggcaaggagccggcctgcagacggatatggcacgatcaaaacatgcccgagccctcacgccgaatcccgtaccgcacctggccaggtgcgctcgccgttctgctggccattgcaggctacgtgggcggcctcgttttctgggacaggcacacgcccggcaaccggccgttgcctgcgggcgaaatgatcgaggtcggccatgcgaggttcgttcccgccagcggatgggagatggacgtgtcccgctccaaggcaggccggtcgctgatgctgttcaagggcggccacaagtttctggtgaccaccggcccatgggcgggcgggccggacgggccgctggtgcggcagcaacggctcatggagcgcggccagcgcttgcgcatcgacggcgacccgtcggacttcgtcacgacctggggcttgcagggtaagacctttgcctactacggctcgaagcttgcaggccgcttctggcaggtggtcgaccttcagcgccggtcgctggtgcagatcgacttctatggcgccaccgacggcctgcccgaggcgatggccgaggcccggagcatgctggagtcgatggacctggaggcgccgctgtgaacctgaacgttcccgaacaacaggacaggggcgactggcccattggcaccgattcgttctttcagccacatcgcgcagccttttgggtattggcggcattgatcgtcaacggcctgttctacacggtcaacatgttctcgatgggattccgcgtggtccccatcaccgcgttgctcggcatcctggtgtgggccatctacacgctggtttttcttctcgtctttcgtgccttggacttgctcgaacagcatccgccggaggctttcgggctggcctttgcatggggcggcctgggcgccgtgtactttgccgcgcccgcgaacatcgccattcagagcttgtgcgccaagctggtgtcgccggacttcgtcgcggcctggggaccggccatcgcggggccgatcaccgaggagttcctgaagcttgctggcgtcgtgctgctggtgctggtggcgcgcaaccagttccagacttatctttcggtgctgatcgtcggtgccatgacggggctgggattccaggtggtcgagaacctcacgtacaccgtcaacgcgtcgatgcactttccgctcgagaaccaggtggtgccagtgctcatcaacctgctgacgcgcggccttttgagcgggctgtggagccacgcggcctacacgacgatcgcctccttcggcgtcgcatggtttctgctgcaccccgagcggccgatggcggtgaggatcgcctgcgccctgctgtgcttcgcactcgcgtgggccatgcacttcatctggaactcgccatggctcgaagacctcttcgatggcggctacggcgagatggcggtattgctcgtcatcaagggcattcccgcgatggccgcagcctggctcttctggcgcgaagccgcccgagagaacggcgcctaccttcatgcgcttgcagcctacttcgtgccggagcgcgagctgatccgtgacgacgaatggctccggctgggggcgcctctgttgcgctacagggttcgcaggcagatcggctggaccttcggcctgcgcgcgaggctgctgaagacgcaattgcagcgcgagcagctgcggctgatccgcaaggcaatgacctacggacgcggggcgcagacgctgcggcatgaagtggcgatacggcgcatacgggccgagctggatccgttgattgcgacgcagccctgaagccacaggcctcggaaaacgcaagacgcgagttctgctgcatggcctcctccgatgacccgatcaagccgacgccttcgcgccgcaagcgccggctcggcgtggctgctgctgcggtctgcgccgcgctcgccgcgggcgtgtgggccgtcgctaccggcacggtcgagattccggagcgcttcaatccgtgggcgccgctcgacgtcgcggcggcgccagactggctcaccggcttcaagctttcccgggcccgccgcgacccagcgcgctgccttgcggcgctggcacaaaccggcatgcagtacgacctgctgcccgaccgcgtcaccggccccggctgcggctttcagaacgccgtcaggctgcgctctgccggcgtgcgcctgggcaccgcgccttcgctcagctgccccatggcgctgtccttcttcatgtgggagaggcacgcattgcagcccgccgccatgcagcgcttcggccaaccggtggtggccatcgatcaccttggcagctatgcctgccgcaacgtgaaccgtggcgaaggggcagtgccgggcgcgtcacgcagccggcacgcgacagccgatgcgctggacgtgacagccctgacgctggccgatggccgacgcatcacggtgctgcaagcctggccccgcgacggcgccggcacaaaaagcacgaacgatccggaggtgctgcttctgctcgatgcgcaccgcggcgcctgtcgcttcttcaatggcgttctgggccccgactacaacgccgtgcacagcgaccactttcacctggagaccggcggctacgacatgtgccgctgagcatccaccagccgagtcataccgcgtttgcggcaataggcattcaggacgcagccggtcccttgcgcaaggtcggcaagccgacccccgcggcatcgaagccaccgtccacggcgagcacctggccgttgatgaagctggcctcgtcgctgcacaagaagcccaccgtgttggccatctcttccggcgtgccgtagcggccctgcgggatggtgtcgtagtagtcggagcggatcgccaccgtgtgaacgagcttggccatctcggtttccaccggccccggcgcgatcacgttcacgcgcacaccggcattgcccagctccaccgcatgctgcttggtcaggtggatgagcgccgccttgctggtgccataggcgacacgcagcgtgctcgcgcgcaggcccgagatggaagcgacgttgaccaccgcgccccgcccgcgctcgaccatcagcgcgccgaacgcctgcgtgcacaagaacgcaccgtcgaggttcgtgccgagcacggcgcgccactcttcgaacgaggtctgcaacactggcttgaacaccgccacccccgcgttgttgaccagcgcatcgacctgcccgaagcgcgcgaccacggccttcgcggcactgcccacctgcgcaggattcgatacgtcgcagtgcacgccaagcacacgttccggctcggccagatcggccaccgcctgatcgagcgtgacggcatcgatgtcgagcagcgcaacgttgtagccgtgcgccaggaaccagcggccaatggccaggccgatgccgcgcgcgccgccggtgacgacggcgacgcgggagggggtggggagatcggtcatggacgggagtttccgcgatggacggagtcagttgacgggcgatggaagccattcttccagagcgactacgaaaatgacaaacacaccgctcacccaccagcgaaccttagaagccaaagaccagcagcaagttgttcgcaggcatcgcatgccgctctcgcaaggcaaggcctctgcgacgcgcctctgccgccacgtcctccaggcggcgtatgccccaggcggaattgcgggcgcgcaagtcttcgtcgaacgccaggttgctcggcgccggtgggacttcttcttcgaagtaaggcccgtaggtgatcagcatcccgccaggaagcagatgccgcgcggccccttgcatcagcgcggcgcatgtggtccagggcgcgatgtgcagcatgttggcgcagtagatcgcgtcgaacttcttttcttcttcagcgaacgctgcaccctgcgttggccattgaggcgccatcacgtcgagcaggagcggcgcgcagagattgggcagtgcggcttctgcaacgcggcttgccagcgcggggatcatgcgtgcgtccgcgtcggtgggctgccagatccattggggcattgctgccgcgaaccaggcggcgtgctggcctgtgccggatgcgatctccagcgcggtgccacgctcaccgaggatgaggatcaatgcatcgaggatgggctgcttgttgcggtcggcggcggggctgtgcggaaggtcgggcatcggtattgggcttggatggttggtttggagggtatcagggccggacggcgaggcgcttgtctaggcgatatgtggtgtccatcacctctggacgacaaggtgtgccacgacagcaagcacaacaggcatgccttgaaacgcgaatgcgtaagcatcctcctacgtcgtccgaaagcaggaacccgtaaggtcatttaaaagcgtacggtcgggatacgttcacagttctcgcaatcgcgcggcagctcgaagtcgtttcacaggagcccgttgcaatgtccgtcccgcagtccctttcccattcgcacatcgatttcgtcggcaacgatttcgaagcgctggcctcccacatgcaccactgtgcacgtgcccacgggcgatggttctcgctgcgaagccacatgcaacgtgtgcgcgcgctcgctgcgggtcgcatcgtcacgatggcctgcgtggccgcggtgttgggcatcggcttgttcgctgtcacttgagcgtcgctgccgtcgtcgaccgcctccaagggctcagtcactacgcccggacccttctgctcggtccgcacgccccgatagcactcccgatccgcgccgaactcttcggcgcccaacgtttcgaacagcacggccacagcctggcccgtgcccaggtggtggaagacgagcaccaccgcgcacgcgaaggcgcgcccttctttccgcgggtcgacgaaaacctcgagtcgctacgcgccgccttcgactacatcgcgctgatctcgctgagcgggcgctatgtgtcgccggcggcggaatggctgctcgacaacttccacctcgtcgaggcgcagctccagcagatccatgacggcgtgccgcgcagctactacgcgcgcctgcccaagctcatcacgccgccgctggcggggctgccgcgcgtgtacggcattgcgtgggcctatgtggcgcacaccgacagcgtgctcaacaagacgctgttcaccgccttcctcaacgcgtaccaggacatcgacgagctcatgctcggcgaactgtgggcgctgcccaccaccttgcgcgtggtgctgctcgaaaacctgcgcctcgtggccgagcgcattgccgagaacaaggtcgcatgcgagatcgcgcacgctgcatgggacgcggcgccgcatctctcggtgcaagacctcgacgtgctgtaccgcgcactgcaaagccacggcctgcaggacagctacctcacccagctgtggcagcgcctgcccgtcgagcacggcgacgacatgcccgcgctggtgcgctggaccgagcagcactgccccaacggcccggcgctgatcggcgacgcgcagaacgcgcaggccgcggccaacctcacggtcggcaacatcatcacgaccctgcgcatgatcggccaggtcgagtggagcgacctgatcgagccggtgagccgctcgctgcgcgtgctgcgcgcactgccgagctttgcgaacgagagcgaactcacgcgccagcagatcacgcatgcgatggagcaggtggcgcgcagcaccgaacggcccgagcgcgacgtggcgcaggccgtggtcacgctggcatccagcgcgccggccgacgaagccggcgcggaaaccgaccgcgccgacggcaccgcgggctactacctcttcggccagggccggcccgcgctgatcgcgtcactgcaggccgacagcccgccgggccgttccgcccacgcagcaaacacgcggcccgcgcgcagccatcgcggctggcgcctgcccgtctacgtgagcgccgtcaccatcggcaccgcgctgctgctggcggccgtggtgcacggtctgccgcatcgcggcgactggaccaccgtcgcggcgttgctgcttcttgcatggccgctgtccgaagcgttgattgcgctggcgcagcgcatcatggcggaatcggtgcgcgtgcaggccctgccacgcctcgactttgcaaacggcattcccgagcggcaccgcgcgctcgtcgtcatgcccacgatgctgggttcgaccgcgaacaactcaaagctcgcgcaccggctcgaacttcactggctggccaaccgcgaggcgcacgcgcagttcgcgctgctgaccgactgggccgacgcctcgcaagcatcgatgcccgacgacgcgcccttgctggacgacgcccagcaacggatcgtcgcgctcaacgccaagtacccgccggcggaaggcgccgcgccgcgcttcctgctgctgcatcgtccgcgcagctggagcgagaccgagcagcgctggatgggctgggagcgcaagcgcggcaagctcgaaatgctgatgcgcctgctggccagcggcgacgccagcggctttcttccgctcgcaccgggccagcagctcacgcccggccgcacgccctatgtgctgacgctcgacagcgacacgggcctgccgcccggcgcgctgcgcgacctcgtgtccattgccgcgcatccgctgaatgcgcccgagatcgacatgccaagccgacgcgtggtcgcgggcttcggcatcctgcagccgcgtatcgtcacgccgttcccgatgcgcagcgagcgctccttcttccactgggtgttcgccgggcagtgcgggctcgacccgtacggcagcggcgcctccgacatctaccaagacgtgttcggcagcggctccttcaccggcaagggtttgctgaacgtgcgcgcggtgcatgccacgctgaacgaccgcctgcccgacagcgccgtgctgagccacgacctgctcgaaggcagcgtcgcgcgctgtgcgatggtcagcgacgtcgtgctggtggaagaccatccgcaccatgccggcgtggccgcctcgcgcgtgcaccgttgggtgcgcggcgactggcagctgctgccgctgatgtggcgcgcgcgccgcttcggcatcgacgcgctgggcctgtggaagatgagcgacaacctgcgtcgctcgctggtggtgccggcgtctttcgcgctgctggtgttggtgatcttcacgcaggccatgccgctcggctgggcactggctgccgtcggcgcggcgctcacgctcggcccgttgctgggtgcgctggccggcttggtgccgacgcggcgcgccatcgagctgcgccacttcttcgacgtgggcgcggtcgacctgctgcgcgccatggccagcgcggcctggcagttcgtgcagctggccgcgcagacgcggttgctgctcgacgcggccttcctcgccacctggcggctggtcgtcagccgcaggcacctgttgcaatggacgacagcagaccaggcgcaggcgcaatccagccaacgactgaagcccttcgtgcgcagcgcggccctcagcagcgcggtgtgcctggtgcttgccgtgctcgcaaactggagtgcctacccggtgcttggccccctgctcttcgtgctctggtccctggcgcccctcgcggcctggtggggcagccgcgtcgacgcgcacgcggaagacccgctcctgcccgcgcagcgcagctacctcgacaagctggcgcaggacacctggcgcttcttcgagcacgtggtgggcccggacgacaaccacctgccgcccgacaacctgcagctcgaaccgcaaccgaccatcgcgcaccgcacctcgccgaccaacatcggcatgtacctgctggccacctgctgcgcgcgcgagttcggctggatcgacacctccgccttgctggcgcgcctcaccgccacgctcgacaccgtcgaccgcatgcagaagcaccacggccacctgttcaactggtatgacactcaaacgctgaagccgctgccgcccgactatgtgtcgagcgtggacagcggcaatttcgcaggccacctcgtggccgtggcgcaggcctgccgcgccttcgcagcggaagaaaattgccagtaccacgaagcacccgcactggaagcattggcgcaacattgcgacgcactgcacgacggcatggatttcagcggcctctacgacgccaagcgccacctgttccacatcggcctgcgcgtcgaagagaacgtactcgacgcgagctactacgacctgctggcttccgagtcgcgcctcttgagcttcctggcgattgcgaagggcgacgtgccgcgccgccactggatggcgctgggccggccgttcctgctggtgagctcccagcccagcctcaagtcttggtcgggctcgatgttcgagtacctgatgccggcgctggtgatgaccgagcccaccgacggcctgctgcaggtggccaacgccgcggccatcgccgagcagcaggctttcggccgtgcgcagaacatgccgtggggcgtgtccgagtcggcctacttcgcgcaagaccattcgctggcgtatcaatactcgcccttcggcgtgccgcgcctggcactgcggcgcacgccgccgaccgaccgcgtggtggcgccttacgccagcctgatggccgcgccgttcgcgcccgaagcggccgtcatcaatctcgagttgctcgaatcgctcggcgcgcgcggcgagttcggttttcacgacgcaatcgacttcaccgcctcacgccagaccgagggccaggacttcaccgtggtgcgcaacttcatggcgcaccaccagggcatgtcgctggtggcgctgtgcaacgtgctgcgcgacgaagcaccgcgccgctggttcggcagtgccgcgctggtgcaggcgcacgagtcgctgctgcacgaacgcacgccgcgccagatcatcggcagcgccgacccgcgcacgccgcccgagcccagccaggccgagctggcgccgctgttccagccgcgcgtggtcgatccgatggggccgggcttccagcccacgcacctgctgtcgaacggccgctacacggtggcactgcgggccaacggcgcgggtgtgagccgctggcgctcgttcaacgtgacccgctggcgcgacgatccgctgcgcgacagctacggcaccttcttctacgtgcgagacgaaggccaggccgagctcacctcgctcaccgccctgcccgcgcccggcgccgactggcactaccgcacccgcttcctggccgaccaggtgcagttcgatgcggccggccccggcctgcaggtgcgcaccacggtgctgatcagccccgagaacgacaccgagctgcgcaacatcacgctgcacaattcgggcgatgaaacgcgcacgctcgaactcatctcgtacttcgagccggtgctgtcgaacccgaaggccgacgaggcccacccggccttcgccaacctgttcgtcgagtcgcgctgggagcccgcgtggcgcgcgctgctgctggcacgcaagccgcgcctgcatggcgatgcggtggtggccgccgtgcacttcgtggcctcggtcgatgccaacgtgctgtcgatcgactgcatgaccgaccggcgcgccttcatcggccgcaaccgcacgctggccacgcccgcgctcgatgcgcagccgaaggccatcaacggcacgccggtgaacggcctggaccccatcgcctgcctgcgcgtgcgcctgtcgattgcgccgggcaccaccgcgcgcctgagcttcgccaccgccgccgacgagagcatcgaggcgctgatgcccagcatcgaccgctacctgcagcccatgcacgtggagcgcgccacccgcatggccgccacgctggcgcaggtgcggctgcgcgacctgagcatcgcgcccgcacagaacctggcgctgcaggacctgacgaccatcctcacctacaccacgccgcgcgtgatgcgcgaccgcgggctgatcgacctgcgccagatctggcgcttcggcatctcgggcgacaagcccatcgtgctggtgtacatccactcgatggacggcatgggtctcatcaacacgctgctgcgcgcgcagccgtggtggggcttcggtggcgtggcctgcgacctggtggtgctcaacggcgaaccgaattcgtacctgatgccgctgcagcgcgagatcgaggcgctgcgctcgcgcgtcgcgcagcagacgcagaacagctttccgcgcaacgacacggccggcttctacctcttgcgcgaccaggacgtggtgccttcggaaaaggccgtgctgtccagcctggcgcgcgtggtgttcacggccgatggccgagcgctcgaagtgcaggtggcggcgttgcatgaggcacgcagcccgacgatcgccgacgacagcagcgcaccggtgcagcaccgcacgccgctgttgacgagacgggcgccgcagttgaccgccatagcgcccaccggtgacttcgacgccgagagcggcgagttccgcttcgaggtcggccccgaccgccgcacgccgcgcccgtggatcaacgtgatcgccaacgcggccttcggcttccaggtgtccgaatggggcgccggctacacctgggccggcaacagccgcatgcaccaggtcacgccgtggtcgaacgacccggtgcaagacccggccttcgagcactacctgctgcaggacgtggcctcgcgcgagatgctgccgctgacgccggccggcggtggcgacggcctcacccgccaccgtgtgcggcacggacaaggctacaccgtcttcgagtgccgccagggcgacctcgcgctcgaaaccaccttcttcgcggaccgcgacgaagccgtcaaactggtgcacgtgcgcgtgcgcaacgaaggcgccagccagcgccgcctgcgcgcgctcgcgatggtcgagtggcaactgggcgccgcacgcggcgaacggcgcaccgtgcattgctggaagcccgaagaccagccggccgtgttcggccagcagcgcgaatcgagcgcgggcttcggcggcagcgcggccttcctgctgctcgctggcctgcagggcgtaacgaccggggccacgcaatggacctgcgaccgcagcgagttcttcgccggccgcggcatcgtcgaagtgccggacacgctggcgcggcgcgccggcagcgggctcgatgcctgcgcggccctcggtggcgaattcgtcgtgggcgccggcgagacctcgagcttcagcttcgtgctgggccacgccggcacggccgacgcggcgctcgaccttgcgcgccgctggcggcggcgcgacgtgcccgaagcgctggcgcaggtgcgcggcttctggaacgacctgctgggccgcctgcaggtgcgcacgcccgacccgctgttcgatgcgctggtcaatcgctggctcgtgtaccagacgctggcgtgccggctctggtcgaaggccggcttctaccaggccggcggcgccttcggctttcgcgaccagttgcaggacgcgatggccttcgcgctcaccgacccggcgcgccttcgcgcccagatcttggtgaacgcggcgcgccagttccccgaaggcgacgtgcagcactggtggcacatgcccggtggtgccggcgtgcgcacgcatttctccgacgacctgctgtggctgccgtacgcgtcggcgcactacgtcgaggtgacgggcgatgcctcgctgctcgacgagatggtcggcttcatcgaaggccccggcatccccgaaggcgccgaagacgcctactacgcgccgcacaacagcggccgcatggccaccgtgttcgaccacggcgcgcgcgccatcgatcgcagcctgaagaccggcgtgcacggcctgccgctgatgggcaccggcgactggaacgacggcatgaaccgcgtcggccacgaaggccgcggcgaatcggtgtggctggcgtggttcctgtgcagcgtggtcgagcgcttcgcacccatcgcgcaagcgcgtggcgagcacgaacgcgccgcgcgctggaccgaggcacgcaccggctggatcgccgcactgcacgacgcgggttgggacggcgcctggttccgccgcgccttcttcgacaacggcgcgccgctgggctcgtcggtcaacggcgagtgccgcatcgacctgatcgcgcaggcctggtcggtgctctcgggcgcctcggacgcggcccacaccggcccggccatggccgccatccagaagcacctgcacgacgagccggccggcctgctgcggctgctggtgccgcctttttcccactcgatcaacgacccaggctacatccaggcctacccgccgggcgtgcgcgagaacggcggccagtactcgcacggtgccgtgtgggcgctgatggcgcaggcgctgcagggagaccatgaagcagcttggcaaagcttcgagggcctgagcccggcccaccgcgcacggcaccccgagcgcggcccggtctacgagctggagcccttcgtgatggcgggcgacgtctacggcgccgcgccgtatgtgggccgagggggctggagctggtacaccggctcggccgcgtggctgcaccgcgccgccgtcgagaccttgctgggcctgaacgtgaagggcaagcagctctcgttgaaaccgcgcgtgccggcgcactggccgggcttcgagatcgcgctacggctcgggacgcgcgagttcactctgcaatggggccacatggaaggcgccgccacgcccacgcatcacctggtggcgggtgaatgggttgattggcactcactgccgccgaattcgaccgtacgggttttggcgtagcgcaacctggctgcacgtcagcgggtcaggatgtgctcgctcacgtccagttctgctgcacccagctgcgcaccgccgcccactcggacgaggtctctatgtagttcagcgtcgcgctcaccaattcgcctacgttcttgtagtcgtccagaccgaacggctggctcagcggcacgttgccgcgcatgtagttgctgccgagcagttgctgggcctggatcgccgccaactccgcggtggcgtccatggtgaggttgagcagcgccgtggccggcaccgtgccatcgctgaacggccacagccaatgcgtgacgccccagtccagcggattggacacggagctgggcggcacgcccaccggattggcgccggtgcccagcgacagcatcacgatgtccgacgtggcggtggcgtagccctggtagatcgcttccacgatcgccgtcatcgaggggttgttggcgaaagtgccgccgtcggcaaagtagccgaagtcacccacctggtacggcgggaagtacgtcggcgcggccgaggtggccagcgcggcgtccaccatgctgatgtcacggtaggtgttgctctggccgttggagatggtgcacggcgcccaactgttgtcgctcgcatcccatagccgcgcggagttgacggccacgaagcggctcgccgacgacaacgcgccggtacccaccagcttctgggcgaccgcctgcaagccggtgttgacgtactggcatctgaagatgcccgggccgctgcccagcagttcttccgtcgactgcgccggcgcacggtcctgttgcttggcctctgcgcccagcaaccagccgttgggctcgaagatcgtggctccttcgttctggtagagattgacgatggcgtcgatgcccacattgctcaccaggcccagcgagatcaggccaccagtggaagtgccggcgaaaccgtctgcgttttggacgatgccgaagcttcggtccaggtcctggatcagcagcgccgtgatgacgccgcgaatgccgccgccgtcgcagcagagaatcttgaaagacatggctgtgctccttgcttgagtggatagatgagaaatgcgcgctcgtccccgacgtgacggggatgcccatcgccgcccacgccggaaaccgaacctgagcactgtggcgcctcttcatgcgccagtccatttcacttcattacaggccggttctggccggtgctacacgaccgtctgcaaaggtattggccgcagcgtggtgctgccctgcatactttctggagacaatggacccggtcgaaaccgagcatgaggggatcaagatgtcagccgacgactggtggaagtgcggaatcgtctatcaggtctacccgcgttcgttccaggacagcaacggcgatggcatcggagatctgggcggaatccgcgcccggctggatcatctggtctcgctcggcgtcgatgccgtctggatctcgccgatctatccctcgccgatggccgacttcgggtacgacatttccgatttttgcgacatcgatccgcgcttcggcacgctggacggcttcgatgcgctggtgcaggaggcccatgcgagagggctcaagctcatcctggacttcgtgcccaaccacacgtcggaccgtcatccgtggttcgtgcagagccgcagcgcacgcagcgatccgcgacgcgactggtacatctggcgcgacccggcgccggacggcgggccgcccaacaactggctcagcaatttcggcggcccggcctggtccttcgatccggccacgggccagtactacggccattcgttcctgaaggagcagcccgacctcaactggcgcaaccccgaagtgcgagccgcgatgtacgaggtgctgcgcttctggcttcggcgcggcgtcgacggattccgcgtcgacgtgctctctcaaatcatcaaggacgcgcagttccgcgacaacccgccgaatccgtacttcgccccgggccaggacccattttttcgctggttgatgctctacaacacggacctgccggaggtgcagccgatcgtggccgagatgcgccgcgtggtcgacgcgttcagcgacacacgctcatcgcgcgtgctgatcggcgagctctacctgccgctcccgcgcctggtcgcctactacggactcaacgccgaaggtgtgctcgaaggcgtgcaactgccgttcaactttcagctgattgcgaccgagtggcaggcggcgcgcatcgaccgctttgtgcgcgactacgaagccgccttgcccgccggcgcccagccgaattgggtgctgggcaaccacgacagatcccgcattgcgagccgcgtcgggccacagatggcgcggctcgcggccatgctgctgctcacactgcgcggcacgccgacgctctactacggcgacgagatcggtatgacggacgtccccattcccgccgatgaagtgcaggacccgttcgaaaagaacaagcctggcatgggcctgggtcgcgacccggagcgaacacccatgcagtggagtgccggagagcacgcgggcttcacgaccggtacgccgtggctgcgcctggcagccgactggcccatgaacaacgtggaagcgcaatcacgcgacgcggggtcgatgctggcgctctaccggcgcctcatcgcgttgcgccgcgcgcagcctgcgctgaaccgaggcaactatgaagcgcttgaaaccgagggcgaggtgctcgcctatgcgcgcaacggcgaaggacagcggctggtggtgctcctcaacttcggcgctaccccggcgccgatttcgccggcgttgatgccgcgccagccgatcgtgctggcatcgaccgatcctgctcgcgccgagttcatcgagggtcccctggtgctggcgcctcacgaaggcgtcgttatcggcaccgtgaacgacaagggtccgccgacacgatgagcaatcaagacttgccggtatggatctcgacgtagctgcgcgcatgccagcgcacgcgcacgggccactttgcgtcggcgatggtttccgaattcacgtccttgccgctgccgtagttgatctgccgatcgggtcttctgttgaggctgatcagcagcacgatgcggctgcccgccgcaagcctgcgagccgtcacgcgttcggtggtgaacgaaagcagctgacgctcgccggcccgaagaagccggcgacgcacgcgatggccggcgtagctggcgcgaaagtcgtagggatcgaacagcagttgatactcgccgctttccgtctgctcatacagcgagatgttgaagtccacgtcctgccgcgagggcgtgatgtcgaacatgccgtgcaggctgccaaagatctcggtgtcctccgggagcggatcactgacaaagctgatgctgttgcgcatcggcagttgcttcacacgcagcacgtccggccacgggatgcgcacgtcacgccgatcggcaagatcgaccgacagccgcgcgctgccaccgccttcagacggcgacggcaacaggcggtgcggttcgtcgcgctcgcgagtgtcgaggtaaaggcgcagcggggtgcgctgcggcgcgtccagcgtcggcacatggcgccactggtccgcgcccatcacctggtagttgatgcgatccaccagcagagaaggcttgttcgcgcccttcaggatgtggtcgatccattgcaagcgtagctcgggcaggtcgacgcgtgcgacggagtccagcgtgtggccgcgcagcgtagccgccgtaccgagccggatcgaggccgcgtcgtaggggccgagcagcagcgtcgtatcggcctctggccggttgcgaagatgctcgtgatggaagtagagcgcgccggcgtctgcgccgtagtagccggcaaagctgagcaccgggatgtcgattcgcgcaaactgctccgccgacggcaagaacttctgccagtagcgatcgtggctggggtgcgtcagccaggtgcggatcagcctgctgcgcttgccaatcaggacgcggtcgatgtcccagtaagggcgattgcctcgataccagcgcgcgtcgagtgcctgccacatcgtgtccgggtcggcgtcggcgtcgacaccggcccgcaggggctcggcattcgcgtgctcctgcgcccagcggaccatggcgttgcggaagatctgcccggccatcggaaagtcgatgcccggcgccatcggcgcgatcgtggcgatggccttgagtgccgccggtctcaagcgggcggcggcccaggcggcgtagccggagtagccgtcgccgagcatgcagacgcggccgtcgctccacgcctgccgggcaatccagtcgatgacggcggcggcgtcttcgccgtcgcggatgaacggccacacggcgcccttaccgtcgggcgtgcgtccgcgcacgtacgccgtgacgccgacatagcctttgacggcgctgcgctgggcgtcgtcctcggcgggatcgagcgtgaagcgcagcagcgtcggcagagcgtcagtcgtgcggccgggccgaaccaggctcgcgaagatgacacccccgcgcacgggaatcctgacgtcggcctccgccacgtagcgggcgcggttttccgccgcgaacaattcgggcagcagcgcaccgaagctgcgacgcgactggtacgaatgccaggttcgcacgagcgccagagcatcggcctccgggaggctgcccttcgcgcgccagagatcgaaagctcgacgcagcggctctctgtataccgccggcggaatttcgagccgcgccatgatggcctgggcttgcgcgttgtcgagcggcgacaccagttcccggaacgagcgcgcgtaggcttcggcgaagccgagtccccccgcttcgagcgtgcgcgcatgcgcatagatgccatcgaggatcgcacgctggaccaggtcgtcgaacggcttgcctttacggcggctgcgcagggacccgctgctgtcggaggctgcacggtaggcgccgctgacgatctgcagagcggtcaggttggccaggaagacatcggtgtccgcctcttggtacaccggcaagatgcgctgggccagatcccgcatcaactccgccgccgtggcatcgtcaggatcgcgagggggccggaagccgaaatccgctccccaagcccacgcgggcagcgcaagaatcacgcgcgtgagggcgcggcgcacacgactgacggtcgactcgcggtgtctcatggtcgctgctcctggggcacggcgtttggcgctttgaccagatgcaccacctgcgtgaacagccggtcgtgcgcttctccggccgagcctatgtggacgatgcccgtgtgcgtgagcttgcccagcaggtcgatgatgagttcgagcgtgtcgtcgtcgaacgcgccgaaggcttcgtccatcaccagccagggcggtgcctgcagcaccacgcgggcgaagcccaggcgcaactgctcgtccatgctgagctcgctctcccagcgacccgtcttgttcagcaagggctccaggcgctggaggcccacactcgccagtgcggccaccgtggcttctctcgggtagctcgacggttccattgggtacgacagcacttcggccagcgtgccgcggggaatgtagggcgtgccgcgcggcatgtagtggatcgtctccccggcgggccggcgcacgatgccggagccccagggccagaggcccgcgagcgcccgaaacagcaaagtcttctcggtgcccggcgtgccgaggatcaagacgcgctgaccccggtgcacgacgagacccggagcgtccagccgatcatggccgctccaggagcgaacctcgagcgcttcgatcgcgagcgccccggcttcgccctcctcataggcgatgcggctgccgcctgtttgtgcctccagatcggacgccagcatccggcgcaagtcggcaacgcgcagcagcgtggcgcgccagtcggcaatgatgctgaagttgtcgacgaaccagcgcagcgacgactgtgcctgcgtgaaggccgcggcggccatcatcaagccgccgaacgaaaccttccccgagaagtacaggggtgcggccaccagcgtcggcgcgatgatggtgacccagccgaagcccgcggtgacccaggtcaggttggtcagcccgagcaccacgcgcgacgtggcgtgcaagacgtcgcccaaatgcatggcaacgcggcgcttctcgtcggcctcgcccgcagccagtgagataccgtcgagatgctcgttgatgcgcgtcagcgagaagcgcaattcgccttcacgcgcgtagcgctctgcgttgcgcgagatcaggccgttgccgacccagtaggtgaccagggagccggcgaccgcataggcaatggccgcccacaacatgaagcccggcaacacatggtccttgccgtcgaagaagaggctgaagtccttggagatgacccacagcacgctcgcaaagctgccgaacagcatcgctgcctgcaacagacccacgccaagggcgaccgacagatcgcacagcttcagcgcgtcgtcgtgcatgcgctgatccggatgggcccccatcgggccgctggcctggagccagaacgcccggcgcggctgcagccacagccccacgagatcattgaccacggcctcacgcagcttcagctgcaaggtttcgcccagccacctctgcgcgacgttcaagaccagcagcgcgcccgcaatgaccgcgaagacgcctacctgcacgacgaattcgctcaggtcgcgacgcgagatcgcatcgtagaacggcttgttccagctattgagctcgatctgcccatacgccgtgagcgcaacgaccacgacgatcgcgcccatcagcgcgacaagcgttttcgcgaccggggacacgcgcaaggcgccgagcaactcgctgacctgacgaaagaaaccggtcttcgcagccggctcggcacggttctctggccttgcgctcatcgcccccgctgcgcctgacaagcggcggccgcgaggcggcgcgccgagacacacgaaatgaacgcggcgtggctccaggccagttgcttggccgaggtctgcgcgccgctgcgctggtcgaactgttccgacagatcaccaccggccggtgtgtatgcgcgtacggtggcgaggtaggcgtcaccgcgccccatccactggttccaatggcgtgcatcgccgcccatcgccgccgcggcgcggaaacagaactcggcggcgccgagcgtcgagaagtagtacgcgccgcccgagtagtacacgtcgccggcgtaccggcccatcgccgcgccacggcctgcgccgcggccatggttgattggataggctgcatcgaacagcgcgtcgaggcgctccagcgtggcctgcatacgcggatcggccggtccatgcacggcctcggtgccgaggctgccgaggctgtggatcgccgacaggatcaccgcgatgtccagcgccttcggactgggcaggccgtccgccagcacgcgtgaacggtagtagccgcgcgtcgagtcgcgatcgcctgactgctcgcctcgctcgtctcgttcatccacccagtagtcgtcgagcaggcgccgcacggccccagactcctcccggcagcgctgcgcctgcgccgtgtcgcccaagccctccagccatgccgcgccttcggccagcgcggcccctgcgacgcgcagtgtgtagtagtggtggccgagttcttcctcccagatgtcgtatgacggctcgcgccagtgacgcagcgtgaagtcgatgtcgaaacggatcagcggcgtgatctccgccagcagggccgcgtcgaggtgcccgccggccacccagcgcagcagcgccaacgcgcgcaatggaggcccgtcgtgctggggtcgcgcccattggaggacatcgagcgtgccgtcggggttcaccctcgtttcggcgacgacggcatcgccgtggacgctcgcgaggtcatggtcctcgcgcagatactgcaggagttcgggggccgcgcgcgctctgcggtcctgctccgcggcaaccgcgcggccgtcgagcccgttcacggcaatgctgaagcggatgaaatcgcgcagatgctgcagggcttcgtcgccgacgcgcccttcggcgtagagcaggcgcagtgcatcgatgacgacggcggaatcgcggaaccaatgaaagaagtagtccgggtccgggttgtagtcggcgagcacgggcgaagcgacgatggcgccgactatcggccgtatggtctggccgaagcccggccgatgcttgacggtcgacaccggcgagatgctggacagcatcgccgtcgccgaatggcgcagctgtgtttcgagccaggactcgaacgccgggtcttccaggctcgccacgctgaaggtcacggtgcgggcgacccgagacgcgggctgctgaagtccaggcgccgcagcccggcctgcacttcgggcacgctcatgaacagtttccacagaaggcccgtgcgatggttctccatcatcacgacgatggggccttgatcgatcgcaagataggtgtctgcgaaccagtctcgctgctcgcagaacgcatcgacgaagccgtagtctctccacaaccgctcgccatgcacgctgaggaaatgccgcaccaccttcatcacctcggccggcgcgtacggcaggctggccagtgcggccgtcggcgaaatggtgccgttgtcgatgtccggagcgtgcgcgaggtagccgtaggggtcgtcgctggcggtcaggccccagcacgattcgccgtagcccgcgtggccctgggggttggcgaggcagtgggcacggttgatctggacgtggcggcagttcagatcccaatactcggcgtagcgatccttcaagccgcgcggatcgaggccgcagaacgagtaatgcgtgaagaacagcgggccgccgtaaggcatgccaagcggaatctcgatgccgtagtacgactggccgttgaggaagccttcgcccgccgcgaagccgcggtggtacacccgcggatcgatcgcatggcggggcgcggccgcggccagcacgtaggtgatgaggcactcgttccagccgcgcacttcatggttcattgcccagccgtgtttcgggctccagtgccagtacagcacgtcctgcccgccctgagtgaaccagttccattcgacctcgtgccacagcgtgtcgaagtccgcgcgcaaccggcgcgccatggccgtgtcctcgctgaaatactggcgcgcacagagcaggcccatgcagaggaacgaggtctcgaccagatcgcccgcatcgtccttggggctcatcgggatcgtctcgccgctcgccccgtccatgaagtgcgggaaggcgccgtggtagcgcttggcgcgaaagagggcgtcgcgcatgcgccccaggcgctccagcgctgcgtcccgcgtgacccatccgcgctccaccgcgacgatcaaggccatgatgccgaagcccgtgccgccgatcgccaccctctcgtccgccaggtcttcgcccgtggcgccgacgagcgtgcggcggtcgagcgccaggccgctggcggcatccgcaccatcccagaaatagcggaaggtctgccgctgcacggcgtcgatcaaggcttcatcgggcagggctgccagtgccctcgggttcctgtcatccttcagcacgaacggctcctttcgttgtcgtctcggtaacacgtttggtttcaccgaattgtcggcagcgcaacgcggccgagggctctccgcccgcagcatgccatcattaaggcccttgggttctattcgaaatccctgatgagccgcatcgataccctcatggcccggatgacgctagccgaaaagctgggtcaactgacgatgactgcctccagctacacggtcaccgggccggtgctcgcgggggactccacgcagtcgatcatcgacggcaccgtcggcaatctgctgaacatggtcggcgcaggccccacgcacgagatgcagcggctggccgtcgagaagtctcggcttggcattccgctcttgatcggcctggacatcattcacggccatcgcacgctctttccgattccgcttgcggaggccggcaccttcgaccaagacctctgggagcgcactgcgcgcgaggctgcgcgcgaagcctccgccgacggcctggccatgactttcgcgccgatgctcgatgtatcgcgcgatccccgctggggccgcaccgcggaagggcccggcgaagacccttggctgaacgcacgcatcgcacaggccaaggtgcgcggtttccaggggaccgacctgtcatcggccgattcgctggccgcctgtgcgaagcatttcgtcgcgtacggcgcagtcaacgcggggcgggagtacgccgccgtggacatctccgagcgcaacttgcgcgaggtgcatctgccgggcttcgcagcagcggtccgcgccggcgtcgcgacgctgatgcccgcctttaccgatctcaacggcgtgccgatgacggcgcacatccctttgctgcgcgactggctgcgcggcgagatgggctgggacggcgtcatcgtcagcgactacaacgcgatcgcggaattgatcaagcacggcgtcgcggccgatctcgccgatgccgcggtgctggcgctgaaggccggcgtcgacatcgacatgatggccgacgcgtatcgcaagggtctgcccatcgcgctcgagcagggacgggtgacgatcgaagagatcgacgcgagcgtgcgccgcgtgttgcggctcaaggagcagctcggcctgttcgacgacccctaccgccgcggcgcgacaacaccggagcccgcggcggttgtcgccgagcggcacacgctgtcgcgcgacgccgggcgcaaggccatcgtcatgctgaggaacgagcgggacaccctccccttgcctgctgcaccgaaggcactgtgtgtcatcggcccgctggccgacgccagcaccgagatgaaaggcccatggtggggtgccggcgaacacgagccggccgtcagcgtgcttgccggcttgcgcgccgcgctgccgcagaccgacatacgccatgcacccggcgtcgccatcgagggcggcgacgacagcggcatcgaagccgccaccctgctgtgcgacggcgccgacgccgtcctgctgtgcctgggcgaacgtgccacgatgagtggcgaggcggcgagccgcgccacgcccgcgcttcccggccggcaacaggctctggccgaagcggtgacggcacgtgcacatgcgctcggcattcccgtcatcgcaatcttgttctcgggccgcccgctcgtcgttccctggctggccgaacacgccgatgcgctgctggctgcgtggttcctcggcatcgaagccggccatgcgatcgccgacgtggtcacgggccgggcaacgcctggcggtcgcacgccgatgagctggccgcgcgccgtggggcaggtgccgatctacttcggccagcgtcccaccggtcggccgatcaaccctgccgactacttcacgagcaagtaccaggacgtcgagaatacgccgctgtatgccttcggccacggcttgacttacggccggtttttatacgacgagcttcaggttgagccgcggcgcatgcgcgagcaggacacgctgaagatcagcgtcagactgcgtaacgttggcgcgcgcgaggctgaagagactgtcttcctgttcgttcgcggcaagctgagccgcgtcacccggccgttgctggaactcaagggctacgccaagctgcggttgatgcctggcgaggccggctcggtgagcctggagctgccggcggccgagttgcgctacctcgggccggacctgcagcccttgttcgaggcgggcgaagtcgagatcctcgtcggcccgagtgccgaggaatcagggttgctgcgccagagcatcgagttgtgttgaaaccctgcggatttcatcgacgatgccggcgaaggtctagttccgaaggtagaccggccgttcgtgaagaaaagtgccactgcctgcaatcgtcagccgccgacattcgacgggggcgaaggcgaagggcggcaaccagtctggagcgggcatgcctgaagggcggctaacgcggcaagagcggtcggtggacttatgctcgtgtactaccgtagtcggccagaagccgccactcggcaatgtcagttttcgagaagtctgtcatgatcaatcggctgccgcttttgtctgaaagatgcgctccaaacgagtcttgccgatttgccaaatcatttcgaggcgcaccccgatggtttgattgtcgacaccacccaatggtgggaggaacactgagaaagcctctcaagtcacttccgccaagtagttgattctcaaggaatcttcagtgtgactttcgggcgatttgcgggcgcggccgattacttcgctaacccttccatcgagcggacactcaacgggctacgcccggcgcctgccgctcatgtcaaacgcaatgtctgaacgcaccaagtggcggcggccgtcagttccgggagcatgcgttgtcctggcatacctctttctgacgtcgtgcagctatgcacccagggttcccgctgcaggcgacctgttcggacaacacgttagaacgaccgtggattcagaagtggcgcgttactacctggaaaactacctgcagggcgaagacgagaaccacgctctgagtggcaggatagatgctctgcatcgcagagtatgttcgatccccgccgtcgagagaggatctcagcgcactttcgcgggtgttctcggttgatttcgcagcattgttcctcgcgcaccggctcctgaccgacgaatgcaacagggcgctgaaccagtcctttgcgagctacctcaagtttgaggccggcgtcaaccccgggatcgtttcctcctacgtggtgctcttcgttccgggctgggattacgcacggaacggacacgtgaccggcgccgattttgccaagccacgcgagcttgttagccgatttggcttggagaaccacttggtcgaactacctccgaccggttctgtggagcggaatgcaactgttctggcttcagagattgccaggcgaagccgctcgggaaaaaagatcattctggccagcgcgagttccgccggacctgccgttcaacttgtcctaggcgagatgctgagcgaaagggaccaggactcggtcaaggcctggctcaatctcggcggcatccttcagggcagcccgcttgtcgactatcttgaggcgaggccgtggctgttcagcccgatcgtctggcttaaagggtgggagaaggaggcgattcgcagcatgtctacgagccggagcagaagccgcttcgcgcgcctggacatgggttccggcattctggttgtcaactacctgggtattcccctgtcgggacagctcagtagattctcgcgagacaactacccgatcctcagctcggatgggcctaacgacgggctgacgatgcttgcagatgcgatcgccccgaacagcctgacaattgtggctcttggaagcgatcacttttttgccgaagatccgcagatcgacgagaagacagtcgccctgatgaagctgatgctggcctacgtggagagcgacataacaagcggttccagccgatgtcctcgcctacggatcggccacggctgaatcacggcgataggcccgcgggcggctcagctcgaacgttagacctcaaagtccacccgggaggtgctcatgcccaatggcgacgagaagatctgtgcaagtgtccaagtccaacttcagactgcttgcgggctttcctttacatgctctgaaaggtagctctgggcccgattgcgacgttcaggcttcgcgatcttaggaccgcaaaccagtctgaagcagcctcttgagcaatgcattcctcggcatccggcagcagcaactcacccgcccccaaactccctcgcatgctccaccgcatacttgatcaattccgcctgcccttcgatccccagccgccgcttgatactctgccggtgcgcctccaccgtacgcacgctaagccccaaatcccgcgcaatctgcttgctcgattcacccctgcctagcgcagtgagtatttcgctctcacgcggggtgagcaacggcctcggcgcctgattgcgaaacagcttcttcgacacggccgggctcaaaaaggtgccaccacctgacacggcctctatggcggcgacgatctcggccgctggcgcgtctttcagcacatagccgcgcgcgcccacctgcagggccttctgcacgtactctgggttgtcgtacatgctgagcatcaccacgtggggcgcgggctggcgttgcagcaccagcgcggccaggtcgatgccgttcatttctttcatgccgacatccatcagcagcaggtcgggcttgagcgattcgatcaaggccagcgcctcggctgcgctgccggcctcgccgacgatctcgagattgggcatggcgccgagccttgcgcgcaggccatcgcgcaccagcggatggtcgtcgaccagaaagaggcgaatgggggcggcgtctttattcgtcatctggctactcaggctttgcgctgcgggtcggcacttcggccacgatggtggttccgccttcgccggatgtcacgcggaggcgcccgccgatggactccatgcgttcgcgcatgttgcgcaggccaatgccgcgccgcgggtcgagctgcatggcgtccacgtcaaagccgatgccgtcgtcgccaatctcgagccgcacgccttcgtcgtcgaaaaagcccaggtcgatgtgcacgcggtgcgcctttgcatgcttgcgcacgttggtgagcgcctcttgcgtgacgcggaaaagtgcggtcttggcttcttgcgagagttcgtaggcttcgccctcgatcatgatcgacgcatcgatggcgccctcttcggcaaactcgtcgcccaggcgctggagcgcggcgggcaggccgagggtgtcgagcaacgcaggccgcaggcggtgcgagatgcggcgcacctccagcagcgaatcgttgagccgttgcagcgccttggccagtgcgggcggtgcggcctggctttcgcggtcgagcgcttccacggcggattcgatcagcagcttggccgagaccagcgtttggctggtgccgtcgtgcagctcgcgtgcaaggtggccgcgctcttcttcctgcgactgaaccacgcgccgcgccaacaggcgcagcttggcttcggccacgcggtgctcgctgaggttgagcaggaggccggtggcgctcaccacgcccaggcagagcgcggcaatgccggcaatccagagcagcgtggtggtgacgttgctgctcatctggcggtcgagcgcctgcatcgtcgtttcgatgtcgtcaaggtaaaggccggtgccgaccatccagttccagcgcggcagcgccgtgacgtagccgagcttgggcgccatctgctcgctggagggcttgcgccattcgtattcgacaaaaccgccgccggcccgcgcaccggcaatcaggtcctggatggtgaagcggccgtgggcgtcgcgcaggtcccagagattcttgccgacgaggtcgggctggcgcgaatgcatgagcgagcggccctgcatgtcgtagacgaagaagtagccgtcgtcgccgtagtcgagcgcggccaggcggcgcagggcttcgttgcgggtttcgtcgtcgtcctggccggcgtcgtacagcgggcgcacggtgctcacggccaggtcgacatagctgcgcagttcgctgcgccgctgatccatatagcttttttcgatgagcgcgcgttcgcgccgggccaggtcatgctcctggtggcgcaccgccagggccaccagcaccagcgcaaccagcagcggtgccacagccagcgcgacgatcttggtgcggaggttcatcggggggcaagactaccaccgggcgcggccatgagcccgtcgcctgacggcgctcactcagtgcacactggtcggccggcccgaggccacccaggcatcgagcccaccggtcaatggcagggcccgccgcgcaccgcgcgccagcagcacgcgcgcggccagggccgccgacacctcgttggggcaattgcagtaaacgaccacatcgcgcccgccgacgtgcggcagttcggggtgccgctgctgcagcgacttgagcgtgtacgccagcgcgccgggaatgcggcgcgggtcgacctgcacgcccgcttcgccgcgcacgtcgatcaccagcgggggcgtctcgctggccagcagttcatgcagctcttccacggtgatgcgcggcatgccggtgagccgcatgaacgcgcggcggcgccagtagcgcaccgccagcatcacggccagcaccaccaccagcgccacggtcgcaacgccgccggcctgggccagcatggccagcacgtcctggatctggtcgcgaaagatccagcccagcccgagaaaaaggccggtccagaccagcgcggcgccaatgtcgaagacgatgaagcgccacaccggcatgcccagcgcaccggccatcggtggtgccaccaccgagacgcccggcacaaacttggcggccaccagcgagagcccgccccagcggccgatgagcgattcgccgcgccgcacgcatgaatcgggcgacagcgagatgcggcacagaaggcgcatgaagcggtagccgaagcggcgcccggcatagaaccaggcgccgtcgcccagcaggttggccagcaccgcggccagcaccacgcccgccaccgagacgttgccggccgccagcagcgcgcccgacaccaccagcacggcggccgcgggcaccggcaatccgaggcgcgcggcaaagctcgccgcgaagacgatcgcgatcgcgttctgcaccagcagcgacatcagctgtgccatggcagcagcaacagcaacgcgaggttggggttcactcgtttggggcggcctagcgcggcgcgtcgcccttgcggtattcggccgtgagctcgtcgagcctctgcttcagcgcggggtccagcttgtaggcggccgcggccagcgtggcgtcgagctgctcggggcggctggcaccgagcagtggcgcggtgatgagcgggttggccatgacccaggccaccgccagcgtggccagcggcacgccggcttcgtcggccagcttgtggagctgtgtcacggtgtcgaagctgcgctcgttccagtagcggtcctggtacatgccgccggccgtgccgagcgtgaagcgggtgttctcctcgggcgtggcgccgggcttgtacttgccggtgagcaggccgccggccagcgggttgtagggaatcacgcccaggccctcttcgcccgccagcggcagcaactcgcgctcgatctcgcggaacagcaggctgtagcgcggctgcaccgacacgtagcgcgtgagcttgtgcagctcggccttgccaagcgcgcgggccagccggtaggccagaaagttggacacgccgatgtagcgcgcgcggcccgacttgacgatgacgtcgagcgcctccaggctctcttcgagcggcgtctcgcggtcgtcgctgtgcagctggtacaggtcgacgtggtcggtctgcagccgcttgagcgaggcgtcgatggcgtcgagcaagtgcttgcgcgatgcaccctggtcccagctgttgggcccgaccttgccgaccgccttggtcgccaccacgaagcggcggcggccggtggggccctgcttctgcagccagcggccgatgatttcttcagtgcggccggtggtttcgacggtgccgccaagcgggtacacgtcggcggtatcgagaaagttgatgccaccctcggcggccttgtccagaatgcggtgcgacaccgcctcgtcggtctgcaggccgaaggtcatggtgccaagcgcaagccgcgacacggtaaggcccgtgcggccgagacgggtggtgggaatgctcatggtggtctcgatcgagagagatgacggagaggaagggcggcggccatcatagacacggccgcgcaaacctgctggcacccccgatatttcaggtggcttcgagatgcacgccgggcgcgccgcgctccaccgcaaagcgggccatcggcgcgacggcgctgtctgcggatttctcgtcttccacggcgcggaactcgaccgtgcagccgcgcgcatcgaacgccatgtgcgcatagccgcgcttgtcgccccggccgtagcgcaggtggtcgttcttggcgagcaggttggtcacgttggcggcgctgggcccttcggaggtgatggcgccgccgacgaattcggtcgccaccgccgggccttgcggctcgcggcgcagatcggcagcccagaaggcgtgcacgtcgccgctgatgaccagcgcatcaccgccgcgcgccttgttggcggccaggctgtcgagcaggcgcgcgcgggacgcggcgtagccgtcccagccgtccatccagtagccgtgctcggggccgcgcttgcggtcggcctcggccagcaaggtgggctgcgcaatgaccgtccagcgcgcgggcggcgcggccagttcgttcgcgagccaggcttcctgcttcttgcccaggaggctgcgctccggcgcgagtcggtcggcacagtcggccaatggcgatgcactgcggccggccaggcaggcgtggtgcgagcggtactgccgcccatcgagcaggaacacgtcgagcatgcggccgaagcgatggcgcccgtagatggtggccgcggcaccggtcggccgcatgctggcgggcacgggcatgtgctcgtaccacgcctggtaagccgcggcgcggatggcaagaaactgcgcggggtcgatggcgcgcggcgacacgtcgtcggtgtagtcgttggccacctcgtggtcgtcccaggtcacgagccaggggaacgcggcatgcgcggcctgcaggtgcgggtcggtcttgtagagcgcgtagcggtcgcgaaactcgcccagctgcgtgggaatgccgccctggtggcggcgcacatggcgcgagccccatgagctttcgtagatgtagtcgcccaggtgcacgacgaagtcgaaaggctgcgcggccatgtcgcggtaggcggcgtagtagccctgctcgaactgctggcacgacgcgaaggcaaagcgcaatggttgcagcgcggcatcggcttcggccggcgcggtgcgggtgcggccgacggggcttcgcgcgccttcggccgtgaagcgataccaataaggccggccgggcgcgaggccccgcacttcggcatgcaccgaatgcgcgagcgccgcaacggccgtggccctgccctccgcagcaatgcgggcaaagttttcgtcgtgcgccacttcccagcgaacgtcgaccgatgcgtcgcccatgccgccgccctgcagcggatcgggcgccaggcgcgtccacagcaccacgccgtcgggccttgggctgcccgatgccacgccgagcgtgaagagttcgcgcgaactttgttgttgcgcgttcagccggaggaacggatggcccagcgatgcagccgccatcccgctgagcagcaggcggcggcggcgcgagacaggctgggccgccctcatgtcttttcgcgcgcggccagggccaggtcggagcggtcggtggtgatctggcgcacgggcatggtgagccattgtgcaatttcctcgcgcgggtcgatgacccaggcgctcaccgtcgggtgcggccgggcactgcggccacgcagcgcgccagcgagtttgcgcgttcgatctacgaagcgctcggcgcgcgctgagcggcgtcgggccgctcgctggcgcgtgcactcgccaccgcccaccagaacacacccatgccggccagcgccagcaaggcgccgacccagccggtcgacgtccagcccaggcccgcggcaatggccacgccgccgagccatgcaccgagcgcattggccatgttgaaggccgagtggttgagcgcggcggcgagcgtctgcgcgtcgccggccacgtccatcaggcgaatctgcagggccgggccgatggcgacggtggtgccgatgaggaacacgttgaacgccgcggtaaagacgttgtgcgccgcgaacgtgaacacggcgagcaccagcgccgcatagacgagcaggccgccgatggtgcgcatgagcgacttgtcggccaggcgcgaaccgacgaggttgccggcgaccatgcccaggccgaacagcgcaagcacgaagggcacgccgcccagcggcaggcccgccacctcgatcagcgtgggcttgatgtagctgaacaccgagaacatgccgccgaagccgatggcgccgatgccgagcgtgaaccacacctgcttgcgcttgagcgcgcccagttcgcgccaggggctggcacctgcgggcgccgcaaggtcggggatgtcgcggcgcagcagcaccacggcaatgagtgcgatgacgcccacgaacacgaaggccgcgcgccatccgaaaagctggccgagccaagcggcaatgggcacgccgaccagcgtggcgccggtgagccccagcatcacgaggcccacggcccgcgcgcggcgccccggtggcgccagcgtggccgccacgagcgcggcaacgccgaagtaggtgccgtgcggcagcccggtcgcaaagcgcagcaggttgagcgacatgtagcccggcgccatggcgctggcaaagttgccggcggcaaacacggccatgagcgcaaccagcagtgcgcggcggcgccagcccgcggcgagcaccgcgagcactggcgcgccgatcaccacgccgagtgcgtaggcgctgatgacgtggccggcctgcgggatggtgaccgcgatgtctttcgcgacctcgggcagcagccccatgatcacgaattcgccggtgccaatggcaaagccgcccacgccgagggccagcacggcccgcaggaagtcgacgcgcgatgcggaagaggaaacggaaagatcggtatccgcgctgtccagcgcgggcggggaggcgttcaaggccaggctcctgggagggtgcccggcggcgacgggcagaggcctgattttagggtaaaccctgaatttttgctgatacagccatgctgtccggctggtaccgccgtgccggacgatggccggccgggatgcttagatcgccacgagctggcgcacgccctgcgcttccatgtcctcgccgaggccgcgcgcgatcacttcgccgcgctccatcacgaggtagtcgtcggccagctcctgggcaaagtcgtagtactgctcgcacagcacgatggccatgtcgccgcgatcggccagcatgcggatgacacggccgatgtccttgatgatgctgggctggatgccttcggtcggctcgtccaggatcagcagcttgggcttgggagccagcgcgcgtgcaatggccagctgctgctgctgcccgcccgaaaggtcgccgccgcggcggttgatcatctgcttgagcacggggaacaactcgaacagttccgccggaatgggcgtgctgccgctcttgtaggctaggcccatgcgcaggttctcttcgaccgtgaggcgggcaaagatctctcggccttgggggacaaagccgatgcccgctcttgctctttcatacggcgtggccttgtggatcggcttgccttcgagttcgatgctgccgctcttgatgggaacgaggcccatcagcgacttgagcagcgtggtcttgcccacgccgttgcggccgagcagcacggtgaccttgccgagcgtcgcctcgaagctcacgtcccgaaggatgtgggagccgccgtagtactggtggatgttttttactgtcagcattttggggacgccttcctttgtctttgttggaggcgcccggggtgcggcacggcgcgatcggccccactatgccggcccttcgggctcccctgcggtgctcgcatttcgcggggtctcgcagaactcgcttcgctcaaacagctgcgagccctgatccgcgaaacgctgcgctcctcggcggcacagaggggccgcccacaccgcgccgcaccccgggcgctggccgtggcgttaatgccgcctgccctcaccccagccctctcccgaagggagagggaggaagtcagggggtacaccatggctctgtccacggcgatgggggttgagcccttgggtggccgttgaggcaccgccgagcagcgcagcgacgggcggatcagggctcgcagctgtttgagcgaagcgagttctgcgagaccccgcccgtcgcgagcagcgcagggaagcccgaagggccggtgacgtcggccgcccaagggctcaacccctatcgacgcaccccgaacagaatcagcgaccaagatagacctcgatcacgcgctcatcagcctgcacctcgtcgagcgtgccttgcgccagcacggagccgtcgcacagcaccgtgacaatctcggaaattgttcggatgaagctcatgtcgtgctccaccaccatcagcgaatgcttgcccttgagcgtgagaaacagctctgccgtgcgcgccgtttcctcgtcggtcatgccggccacgggctcgtcgagcagcagcagcttcgggtcctgcatcagcagcatgccgatctcgagccactgcttctggccgtggctcaggttgccggccaggcgggacacgctgtcggccaggtggatggtctgcagcacttcggcgagccggtcactctgcgcggagtcgagcctgaacagcatcgacgcgcgaacgcccttgttggtcttgagcgcgagttcgaggttctcgaacacggtgagatgctcgaacaccgtcggcttctggaacttgcggccgatgcccagctgcgcaatgtcggcttcgcgatggcgcagcaggtcgatggtgctgccgaagaaaaccgtgccttcgtcgggccgcgtcttgccggtgatgatgtccatcatcgtcgtctttcccgcgccgttcggtccgatgatgcagcgcagttcgcccggcgcaatgtcgagcgacagcttgttgatggccttgaatccgtcgaagctcacgctcacgtcttcgaggtacaggatgcggccgtgtgtcacgtcgacctcgcccggcgttgcaatgcggccgaaatccgcggaacggccgccggactcggtgctgccgctcatgtagggcatgcccgcggcgcgggcggcgcgctcggcgccggcttccatcaggtcgggcgtcatgcgcgcgctcccttcacctcggcggccagcggcgcgtgcagcgcctccggctccacgccttgcgcggcggccatggcgcgctgcgcttcttctcggccggcgcttggcgcggtcttctcgcgcgacagccatttcttcaccagccccacgatgccgttcggcaagaacagcgtgacggcaatgaacaaggcacccaaaaagtacagccaatactcggggtacgccaccgtcagccagctctttgcgccgttgacgatgaaggcgccgatgatcggaccaatgagcgtggcgcgcccgcccaccgcagcccagatcgcgatctcgatggagttggccgcgctcatctcgcccgggttgatgatgccgacctgcggcacgtacagcgcacccgccacgccgcacatgacggccgagatgacccagatcgtgagcttgtagggtagcgggttgtagcccgagaacatcacgcgcgtttcggcatcgcggatggcctgcagcacgcgaccgaacttgctgccgatgagccacctggcaaacaggaagaagccgagcagcgtggcgcccgtgagtgcaaacagcgtcatgcgcatttcttgcgtggcaatcggaatgcccaggatgcgcttgaaatcggtaaagccgttgttgccgccgaagcccgtctcgttgcggaagaacagcagcatggccgcgaaggtcatggcctgcgtgatgatcgaaaaatacacgcccttgatgcgcgagcggaacgcgaagaagccgaacacgaaggcaatgaggcccggcaccgcaacgatgaggatgagcgtggcaacgaagctgtcgctgaaggtccagtgccagggcagcgtcttccagtcgagaaacaccatgaagtccggcaggtcgctcttgtagttgccgtcgcggccgatctggcgcatgaggtacatgcccatcatgtagccgcccagcgcaaagaagaggccgtggcccagcgagagaatgccggtgtagccccagatcaggtccatggccagcgcgcagatggcgtagcacatgatcttgccgaccagcgccaccgcgtagtcgctcatgtgcagcgggctgcccgccggcaccaccatgttgagcaccggcgccacggcgcacaccacgatcagcgtgacgaagaaggctgtccagcccttgccgctcaagagcggtcctttggttggcaatacgaccttgttgttgctcatgcctctgcgctccggcccttcatggcgaagatgccctgaggtctcttttgaatgaagatgatgatgaagacaagcaccgcgatcttcgcgagcaccgcgcccgcccagccttcgatgaacttgttgagaatgcccaggcccatggccgcatacaccgtgcccgcgagctggccgacgccgcccatcacgaccaccatgaagctgtcgacgatgtagctctggccgaggtcggggccgacgttgccgatctggctcagcgcacaacccgcgaggccggcaatgccggagccgagcgcgaaggcgtaggtgtcgatgcgcgcggtgttcacgcccatgcaggaggcaatgggccggttctgcgtcacgccgcgcacgaacaggccgagccgcgtgcggccgatgagccagcccattgcaagcagtaccagcactgcgaagatgatgatgcaaatgcggttccacggcagcgtgacgttgctcagcatggtgaagccgccgctcatccagccggggttttccacgccgacgttctgcgcgccgaacagcgagcgcacgagctgctgcagcatcaggctgatgccccaggtggcaagcagcgtttcgagcggccgtccgtagagaaagcggatcacgccgcgctcgagcaccgcgcccaccagcgccgaactcagaaacgccaccggaatggccgccaccaggtaccagccgaaggccgcttcgggcatgtagcgctggaagatgccttgcatcacgtaggtggcgtaggcgccgatcatcatcagctcgccgtgcgccatgttgatgacgcccatgaggccgtaggtgatggccaggccgagggcggcgagcagcagcaccgagcccaggctgatgccgctgaacaccgcgttgatgcggtcgccccacaccagcgagccgtcgatgctggcaatggaagcgacgatggcggccttgacgtccgcttcggtttcgtcagcgagccgctggttgagcagcagcttggtgtcggggctgctgttggcgccgagctccttggccgcggcaaggcgcctggccttgtccgcgctggtgagcatgctggcggcgcgcaccagttccagctgcgccttgatgccggggttggtctcggcggccagcgccttttcgaccatcggaatgcgcgattcgtcgggctccttgaagagcgcctgcgcggcttcggcgcgcaccgcatcgtccttgctcgtgagcttgagcacggcttgcgcggcatcgagcgcgccgcgcatgaggttgttgttgaccacgtcctcggccgtgtcgggcaccttcaattcggcgccggtcacggggtcgtagcctttgtcgtccttcatcacgaagactttgtcttcggaatacttgaccgcgtcctcggacatggcctggatgaatgcggcggtcttgtcgtcggccgtgagcacggccttgttgagcgcggtgatgcgcgattcggattcgcccgaggcgatggccttggcttcgtcggcggtcagcgcgtggacggccgatgccatgagcagcatggcggcgagtgcgcaatgaagggatcgtcgaagcatggtgaatgagatcgtgttgccccctctccccttggggagagggttggggtgagggcgggcagccttccaacagacacggcggccagatcgaccgccgttgccctcacccccgccctctccccgaggggagagggagcaagagagggacttgccgacgaattacagcgacttgccagccggctggtcaggcttcttgtcgttgccttcgatgtacgggctccacggcttggccttgaccgggcccggcgtcttccacaccacgctgaactggccgtcggccttgatctcgccgatgaacacgctcttgtgcaggtgatggttcttctcgtccatcttcgacacgatgcccgagggcgccgtgaaggtctggccggccatcgccgcgatcaccttgtcggtgtcggtgctcttggccttctcgacggcctgcttccacatgtggatgccgatccaggtggcttccatcgggtcgttggtgagcggcttgtccttgtggccggcaatgttcttggccttggcgtaatcgccccactgcttgatgaacgccgtgttggtcgggttcttgatcgacatgaagtagttccatgcggccaggtggccgaccagcggcttggtgtccacgccgcgcagttcttcttcacccaccgagaaggccaccaccggcacgtccttggccttgaggccggcgttgccgagttccttgtagaacggcacgttggagtcgccgttgatggtcgacaccacggccgtcttgccgccggccgagaacttcttgacgtcggcgacgatggtctggtagtcgctgtggccgaagggggtgtacttctcgtcgatgtcggtgtccttcacgcccttgctcttcaggtaggcgcgcaggatcttgttggtggtgcgggggtacacatagtcggtgcccagcagcacccagcgcttggcgccgccgccttccttgctcatcaggtagtcaacggccggaatggcttgctggttgggcgcggcgcccgtgtagaacacgttcttcgacagctcttcgccttcgtattgcacggggtagaacaggaggccgttcatttcctcgaccaccggcagcaccgacttgcgcgacaccgaagtccagcagccgaagatcaccgacaccttgtcctggccgagcagctgcttggtcttctcggcgaacagcggccagttggaagccggatcgaccaccacgggctcgagctgcttgcccagcacgccgccctttttgttgatgtcctcgatggccatcagcaccgtgtctttcaacacggtttccgagatggccatcgtgcccgacagcgagtgcagcacgccgaccttgatggtgtcggcggcaaaggccggcgcagcggagatgctggccagggcgacggcggcggtaagcgccttgagtgtgaaacgacgttgcatgtggactcctgctccagggtggttgaaacctttgtcgccggctggccggacgatggaagggagtctgcggattcgcccgcccgcgagaaatacgccgggtggcgtacacggaggtactcagggcggccgacctgcaattcggctcggccacacactctttctacgcgcgtgatcctcgtggcaaaaacccattttgggctttaaaatgcccaaaatgggtaagttcttgtcgcccgccgcgcagatcgagaggcccgccagcttggcggatgccctgttcacgaccacccagcaacgcgtgcttggctatctcttcgggcagccggaccgcagtttcttttccaccgaattgatcaagctcaccggcgcaggctccggcgcggtgcagcgcgagctcaagcaattgaccgacagcggcttgctcatcacatcacgcgtgggcaaccagaagcactatcaagccaacgccgcggcgccgatctacgacgagttgagcagcattgttcgcaagaccttcggcctcgcaggtccgctgcgcgaagccttggaaccgctcgccgcaaaaatcgaagccgccttcgtattcggctcggtggccaagaacagggatacggcctccagcgacatcgacttgctgctgatcagtgaagaacttgcgtattcggacctgtttctcgccctcgatgcagtgtcggcacgtcttggccgtacagtgaacccgaccatgttcacaagaaaagaactgatgcgaaagcacaaagacggcgagtcgttcgtgaagcgcgtcatggaacagcccaagctctgggtcatcggtgacgcgcatgccctccccgcttgaaaacctgtgcggcccgaccaagccgctcaccgcagaacccccggatgctcgcgaattcgcgggcctgctgcgttctggccttgcacgcctggcggatgcccaggtgatgcaactctccgtcgagggccgattcgatctcgcatacaacgccgcgcatgccatgtgcctcgcagcgctgcgttggcatggctatcggtcgagcaaccgcttcatcgtcttccaggtgttgccccatacgttggagttgggaccggaggtgtggagggtattggccaaaggccacgaaatacgaaacctcggcgagtacgaaggcaacctgaatgtggatgagcgcatcgtccgcgatctgatcgcagcatgcgagcgcgtagcctcgaagctctctgaactgccgccgcccaggctggactaggcattcgcggccgaaatcaaacttcgggcctcgcgcttgaattgggccaccgcaaaggcccagaccatgcgcgtcgcatcgggccctcccgggtcgctgaaaagcagccgggaagcgccgccgctccacgcgtgccccaggcgctcaatttcgcacagcgtgaccaccgcgcggcctttgcgccggaactcggtcacctgcatggggtgccgcttgccgcgttgaagcgtgcgcggcgtccccggcttggcacccagggccgtggcccatacggccgcgctgctgacggcattgctcggcgccaccacggcatctgcggtgccatgcagcaccagcatcggcggcaaggttgcaaagacggcagccgcgcccatcgccttgccgaccgcggtggacggcatgggcggcgtgtgctgtccgcgcatcgcgccaagggcggtggccgaagactttgccgcacccggcgccacgcccgaatgcatgaccacggcgcgaaagcgcagcgggtagcgcgtggccagcagcgccgccatgctggcaccggccgaaaggccggccagtgcaatgcgctcgcggtcgaccggatacagcacgcaggcctggtcgatggccgccatcaacgtggcggcctcggcatcggccttgcccgagcggcgctcataccagttccagcagccttggggatgggccagcctgtcttgctccaggtacagcaccaggaagcgctgccgcactgccagcgtattcatgcgcgtgctggccgcaaagtcgcgccccgtctggccacagccgtgcagcatgaccatgagcggcagcttttcgccgggcgcgagcttcaggtcgacgggacggaacaggtgatagccgcgtgcaccgccggggcccagcgccatgccgctgagccagtcgcccctgccgggcggcggcttgagccgcttggcggtggcgcgctgcacctggcccgtcacgcgcttgctgttgctgagcgtgagtttggtgagtgccttcaggttgcgctcgtaggcgcgggcgaacagggatgcagtggaacgacggaccatgggcgcagtgtgagggcaaagcgccggccggccaaacggccgcgaggcctcagtagatttccggcacgatcatgtcggccggcacgggctggcgcaaatagtccgcatggcgctcgcgcgccggcaggtcgaccggcggatgcggcacctcctggtagggcagctggcccagcaggtggctgatgcagttcagccgtgccttcttcttgtcaaccgcctgcaccacccaccagggcgcttcgggaatgtgcgtgcgctccagcatgatctccttggccttggtgtattcctcccagcggcggcggctttcgagatccatggggctcagcttccattgcttgagcggatcgtgaatgcggccgagaaagcgcatgtgctgctcgtcgtcggtgatggagaaccagtacttgatgagcttgatgcccgagcgcaccagcatcttctcgaactccggcacggtgcggaagaactcttcgtattcgtcgtcgctgcaaaagcccatcacgcgctcgacgccggcgcggttgtaccagctgcggtcgaacagcaccatttcgccggcggccggcaggtgcgcggcataacgctgaaagtaccactgcgtgcgctcgcggtcgttgggggcgggcagcgcggccacgcgggccacgcgcgggttcaggcgctgggtgatgcgcttgatgacgccgcccttgcccgccgcgtcgcggccttcgaaaagaatgaccaccttctgcttgctgtgctgcacccagtcctgcagcttcacgagctcgccctgcaggcggaacagctccttgaagtaggcctggcgagcagccttgtcggttgtttgcgccgcggggtcgagcccgtcgatgttgcggtcctcgatctccagctctagctcttcgtcatagctgtcgatcaggtcgcgggcgatgcgttgcatcaggtcttcgtggtctggaagtgcgctcgtcagcatcatggcaaggagaagaggtgtggggtagaacaaagcatgctgcccgccgcatatgaccatcgcgtgacaacctgcaatccgccgacacgaagttgtcataaatggcgaacaccatccgggacacacccttttgtctttcctgatccacacgcaccttgccggcactccatgacctggccgccaattcgtacggcggcgacgaagccgggctgatctgcggctacctgttcgacgccgatgcgccggagcctgtgcgggccatcgattcggcgcaggctgcggcctggctggatacgggtgcggtacaggacggccccatcgcagcgccgggccgcgcgagttcccccgcattcctctggctgcacttcaacctgagccacgcccaggccgagcgctggctgttgcgccatgcgcagctgtccgacaccttctacgaaacgctgcacgagggcctgccctccacgcgcatcgagcgtgctgacgattcgctgatagcggtcatcaacgacgtgcacttcgagttcagcttcgagccctcggacatctcgacgctctggatcagcgtggggccgcgcctggtggtcacggcgcgcgccaagccgttgcgctcggtcgatgcgctgcgcacggcggtcaaggccggggacgcgccgcgctcgagcaccgagctgctcgagcacctgctgcgcgcgcaggccgacgtgctggtgaagatcgtgcgcggcgtcacttcgcgcatcgaccgcatcgaggacgagctgcttgccggccggctcgaccacaagcgcgcgcggctcggcgtgctgcgccggctgctggtgcggctgcagcgcctcttggcgcccgaacccgccgccctcttccgcctgctgcaagggccgccgggctggatggcagagcccgacgtgcaggagctgcgcggctcgaccgaagagttctcggtggtgctgcgcgacatgcaggcactgcaggagcgcatcaagctgctgcaggaagaaattgccgccaacgtgaacgaggacaacaaccgcagcctgttcgtgctgacggtggtgaccgtgctcgcgctgccgatcaacatcctcgcaggcctgtttggaatgaacgtgggcggcattccgctggcggagcacaagcacgggttctggatcgtggtggcaatcgttgccagctttaccgctgtggccgcctggacggcattccgcaagaagcgctgaggcgcatcggcaggcgcagtaatgctatttatttaatagcaaccacaatagcatccatgcgcctgcatcgatttccagacccaatagaatgacgttgtgtccaccattctcaatgccgatctgcactgccattccgtggtctccgacggcaccctgacgcccgaggaactggccgcgcgcgcggcagccaacggggtcgagctctgggcgctcaccgatcacgacgaggtcggcggccagtaccgcgcagccgccgcggcacgcgccaacggcatccgctatctcaccggcaccgagatctcggtgaccttcgccaacgagacggtgcacatcgtcggcctgggtttcgaccccgccgacgccgcgatgacacagggcctctacgacacacgcggcggccgcggcaagcgcgcgcaggaaatgtccgaggggctggccaaggtcggcatccacggcgcctacgaaggcgcgctcaagttcgtcggcaacccggagctgatctcgcgcacccacttcgcgcgcttcctggtcgagcagggccactgccgcgacacgtccgaggtgttccgcaagtacctgaccgaaggcaagcccggctacgtgccgcaccgctgggcctcgttgaaggatgcggtgcactggatcacggccgccaagggcatggccgtcatcgcgcacccggggcgctacaagttcacggcgaacgaggaatacgcgctgttcctcgaattcaaggcgcatggcgggcaggcgatcgaggtcgtcaccggcagccatacgacggccgaatacgtcgagtacgccgacaaggcgctcgagttcgatttcgccgcttcgcgcggcagcgatttccacagtcccgacgaaagccactgcgatctcggcaagctgccaccgttgcccggtgcgctcacgccggtgtgggaactgctcagcgaccgcatccagcagtgagccagacccacgggcccggcaccgacagcgcggcaacggcggcactggcgagcgcccgcgccgcgtcgcgccaggcgcgcgacaccgaatccggacgcatcctcgcgggcatcggcctggtgctggtggcggtggcctgctttgccacgctcgacaccgccaccaagacgtccaccgccgccgtgccgatcctcatgggggtgtggttccgctatgccttccaggcggtggccaccacggcggtgctgctgccgcggcacggcaccgcgctgctgcgcacgcagcatccgcgctaccagctgctgcgcggcgcgctgctgctggtgtcgagcacgctggccttcctgagcctgcgctacatgccgctggccgagttcacgtcgatcgtgctggtcgcgccgctggtcatcacgctgctcgcggccaccacgctcaaggagcatgtctcaccgctgcgctgggtgctggtggcggggggattcatcggcacgctggtcatcctgcggccgggcggcggtgcattcagctgggccgtgctgctgcccgtggggctggtgctgaccaatgcgtggttccaggtgctcacgagcaagctggcgcaaaccgagaatccgctgaccatgcatttctataccggctgggtcggcgcgctgatcgcctcgctcacgctgcccttcgtttggacggcgctgccctcgtggcactggtgggccttgctgtgcctcatgggtttcatgggcacggtggggcatttcattctcatcctggcctaccagcgcgcgccggcctccacgctcacgccgtacctctatgcgcagatcgcctttgccatgctgggcggctggcttgtcttttcgcacgtgcccgaccgcttctcgctcatcggcatggcgatgatcgccgtctgcggcgctgccggcgcctggctcaccgtgcgcgagcgccgggtgcccatcgaaccggcggaatcctgatcaggagcttttttcttcatggcccagtacttcgaagtccatcccgacaacccccagcaacgcctcttgaagcaggcggcggcgctgctgcagcgcggagagatcgtggccgtgcccaccgattcgagctacgcgctggcctgccatctggacgacaaggacgcggtcgaccagttgcgccgcatccgccaggtcgacgagaagcatcacctcacgctgatctgccgcgacctgagcgagctggccaactacgcgcgtgtggacaacaaacaataccggctgctgaaagccgccacgcccgggccctacaccttcctgctcgaagccaccaaggaggtgccgcggcgcgtgagccacccgcagcgcaagaccatcggcctgcgcgtgcccgaccacaaggtgctgctcgaactgctgatgctgcacggcgcgccgctcctggccaccacgctgatcgcgccgggagaaaccgaggcgctgaacgacgcgcagaccattcgcgagcgcttcgagaagcagatcggcgccgtcatcgacgcgggcgcctgcccttcgcaacccaccactgtggtggacctcacgcccatgggctcgggcgacgatccggtggtggtgcggcagggccgcggcgcgctggcggtgctcggcctctgacaagcggcaccgaagctttcactctgtctgacacaatcgcacagtggatatttccaacctgatacagacggtacttatttacgcactgcccgtggtcttcgcgatcacggtgcatgaggcggcgcacggctatgtggcgcgccatttcggcgacaacacagccgaagtgatgggccgcgtcacgctcaacccgatgaagcacatcgaccccatcgggaccatcctgatgccgctgatgctgtactttgccacttctggagcctttcttttcggatacgccaaaccggtgccggtgaacttcgagcgcctgcgccatccgaagcgcgacatgatctgggtggcgctggccgggccggcatcgaatttcgtgcaggccattctttgggcgctggtgctggtcgggctcattgcaaccggcgtggatgaaacctttttcatcaagatggcgcagggcggcgtgctggtcaacctcgtgatgtgggctttcaacctatttccgctgcctccgctggacggcggccgcgtgctcgcgggcctgcttcccaacggtgcggcgcagaatttcctggcgcgcatcgagcccttcggcttcttcatcgtgatgggcctggtgctcgcgggcatcgtcagcaccttctggctgcgtccgctgatggacgtcggatacaccgtcatcaacctgcttatctcaccgctcacggctttgctgcgttaagttcctctcccatggctacgtcttcttccgctcccctgcgcgtcctgaccggcatcacgccgtccggcacgccgcacctcggcaattacgtcggctcgatccgccattcggtgcggcagagcgtcgcgccgggcgtcgagagctttttcttcctggccgactaccacgcgctcatcaaggtgcaggagccggcactcatccagcgctcgacgctcgagattgccgccagctggctggcctgcggactcgatccggaacgcgtcaccttctaccgccagtcggacattgtcgagattcccgagctgacctggttcctcacctgcgtgaccggcaagggcgtgctcaaccgcgcccatgcctacaaggcgcagctcgacaagaacatcgccaagggcgaagacccggatgccgacgtgacggccggcctcttcatgtacccggtgctgatgggcgccgacatcctgatgttcaacgcgcacaaggtgcccgtggggcgcgaccaggtgcagcacatcgaaatggcgcgcgacatggcgcagcgcttcaaccaccagtacggcgagcacttcacgctgcccgaagccgagatcgacgatgcggtggccaccctgcctggcctggacggccgcaagatgagcaagagctacggtaacaccattgccatgttcgcgccgcgtgcgcagctgcaaaagcagattgccagcatcgtgaccgactcgcgcgcgcccggcgaacccaaggacacagagggctcggcgctgttccagatctaccaggcctttgccaccgccgaagaaaccgaggcgctgcgcaaggcttatgccgaaggcatcggctggggcgacgcgaagcagatgctgttcgagcgcatcgacctcgaagtggcgccgctgcgtgcgcgctacgaagcgctgatgaacgacccggcggagatcgagcgcattctgctcatcggcgccgagaaggcccgcaagctggcccgccccttcatggccgagctgcgccatgccgtgggcctgcgcaacctcgcggcgggcagcggcaaggacggcgcccgcaaggccaaggttgccaagccgagtttcaagcagtaccgcgagcgcgacgggctgttctatttcaagctgctcgatgcgcacggcaccgccctgctgcagagccgcggttttgcctcgccgcaggaagccggccgtgccattgccgccttgcagcagcagcgtggcgcggcattggccacgctggccgaccggctcgagccggccgggccggaagaattacgcgccgcgaacgaggcgctggaggcactggcggaagcaacagcccctaccaacgggagttgatccggcaatatccatcggctacccgccgaggaagacgaaagaagacggtgcgatcactaaggaagaaaacatgagcatttatgtcatcgacgaccaccccctgatgcgcgacgccatcgtgatggtgttgcggcgcctgcggccggccgagaatatcgtcgagctcgagcgtctcgacaagctcgcgagttcggtccagcagcgcggtgcgcccaccctcttctgcctggacctgaagctgcccgacaccaacggcgtttcgggcgtggtcgcggtcaagcaggtctaccccaacgtgccgatcgccgtgtattcggcggcgccggccggggacatggaagacgcctgcatcgaagcgggcgccgacacgtacatcgagaagtcggccagctcggccgagctgaccgcggccctgcgcggcctgctgatggccggctccgaagaaggggaagagcccgcgctggccagcaacagcaagctctccaagcgccagacgcagctgattgccatgctcgacaagggcatgagcaaccgcgacatcgccaccgacctggagatcagcgagcacacggtgaaggtgcacctgtggcgcctgttccgccggctgggcgtgaagagccgcacgcaggcgctgcactatgcgcgtaccaatgggttgatttcaagcaactaggctcgcccccagtctgcgcgcacttcgtgtcgcttcgccaaccccctaccgggggcaacaccagaggcccggcgaagccggttcctcggtagagcttggctctcccccagtcttcgcgcacttcgtgtcgcttcgccaacccccttccgggggcaacaccaccggcccggcaaagccggttccgcggtgtttctggaaggaatcaaaccgcgcctcgtgcgcggttttttattggggcaagggtgtcagccgccggaggcgctgacgcgggcttgggcgacggcttcgtcggcgtcgtgcagtgcgacgcgaaacacgctgccgctgccgaggcgggagcgcacgctgacggggtggccgaggacgtgcgacaggcgggcgacgatggcaaggccgaggccgaagccgtcggaggtgccggcgtggtcggcgaccttgtagaactccaggaacacgtcgcgcaggtgttcgggcgcaatgccgatgccggtgtcccacacctcgatgcgcaggccgtcgcgcgtttgccgcgaggccagcagcacgccgccgtcggtggtgtacttgatggcgttggcaagcaggttgccgatcatgcggcgcacgcggatcgggtcggtgaggaagctgccctcggtcacgtgcacgcgaaaatcgaggccgcggctttcggccacggggcggtactgcagttcgaggtcatggagcagctcggccacgtccacgcgctcgatgtgcagccgcacctggcccgagtcgatgcgcgccagatcgaacatggagtcgaacagcgcgttcacggcatgcgtggcgcgaacgatcttgggcgcgagttccagcaccagctccggctcgttgcgcagccagtcggcgtacagggacaaggccagcacgggctggcgcatgtcgtgcgcggcgctggccaggaagcggttcttcatggccacggccgccaccgcggcctgccgctgctgcgtgagcgacttgatcaggatgtggttgtggaacagcagttccaggctgttgcgcgccgtctcgtggatgtggcgccccgcgcgcagcagcagaaaccaatgcaggatcggcaagatcggcatcaggaagccgtactggaaatgcggctccacgatgttgatgctcacgagccggatcagaaccgctccgagcatcgtgatgaacagcgtattgacgtagcgcttgagcagcggcgggtgcagcgccagcccgttgagcggaaaagtgccgacgccggccacgatgagccagctcatgaactggttgacctgcggcgtgcgctcgaagaacagcaggatcgacgcgccccagaccaccgcgctggtgctccagatgaaaccgtagcgctcggtgaactgctgctgcgcggctgcgctccggcccgcatagcgcacggcatagaccttggcgccccaggcacggcaagcggtggcaatgaagcctgcggccagccacgtgagcaactcccagtgcgggatgtagctccagttgaggccgaccatcaacggcatgagcgccgccgagaccatgtaggacccgcgtgcggaccgcatcagactgcggatcagctcgccgcgtacccacgattcagcttcatcggccgaagccgggaccggtgtcacgctcgcgatcgacgcattggccatgtggcgctgagccctctttttagttttcgactacaggaaccgcccgcaagttgcggggaatgaagaggtggcgatcttaacgggcggatgcggccttcccgggcatcggcacggcaccttgatgggccctgcgaacgaagcgcaaaggccgggaaacgaaaggtattgttttgccggcgcgggcggccgagcgaaggaagtcggcgggaagacaggaaaaaagacaggcaaaaaaatagcccctttgcggggccattctggaggagagggagggattcgaaccctcggtactatcgctagtacgcctgatttcgagtcaggtacattcgaccactctgccacctctccggtgctgtcgagcctgcgattctagcagacaaaaacgggggttttgaagccccggggccatcagccgcgcagcagttccttcccgcccaggtaaggccgcaacgcggcggggatgctgatcgagccgtcttcgttctggtggttttcgagcaccgccaccagcgtgcggccgaccgccaggcccgagccgttgagcgtatggacgagttcgttcttgccctgcgcgttcttgaaccgggcctgcaggcggcgcgcctggaaggcttcgcaattggacaccgagctgatctcgcggtacgtgtcctgcgccggcagccacacctccaggtcgtaggtcttggtggcgccaaagcccatgtcgccggtgcacagcagcaccacgcggtacggcagctccagcgcctgcagcacggcctcggcgtggccggtcatctgttcgagcgcttcgtagctcttctcggggtggacgatctgcaccatctcgaccttgtcgaactggtgctggcggatcatgccgcgcgtgtcgcggcccgcgctgccggcttcggagcggaagcacggcgtgtgggccgtgagcttgatcggcagctgcgcctcggccacgacctcgtcgcgcacgaagttggtcagcggcacttcgctggtgggaatgaggtagagcgccgaatggtcgggcgcgggttcgccgtcctggccgcccttcttggcggcgaacaggtcgccttcgaacttgggcagctggccagtgccgctcaaggtggcggcgttgacgatgtagggcacgtagcactcggcatagccgtgcttctcggtctggatgtcgagcatgaactgcgcgagcgctcggtgcaggcgggcaatcggccccttcatgacggtgaagcgcgagcccgcgagcttggcgcccatctcgaagtcgagccccagcggcgcgccaaggtccacatggtcctttggcgtgaacgccagcggcgcggcattggcgccggcgccgccctgggggctccagcggcgcatttcgacattggcggtttcgtcctcgccgaccggcacgctggcatgcggcaggttgggcaccgcgagcagcagcgcctgcagttcgggctggatttcttcgaggcgcctggattgcgattcctgctcggccttgagcgcgttgacttcggccatcagcgcatcggtcgattcgcccttggccttgagcgggccgatctgcttgttcagcgtattgcggcgggcctggatttcctcggtgcgggtttgcagcgtcttgcgctcggcctcgagcgtggtgaacgccgccacgtcgaggtagggctggtttttcttgcgtttttcgaggccggcgacggcggaggccaggtccttgcggagcagagtgatgtcaagcatggggggattttaggtgggcgtagcatcttcctccccacacctcaaccgaagggaaagagcgatgcaagcctatctgacattcaacggcaacgcggccgaggcactggccttctacgcgaaggcgctgggcggcaaggtcatcttcagcatgacgttcggcgaaagccccatgggcgccgaaacacccgccgcgtacaaggaaaagatcatgcacgccacgctggaggctcgcggccaccagctgatggcctccgacatgccgcctggcatgcccttcgagggccacaagggcttttcgctgtcggtgcagggcaacaacgtggacgaagggaaaaagctcttcgacgcgctggccgagggcggcgaagtgacgatgccgtacggcccgcagttctgggccgtcggcttcggcatgctgaaggacaagttcggcgtgccgtggatggtcaactgcgaaaaataaaaggacttcaggcgacggtggcggggtcgacgttcgcgccgcagacgatcaggcacaccttctcgccttcgcgcggcaggtaggcgccggtctgcagcgccgccagcggcagcgcggcggccggctccacggcgagcttcagttccttccacagccactgctgcgcggcgcggatggattcgtcggacagcagcagcgcgtcctgcacgtacttctgggtaatttcccacgagatggcgccgatgcgtcgcgcgccgagcgaatcggccgcgatgccgcccacatcgacgtcgaccggctcgccggcctcacgggcgcggaacagcgtgggcgccttctcgggttcgagcgccaccacgcgggcgcgcttttggaaccagccggcgaggccgccgatcaggccgcccccaccgacgctcacgagcaccgcgtcgggcaggccgccctcggcttcgatttcgacccccagcgtgcccgcgccggccacgacttcgggctggtcataggcatgggtcagcagggcgccggtttccttctggcgcgtgaggcaggcagccagcgcgtccgggtacagctcgccgacaacgatcacttcggcccccagtgcccgcagccgcgcacgcttggcttcgggcgagacgccgggcaggaacacctggcagcgcacgcccagcgccttggcggccgccgcggtggcaatgccggcattgccgcccgaggccacgaccacgccgctcgcgggaatgtcgttggccagcaggcggttcatcatgccgcgcgccttgaagctgccgctcacctgcatgtgctcgagcttgagccacagctccacgccgggcacttcgatgccgaaagcggaagccggcaatttccagagcggcgtctggcgcaggaaggtgccggagcgttcgcgcagccggcgggaggcgccgtctatttcaaggcgccagtcggtgttttcgttggtcaagagatatgtccaggaggaggaatgtcgtcgagcttgaggcccttggggagcggaaacttgatggtttcctcgatgccgtccatcttgcggaccgacaccgcgccgagcgccctcacccgctcgatcacctcgcgcaccagcacttcaggggccgaggcgccagccgtgaggccgatgcggcccttgccctcgaaccattcgggcttgagctcgtcggccgaatcgaccatgtagctttcggtgccgaggcgctctgccagttcgcgcagccggttgctgttggagctggtggggctgccgaccacgatcaccaggtcgacctgcgggctcatgatcttgaccgcgtcctggcggttctgcgtggcgtagcaaatgtcctgctgcttgggctcgcgcaccttcgggaaacgcgcgcgcacggcggccgcgatttcggccgcatcgtccacgctgagcgtggtctgcgtgacgaccgcgagcttgtcggtctgcgcgggcgccaccttggccacgtcttccacgtcttccaccaggtggatgccgctcgaaagctggcccatggtgccttcgacctctgggtgccccttgtggccgatcatgatgaattcgtagccttccttggcgagcttggcgacctcgacgtgcaccttggtcaccagcgggcaggtggcgtcgaaaatttcgaagccgcggtcgcgcgcctcctgctgcaccgccttgctcacgccgtgcgcgctgaacaccagcgtggcgccgggcggcacgtcggccaggtcttcgatgaagatcgcgcccttggccttgagttcgttcacgacataggtgttgtgcacgatctcgtggcgcacatagatgggcgcgccgaacttggcaagggcacgctcgacgatctcgatggcgcggtccacgcccgcgcaaaagccgcgcggttcggcgaggatgacttcttcgaggctcgggttcatagcactccgatcaggcgcacctcgaaggtcacgggctgtccggccagcggatggttgaaatcgaagcgcaccgcggtctcgttcgattcgaccaccgcgcccgcgtagctgcccgtgccgtcgggcgtgggaaactgcaccacgtcgccgaccgcgtattgctcgtcggggtcgcccatctgcgccagcagcttcctggccacccattgctgcatctcggggttgcgctcgccaaaggcctcgccggcgggcagctcgaaggtggcgtgcgtgccctcttccaggcccatgagccgctgctccatggcgggcgaaagctcgccggtgcccagcgacagggtcgcgggcttgtcggtgaaggtgttgatgatgtcgcccgccggaccggccagccggtagtgcagggtcaggaacgagccggaagtcacaacgtgggacatgggtgcagtggaggtaggcaaagacaaggtgggtgtcccgataaactggactgcattttaaggagcgggcgcgttcgcctgccctttcagggtttcaccaggtttccgatggcattcaaggatctccccgcccacgcccgcccgcgcgaaaaactcatcgcgcggggtgccggcgcgctggccgacgccgaattgctggcgttgctgctgcgcacgggcgtggccggaaaaaacgtgctccagctcgcccaggagctgctcgaccacttcggaggcctttcggggctgctccagaccggcgccgaggatctgaaggtgatcaagggcatgggcggcgacgccaagcgcgccgaactcatcgcagtgctcgaactggcgcgccgcgccatggccgagcgcctcaaggagcgcgcggtgttcgactcgcccgaggcagtcaagcagtacctgcagctgcacatcggttcgcgcgcctacgaggtgtttgcggtgctgtttctcgacgcgcagcaccggctgatcgtgctcgaggagctgtttcgcggaacgctcacccagaccagcgtctacccgcgcgaagtggtcacgcgcgcgctgcaccaccgggccgcggccgtggtgctgtcgcacaaccatccgagcggcagcatcgaaccctcccgggccgacgagtcgctgacgcaaacgctgggcgctgcgctcgcgctgatcgacgtgcgcgtgctcgaccacgtgatcgtcagcgccggccagagcttgtcaatggccgagaaagggctgctctgatggcttcccgcacgccgcccatcaagaacctggcggacctgaagcaggtgcagcgcgcgctggccgaaacccgcgagcgcgaagcggccgccgcagccgccagggccgctgcggaacgcaagcgcgccgccgagaaagacctgttcacgcgcgccatcggtgccacagagccgcttcgccgcaaggccgcggtgccgctcgcgcccgagccgccggcacccatccccgtgcagcaccagctcgacgaacagcgcgtgctgcgcgagtcgctgtccgacgaattcgacgtgaccaccctgctcgacgtggacgacgccatgagctttcgccgaccgggcatcggcaccgacgtgaccgcgcggctgcgcaagggcgactggagcatccaggcacaggtcgacctgcacggcctgcgcagcgacgaagcgcgcgaggcgcttggcggcttcatccgcaacgcgtacaagcaagggctgcgctgcgtgcgcgtggtgcacggcaagggcctgggctcgccgggcaggcagccggtgctcaagaccaagacgcagcgctggctgatccagaagaacgaggtgatcgccttcgtgcaggccaagcccgccgaaggcggagccggcgcgctggtggtgctgctggccccggctcggcgttgaccgcggcaggccgctaggacaagtggttcttcagcgggatcgacgcatccgccaccgccgccgcatcggggctgcggcccgcttcgagcagcttgcggctcatcatgtgatcgaccggcgcattgaccgattcgacgcatgcgagctgcccgtcgacataatggaacagcgagaacgcatcgggcttggggccggcgcggcgcacgctggacaggcccggcgtgccctccgccggcatcaggcccgccatctgcaggcgcatgctgccctggtcggaccagaaccacgccacgacgtcgtgcgggcgcggcgcgccggtcagcgtggccacggccgtgcgcgcctggtcgttcgcgttctgcaccgattcgagccggagcgcgcggcctgcgcggcgatcgggaaagcgcgtgcagtcgcccacggcgagcacgtcggccgcgctggtctgcatgtggccatcgaccacgatgccgtcggcgcactcgatgcccgcggcctgcgccagcgccgtctcgggcaccgcgccgatgcccagcagcagcaggtccacaggctgcttcacgccgttgacctggatcgacagcagccgctcgccctcgacctcgaacgcgccggtgcgtgcgccgagcacgatgtcgatacccgctgcgcgatgcgtcgcgagcacgtgcgccgacagctcgggagacacggcgcggcccagcagccgcggcgcgctctcgatcacctgcacgctcttgccgagcgccttggcggtggccgccacttcgagcccgatgaagccgccgcccagcaccgtgacctgctgcgcagcagccagccgcgaacgcaggcgatgcgcttcgtcggccgcgcgcaggctggcgacgttctccagccccggcttcaggtcgggcatctggcgcgcacgcgtgccggtggccagcaccagccgctcccacggcaggatcgcgcccgaacgcaaggtgacggtgtgcgcctcgcggtcgatggcgaccgctgcgtcgcccaggtgcagcgtgatgcccgcttcgcggtaccagtcagcggccttgtgcggctgcgtggtttcctcggcgctcttgagaaaggccttcgacagcggcggccggtggtacggctcgcaagcctcctcgcagaccaggtgcacgcgagcgccctgcccggcttcagccagccccgcgcaaagctgggccgcagcgtggccgccgccgatgatgacgatggaattcatggaagaggatctttcggagtcgttgtctatcttgttattcgccgcgattgcgcatccagtcggccgtctggaagaaagagtcacgcaagcgcgcgcgcaatccctcgggcacgccggtctcgcccatggcctggtccatgcaggccagccactggtcgcgctccttgatgccgatgctgtggccgccaatgctttgcggcagatggcgcgcgcgcagcatcggatggccgaagcggtcggtgtagtgctgcggtccgccgagccagccgcacaggaaccagaagaggcgctggcgcgcgttgtcgaggctggtgccgtgcaccgcgcgcagttgcgcataggccggctcgagttccatcaggtcgtagaagcgatcgaccagcgcctgcaccctgggttcgccgccgatccattcgaagggtgtgtcgacgggtggcttttcgtgaatctgcatggcgggagtatccctctgtgcgcctgtcaggcctgcacgaggttcggaattcccacgtcgggattcacgtcagcctcgtagtccacgccgtcgatgccgaacccgaaaaggcgcaggaactccgccttgtagccggcgagatcggtgagttcgtggacgttctggctcgtgacctggggccagcgcgccatcacacgcgcctgcacttgcggagacagttccttgtagtccgcgcgcagccggccctcctcgtcgaggtgcggcgcgctgccgtagaggctgtcggcaaaaagcccatggacctgctcgatgcagccctcgtgcgtgccctcggccttcatgaccttgaacagcagcgacaggtacagtggcatcaccggaatcgccgagctcgcctgcgtgacaaccgccttcagcaccgagacgcgcgcatcgccgcccttggcggccagcccggcgcggatgccgagcaccttctggtcgaggtccttcttggcggcgccgatcgagccgttccagtagatgtcgtgcgtgatccgctcgcccaggtaggtgaaggcggtggtcttggcaccgtcggccagcacgccggcggcctgcagtgcgtcgatccacatctgccagtcttcgcctcccatcacggccacggtgtcgtcgatctcttcctgcgtggccggctcgagcacggtgtccttgacgacttcgttgtcggtgtcgaggccgcgcaggctcacggccttgccgatgggcttgagcgtcgaattgaagacctcgccggtcttcggatgggtgcgccgcggcgcggccaggctgtagacgacgaggtcgacctggcccaggtcctcgcggatcgcatcgatggccttctgcttcacgtcgtcggaaaaaccgtcgccgttgatgctcttggcgtagaggcccccttgcgcggctgcgcggtggaaggcggccgagttgtaccagcctggcgagccgggcttgttttcgctgccgggccgctcgaagaagacgcccagcgtgtcggcgccgcagccgaaggccgcggtgatgcgtgcggccaggccgtagccggtcgatgcgccgatgaccagcactctcttcggcccgcccgcgatccttccctcggccttgacgtagtcgatctgctgcctgacgttggcctcgcagcccgcgggatgggtcgtgacgcagatgaagccacgcacgcgcggtttgatgatcatgaagagctcgctgaagatggatgccgcgggggccggggcgcaggtttttgcgccgcgaatttaacccaggccgtgccagggccgatcccgcaaggccatatgcatatgtcgattgaggatttaataatctcgggttttgttgatagggtccagccctttgtcttttcatccggagtgagaacaaccatgcgccacaccctgctcgccgcggccctcgccgcctccaccctgctgacgggcatcgccgcccatgcagaccagcttgccgacatcaagaagaagggcgaactcgtggtcggcgtgctcggcaccgacgagcccgccactttcatcgatccgaagacgcgccagatcgtcggctacgaggtcgatctggtgaacgccatcgccaagaagatcggcgtgaagccggtcctcaagcagatcgcggtggccgcgcgcattcccgagctgcagcagggccacgtcgatctggtggccgccggcctcacccacaacaaggagcgggaggcgcagatcgacttttcgctcaccaccttcgtcacgggccagaaggccatcgtgaagaaggacagcggcatcagcgacgtgccccagcttgccggcaagaaggtgctgaccatccgcggcggcacgcaggaacccaatatccgcaaggccgtgcccacggccgaggtcgtgaccttcgacaccagccagcaggccttccaggcgctgcagcagggcaagggcgtgggctacgtggacgacgaggccgcgctgctgcgcagctacgccaagctgggcccgcagaaggcccagtacgtggtgctcaagcagaacctgagcaccgaggcgctggccatcggcatcaagaagggcgagagcgggttgaaggccgtggtggacgagaccctgcgcgagctcgagaagtcgggcgaagcgcagaagatcttcgtcaagtggtacggcccgaacacggcttccggattccagacgcgcgacttcaagctcgagagcgacaagatcgactgatttggtatttctccttccccctctgggggaaggcagggatgggggcaagcggcctttgaacaggccgcggcgcatcgatcgccgtcgtgcccccaccccaaccctccccccgcgggggagggagccaaattccctgcgacgcggtgatactgtcgccccccatgcccctgttcgactattcgttgctgctgaccggcaagtaccacgacatgctggtcgcgggcctgctgctctcgctgcagctgctggcggcctcgctggtgctggcactgcccatcgcgctggtggtggcgctgcttcggctgtctccgctcgcaccgctgcgctggctcggtttcgcgtacgtggagacgatccgcaacatcccgctgctcgcgcacatgctgttctggtatttcggcgcgcccgagttgctgcccgagggcatcaagcaatggctctatgcggggcatatcgaggcctacagcgccatcatcgcgctgtcgctctatacggccgcgttcatggcggaagacatccgcagcggcatccgcgcgattcccaccgtgcagttcgaggccggccgcgcgctgggcttcgggtttctgggcaccatgcgccgcgtggtgctgccgcaggcgctgcgcgtgacggtgccgccgctcatttcgcagacgctgagcctctggaagaacacctcgatcgccaccgtgatcggcgtggccgagctgatgtaccaggccgggcaggtcgagagcgcgacctttcgcagcttcgagtcgttcgcgttcgcgagcgcggcgtacctgacggtgtcgctcgcgatcacggggctggccacttggtaccaccatcggttcccggtgcggaccatctagagaagtgttgatgagatgctagagatcatcaacgactactgggtctactttctcatcgggcagtacccgaacgggccgctgggcgggctggtgctcacgctgctgctcgcctcgtgcggcctggtgctcgcgctgccgctgggtatcgtgctgggccttgcgcgtgtgagcccgtggcgctggttgcgctggccggtcacgggcttcgtgttcgtggtgcgcggcctccccttgctgatggtgattttctgggcctacttcttcctgcccagcgtgacgggcgtgaagaccgaccagttcaccaccatgctgatcgcgctcgtggtgttcgatgcggcgtaccttgccgagatcgtgcgcgccggcatccagggcctgccgcgcggccagatggaaaccgcccgcgcgctgggcctggactacggccgcgcgatgcgcctcgtggtgctgccgcaggcactgcgcagcatgctgccctcgctggtgaaccagttcgtctcgaccatcaaggaaacctcgctcggctacatcatcgggttggccgaggtgtcgttcatcgcgacgcagatcaacacgcaggtgttcaccaagccggcgcagatctacctgatcctgggcctcacctatttcatcctctgcttcgggctatcgcgcttcgcctactggctcgaacgccgtctcgcgcggcgcggcatgtccatcgccaaccccacttcggcccccaaggtatccgcatgatcgaactgcagaacgtcaacaagtggtacggcagctaccaagccctggtcgacatcaacgagaccatccacaagggcgaagtggtcgtggtgtgcggaccgtcgggctcgggcaagtccacgctcatccgcaccttcaaccggctggagccgatccagtcgggccgcattcttttcgaaggcaaggacatccatgcgccaggcaccgacgtgaatgcattccgctcgcgcattggcttcgtgttccagcagttcaacctgttcccgcatctcacggtgctgcagaactgcacgatggcgccgatgcagctgcgcggcctcacacgcaaggaggccgaagagcgcgcgatggcgctgctgcagcgcgtcggtcttgcgaacaaggccaacgcctggcccagcgagctctcgggcggccagcagcagcgcgtggcgattgcgcgcgcgctcgccatgcagccgccgctgatgctgttcgacgaacccaccagcgcactcgaccccgagatggtgggcgaggtgctgctggtgatgcgcgacctcacgcgcgacggcatgacgatggtctgcgtgacgcacgagatgggctttgcgcgcgaggtggccgaccgcgtgctgttcatggacgagggcaaggtgctcgaacgcgccacgcccgacgactttttcaaccggccgcagcatccccgcgcgcagcagtttctttcggacatccgctcgccctttgcgcgcgacgcatgacatgctctccatgcccatgaccgacacgcagacgcttcccgtgatcgatgtcgccccgctcgtggccggcgcgcccgagcgcgacggcgtggcggcgcaggtcggcgccgcatgccgtgcgcacggcttcttctacgtcaccggccacggcgtcgatgtagcgctggtgcggcggctcgaagacctgagccatcgattcttcgaactgcccaccgagacgaagatgcaatggcgcatggccctgggcggacgggcctggcgcggcttcttcccgctcggcggtgaactcacttcgggccggcccgactggaaagaaggcctctacctcggcaccgagctacccgcctcgcacccgctggtgcagacgaagacgccggtgcacgggcccaaccttttccccgacgtgccgggcttgcgcgaaaccatcctcgactacatggcggccgtcacgcagctgggccaccggctgatggagggcattgcgctgagcctcggcctgccggcggcgtacttcgccgagcgctacacggccgatcctctcatcttgttccgcctgttcaactatccgtcgcagcccgtgcccgagggcctcgacgtgcagtggggcgtgggcgagcacaccgactacggcctgctcaccgtcctgcaccaggacgacgtgggcggcctcgccgtgcacacgccgggcggctggatcgacgcgccgccgattcccggctccttcgtctgcaacatcggcgacatgctcgaccgcatgaccggcgggctctacaagtcgacgccgcaccgcgtgaggcgcaacacctcgggccgcgaccggctgtcgtttccgctattcttcgacccgaatttcgaggcgcgggtgcagcgcatcgaaggcctcgcgggcgcggaggcgcgcgacgacagcgccgagcgctgggaccgcgccaacgtgcacgccttcagcggccgctacggcgactacctgctcgccaaggtgtcgaaggtgtttccgcagttgcgcgacgaggtgctctgaagcgctctcgatggagggccggcgggggcgtcgatgaattcatcttcccagttgccgacatccgcatcgggatcggaaatgggcacgagcttgtcgctgcggcaatagaaggtccagccctcgaacagcacgtcgtagtaagtgccgggcaggtagcgctcgctgggcgcctcgtagagcgccgagaccacctccacgatgcgtccgacggcgcgctcggtcatcggcgacgcgaggcagctgtcgagcacgtggcagagggtcccgatcttgatcatgtgcgtatcacctggccgggaaaccaccgcggcacatgggcgagggcctcgtgaagggagtcgagcacatggaacgcccgctcgacgatcgacgcgggcgggtgcttgagatccggcacgatcacgactcggaggcccgctgccagcgcggccttggcgccgttctcgctgtcctcgaaggccacgcattccgccgggtcgacgcccaggcgcttcgccgcgagcaggtagagcgccggatcgggcttcgcgcgtgccacctcgtcgccacctgcaaaagcgtcgaagtgatggagcacgtcgaggctgccgaggcaggcctggatctgcccactggtcgaagacgatgcgacggcgcaacgcgttccgcgctggcgcagcgcgcccaggaactcggccgcgccgggcttgatcggaaacatcggaaggccgtccgcccgctgcagttgcagcagtttgcgaacgtgcccgatggcatggcgataggcttcaggcccgccgagcagcgtgccgagaatcagctcggactccgcggtggcaaggcccaccacctgcagatactggctgtgcgaaagctcgatgtcgagcgtgcgggccgcttcgatccaggcagccatgatgggccgctccgaatcgatcagcagcccgtccatgtcgaagatggcggcggcgaacatggagcgaatgctaagccagcacgcgcggccggtgttgacccggtcagtcgcgcaccagcgcccggttcagccccagcgccgccagcgtgccgaccgcgcccgacagcagatacacgctcacataggccagcccgaaattcgccgacaggcccagtgccaccagcggggcaaaggcggcaccgatgagccacgccaggtcggccgtcagtgcggcaccggtgtagcggtacttgggctcgaagttcgaggttacggcgccggccgcctggccataggaaagccccagcagcacgaagcccagcagaatgaagatgtcctggccgatgcggccgccgtcgagcagcgtgggggcaaaaccactgaacaccgcaatcagcgcggccaggccgcccagcgtgaaacggcgccccacgcggtcggcgatcacgcccgaggccacggtaccgccggcgcagaacaccgcgccgatcatctgcaccaccaggaactcggtgatcgactggtcggaatacagcgtgatccacgacagcgggaacaccgtgatcaggtggaacagcgcatagctggccagcgcggcgaaggcgccgatcagcaggttggcgccctgggagcgggtcagctcgaccacgctggtgggttgcagctcgcgctcttcgagcaggcgggaatactcttcggtggccaccagcctgaggcgcgcgaacagcgccaccacgttgatcgcgaaggccacgtagaaggtgtagcgccagccccaatcgagaaagtccttgatcgagaggctcgcgtagaggtaggcgaacagcgcactggcaatgaagaagccgatgggcgcacccagctggcccagcatggcataccagccgcggcggttcggcggcgcgttcagcgccagcaacgagggcaggccgtcccatgagccgccgagtgccaggccctggcagaagcggaacaccgacagcagcacgatcgccgtgaacccgatgctctcgtagcccggcaggaaggcgatgcccgcagtggaggtgcccagcaggaacagtgcgatcgtcagtttggtctcgcgcccgaatcgtcgctggatcgccatcgagatgacagttccgaacggccgtgcgatgaacgcgaacgaaaagaccacgaaagcgtagaggatgccctccaggcgctgttcgaacggaaaaaatatgtacggaaacaccagcaccgaggcaatgccgtagacgaagaagtcgaaatactcggaggcgcggccgatgatcacgcccaccgcgatctcgcccggggcgatgtgcgagtgatcggcgtcgctctggctggcgccgtttccggacgtgttcggcacaggctgtgcgccttgcggactgatgctggacgtcgtcgtcattgcgttttgtaattcgggtgtcaccggcagtgacaaaggtagaccattgaacagaggttccaagcgtctcaccgaatggggattcccgccataggacaaaacgtccaataggcggcgggcgcctttggtcgtagattgtggagtctttgcgcagcccacgcacctctttctttctcttcggcatgcccaccctccactcccttcgccgatggctcctgttgctccccctcgccttgctggcgggctgcaacacggtgctcatgaacccttccggcgacatcgccaaccagcagggacgcctgatcgtcgtctccaccgtgctgatgctgatcatcatcattccggtgatcgcgctgaccatcttcttcgcctggcgctaccgccagtcgaacaaggaggccgactacagccccgactgggaccactccacccagctcgaactcgcgatctgggccgcgccgctcctgatcatcattgcgctgggtgccatcacctggatcagcacccacacgctcgacccgtaccggccgctgagtcgcctggacgccgagcgcccgattcccgccgaagccaagccgctggtggtcgaagtggtggcactcgactggaaatggctcttcatctaccccgagcagggttttgccacggtgaacgaaatggccgcgccggtcgaccggccgatcactttcaagatcacggccacctcggtgatgaattctttcttcattcccgcactggccggccagatctacgccatgccgggcatggaaaccaagctgcacgcggtcatcaacaagccgggtgagttcgagggcttctcggccaactacagcggcgcgggcttctcgggcatgcgcttcaagttccacggcctgaccaacgacggctttgaagagtgggtcaagaaggccaaggccggcaaggacggcgaactcagccgcgaaacctacgtgaagctcgaagcgccaagcgagcgcgaccccgtgcgccactacgccagcgtggcgcccgacctgtacgacgccatcctcaaccgttgcgtcgaccgcaacaagatgtgcatgaagcagatgatggccatcgacgccgagggcggcctgggcaagcccggcgccttcaacgtggccaccaaggcaaccgcctggcagcccgacagcatcaattccagttcgccgacgcgcaagtacgtcacggcgatgtgcaccaccgaagaatgacgatgttcgagaaccttgacctgacgaagctcatcttcggccgcctcacgtgggaggcgattccctaccacgagcccatcctgcttgcgacctttgcggccgtggtgctgggcggccttgccgtcctcggcgccctgacctacttcaagctgtggggcaccctgtggcgcgactggatcaccagcatcgaccacaagaagatcggcatcatgtacatcatcctcgggctggtgatgctgctgcgcggctttgccgacgcgatcatgatgcgggcccagcaggccatcgccttcggcgacaacgccggcttcctgccgccgcaccactacgaccagatcttcaccgcccacggcgtgatcatgatcttcttcgtggccatgccgctggtcacgggcctcatgaacttcgtggtgccgctgcagatcggcgcgcgcgacgtggcctttccgtttctgaacaacttcagcttctggatgaccaccttcggcgcgggcctggtgatggcctcgctcttcgtcggcgagttcgccaagaccggctggctggcctatccgccgctgtcgggcattctcttcagccccgacgtgggggtcgactactacatctggtcattgcagatagcgggggtagggaccctgctctccggcgtcaacctgctggccaccatcgtgaagatgcgcgcgcccggcatgacgatgatgaagatgccggtgttcacctggacggccctctgcaccaacgtgctgatcgtggcggctttcccggtgctgaccgccgtgctggccctgctgtcgctcgaccgctacgtcggcaccaacttcttcacgaacgacctcggcggcaacgccatgatgtacgtgaacctgatctggatctggggccaccccgaggtctacatcctgatcctgccggccttcggcatcttctcggaagtggtctccaccttctcgggcaagcgcctcttcggctacgcgtcgatggtgtacgccacggtcgtgatcaccatcctgtcgtacctcgtgtggctgcaccacttcttcaccatgggctccggcgccagcgtgaactcgttcttcggcatcacgacgatgatcatctcgatcccgacgggcgcaaagatcttcaactggctcttcaccatgtaccgcggccgcatccgcttcgagctgcccatgatgtggaccatcggcttcatgatcaccttcgtgatcggcggcatgacgggtgtgctgctcgcggtgcctccggccgacttcgtgctgcacaacagcctgttcctgatcgcccacttccacaacgtgatcatcggcggcgtgctgttcggcatgctggcgggcatcacctactggttccccaaggccttcggctacaagctcgatccgttctggggcaagtgctcgttctggttctggatcgtcggcttctggttcgccttcatgccgctttacatcctgggcctgatgggcgtcacccgccgcatgagccacttccaggacatgtcgctgcagatctggttccaggtcgccgccttcggcgccgtgctgatcgcgctgggcatcgcgtcgttcctgatccagctggtggtgagctacatccgccgcgattcgctgcgcgacaccacgggcgacccgtggaacggccgcacgctcgagtggtcgacctcgtcgccgccgccggcctacaacttcgcgttcacgccgcgcatccacgacaacgacgcctggaccgacatgaagcgccgcggctacgcgcgcccgctcgaaggcttcacgcccatccacatgcccaagaacacggccgccggcttcgtcatcgcggccctggcagcgacctgcggcttcgcgctgatctggcagatgtggctcgtagcgggcatcggcttcgtcgccatgctggccgccgtgatcatccataccttcaactacaagcgcgactactacatccccacggaagacgtcgtgcgcaccgaggccgaacgcacccgcctgctgggagccgcccatgtctgataccaccgctctgcaaactcccgcgggcgtccacgcccacagcgaccagacgggcaagccgcccgtgttcgagctgttccacgtcggcaacgaccaccatcccgagaacggcacgctgctgggcttctggctctacctgatgagcgactgcctggtcttcgcctgcctgttcgcggtgtatggcgtgctgggccgcagctacgcggccggcccctcgggtgccgacctgttcgacctgccgctggtggccatcaatacctcgctgctgctcttctcgtccatcacctatggttttgcggtgctcgagatgcaacgcaagcgcatgggcggcacgctggtgtggctggccatcaccggcctcttgggcgcgggcttcatcggcctggagctgtacgagttcgcgcacctcctccatgaaggcgcgggcccgcagcgcagcgcgttcctgtcgtcgttcttcgcactggtcggcacccacggcctgcacgtgaccttcggcatcgtgtggctcgtcgtgctgatgatccagctgcccaagcacggtttcaccgccgcaaaccgccgccgcctgatgtgcctgtcgatgttctggcacttcctggacgtggtgtggatcggcgtcttcactttcgtctacctgatgggatcgatgcaatgaccgcccccaccaccaacgccgcgcacagccatgatgcgcacgacgaccatcacgacgacggccccgtcagccacagcaccttcaagggctacatgaccggcttcgtgctggccgtgatcctgaccgcgattccgttctggctcgtgatgggcaaggtgctcaccagcacgcacaccacctcgctcgtcatcctgggctttgccgcggtgcagatcgtggtccacatgatctacttcctgcacatggacgccaagtccgagagcggctggaacatgctggcgctgatcttcacgatcgtgctcgtggtgatcacgctggccggatcgctctgggtcatgtaccacatgaacgccaacatgatgccgatgtcggtgcacgacatgaagaacatgccttgacgccaccgccgccagaccacagcacccaaagcctcgacacaccggccggccgccagcgctccgcggcggcccgggcggcgctggcggtctgcgcggcactggcctttgccggcttcttcgcgctcggcacctggcaggtcgagcgccgggcctggaagctcgatctcatcgcccgcgtcgaacagcgcgtgcacgctgcgcccgccgatgggcccggccccgagcgctggccgcaggtcaacgcggccgccgacgaataccggcgcgtgcgcctcaccggcacctttctccacgacaaggaaaccctggtgcaggccagcacccggctcggcgccggcttctgggtgctgacgcccttgcgcgctgccgatggcagcatcgtgctggtcaaccgcggcttcgtgccgcccgaagcgcaggggcgcccggcgcgtgccgccaccgagccccagggcgaaaccatggtgaccgggctgctgcgcatcaccgagcccaacggtggcttcctgcgcaagaaccagccaggcgaagggcgctggttctcgcgcgacgtgcaggccattgccgcggcacgcggcctcggcaacaacgtggcgccgtatttcgtcgatgcggatgccgcgccctcttcgtccagcgcggcccccgcctggcccgccggcggcctcacggtcatcgcctttcccaacagccatcttgtctacgccatcacctggtacggcctggcgctgatggtcctggccgccgccgggtacgcctggcgcgaggggcgcaggcgccgcagcggcgaaaatgccgccaatgcccaagccagcgcccgtccagatgcccgccgcgactgagcctctcgccgtcgcgggagaactgcacgcgccccgcgcgggcgtggcaagcctggacaacgccaccggccacaagaacatgcagcagctgatccagctgcgctggttcgcagtggtcgggcaggtggccaccatcctgctggtgcactacggcttcggcatccggctgccgctggaccacatgctgcaggtgctgacctgccttgcgctcttcaatggcgtgagcctgctgcgctcgcgcagccttcgccgcgtgaccaacggcgaactctttctcgcgctcttggtcgacgtggccacgctcaccgcacagctctacctgagcggcggcgccaccaatccgttcgtctttttgtatctgctgcaggtcatcctgggcgcggtgctgctcaaggcctggtcgacgtggaccatcgtcgtcgtcaccagcctctgcttcgcggggctggcgcttttctcgcgcccgctcgcgctgccgctcgaccacgaccgcgggctctggagcccgtacgtgcagggcatgctgatctgctttgcgctcaacgcggcgctgctggtggtgttcatcacgcgcatcagccgcaacctgcgcgcacgcgatgcgcggctggccgacctgcgccagcgcgcgtcggaagaagagcacatcgtgcgcatgggactgctcgcatcgggcgccgcgcacgagctcggcacgccgctggccacgctggcggtgatcctcggcgactggcgtcggctgccgcatttcagctccgaccccgagctgctgaccgaagtggccgagatggagctgcagatccaacgctgcaagagcatcgtgagcggcatcctgctgtcggccggcgaggcgcgcggcgagtcgtcggaagagaccacggtgagcaccttcctcgacgagctggtcgaggaatggcgcaccacgcggccggtcgaagacttcgactacgacaaccgctttggccaagacctgcccatggtttccgactcggccctgaagcagatgatctgcaacgtgctcgacaatgcgctggaagcctcgccgcactggctgcgcttcgaggtggcgcacgacgccgacgcgctgactctcaccgtgaccgatgccggcccggggttcctgccgtccatcctgaaggagttcggcaagccctaccagtcgagcaagggacggccgggcggcgggctcgggctgttcctggtggtcaacgtggcgcgcaccctgggcggccgcgtcgcggtgcacaaccggcccgaaggcggtgccatcgtggccatcacgctgccccttgcggcgatcgtgctggaagaagaggaagaagaagaagccggcgaagagacgccagccatcgacgccatcgaaaaaacgaaagcccatgacggaaaccgctgaagccgagcgccagttgctgatcgtcgaagacgacgcggccttcgcacgcacgctcggcaagtcgttcgagcgccgcggctacgcggtcacgcacgcgagcaatgccgaagaagtcgagaccctgctgcagacgcatgcacccggctacggctatgccgtggtcgacctgaagctcaacggcgaggcctcggggctggcgtgcgtgcagatgctgcaccggcacaaccccaagatgctgatcgtggtgctcacgggctttgccagcatcgccacggccgtcgaggcgatcaagctcggcgcctgccactacctggccaagccctcgaacaccgacgacatcgaggccgccttcggccgcgccaccggcaccaccgaggtggaactgaccaaccgatcgacttcgatcaaaacgctcgaatgggagcgcatccacgagacattggccgaaaccggcttcaacatttccgagaccgcgcggcgtctcggcatgcatcggcgcacattggcacgcaaattgggcaaacagcaggtcaagtaacatgacttgccggcttcacgaaattccgcggaaccaattccaatccaggagattctgttaccaatgacgaatcgacaaccgatgcagttgcagcaagccattccagtccaagcggacaagcggcctccgctggcccgcgaccagaccacgctggaagaaatcttcaatgcattgagccacggcctcggcctgctacttgcgattgcctctctgcccatcctggtctacagcgctgcccagaaggggcaagccgcgagcgtcgtcggcgcatcgctctttgcgggcacggccatcgtgctgtacctgatctccacgctgtaccacgcgctgcccatgggcagggccaaggcgtggttcaaccggctcgaccacgcggccatctaccttttcattgcgggcagctacatgcccttcctgttcggcgtgctgcgcgggccctggggctggaccctgttcgcagcggtctgcgccgcggccgcgctgggcgtgggtgccaagctgttcaaccggctgcggcatccgctgtggtcgaccggcctctacgtggggatgggctggatggcgttgatggcggcggtgccgctgtacgaacgcatgtcgcccgcggggctggggtggctcgtggccggtggactcttctacacggcgggtgccgtggtcttcctgttcgacaacaaggtgcggtttgcgcactttgtctggcacctgttcgtcctggcgggcagtgcgtgccatttctttgcggtgctctggcactcgcacgggtgatctttttttggccggttccgttcagggcgtgtgcacaggccaccgggtactcccctccgcgaatgtcccccgccttcggctcctcctttatttcgctgcggggagcacccggcgccctgtgcacaccaagcgccgtgcttgttccacccgatcaaccactgctctgtccaacgcccccgctggcggggtgccttgcgcagcgaaataaaggaggagccgcaggccgggggacattcgcggagaaaggtactccgtcggcgggagcgccgccctgaagaacactgccttcagtagtgcggcggcagctcgtcccggagattgcgcgccgccccctcctgccccgcgttctggctttgctgtttcaactgggtgacctgaaggaccaagctgtcgatctgctgctgttgacggtagatcgtcatgttcagctgctcgagcaggtcctcggcatagctcgacttgatctcgagctcggtcagccgttctgcgagtttgttcggtggatattccatgccgctattggacaggaagattcccctactcactccgccgcccgccgcagcgtatcgaccaccggcctgcgcagcacgtcgcgcagcccccaccagcctgcggacagcgccagcaccgcgcccgcgagcgcaccggccaccggcacgatgggggacgcggtccaggtgaagtcgaacacgtagcgtgccaggccccagccgatggccgaggccacgatgctcgccaggaagcccgcgagcaagcccacgcccacgagttcggcgcgctgcacctggcgcagcaggctggcccgcgcacccaccgcgcgcatcaccgcgaactcgcgcgcgcgctcctcacgcgtggccgtgaccgcggcaaacaacaccaccagccccgcggcgagcgtgaagccgaacaggaactcgaccgcgcgaaccacctggtcgagcacgcgctgcacctggttgatggtggcgctcatgtcgacgttggtcacgttggggtagctgcgcaccagcgcgttgtcgaagccccgggtttcgggtgcgcggaaggcgcccatgtaggtcacgggcacgtcgggcaacgcggccaccgtgtacatcacgaagaagttggcatgcagcgagccccagtcgaccttgcgcagcgatgtgatgcgcgcgtcgttctgcatgccgccgatgtcgaagcgcatcgtgtcgcccaacttcaggccgagggtctcggccaggccttcttccacgctcacttcgcccggcgcatcgggcttccactcgcccgccaccacggcgttgtgcggcggcgcctgcacgctgttgctgaggttgaactcgcggtccaccagccgcttggcgcggtcttccacgtagtcgtcgggcgacaccggcttgccgttcacggccaccagccggccgcggatcatcgggtaccagtcgaacttgctcacgccggcatcgcgcagcgacttctggaacgcggtgctctggtcgggcatgacgttgatcacgaagcggttgggcgcatcgggcggcgtggccttgcgccagctcgcgaccaggtcggtgcgcagcagcaccagcagcaccagcgccagcaggcccacggcaagtgcgctgacctgcaccaccgcgtaggccgggcgcgccgagatctggcgcgtggccagcaccagccagcgcggggcggtggtttcattgacgctgcggcgcagcaccttcaccgcgagccagctcaggagcgcaaacacggccaccgcgcccgcgaagccgccaacggcgatcaggcccagcttcaggtcgctgctggcggcgatcagcaaggccgcgaaaccggccacgccgatgcccagcaccgcgagcgacgcgggcttgagcccgcccacgtcgcgccggatcacgcgcagcggaggcaccctggccaattgcagcaccggcggcaggccgaaggcgaacagcagcgtgagccccatgccgagaccgaacgccacgggccacaaggtggccgcgggcagcgcggtttcgaccagccccgcgagcagcaccacgaagacgtagtgcacgccaaagccgagcgccacgccgaggctgctggccgcaaggccgacgaccgcgaactcgaaggagtaagccagcgcgatggtgcgctggctctggcccagcacgcgcagcatggcgcagtcgtccagatggctggccgcgaagccgcgcgcggccagcgccacggccaccgccgagagcagcgccgcgagcagcgcgaccaggctcaggaatttctcggcgcggtccagcgtctggcgcatctcgggacgcccgccctcgaaggagtcgagccgcacgccgcgcaggtcgcccttcttgatcgcggcctcggcccagtcggaaaagcgcttgacggccgcatcgtcgcctgccaccgcataccggtagccaacgcggctcgcgggctggacgaggccggtgcgcggcacgtccgcctggttgagcatcacgcgcggcgaaaagctcatgaagcccgctccgcgatccggctcgagcgtgatcacgcggccgacgcgcagactggtgtcgccaagaagaagcgggtcgcccaccttgagccccagagagtcgagcagcgaggcatcgacccacacctcgcccggcgttggtatgtcgcgcgtgatggtgccgggcgcctcggcggtgctggcggtctgcaggctgccgcgcaacggataacctggggccaccgccttgagcgccaccagcttgctggcgccgccctgggcatcgtcggcccgcgccatggtcgggaagccgtaggtgccggtcccctgcaggccgaatgcgcgggcctgcgcaatgaaggtcgggggcgtggggttgtcgcttacgaccacggcgtcgccgccgagcagttgccgcgcatcgcgctgcaagccgccctgcagccggtcggcaaagaagccgaccgcggtgagcgcggccacggccagcagcacggcaacgatcaagaggcgcagttcgccggcgcgcagatcgcgccaaagggtgcgccagccaaggcgaagggaggcattcatgggcgagacgatagccgacgcgcgtgcgccggcgcctttcaggggcttaccgcaaggggtggacagccttaggccggacttcggcgtgcgagttccggctgcagcaccagccgatcggcgcccgcgtagcagacgaagtgccggttggtcgcgcggccaatggcgcacaggcccacgcgcgtggccacctcatggcccatctgcgtgatgccgctgcgcgagaccacgatgggcacgcccatctgggccgacttgatcaccatttcgctcgtgaggcggccggtggtgtagaagacccggtcgccggccagcgcatccggcggctgcatggcgcaccagcctgcgatggtgtcgatggcgttgtggcggcccacgtcctcgacgaagcagtgcatcgtggcctcggtaccgccgggctcgagcgtgaacagcgcgcagccgtgcaccgacccggccgacttgtaggtgctctcctggagccggatggcgttgaccagcgcataaagctgcgcctgcgtcatgcgcgtgggcggcagccggagattgtcgatgtcggccatcaggtcgccgaacacgctgccctggccgcagccggtggtcaccaccttcttggcggtgcgctcctcgatgcggtcgatgccggcgtgcgtcttgaccgcggcggcgcccacctcccaatcgaccgtgaccgactccacgtcgccggccgattcgatgagacgctggttcagcaagtagccgagcaccagcagttcgggctgggcgcccagcgtcatcagcgtgaccaactcgcgccgatccacgtacaccgtgagatcgcgctcggcgggaatggagaccgtgccgcgcgcgccgtgctcatcgacaacctcgacctcgcgcgtcagtgcggcgcgggcctgtgtgagacgtggaagcggcaacggcggcaacggcgttgtcactgcgccttcttcggcgcaggattgacggcggcgtcaggctgcgtggtgctgggcggcgaagcagccgtggtggccggcgaatgcgcgcccgcagcctcgatgggcttggcgtccggcggtggcgcataggcaaaggggccggggtcggcgcagggcggcgtggcaaccgccgtcggcaccggcttggcggccgaggctgcgcttgcgcggtacttggccgccacgcggtcctgcgcctggcagagcttgtagccatcgaccttggctgtccacgcggtcttggcggcggcttcggcggccttggccttggcttcgggagtggcggcgggtggcgggagcttggcccacgccacgggcgcggccagcgcgagcaccagcgcgcagaaattcaaagacagcgtcggctttttcatgagggagttccttcggcgggtatcgcgggccgcgcagcgggcggcaccgccgagccgtccggcaccgagcgctgcgccggaatcttgcccgcgacgatgtcgtcgtaccagagctcgtggtgttccttggcccaggtctcgtcgacgtagccggtgcgcatggctttgtaggcgccggtcatgccgagcgtgccgatgaagatgtggcccatgatcatcgcgatcatcagcagggttgcaatgccgtggaccatgtgcgccacctgcatctcgccgcgcgtgtagacgaagccgggcagcagcttgtccaggaagagccccgagccgatgacgaaggagccgaggaacagcacgccgccccagaacaccaccttctcgcccgcattgaagcggtgcgacggcacttccctgccgccgaagaggccgccgaagcgcgcaagccatttcaggtccatggcgcgcggaatgttgtcgcgaatgaaggtgaagaccatgaacacaatcgtcaccacgaacagcggtccgacgaagttgtggacgttcttgagcgcgtaggcgatccagccgaacagcgtggcacccatccagggcaggaggaagaacttgccgaaggccatcacgaggccggagatcgcgagcgtgacgaacgcgatggcgttcgaccagtgcgtggcccgttcgaagggcgtgaagcgttcgatcttgcggccggtttcctggccgtgcaggcggatggggccgcgcgtgaaatagaagatggccagcgccagcagcgtgacgaacagcagcgccgcaccgtagggaatgatccagtcgttgcgcacctgccgccaggcttcgccggcgttggtgaaacgcgaacccgggtactgaacgaaaggctggatcaggttgccggcttcgggcgcttcgctcttcggcaggctgctgtggccggtcacgccctgccccacctggcgccacatgggcgcgttgttgccgggctgcaccttcatgcgctcgccgttggtctggttcgcgtagttggggtcggcgctggcttcgggcttgacctcgaagatgttctggccgcggatgccgcccgcggccggtgccggcgcgggggtggcagcgggtgtggatgcgggtgcggctggcggctgcgcctgcccgaaggccggacccagcgcggcacagcaaagaaccagagcggtcagcgcttgcttcatgggctctccgttcagttctctttgttgtattcgttctgcccgttctgcgcgcgggtcttgagctgctgctcccaggcggtcttgtcgccgaccttccagccgggtgcggtgaacaccgtgccggcgttctccttgttgctcgttccgctccagggcacggcgtcgcgcttcacgccctgcgtgttggtctgcggcttctcgccgcaggccacgaggcaagttgcggccagcgcaacgcccagggcgaggaggcccggccgcttcatttctgcactccgttcacgggcggcttgcccgcttgctgggagccgtaggcggtgccccagccccagacctcggcacccttgccgcgctggaccacgcgggtgcggaagatgtcggccaccacgtcgccgtcgccggccaggagcgccttggtcgagcacatttcggcgcaggcagggagcttgccttcggccagccggttgcggccgtacttctcgaactcggcttcggagccattggcctcggggccgccggcacagaaggtgcacttgtccatcttgccgcgcacgccgaaggtgccttgcgacggaaattgcggcgcgccgaacgggcatgcgtacgagcagtagccgcagccgatacacacgtccttgtcgtgcagcaccacgccttcttcggtgcggtagaagcattgcaccgggcacaccgccatgcagggcgcgtcggagcaatgcatgcaggccaccgagatcgacttttcgcccggcaccccgtcgttcagcgtgaccacgcggcggcggttcacgccccagggcacttcgttctcgttcttgcaggcggtgacgcagccgttgcattcgatgcagcgttccgcgtcgcagacaaatttcattcgtgccatggtgcctccttatgccttttccacattgcagaccgtggtcttggtctcttgcatcatggtcacgctgtcgtatccgtaagttgttgcggtgttgatcgcctcgccgcgcaccacgggggctgcgccggcggggtagtagccgagcatgtcggcgccctgccaatggcccgagaagtggaacggcatgaacaccgtgtcgggccccacgcgctcggtcaccagggcctgcacgttgagctttgcgcccgtgggcgtgtgcacccaggcacgctcgccgttgcgaatgcccttctcggccgcgaccttggggttgatctcgatgaacatctcctgctgcagctcggcgagccaggggttcgagcgggtttcctcgccgccgccctcgtactcgaccagccggcccgaggtcatcacgtacgggaatttctcggccaccttgtcggcgatgttcttctgctgcacgctcttgtagagagtgggcagccgccagaacgccatcttgtcgtcgtgcgtcgggtacttggccatgaggtcgggccggttgccgtagagcggttcgcggtgctgcggaatcgcgtccgggaagttccagaccagcgcgcgcgccttggcattgccgaagggatggcagccgtggttcttcatgaacacgcggatcatgccgcccgagctgtcggtcttccagttcttgccttcggccttcggcttctcggcctcggtgagctcgtcccaccagcccagcttcttgagcagcacgtggtcgagctcggggtagccggtggtgatgtcggcgccgagcgaatgcgagccatcctcggccagcaggttcttgccgtcgcgctccacgccgaagttcgcgcggaagttgccgccgccttccatcacgtgcttggacgtgtcgtagaggttgggcgagcccgggtgcttgagttcaggcgtgccgtagcagggccacggcaggccgaagtaatcgcccgtgaggtcatagccgttgaccttgtccttcacgccggccttcaccttgagcgtgcgcacgtcgaaggcccccatgttgcgcatgtgcgcctgcagccgctcggggctctggccggtgtagcccacggcccagcaggtcttgttgatctcgcgcaggatgtcgtcgggcaggggctcatccatgcccttgaccttctgcatcttgaagttcttgctgagctccttgccgaagcccaggcggtcggcgaactgctgcatgatcatgtggtcgctgcggctttcccacagcggctcgatcactttctcgcgccactggatcgaccggttcgacgccgtgacggagccgctggtctcgaactgcgtgcacgcgggcagcaggtagacggcgcggttcttgttgaggtcgtcggggttgccgggcatggcggccatggcggccgtggccgagggatacgggtcgaccaccacgagcaggtcgagcttgtccatggcgcgcttcatctcgaggccgcgcgtctgcgagttgggcgcatggccccaatagaacacgccgcgcaggttcgagtcctggtcgatcagctcgttcttctcgagcacgccgtcgatccaccgcgacacggtgatgcccggcttgctcatcatcgcgggcgacgcaaagcggcccttgatccattcgtaatcgacgccccaggtggcagcgaagtgcttccacgaaccttcgacgatgccgtagtagcccggcagcgaatcgggattcgggcccacgtcggtggcgccctgcacgttgtcatggccgcggaagatgttggtgccgccgcccgacttgcccacgttgccgagcgcaagctgcaggatgcacgaggcgcgcacgatggcattgccgatggtgtgctgggtctggcccatgcaccacaccacggtgccggggcggttctcgttgagccaagtggccaccttgagcacctgcgcctctttcacgccgcaggcctcctcgaccttgtcgggcgtccacttggccaggacctcttcgcgcaccttttccatgccgaagacgcggtcgttgatgtactgcttgtcttcccagccgttcttgaagatgtggtgcaggatgccgaacagaaaagcgatgtcggagccggagcggatgcgcacgtactcgtcggccttggccgcggtgcgcgtgaagcgcgggtcgaccacgatcatcttgcacccatgctccttggcatggagcatgtgcagcatgctgaccgggtgcgcctcggcggcgttggagccgatgtacatcgccaccttggcgccgcgcatgtcgttgtacgaattggtcatggcgccatagccccatgtgttcgcgacgccggcaaccgtggtcgagtggcagatgcgcgcctggtggtcgcagttgttgctgccccagaagctcacgaacttgcgcagcagatacgcctgctcgttgctgtgcttggacgagccgatccagtagaccgaatcgggcccgctggcctggcgcaggtccttcagcttggcggtgatctcgttgagcgcggtgtcccagctgatgcgctcgtacttgccgttgaccagcttcatcgggtagcgcagccggtattcgccgtggccgtgctcgcgcagcgcggcgcccttggcgcaatgcgcgccgaggttgatcggcgaatcgaacactggctcctggcgcacccacacaccgttctcgaccaccgcatcggaggcacagccgaccgagcagtgggagcacacggtgcgcttgatttcgaccttgccggcgccgatcgcggtgggccgcgcatcgcctgccgcctcggccttgcgcatcagcgtgagctggccggcggccaggcccacgcccacaccgagcccggaacgccggagaaaggcgcgccggtccatggtgggcagcgcgcccgaaaggccgcgccgcaggctgtgaatgaacgcggaagactcgcgttccccttgccgcgagacagtgttcgcgggggctgttttcttggtcaacaacatcttggggtccgcttcaggccgaagcggtcttgtaatagcgcttgacgtgttcgctcagcgaatagccgccgcccttttcaggcgcgggcttcgccgcgggcgcggcagcttcgaccgccacgggggtgtcgaccaccttcggaagcaccgaaaccgcggcaaccgcggcaccggcgctggcggcacctaaaaagaaacctcgacgcgaggccggcttgatgccggccgcttggctgtcctgcatgtgatctccaggagtggctgggggcaaaccagatatgaactgatttgcatacatctggatactagtcgagacccttaatcccgacaatcaaactcttccattgatgcgatcaatcgagcatgtcgaagccctgaacctcgatttcggcgaaagcgcgggtgaacccggccagcgaggcatagaaatgcgacttcggatgttgcgccactgcgtcgcagagcgtcggcagccacgactgcagatgggtggcgaaaaaagcctgttgctgcgcaaggttggctaccgctgcgtcgtcaccggcaataaggtagcgcattacctcgaacagacaggcaacatggtcttcgctttcggacacggcctcgccgcgcgccagcccgaggcgggcgaggtcggtgcgcagttgcgccagcggcttgtcgttgagaaagccgctcaggtagtgcgagccgaaaaggtagatctcgggcttgcccatgccgccgaacagcgcgtcgtactcggcatgcaccgcggcggcatcggtgccgcgcgccgcgccgaccagctgccgccagggctcctcgagaaaggcgccggccgcgggcgcctcggtcggcgccacgccgaaggcgccgagcagttcggcatcgggcgcggcataccagaggcgcgcgagcaggccgtagacctcggcccgcgcaatttcctcgtcgagcgccgaggtcattggaggaaattgactcatagttgcgtgatcttcatctcgttctgcgcgctgtacaggtcgatcacccggcagtcgctgcacatcttgagccgctcgagcgcctcgccctggaacatggcgtggcccgccagcttgccgagcatcgcttcgatggccttctgcgtgccgaagggcttgctgcagcggatgcaagcccagggcttggcctcgttgagcaccacgggctgcttgcgctcgggggcagtcgaaagccggggcacgagcgcaatcgcgttctcggggcaggtggtggcgcaaaggccgcactgcacgcagttcttttcgatgaagcgcagctgcggcgcattctggttgtcttgcagcgcgcttgcggggcaggcgctcacacaagccaggcacagcgtgcagctgtccttgttgacggtgatcgcgccgaagggagaaccgtccggcagcggaatttcgaggggtgcggcggcatcggcaggcggcgccgaaagcgccggcgcctgggccatcaggtggtccagcgtcatctcgagcgtgccgcgcttctcgccgccgacggcaaagcgcgccgcactgccgggcacgcgctgccgcgtggcgcgcaggccggccagcgccgcatccagcgcggcgggcgtggcggcctcgatcaggtggaagtgcgtgccggtgtagccgaggccggtgagcagcgcctgcgccacggccatctgcttcttgagtgcgtccaggtactgaggcgcctcttcgccggtggacagcaccgccacctgcgacgcgccgaacgcaacggcgctgagccagaggtcgatgccggtgctcgcgacatgcatcagcgccaccggcagcacatgcgccggcacgccgccgaggccgtcgcgcttgccgcgcccgagctgcgcctcgcggccgagccgttcgaccagcgcctgcccgccttcttcgttgtgcagcagcaccgtggcgtcgcggccgccggcgcccaggtaggtggcgagcagcgtgcgcagcttgcggccctggtcgggcgtgcgcggataggtatagcccagcgcgccggtcgggcatacggtggtgcaggcgccgcagcccacgcagagctgcgggttcacgacgatgcgctggcgctccttgtcgctggagatggcgtgcgccgagcacacctcgacgcaggcgttgcagcccaccacttcgttgcggctgtgggcgcagagcttctgcttgtagtcgaagaacttcggcttctcgaactcgcccaccagctcgcgcaggcgcagcagggtcgacaggccttcgccattcgccagcccgcccgccaggtggaaataaccttgcggcggcgcatgccagtcgatcagagcggttgtgcccaggtcgagcaccaggtcgaaaccggcatcgagcgcctcgggcgcccggccgaagttgatggcgccggccacgccgcagactttttcgcagtcgcggtgcgaggtgcacttggccaggtcgatctggtagtcgagcccgatcgcctgctcggggcaggcgctcaagcaggcattgcagcgcgtgcacaggtcgagatcgatagggttgtcccgcatccacttgagcgagaaagcgccgagccagccgtcgagcgatgcgatacgccccgccatcacgggccagcggcgttcctgcccgccgccgctggcgcccgggccggtggaaaagatcgagacctgcagcgtgtcggccaccagcgcggcggcccgctcggcctggtcgagcgggccgacgatcaggagccggccctggctcgcgtagctcacggtcgagaccggatcgggctccggcaggtgggccaccgccagcaaggcggcaatcttggggctggcgttcttcgcgtcgcgactccagccgccggtttcgcggatgttgacgaagcggatcggcgaggtcgcgccttcggtctgtccagcgagctcggtgaacagcttgcgctcctgcgtgcacgcaaccaccacctcgtcgcccgagcggatggcgcgctggaaagccggcgcctcgcggcggcacagcgtggaatgaaggggaagcgactcagccagcgctgcgccgagcgtcttcggctcgagcggcatcgtctggttgcagtcgcagatcagcgtggtggtcatcggttttgtggcttgcgggttgcgcatcggcaacctgctggctggggatatctcccggaggctcggactgtgccacgtccggcggcgcggcgacgtgcggggtttccgcgggttctccggatcgttgcacttgctcttcttcctcgtgctcgaacagcttgaggaacttggcactggccatctggcgcagcacgctgtcggggatcggcgtcgatttggaatagtcgtcgacgtaggtgtccaggccgtccatcacattgaactgcgggtcggcaaagagctttctgaaggcggtgttttttacctcgggcgcgacgttcctggccacgaagggccggaagtcggactcggacgtgagggcttccgcatcggcgagggtgggtgggggtgtttccccctgcccttcggcgggaaggccggccgcggtgctctgggccgcgggcaggggcgcggcggtttcgacgcgcgcagcggccgcgccttgcacctcgtccgcgtcctgcaaggcgggaggcggcgaaagctcttcgcgtgcttcctttttgcgccgcgaccagcggtcgaagaagttctcagacatcgcccgctccgggtccgcgctttttctcggtcgacacggtggccgggttgccgaagcggtcgaccagcgggcggaaactctcgggccgcttgcggcgcttgggctccatcacgtaatgcgcctgcacgaagccgcgcatccactcgatcacgtcttcgggcgcgggcacctgctccacggtttcctgcgcgtcgagccagcgcccggcttcgttgtagctgaggctcaccaccaccggccgcgccagcggctcgtcggcaatggtgggttcttcctccatgcgccaaagcacgaaccagcagggcgcgggcgtggtggcgttcaggtggtaaccctccacgtcgtcgcggaacagctcggtcttgaagccggggtgcagccagcgctgggcacgctcgctcgcctcgagcaggcgcggctcggtgccgaagccgggctggtcggggccgacgctttcgagaatccagcgccaggactgccaacggctgtcgacacgttcgcggcgcatcacaacggcaacatcgatggaaggattcatgccgcgatcgtagcgctgccgcaaggcgcttttgcggcgagggtcatccgcgtcctccgccggccggctcacgcgccgcgcgcgtcccgcagcagcagcccgcgcagctttcgatgcagcggcgtggcttcggtggccggcacgccgcccacctcgcgcagcgcgaaatcgcggctctgcgcgttgtgcaggtcgatctcgcgcaccacctggccgttgtcgtagacaaaagccacgtcggccagcgccagcacgtcgtcgatgtcgtgcgtgatcatcagcaccggaatgccccattggcggcggacctgcgcgagctcgttgcggagttcgctgcgcagcatcgggttgagcgcggcaaagggctcgtcgagcaacagcacctgcggctggcaggccagcgcgcgggcgagcgccacccgctgctgctggccgcccgacagcttctgcggccggctgtcggccagcgccgccagaccgaagccttcgagcagcgactgcaccatctcggcctcgcgcggcggcagcttgcgctggtgccacgcggtcaggccgaaggccacgttctcacgcaccgacaggtgcgggaacagcgcgtagttctggaacaggtagccgatgcgccgcgcgggcgccggcacgtcgatgcggcgcgcggagtcgtagagcgtgcggccgtcgagccgcacatggcccgcggacggatgcagcagccccgctatcgcttgcagcgtgagcgtcttgccggcgcccgagggcccgtaaagcgcggcaaaaggcacgtcggtcgcgaagcgcgccgccaggtcgaagcggcgggtgccgtcggtgaccgtgagcttcaggtcgacgtcgatcatggtttgccgaagccgtagtgcgccaggacttcgcgcgcggcgtcgctcgaaagaaaagccacgaaatcgccggccagcgctttctgccggctgtcggcgaccaccgcgaccgggtaggtcaccggcatggaggttgccggcgcgaaggcgaccctgaccttgtcgcccatcaccgccgcatcggtgcggtagacgaagccggcttcgacctcgccgcgggccacgtagtcgagcacctggcgcacgctgtcggcctgcacgaacttgggctcgagcacgctccagagccccgccccttccagcacctgccgcgtgtagcggccgaccggcacggtggcggtcttgccgaccgcgattttccgcacacccgcgccggcaagatcttgcagcgaccggacgcctgccgcgtctctcagcggttcgatcagcaccagggcgttgctcgcgaagttccggcgcgtggccgcatcgatgagcttctgttcggcggcgcggcccatggtctcctggtcggcgctggcgaacacgtcgaccggtgcgccctgcgcgatctgctgcagcagcacgcccgaagccgcaaagttgaagcgcaccgtggcgcccggcctggtggcctcgaacttcggccccagcgccttgaacgcgtccgtcaggctggccgccgcggacacggtgatctgctgggccgccgcgcccagcggcagcgccaaggccaagacaagagacaggaggcggagcggacgcatggaggttctcgggtaagggtgagccagtcagcgaagcgagaaaaagcggttcgacagcaccagcaccgtgaccgacagcacggacgtcaccaccaccagcagcaacgccagctcgtcatggccggcctgcacggcgtcgtagatcgccatcgacaaggtctgggtctgctgcggaatggagcccgccaccatcagcgaggcgccgaactcgcccatggcgcgcgcgaacgcgagcagcgtgccggccaggatgccgggccaggccagcggcagcgtgacacgcaagaacaccgagagcggcgactggcgcagcgtgctggcggcggcttcgagcgagcggtcgacccccgcgaaggcggcgctggccgacttcagcaccagcggcagcgccaccacggccgacgccacgacggcgccatgccagctgaagatgatggaatagtcgaaatgctcgcgcagccagctgccgagggggctatggcgccccgcggccaccaggatggcgtagccgatgaccgtgggcggcagcaccagcggcagcatgaacaccgcctccagcaccgtgtcgcccggaaaacgcttgcgcgcgaacacccagcccagcgccacgccggcaacgagcgccagcagcgtcgcgaccgcggccaccttgagcgacagcaccaacggaaaccagtcggtcgaagcgatgagggagttcgtcgtattcatgaagatacaacgcaattgttgcacgaacggactttcccccttgaaaagaggtccgtggcggctgcgggagagtggcgccgatatcctttcggatacagcgcgggcgatggatcagggcgccagcaggcgcgtcagcgcgcggacgtcggccgccgtggccaggcgcgcagcgttctcgatggcgcggtaatgcttgacgatttcctcgcccacgggcgtgagcgcggtgccgccgccgcgcgagccgccggccgccgtgttcacggccggggagctcagggcgtggttcatctcgtcgatcagcatccaggcacgccggtacgacatgcccagctgccgcgccgcggccgagatcgagccggtctccgccacggcctccagcacggcgatcttgccggggccgatggcgatgctgtcgtcccggtagatgcgcaggcggaactggactctggttttcatgccggtgggggtgagcggtgcgggggcgtcggggcgcaaaggttaaaccatgcccgcgccctcgcccaccgcccgcgtcaatccacctttgccagcacgcccgagccggttccgtagccggccgccgccatcggctggccgccgcgcgcaatgcgcaccgcgcagtacttgaactccgggatcttgcccatcggatcgagcgcggcattggtcatcaggttggccgccgcctcgtagtaggcaaagggcacgaacaccgcgccgttcggcgtgccgtcgtcgcgccgcacgtggatggccacctcgccgcggcgcgactgcacggtgatcacgtcgccggcctggagccccagcttctgcagatcggcctggttcatcgacgcggtggccatgggctcgagcgcatcgagcacggtggcgcggcgcgtcatgctgccggtgtgccaatgctcgagctggcggcccgtgatgagcacgaacggatactcggcgtcgggccgttcgttggccgggatgatgtcggcgggcaccagcttcacacggccgtcggccgtcgggaagtcgtcgatgaacacggtcggctggcccgggtcgtcctcgctcaggcaggggtaggtcacgctcgaatcgcgctgcagccgttcccagctgatgccgctgatcaccgcgtgcatggcctggcgcatttcctcgtagaccgcggccacgccggattcctcgccctcgtagttccattgcaagcccatgcccttggcgatctgctggatgatccagagatcgggccgcgcgtcgcccggcgggttgagcgcccgcttgcccagctgcaccatgcggtcggtgttgctcaccgtgccggtcttctcgggccaggcgctcgcgggcagcaccacgtcggcgagccacgcggtctcggtcatgaagatgtcctgcaccaccagatgctccaggctcgcgagcgcatggcgcgcatggttcaggtcggggtcgctcatggccgggttctcgcccatgatgtacatgccgcgcaccttgtgcggatcggtgtcgggcgccagcgccttgtgcatgatctcgaccacggtgtagcccggcgtcgcgtccagcggcgtgccccagaagttctcgaaccacgcatgcaccgccgggttgtcgacgcgctggtagttggggaacatcatcgggatcaggcccgcgtcgctcgcgccctgcacgttgttctggccgcgcagcggatgcaggcccgaacccggcttgccgatctgcccggtcacggtggccaaggcgatgaggcagcgcgcgttgtcggtgccgtgcacgtgctggctgatgcccatgccccagagaatcatcgagccctttgcggtggcaaaggcccgcgccacttcgcgcagcgtttcggccggcacgccgcagatgggcgccatcgcctcggggctgtagcccttgacgttctcgcgcagcgcctcgtagttgctggcacgcgtgcgcacgaactcctggtcgaccaggccttcgtcgatcacggcatggatcagcgcattgagcatggccacgtcggtgtcggccttgaactgcagcgtgcgccaggcatggcggctgatgtcggtgcggcgcgggtcggccagcacgatcttcgcgccgcgctgggcggcgttcttcatccaggtggcggccaccgggtggttcgccgtgggattggagccgatgacgaagatcagccccgcatgctccacatcgttgacctggttgctcaccgcgcccgagcccacgccttcgagcagcgcggccacgctggaggcgtggcacaggcgcgtgcagtggtcgatgttgttgctgccgaagccggtgcgcacgagcttctggaacaggtaggcctcttcgttgctgcccttggccgagccgaagcccgcgagcgacttggcaccgtaggtgtcgcgcaggcccgcgagcttgccggtggtgagcgccagcgcttcttcccaggtggcctcgcggaaatactcgctccagtcgccgggccgcggcgcatcgccgaagtccttcggcacgccggccttgcggatcagcggcttggtcaggcgctgcgggtggtgcgcgtagtcgaagccgaagcggcccttcacgcaaaggcggttgtggttggccggtccgtcgcggccatcgacgctgacgatcttttcgtccttcacgttgtaggtgacgaggcagcccacgccgcagaacgggcacaccgaatcgaccttgcggtcgacctgctgcgagccgatgtggctcttgggcatgagcgcgccggtcgggcaggcctgcacgcattcgccgcaggccacgcaggtgctgtcgcccatcgggtcgtccaggtcgaacacgatcttgctgtcgccgccacgcagggcatagccgatgacgtcgttgacctgctcttcacggcaggcgcgcacgcagcggttgcactggatgcaggcgtccaggttgacggccatggccggatgcgagatgtcggtcttgggctgctcgcggcgcagcgccttgagttcggggcgcaccgcgatatcgagctttttcgcccaggcgctgagctcgccgtgctgctgggtggcgtcgtcgccgatccatttgtagccttggtcgggcatgtcggacagcagcatctcgacgaccattttctggctcttgagggcccgctcgctggtggccttcacttccatgcccgccgtgacgttgcggcagcagctaggcgccagcgtgcgctcgcccttcacctcgaccacgcaggcgcggcaatttccgtcggcgcggtagccgtccttgaagcacaggtgggggatttccacgccatggcgctcggccgccttgtagatggtttcgccatcgaaggcctggatggattggccgtcgagcgtgaattcgatggtctgcggcatcagctccgcgagcttggacggggcgttcatgccacctcctccggaaaatattgctggatgcaccgaatcggattgggcgccgcctgtccgagcccgcagatggaagcgtcgcccatgacctgcgcgaggtcttcgagcgtggtgttgtcccacaccggcgcctgcatcagcgccgcggccttcgcggtgccgacgcggcagggcgtgcactggccgcagctttcgtgctcgaagaatcgcatcacgttaagcgcggcatcgcgcgccctgtcgtgttggctcagcaccatcacggcggccgatccgatgaagcagccatggggctgcagcgtgtcgaagtcgagcgggatgtcgttcatgcgggccggcaggatgccgcccgaagcgccgccgggcagataggcatagagcgagtggccgtcgagcatgccgccgcagtattcgtcgatgagctcctgcaccgtgatgcccgcaggcgcgagcttgacgcccggatgcttcacgcggccgctcacgctgaagctgcgcaggcccttgcggccgttgcggccgaagccgctgaaccaggcggcgcctttttcgacgatgtcgcgcacccagtagagggtttcgaagttgtgttccagcgtcgggcggccgaagaggcccacctgcgcgatgtatggcgggcgcatgcgcggttcgccgcgcttgccctcgatgctttcgatcatggccgactcttcgccgcagatgtaggcgcccgcgccgcgccgcagctcgatacgcggcagcgcgcagggcggatcggcctggagccgggccagctccctttccagcaacgcacggcagtcgtggtattcgtcgcgcaggtagatgtagcactgctcgatgccgacgatctgcgccgccaccagcaggccttcgagaaagcggtgcggatcgcgttcgagataggtgcgatccttgaaggtgccgggctcgccttcgtcgatgttcaccgccatgagccggggcgccgactgatcgcgcacgatgcgccacttgcgccccgccggaaatcccgcgccgcccaggccgcgcaggcccgagtcttccatggtcttgatgatggcctcggcgtcttcctcgccgttgacgagcgcggacgcgagcgcatagccgccgtgtgcgcggtaggtggcgtagtcggtgaaagccggcatgcgctcgatggcgccgggcagtggcgagatgcttttttcggcgaatgcggcggcatcgaagtacgcgaccgtggcttcgtcgggatcggacttcagggcctgcaacactttgccggtggtcgcgagcggcactgcctgctggtcgacgaccgccacgggcgcctgctcgcagcggccgacgcagggcgcggcaatcacgcgcacgtcgccgccttcgaccccgagcagttcgggcagccgcgccagcagatccctggcaccggccagttcgcaggccaggccgtcgcacacgcgcacggtgagtccgggtgccgcatcgtcgccgcgcaccacctcgaagtggtgatagaaggtcgcgacctcgtagacctcggccatggggatgttcatttcccgtgccagcgccaccaggtggcggtcgtgcaggcagcggaaggcgtcgttgagcttgtgcaggtgctcgatgagcaggtcgcgccggtggccctcggccggacgcgcgccgatgagcgtgcgcacttcgacgagtgcggcttcctcgggctggcggcccttgagcttgctcttgcggcggatgcgctcgcgcatctcgtcggcggtggcgagcggcacgatggtgtgcgtcggggccgccgtggtggtcgttgtctcgcgggtcgtggctgggtggttgttcactgcctaggccttttttcggatgtctgtctggctctgccccgagcggatgctgggaggctgaccgagtgtgtggggccgccctgggtgcgtcaaattcgatcggcgcatcgatcgattcaataactaaatggtgcgcccgctcagggccggccgccagctattcgccgagcgcgccgctgtgcagccgcacctgctcgcgccaggccggcgtctgcaggaaaacgagggcggcatcgagcgcacgcgaggggcgcacgccggtctgggtcatgaagcccagcggggtcttgacctcgggccccaccagcggcagcgcctccagttcgcggtagctgcgcaccgccgcgaccatcgaccccggcagcacactgctgacgctgcctgccagcacggccaaggcaagggtaagtaccgagttggtctcgatggccggctccaccacggtgtcggcttcgcgcaacgcctggtcgatgatggagcggttgtgcatgtcgggcgtgagcaggcacagcggcagcttgccggcgtcggcccacgacatcggccggccgatgcgcagccggtcggccgagggcttggccgcgcggcgcagcagaaagtagtgctccacgctctgcggccatgccgtgagcttgatgcccggcaggtgcatgcgctcggtatagccgagcgccaggtcgacggagaggctttccaaccccatttccaggtcttgcgagctcatcgacagcacggccggcacgatgcccgggtgcagctcgtgcagcatcgccgcaaagcgcgacagcatcggaatggcggtgggcaccgccgccatgcgcagtcgcccgcgcggatggccctcttcgctgcgcagctcctgctgcagcacctcgttgtcgcgcagcatgcgctgtgccgtggccagcacacgctcgccttcgtgcgtgaggcccacatacacgcgcgcccgcttgacgatgaccacgccgaactcgccttcgagcgagcgcagcgcattcgacaacgccggctgcgtgatgtggcaggcctgcgccgcgcgcccgaagtgcttgtgctcgctcagtgcgaccaggtagcgcatcgacgcgagaagattcacggggcgcgccgccgatcaggtgttcttgctgatggaaatggtcgggaacttggccgagaagtccttggccttttcggcgatgcccacggccacctgccgcgcgacggccttgtagatgcccgccacttcgccgtcggggtcggccactacggtgggcttgccgctgtcggcctgcagccggatgttgatgtccagcggcagcgcgccgaggtattccatctggtactgctcggccatcttcttgccgccttcggagccgaagatgtgctccacgtggccgcagttggagcagatgtgcaccgccatgttttccacgatgcccaggatcggcacgccgaccttctcgaacatcttgatgcccttcttcgcgtcgagcagcgcgatgtcctgcggcgtggtgacgatcaccgcgccggtcatcggcacccgctgcgaaagggtcagctggatgtcgccggtgccgggcggcatgtcgacgatcaggtagtcgaggtctttccagttggtctggcgcagcagctgctccagcgcctgggtggccatggggccgcgccagatcatggcctcgtcctggtcgaccaggaaaccgatcgacatgacctgaacgccgtgattctccagcggctccatggtcttgccgtcctcgctctcgggccggccttcgatgcccagcatcatgggctggctcgggccgtagatgtcggcatcgagcagcccgacggccgccccttcggccgccagcgccagcgccaggttggccgccgtggtgctcttgcccacgccgcccttgccggacgccaccgcgatgatgttcttgacgttgggcatcagctgcacgccgcgctgcaccgcatggctgatgaccttggtcgtgatgttgaccgagacgttgctcacccccggcaccgtctttgcggccgccaccagcgccttgcgcagggctgggtgctggctcttggccgggtagccgagctcgaggtcgaacgaaacgtcgccttcggaaatctgcaggttcttgagcgaacgcgtcgccacgaaattcttgccggtgttcgggtcctggacggccttgagcgcgtccatgagcccttctggggtgagtgccattgatctaactcctgaatggcgggtagtctagtggcttgccaccggcccccgggcgcttcggccgcttcgccttcccgctgccgggggcaacacccgcaaaccacgggggatgcaagcgctttttgaacagccacagcaacaagaacaatgcctccgacacccccggtcaccggtcttttgctcaccggcggcggtgcccgggccgcctaccaggtcggcgtgctcgaagccatcgccgacatccgccgcgcggcgggtttcgccggtcagggcaatccctttcccgtgatcaccggcacctcggccggcgccatcaatgcggccgcgctggcctgcggcgccgacgacttcgaccaagccgtggcgcgcatcgcggaggtctggcgcgacttccacgccgggcaggtctaccgcgccgattcgctctcggtcatcggcagcggtacgcgctggcgcatgctgctcgggctcgggcgcttcgcggccagttggatgcgcatcaagccgcgctcgctgctcgacaacacgccgctggcccagctgctgggccgcatggtgccgctcgaccggctgccccggctgatgcaggagggccacgtgcaggcgctggccgtcaccgcatcgagctacagctcgggcgagcacgtcaccttcttcgaggcggccgtgccgatggagccctgggtgcgttcgcagcggctctcggtgcgcaaccgcatcagccacgcgcacctgctggcctcatcggccattcccttcgtgttcccggccacggcgctgccgatgcaggggcataccgaatatttcggcgacggttcgatgcgccagtcggcgccgattgccgcagccatccacctcggcgccaagcgcatcctggtgatcggcgccggccgcatgcacgagccgcgcgacgccgacgcgcccaacacctacagcggctatcccaccatggcgcagatcgcgggccatgcgctgtcgagcatctttctcgatgcgctggcggtggacatcgagcggcttcggcgcatcaaccacacgctcggcctcattcccgaggaagcccgcatgtcgagttcgctgcgtccgctcgacctgctggtgatttctccgtcggagcggctcgacgtgatcgcggcacgccatgtcgatgccctgcccggcgcggtgcgccacctgctgggcggctccaaggctgcggccgatgtgaagggcggcgcgctcgcaagctacctgctgttcgaatcggcctacacgcgcgagctgatggcgctcgggcgggccgacgcgatgcggcagcagggcgaggtgctgcggttcttcggctgggaagcggcggcctgacggagatcagcgcgcgccgccgcccgctgcggaaaggcccgccagcagcaggtccaggctcgcttggaactcctggtcggccgtgcttgcggtcgctgcattcgcgatgtcgatcaggtgcgcaaagcggtcttccggcaaggcccggaatcgttcgatggtgagctccgccgattccgacgcctgcagcgccagcgggcccgcaagctccgactgcgcgagccccgtgatcagccccgacacggcccggaaggcgacgagcagcgcctgccccgagcgcccgctgcgagccagggcgcgcagcatcgcctcggtcacgtcgaagacggccggcgaacggcttcggcgcgtgaggatcagcgcaatggcatggggatgggcccgcaccgcctgccacaacgccgtggcgatggcccggacttcgtcctgccattgcgcgtgttcggcaagcggccagcgcgcttggccgatcaccgcctccaccaccaagaggtcgatgtcctcgcgctgcgagacgtagttgtagagcgtcatcgcgccggtgccgagctcgctggccagcgcgcgcatcgagagccccgccagcccttccctgtcgacaagagccaatgccgcggcctggagttgcgaatgcgtgaatttggcgggtcgtcccataagggtggatgttgacgcagttcggaagacgcgagtatattcaattacgtacagcgtacgtttaaagaggaaagtccatgaaattcgcacccggcgacaccgctcccgccattgccgacagcaccatccacggcaagcctgcccatgttccggacccgctgccgcgctacgtgcatcttcagttccggcgtttcgcgggttgcccggtgtgcaactttcatctgctcaccatgggcaggcgccatgcggaaattgccgcggccggcattcgccagctcgtcttctttcattcggcgcgcgaagaaatgctcaagtaccaggcacagcttccgttcgattgcattgccgatcccggcaagaagtatttcaaggcgttcggcgtcgagacctccgtgcgagcgctcttgaatccccgcgtgttctggagcgggctgcggtggatcctggcagccaggcgcctctacacccgggccgagaacggcatcctgggtctgccggcagactttctcgtcgacgcgcaggggcgcatcgtggcgtgcaagtacggcgcgcatgcggacgaccattgggaagtcgacgaattgctgcagctggcccgcaaggcaccgcctctgcaggcgatgccgctcgcagccaccgcgtcgcccagctagcgcccgcgcgccggatcaccccgcctctgaaatcccgagttccgaacacacccgccccaccagcgccctcagcgagacgagctcggcctcgagccgcgccacgttggccttgagcgccgcgacctcgccgagcgatgcatcgtgcgacgcatacgctccctcggccgaaccgccacccggaccggcaacctcttccgccggcgcgccgctcagcagatgcgcccagcggctttcgcgcgcacccggcaggcgcgcgagcttcaccaccaaggcgccggccggacgctcggcgagttcgtcgagaaagccctcgaccgacgagatatcggcgaagttgtgcatgcggtcgcaggcaatgcgcagttcgccgggcgtttgcgggccgcgcagcatcagcacggtgagcaggatgaccgattgcgacggaatgcgcagcacccggtcgatgttgtgctcgtagcgaaaggcccggccgccgctggtttccgccaccaggctgtagcccttcaggctgtcgatggcggcctgcacctgcgcctcgcccagttcgagcaccgggttgcggctggtcttctggttgcagccggacaccagcgaattgagcgtcagcggatagctgtcgggcacggtgcgctgcttttcggccaatacgccgagcacgcgggtttcgacgagcgaaagaatgggaagggcctgggtcatttctcaaagaatcctgaatgaaagcgcggtgtcccgaagccggttcatggcaccgccacgccgagtatcgggcccagctcgcggacgaaatcgccgcgccgcagcgcgagcgaatgcaatgccgagacggtgccgtcgagatagagcgcgtcgcggcaacgcagcacgtcgcgaaagtagagggcgaattcgtagaagttcacgggctgctcgctgatcacgaagatcgcggtatggcccgacacgcccacgccgttgcggatcttccgcgaatccgagtcgggaatgaaagcgggatgcaccctgccgcggcgcagcagcaacgggcccgactgcgtggccagccgaacgcccttggacagcgccggatattccgaagactcgaccacgcgcggcacccccgcgccggacaccaggaacacaccgttcggcttgaggaagaagttgccctcgcccgccgacaggttgagcggcgaaacctcgcgtccgtcctgcaccaggaggcccaccggggaaaagtcggcgtggtacatgccggcattcatcgcgaacaccaactgccggttgtgcccggcgagccacgcctcgaggcggtcgaagcgcttgaactcgacgccggcatcgtcgcgcaggaacagctcgagccgctccttgcgcaaatcgatcttcacgacggtgtagcgcggctcggcatcggccgctcgggcggccaggctggccgcggcggcgacgcacaaggccagcaggagcagcagctttctcatgaagtcccggaaagccgcctccgcttcagccgttctggatgcgactgaccagtgctttcgtgaacgccgcagtgcccgcggtgccgccgaggtcgccggtgcgcaccttgtcgatgttgagcgtgtcgtcgatggccttgcgcaggcgcgtggcaaggtcgggcagcctgacgtgctcgagcatcagcgcggcggccaagagcagtgcggtggggttggcaatgcccttgccggcaatgtcgggcgccgagccgtgcacggcctcgaagatcgccgcatcggcgccgatgttggcgcccggtgccatgcccaggccaccgaccaggcccgccaccaggtcggacaggatgtcgccgaacaggttggtcgtcaccagcatgtcgaactgccaggggttgagcaccagcttcatcgcgcaggcgtcgacgatgatcgtgtcgagttcgaacttgcccttgtacttttcttcatagagccggaggccggtctccaggaacaggccggtcagcaccttcatgatgttggccttgtggaccagcgtgaccttcttgcgccccgtggcaacggcggtctcgaaagcgtattcgagcaggcgcaggcacccctggcgcgtgttgatgccggtggccatgcccacggcatgcgggtcgccgtcgatgcgcacatagtgctcgtggccgatgtacaggccctcgaggttttcgcgcacgaccatcaggtcgatcttgtcgaagcggccgcccggaatgatggtgcgcgcggggcgcaggttggcgtacagctgaaattcttcgcgcagccgcacgttcgacgagcggtagccgccgcccgaaggcgtctccagcgggcccttgagggcaaggcgggtgcggcggatgctgtccagcgtggcttctggcagcggatcgcccgaagcctggacgccgccgaggccggcaatctggcggtcccactcgaagggcgccttcagcgcatcgagcgcggccagggtggcgtcgacgatttcggggccgatgccatcgccgggaatcagggttgcggaaatgggggtggtcatcggaaactcgctttctgtatatctatcttgtatatctcttcgccatatggggagggagcgtggcgaaacgcgcggggtggagcatacgtcgcgccggagacaccccggcgccgttcgggtcactgggggtccggaacctctggtcgagcccccgggatcgggggtcttcggcagggtgcggtgccgccacctaaaatgcccggttcccgaatgcggccccaggccgccttcgttgccagcaagttcgccactcccgaaagcgcccttcccgatgtccgccccgcgcaagctcttcgttaccaccgccctgccctatgccaacggcaagttccatatcggccacatgatggaatacatccaggccgacatctgggtgcggaaccagcgaatgaatggcgccgaggtcaacttcgtctgcgccgacgacgcgcacggcgccgccatcaccatcgcggccgacaaggccggcgtgacgccgcaggccttcgtggccgagatcgccgcgggccgcaagccctacctcgacggctactacatctccttcgacaactggcactcgacggacgcgcccgagaaccaccagctcgcccaggacatctaccgcgacctgcgcgccaacggcttcatcagcagcaagagcgtcgagcagttctacgacccggccaagggcatgttcctggccgaccgcttcatcaagggcgaatgccccagctgccactcgaaggaccagtacggcgacaactgcgaggtgtgcggcgccgtctacgcgcccaccgagctgatcaacccctattcggccctgtcgggcgccaagcccgagcttcgcagctcggagcacttcttcttcaagctctcggacccgcgctgcgaggcctacctgaaagaatggacggccgccgccggccacgtgcagcccgaggtgcagaacaagatccgcgagtggctctacaaggacgacgaaggcaagggcggcctcggcgactgggacatcagccgcgacgcgccctacttcggcatcgagattcccgatgcgccgggcaagtacttctacgtgtggctggacgcacctgtgggctacctggcctcgctgaaaaacctgcttgacaagcgctgcatcgagcttggcggcgacggcatctcgtacaccgagtacatggccgatcccgacctggagcaggtgcacttcatcggcaaggacatcatcaccttccacacgctgttctggcccgcgatgctgcatttcagcggccgcaaggcgcccgatgccgtgtacgtgcacggccacctgacggtcagcggcgagaagatgagcaagagccgcggtacgggcatcgacccgctcaagtacctctcgatcggcctggaccctgagtggctgcgctactacatcgcggccaaactcaacggccgcaacgaggacatcgacttcaaccccgaggacttcgtggcgcgcgtgaacagcgacctcgtgggcaagtacatcaacatcgcgagccgcgcggcgggcttcatcggcaagcgcttcggcggccagctgggcgaggtgtcggccgacggcgacgcgctgctgttcgcgctgcgcgacgcggcgccgcagctgcatgcgctctacgacggccgcgactacgcccgcgcgctacgcgaggtgatggcgctggccgacaaggtgaacgagtacgtcgatcagaacaagccctgggagctggccaagaaggaaggccaggaggcgcggctgcacgacgtgtgcaccgtgtgcatcgaggctttccgcctgctcacgctgtacctgaagccggtgctgccggcgctggccgtgaacgtcgaggccttcctcaagatcgcaccgctcgcgtgggccgatgccgcacaggcgctgcccgtgggccatgccatcggcgactacaagcacctgatgcagcgcgcggatgccaaggtggtcgacaagctgttcgacgcacctgaaccggcgcctgccgccgccgcggaaacggcggccgatgcgctgccgggcggcgaggccatcgcgcccaccatcaccatcgacgatttcgcgaagatcgatctgcgcatcgcgaagatcgtggcctgcgagaaggtcgagggctcgaccaagctgctgcggctgacgctcgatgcgggcgaagcgaagacccgcaacgtgttcagcggcatcgcctcggcctatgagcccgagcagctggtgggcaagctcaccgtgctggtggccaacctcgcgccgcgcaagatgaagttcggcctcagcgaaggcatggtgctggccgccagccacgccgacgaaaaagccaaccccggcatccacgtgctcgaaccctggccaggcgccacgcccggcatgcgggttcgctgaccccaaggacctcccatgctcaaacgcaccctcctcctgttgtcattcgcagccatgctgagcggttgcgcggtggtgactgtggccggtaccgccgtgagcgtgggtgccagtgcggtcggcctggccgcggatgcggccatcggcaccgcgcgcatcacgggcaaggccgtgggcgcggcggccgacgcggtgattccggacagcgactgaacggcggccacccgggccggcgcggggtacacaatgagtgccccatgcagtcaccgctgaacatcacccgctttcgcccgcgcctgctcgacgccctggcgggctacgaccggacgcgttttttcaaggacctggcgcgggcgccacggtcggcatcgtggcgctgccgctggccatggcgtttgccatcgcctcggggctcaagcccgaggccggcatctggacggcgatcatcgcgggcttcctgatctcgctcctgggcggctcggcggtgcagatcggcgggccggccggcgcgttcatcgtgatcgtctacggcatcgtcgaacgctacggcgtggcgaacctgctgatatcgaccgcctgcgccggggtgctgatgttcgcggcggggctgttcgggctgggacggctggtgcgcttcgtgccgctgtcgatcgtggtgggcttcaccaacggcattgcggtgctgatcctgctgtcgcagctcaaggacctgctcggactcacggtggcgaagatgccggcggacgtgttctcgcagctgcatgccatggcgctgcagatcggcaccttcaacccttatgccttcgcgctggggctggcctgcgtgcttggcctggcggtctggccgatgctgctgcgcgatgagtcgaaggtgggccacgcggtgcagcgcctggcgggccgcatggcgcgctcgcgcgcggtgctggtgggcgcgcgcttgccgggacccatcgtggcgctggtgacgctcacgctggtgtcatggggtttcgagctgccggtggaaaccatcggcacgcgcttcggcggcattcccgagggcgccccggccttcgcgctgcccgacttttcgtgggaaacggtcaagcagctggttacgcccacgctgaccatcgcgctgctgggcgccatcgagtcgctgctgtgcgcccgcgtggccgaccagctcagcggccagccgcgccacgacccgaatcaggagctgatggcgcagggcattgccaacctggtcacgcccttcttcggcggcatgccggccaccggcaccattgcgcgcacggtgaccaacatccgttcgggcggcagttcgccgattgccggcatcgtgcacgcggtcacgctgatggtggtggtgctgctggccgcgccgctggcgcgccatgtgccgctcgcggtgctggcgggcattctggtgttcgtgggcctgaacatgggcgaatggcgcgagttcacgccggggcagctgcggcacttcagccgccactaccggctgctgatgctcggcaccttctttctcacggtcgtgttcgacctgacggtggcggtgcaggtaggcatcgtgctggcttgcgccctcttcatccggcgcatgagcgggcttttcagcgtcgagctggtcacgatgcagccaccggtgctcacctatcggctctacggcgcgctgtttttcggggccgcggccaagctggacgaggcggtgaacgcggccgagagcgcgccgcgcggcatgacggtggtgctcgacgccacacacctcatctacctggacgcgaccggcgtcgatgcgctgcgccagctgcaccgcgcggtgctggcgcgcgacgggctgctgcgcctggagtcgctgcagccgcagccgctcgaggtgatcgtgcgctcgggattcgccgacgagctgacgagcggccagccgcacgcggccgagggctagtttgcctcggcgccccggtcgggcgacgagccgctgcgcaccacgcgctggtcgtcgttcaaggtggcggtgaacaccatgggcgaattcggcggctggacccagcgccattcccattcggtttcgcgcttgagcgcgtagggcgtgaccttggcgggcttgccgagcagcttgcgcaggtcttccatcatcatgcccggctgcaccttggcaaagttctcgggcgtcagcacctggcgcagcgcgctcatcttgccgtcggcgccgatggtgatcatgtagttcttctggccctgcggctggcggttgtactcgagcacccggccgttcggcgcgtcccagatgttctcgggctcgccgaacctggcgcgcacgtcggcctcggtcgagacgccctcctccagctcgccgatgcgctgcgggtcgcatcccgaaagccccatcaatgccgccgccaataacgctgttgcacagccgatccgccactgttgtcgtcgcttcatgccatccccggtaaaattcgcgcttcaaaggtccagtctatgtccatcttccgccgcccccactacacctccgagatcaccagcttcatcgaggagatgaaagaaaagaagccgacgctggaagccgaacagcgcgccggccgtgccctgctgtgggacaagcacctcgaccgcagcctgctcgaggaatacagcgaggccaacgtaccgcagcagccgtacgtctaccagacccaagtcaagtaatggtgcccagccggcatccatcgttcgtcctcatcgcctgcagctattgaaatgatagcaagcacccgatgaagggcaacgaggacaacgacacgctcgtggccagcatgcctgaggtggtcgaccaggtcgcgctcgccaggctctatggcgagccgttgttcgcgatgccgaaggacctgtacatcccgccggaggcgctgcaggtctttctcgaagccttcgaaggtccgctggacctgctgctctacctgatcaggaagcagaacttcaacatcctcgacatcccgatggcggggctcacgcggcagtacctgagctacgtcgacgagatccgccagacgaatctcgaactcgcggccgagtatctgctgatggccgcgatgctgatcgagatcaagtcgcgcatgctgctgccgcccaagaaggtggcggaaggcgaagaggccgaagacccgcgcgcagagctggtgcgccgcctgctggagtacgagcagaccaagctgcaggccgccgccatcagcgccatgccgacctacgggcgcgacttctggaaggggcaggtctacatcgagcaatcgctcaagccccgctttcccgacatgaacgtggtcgagctgcgcgatgcgtgggccgacatcatgaagcgcgccaagctcgtgcagcaccacaagatctcgcgcgaggaactcaacgtgcgcgagcacatgagcatcgtgctgcgccacctgcaggggcagcgcttcgtcgagttcgagaaactgttcgacccgtcgcgcggcgcgccggtgctgatcgtcaccttcatcgcgatgctcgagctcgcgaaggaaacgctgatcgacatcacgcaggcggaagccttcgcacccatctacgtgcgcctggcgtactcgccggcctgacagcggagcccggcgtgcgcgacttcgacgtcctcatcgtcggcagcggcctcgcaggcctctcggccgcgctgcacctggcgccgacgcaccgcgttgccgtgctgaccaagcgcgcattgagcgacggctccagcgcctgggcgcagggcggcattgcggccgtgctggccgcgggcgacagcttcgatgcgcatgtggaagacacgctggcggccggcgcgggcctctgcgaccccgaggccacgcgcttcgtggtcgagcatgcgcccgaggccatcggctggctgcgcgaactgggcgtgccgttctccgaagaagcgaaggaaaacggcgggggcctgcacctgacgcgcgaaggcggccacagccagcgccgcatcgtgcacgtgaccgacgcgactggcgcggccgtgcagcaggtgctgatcgagcgggtgcgccgcacgccgaacatcacgctgttcgagcatcacacgctggtcgacctgatcacggggcccaagatcgggctcgatgacccggcctgcctgggcctctacgcgctggacgacgagaccgacgaggtgctggccttccgcgccccgcacaccatcctggccaccggcggcgctggcaaggtgtacctgtacacgaccaaccccgacaccgccactggcgacggcattgccgctgcgtggcgcgcgggctgccgggtgtcgaacatggaattcgtccagtttcacccaacctgcctgtaccacccgcacgccaagtccttcctgatcagcgaggcggtgcgcggcgaaggcgggctgctgaagttgcccgacggcacgcgcttcatgccgaagcacgacgagcgcgccgaactcgcaccgcgcgacgtggtggcccgcgccatcgacttcgagatgaagaagcacggcctggactgcgtgcacctcgacatctcgcaccagccggccgcgttcctgaaagagcattttcccaacatcctcgcgcgctgcgcggagctgggcatcgacatcacgcgcgaacccattccggtggtgccggccgcccactacacctgcggcggcgtgctgagcgatctcgccgggcgcaccgacgtgcccggcctctacgccatcggcgaaaccgcctgcacgggcctgcacggcgcgaatcgcttggccagcaactcgctggtcgagtgcatggtgttcgcgcgcgccgcgaccggcgccatcgccgcggcaccggcgcgcggcagcgcccaactgcctgcctgggacgacagccgcgtcaccgacgccgacgaggccgtggtcatctcccacaactgggacgagctgcgccgcttcatgtgggactacgtgggcatcgtgcgcaccaacaagcgcctggagcgcgcgagccatcgcatcgcgctgctgcaggcagagatccaggagttctatgcgaacttccacgtcacgcgcgacctgctcgaactgcgcaacctggtgcaggtggccgagctgatcgtgcgctccgcgcagtcccgccacgagagccgtggcctgcatttcagccgcgactatccttcgctcgccgagcccaccgcacccacggtgctggtgccgccggccgagtgatcgacccacccgcttcgttttcttcacccaaggatgcccggccaccgacgcccgcagggagaaacccaaccatgtcgaacaccacacccatcgctgaaacacccccggcctcgccctacggcacgctgccgccggcctccccgctcgcctcgcgcaagcccgtgagcctgccgcgcctggccgacatgcacgcgcgcggcgagaagatcgccatgctcacggcctacgacgccaccttcgcggccatggccgacgcggcgggcgtcgactgcctcctggtcggcgattcgctcggcatggtctgccagggcctgaacagcacggtgggcgtgagcctggacaccatgcgctatcacaccgacagcgtttcgcgcggcctgcgccgcgtgctgggcacggcctggctgattgccgacctgcccttcggaagctaccaggaatcgcgcgaacaggcgctcgccagcgccaccgtgctgatgcaggccggcgcgcacatggtcaagctcgaaggcggcggctggaccaccgagacagtgcgcttcctggtcgagcgcggcattccggtgtgcgcgcatctgggcctgacgccgcagaccgtgcatgcgctcggcggctaccgcgtgcagggcaagggcgatgctggcgtgctcctgaagcagcaggcccacgcgctgcaggacgcgggcgccgcgatgctggtgctcgagatggtgccggccgcgctggccgccgaactcaccgccgagctgaagcactgcgccaccatcggtatcggcgcgggcaaggccaccgccggccaggtgctggtattgcacgacatgctgggcatcaacctcggcaagatgccgaagttcgtgcgcaacttcatggccgacgcgtcgggcgtgctgcccgccctcaaggcctatgtgcaggccgtcaaggacggcagcttccccgacgaccaacgccacgcctggtaaggaaccgagaccatgtacatcgcacacaccgtggccgagcttcgcgaccatctggccgcgttcaagcgtcccgccttcgttcccaccatgggcaacctgcacgacggtcacctcgcgctgatcaggcaggccaagccgctgggcgacgtgacggtggcgagcatcttcgtcaatcgcctgcagtttctaccgcacgaggatttcgacacctacccgcgcacctgggacagcgactgcgagaagctgcgcacggccggctgcgacgtgctgttcgcgcccgatgaaaaggcgctctaccccgagccacagacctgcaaggtgcatccggaccctgcgctggccgacattctcgaaggccacttccgccccggcttcttcatcggcgtgtgcacggtggtgatgaagctcttcagctgcgtgcagccgcgcgtggccgtgttcggcaagaaggactaccagcagctgatgacgatccgccacatggtgcggcagttcgcgctgcccatcgagatcgtgggcagcgagactttccgcgccgacgatgggctggcgctgtcgtcgcgcaacggctacctgagcaaggaggagcgcgcggaggccgtgcagctctcgaaggcgctgaaggccatggccgaagccgtgcaagccggcgaacgcgatttggccgcgatcgaagcacgggcaatgcaggcgctggcacagcgcggctggcagccggactatcttgtgctgcggcgccgttccgatctgcaggcgcccacctccgccgatctggccggcgagccgctcgtggcgctggccgcggctcggctgggcggcacgcggctgatcgacaacctcgaaatcgacatctccagctcatgacctacagcgtcaaggaaatcttctacaccctgcagggcgaaggcggccaggcgggcatgccggccgtgttctgccgctttgccggctgcaacctctggaccggccgcgaggaagaccgcgctgcggccgtctgccgtttctgcgacaccgacttcgtcggcaccgacggcacgctcggcggcaagttcagggatgccggccagctcgccgacaccatcgccgcgcagtggccggcgaacgatgccgagcaccggctggtggtgctgaccggcggcgagccgttgctgcaggtggatgcggcgctggtcgacgcgctgcatgcgcggcgctttcgcatcgcggtcgaaagcaacggcaccgtcgtggcgcccgaaggcatcgactggctctgcatcagccccaaggccggcgcgccctgggtgcagcagcgcggtcaggaactgaaactggtgtggccgcagaccgaattcgacctcgacacgatggcgcgcacaggcgagttcacccaccgcttcctgcagccgatggacgggcccgaccgggtcgcgaacaccgaactttgcattgccgaatgcatgaagcagccggtttggcgcctgagcgtccagacccacaagatcactggcatccgctaagcgcggagagacttttcagatgcgattcactatcagccaacgctttttcttcgacgccgcgcacacgctgaagcgcgacatcgaggtcgaaggcagccgccgtatccacggccacacctaccacgccgaagtctggctttcgggccagcgcgatcccgtgacgggcatggtgatcgacctggggctgctgcgccgccgtctggacgaggtgcgcgaactgctggaccaccacctgctggacgacgtggcggggctgcatccgccgacgctggagaacctctgccttttcattgccgatgcgctgccggaattccacgcgtcgctcgcgcgggtacgggtgtggcgagaggcactgggcgacagctgcacgctggagttctaagggttttactccctctccccttggggagagggttggggtgagggctgcggcagcaaagttagcgcgatgttgcgaggcccgctgccctcaccctagccctctcccagagggagagggacaacgcgaattcaggcggcgccgatgcctgcgatcaggctgccagccggctgaccattcttcagcccggccgtaaacgccagcatccggtcaatcggcacccgcgcccgcagccccagcgccggatcgacgtgaatctcgcccgcaccggtttccagcgcgttcgcgagttccaccagcccgttcatcgccatccaggggcaatgcgcgcagctcttgcatgtgcccccattgccggccgtcggcgcttcgatgaaagtctttccggggttcagcgtgcgcagcttgtgcagcatgccggtatctgtggcgacgatgaattccttcgcgtccaggcgccgtgccgcattcaggatcgcggaggtcgagccgaccgcatcggccagcgcaatcacgtcggccggcgactccggatgcaccagcaccttggcggccggatggtctttcatgagcagctcgagctcgagcgccttgaactcgtcgtgcacgatgcaggcgccgttccagctcaccatgtcggcgccggtctgccgctggatgtagtcgcccaggtggcggtcggggccccagaggatcttgcggccctgtgcgtgcagcgcgctcaccacgtcgagcgcgcagctcgacgtgacgagccagtcggcgcgcgccttcacggccgcgctggtgttggcatagacgaccacggtacggtcggggtgctggtcgcagaaggcgctgaattcgtcgaccgggcagcccaggtcgagcgagcaatgggcgtccaggtcgggcatcagcacgcgcttctcgggcgagaggatcttggcggtctcgcccatgaagcgcacgcccgacaccaccagcgtggtggcggcatggtcgcggccgaagcgcgccatctcgagcgaatcgctcacgatgccgccggtttcctcggccaggtcctgcaggtcggcgtgcacgtagaagtgcgacaccatcaccgcattgcgttcgcgcagcaggcggcgaatgcgctccttgagtgcgatgcgctcgccgggcgagggctcgggcggcacgcgcgcccaggcgtggcgggtgtcgcaggcggcgccggcgccctgcgccgcgggctgttcgtagtcgacgtcgatgacggaagcggtcgccatggcggttcagtgctcgggttggaagcgcatcgaataatcgatggccttgacgtccttggtcaacgcaccgaccgagatgcggtcgacaccggtttcggccagggcgcgcaggccctccagcgtcacgccgccggatatttcgagcacggccttgcggtcggcgccggcctcgtcgttgatgcgaaccgcctcgcgcagggtcggcaggtccatgttgtcgagcagcaccatgcgcgcgccggcttccagcgcttcgcgcagctgccccagcgtttcgacctcgacctcgacgaaggctgcgcgctctgccgcgggtgccacggcacgcagcgccgcggccacgccgccggcagcagcgatgtggttttccttgatgagcaccgcgtcgtaaaggccgatgcgatggttcaggccgccgccggtgcgcaccgcgtatttctgcgccaggcgcaggcccggcagggtcttgcgggtgtcgacgatgcgggcgcgcgtgccgcgaaccgcatcggcgtacagggcggtcttggtggacaccgcgctcagcagctgaagaaaattgagcgcggtgcgctcagccgtcagcagcgcgcgggcgctgccctcgatttcgagcacgacctgatcggccgcgcagcgctcgccctcgccgtacagccagcggatgcgggcctctggatcgagctgccgcacggtggcttcgacccagggcgcaccgcagaccacggctgcctcgcgcgccagcacgcgggcaacggcgcggcggccgggatcgaccagcgaagcggtcaggtcgccgtcggccacgtcttcctgcagtgcgcgggcggcgtcggcgtgggccagctcggccacggccggcgccgaaaaatcaaagcgaaggctcatggctctcttgtctcttcagtcttgttggggtgaaccgcgcgggtccgcgggcgcgagcaccgactcgggcaccggatcgcggccggtcagcgaggcaacggcctccttcgggctcagcttgccgtcgagcagcgcgaccacgccttcggcgatgggcatttcgacgcccaggccccgcgcgcgctgcaccacggtgcgtgcgcaatagacgccttcggccacgtgccccagcgaagccacggcctctgccagggtgcgcccctgcgccagcagcaggccgaccttgcgattgcgcgacaggtcgccggtcgaggtcagcaccaggtcgcccaggccggaaaggcccatgaaagtctcggcgcgcgcaccgagcgccaccccgaagcgcgtcatttccgccaggccgcgcgtgatgagcgcggcgcgcgcattgagccccagcgccagtccgtcgcaaaggccggtggcaatggccagcacgttcttgaccgcgccgccgacttcgacacccacgatgtcgtcgttggcatagacgcgcaaggccggcccatggaaggcatcgaccagcgcgtcgcgcaccgccgcatgcgggctcgcggccaccagcgcggtgggccggccttcagcgacttcttgtgcaaagctcggcccgctgagcacgcccgctagcaattcaggagcaacctgcgcccatatctcgtgggccagcaagccaaaggaggcgggagattggtcaagcgcaggctcgacgcccttgcacagccacgccaccggcacggtcgtgccgcgcaaatccttgagctgctggcgcagggcggccatgggcgtggcgactatgacgagttcggcgcccacccgggcttggcggagatcgccggcccgcaccgtgagcgagggcggcaaagccaggccaggcaggtagcggatgttttcgtgcgcggccgagatcgcggcggcctgggccgcatcgcgcgcccagagcgtgacctcgtggcggcccgccgcgttgacagccagcgccgtgccccaggcaccggcgccatgaacgcagatcttcatcggcgttgcggcgtcgtgccaggtttactgcgcgagggtcggcgagggctggccggcggcctgagcctgctgctgctcgtacatcgcctggaagttgatttccgccaggtgcacgggcgggaagccgccgcgctggatcacgtcggccacgttgccgcgcaggtacggatagacgatctgcgggcaggcgatgccgaggatcggacccatctggtcttcgggcaggttgcggatctcgaagatgccggcttgcttggcttcgaccaggaacacggtcttgtcctggatcttggtctgcacggtggccgacacggtgatttcgaagatgccttcagccaccggctgggcgtccacgccaagctggatgtcgacggtgggctgctcctgctcgagcaggatggcgggcgaattcggctgttcgagcgacaggtccttgaggtagacgcgctggatctggaaaacgggatcttgggcttgctggtcggccatggctgaactttcgaggatcaaaacaatgcccgccggggagaggttcccgcagcgggctgcagatgaatggactgaagattatcgcccgacgcccggaccgcttccgcgacgtccggctgctttgtgtatcaggcgccctgcaggagcggaaccaggccgccgcggctgtcgagcgccatcaggtcgtcgcagccacccacgtgggtgtcgccgatgaagatctgcggcaccgtacggcggcgggtgacctccatcatggtgttgcgggcaaccggatcgctgtcgatgcggatttcttcgatctgctcgacacccttggacttgaggatctgcttggcacgaatgcagtaggggcagacggcggtggtgtacatcttgacggcttgcatacgctctagctggggaagacttaggctttttcaaccggcaggttggcctctttccaggccttgaggccgccagcgaccgcctgggcctgctcgtagccgagtttcttggccatggccacggcgcgatgggcgcgggccccggtggcgcacaccagaagcagcggcacattcttgttcttgaccgcgccggtcagcttttcctcgagctggttcaggggcacgttcttggcgccgatcatgtggccggtggcgaactcttcgggttcgcgcacgtcgaccagcaccgcgcgttcgcggttgatgagatgcaccgctccctgggccgtgagcgtgccgccgctggcgccgcgaaccagcggccaggccagcatgccacccgagctgagcgcgatcaggatcagcatccagttggcggtgacgaattcgatcaatttcacgggggttccttggatggcaaacccgggattttagaatgctggttttcccaagcgctgccaaaggcttcccacatgcacaaactggtactgatccgccatggcgaatcgacctggaatctcgaaaaccgcttcaccggatggacggatgtcgacctgaccgaaaccggcatcgagcaggccaagcaggccggccggctgctcagggccgagggctacgacttcgacgtggcctacaccagcgtgctcaagcgcgccacccgcacgctctggcatacgctggacgagctcgaccgcacctggctgccggtggtccattcctggcgcctgaacgagcgccactacggcggcctgcaggggctgaacaaggccgaaacggccaagagatacggcgacgagcaggtgctggtctggcgccgcagctacaacacccctcctccgccgctggaagccgacgacccgcgcagcgaacgcagcgacatccgctacgccaagctgtcgcccgagcagattccgctgaccgagtgcctgaaggacacggtggcgcgtgtgctgccgttctggaacgaatcgatggcgccggccatccgcgccgggcgccgcctggtggtggcggcgcacggcaattcgatccgggcgctggtcaagtacctggacggcatttcggacgacgccatcgtcggactgaacattccgaacggcattccgctggtctacgagctcgacgacgagctcaagccgctgcggcactactacctgggcgatgccgcggccgccgaaaaggccgccgcggcggtggcgtcacagggcaaaggctgaagaaaagaaaacccttgtcggcggtcccccgtggaaccccggcaggcaatttgcttccaagctgtgtatattggctcgacagccgacaaggacaatcactcatgatgggccagaaattgaagattaccggctgggtcgccgctggcgccgttgccggcgtccttaccaccgtctcgttgcagacggtcgcgcgcggctcgcttgcgccgctcccgctcgaggaattgcagcagctcgctgccgttttcggcatggtcaagagcgactatgtcgagccggtcgatgagaaaaagctcatttccgacgccatttccggcatggtggcggggctcgacccgcattcccagtacttcgacaagaagtccttcaaggaattcagggaaggcacgaccggccgattcgtcggcgtgggcatcgagatctcgcaggaagacggcctcatcaaggtggtgtcgcctatcgagggctcaccggccttccgcgccggcctgaagccgaacgacctgatcaccaagatcgacgacaccgccgtgcgcggcctgtcgctcaacgaagccgtcaagcgcatgcgcggcgaggccaacaccaaggtgctgctgaccatcttccgcaaggacgagagccgcaccttcccggtcacgatcacgcgggaagaaatccggacccaatcggtgcgcggcaaggtcatggagccgggctacggctggatccgcctgtcgcagttccaggagcgcacggtcgatgacttcgtgaagaaggtcgaagacatctacaaggaagagcccaacctcaagggcatggtgctcgacctgcgcaacgacccgggcggcctgctcgacgcggcggtggcgatctcggcggccttcctgcccgaaaacgtcacggtggtgtccaccgacggccagttggccgagagcaagtcggtctacaaggcggcgcccgagttctaccagcgccgctccggcagcgacccgctgcgcaacctgcccgccgccctcaagaccgtgccgctggtggtgctggtgaacgaaggctcggcgtccgcgagcgaaatcgtcgccggtgcgctgcaggaccacaagcgcgccaccgtcatgggcagccagaccttcggcaagggctcggtgcagacggtgcgcccgctcggaccggataccggcctcaagatcaccacggcgcgctactacacgccgagcggcacctcgatccaggccaagggcatcgtgcccaacgtgctggtcgacgaaagcgccgagggcagccccttcgcagcccttcgcatgcgcgaggccgacctcgagaagcacttggccagcggccagggccccgagaccaaggacccggaacgcgaaaaggcccgcgacgaagcccgcaagcgcctcgaggaagaagccaagaagccgccgcaggaccgcaaggtgcccgagttcggcaccgacaaggactttccgctggtgcaggcgctcaaccgcctcaagggccagccggtgctcgtgagcaagacgcaggtcatcgtcgacaacaaggaagagaagaaggaaaactgaagcacgcacctgccaaggcagggcgggccgaggcgcgcatggacgatcacgacctgctgcgctattcgcggcacatcctgctcgaggagttcggcatcgacggccaggagcgcgtcagtgccgggcgcgcgctggtcatcggcgcgggcgggctgggttcgcccgtggcgctgtacctcgcggccgccggcgtcgggcacatcgtgctggtggacgacgacgaagtcgacctcaccaacctgcagcgccaggtcgcccacacaaacgcacgcgtgggccgcctcaaggtcgaatcggccgcagaggccatgcgcggcatcaatcccgacatcgccatcgagacgcacgccctgcgcgcggacgaggcgctgctcttgcggctggtcgcggcggctgacgtggtggtcgactgctgcgacaactttgccacccggcacgccgtcaaccgcgcctgcgtggcgcacggcaagccgctggtggccggtgcggccatccgcttcgacggccagctgagcgtgtacgacacgcgcgaccccgcctccccctgttatgcgtgcatctttccgcccgacgcggccttcgaggagacgctttgcgcggtgcttggcgtgttcggcccggtggtcggcaccatcggcacgctgcaggccagcgaagcgctcaagctgctggcggggatcggtccgtcgctggcgggcaagctcctgatgttcgacgggcgccgcacggcgttcgacatgctgaagattgcgcgcgatccgcattgcagcgtgtgcgcgcaacgcccagcaacaggaacctgacgggtagcgcggcgccaaaaggcggcgcagcaggcgcagaaggcctcagcgctgctgcttcgcgcccttcgccttggctgcaccggcggcagccgcaccggttgaaggtttgttggcttgcgccagcacacccttgcaatcggcatcctcgcccggcccggtctcgacggtggcggccagggccagcagcggattgagcgcgcccagcaccagggcggcgatgccgcgctccgccagagacgccgcctgcaccccgccggtcggcgccccgaaggtgccgccgatgaccagcggcgagcgcagcgacaggaagctcttgtccttgggctctgggcgcaccacgaagtcgagcttttcggtcgccaggttggcctggccgctgccatagaaaacggtgtcttcggtgtccagcaccatgctgcggctggtcatgacgcccttgttgacgtcgaaggccatggcggcgcagcgcagttcgacgttctggtcgccgcgcagcagaaacttgatgatctcggcgccgtccagccccatgaactcgagcaacaggttgctgaaccgccctcggccggtcagtgccgcgacgtcgcccgaggcgccgccgagccagcttgccaccgaggttccccggcccgacagattgatccggccatccagcctgctgaagctgcttcgcatggtctcgatcttggggatcaggcggttgagctgcacattgcgcaggtcgagcgaggcgcggatgtccgccgggttctgggtggcgtcgatgcggatggcgccagccagcttgccgccgcccacgcccaagtcgagcggctccagcacaagcacgctgttgttcagcttgatctgcacgctgccgcggtccagcggcatgtcgcgcacgttcttgatccggtcggccacgtacttgacgtcggcgttcatcgcgcgcagccggtcgaagtcgagggtggcgctcggcagcaccttggcgtcccggccgcgcttgacctgcttgatggtggggggcggtgccacgccttcgaccgccttggccgaccgttcggtgggcggcaggccgatcagcgggcccaggtcatccatgtccatcacccgggagcgcagttcgcccgcgaggtgcggcaccttgcccgattggtcgaagcgcatgtcgccggcaatgtcggacaggccgagcctgcccttgagtccagccacctcccattgcttgccgcgcttgcgcagatcgccgctcagcgcatagggagacgtttcaggcagcgcaatgcccagcagggggaacaaggcgccaagggtctggcccttgaggtcgaacttcgcgtcaatgccgtcgaggtcggcaaagtcggtcaccgtgcccgaggccttgagccgcgtctggccggcagcggcatcgacctccagcggaaacggctgcccgccggccgccttgagctgcagcacgttgcccgtgcgcccttcggcggtcagcggctggcccttgtagcggcccttgatgcggtagctgagcggaagcgtgccaaggctggtgtcgtaattcacgtcggcgtgcaggtcgactcccaggtgcttggccaggaaatcgaccgcaccgctgtcgacctgcatcaggccgatgacgggaacggtgccgggatcggaggtgtccttgccgagcgcccaggtacgccgcccgtcggcttccatctgaagaccgagggtgggcgagacgagcgccagccggggaatcacgaccttctgcctgatgaggggccagagccggatgtcgaattcgccgcgctcggccttgaccaggtaggggtcgcgcgcccaagggggattggcgaactcgatgccgtcggccttgatggtggctccgcgcagcccgagcccgacgtcgagccggcgcgtgatctcgaacttgcgcccggtcttttcgctgacatagcggttcaggggttcgcgcagcgtgtcccacggaaagaacgccagcaccaccgccagcagggcgagcagcagcaggaaagcccccagcaccttgagccagagcggtccgttgcgaagctggttgcgaaggacgacattcgttgccatgccgtctgaataaacctgccttggcgtttcacgggtcggcagtggaccgcaaaaaccgtgaggcattgcctacggaatgacgagataaagcggcttcgtcagaacccgcctacaacacgctccccccgaaccctgcatgatgcttgccggcggggcatcaatctcaatgcgcagacacactcgccggcaggagttcggagacacctgccaacgtcagaggaagcgcggttcggcatggataccagattgcagacctatatcgtcgaagacaaccccacgatccgtgaaaacctcattggcactctggaagaacttacctgcacgacggttgtcggctttgccgaaaccgaagcacatgcgaggcagtggctgcacgaccatagcgaagagtgggatttggcggtggtcgatctttttctcaagcagggcagcggactgggcgtgctccaggcctgcaccacgcgacgggccaaccagaaggtggtggtgctcagcaactatgcaacgcccgacatccggcggcgctgcgccgaattcggtgtcgatgcggtattcgacaagtcgaacgagatcgacgcgctggtcgacttctgcatcctcgaggcagcggctcaccgccccgccgcggacactgaccgaggaaaataaaaaagcggccgcaatgggccgcttcttcttcgacgcggggctttcgccctcaatcgatcagcttgttcttcagcgcgtagtacgtgaggtcgctgttggaagacaggttcatcttctccatcaggcgcgtccggtaggtgctgacggtcttgaccgacagcgagagcgtcttggcaatgtcgcccgcggtctcgcccttggcaagcttcaggaacacttggaactcccgctccgaaagttgttcgtgcggcgcagcatcgtccttgcggtcgagctggcgtgcgagcaactccgccaccgccggcgtgatgtagcggcggccgagcgagatggtgcgaatcgcattgacgatctcgatcgggtcgcactccttgttgaggtacccactcgcgccctgccggatgagattcatcgcgtagtgctcttcggggtagccgctcaggatcaggatgcccacgtccggcgccttggcgcggatcatggcaagggcgtcgatgccgctctgcccgggcatggaaaggtccatcaccagcacgtcgagttcggtggtgcgcacgagttcgatcgcttcgcggccgctggcggcttcgccggccacgcgcaagtcgacgtgctcggagaagaactgcctcaggccagatctcacgatggcgtggtcgtccacaattccaattttgatcatctgttactttcttcgttgtgtcgcatctgtggaagctgcaacatgccggtcccctgctagttatcgattattcacgaacttgtgttgaaagcaccttcgaaagtttcatgcactggttagcccctccaaaaatggccgtgagcctcctgctcgcggcgctggctgcgctggcactcgttggcatcaacgaggccggttaccgccagtcgagccgtgccctggcggacatcggcgaggcgcaaaaggtgcgcgccacgctcaaccttatcctgcagaacatgctcgatgccgagaccggccagcgaggctatctcctgaccggcgaaaccagctaccgccagccctacgacgcggcggtcaaacaggtcgacgggcatctggccacgctacgccaactttacgccgaacggccggccgagcgtacgcagttggcggagctttccaagcacgtgctgcgaaagatcgccgaaatggacatgagcgtgcggctgcggcaggacggcaaagacgacgcctggaagttcgtcatcacgaccgacgtcgggcgcgaggaaatggacgccatccgcaagagcgccctcgacctggtcgcaaacagcaacaggaccctgaacgaaagccaggcgcaggtgaagaaatcgctgcagctggcgcgcatcggcaccgccatcgtggcgctcgcggccttttttgcgtttttcctgtacctgcggcagacgcacgcgctgcgctccatcggggaacgccagcaggaaacgctgcagcgggaacgcaacgcgctcgaagacgaggtgcgcgaacgcaccgcgtcgctggccgagttggccacccacctgcaggacgtgcgcgaaacggagcgcggctatctcgcgcgcgagctgcacgacgagctcggctcgctgctcaccgccgccaagctggacgttgcccgtctcaagtcgaggttgctcgaagcgcccgacgccacccagcggctgcagcatctgaccgagctgctcaacagcggcatcgcgctcaagcgccgcatcatcgaagacctgcggccttcgtcgctttcgaacctcggactggtcgcgtcgctcgagatcctcgggcgcgaattcgcggagcgctccggcatccaggtgcagatggcgctcgaacccgtgaccatggacgaatcgcgccagctcacgatctaccgcatggtgcaggagagcctcaccaacatcggcaagtacgcggaagccagcgaggccacgatcgtcctgaagaactacgagaaccacgtgatcgtggaagtcgccgacaacggcaagggcttcgatcccctgcgcgtccacccgtcgacccacggcctcgcgggcatgcgccaccgggtcgaggccgcccggggcaggctcacgatctcgtcgacgccggggcgcggcacccgcctgagcgccatgctgcccaccgtcaaggtgctctgacgcagcaccgcgggctgcgccgccggctcacttgcgcgactcgccgcgccggcggtttccgaggaactcggccatctcctacgcaccccgcgcccggttgctgacaggcccccgcgggggggccacttaaggttgcttccgagccgttcatcctcttcttctttttgaacgggccttcctaaaaactacgagcgaagcctcgaaggagtccacatgttgtactacgcagtggtgtttctggtcatcgccctgattgccgccgtgttcggttttggcggcattgcagccagcgcggtagggatcgcaaagatccttttcgtgatcttcgccgtgcttgccatcgctagttttctggccggcttgctcaggcgcaagtagcgtcgttacgatcagcaggctcccgcaattcatctcccggaaaggaaattctcatgaacacgacgaccaagactccctcgcaaattgccgacgaggcgcgccagactgccagcgacgccgtcgacacgacccgcgcctatgcacagaacgcagtgaatgcggccggcgagaaggtgcgcgaactgcgccgcgatgcggaacccgcggtcgagcaactggcagcgcgcgtgcagcaggcagtgcagcgcggcctcgatgcggcctcgaccacgagtgcccgtgcccagcgccggctcgaacaggcagccgacgtcaccggccgctatatctccgaccagcccgtgcgctcggtgctgattgccgccgcagccggcgccgcaatcaccgcgctcatcgtgctggccagccgcaaccgtcgggacgactactgatccgctgctgctgatacgacgttccaccgatcccgcgcaccatgcttcatccgatcttttccacggtgctcgggcatccggaactcattgccgaacacgcggcgaactacgcggccctggtgaggcaggaggcctccgaggccgggcgcggcatcgtcgcgcgcatcgtggctggcgtgctggcggcggccagtgccatgctggcgctcgggctcatcggcgttgcggtgctgatgggcgtgctgcatggcagcttccactgggtgctggtggccgttcccggcgtcgcgctggtgattgccggcatctgtgcctggctggccgcgcgtccgtttccggcctacggattcgacgacctgcgcgagcaggttcatgcggacctgacggcattgcacgaagcaggagcccgccatgaacgacgctgagcgcacttctctcacgccgaaacagcggcttgccatttcgcgccgggccctcgtcagagagttgaacggcgacgacgagccggacgaccgtccccgcggcaggcgcggtgcggcgccgcaagagccggcgggaatgcccagcgtcgacgacgccggggaccccggccatccgttccgcggccaccgaagatggatctcgatggcgcgcagcatgaccgaacgctggtggcgccgccatccggcccatgcaatgggccagcttgcgcggcccgtgctcgagcactatgcccgcaaggaaccggccaagctcatggcgatcgctgcggccaccggcgcggcgatggtgctgctcaagccgtggcgcctgctctccttcacggcggtgctggcggctgtgctcaagacatccgacgtggctgacgtcgtcaacacgttgatgcagaaaaacacaagcccacgaaaggacccttcatgaatgcccatgtttccacggccacgaacccggcaggacacaagcgcctggtgctcgacgagatagccatcggcgaggcagccaagagcctcgacgaaggcgccgtcacgccgagctacggcccctggcgggacgacgtcgtgaagctgctgaacgacgcgctcgccaccgaactggtctgcgtgctgcgctacaagcgccactacttcaccgccaacggcgtgtcgtcgccgaagatcgccgaagaattcctggtgcacgccaacgcggagtcgggccacgccgaccgcatcgcggagcgcatcgtgcaattgggcggggagcccgactttgcgcccacgcacctgctcgatcgcagccacgccagctacgacgaatccaccgacctgcaagccatggtgcgcgccaacctcgtggccgagcgcattgcggtagaaacctaccgccagatgatcaatctcatcggcgacaaggacccgacgacccggcgcatgctggaagacattctttccgacgaggaagagcatgccgacgaactgaaagactggctcggccactgacgcagtccaagcagtcccgtcaccttgagaaaagcccgggcgaaccgggctttttgcttggcaagggagcgaaggaaacgctcagcccttcacctcgagctggttgttcaccgaggtcacgccctgcacgcccttggcgatctcctcggcacgcgccttggcagcggcattgggggcggggcccttgaggctcacgacgcctcccttggtgtcgacgtcgatcttgagtgcgctcaagtccggatccttcgcgaggccggcggaaaccgacgaggtgatcgcggcatcgtccaccgacgcggacatggcggcgccagcgctcttggcggcgtccttcaggttggccatcccttccttcacctcggcggtggtgttggaggcgtcgatcttggccttggcatccttgacggcctctcgggtcttggcagcagcggtgtcggcagccttctcggtcttcgagatggcactgtcgagcttctcgccggccgtgcggttgtccgacttgtcgcatgcggcgagcgtcagcgcggcgccgaccagcagtacgtagagccatgtgcgcgagtggggcgtggcggtggtttgtcgagtcttgttcatttgaaatcctccagtcgctcgcagggagcggggaaaaaaggcacggccacggcagtggccgtccccactctagctttcatgcaggccggccagggggtggccggcggcccgaaatcctgtaggacaggaaaggtcaagccgtgacgatccagccttcgagcggatcgaaccgctccggcaggccatagcccggcccgggtgtggaagcgcgctgtgcgctccaggccgcctgtaccaggcaaagcaccgcatcgatgtggtcgccgcgggcgtcgtccagcaactcgctgcgctgcacgcggttgagctccagccgcaggccgagccgcgaggcgcctgcctcgagcgcggcgagcaggtcgcctcgcgccgccagccgctcgggcgtctgcctggccagctcgtcgctcttgtagctgcggcgcccgatcagctcgcgggcgagcagccccggataggcctccagcgccacgcggccgccgtggctgccggcgtgcaggccaggcaggctcgcgcccgcggccagcagcggcggcacacctgcatggagcatgaaggcgaccggcgggttgacccatttcatcgacgtgctcgaaccggcgggcgcatcggtcgcccggtgcgcgaacttgccgccgaccggccggcccgcgcagaaggcggcaaaggtggctcggatgtcggcgcgactcaggctgacgtagtgggcgatgagcgcatcccactcctgcggccagcgcagatgctcgaccagctcacgcggaaggccgaacggaaaatcgaagccgccgatccattccggctcggtgcaaagccaccgggcccaggcatcgagagtcgtgaagcgctgcaggcctgtcagcgccagggtgcccgcatcgcccgtgctgcccatgccgcccatggccacgacgatcggtttgcgcggcgtgggtgcgcatgagaaatcgcaaccggtgagcagcatcgcgccagctctcaccccagcgcaagcgccaccatgccggcggcgatgaatgcggagagcgacacccccgaactacgcgcttcgcgcgagcaagcgacaccctcgggggcagcgaggacgcgaagcgccgtgcgtgggggccacgtgacctagtggcggccgacgatggcggcggtggccatcagttcttcgagcagcgccagcgacaccttgcccgacaccgcgtacggattgagctcgggcttttccgaatacttgagcagcgtcgaggcattgagcttggagaggttgacctgccccatggtccagccgccgaagcggcgctcggaaatttcttcgtagtgcagcaggaccacgtccttgtggcgcgcatcgcgctggatgtggccgtacagctcgctgatggcggtgcgcccgccttcgatggcctgcaggaaggtgccggcgccgtagcaaagaatgccggtgatgccgcaggccgtgttgtgcgagcgcgattgcgcgaggatggcctcgatggcctcggggctggtgtcgacggcgcggctggcgtagagaagtctcacgagcatgatcaggcctcccgccgggccaccccaagggaggcctgcgccccctcggggggcagcgaatacacgaagtgatgagcgtgggggttcatttagctccttctcggcaggagggaaaggaattcgcggcgcaggctcgggtctttcaggaacacgccgcgcatcacggagttgatcatcttgctgtccatttccttcacgccgcgccaggccatgcagaaatgctcggcttccatcaccagcgccaagccgtcgggctgggtcttttcctggatcaggtcggccagctgcaccacggcttcttcctggatctgcggacggcccatgacccattcggcaaggcgggcgtacttggacaggccgatcacgttggtgtgctcgttcggcatgatgccgatccacagcttgccgatgatcgggcagaagtggtgcgagcaggcgctgcgcacggtgatcgggccgacgatcatcaactcgttcaggtgctcggcattcggaaactccgtgagcgaaggcggcgccacgtagcggcccttgaacacttcgttgaggtacatcttggccacccggcgcgcggtgttgccggtgttgtggtcgttctcgagatcgatcaccaggctttcgagcacgcccttcatcttgacctcgacctcgtcgagcaaagactcgagctcgcccggcgcgatgaactcggcgatgttgtcgttggcgttgaagcgcttgcgcgcggccgtcaggcgctcgcggatcttcaccgagacgggtgtgccctcgtcgtcattgttgccaccagggcgcggttccacgtcggttttcctcagcatccgcgcatggtatcagcgaacgcattttggctgccggggcgggagaagcagcgcgcagggtgcgaagcgcgccggctcgggcctcaaggcagcgtgaaatcggccaccagcggcaggtggtcggacatgcgcgcccaaattggcccccgcggcaccgagcaggcggccggctcgagttgccgcgcgtagatgaaatcaagctgcgccacgggcaggcgcgaaggataggtaagcgtcggcggaccgcgcaggtcgctggtgtcgcgcaggcccatggcgttcatggcgtggcgcatgcgcgcgccccagtcgttgaagtcgcccgcgaccaccaccgcctcgccagccggcacttcgcgttcgatgaactcgcgcagccgggccacctgccgcacacggctgcccttgatgagccccaggtgcaccacgatggcatgcaccggacgggcctccacctcgatgacgacgtgcagcagcccgcgctgctcgaagcgatggtccgaaatgtcctggtggccggtacggatcactggccagcgcgtgagcaacgcattgccgtgctccccgtggcgcgtgacggcattggtttcgtagacggcggtgtagccctcgggcgccagaaaatcggcttgcggcatctcgggccagcgcgcaaaacgcgcctgcgcctgccggttcatcttgcgcacctcttgcaggcagacgatgtcggcgtcgagctgctcgatggcgtgccccaggttatggatctcgaggcgccgggcaggtccgatgccctgcacacccttgtggatgttgtaggtcgcgacccgaagtgcatgtgccggcaggttcatcgtgcaaattctggcagcaacagaatggcttcggcattcgatggggaaaagcacgcatcggcggcctcgcgataaggcagccatttccaggccgtgtgctcgcgggggtggagcgtgggcaccacgcgctcgggcacgcagagcccgaagagatgctcggtgttgtgcgtgatgccgggttcgtagcgcgcacgccagcccgggtagatttcgtagacgttgcgcagctgccagtcgaccagttgcgccgccagcgggctgccctccccgcactggataccggtttcttcggccacctcgcgcgccgcggtgagcgcgagcggctcgtcgagcacgtccttgctgccggtgaccgactgccagaactcatgggcgtcggcgcgctggatcagcagcacatcgagcgcaggcgtatgaatgacgaccagcaccgactccggaatcttccagggccgggcgatggtcgtcatggtcgcatcaggcgggctgctggacgttgcgcagccggatgtggagctcgcgcagctgcttctcgtcgaccgggctcggcgcctgcgtgagcaggtcttgcgcgcgctgggtcttggggaaggcaatcacgtcgcggatcgactcggcgccggtcatgagcatgaccaggcgatccaggccgatggcgatgccgccgtgcggcggcgcaccgtactgcagcgcgtcgagcaggaagccgaacttgagctgcgcgtcctcggcattgatcttgagcgcgcggaacaccttgctctgcacttcctcgcggtggatacgcaccgagccgccgcccatctcgatgccgttgagcaccatgtcgtaggccttggcaatgcacttctcgggcgcggtgtccatgaggtcttcatggccgtccttcggtgcggtgaacgggtggtgcacggccgaccagcgctggccttcctcgtcgaactcgaacatcgggaagtcgaccacccacagcggcgcccagcggtcgtcgaacaggccgctcttcttgccgaaggcgctgtggccgatcttcacgcgcagcgcgccgatggcgtcgttgacgaccttttccttgtcggcgccaaagaacaggatgtcgccgttgcgggcacccgtgcgggcaatgatttcggccagcgccgcgtcgtcgaggttcttgacgatggggctctgcaggccttcgcggccggcctgcgcgtcgttgaccttgatgtaggccaggcccttggcgccgtagatcttgacgaactcctggtaggcgtcgatctcgccgcgcgagaggccgccttcggcaccgccgcccggcacgcgcagcgcgaccacacggccgcccttcatggtggcggcattcgagaacaccttgaactcgacgcgcttcatgagttcggtgagttcggtgaattcgagcttcacgcgcaggtcgggcttgtcggagccgtacttgaacatcgcgtcggcatagctcatggtcgggaacaccggcaggtcgatgcctgcggcattgcggaacacggtgcggatcatgccctcgaacatctcgcggatttcttcttcggcgaggaacgaggtctcgatgtcgatctgcgtgaactcaggctggcggtcggcgcgcaggtcctcgtcgcggaagcacttcacgatctggtagtagcggtcgtagccggccaccatcaggagctgcttgaagagctggggcgactgcggcagcgcgaagaagctgccgtcgtgcacgcggctgggcacgaggtagtcgcgcgcgccttcgggcgtggacttgccgagcatcggggtctcgatgtcgatgaagccgttggcgtcgaggaacttgcgcgtttccatcgtcaccttgtagcgcagcatcatgttgcgctgcatggccgggcggcgcaggtcgagcacgcggtgcgtgagacgggtggtttccgacaggttgtcgtcgtccagcaggaacggcggcgtgaccgacgggttcagcaccttgagctcgtggcacagcacttcgatcttgccgctcttgagctggtcgttggtggtgccttcggggcgcgagcgcaccaggccggtgatctgcacgcagaactcgttgcgcaggttttcggcgacggcgaaggtgctggcgcggtcggggtcgcacaccacctgcacgtagccttcgcggtcgcgcacgtcgacgaagatcacgccgccatggtctcggcggcggttgacccagccgcacagggtgacggtttggcccatcagggcttcggtcacaagaccgcaatagtgagtacgcatggccatatcttgaaattccagcgccgcgaaggcgcgttttctacttgatcgcgatggacgaggggccgccgggaacgaccacccccatcgagacgatgtacttgagcgcttcgtccacgctcatcttgagttcgatgcagtcgctgcgcttgagcatcacgaaatagccgcccgtgggattgggcgtggtcggtacgtagacgctgaggtagtcgccgccgcccaggtgctcgaccacgtcgctacccggcgtgccggtcacgaaggcgatggtccagactccttcgcgcggccactgcaccagcacggcggtccggaaggcattgccattctcggaaaacagcgtgtcggagacctgcttgacgctcgaatagatggagcggacgaccgggatgcgccgcaccacggcgtcgccccagccgagcaggcgcttgcccacgaaattgctcgcaatggcgcccacgcccagcaggatggccagcgtaagcagcacgccgagcccgcgtacgttgttgtcgtacagccatttctgccagaccgacggcagcacccagagcgtctggtccagcgtgtcgatgatccacttcagcaccgccagggtgatgaacagcggaacgatcaccagcaagccggaaaacagccatttgcgcagggcgagcatggtgtgtgttctcaggcgcccttggcggcggctgcaggggctggcgccggagcaggaataggcgcgggggcgggcgcagggctcgaagcttccgcggtcttggcggccgcggccggcgcggcggcggaatcgccattggccgctgccggggccgttgcgggctcggccttcttgccgccgccatcgcggaaatcggttacataccagccggaacccttgagctggaacccggcggcggtgacttgcttctcgaacgcactcgcgccgcacgtcgggcacaccgtgagcggcgcatcggacattttttgcagggcgtccttggcaaagccgcaggcgctgcacttgtaggcgtagatgggcattggaattgagtggaaaagcggcgcgaactcggcgcaaaggcctgacttaggcctggcaaagcccgctcgcaaagccctcgattataagggccgccccgccaacaggcgcgtcttcaggccggttccgtggccagcagccggtgcggcgtgcgggtattggccacccactgcggcgccagcgatccggccaccatgccggtgaacgaggcaagcaccccggccagctgggccggaaatgccgtgccccagggcagcgccaggaacagcagccagacaccgatgccgaacagaatcgaggcgacggcgccctgcgtggtggcgcggcgccagtacaacccgaacaccagcggcacgaaggcgccgaccagcggcacctggtaggcgcccgacaccaactcgtagatgggcgtgccctgcatgcggatggcgtaggccagcacggccgcgctgaagaccagcaccgtgatgcgcatggtcatgaggttctggcggtcggttcccgcgggccggaactggcgccagatgttctcggtgaacgtgacgctcggcgccagcagggtggccgaagcggtcgacttgatggccgacagcagcgcgccgaagaacagcacctgcatcacgaagggcatcttctcgagcaccagcgtgggcagcaccttctgcggatcttccttcagcagctcggcggtctgctccggcatgatcaggagcgcgctcgccaccaggaacatgggcacgaacgcgaacaggatgtacgccacgccgccgatgacagggccgcgcttggcggccttggtgctgttggccgacatcacgcgctggaacacgtcctgctgcggaatggagcccagcatcatcgtgatggccgcggcaaagaagaacaccatgtcgtgccagttgggctcgggccagaacttgaagaggtccttgctgaccgcgaaggccaccaccttgtcggcaccgccggccatgttgccggcgaacacggcaatgacggcaagccccgcgacgaggatgatcatctggatgaagtcggtcaccgccaccgaccacatgccgccgaacagcgtgtaagccaggatcgagaccaccccgatcaccatgcccgccggaatgctgatggcgccggccgagagcacgttgaacaccagccccagcgccgtgacctgcgccgacacccagcccaggtagctcagcatgatgatgagcgagcaggccacctcgacgccgcggccatagcgctcgcggtagtagtcgctgatggtgagaagcgtcatgcggtagagcttgcccgcaaagaacagcccgaccaggatcaggcaggtgcccgcaccgaaggggtcttcgaccactccgttcaggccgccctcgatgaacttggccgggatgccgagcaccgtttcggacccgaaccaggtcgcgaaggtggtcgtcacgatcatgtagagcggcagatgccgccccgcaatggcgaagtcggtggtgttcttcacgcgcctggcggcgtaaaggccgatcgcgatggtgaccagcagataaacgacaaccagcgtcaacagcacggggactctcctctagaacaacttcacgcgtaccagcacctgcatggcgagcaaccccaatacaaatcccatgccaccatagagaatggcctgcagcagccggttggtgcgcttctgcgcggccagcagttccagcagctcgcggcggtggtcggcgggccgattttcaaggaaatcgtgcagcaggcgcggcaattgcggcagcaattttgcatagcgcggcgcctcggccttgagctgctcgaacagcttccggggcccgatctggtcgaccatccacttctcgaggaatggcttggcggtatgccagaggtcgagctcggggtcgagctggcggcccaaaccctcgatgttgagcagggttttctgcagcagcaccagctgcggctggatctcgacgtggaagcggcgcgaggtctggaacaggcgcatgagcaccatgccgagcgagatttcccgcagcggccggtcgaaatacggctcgcagacggtgcggatcgccgcctccagttcgtcgatgcgggtgccttcgggcacccagccgctttcgaggtgaagctcggccacgcgcttgtagtcgcgccggaaaaaggccacgaagttctgcgccaggtattccttgtccgactcggtcagcgtgccgatgatcccgaagtcgagcgaaatgtagcgcccgaaggtctcgggcacgaggctcacctggatgttgcccgggtgcatgtcggcgtgaaagaagccgtcgcgaaacacctgcgtgaagaagatggtgacgccgtcgcgcgccagcttgggaatgtcgacgccggccgcgcgcaggcggtcgagctgggcaatgggcacgccgttcatgcgctccatcacgatcacctcggggtggcagaagtcccagaacatctcgggaatcagcaccaggtcgagcgaggccatgttgcggcgcagctgggcggcattggccgcttcgcgcaccaggtcgagctcgtcgtgcaggtatttgtcgaactcgccaaccacctcgcgcggcttcaggcgcttgccgtcgggcgagagcttctcgacccagccggccatcatggccatgagcgccaggtctttctcgatcacgccgcgcatgttggggcgcagcaccttgaccgcgacctcgcgcacctcgccctcgttggtgcggatggtcgcgaagtggacctgcgcgatcgacgcgctggcgatcggcgtctcgtcgaactgcacgaacacgtcgcccacgggacggcggaaggcgcgctcgatggtcgcaatggccaccgacgaggggaacggcggcacgcggtcctgcaggaaggcgagctcgtcggcgatgtcgggcggcagcaggtcgcgccgggtcgacagcacctggccgaacttgacgaagatcgggcccagccgttcgagcgcctcgcgcagccgctggccgcggggcgcatcgagattgcggccgatggagacgacgcgcgccaccacgcgcagccagggtttctggaagctcgtgagcacgagctcgtccaggccgtagcgcagcgcgacccagacgatgaaaagcccgcggtagaagcgcctcattcgggcgtgctcgccgagccggccgacgaaccgccggcccgctggggcttgcgatcgccgacgaactggcgcagtgcgcccacgacacggcgcgcgccattggcaatggtgtgtgccggcacgtcgccgaccaggcgggcgaggtcgtcctcgacatcccagcgcacgtggtcgaccagccagttgacctcggccgcgagctgcacgtcgccgatgatctgcacagaaggcttgccgccgcgcagcgtggcacgggccagctcgaagggggattcgtcggtgacggtgagcgtgagctcgggcaccgatccggcgggcgccaggtcgagaaggccggcgggcgtggccaccagctccattgtcacgaagcgccactggaagcgcaccacccgcccctgctggcggagcagccgctgctgggcctcgggctcctgctgcagcacatggttcagaaacagcaccgcgcgatgctggatctcgtgcaccgcccaggcgggcggctgcagacgctcgccgatgcgattgaacagatcgtcgagaaaagaaaatggggacgatggtgtagccatgtccccattatcggttctgcggacggcctcccggccgccggaatgcgcttactgcaacgcttgcacgcccgccaccagccagccgctggtgccgctggtgggcttggtcatgttccagacttcgcggaacgggcccgggccggcggaagcatcttcgcggatcatgccggagaactccacgctggccatgtagacgtcagccagttcctcgatgccaagcagcttggcgtcgagcatcacgacttcggtcttgttcgaggcgccgccggtgtggctggcgcgatcggccagctgggtgcggatctcgtcgaccatgccgtcggtcatcatcgagcgcagggtcgtgacgtcggcgcggtcccatgcgtcctgcagggtcacgaagttgcgcttggcggctgcaagaaagccgtccacgtcgaagccgaccggaatgccccacgcctgcgaacccgacagcgccgagccgatcatgctgccgccggccgccgcgcctgccgcggaaaggctgctgccatgccgctcgtcggtgtgtgcgggcgtggcgtcgaaggcgctcgtgttgcgctcccagggccgggccgacgcgtcattgccgacattgttcgggctgtactgcgccggggagccggcattcgccgggttgcccgcgccttcgaaggcgaagccgcccgggcggttggcacccgacgaggctgccgaacgcgccttgaacatgcgccagacgaacagcgcagccatcacgagcagcccgatcaacaggatgttggcaaagccggcgccaaggcccagcgaattcgcgagccaggccaggcccaggccggcggcgaggccaccgagcatggcgccccatggacgcttcggcgccgcggcggcgggcgccggcgtggcgggcttcggcgcggcgttggtcgcgctttgctgcgctggcgcggtgggcgatgcggattcgcgctgcgtcacgttggacgactggcggccgaccgacttgccgccgccgatgcgtgctgcatcggcttgcacgctgaccagggccagcacgcaggccaggaacaaagaactcaaacttttcatgtcgtctcctcttttgagcgaagaattcgcgtcatcaacacttgattccaacatgaagggcgaccacgccacccgtcatgttgtgatagtccacatgcccgaaaccgccctctttcatgagggtcttgagttcatcctgcgcggggtgcatccggatggattcggccaggtagcgatagctcgcatcgtcgcccgccaccagcttgcccaggcgcggaagaacgctgaacgaataccagtcgtaggccttggcaagcggcttggcaaccttcgagaactcgagcaccaggagcttgccgcgcggcttgagcacgcggttcatttccttcaaggcaaggtccttgtgcgtcatgttgcgaaggccgaacgccacggtcaccacgtcgaaatggtcgctcgggaacggcagcttttctgcgtcgcacaccagcgtgggcagcgccacgccggcgtcgagcaggcggtcgcggccggtgcgcagcatggcttcgttgatgtcggtgtgcaccacctggccgctggcgccgaccttcttggagaaggccagcgcgaggtcgccggtgcctcccgcaatgtcgagcacgcgcgaaccttcgcccacgttggccaccatcacggtgtaggccttccaggcgcggtgcagccccatcgacatcaggtcgttcatgaggtcgtaacgcgtcgccacggaatcgaagacgccgcggacgcgctgcgctttctcgctttcgtcgaccttttcgaagccgaagtgggtggtgctcatgggactgatattagggcggaagctcacacctcaagaacgcgaccctccgaagacggcgggcttttgttgctttttcttcaaatagcggggcgccgaaggacgcgccgcgtctgttgcgaggcaatgcttcaggagcggacgcgttcgcgccgggtcagtggctgccgcaggcggcaccgcccttgtcgagcatcggcgcatcgcggtcgacgcccgccgcggcgagccggcgttcgtactcggcccagagctcggcctctttggcgccgagttcatacagcaggtcccacgagaagatgccggtgtcgtgaccatcgctgaagacgggctgcacggcatagttgcccaccggcttcaggtcgaccagttcgacgtcgcgcttgccggtctgcaagatttcctgccccggaccatgcccctgcacttccgcggacggcgagtagatgcgcatgagctcgaacggaatgcggaaggtggcaccgtcggaaaacccgacctcgagcacgcgcgactggccgtgcacggtaatcgattgcggcgtcggtgcgccggcttgcaaacctgccatcagaagctccttgtgcccagtcgggccatcatcgcacgctccaattcgggcaggcgcgcggccacggcagccagttgggaagcattcgcctcgcgctgcaccggagcccagaccgaaccgggaaaatgggtgtcgtcggcaaaacgcgcaatcacgtgccaatgcaggtgcggcaccatgttgccgagcgccgcgaggttgatcttggccggcgacagatgctcgcgcaggcactgctcgaccaccgtcacggcctccatgcacagcgcgcggtcggcggcatcgagatccgaaaactccgccgcatgctcgcgccagatcacgcggtagaaggccggaaagcccgcctcttcggcatggatgacgcgaagcttcgcgccttcgaacacgatgcgacccccggggccttcgcagaacggacagccgggaaccgggccgccgccgatcgtggaggccatggtcataccagcacccgctcgatcccgccctggttggcagcggccacgtattcgggcatccagtccttgccgagaatcttgttggccatctcgaccacgatgtagtcggcttcgagcaggccgttgttcaggtcattgccgtagcgcgagaggccttgcaggcagctcgggcagctggtcaggatcttcacgttgtccttttcgccgacctggccgttcgcgcgcaacgcggcctcgcccttcttgagctcttcttccttgcggaaccggatctgcgtcgagatgtcgggccgcgacacgcccagcgtgcccgactcgccgcagcagcggtcgttcttgagcacgttgtcgccgaccagcgccttcacggtcttcatcggatcctgcagcttcatcggactgtggcaggggtcgtggtacaggtagccgccaccgcccgcatcggccagcgtgatgcccttttcgagcaggtactcgtggatgtcgatgatgcggcagccgggaaagatcttgtcgaactggtagccctgcagctggtcgtagcaggtgccgcagctcaccaccaccgttttgatgtccaggtagttcagcgtgttggccacgcggtggaagagcacgcggttgtcggtgatcatcttctcggccttgtcgaactggccgctgccgcgctgcgggtagccgcagcacaggtatccgggcggcagcaccgtctgcacgccggcatgccagagcatggcctgcgtggcgaggcccacctgcgagaacagccgctccgagccgcagcccggaaagtagaacaccgcttcggtctccgacgtggtggccttcgggtcgcggatgatcggcacgtagtcggcatcctcgatgtcgagcagcgcgcgcgccgtctgcttcggcaggttgcccggcatcttcttgttgatgaagtggatcacctgctccttgatcggggccgggccgagcgtggccggcggcgcagcggtctgcttcttggccaggccgcgcagcaggtcgttggccaggcgctgtgccttgaagccgatgcccaccatgcccgcgcgcactgccttgatggtctgcgggttggtcgcgttgagaaagaacatggcggccgcattgccggggcggaagctcttctgccccatcttgcgcagcaggttgcgcatgttcatcgacacgtcgccgaagtcgatcttcaccgggcacggcgtgaggcacttgtggcacacggtgcagtggtcggccacgtcctcgaactcttcccagtgcttgatgctgatgccgcgccgggtctgctcttcatacaggaaggcctcgaccagcagcgaggttgccaggatcttgttgcgcgggctgtacagcaggttggcgcgcggcacgtgggtggcgcacactggcttgcacttgccgcagcgcaggcagtccttcacgctgtcggcaatggcgccgatgtcgctctgctgcatgatcagcgactcgtgccccatgaggccgaagctcggcgtgtaggcgttggtcaggtcggcatgcagctcgacgttttcgccggcgggcgggcgcaccagcttgcccttgttgaagcggccttcggggtcgacgcgctgcttgtagtccatgaagggcttcagctcttcgtcgctcaggaactcgagcttggtaatgccgatgccgtgctcgcccgaaatcacgccgtcaaggctgcgcgccagcgccatgatgcgcaccaccgcggcatgcgcggtctgcagcatgtcgtagttgtcgctgttgacgggaatgttggtgtgcacgttgccgtcgccggcatgcatgtgcagcgccacccacacgcggcccttgagcacctgcttgtgaatggcggtgcactcggccaggatcggcgcgaactcggccccgctgaagatctcctgcagcggctggcgcagctgggtcttccagctggcgcgcaaggtgtggtcctgcagctgcggaaacagcgtgtcgacgtcgcgcagccattcggcccagagcgcacgcacgctctgcaccagcgccacggcctgcgccacgcggtcttcgagcagctcggccgcgggaatttcgtgcgcatcgtcggtcttgccgagcggcaggttgccgcgcagcagaaaggcctcgagggcgtcggtgagttccagcttgttttgcagcgagagctcgatgttgatgcgctcgatgccgtcgctgtactcagccatgcgcggcagcggaatgaccacgtcttcgttgatcttgaaggcgttggtgtgcttgctgatggccgccgtgcgcttgcggtcgagccagaatttcttgcgcgcctcggggctgatggcaatgaagccttcgccgctgcgcgaattggcgatgcgcaccacttccgacgtgacgcgcgccacggcatcggcatcgtcgcccgcgatgtcgccgaacagcaccatcttcggcaggccgccgtgcttcttcgacttggtggcgtagcccacggccttgaggtagcggtcgtccagatgctccaggcccgccagcagcacgccggagcgcttctgctcggcgaacatgaagtccttgatctcgacgatgctcggcaccgcatccttggcgttgccgaagaactccaggcagacggtgcgcgtgtgcgccggcatgcggtgcaccacccagcggcagctggtgatgaggccgtcgcagccctctttctggatgcccggcaggccggagaggaacttgtcggtcacgtccttgccgaggccttccttgcggaaggtgcggccggggatctcgaggcgctctgtgcgcagtttggtcttgccgtcggcggcgtaatactgcagatcgaacacggcgctttcggcgtcgtggatcttgccgaggttgtggccgatgcgcgtgacttcgagccattcggcctgcggcgtcaccatgcgccacgaagccaggttgtcgagcgccgtgccccagagcacggccttcttgccgcccgcgttcatcgccacgttgccgccgacgcatgaggcctcggcggaggtcgggtcgaccgcgaacacatagcccgcgcgctcggcggcgtcggccacgcgctgcgtgactacgcccgcctcggtccagacggtggccacgggtgcatcaaggcctggaagcgagaccatctcgacctcggtcatggcctcgagcttctcggtgttgatgaccacgctcttccacgtgagcggaatggcgccgccggtgtagccggtgccgccgccgcgcggaatgatggtgagccccagttcgatgcagcccttgaccagcagggccatctcggcctcggtgtcggggcacagcaccacgaagggatattccacgcgccagtcggtggcgtcggtcacgtgggacacgcgcgagaggccgtcgaacttgatgttgtccttggccgtgaggcgacccagcacgcgcgtggccttgcggcgtagagccgccacgtcgcgaaaagcagtatcgaaggcggcaacggcctggccgacgagccccgtgagttcgcccacgagctggtcgcgcggcaggtcgctgtcgggggtgcggcgcttctgcacttcgcccagccggtgcttcagggcgtcgaccaactgcccgcggcggcgtgggttgtcgagcaggtcgtcgacgaggtaagggttgcgctggaccacccagatgtcgccgagcacctcgtagagcatgcgggccgaccggccggtgcggcgctcggcgcgcagggtctggagcagttcccagccgcgctcgcccaacaggcggatcacgatctcgcgatcggaaaagctggtgtagttataggggatctcgcgcagtcgtacaggctctgcggcctgcgacaacagcgtggtcaacgcggtcggagcattcatcgggggtggcacctcggccaggcgctgcgcgcccatctagccgggggtgggattttagggcagggaccggggtcttgccttgggctgccgctgtacccctgttgggaggcgtcgggcacgcggtatggcgcgggggttgaggccgtctgccctcaccccaaccctctcccagagggagagggagcaagaccggaactaggcctcagaacagcacgcggctgcggatggttccgttcaccttggccagtttctccagggccaggtcggaataggccgcgtcgatgtccgtcaccacgtagccgatcttctcgttggtctgcaggaactgcgaggagatgttgatgttgttgtccgagaagatcctgttgatctccgacaacacgcccggcacgttgcggtggatgtgcagcagccggtgcttgccagggtgggccggcagcgccacctcgggaaagttgaccgaggaggtcgaggtgccgttgtcgctgtacttcaccagcttttccgccacctcgaggccgatgttggcctgcgcctccatcgtcgagccaccgatgtgaggcgtgaggatgacattgtcgagcccgcgcaacggcgactggaactcgtccttgttggttcgcggctcgaccgggaagacgtcgatcgcggcgcccagcagcttgttctgcttcagcgcctgggccagtggctcgatctcgacgaccgtgccgcgcgaggcgttgatcaggatcgaacccggcttcatggcggcgatttccgccgcgccgatcatccattgcgtggcctgcgtctcgggcacgtgcagggtcacgatgtcgctctgggccagcagctggtgcagttcgcgcacctggcgcgcattgcccagtggcagcttggtcaccacgtcatagaaggccacgttcatgcccagggcctcggccagcaccgacaactgggcgccgatggagccgtagcccacgatgcccagcgtcttgccgcggatctcgaatgcgttctcggccgacttgagccagccgccgcggtgcgccaccgcgctcttttcaggcacgccgcgcagcagcaggatggcttcggccagcaccagctcggccaccgagcgggtgttggaataaggcgcgttgaacaccgccaccccgtgctcgcgcgcggcctccaaatcgacctggttggtgccgatgcagaagcaccctgccgccaccagcttctgggcggccgcaaagacctcggccgtcaattgcgtgcgcgaacggatgcccaggaagtggacgtcggcgatcttggccttgagctccgcatcgggcagcgcacccggcagcgactcgatgttggtgtagcccgcggcgcgcagcacctccacggccgaagggtggatgccctccagcaaaaggaacttgatccggcttttttcgagggaggttttgctgctcatgacgtactcgcggaagccccggccgcggcaacaggctaggccgaaaaaggcgaatgcgatgctagcatgctgcggcgcaacatgaagacccgcgccctgccggaagccttgcgccaaaggggttttcccgattggaagatgacagaggtccgtgcgccaatgtgacgcggatgtgtcatccacatggcctagcatccgcgctttcatttcccatcaggagtcttcatgcgattcaagacgctcgcgctggcatcggcgctggccgccaccacgctgttcaatgtggcccacgcccagaccgaaatccagtggtggcattccatgagcggcccgctcggcgaatgggtcaacgacctcgccaagcagtacaacgccagccagaaggacttcaaggtcgtggcgacctacaagggccagtacgacgaatcgatgaccgccgccatcgcggcctaccgtgccggcaatgccccggacatcctgcaggtgttcgaggtcggcaccgccaccatgatggcctccaagggcgcgatcaagcctgtgggcgaggtgatgaattcgggcggcgccaagttcgaccccagcgtgtacgtgcccgccgtgtcgggctactacaccgcgcccaatggccagatgctgagcttcccgttcaacagctcgacgaccatcttctattacaacaaggacgccttcaaggcggccggcctggaccccgagaaggcgcccaccacctggcccgaagtgatcgccgcggccgacaagctcaaggccagcggccacaaatgccccttcaccaccagctggatgagctggacccagctcgagagcttctcggcctggcacaacacgctctatgcgacgcagaacaacggctttggcggcacctcggcgcgcttggccttcaactcgccgctgcaggtgaagcacttcgagaacctggccaagatgtcgaaggacggcaccttcgtctacaagggccgcaacaacacggccgacgccgccttcccctcgggcgaatgcgcgatgatgaccggctcctcgggcctgtacgcgcgcgtggccaaggacgccaagttcaagtacggcatctccaccctgccctactaccccgacgtgaagggcgccccgcagaacaccgtgatcggcggcgccagcctctgggtcatgtccggcaagccggccgaccactacaagggcgtggccagcttcttcaccttcttgtccgacaccaaggtgcagtccgacagccacaagcgcacgggctacctgcccatcaccacggcggcctacaagctgaccgatgcttcgggcttctacaaggacaacccaggcaccgacgtggccgtgacgcagatgatccgcaagaccaccgacaagtcgcgcggcgtgcgcctgggcagcttcgtgcagatccgaaccatcatcgacgaggaaaccgagcagatctggaacggcaagcgcaccgccaaggaagccctcgatgccgccgtcaagcgcggtaacgagcagctggagcgcttcgagaaagcaaacaaaggctgaagctccggtcggctctgcgccgaagtagactcgcccgcccgccactgcaaaagccgtgggcgggcgtttcgttttttgagggattcgaggggctatggaaaaacgcgttctattccgatcggcatggctgccatggctgctgatcgcgccgcagatggcggtgatcctggtgttcttcttctggcccgccagccaggcgatctggcagtcgatgcagaccgaggacgccttcggcacctccaccgtcttcgtgggcctggagaacttcaagaacctgttcgatgacccggcctacatcgagtcgttccaggtcaccgcactgttctccgtgctggtggccggcatcggcatctcgatatcgctcctcctggcgatcttcgccgaccgcatcctgcgcggttcgttgttctacaagaccttcctgatcattccgtacgcggtggcgccggcaatcgcaggcgtgctgtgggtgttcatgttctcgcccagcatcggcgtggtgagctacggcttgcgccagatgggcatggactggaaccacctgctcaattccaatcaggcgctgtcgctgatcgtcgtggccgcgatctggaagcagatctcctacaacttcctgttcttcctggccgggctgcagtccattcccaaggcactgatcgaggccgccgccatcgacggcgccggtccgctgcgtcgctttctgaccatccagttcccgctgctgtcgcccaccacctttttcctgctggtgatcaacgtggtgtacgccttcttcgacaccttcgcgatcgtgcatgccacgaccgaaggcgggccgggccgagacaccgcgatcctggtctacaaggtctggcacgacggcttccgggctctcgacctgggcggctcggccgcgcagtcggtggtgctgatggtgatcgtcgtcgtactcacggtgatccagttccgctacgtcgaaaagaaggtccagtactgatggcgcatcctttcccttctgcattctttctccggagcaaccgccatgattgaacgccggcccggcctcaccgtcctgtcgcacgtggtgctgctcctgggcatcgccatcgtggcctttcccatctacctggccttcgtcgcctcgacccacacacgcgacgagatcctgcgtgtgcccatgccgcttgtgcccggtgcgcacatggtcgagaactacaccgcggccctccttggcaccgagacgcagggcgcgcgcgtggtggtgggccgcatgatgtggatcagcctggtcaccgcgctggtcatcagcatcggcaagatcgcgatctcgctgctctcggcctttgccatcgtgtatttccgctttccgttcaagaagatcgtgttctggatgatcttcgtgacgctgatgctgccggtggaggtgcgcatcctgcccacctacaaggtgctggccgacctgaacatgctcaacacctacgcgggcctgaccatcccgctgatcgcgtcggccacggcgaccttcctgttccggcagttctttctctcggtgcccgacgagctggtcgaggccgcgcgaatagacggcgcggggccgatgcgcttcttcaaggacatcctgataccgctgtcgcagacttcgatcgctgcgctcttcgtgatccagttcatctacggctggaaccagtacctctggccgctcctggccaccaccagcgaggacatgtacccggtggtcatcggcatcaagcgcatgatcgcctcgggcgacgccgcggtcgactggaacctcgtgatggccaccgccatgctggcgctgataccgccggccatcgttgtggtgctgatgcagcgctggttcgtcaagggcctggtcgacacggagaaatgagcccacccccgaagcggctcacttcgtgtagccgcctccccctcgagggggcaacaccggcggcccggcagagccggttccgcggtgtttcccggcttggggcgccagccacaacctgatatttaaaaccgacaacatgtcagccatttcctttcgcaacgtcatcaagcgctacggcaagggtgccaaggccaaccaggtcatccacggcgtctcggccgaggtgaacaagggcgaattcgtcgtcatcgtcgggccctcgggctgcggcaagtccacgctgctgcgcatggtggccggcctggaagacatttcggccggtgacatcgccattggcgggcgcgtggtgaacctgctcgaaccttccgagcgcgacatcgccatggtgttccagaactacgcgctctatccgcacatgagcgtgttcaagaacatggcctatggcctgaagatcgccaaactgcccaccgacgagatcaagactcgcgtcgacaaggcggccaagatcctcgaactgggccacctgctcgagcgcaagccgcgcgagctttcgggcggccagcgccagcgcgtggccatgggccgcgccatcgttcggcagccgcaggtgttcctgttcgacgaaccgctgtccaacctggacgccaagctgcgagcgcagacccgcctggagatccagaagctgcaccgcgagctcggcatcacctcgctgttcgtcacgcacgaccaggtcgaggccatgacgctggcgcagcgcatcatcgtcatgaacggcggcgtgatggaccagttcgcaacgcccgaagaggtctacaaccggcccgccaccaccttcgtagccagcttcatcggctcgccgccgatgaacctgctgcgccatgcgcctggcgtgcggcccggccagatcctcggcattcgccccgagcacatgaagctcgacgaaagcggctggtccgtgcaggtcgagtcggtcgagctgctgggcgccgagcggctggtgtatgggcgcatcggcgaagagcagatcatcatgcgcaccgacgaaagcgaccacccgccagtcgcgggggacacggtaaaaattgcggcgcgccaggacaagctgcactggttcgacgccggttccggcaaacgggcagactgaacgatgccagcgctgcagccctggccctaccctcgctggatcgcgcaccgcggcgccggcaagctggcgcccgagaacacgctggccgctttccggctcggtgcctcgcacggctaccgcatgttcgagtgcgatgccaagctcagcgccgacggcgtgccttttctcatgcacgatgccacgctcgaccgcaccaccaacggccatggcacgggcggcgcgcaaccctggagcgcgctcgcgcagctcgacgccggtggatggcattcgcgcgccttcgcgggcgagccgctcgccacgctcgagaacctggcgcgcttctgccttgccaacggccatctgctcaacatcgagatcaagcccacgccgggtaccgagcgcgaaacgggcgaagcggtggcacggctcgcggcccagctttggcagggcgcagccattcctccgctgctcacttccttccaggccgaatcgctggcgggagcgaaggcggtccagcccgagctgccgcgcgggctcctgctcgacacgctccgggagggctggcttgcccttgcaaccgacctcgactgcgccgccatcgtctgcaaccacgcactctgggacgccgccacggtggcgcaagtgcacgacgcaggcctgcgcgcgctgagctacaccgtcaacgatgaatgggccgccgagcggctgatcgaactcggtaccgacggcatcatcaccgaccgcgtcgacctcttcagtcccgccgcttgaccgctgccggccgcagcggctcgtcacacgttgcaacgagccgcgccgcgggccggaaatggcgccttctatgatggcagccatgagtttgatcccccgcctgatggccctttgcctggccgccttgctgtcgtgcggcactgcgatggcgcagcccgacagcaacatcggcagcagcagcaccgccacggctcccgtgcccgaacccacggtggccgaactgcgcgagcagctcaccaagatcaccgcctccgccgattccaacgaggacatgcgcaagctcctggcgcagatcagcgacatcggcacgcaggccgacaagttcgtcgccgcgcgcgccagcgaactggccgacctgaacgcccgcctcggggagctcggaaatccgccggccgccggcgccaccgaagacccggacatcacgcgccagcgcagccggctgacaaaagaacgcaacgcgctggatgccgacatccggctggcgcgcctgctctccatcgacgtgcggcagcgcgccgccgaactggtgacccagcgccgcgagctcttcgaggcgcagatcaccgagcgcgccgcttcgccgctgaccggcgagttctggcgcgacctggaggcggcgtggccgaacgacctgacgcgcctgaaggcgatggtggctggcctgcgcgacgggctcgcgcaagcgatgcaggaggagacgcggatcgccctggttggcgcgctgatcctggcgctcttgctcgcggtgctcggcaactgggtggccgagcatctgctgacgcgcatcgccgcccgggtgctgccggcgggccggcttcggcgttcgctgctggtgattgccatcgtggcgagccatgtgctgctggtcgctgcggccgcccacgggttcgtgcgcgtgctcgaggaatacgccacctgggagtcgcaggcgcgcaaggcgatgcgttcgatggcccaggcgctggtgttcatggccttcgtcatcggtttgggccgcggcctgctggccacccgccggccctcgtggcggctgccgccgattcccgacgccatggcgacacgcctcgcgccgctgccgtggctggtggcgatggtggctgcactggcatgggcgccggtcgagatcaatgcgttggtcgaagccagctttgcgaccgtggttgccacgcacgtgctcaccgcgctgatgctcaccgcgctggtcggcgcggtgctccggcggctgcggccgctgcgcgccgatacgcccgacgccgacctgccggagcggccgatgtgggtgggcctgctggtggcctgcatcggcgtcctgatgctgtcgatctgggtgctggtggccctgggctacgtggcgctcgcgagcttcctggcctcgcagctcacctggagcggcatcgtcgcggccgccttctacgtgctgttcaagtttgccgacgacgtcttcatggccggcgtgtcgtcgcgcagcaccttcggccagcgcctgcagaaaagcttcggactcgcgccgcagacgctcgaccaggcggccaccgtgctctcgggcctgagccgcgtggggcttttcttctacatgctgatcgcgctcgcggcgccccttggcaccgggcccagcgaagtgttccagcgcagcggcaagttcggcaccggcgtgaaggtgggcgaattccaactggtgccgggcgccatcctgagcgccatcgccgtagcggtgatcggcttcatcgtgctcagggtcttcaagcgctggctcgcgcgcagctacctgcccagcacgcagttcgaacccggcatgcaaagctcgatcaccacgctgctcggctacgtgggcggcatcctggtggtcgcgttcgcgctgtcggcgctgggcatcggcatcgagcgcatcgcgtgggtggccagcgcgctgtcggtgggtatcggcttcggcctgcaggccatcgtgcagaacttcatctcgggcctcatcctcttggccgagcagccggtgaaggtgggcgactgggtggtgctgggcaccaccgagggcgacgtgcggcgcatcaacgtgcgtgccaccgaaatccagctcggcgaccgctcaacgttgatcgtgcccaactccgagttcattaccaagaccgtgcgcaacatgacgctggccaacgccgaaggccgggtgctcatccgcctgccgatgccgatgaccaccgacgcgcagcgggtgcgcgagctcatcctggaagcatgccgcgcgcacgaaggggtgctcgagacgcccgcgccttcgctcacgctcgagggcgtcgagggcggcctgctcattttccaggccattgcgtatgtaccgagcccgcggctggcgggcggggtgcgcagcgacctgctgttcaccattcttgagcgcatgcgggtggagcggatcgagctggtgccgtatgcggcggtgccgccgccagtggctggtggcgagacaggaccggtggccgcctaggtgctgggccgatcaccccgaatctttcgttgactgaagcaacatccagaaacgcccctcgggatcgggcgctttccagcccctacctttgccagccgcgcgacaccagccattggctggtcccgcacgcaagcacgagcgcggcgtaggcgcccatcgtgccatcgcgtcccgaaaagatcagcccgcccaggagcgccgccgcgccggcgccgcaattgaccgcggcttgaacccaccaggcgggcgcgccggactttcgccccaaaaccccgcccgccagcgcgcacacgaatccgaccgccagggcgggtgccaggaagttgagcagatgattgaggagatccagcagggacatggagggggataagagaggcgagaggcggccaaacccctcggcagccgcatagctcctgctgattttataatcagcggatatgtcagtctgggccctcgggttgaaccacacgaccgcgccgctcgacctgcgcggccgcttcgcgttcgcgctagaccagctggctcccacgctgcacagcctgcgcagctcgtttgccgccggccgccacccccaggtcgaagccgcgatcatctcgacctgcaaccgcaccgaaatttattgcgccgccgagcatgcggcgctcgaccacacggtgggctggctggccgagagcggcggcgtggcgcccgccctgctgcgctcgcatgcctacaccctgcaagatgaccaggctgcgcgccacgtcttccgcgtggccagcgggctcgattcgatggtgctcggcgaggcccagatcctcggccagatgaaagacgccgtgcgcgcggccgaaaccgccggcgcgctcggcagcacgctcaaccagctgttccagcgctcgttcgcggtcgcgaaagaagtccgcaccgcgaccgagatcggcgcccattccatcagcatggcggctgcggccgtccggctggccggccagctcttcgaagacttgcacgagacgcgcgtgctgttcgtcggcgcgggcgaaatgatcgatctggccgccacgcatttcgcggccagggacccgaagtcgatcgccattgccaaccgcacgctcgaacgcggcgaaaagctggcatcgcgcttcggtggcgaggcgatgcggctggccgacctgccgaaccggctggccgagttcgacatcgtggtgagctgtaccgccagcacgctgccgatcatcggcctgggcgccgtcgaacgcgcactcaaggcgcgcaagcaccgcccgatgttcatggtcgacctggccgtgccgcgcgacatcgagcccgaagtgaaggcgctcgaggacatctatctgtacaccgtcgacgacctggcgcaagtggtgcagcagggccaggccaaccgacaggccgcggtcgcgcaggctgaggtcatcatcgacgccggtgtgcagagcttcatgcactggctgggccagcgcggcacggtgccgctgatccagcagctcaacgcccagaccgacgaatggcgcgcggccgagatcgcacgtgcgcgcaagctgctggccaagggcgaatcggtcgatgcagtgctcgaagccatgtcgcgcgggctcacgcaaaaaatgctgcatggcgcgctggccgaactgcatgcgggcgatgcggcttcgcgcgagcagacggcgcacgccatttcgcgcctctttctgcgcaaagagcgttagcgacgcttgccgccgccggcccggcctggttgccgcggcctccccgcgccttgccgccgcgagccgcgccccctcttcttttcggcccctttcgacgtgaaaacttttctgcgccaccaactcgagcgctacgtgcagcgcctcggcgaactcgacttcctgctttcgcgcgaagacatcatgagcgacatggcgcagtaccgcaccatctcgcgcgagcatgccgaggtgacgcagatcgccggccgctacgaacgctaccggcagcgcgaggccgacatcgccggcgcgaaagagatgctcgacgatcccgacatggccgagatggctcaggaagaaatcgccggtgccgaagccgagctggtgcagctcgaagaagagctgcagcgcctgctgttgccaaaggatccggatgacgcgcgcaatgcgttccttgaaatccgcgccggcaccggcggcgacgagtccgcgctgttcgcgggcgacctgctgcgcatgtacacgcgctactgcgagcgagccggctggcgctgcgaagtggtgagcgaaagcgagagcgagctcggcggctacaaggaagtggtgatccgcatcgtcggcaccgacgtgttcggtcacctgcgcttcgagtcgggcggccaccgcgtgcagcgcgtgccgaccaccgaaacccagggccgcatccacaccagcgcctgcacggtggccgtgctggccgagcccgacgagaccgtggcggtgcagatcaacccggccgacctgcgcatcgacacctaccgcgccagcggcgcgggtggccagcacatcaacaagaccgattcggccgtgcgcatcacgcacattcccaccggcatcgtggccgaatgccaggacgaccgcagccagcaccgcaacaaggccaaggcgctgcaggtgctctcggcgcgcatccaggaaaaggagcgcagcgagcgcgccgccaaggacgccgccatgcgcaaggggctgatcggcagcggcgaccgttcggaccgtatccgcacctacaactttccacagggccggctcaccgaccaccgcatcaacctcacgctctacaagctgctggccatcatggaaggcgacctgggcgacgtgctggacgcgctgcgcgccgcgcgcgaggccgagcagctggccgagctggagtcgagcctgccggcatgacgatgacgacggcctccacacccgccaccgtggcgcaggcgctggccgcgtccgtggcgctgggcatcgaccggctcgatgcgcagttgctgctgctgcatgcgctgggccgcgccccgcatgaccgcgcgtggctgctggcgcacgacaccgatgccatttccggcgcggcatgggcggcgctttcagcgcagctgtcgcgccgcctggccggcgaaccggttgcctacctgctcggcgaaaaggagtttcacggcctcgacctgcgcgtggacccgcgggtgctggtgccgcgtccggacaccgaaacgctggtcgactgggccctgcagtgcctcgaaggccgcacggcgccgcgggtgctcgacctgggcaccggcagtggcgccatcgcgctggcactgcagcatgcgcggcctgatgcgcaggtcgatgcggtcgatgccagcgccgatgccttggccgttgcaaaggcaaatgcccagcgcctggccctgccggtgcgcttcagccaggcgcactggctcgatggcgcggccagcggctacacggtcatagccagcaacccgccgtacatcgccgccgacgacccgcacctgcccgcgctgcggcacgaacccgcggccgcgctggttgccgggcccgatgggctcgacgacatccgccagatcgtgcgggacgctccgctgcacctcgcggaaggcggctggctgctgctcgaacacggccacgaccaggccgcggccgtgcgccaactgctccaaacgcacggttttgccgaagtccaaagccgcgaagaccttgccggcatccagcgctgctccggcggagtctggcgcacggtgaaataatcccctcagcccatttttcaggagtccccatgtccgacgcccagcaacgcatcgacgatctcgtcaaatccaacgacctcgtgctcttcatgaaagggaatgcgagttttccgatgtgcgggttttccggccgcgcgatccagatcctcaaggcggtcggcgtcgacaccaaggcgctcaagaccgtcaacgtgctcgaagacgacggcatccgccagggcatcaaggaatacagtaactggcccacgattccccagctctacgtgaagggcgaattcatcggcggctcggacatcatgatggagatgtacgagtcgggcgagctgcagcaggtcctgggcggcagcaaccccgcctgatttttccgctcccgccatgagccacgaccacgacggccacgcgcacggcggagagtccgcgccggcctggaagcacgacggcgtgcgcgtgatcccggccaaccagctcgacgccaacaccgcgcagacgcccggcatgaaccgggcggcggcgatcaacttcgcccgcgtgggtgcacagaagctctgggccggcaccgtcaccatccatgccgatgccaagaccggcgcccatcaccatgggcacctcgaatcggtgatctacgtggtgcgtggccgggctcgcatgcgatggggcgagcagctcgagttcacggccgaagccggtcctggcgatttcatctacgtgccgcccttcgtgccgcaccaggaaatcaacgccagcgcgaccgagtcgctcgaatgcgtgctgtgcagaagcgacggcgaggccgtggccgtcaatctcgacatcgagcccgtcgaaaaacctgaatcggtactctgggtcgacccgacgcatccgcacggcggggtctagcctcgccagtcatggcaccatggcactcttcgccgtgccgccatgactcttacccaaagcctgctcatcatcgtcttgctgatcgcgatgagcgcgttcttctcccttgccgagatcacccttgccgcctcgcggcgcctgcgcctgcgccagatggccgacgatggcgatgcacgggcggaaaaggtgctgcgcgtgcaggagcagcccgggcactacttcaccgtggtgcagatcggcctcaacgcggtggcgattctcggcggcgtggtgggtgagggctcgctcagcccgtacttcgcgcgtttcttcgagaactggatgagcgtcgaggcctcggcgaacgtggcgttcctgtgctcgttcgtcatcgtgattgcggttttcctggtgtttgccgacctgttccccaagcggctcggcatgagcgatccggagcgcattgccgtgcgcatggtcggcccgatgctggtgctgatcaccaccttcaagccgctggtgtggttcttcacgcgctcgaccgacatgctcttcaagctgctcggcatgccgctggtgcgcgacgacaagatcacctcggccgacatcctggccatgaccgaagccggcgcgcgcgcgggcgtgctggccgtgcgcgagcagcaggtgatcgccaatgtgttcgagctcgacacgcggctggtcagcagcgtgatgacggtgcgcgacaacatcgcctggttcctgcacgacgacccggagtcggtgctgcgggcgcgcatcgtggccgagcctttttcagcctacccggtgtgcgacggcgacatcgaccacgtgctcggctatgtcgacgcgaaggagatgttccagcgcgtgctgagcggccagccgctggccttcgaccagggcctgacgctgaacaaggcgctggtcgtccccgaccggctctcgctcacggaagtgctcgagcagttccagcaggcgcatgaagacttcgcgatcatcgtcaacgaatacagccttgtagtgggcgtgatcacgctcaacgacgtgatgagcacggtgatgggcgacctggtgtcgctgcccgacgaggaacagatcgtgaagcgcgacgagaactcatggctgatcgatggcgtgacgccgatccaggacgtccagcgtgcgctgcacatcgacgagctcccgcatccggacgactacgaaacgctggcgggctttttgatggtgatgctgcgccgggtgcccaagcgcaccgacagcgtgagctggggcggctataccttcgaggtgatggacgtcgacagctaccggatcgaccaggtcatggtgacaaaaacttagctggcccccagtctgcgcgcagaggtcaggctgccgaacggtccctgtccacgaaggtccagaggcgctggttcgcgaacaccgcgctggggtacggcgcctttccgcggctgccgttgtagcggccgagggtcatgtagaggtcgccgttctcgcggtcgaggtagtggcgcaggatgacgcagccgaagcgcaggttggtctgcatgtggaacagcttggcgggatcgctgtcgccgatcacgcgggtccagaacggcatgacctgcatgtagccgcgcgcgccggcgctggagacagcgaacttgcggaaattgctctcgacctggaccagcccgagcaccaggctcacgtcgagccccgagcgcttgctttcgtaccagacggtctgcaggaattccttgcgcgtcggccagtccgcgatttttttcttgaggcgctcgctcatctcgcccagccagcgcaggtaggtcaggcgggcctcggtgtccgagaactcgggcaccggcggcgccttgttgtgcacggccgaactcagtgcagtgcgcaccgaatcgatcagcggctcttcgatctgcgcgccagcgcgggcggcctgcggcagcgacagcacggtcagagcgcccgcggtcacggcgccgcccaggcaccggcgtcgcgagagactgccctccaagctcatttcgcgagcttgccgatgatgaattcggcgacgcccaccgccggcaccttggtggcggcagtgtcgcggcgatgctggtattcgagctggccttccttcaggccgcggtcggagatgaccacgcggtgcggtacgccgatcaattcccaatcggcgaacatcgcgccgggtcgctcgccgcggtcatcgagcagcacgtcgacgccggccgcgagcagttgctcgtagagcgcctcggcggccaccttgacctctgggctgcggtccatgccgatggggcagaccaccacggtaaagggtgccagcgcgtcgggccagatgatgccgcgctcgtcgtggttctgctcgatggcggcggcgggcaggcgcgtgatgccgatgccgtagcagcccatctcgaggaactgcggcttgcccgcttcgtcgaggaaggtggcgttcatgtccttgctgtacttggtgccgagcacgaacacgtggcccacctcgatgccgcgctcgatcgcgagcacgcccttgccgtcgggcgaggcgtcgccgtccaccacgttgcggagatcggccaccaggtcaggctcgggcagatcgcggccccagttgacgccggtcatgtggaagtcgatctcgttggcgccggtgatccagtcgcccagaacggcggcctcgcggtcgaccacgagcttgaccggcttcttgaggttgagcgggccgaggtagcctggcttacagccgaagtggtcttcgatctcggccagggtcgcgaagcggaagcccttgtccaggccgggcaccttgccgaccttgatctcgttcatgtcgtggtcgccgcgcaggagcagcagccagacctgcgaacccttgaggttgccggccgcatcgaggatgtcggtcgcgagcaccagcgacttgacggtggtcgagagcggcacgccgagcagctcggccacgtcggcgcaggtgctcttgccgggggtcggcgtcttgtggagctccttggctgccgcggggcgcgggccggccggggccagtgcctcggccttttccatgttggccgcgtagtcgctgcccgggcaatagacgatggcgtcttcgccggtggcggcgatcacctggaactcttcgctcaggtcgccgccgatggcgccgctgtcggccgccaccgcgcggtagcgcagcccgaagcggtcgaagatgcggcggtaggcatcggccatgacctggtagctggccttggcggcgcccaggtcgcggtcgaagctgtaggcgtccttcatgatgaactcgcgcccgcgcatcaggccgaagcgcggacggcgctcgtcgcggaacttggtctggatctggtagaagtttttcggcagctgcttgtagctgcggatttcctggcgcgcgatgtcggtcaccacctcttcgctggtgggctggatcacgaagtcgcggtcatgccggtccttgatgcgcagcagctcggggcccatcttgtcgaagcggccggtctcctgccagaactcggccggctgcaccacgggcatcgtgagttcgacggcgccggcgcggttcatctcttcgcgcacgatcgcctcgaccttgcggatcacgcgcagccccatgggcatgtaggtgtagatgcccgtgccgagcttcttgatcatgccggcccgcatcatgagccgatggctcgcgacctcggcgtcagcgggcgcttccttgagggtggagacaaaaaatcgggaagctttcatcgggatcgcgcgtgatggaatcggtatgggatgtgggggacaactctccggggagaccctgagagcctggcatcggtcgcttgccgagggcaacccggcatgcataatcgactcagttcaaaaattggggtttgattatgctcgaccgggacggcttcaggcccaacgtcggcatcatcctgctcaaccagagaaaccaggttttctggggcaaacgcatacgcacgcattcctggcagtttccgcaaggcggcatagaccgcggcgaaagtccggagcaagccatgttccgggaactgcacgaggaagtggggctccatccggagcacgtgcgcatcgtggcccgtacccgcgactggttgcgctacgaggtgccggatcggttcatccgccgtgacgcacggggccactacaagggccagaaacaaatctggtatttgctgcaactcatcggccacgactgggatctgaacctgcgtgccaccgaccatcctgaattcgacgcatggcgctggcacgactactgggtgccgctcgacgtggtcgtcgagttcaagcgcggcgtctacgagatggcgctgaccgagcttgctcgctacctgccacggcaggatttccgcaaccgcttccttcgcagcaacgtacgcgcccgtgaattcgagcgccacatgccagacggcggcgcacccgcgggcctggatctgccgcccggcggcagtttcgacccgcatcccgacatccattccgcgagcgatgaaccttctcctcccccgaacaaaacgcccttccttccgtcgcaacgttgagcgcattctgcttctcgcctgcttcggcatccttgccggctgcgcatcgggcaaatacgacaccgacaaccccgactgggcgcagtcgggcatgccgccgccgcccaagcgctccgaggcggacgccgaatgggtagaaaccgcggcaccgccgccgccggccttcagcgaaagccggctgctgccaatcgaaatgcctccgtacatgagcctgaagttcggcatcgacccgaacacgatcgccatcacgcgcgacggcatcgtgcgctacgtggtggtggcgcagaaccgcaatggcggcggcgtcaatgcgttctatgaaggcgtgcgctgctcgaccggggaaatgaagagctacgcccgctacaacaacggcgcctggcaggaaacgaagacgccggagtggaagcgcatcaacgacctgaactcgcgctacgccaaggcgctgtcgacccaggcgctgtgccgcggcaacgcgccgcgcaactcggtcggggacatggtccagaacctgcgcaatccggttcgcgaagtgcagtgaacccgtaacggggcctcgcgccccgttttttacgtcagccgggcatcagcaccatgttgtcgcggtggaccatttccggctccgccacgtaacccagcaatcgctcgaactcgctcgaaggcttgcggcacagcagccgcgcttcgacgctcgagtagttggccaggccgcgggccagttcgacaccgtcgacatcgcgtaccgcgatcacgtcgccgcgcgagaactcgcccgacacgctggtcatgccgatcggcaacaggctcttgccctcggcgcgcaccttggctgcggccccggcatcgaccgtgaccgcgccgcgcaactgcaggtggtcagccatccagcgcttgcgcgcctggtgcttggccgtctgcgccaccagcaaggtgccgatggattcgccacgcgtcaggcgcagcagggcatcgggttcgcgcccccaggcaatgaccgtggaagcacccgacccggccgcgcgcttggccgcgaggatcttggtgatcatgccgccgcggccgaggctggagcccgcgccgcccgccatggcttcgagggcggggtcgccggcggccgcctcatggacgaactttgcgtcagggtccttgcgcgggtcggccgtgtagaggcccttctggtccgtgaggatgatcagcgcatcggcttcgaccagattggccacgagcgcgcccagcgtgtcgttgtcgccgaacttgatctcgtcgttgacgacggtgtcgttctcgttgatgaccggcaccacgcgcagcccgagcagcgtgacgagcgtcgagcgcgcattgagatagcgctcgcggtcggccaggtcggcatgggtcagcagcacctgggcgctgccgatttcgttctcacgcagcttggtctcgtacatctgggccaggcccatctgcccgacggctgcggccgcctggagctcgtggacctcgtgcggccgggtgcgccagccgagccgcttcatgccttcggcaatggcaccgctcgacaccatcacgacctcgcgcccgccctgcaccagcaccgcaagctgccggcaccactcgccgatggcgccctcgtcgaggccgcgcccttcgttggtcacgaggctggagcccaccttgacgacgattcggcgggcatcccgcaaggcagtggatccggagttcgaggtcattggaggctttggcggtcgtgtcgtgaatactgcgtgttcggctgtctatctatgaagcagcatcggctgccgatgctcagcggcgctcaggccggatcgggcggcagctcggcaaagcgcggatcgacctcgaccggcacctgctccgccacctgctgcgccttgatgtgctggtagaccgcctgcacaaggtgctcgcagccttcccgcgtgagcgcggagatctcgaacacaggccccttgaagcgcatgcgcttgacgaagtctttcacgcgcgccgcgcgttcgtcgccgggcaccatgtcgagcttgttgagcacgagccagcgcggcttctcatagagcgcggtgtcgtactttttcagctcgccgacgatggcctttgcctgtgccaccggatcgaccgcgtcgtcgaagggggccatgtcgatcacgtgcaacagcaggcgggtgcgctggaggtggcgcagaaacaggtggccgaggcccgcgccttccgacgcgccttcgatcaggccgggaaggtccgccaccacgaagctctgctcggggccgacgcgcacgacgccgagattcggatgcagcgtggtgaagggatagtcggcgatgcgcgggcgcgcattcgaaatggcgctgatcagggtcgacttgcccgcattcggcatgccgagcaggccgacgtcggcgagcaccttcagttcgagcttgagactcttcttctcaccgggccagcccggtgttttctgacgcggggcacggttgatggcgctcttgaagcgcatgttgccgaagccgccgtcgccgcccttggcgatggtgacgacctcgccttccgtcaacagctcgtacagcacctcgcccgtctcggcgtcggaaatgatggtgccgaccggcatcttcaacacgatgtcgtcgcccgcggcgccgaacatgtcggagcccatgccgtgctcgccgcgcttggcctcgtgtcggcgcgagtagcggaagtcgaccagggtgttgagattggaatcggccaccgcgtagacgtggccgccgcggccaccgtcgccgccgttggggccgccgaattccttgtatttttcatgacggaacgacacgcagccgttgccgccatcgcctgcggcgatgtcgatgaaggcttcgtcgacgaacttcatggggtatccagtgtacaaatgaagaagccccggcaaagcggggcttcgagctgatcgaagggacctgggcttatgccgcgggggtcacgttgaccatgtgcttgttcagtgcgcccttgacgccgaacgacacgtggccgtcgaccagcgcaaacagcgtgtggtccttgcccacgccgacattcacgccggggtggaactgggtgccgcgctggcgcacgatgatcgagcctgcgctgatcagttcgccgccgaacgccttcacgccgagcatcttgggcttggaatcgcgcccgtttcgcgttgagccgccgccttttttctgtgccatggaatctgctccttagccggcgatcgcgccgatttgcagttcggtgaactgctggcgatggccttgacgtttttgatagtgcttgcgacggcgcatcttgaagatgcgaaccttgtcgtgcttgccgtgcgacagtaccgtgactgtcaccgttgcgccggacaccaggggcgtaccgaccttgatttcgctgccgttgccgactgcgagaacctgatcgatcacgatttcctggcctacatccgcagcaatctgttctactttaattttttcgccggaagcaacgcgatactgcttgccgccggtttttatgaccgcgtacatgtgaacctcttgggaatatgagctccgcggcgaattccgcagagcccaagattctagcacggtttgcgcgcgctaacatggtttaagcgcgaagcgcgccggaacagcacgcgctcctccctataatctgcgccttccggtcttgtgccgctgccaccttcgtactcagacgcgccgcgcgcaaacgctttgccagttcacgccgccgatacctcccccaccgccaccgtgctggatttgatcgccggcgacatggtcgaagtcgaccgtgtgatctcgcggcgcctcgatacgggcgtgcccctggtcagccaggtttccaagtacatcatctccgccggcggcaaacgcctgcggccggcgctgctgctcctcatgtcgggcgccctcggatacacgggcgagcagcgcttcaacctggcagcggtggtggagttcatccacacggccaccctgctgcatgacgacgtggtcgacgagtcgaccctgcgccgcggacgcccgacggccaacgaatcgttcggcaaccccgccagcgtgctggtcggcgacttcctgtattcacgcgccttccagatgatgttggatgcaaacaacatgcgcatcatgcaaattctggccgaggcgaccaacgtgatcgcagaaggcgaggtgctccagctgatgaacatgcacgacgcgtcgctggacgaagcggcgtacctgcgcgtgatccgctccaagactgccaagcttttcgaagccagcacacggctcgccgccgtgctggcgggcgccgcgcccgaggtcgaggaagcttgcgccacctatggccaagcccttggcacggcgttccaggtcatcgacgacgtgctcgactacgccggagacgcccacgaaactggaaagaacgtgggcgacgacctgcgcgaaggcaagaccacgctgccgctgatcttcgccatgcggcgcggcagccccgcccagggcgcgctggtgcgcgcggccatcgaggccggcgacacggcccagcttggcaagatcgtcgaaatcgtccacagcacgggcgcgctggaagcctcgcgcgccgccgcggccgacgaggcaaaacgcgcgattcatgcgttgcgggactttccgtccaatttgcacgccgacggtttgctacaattggcggctcagttgcttgagcgacgtgcctgaacacctcacaagagttggcaaggacgacttctctttttctgcaaccaatcggggtgtagcttagcctggtagagcgctacgttcgggacgtagaggccggaggttcgaatcctctcaccccgaccagtcttttcggctggcaccaataaatgcccatgcctgttgctgcgtagcgatttacatggcgagggcgttcagcgatgatcgtgaagcactttttcacatcttttgcaatttcgctgaatggctgccgccgaacttcctgttaaagaaaacacgcaaatcgccctcccgggccttgcgcgcgccctggtttcagccgggaagcttcctgcgaagactgcggaagacatctaccagaagtcgctgagcagtcgcaccagcttcattgccgagctgaccggcagcggcgccgtatcggccgccgacctcgcccacacgctatcttcagctttcggcgcaccgctgctcgacctggacgccatcgaccaccagcgcctgcccaaggacctgctcgacccgaagctgtgcctcgcctaccgcatcgtggtgctgagcaagcgcaacaaccgtctcattgttgcaacagcggacccctcggatcagcaggcggtggaaaagatcaagtttgcgtcccagatgggcgtggactgggtcatcgcggaatacgacaagctgtcgcgcatgatcgaggccgccgctgtcagcgcgtcggaaaccctcaacaacatcgtcggcggaggggatttcgagttcgacgatgtcacggccgatacatcgggcgatgccaacgaacaggcggccgtcgccgaagtcgaggatgccccggtcgtccggttcctgcacaagatgctgctcgacggcgtcagcatgcgtgcctcggacattcacttcgagccctacgagcacaactaccgcgtgcgctttcgcatcgacggcgaactgcgcgagatcgcgagcccgcccacgctgatcaaggacaagctggcttcgcggatcaaggtcatttcgcggctcgacatctccgagaagcgcgtgccgcaggacggccgcatgaagctcaagatcggcccggaccgcgtgatcgactttcgcgtgagcacgctgcccacgctgttcggcgaaaagatcgtgatccgtattctcgacccgagcagcgcccgcctgggcatcgatgcgctcggctatgacgccgatgaaaaggaacggttgctgaacgcgatcggccgtccctacggcatggtgctggtgacgggccccacgggttccggcaagacggtgtcgctttacacctgcctgaacctgctgaaccagcccggcgtcaatatcgccacggccgaagacccgtccgaaatcaacctgcccggcgtgaaccaggtcaacgtgaacgagcgcgccggactcacgttcgccgccgcgctgcgcgctttcctccggcaggatcccgacatcatcatggtcggcgaaatccgggacttagaaaccgccgacatctcgatcaaggccgcgcaaacgggccacctggtgctttcgacgctgcacaccaatgacgcgccgaccacgctcacgcgcatgcggaacatgggcattgcgccgttcaacatcgcctccagcgtcatcctgatcactgcgcagcggctggcccgccgcctgtgccatttgtgccgcgcgccggccgacgtgccgcgccaggccctgctcgacgcgggcttcaaggaagctgaactcgatggctcctggaagccctatcgtccggtcggctgctccgtgtgcaatggcggctacaagggccgggtcggtatctaccaggtgatgccgatctccgaaacgatccaggccatcatcctgcgcgacggcagcgcgctggacattgcgcgccagtccgaggccgagggcgttcgctcgttgcggcagtccggcctcagaaaagtcatgcaagggctcacctcactcgaagaagtggtggcggtcaccaacgaataacgaacgaacacactgcaaatcggagatcgaatggcaacagtggcatccacccgcacctcaagcacgctcaaggaatccgtctacgagtgggagggcaaggaccgcaacggcaagctggtgcgcggcgagcttcgggccgccggcgagaaccaggttcaggccgctttgcggcgccaaggggttctcgcatccaagatcaagaagcgccgcatgcgctcgggcaaggcgatcaagcccaaggacatcgcgatcttcacgcgccagctggcaacgatgatgaaggccggcgtgccgcttttgcagtcgttcgacatcgtcggccgaggcaatgccaacgcaagcgttgccaagctgctgaacgacatccgcagcgacgtggagaccgggacctcgctttcggccgccttccgcaagtttccgaagtatttcgacaacctctactgcaacctggtggaagccggcgaagcggccggtatcctggaagacctgctggaccgcctggccacctacatggagaagaccgaggcgatcaagtccaagatcaagtcggcgctgatgtatccgatttccgtggtcgtggtcgcgttcgtggtgattgccatcatcatgatcttcgtgatcccggccttcaaggaggtgttctcctctttcggcgcagatttgcccgccccaaccctgatcgtgatcgggataagcgagttcttcgtctcctactggtggctgatcttcggcgggatcggggggggcatctacttcttcctgcaggcctggaaacgcaacgaacgcgttcagcgggtcatggaccgcgcgttgctgcgcgtgccgatcttcggcacgctgatcgaaaagtcgtgcgtggcccgatggacccgcaccctcgccaccatgttcgccgccggcgttccgctggtcgaagcgctcgactcggtgggcggtgcgtcgggcaacacggtgtatggcgatgccacggccaagatccagcaagaggtctcgaccggcaccagcctcaccacggccatgaccaacgtcaacctgttcccgtcgatggtgatccagatgacggccatcggagaggaatccggttccatcgaccacatgctcggcaaggccgcggacttctacgaatccgaagtggacgacatggtcgcgggcctctccagcctgatggagcccatcatcatcgtgttccttggcacgatcatcggcggcatcgtggtgtcgatgtacctgcccatcttcaagctgggccaagtcgtctgatgctggtttcgcaggagttcgacgccgcttttgccggcgtcctcgggttgctggtcggcagtttcctcaacgtggtgatctaccgcacgccggtgatgatgtaccgcggctggctggccgatgccgtggccaacctgatgtcgtcgaaggatgttccatcgctctggtcgctggtcttcgggccgaagaccgcgcccccgccgggcctcgaagccgcggccgacaaggctgcgctggcgatcgagggcctgccgcccttcgacctggcccgtccggcctcgcgctgcggagcctgcgggcacaagatccgctggtacgagaacattccggtgctgagctacctggtgctgcggggccgttgcgccgcctgcaagacccacatcagcccgcgctatccgctggtcgaactgatcaccggggcgctcttcgccctttgcgcctaccgcttcggcctcacgcccaccggcgcgctctgggccgccttcgcggcgctattgatctgccagttcctgatcgatttcgacacccagttcctgcccgacgcgctcaactatccgctgctctggctggggctcatcggcgcggccatgggctggaccggcgttgcgctgagctcggcggtctggggcgccgtgttcggctacctgagcctctggcttgtgtaccatggctatcgcctggtcacgggcaaggaaggcatggggtatggcgacttcaaactgctggctgcgctcggcgcatggctcggggccgactacctcattgccatcatcctcgtctcatcgctggtgggcgccgtgatcggcctcacgctgcgattcgtcggcaagctggcgcacaaggacattcccatggccttcggccccttccttgccggtgcaggcctcgtctgcctcgtggcgggccccgaactcgtccggcaatggattcccttcgctttcccgctcggcgcattcgcccgctgaagagccagtgatgcggcgcatcggcttgacggggggcatcgggagcggcaagagcaccgttgccgcactgttggttgcggagggtgctgtactggtcgacaccgacgcgatcgcgcgccgcatcgcacagcccggaggccttgcaatgcctgccatcgaggctgccttcggccgggcggccattgcgccggacggcggcctggatcgcgcaggcatgcggcaactcgtgttcaccgaccacagcgcgagaaagcgccttgaatcgatcctgcacccgctgatcggtgccgaaacggagcgccttgcgtccgcagcgggtccggatgccgtggtggtcttcgacgtcccgctgctggtcgaatcgggtcgctggcgggctctcgtggatcgggtgctggtggtcgatgccagcgaggaaacgcagttgcggcgcgtcgtggcgcgctccggctggacagacgaagccgtgcgcgcggtgatcgcccagcaagctgcgcgcaagttgcgccgggctgctgccgatgcggtcattttcaacgagacgctctcgctggaggaactcggcggcgaggtgcggagtctctggaagcggtgggctccgcccggcacgcgataatccgagacttgccgccgcagcggccgcataacgatcaagacaaaaaggcgctcgccggagtgccctccctcccgcgatgcttttcaattcgtatccctttatttttgtcttttttccgctggtcctgatcggcttcttcctgatcggcaagcgcaacgcccggtccgcggcgggctttctcgccctggcctcgctgttcttctatggctggtggagcgtcaaggcgcttccgctcctggtggcgtccatctgcatcaactactggttcgggctgcgcctctcgcccgcgccggaccggaacgaccgcaagcgaaagtcgctgctggtgatcgcactggtggtcaacctgggtgtgcttgcggtcttcaagtacgccaacttcttcgtatcgaacgtgaacgacggactcgccgcggccggcctgtcgcagattccgatgctgcacatcgtgctgccgatcggcatctcgttctacaccttcacccagatcgccttcctggtcgactgctggcaaggcaaggtgcatgagcgcagcttcattcactacgtgctgttcgtcacctactttccgcacctgatcgcaggtccggtactgcatcacgcgcagatgatgccgcagttcgcgaatccggccacctaccggctcgacccgaacaaggtggcgctcggcgtggcgatcttcaccttcggcctcgcgaagaagctgctcattgccgacccgatgggccaatacgccgacatgatgttcaacggcgtgcacaagggcatcgagcccacgctctacacctcatggttcggcgcgctggcctatacgctgcagatctatttcgacttctcgggctattcggacatggccgtcggcctctcgctatgcatgggcgtgcagctgccgctcaatttccgctcgccctacaagtcgaccaacatcatcgaattctggcggcgctggcacatctcgctgtcgaacttcctgcgcgactatctctatgtgccgctgggcggcaaccgcaagggcccggcgcggcgctacctgaacctgttcctcacgatgctgctcggcgggctctggcacggcgccgcatggaccttcgtgatctggggtgcgctgcacggcgtgttcctgatgatcaaccacctgtggaatgccaaagtgcggcgcaacgccaagccgggccgcgtggcccacgtgctgggctggctgctgaccttcctctgcgtggtgctggcctggatcgtcttccgcgccgacggcgtgcatacggccatggccatctacaagggcatgctcgggttgcatggcgccccggcctcggcgttcagcgaactcggccccgtgccgttccgcaaacccgagttcttccagaccatgctggtcggcatcatcatttgccttgcgttgcctccgacgatctcgctcgagcgctggattccccatccgaaggcggttgcgggccagcccgtcatggcgtggttctcctcggccgtgctcgcgatcggcactttcgcgctcttcgcctggtgcgtctcgaagctgggcaactacagcccgttcctctatttccaattctgattcgacatgacgacgcccgccaaagtctggctgcgattcttcctcatcggctacatcgccctgatggtgctgtggatcgtttcgctcaccagccccgtgccttacggcgacctcacgcggatcggccgcctgtcagaacgcgagttcggctggaccgctccgccaccccaggtcgaccctgccttgctgaagggcacgcccgtcgaccaggccgacgtcctggtcatcggcgacagcttctcgatgaccttccgctggcagtccgtgcttgccaaggccggctaccgcgtctcgaccacctactggggccagtatgaaaatgcgctctgcggcgacttcgaccagtggatcgcacgcaccggcttcaagggcaagctgatcatcatcgagagcgtggaacgcctgctgggcgaccgcaccaaggacagcatgaagtgccagaagatgatccggcccttcgacgccatggaccacccgctgatcacgccggacgaaaccgtgccgagccccgcacccaactggaacgtgcagttcatgacggggatcacgacctactacaacacctggaaagcgaaaaagtctgcaacagacattcacttcgactggaacacctgggtgcggccggtgcccgatggttgcaagctcttctcccatcgctcctgcgacaagatgccttttttcgccgaagatgacgacaatggcccgctgactcccgcgcacctcgagtggatgaagaatttcacaaaggcgcacggcaagcttcctatcatgtggatggtgattcccaacaagaccaccgtgtacctgaagcccgattactccaaggatttcgaagccgggttccgcgcgtccggcctcgggcccgatctctacgcgttcacgcgcgagaagcacacgcagattcgcgacttctatttctcgaacgacacccacatgtccatgcacggccagctcgcgctgggagaacgcatgctcaccgccgtgcgcgaagtgctgcccacgcccccatcgaaatcgccctgaagctatgatggcgcgacaggaaaccgacaaaaacgcgtgatcctctacgagtaccctttcaacgagcgcatccgcacctacctgcggctggagcacctcttccgccggctcggggaactggtgccctcggaatccgcgctctcgcatcactacgcgctggtcacgatcttcgagatcatggacgttgccgcgcgcgccgacctcaaggccgacgtgatgcgcgatctcgacaagcacaagaacgtcttcaacggctaccgcggcaatccggccatcgccgaagccgtgctcgaccaggtggtgggccagctcgagcgcaacttcgcaacgctcaacggcgttgccggcaaggctggccaggccctgaccgaaaacgagtggctcatgagcattcgcagccgcgcgggcattccgggcggcacctgcgaattcgatctgcccgcctactacgcctggcagcaccgcagcgcggcaagccgccgggccgatctcgaacgctggtccgccacgctgtccccgctggccgaatccatctacctgctgctcaagctgctgcgcgatgccgatgtaccgtacaaggtcattgccacgggcggccagttccagcaaaacctgccgcaaggccgcagcttccagctgctgcggctacgcatcgatcccgcgctcggactcattcccgagatcagcggcaaccggctcatggtttcagtgcggctgatgcggcacgaagccgacgaccggctgcattcaagcacggacgacacggcattcgaactcaccctttgcgcatgagctccggcctggccgttccgaagggggctcgcaccgcagtgcggagcacggaggttacttatcaatgagcgacgtgaacaagatcggcgagcggatcgtccgctgcccctcgtgtggcggcgacagtgtctacgccgagcgcaacccctatcgcccgttctgcagtgcgcgctgcaagggcatcgatttcgggggctgggccagcgaggagttccggatgccgacagaagcgccggccgacgacgagcccttcggcgacccgaagaaagtccaataagcgcaccttgcgctacggcgcgagaaagacgcggtccagatagtccgcgtgctcgcggacgtacgccggacgcaggtgctcccggtccttgtaggccggtgcatcgtcgggtgtcgcccggaggcactgcccctctgcacagagccttgccatcacgtcgatcggctctgcgccgctggagagcgcgagcgcgcgcaactgctcattgagcctcgcctgttccggcggcaggggtgcggcaggcgtgctggtcagcgccaccatcttgcccatgcggctgccttcgatgaggcgccgcggctcgaactcggggccgctggcgttgtccagcaacaggtagacttttttcttgtgctgcaccagctgcaccaggagcttttcgagcgacgccagcgagcgcccgaggccggcgccgccattgttcacgaggtaggccgacgcaccctcgtgaaagtagaacggcaacggaaagttgcccgtgaaatagcagttccagcaagcgccgaccaccacggtgtcgaaccgcggatcgacggccagcgcgagcatttcgcggcgcgcctgctcgcagcccggattgccctccgcagcaaccatgccgggcaccggcgggcaggcgccgtaggtcgagaagaaggtcgtcgccatgcgctcgggggcgcggcgtgcgagctccattgcacggggcgcgtattgcaggatgtggctgtcgccgatcagcaagaccttccgagacccgtcgcccacgcgcttgaccggaaaggcgccgatcttctgctgctcgaagccggcgtagtagttgtcgtccacggtggcgtcggtcaccttgcgcagcaggtcgctgccgttgcgtggcggcatgccgcccagcgccagcagcccggtgaccgcgatcgccatgctgccgcccacgagcgtgcgcagcatgccgacgtgcacccgtgccctggtgaagcgctcgacgaagcgataggtaagccaggccagcgccacgctcgccagcaccatcgccgcacgcacgatgggcgccggctcgccttcgttcacgatgcgtgcgtagaccagcaagggccaatgccacagatagagcggatagctgatgagaccgatccacaccatcggacggctggcgagcacatacctgttcagcacccccgcaggcccggccgcgatacagctcgccgcgcccagcgtgggcagcaatgcccaccaccccggaaacgccttgtcgctgcgggtcatcacgagccccagcacgatcagccccacgcccatgcacgactgcacgtggctgcgccaggccggcaccggctccttggcgggctgcaggcgcatacaggccaggatgccgcccaccatcagttcccagaagcgcgaagcgggtgagtagaaggccgccgtgcgaaaaggatggatcgtcagcacgttgaccagaaacgaaaccaccgccagcacccagagcaaccggagaatcggccagcgccggcgccaggccagcgccagcagcatgggccagaaaatgtagaactgctcctcgatgcccagcgaccacaggtgcagcagcggcttggtctccgcggccgtatcgaaatagccggcctcgccccagaagatgaagttggcaatgaaggccgcgccgcccgccgcctgcttgccgagttcggtgaactccctgggcagcagcgcataccagccgaaggcgagtgtggccagcagcaccagcgtcagtgccggaaagatccgccggatgcgccgtgcatagaaatcgcggtagctgaaatcgcccgccgcatggctctgcatgatgatcgtcgtgatcaggaagcccgagatcacgaagaagatgtcgaccccgatgaagccgcccggcaatgcgtcgggaaacgcatggaaggccagcaccgacgccaccgccacggcacgcaggccatcgatgtcggcgcggtacttgggatgcagcatgtcttgtctcaggcccgcggcgcccgcaggccgcgcttgcccgacctcgcggcccagtccatcaggccagggtcgaaaccgccagcgccgccgacgcgggcagcccgcgttcctgggtcagccattcgagcaccggcaaggcgcccggcagcaccggggccacgtcgagcggcagctgctgccagcgcatggcctgcccttcgcgcatttcgaactcgccgctccaggccgtgaccttgcaccagtgcaatcgcaccagcgcatgcgggtagtcgtgttcggtcactttccagacctcggcgcccgcgatggtgatgcccagttcttcgtgcagctcgcggcgcagtgcctgctccacggtttcgccggcctcgatcttgccgcccggaaactcccagaagccggcgtaggccttgccctcgggccgggtcgacagcagcagcgcgtcgtcggccgggcggatcagcacgccgacagccacctcggtgtgcttgcggccttgggactgcggctgtgcgctcatgcggaagcccgcccggcatagtcgcgcgcgaactgataggccacgcggccgctgcgcgaaccgcgctccagcgcccataccagcgcctcgggacgcgcggcctcgatggcggccttgtcgacgccgaacgacgacagccactgcgcgacgatcgccaggtattcgttctggctgaagggatagaagctcacccacaggccgaagcgctccgacagcgagatcttctcctcgatcacttcgccgggatgcacttcgccgtcctcggtgtgggtgtagctgaggttgtccttcatgtattccggcagcaggtggcgccggttgctggtcgcgtagatcagcacgttgggcgtggccgccgcaatcgaaccgtccaggatcgacttcagcgccttgtagcccggctcgccctcgtcgaagctcaggtcgtcgctgaacacgatgaatttttcgggccgctgcgacaccacctcgacgatgtcgggcaggtcggtcagttcggccttgtcgacttcgatcagccgcagcccctgcggcgcataggcctgcaggcaggcgcggatgagcgacgacttgcccgtgccgcgcgcccccgtcagcagcacgttgttggccggcttgccctcgacgaactggcgcgtgttgcgctcgatcttttctttctggacgtcgatttccttcagcgaatcgagcgccatcgaggccacgtgtttcaccggctcgagcacgccatggcccgagctccggcgacgatagcgccacgcgatcgacgcgttccagtcggccggtgccgccagcggctgcggcaggatcgactcgatgcggccgatcagctgttcggcgcgctccagcagcttctggaattgctcattcatgacctgtaatcagcattgatcgtgacgtagtcgtggctcaggtcgcaggtccacaccgtttcgctcgcgttgccgcggcccaaccggatgcgcaccgtgatctcgctctgcttcatcacgcgctggccgtcttcctcgcggtacgacgggttgcgcccgcccttgacggccacgtgcacgtcgtccaggaacaggtcgatgccggtctggtcgagatcggcaatgcccgcatagcccacggccgccaggatgcggccgaggttcgggtcgctggcgaagaacgcggtctttaccagcggcgaatgcgcgacggcataagccacctgcttgcattcgcctgcatcacggccgccttcgacctggatggtgatgaacttggtggcgccttcgccgtcgcgcacgatggcttgcgccagctggcgagccacgttctgcatggcggccaccagtgcctggccgtcggccgactccagcgaggtgatggtggcgtgcgcagccttttgcgtggcgatgaccacgaaggagtcgttggtcgaagtgtcgccgtcgatcgtcacgcggttgaatgaagcatcggccaacaacctggccagcggctggatcagcgaaggatcgatcttggcgtcagtcgccatgaagcccagcatggtcgccatgttcgggcggatcatgccggcgcccttgctgatgccggtgacggtgacggtggcgccgccgatttgaacctgctggctgaaagccttgggaatcgtgtcggtggtcatgatgccttcggcggcacgtgcccagtggttctccgaagcgtcggccagcgcggcgggcaggccggcttcgatgcggtccacgggcagcggctccatgatcacgccggtcgagaacggcagaatctgctccggcgcgatctccagatgacgcgccagcgcgatgcaggtggagcgcgtgcgcatcaggccgtcttcgcccgtgccggcattggcgttgccggtgttgatgaccatcgcgcgaatgccgtagtgggctgccaggtggtcgcggcagacctgcaccggcgcggcgcagaaacggttctgggtgaacacgccgccgaccgccgcgccttcatcgatcagcacgacggtcaggtccttgcgattggccttgcgcacacccgcttcggccacgccgatgcggacgccgggcaccgcgaacaaggcggcaggatcaggagcggacaggttcacgggcatggcggttatttctcttcgggagtttctgggtcagctgagtttgccgtggcagtgcttgaatttcttgccgctgccgcacgggcatgggtcgttgcggccgacgcgtgcaaacgccgcggcttcggcgcccaggctgccgagccccaggcccgcggccgcgatgcggcgctggttttcttcatcctggcgcacctcgacctcgccggtttcggtcggcgcgctgtaggtgatgttcgagacgttctcgccgcggctctccatcgcttccgccgcctcttcgagctgctcgcccgactgcacgcgcaccgtcatgagctggcgcgtgacttcgttcttgaccgagtcgagcagctggccgaagagttcgaaggcttcgcgcttgtattcctgcttgggctgcttttgcgcatagccgcgcaaatgaatgccctggcgcaggtagtccagcgaggccaggtgctcgcgccagtgcgtgtcgatgccctgcagcagcaccatgcgctcgaactgggtgaagttttcctggccgatgagtgcgaccttggcaccgaagctgtcgttggcggcattcaccaccttctcgacgatgtcctcgtcggacacggcctcggccgcctcgatttccttcttgaggggcatgtcgatgccccactcgttggacagcgccttctcgagggcgtcgaggtcccattgttcctcgaccgattcggccggcacgtactgccgcacgaggtcggtgaaacagccttcgcgcagcgccgcgatctgcgccgtcaggtcggccgcgtcgaggatgtcgttgcgctgctggtagatcaccttgcgctggtcgttcgacacgtcgtcgtattcgagcagctgcttgcggatgtcgaagttgcgtgcctcgaccttgcgctgcgcgctctcgatgctgcgcgtgacgatgccggcctcgatggcttcgccgtcgggcatcttgaggcggtccatgatcgccttcacgcggtcgcccgcgaaaatgcgcatcagcggatcgtccaggctcaggtagaagcgcgaagagcccgggtcgccctggcggcccgaacggccgcgcagctggttgtcgatgcggcgcgattcgtggcgctcggtcgcaatgatgcgcaggccgcccagcgacttcacgaattcgtggtccttggtccactcggcgcgaatgtgtgcgacgtcggcctctttggcggcttcgtcgcggccttcgtcgttctcgatcgcctcgatcatcttctcgatgttgccgcccagcacgatgtcggtaccgcggccggccatgttggtcgcgatggtgatcatcttcgcgcggccggcctgcgccacgatgtcggcttcgcgcgcatgctgcttggcgttgagcacctggtgcggcagatccgccttggtgagcaggccgtcaatgatctcggagttctcgatcgacgaggtgcccaccagcaccggttgcccgcgctcgtagcactcgcggatgtcctggatcgcagcctcgtacttttcgcgcgtggtcttgtagacgcggtcgagctggtcgtcgcgcttgctgatgcggttcggcggaatgatgacggtctcgaggccgtagatttcctggaactcgtaggcttcggtgtcggccgtgccggtcatgccggccagcttgttgtacaggcggaaatagttctggaaggtgatggaggcgagggtctggttctcggcctggatctgcacgccttccttggcttccacggcctggtgcaggccatcgctccaacggcggcccgtcatcaggcggccggtgaattcgtcgacgatgacgacctcgccctgctgcaccacgtaatgctggtcgcggtggtacaggtgccgtgcacgcagcgccgcgttcaggtggtgcatcagcgtgatgttggccgggtcgtagagcgaggcgccttcgggcagcagcttgaattcgctcagcagctgctcggccttctcgtggccgtcttcggtcaggaacacctggtgcgtcttttcgtcgaccgtgaagtcgcccggcaccgtgacgccctcgcccgtgcgcggatcggcctcgccctcttgcttggtcagcaggggcaccactttattgatggccaggtacaagtcggtatggtcttcggcctggccgctgatgatcagcggcgtgcgggcctcgtcgatcaggatggagtccacctcgtcgacgatggcgtagttcaggccgcgctgaacccggtcgccgggctcgtacaccatgttgtcgcgcaggtagtcgaagccgtattcgttgttggtgccatacgtgatatcgctgccgtaggcctgctgcttttcctcgcgcggcatctgcggcaggttgatgcccaccgacaggcccaggaagttgtacaggcggcccatccactgggcgtcgcgattggcgaggtagtcgttcacggtgaccacgtgcacgccgttgccggtcagcgcgttcaaatacaccggcagcgtggcggtcagcgtcttgccttcgccggtgcgcatttcggcgatctttccgttgtggagcgccatgccgccgagcagctgcacgtcgaaatggcgcatcttcatgatgcgcttggagccttcgcgcacggtggcgaatgcttccggcagcagggcatcgagggtttcgcccttggcgatgcggtccttgaactcctgcgtcttggcgcgcagtccgtcgtcgctgagcttctcgaactcgggttcgagcgcattgatgcgctccaccgtcttgcgatactgcttgaggagccggtcgttgcgactgccgaaaatctgggtcaggaagttggttgccattggcgtggagatggacgggcacctgacacacaggcactgcgaccggattccctaagatatggtgaaagcagttgggcgcgccttcttcgaatgcaagcctcgaaagcaagcggctccagaccgatctgccggcgcaagcgtcggcaaaccgggcattttagctgtcttgttccatcctccggattacccatgaatcgccgctccgtccctcccttcacgctgcagcaggccgctgaaggctcgcccaccctggcgagcctgattgcgcgcgcgcgcgacgccagcgagcggctgcgggcggtcgaaggattgataccgccggccatgcggcccgccgtgcaggccggcccggcggaaggcgacgtgtggtgcctgctggtcaatggcagcgccgcggccgccaagctgcgccagctgtcgccgatgctggtcacccggctgcgcagcaagggctgggacgtgaacacgatccggatcaaggtgcagtccgggcgctgaacaaaaaaacggccggccgcgcaaaccgcccggcccatcgggacctggcttattgcggctgaagcccgatgtcgtgcgccaccttctgccagcgctcggcttccgcgcgcatgaaagcccgcagctcgcccgtggtggaacccttcagctgcacgcccagcaccgccatgcgctccttcaccgacggatggtccagtgccgcgatcgcctcgcgccgcagccgctcgatcacctccagcggcgtggtggcgggcgccaccatggcccaccactggtcgatctcgaggcccttgagcccgctctccgccaagccgggcacgtccttgaggcccggaatgctcacgcgctgcgcgctcgtcaccagcagcgggcggatcctgttgccgcccaggaggctggaaccgctggccagcgtcgcgaagtgcccggccaccgtgcccgccgccacgtcggtgagcgccggcgccgagccgcgatagggaaccatgttgaacttgatcttcgtgcggctcgccagcagttcggccgccagatggctcaccgtgccggcgccgctgtgcgcgatggccggcggcatcggccgggcggccgccgtcttgatgaaggtcttgaaatcccggctgtcgtcgtccatgcccgcaaagaaaacgagcggcgacgtgccgatcatcgtcaccggcgtgaagtcgcgcagcaggtcgtagggcaaccgcgtcgtcaccgcgggcgcaatggcgtgcggcaactcgacgatggaaagcgtgtagccgtcgggcgcggccttggccgccgcctcggtgccgatctggccggcggcgccggggcggttgtcgacgatcaccgagctgccgatcgtctggctcatgcgctgcgccatggcgcgcgcaatggcgtcggtgctcccgccagccgcccacggcacgatcagcttgatgggcttgtcgggaaaagccgcccaggcgcgcggcgccgcggcggtgaacagggcggccgaaccggcagccaggaaggcgcggcgttgcattgcttgcatggtttcgattccttttgtgtggctcggacgttcaggcggcctggtcgggccaggtcgggtcgcgcgaggcgttggcggtgagcatcagcaccacgtgggcgtcgtcggcaatggcatggctttcgcgcagctggcgcagggcgtccaatccggccgccgcgcacagttcggcgctcacgccggccgccgtgagctttcgccgggccgcgcgggcctggtcgtcgctcaccaccaccgcgccaccgccggaggcgacggcggcctgccactgcaggaaagtcacggtggccccggcggtggaaaactgcgccgtgtcgccgggatacatgccgttgatggcgccgccggcaagcacgcgcgagaggcgcgcaaaaggctccaccagccagagccgcggcaggcgcgaaatgcgtccggcggccagcaggtcgcgaaagcccgcgtagatgccccaggccagatcgccgcgcgccgtggggatcacgacatgatcgggcaggccgccgtcggtcaggcattccagggcaatgggcttgtagccctcgatcgccagcggcgcgcttcccaatgccggcaggcggtagttggtcagtgcgaaatagcccggttgttgtgagcgctcacgcacgaaatcccagcggccggcgttgtccgcaaagctgtggcgccgggcacccagggcgtcgagctgccgtgcataggcggcgggcaagccttcgtaggttgccacttcgcagaccaggcctgcggcccacgcgtagtgcgccgccgagatcgcggcattgcccgaagaggccagcaccagcgtgtgggcaccgaagtccagcgcctgcgccacgcccacggcggtcatgcggtccttgtgagagcccgtggggttgcgcgattcgtccttgatcgcgaggcgtgccacgtcgaactgccgcgccagctccggcatgtccgcgagcggcgtcccgccctcgcccagcgtgaagcccggcatgtagggcatggacacggggctgccgctgtcgggcaggtagctggcgcgcaatccggcatgaatgccggtgttccggcaggccgggcagccatcgttcgccaatgtgagcggatagggggcatcgcatcgcaggcactgaaagccttgcaggcgagggtttctcaccggcggcagcgttcgggccagcgcgccgcccgatgggtttgccgatgggtcgggaagtgcggcggacttgaagtccagaacggacggaggtgtgttcacagggggtcttggcagggaagtcgtgcccaaatcttaggcatctggaaataaaatcatctagcctgaaatactcaagcgataaaaaaacttatcgatgcgcttcaccgaaatagagacgttccgggccctgatgcgcgccggctccacccgcaaggccgcggcactgctgcatgtgacgcaacccgccatcagccagtcgctcaagcggctcgaggcgcaagccggcatgctcctgttccagcgcaccggtgggcggctggtgcccacgcccgaggcgcgcgcgctgtggaccgaggtggagcgcgtcttcatcggcatggaggccatcgagcaccgcatgcgcagcctgcgcgacttcggcaccaaccagctcgaactcagttgctatccggccttcggcctcggcttcatgccacgtgcgctggaacgcctgaaggcacaccggggcgatagtccctggccgcaggtgtcgctgcaggtgctcagctccaaggacgtgcgcgaccgcgtggcaaagggcgtctccgacttcggcctgatggccgacgaactgccgctcgaaggcatcgagcactcgaccttcgcgcggtttcccggcgtggtcgtgatgccgcaaggccatgcgctggcgcgcttcaagtgcatcgagccggagcagctcgcagaagcgcctttcctggccctgaaccccgaggacccttcgcaccgcgggctcgaaaccgcactggccgaacgcggcgcggcgcttcgggtgatggtgcagacgccctacgcggccagcgtgtgcgagatggccgtgcgcggcctgggcgtgggactggtcaacccgatcaccgcgctcgactacgcggaacgtggcctcgtggtgcgccggctctcggtcgacgtgttttttagctgcgtgctggccctgcccgcgggcaaggtgctgtccaccaccgcccgcgactttctttcgctcatgcgccagcaactggcggaagacgagaagcgcatccagcgttacctgcgctgattccgcacgggcctacttccaggcgaactcgtggttcagccccacgacaaagccgcgcacgccctgcggtccggtcctcgaagcgctgatatccacgctgatcagcggcgtgaggctgaagcgcccgccgatgcgcgaggtccagacgcccgcagcgcggctgcgctccgcaatgagcgagaccttgtcgtcgagcgcccactccgcggccagcccgccgcgcggcgtgcgagccccggtgccggtggcccaatcggcgccgaggttggcgtgaatctgcaggctgctcgtcgggcgccacgtgagcggcagcacgaactgcccacccgcacggccaccgcgcgtcaggtcgaacgcggcaccgagagaaagtgccgcgctcaacggcgcgtcggccgccgcgccgaagaaattccatttgacctgcgggcctgcgacgaccgagtgcatgcccgcggctgaaaaccggtcgaggttcagccccagttcgacaggccccacgcggcaggacgggccgatgtgcagcccgtttaccggctccggaccggtgcggccccaccaggcttcgtactggcattggcccggatcgagcgtgccggcatcgtcgacatcgaaatgccccgcggcctgcgcccccgtgctcgaaaggctgcaggcagccgcgagcagccaggcggctcgcggccgtcgaatcatttttgtgcgtttgttgtctttcatcgcctgcatcccccgaggaccgggagattctagggatgaagacaccccttcagatctcgaactgcggctgcagctcgcgaatgcgcttgatggccaccccggcggcggccgtgcgggtctcgacgccgagcttcacgtacacccgctccaggtgcttcttggccgtggcggggctgctgccgagaatttcgccgatgtccttgttggtcttgcccttcaccacccagtagagcacctcggcctcgcgcgccgtgagcttcaggctcaggctcatggcctcgatcaccgcggtatccgaaacctcgcgcatgacgatcatccactcgtcgccgtcgtcgtcctggccggtctgccgatgcaggcgcaggctgaggctgctcgcgctcggcgtgccacccacgctcgtcccggcggcgccctgcacgatggaaagtgccggcggctcgatgccctgctgcctggcatcgggcgcgtggcgccgaagccactcgagcaccacgggcggcgtttcgggcgcgcgggtgtcgcaatagcgctgcagcaggtcgcgcgcgagcgccgtctgccagatcagcttgccctcgggcaggcgcacggtaatgctggcgtagccaaaggcgtcgagcgcattgcgcgcctggccggcctgccgcgcatcctgccgggcgcggcgggcgccctgcaggtgcacgttcatgcgggccagcacttccttgggcttgatcggcttggtgacgtagtcgacaccgccggcctcgagcgcggccacgaggtgctcggtttcggtgagcccggtcatgaacacgatgggaatgtgcgccgtcgcggcattggccttgagccggcgcgccacctcgaagccgtcgatgcccggcatcatggcgtcgagcagcacgatgtcggggcgcgcctgcgcggcacgctgcagcgcctgctcgccgttggtggcaatgagcacggtatagcccgattcgtcgagcgcgtcatgcagcaccgcgaggttgtcgggcacgtcgtcgacgatcagcaccaggtcgctgttggcgccctgttcgcgcagcgttttcgcaagcggtgtggtttccatgagacttgatcttcaggccgcgctcaccgcggcggcaagcgcccggcccatggcctcgaactggaactggcgcgcgagcacgcgctgcgcctcggtccaggccaggcattcgggctgttcggcgtcgatttcgtcgagctggttcatgatgccgcgaaaatagcccaggctcaccgcttcgtcgagggcgcgcagcctcgccatcgaaggcgcctgcatcgcgcgcggcgcggtggcgggggtcggcttggcggccgtgtcggtccatcgcaggccgaggcggcgttcgagccagtcgagcagttccgtatggcgcaccggcttgacgaaaaaatcttccggcgcaatgcctgcgtcgttgtccaggcccttgtcgaaggcattggccgagacgatggccacggaggcctcggccaggccgagcttgcgcgcacggcgaatcgtctcccagccgtcgatgcccggcatggcaaggtcgacgaacatcgcatcgggccggtagccggccgcgatgaggtcgagcgcgtcgtggccgctggcggcggtgcgcaactcgaagccgagcggcgccagcacatggccgagcaggtcgcggtcggcctcctcgttgtcgaccaccagcagccgccggcgaggtccttcgtagccgcgccgcgcgcgctgcaccggagccggccggcccgaggcgctcgccgtgtcgtgcacgcgcggcaaaaaaagccgcacgcagaacagcgagccttccccgggcgtgctgcgcaccttcatctcgccgcccatcaggtcggtcagcatcttggcgatggtgaggccgagccccgcgccgggcgtggaggccgcagccgcatcgccgcgcgcaaagggctcgaagatgcgttcgatgtcttcggccgtcatgccgggcccggtgtcctcgatctccaccgaagcgaattcccgcgcatacgaaagccgcagcgtcacctcgcccgcggccgtgaacttgatggcgttgcccagcaggttgatgaggatctggcacacccgcttctcgtcggcacgcaccaactcgggcagggtgcccgtggtctcgaagcgaaagcgcagccccttctcggccgcctgcagctcgaacatgtcggccagctcccgcagggtgtcggcaaagcgcatcggcctcgcatgcagcgtgagcttgccagcctcgatgtgggcaatggccaacgtgccctcgatgagcgacagcaggtgctcgccgccgcgcttgatcaccgccacggcttgctggcggtgcggcggcacggactggtcttcgcccatcaactgcgcatagcccaggatgctgttgagcggcgtgcgcagctcgtggctgatggcgctgatgtaccggctcttggcctggttggcctggtcggcggcgcgccgggcctcgtcggctgcgagcttggcctgctctgcgacctcgcgcgcttcatccgcggtctgcttggcggactgaagcgcacggtcggtcgcgcggtgcaactcgatctcgcgcatcagcaagtgggtctgccggttcgattcctcctgcgcgaccctccggctctggtgcgccagcaccagccaccaggccacgacgcccgcaatcaccagcaacgccatgtaggccttgagaaaaccggagcgcaacgacgactgctgcacgctggccagcgcctcggccagttccgattgcgatgcgatctgcagcgcgctctcgcccaatgcgcgcagctcctgctgatagagcacgccaaacaccaccgccagcaccggcacgatgatcagcatcagcaacaggaagtgcccgagcccggtgtcgagatagcgccaactgaagcgcggcagcagccagcgcagcgccgaagaccattgcgcggagaggctcgcatgcggcttgcacaggtcgccgcagcgcgcatcgagcgtgcagcacagcgagcagatcgcgccctggtaggccgggcaatgggccatgtcgggcccttcgtactcgcgctcgcagatcacgcagtgctgcaccttgaggcgctggtagctgccttccgctccgtcctcgtgcaggtcgtgctcgacccgcgcccagcgaaccgcacgcgggcccgtggccggcgcaaaggcgaccgcgccatgcgcgaccgagccgcgcgccaggtagtacttgccgccggtggcccaggccaggagaggcgacaccaccagtgccgtgccgagcgcgatgagcgccgagaacgcctgcgccagcgggccgaagacgccgaggtgggcggtgatggacagcagcgaggccagcgccatcgcaccgacgcccaccggattgatgtcccacagatgcgcccgcttgaactcgatgccgggtggcgacaggcccagcggcttgttgatgacgaggtcggccaccaccgccatcatccaggcgatggcaatgttggcaaaaaggccgagcacgtcgcccagcgcctcgaacacgttcatctccatcagcatgaaggcgatgagcgcgttgaacaccacccacaccacgcgccccggatggctgtgcgccacgcgcgagaaaaaattgctccaggccagcgagcccgcataggcgttggtcacgttgatcttgagctgcgagatcaccacgaacagcgcggtcgcggccacggcccagccgtagttcgggaacacgtactcataggccgcgaggtacatctggttcggatcgaccgcgcgctcgaccggcaccatgtgcgtgatggccaggtaggccagcagcgcgccgcccagcatcttgaccacgcccagcaccacccagcccggcccgccggccagcacgccagcccaccagcgccgggcgctccccgccgtgcgcgcgggcatgaagcgcaggtagtccgcctgttcccccatctgggtgatcaatgcgataccgaccgtcagcgcggcgccaaacaggtgcagatcgaagcccttggtgctcgctttcgacccgttgtagtgcacgatgccagcgaacgcaccaggatcgcgcaccagcacgaagacaaaaggcaccaccagcatcaccagccagagcggctgcgtccacagctgcagccggctgatggccgacaccccgtgggtgaccagcggaatcaccaccagcgcgcacaccaggtagccccagaccggcggcacgccgagcgccagctcaagcgcatacgccatcaccgcggcctcgagcgcaaagaagatgaaagtgaacgacgcgtagatgagcgaggtgagcgtggagccgatgtagccgaagcccgcgccgcgcgtgagcaggtccatgtcgacgccgtagcgcgcggcatacacgctgatcggcacgcccgccaggaagatgatgagccccgtgaccacgatggcccagaacgcattggcgaagccgtattgcaccagcagcgttgcgcccacagcctccagcaccaggaacgacgccgccccgaaggccgtgttggccacgcgccattcggaccacttgcgaaagcgctgcggggtgtagcgcagcgcgtagtcctcgagcgtttcgctcgccacccagctgttgtagtcgcgccgcaccttgacgatgcgctggggcgcgtcatcggggctggtggaagtctcggcggggttcacaccgtttcggtgcatctttcgtgccatccatacgtcgtttggcgaacaccggcacgactgttgcaaagctgaagcctgcccaataatggcccgacctccacgccctccgatgccgctcccatggaactgaccccgcgcgaaaaagacaagctgctgatcttcaccgcagcattgctggccgaacgccgcaaggcacgggggctgaagctcaactaccccgaagccgtcgccctgatctccgccgccgtgatggaaggtgcccgcgacggcaagagcgttgcggcgctcatgagcgaaggccgcacggtgctcacccgcgccgacgtgatggacggcatcgccgagatgatcccggacatccaggtggaagccaccttcccggacggaaccaagctggtcaccgttcaccagcccatcgtctgactcccgctccagaacaagaaagacctgccatgcgccacaacgcttccaagacccttgccctcgtcgccctgctgctgccgtttgcggccagcgcccacaccggcgtcgacggcggcgtgcaccacggcttcgtcaccggctttttgcacccgctcacgggtgccgatcacctcgcggccatggtcgcggtcgggctctggagtgcgctggccgcgcgccgcgcctggcccgatctgctgtgggcgccactggctttcgcgggcatgctgctcgtgggcgcgctgatgggactggcgggcgtgcagctgccagccgtcgaaccgatgatcgcggcctcgctgctcgtgctgggcctgctggtcgccacgcgcatccgcctgccggccgcggtggccgcggcggtggttggcgtgttcgccatctttcatggcgtggcgcacggccacgaactcgcgggcgagcaaggcgcggcgttgacgctggccggcatggtcggcgccaccgtgctgctgcacctcgcgggcatcgcgttcggctgggcgctgcgccacgccaatgcctggctgccgcgcatggcgggcgccgccgtggtggcgctgggcgccacgctgctctcgcaggccgtctgaacaaaggcaccgccaccatgacacccggcgaacttttcaccgatgagggcgagcacatgctcaaccctggccgccgcaccctcacgctggtggtgcagaacaccgccgaccggccgatccaggtcggctcgcactatcactttgccgaaaccaacggcgcgctcggcttcgaccgcgaagccgcgcgcggcatgcggctcaacatcgcttcgggcgccgccgtgcgcttcgaaccgggccagcagcgcaccgtcgaactggtcgacttttcgggcgatcgcatcgtctatggctttcgcggcctgatccaagggaagctctaaaaaatggccaccatcgggcgacgcgcctatgcagaaatcttcggccccacggtgggcgaccgggtccgccttgccgacaccgacctgctgatcgaggtcgaggccgactacacgctgcgcgccggcggctacggcgaagaggtgaagttcggcggcggcaagacgattcgcgacggcatggcgcagtcgcagcgcaccagagcccaaggcgccgtcgacaccgtgctgaccaacgcgctgatcctcgaccactggggcatcgtgaaggccgacatcggcctgaaggacggccgcattgccgccatcggcaaggccggcaaccccgacgtgcagccgggcgtggacatcgtcatcggcccgggcaccgagatcatcagctgcgaaggcaacatcgtcaccgctggcggcatcgacagccacatccacttcatctgcccgcagcagatcgaggaagcgctcgcttcgggcgtgaccaccatgctcggcggcggcaccggcccggccacaggcaccttcgcgaccaccgccacgcccggcccgtggcacatcgaacgcatgctgcaggccgccgacgcgttccccatgaacctgggcttcctgggcaagggcaacgccagcctgcccgatgccctgcacgagcagatcgaagccggcgtcatgggcctgaagctgcatgaagactggggcaccacgccttcggccatcagcaactgcctggacgtggccgacgccaccgacacgcaggtcgcgatccacagcgacacgctcaacgaatcgggctttgtcgagaacaccatcgcggccgtgggcggccgctcgatctgtgcctttcacaccgaaggcgcgggcggcgggcatgcgcccgacatcctgcgcgtggtgggcgaggagaacttcctcccctcttccaccaacccgaccatgccctacaccgtgaacacgctcgacgaacacgtcgacatgctcatggtgtgccaccacctggacgccggcattgccgaggacctggcctttgccgagtcgcgcatccgcaaggaaaccatcgccgccgaagacgtgctgcatgaccttggcgcgatcagcatgttcagctccgacagccaggccatgggccgcgtgggcgaagtggtcctgcgctgctggcagaccgcgcacaagatgaagctgcagcgcggcaagctgcccgaggacaccgagcgcaacgacaactttcgcgccaagcgctacgtcgccaaatacacgatcaaccccgccattgcgcacggcatcgcgcacgaggtcggctcgctggaggtcggcaagtgggccgacatcgtgatctggaaacccgccttcttcggcgtgaagcccttcaccctcatcaagggcggcaccatcgccatggccgccatgggcgaccccaacgcgtcgattcccacgccgcagccggtgcactaccggccgatgttcggcagctacggcggctcgctggccaggagttcgctcaccttcgtctcgcaggccggtctggccgcgggcatcaaggaacgctacggcctggcgaagcacctgagcgctgtgaagaacatccgcaacgtgcgcaagaaggacctgatccacaacggctacacgccgaagatggagatcgatgcgcagacctatgcggtgcgcgccgacgggcatctgctgacttgcgatccggcggtgcagctgccgttgacgcagcggtatttcctgttctaggtgcgcgttcagccagaacgagcctgcaggtgttcgcgaatccaggccgcaaagctgctctcatcgatggcgctggcggcgacgtcgaacatcacaagggttgcttcagtttgcgtgacgaccaatcgctggccgttcaaggcaagaaacaaacccacggcgagaaaggctacgcgcttgttgccatcgacgaagggatgattctgggcaagccctatgccgtaggccgctgcgaggtcggcgaggtcaggctcgccataggccacgagcttgagcggccgcgccaatgccgactgaagcaagccttcatcacgcaagcccgatgcaccgccgtgttcggccaggctctcgtcatgcagcagaacgagcgtgcgctggtcgatccaacgccaagcgctcatttggcaagctggtggaaggtgtcgcggtactcgcgcatgaactcgcggcccagcttgagctgctcatccaccgcagggtcgtacggcgtcagggtgacaccgttggccgcctccgtcatgaacacggtgtcgcccttttccagcttcaaacgtgccaagacttccttgggcaggatcactcccacagagttgccgatctgggtcagtttgagtgccgacattggaatcccagagttataacgattgttatattatcggcaacttaccgccgaaatcaagctcgccatgctcaccgccaacaaactcatgccccaaggccgcggccttgcgcccgtgctgctgaagcgcgccgccaccatcgaactcgactgggacgtgcgccagaaaagccgtttcgacgcgaccgattcgcagggtcggcagatcggcgtgttcctgccgcgcggcactgcggtgcgcggcggcgacgtgctggtggccgaagacggctcgctggttcgcgtcatcgcggcgccgcagccggtgctgcgcatcacgcattgcacggcccacggcacgccgttcgacctgacacgcgcggcctatcacctgggcaaccggcatgtgcccatcgagctcaaacccgaccacctgaagatcgaacccgaccatgtgctggccgatatgctgcgatcgatgcacctgatcgtcgtcgcggtcgaggaagccttcgaacccgagggcggcgcttatggatcgcaggagcattcgcacagcggaggccatggccatgaccatgcgcatgaccacggtcactcccatgcaaaaggccccaagccgctggtactcgcaccggagctgctggacgacgatcatgaccatgcgtgattcagagcggtggttgatcgagcggaacaaccgcagcgcccggtgtgcgcagggcgccgggtgctccccgcagcgaaataaaggaggagccgaaggcgggggacattcgcggaggggagtacccggtggcctgtgcacgcgccctggacaagagcacttcaaaagctgacatgtccgacgcgtccaacaacgcccacagcctcctgcagctcatctggctcgcctccccggccctgcctgtcggcggattttcctattcggaaggcgtcgaagccgcagtggaatgggccggcatcgattcggaggccaaggccatcgaatggctctcagaccagctgtacctgagcttcgcacgcggcgacctcgcactggtcgcgcaagccatcccggcctggcgcgcgggcgacgccgaacggatccgcgcgctcaacgaatgggtcctggccacgcgcgaatcggccgagttcttcctgcagaccgagcagatgggccgctccttcgtcgagtggctcaagctgcaccacgcggacacggccgaggtcttcgtggacctgcccgcaagctaccccattgccttcgccttcgcgctgagccgcaccggcgccacgacacacgacggctgcctggccttcgccttcggctgggccgagaacatggtggccgcggcggtcaaggccgtaccgctgggccagagcgcgggccagcgcatcctggcgcggctggcgcacgaaatccctgccgccgtcgcccacgcgatgcgcctcggcgacgacgagcgccaggcctttgcgcccctgctggcggtgttgtcggcccgccatgaaacacaatactcgcgcctctttcgaagctgactgaaccggacaacgcccatgacctccgccctgcaccacattccccatcgcaccaagaaactgccgccgctgcgcgtgggcatcggcggaccggtcggctcgggcaagaccacgctgctcgagatgctctgcaaggcgatgcgcgacaagtacgacctgatcgccatcaccaacgacatctacaccaaggaagaccagcgcctgctcaccgtggccggcgccctgcccgccgaacgcatcatgggcgtggagaccggcggctgcccgcacaccgccatccgtgaagacgcctcgatcaacctcgaggccatcgaccgcatgctcgaagactttcccgatgccgacgtggtgttcgtcgaatcgggcggcgacaacctcgcggccaccttcagccccgagctgtcggacctgaccatctacgtgatcgacgtggccgccggcgagaagattccgcgcaagggcgggcccggcatcaccaagagcgacctgttcatcatcaacaagaccgacctcgccccgtacgtcggcgcgaacctcgacgtgatggagcaggacacgcagcgcatgcgccgccagcgcccctacgtaatgaccaacctcaagacccacaccggcgtggccgaggtggtggcgttcatcgaaaagcgcggcatgctcaccgcggcctgagccgcttcgtcagagcgcggtccggtcagcgcgtcgacgccgcggtctgccccaggagcggcaggcgcaacgtcagccccagtgcaccgcccgcatgcggcgccgcgtagatgcgcccgccatggcggcccgcaatgcgctcgcacacgcgcgcactcgcggcatgcgcggccgcctgcgttgcctcgaggaacctcgcgagcggcgggctcgcgtcggctgcgtcgaggtctcgccaatggaccacggcctggccgctttccacgcgcgccgaaacctgcagcgtagccccgggcgacatcacgttcgccgcatacctggctaccttggagagcagttcctccagctcggcctcgatgccgaacacgggcaccacctcgtgtggaacccggatgtcgaaacggatggggcgatcggaggcgcgctcgcgcagcgaggcaatgagcggccgaagatcctgcacgctgctctggctcatcttctggcgcgcttcgcacttcgcttcctctgccatttcacgcgccagcctgccggccttcacgttggagatgaacagcgacacgatgaaggccagcactgcggcgagccccagtccgacggccagggcgatgcccaggcccaggttggtggaatacatggaatcctccgtcttcaatgtcccgggccaggccggaactccagttcgccgccagcgccgcgctcgcagctgcccgacaacgcatccgcgcgccggccgggcagcacggggcgcccgccttcaggctggccctcgcaaacattccaggacgcgagtggcggcgcatagccgccgggcggcatcggcgcagcgccgtgaaagcccgggtacggccccctgcccggcggcgggccgaagggcggaggcggcggaagcatgatgcagcccgaaaggacggccgcggcgagcacgcccgacaagtgatggaatctgatcatttgaaactcacgaacaagttcacgagcgcatgcggcagggctgcgcactgcgctgccctgccgcacactgcctttgacgtcagaaggcgtgacggatgccgaagtcgtagccggtggacgaacgcggcaagcccgtgtagctgacgccggcgctgccgtagcccgtggtgctggcagcactcaggctgccggtgtaggccgcgtcgttgcggttgttcacgcgcgcaatcgtggcgtacagggccgtgcgcttcgagaggttgtgcacatagccgagcgccagcttctgaacgcgcggatcttcgccggtgatgccgacggcgccttcgttgtagcgaaccgtggaatacgacgcacggatgaggcccgcacccaccggcatgctcgcgccgatcaggtagccgttgtagctgtcgtggctgtcgccgacggcgagctcgaacttgttcttcacattcgagagttcgccgaacagcttgacgggaccgaagtcgtacgacgcacccaggttgatggtctgcaccttgcgggtcagcgccgtggtgtcggtggcgatgttctggcccaccgcaagggccacgtccaacggaccattcgcatagccgaaacgtccgcccacatagcgaccggcgttggtgttggtcgacgtcgtggtggtgccggagtcggtgtccgtgttttcgtggaagctgtattgcacctgtccgtagaagccgccgaggttcggtggcaggaagtagccgaccatgttgctggcgcgcgtgtaattggcattgttcaggccggtgctgccgctcactgtgctgatcacgttggtacctgagccgttggtgccgaacggatcgaagacggagtcgttccagaacgtggcggtgtagtcgcggcccagccgcacttcaccgaagccgcccgagaggctcacggtggaacggcggttgaaggtcgaaacgccggtggcgccgtcgtcgttggtgatcggtgcttcgagccagaagctcgctgcgagcccgccaccgaggtcttcggtgccgcggaagccgaggcggctggagttgtagcccgagttggcgaggctccacttgctctgctttgagctcaagcccgtggtcgcgtcgcgcgaggtggccgactggtaggtcacgccggcatcgacgacgccgaacaacgtaacggacgattgggcagaggccaggccggtaacggccagcgcggcgagtgccgtgagggatttcttcattcaggtttctccggttttcagcagctcttcatcgagcagctggacggatggtcctgttcaaatttggaggaatctggtcgatgccgcgcgctttgcaccgactgttgtttgtgcgcacgcccaagcccttcaaatgcacaaggcttcataccagaaatctcccaaaagccgcgcaatgctcggcaaccgaaggagcccgacatgaccattgcattgcagaacaccatcgcagcctcgctgggtgtgcagcagctcaccagcgcattcagcccggccttttcccacctgcgcatacttcgcaacctgatcattcccatgcccgaggggagcccggttcgcaccgcacagatcgatgcggtgctggtgtgcgaaaccggcatctacctgttcgagatcaaggcctggcgcaacgccttcgtctaccgcaagaaatcggaccaggcgccgccgcgctggttcctgcggctgcaaggctgcacccgcgcccgcgaagtcaaagaccccgcatggcagggcgggcgcaagaccacgcagctgcgaagcctcttgagcgacgacctgcgtctgcagtacttcgtgctgctgccctgcgagggcgtcgagctcgaaggcgtgatgccggccgcggtgatcacgcagcaggacctgccctacatcgcgcgcctggtgcgcaacaacgggcgcaccgcgcgcacctatccgctgctcgatgccgaggccatcgaccgcacggcgcagcggctgctcgacatccagggcggcctctcggtcgaagaccacgtgcagaactgccgcgagagaagcgagcagatctcggtgcgctggaacatcgcgggcgcaaacaacgccatgagtggcatcggactgcaatagcacgcgccgcgggcacgcccctgcgtgtcggagggagtcccagatttctccgactttggcgggaaccatgcggcgatatgaatccatccaagtccgcagcggccgtcgctgcattgctcaccgcgcttacatgcggcccggcctgggccgccgatccgttcaccgtcagggacatccggctcgaaggcctgcaacgcgtcgagccgggaacgatcttctcgaccctcggcatcaaggccggagacacctacagcgacgaacgcggcagcgcggccatccgatcgctgttcgagctcggcctcttcaaggacgtgcacatcgacatcaacggcaacgtgctggtggtggtggtcgaggagcggcccaccatcgcggacgtcgattttgtcggcagcaaggagttcgacaaggccgtgctgcaaaaagcgctgcgcgaagtcggcctagccgatggccggccctacgacaaggcgctggccgatcgtgccgagcaggagctcaagcgccagtacatcagccacagcctctacaacgcgcaggtcatcaccaccgtgacgccgctcgagcgcaaccgcgtgaacctgaccttcaccgtgaccgagggcgagtcggcgcgcatcacggacgtgcgcgtggtcggtgccaaggccttcagcgaaggcaccctgctcgacctgttcgaccaggacaagggcggctggctgagctggtacaccaagtcgaaccagtattcgcgcagcaagctcaatggcgacctggaaacgctgcgctccttctacatcacgcgcggctatctcgagttccgcatcgactcaacgcaggttgccatatcgcccgaccgcgagacgatcacgctcacggtcaacatcaccgaaggcgagaagttcgcggtggccggcgtcaagctggacggcaactacctgggccgggaagacgagttcaagtcgctcgtgacgattcgcccgggccagccctacaacggcgaagacgtgagcgccaccaccaaggccttcaccgattacttcgggaccttcggctacgcgttcgcgcgcgtgaaggcggaaccggagatcgaccgcaccaaccgccgcgtcgtgatggtgctgcgggccgaaccctcgcggcgcgcctacgtgcggcgcctgaacatcggcggcaatgcgaggacgcgcgacgaggtcatacgccgcgagttccgccagtacgagggcgcctggtacgacggcaacaagatcaagctctcgcgcgaccgcgtggaccggctgggcttctttaccgatgtgaacgtcgaaaccaccgaggtgccgggctcgcccgacctggtcgacctcgcggtcaccgtggccgaaaagccgaccggctcgctgcagctgggcgcgggctattcatcgaccgacaaggtgtcgctgagcttcggcatcacgcaggagaacgtgttcggctcgggcaactacctggggctgcaggtcaacacgagctcctacaaccgcaccatttccctcaccgccaccgacccgtacttcacgccgggcggcatctcgcgcacgttcaacgtgttccacaccaccacccgcccctactacgaagcggacggcaactacaagctcgcgagcgacggcggttcagtgcgcttcgggctgccgctgggcgagctggacacggtgtatctgggcatcggcgtggagcgctacagcttcacgcccggcaccaatggcgcctacacgctggtcgacggctcttacgtctacaccggcacgccgcaggcctatctcgactatttccagtgcacgggcaccgcgccaagcgtggtgtgcgcatcgaagaacatggtgggcattcccgcgaccatcggctggggccgcgacgaccgcgacagcgcgctggtgcccaccagcggccgcctgcaaaccgccaacctcgaggtgggcgtgggcagcgagctgcgctacctgaagaccaactaccagtaccagcagtacttcccgctttccaagcaatacacgctggccatcaacggccagctcggctacgcaagggcgctcggcggcaccgcctaccccatcttcaagaacttctatgcgggcgggctgggctccatccgcggcttcgagcagaactcgctggggccgacggacgcggtgacgggcggtgcgctcggcggcacgcgcaaggcgatcttcaacatggaattcagcacaccttttccgggcgcgggcaacgacaagacgctgcggctctacaccttcctggatgccggcaacgtgttcgcggaacgcacggcgagcatgaccgacgcacagtggaaagcccagaaccgccttcgcgcatcggctggcgtgggcatcagctggatctccccgctcggtccgttgcgcctggcctatgcggtgcccatcgtctaccagaagctcgacgaggccaacggcattgccgcggaccggacccagcgcttccagttccagatcggcacctcgttttgaagcgggagcacccatccatgagccgcatcctgctggttgaaaaaggccgcgacatggcctcattgctgctcgaaggcctgcagcgcgccggccatcatgtcgagcacatcgacgacggtgttgccgcactcgaccgcatcctcacgtcgccgcccgcgctcacgctgctcgacacggcgctgccgcgcatcgacggcttgcgggtgctcgaggaagtgcgctcgcacagcgaccatccgatcatcgtgctgaccgcgcgcacccgcgaagcggacatgctgcgcgggctcgacctcggtgccgacgactacgtgtgcaagcctttttcgccccgggaggtggtggcgcgcgtgaacaccgtcctgcgccgacatgcgcagcggcggcgactggccacgccgtcgccttcggtggcgttcggggacgcgccgggccgcgtacagatcgagggccggccggctgtgctcacaggccgcgagctgcgcctgttgcagacgctttcccgggagccgggccgggtgttcccgcgctcggcgctgctcgaagccgcattctccgacgcactcgacgtcaacgaacgcgcggtcgacgggcacatcaagaacctgcgcaagaagctcgccgccgcgtcaccttcgcacgactggatccgctcgatctacggcgtcggcttcgtcttcgaggaacggtcggcctgaggccctttgcatgcgggcttcggcggccgggaatcccggccaccggtggccatgatcggtgcaagggtcgacagcgcagagttccccgcgttgcctttgtcgtcctccgggcagccgtcgcgcgcggccagcacagcaccggccatcaggccgcacgaaagcagaaagcctgcggcacgctgaatgaacatgggcccgttgtcctgcagcgcctcggtgcgagagagccacacggcgctcacgcgcggcggggcacattggccccctctccgatgaaccgcggctttctcacctgcgtcatggcgtctccttctttgccgcggtgccggccgcggccgagcgggtggcacgcgcttcggcccagacgaccaccagcgcccacacgtgggtcaccagccagaaaagggcggtcagcgcaaacagcagtgtgtccatgcccgggtcggaccagacttccgaccaggaccacgcggaagccgatggcgcgcaatgggccggcccggcccatgcgagcacggaggccacaagggcttggaaagtcttgttcgggcgtcgatgcatgcgcggattcatggcgtgcatcgtgcgattcgattcgggagaaatatgggagaagcgttctcccatatttctccgcaattcaaaatcaagatcggcggtttccccatgacgcccttcagccccgaacgcatgccgcagaatgcggccatgcatctcccgagcccatgccgcgtctgacgctttccaggaaaatcttcctggcgctggccgccctgctgatcgttctgctgctcagcttcgcgggcctttccatcgttgcactgcagcgaggcctcggctcctacgtggcagagatcgagatccgccgcatggactggctctcccaactgctgctgaagcactacgccgccaacggcgactggaagaagctgcgcgacaacgacgatgcctggcaccgcctgcagatgggccggctcgcggccgtgctcgatggtgccagcagccccgacgaacgaaagcttccccctggtacgaaaaccgcgggccgggcggcaacggccccgagggcagcccagagaacggctcccgcccgccccctcctccgccatcgccccaactcgacctgctgcccaagcggttcgtgccgctgccgccgccatggtcttttcccgatccgcgcgaagccgccgattcgatctaccagcgcctggccgtggtcgacgcgcagggtgcgcacgtggtcggggcgaaggtcgaccaggagaatgccgcgcgcctgccgctgcggcacggcaggtcggtcgtcggctatctgatgctcgcgccggtgcagggcctggagagcgaggccgaccgcgcctttctcgcgcgccagtcgggcgtgatcggcctcaccgggctgtgcgggctggtgtttgccttgttgctgtcgtggctgctggcacgccgctggttccggcccatcgacgacctcacgcaggcggcgcaggatgttgcgcgcgggcggctgtccacgcgcgtggccgtgcagggttcggacgaactcgcgctgctcggcaagaccttcaacgacatggcgcagcgcctggacacggtcgaagcgtcgcgccgcgcctggctggccgacgcggcgcacgagctgcgcaccccgctggctgccatgcgcgccgaaatcgaggccctgcaggacggcgtgcgcaccttcgacgagcgcaccgcgctgcggctccatcggcaggtgatccggctcggccagctggtggacgacctgcgcagcagcatgcgcgagccgcaaagcgacttgctcacgacggcggtgtttccactttcgctgctgaaggaagcactcgaccacacgcgcgaccgcttcgccgcacgcggcattgcggtggaccgcagcgcgatcgacctggtctcggcgtgggcgcagccgatgatcgacggcgacgcgcaccggctgcaccaggtgttcatgaacctgctggaaaacacgctggcctacaccgacgccggcggccggatgcgcatcggcgtcacggtcgatggcgcctggtcgggcaaccgccttacgctgcatttcgacgacagcgcgccgggcgttcccgaggcggaaatgccgcgcctgttcgaccggttgtttcgcggggaatcgtcgcgcagccgcgagcttggcggctccgggctcggcctttcgatctgccgcgcggccatcgaggcccacggcggcaccatcgatgcccaggcgtccgacctgggtggcctctgcgtgaccctcacgcttccgcttgcaaggagcacttcgccatgacccgcatcgtcatcgtcgaggacgagctcgacatcgcctcggtggtgcaggactacctgcgccacgccggctacgaaaccgagcatttcgccgacggccagagcgcgctcgagcacctcatcgcctcgccacccgacctcacgctgctcgacatcatgctgccccggctcgacggcatcgaggtgctgcgccgcgcgcgcgagcacaccagccatccgatcatcatgctcaccgcgcgcatcgaggaagtcgaccgcctgctcgggctggagcttggcgccgacgactatgtgtgcaagcccttctccccgcgcgaactggtggcgcgcgtgcgcgccgtgctgcggcgcaccctgccgcccgatgaccgcggccaggcccggcaaggcacaccaggcctcgtgctcgacgacgtgcactggcgcgcctcgctggagggaacgccgctcaacctcacgcgccgcgagttcggattgctccaggtgctgtcgcggcaccccggccgcatcttctcgcgcgcgcgcctgctggagctggcctacgacgacaccatggacgtgacggaacgcgccatcgacagccacgtcaagaacctgcggcgcaagctcggtgccgtcacgccgtcgcacgactggatccgctcggtctacggcgtggggtttgcgtgggaggcgccagcgcagggctgagcggtcttgctgcgattagaggccgcagccaagctgctttgcttgaaggtgagacgctccgtgcctagactgaagtgcgaaggcacccgcagtgccgggggccaaggagttggccatgtacaagcgcatcctcgtcgccaccgatggctcttcgctctccgagcaggcggttgcaaccgccatcgaccttgccgtgctgacccgggccgaactggtgagcgtcaacgtcgtgcacgtccagccctacggctatttcgaaggctcgatgatgctgaaccagcgcgaaatcgaagcctcgcaagagcaggccaaccagaccggccagcgcctcgtcgatgcggtccagagcgccgcaaccgccaagggagtccgcagcacgcaggccatcgtcatgaagtcgaaccaggtggccgaggccatcatcgcgaccgcaaagaaccagcagtgcgacctgatcgtgatggcctcccatggccggcgcagttttgcgcggctgctgatgggcagtgagacgctgcatgtgctgacgcactcgcacattccggtgctcgtgctgcgataaccgcacggtgtaggcgggaaaaagcgcccctttgactccatctgcggcctctgcacaaccgtggaaggtaaagtccacggcattgctgcatcacgcaaaggccgtcccaagggagtctgaatgaaatcgatgttcccccgcctcgcgggctggaccctgctgatcttgtcggtcctggtggccatctgcgtcgcggttgccctgagcttcgactggaatcgcgccaggccctggatcagccaacgcgtcagcgaagcgaccggccgcccgttcgcgatccagggcgacctggttctgcagtggggcagccccgaggccgaaaccggctggcggcgctgggtgccctggccccggttgaaggcacaagacatcacgctgggcaatgccgaatggggcaagaccggcccgcacctggccgagatcaagcagctgaccttctccctcaacccggtgcatttgctgaaccgcacgatccggattccgacgctggaactcgacggccccgtgctttcgctcgaacgcaccgccgacggcaagaacaactggacgctggcatccggcaccaccacggccccatcggtctggaagctcgagctgcagcggctggtgctgagccatggcacggtcaagctcgtggatgccacggcaaagctcgacctgaaggtcgacatcgacagcctgccgaaagaaagcgccgagggctacggcatcggctggaagctcggtggcaccttccggcaaacccaggtgcgcggaagcggccaggccggcgcagtgctttcgctgcagcaggacaacaagccctacccgctgcaagccggcgtgcagatcggcgccacccgcatcgacgtcgtcggcacgctgaccaaacccgacgcgctggcggcgctggacctgcggctcaagctctcgggtgccagcatggcgcacctgtaccccatcaccggcatcaccctgcccaacacgccgcctttcagcaccgaaggccatctggtcggcaagctcgacaaggccggcggccgctggctctacgaaggcttcaagggcagcgtgggtgcgagcgacattgcgggcacgctggaatacatctcgcagcagccgcggccgctgctgcgcggtcaggtgcaatccaaccagctgcgcctgcaagacctggcgccgttgatcggcgcggactccaacgccagcaaggccaagcggggtgcgcctgccgtccagccggcggacaaggtgctgccggtggaaaagttcgacacggcaagctggggcagcatcgacgcggacgtgaagtttgcgggccgcaagatcctgcatgcgaaggacctgcccatcgagagcctggtggccgatctgcatctggaggacagcgtgctctcgctcacgccgctcagctttggcgtcgcgggcggcacgctggccgcgacggccaggctggacggccggcagaacccgatccgggcgaaccttcagctctcggcacgccggctgaaaatcaaggagctctttccaaccctggacacgatgcgcgccagcctgggcgaagtcggcggcgacgccgcgttgtccgcctccggcaactccattgcagccctgctgggcacttccaatggcgaggtgaaagcgctggtgagcaagggcaccatgagcaagtttctgctcgaagccatgggcttgaacatcggcaacgtggtcgcgacccagctcttcggcgacaggcaggttcagctcaactgcctggccagcgacttcaaggtgacgcaaggcgtgatgcagacccgctccttcgttctggacaccgatgaatcgatcatcaatgtgaccgggctcatcaacctctcgaacgagcaactggcgctggagatccagccgcgaaacaaggcactgcgcgttctttcgctgcgctcgccgctgtacgtcaagggcaccctcaagaacccggatgtcggcgtcgacaagggcgcggtcgcactcaagctgggtgccgcggtggcgctgggtgcggtggcaccggctgccgcgctgctgccgttgttgaacgtgggtacgcaggagttcgcgggatgtgccccgctggaggctgccgcaagcaagaagccgcaggcacctgccgtccggccggtgaagcagcgtcagcaatgactatggctcagggcgcggatccccgcttggccgcgacagctgcccggcacgcctcggcggcgcgatgcgatgcgagctcgaagcagcgcatctgcgccgcgcgtgcaatcgcctcgagcgagcggcgttcctctgccgcctcgacctgaaattcgacgagccatttcatggccattgcgagtgcgatcaaaaggccgaccagggcggccatcaatgtcccccgccagttccggattcgaaaggcggggggttcggggttgtccatcgatcgcgtgggatgacaggcggcttatggcggaggcctgttcgcgttcagcaattgcctttcttggcttgtccgggcgggcagaagtttccacctttttgcgcgccccctccctcgtagacgggaaccacgcagccgctcatgagcaaagagacggcaaaggcaaacatcagggtggcagcggtttttttcatgggggctccttgttgaaattgtgaatcgacggcgcgagcagcctggggccgtccgcataagcgccaagatagagggcgccataacatttttccaggaactgtttcacgctcgggtttggttttcgccggcacggatatctaagatgcaactctgcccagtacttcacgcacttgcaaagatgcgaccgcaattcaacgaacgaccatcgacatccgtcgcgggcccgttcgaaaatcaagcggcgcattccgtcaaactcgcgtgctgtcaccgatagactccacaaccgttctactgaaaaggaactcctgctttgaacaaaaccgaactcattgccgccatcgcggaagacacgaacctcagcaaggccgacgccggccgcgctttcgattccgcgctcgaacacctgtcgcgtgccctggtgcgtggcgagtccgtccaactgatcggctttggcaccttcaccgttgcaagccgtgccgaacgcaccggccgcaacccgtcgaccggccagccgatcaccatcaaggcaagcaagagtcccaagttctcggcgggcaaggcgctgaaggacgccgtcaacgcgggctgattctccccccttcgcatttgcaccgaccggcggcgcgcacgcactcagccctgcgcgctgctccacccgcctccgagcgccttgtacaggttgaccaggttcacggcctgcttgagctgcagttcgatcaactgctgctgctcggcatagagttcgcgctgtgcatcctggctcgagaagtagtcttccaggccgccgcgaaagcgcgtccgggaaatgctggccactttttcaagcgactgcacgcgcgtctgctgcgcctccagctgaggtcgcaggtggtcgtcggcaatcagcgcattggcggtctcccggaaagccacttgcgccgcgtattcatacgacgacatggcggccgcaagccgctcttcgttggcggtgatgttggccgagcggcgcccccagtcgaacaggggcagcgacacaccaagcacgccggcccagctcctgttgccgctgctgagcagcgaagacaaatccccgctgatgccgcccgccagggccgtgagcgagatggtcggcagcatcgcagccttggccgcacccacgcccgaattggcagcttcgacccgcgcataggcggccagcaggtcggggcggcgctgcagcaggctggacggcaggcccgccgtcacaggggccgtcgagcgctctggccagggccgcgcgctgcccgtctcgggcggcaccggctggccgaccagcacgttcaaccactgaagatcctgcgcgacgcgcatgcggtattcctcttgccgcacccgcgcgttctgcaacagcgactgcgcgcgatagacgtcgagctgcgcggcgccgccggccgccttggcgcggccgatcatgtcggcgttggaggagagcccgccttcgttggtattcgccagcgcgagcaacgcccggtcggcgcgcagcgtgagatatgcgttcgacacctcgcccaccaggttcatgcgtgcggccgcgtaatccttgtcgcctgcttcggccaaggcgccgccttgctgcgccgtgctctgctggcggccgaagaagtcgagctcgtacgaggtcacgccggcctgcacatcgaagctgttggacacgcccccgttggtcggtacgttgccaatcgggctgagcgacccctgcggcgtggtctgcgcgcgctgggcatggcccgacagcccgatctgcgggaacagcgaggcgcgggttccggcatacacggctcgagcctcgcgtgccttcgcagcgtagacgcgcaggtcgcggttctgcttgagggcggtgtcaatcagcccgcgcagttcctcgtcctgcacgaaactgcgccagtccaccggctcggcgcttggcgccgtggtgccggccggccattgcgtaggcacggcgaggtcgggctgcttcatcggcggcgtgagattgcatccgctcaccaccagcaccacgcaggttgcgatcaccagcaggaacagccgcagaaagaggcgcatgaagcccgctccaggcgcgccgaaccccgcgctctcgagcaatgccgaagcggctcgccatggccgcacctggactgcgacgtggcttggcggcacggtgaacacgtggctcaccaattgttcgcgctgggcctccgaggtggcgtcgaagcgcagctcggcgcccgcggagcttttgcgcgcaaggcgcgccggtagccagcccacggtatcgacatacacctccagaggttgccccacgcgcatgcgtttcagcggcgccttggcttccaccagggccccgtccgccgcgatgttgacgaagcgtgcctcgccctcacccgccgcggtacgcacccgggtgcgcgcgcgccaggggaagcgctcttcctgctccggccgcggcaagtcgacacaggccatgagcgcggccaggcacagcagcagtgcgataccggtccacacgaggttgagctcgtcgccgggcgtgagcgcctctccgctcaaggccaccgatgcgccgccgagctgcagcgccaccagcagcccgccgaacatggcgaccagcttccagtgcacgaccgtcttcgagcggtcgagccccttgttcgtcaccttgaaaggccggccgaagggccgcagcatcgcgcttgcaagcgtgctggtaacagccatggccgccaccagctggctcacctcgctgaagacgggcaggcagcgccgctcgctgatccagtagctgtaggcccagaacatcacgagcggcggcaaaccgtaggcggcaaaggcctgcggcgaggcatggaagaccgagacgcccgcataccagtacagcgcaggcgccagcatgatcagcgccatgaagggcttgccgagccagtgcagcaggccgtgcaagaagtgcatccgcgccgagaggctgtagcccttgccgcgcagcggcccctggggcaggagcgcgagctgcaccgtgcccagacaccagcggctgcgctggttgatgtagtcgatgatgctctcggccgacaagccgttcgacagccgttcgcccagccagcgcgtaacgtggccatggcgcagcagcaggtaggtggtgtggatgtcttcgcacacgctgcccaccggaaagccgcccgcggcggtgatcaggtcgcgccgcacgatgaacgaggtgcccacgcagaaggccgagtccacggcatccttggccggctgcagcacgtcgaagaacacgcgctgctcgtcgacccagctgtcggtggcgcgcaggttgtgctggatggggtcggcgttgtaatagaactgcggcgtctgcaccagccccaccttgcggtccgcgaacaggcccagcatgcgatagatgatctgccgctgcggcgcaaagtcggcatcgagcaccaggatgtacggcgcgttggtcacgcccgccgaaatgcgcagcccgttgttgagattgcccgccttggcgtggctgttgtcgggccgccgcgcatagtgcacgcccttgcgctcgcaatagtcgcgcagccagtcgcgccgggtgtcgtcgagcacccagaccttcacctgcggatagtcgatggcctgtgcggcgatgatggttttttccagcacggccagctcttcgttgtaggtgcagatgaagacgtccaccgccggcaccttggcaccaaggcgccgcagctcggcttcgccgcggtcggccagcgcatggttgtcgcgccgccgcaccagcatgtggatggacatcagcgtgtagacgatggccgtgagctcgaacgcgaggaacacccacgcaaacagggtttcgaagcccaggtcagacggcggcatggtggcgaccacgcgccacaccgcataccgcatcaacagcagcgccgtgagtccgccaaacagcatgcgatgggaggcgtgctggacccgcccccatgtcatcaagagaagtgcgagccccgcaacgagtgcgttgagctggaactccggtgtggcaatcaggtgggacatggtgaagcagctcctgcggcaatggtcttgccggtaaaggggttgaagcccgtcgcggccagcgcgatccaggcggtggcgccgaggtggggccagcggtagtagaaaaagtcggcacccgccgagtccgggccaatggccaggccggtggagatgcgcgcactgggcgttgcgtagtacaggccgttgccggcgcgctgcgacgccagcagttgccacaacgcttcgggcgccgagcccttgagcgccaccagggttgcggcggcctgtgcggtgccctcggtccagatgccgtcagggttgcgcgagaagccgtagccctcgccggagcgatggttcttctccacccaatcgagcccgcgcgtccaggcgcatgagccctcgggcgcggccagtattggccacagctgcgcgtccaggccagagccctcggtggagatggtggcgccgtcttccttggtgccgatgtagaagcgctgctccgacgggctccacatgcggcgcacaaactcgagcgcggtgcgcgcctgctgccgctccgcgtcggcctgcccgcctgctgcacgcgccgcccacgcggccgtcatggcgatgtcgatgttgtgctcggtcgatttccaggtctgcgcgcgctgcgcgttgtcccagccataccagccgccgttgtagccgtcgggcgcgtttttggcgcgcgtgcgctgctcgatccagccgagcagcttgcgtgcatttgccagatacgcgggcgatggttcggcctcgttcaggttcagcagcagcaaggccgcccaagccacgttgcccgtggctgtgctcacctgataggcatcggcgatccactggttcttggccgtgtcccagcgccccggcagcgcggctttgtcctccgtcatgggacccgcgcgataggcgttgcgcacacgcccatcggccgtgttgggatcgcgctccatcgcacgcaccacggcgtcgccgatgcgcttggccgatgcggcgtcgccgcaggccagcagcgcgatgcccgccagtgcgttgtcgtaggtgaaggccgcgcccaccaacgcaggctccagcggcgtgccctgcttcgcgtcggccagccggtagctggcgaggaacagcggcccggaagcagcgcccttctgatcttccgccacggcgcgccgcagcccctcgcagctctgccgcgcaagcgcttgctgcgccgcgccgccgggctgccgcggctgctgggccaacgccgcggacatcggcagcgccaaggccgccgatgccacggcgcaatgcgccagagtccgggagaacgggaagagctgcatggtttgctttcgaagcgggcggtacgtctgtgcccgtgctcaggacttgaggctggccgataccaccttgccgggcgcgcacaggttgttgcccgcggcggttgcggccgacgacacgtccttggcctcgatgcgcgccaccgcgtagagggagccctgctcggcgaaggggaacggcacgctgtaggtgctctgcagttcttcagacgccaccggcagcaactgctccacgcgcgccggcaccgcggcgccgttttcggtcagggttacgtccagcgtcgagccgatgctgaggcgcttggccacccgcgccggaaacaccgccaccacgccgagccggctgcagtcggtcacgcgcaccagcgaggcacccgccgtgacgtacgcgccttcgggtgcgagcaccgagtgaacctgccccgcctgcgaggccttgatttcgtaagaggacagcttctcgacccggcgccgttcctcgtcttcgagctggatcacctgcttgagctgctggaggatggcggcgccgtcctgctgggcacggccgacgctgttgcgcagcacctcgcgccggcttgcgagcgtctggaagaggctgttgccacccgtgcccacgaacgcaccctgccccgcgctggccaccgtctgggcctgcccggcaaaggcttgctccgccaccgacgcattggcgcgcgccgtgttcagttgcgccatcgacgcgttcatcacctgctcgctgatggcgccctgctccagcaaggcctggttggtcttgaccttgttctcctgctcttcgaccatgctgtgcgccacgtcgcgctggcgccgcgcaatctgccaggcctcccaggcctgggccacggaagcctcgcggtgaaccgaggcctcctgcccgacggacctcatctcctggttgtcggccttgaactggttgcccagctgcgccaactggctctgcagcgcgagatgctgcgaacgcagcgtcgtgagaatctcctggctcacggtcgggttgcgcaccgtggccaccacggtgccgggctccaccacgtcacgcgcatgcaccaccatctgcgacaccacgccgttgataggcgacgtgatcaggccgacaggcgcctgcagcaccgcccgcgtggcctgcgaagacagcagcggctggaccagtgtggccaccatcagccacagcacgaaggccagcagcgcataggccgccagcttgggaacgaaggcgcccgcctgccggcctcgatgagggctgcgcggaacccgacgggccctcgcgctggcagtgcggcgatcgccgcggggaaaaacaaatgaaggcagtttcgacacacgcataccccacctcttgatgcgaaggcgtgcgccggaaatcggcgcaacatccatgaatgaaagggaactcgcctgtagcccgaacggagccgccggcgcctcgagggccgccgcgtccgcatgctgcagtgcaatacgaaggtacggccaaagccgatttaccactgcttcggtgagcaacaagatgtgcggacttcacatcctgaccgaccattcggtcgagctaacttcctacagtggcgtcggatttatcgctgttgacaacgaaaggcctcgtccggcaggcaaaggcggccggtttcaggactgcccagcaagcgctccaagccgcgtccgcaaaaagcgccggagcgcggaaatcgagccatcgggatgcggcagccgcgacctgggttagccgaacatatccggtaaccaacccgtgcgactctgacggatttaggcaacgccgaggccgagaaaaaagcggccagcgtgccattccgcaacggtctcgaaggggtcgcgcttccgcccgcacaaggcacttcacgaggcggccgtttacaagcgccgtacgcacgacacagcgcaatacaagcacctgcacagttgcattcatagtgctcatccgcggtctctggcgccttgccaaggagtttgcgaaagccaccccacaacgcccttcggccaccttaccgagggcccatcggagcacaagtcgtgtcatcgccgaaaaagaatgccgccttcctcgggtcgatctcgggccacagcctccgggcgtggctgtggagcgcaggaagaagcaggcctcgttcgcgtgcaccggccggatctagcgcgcagagatgtagcgttttttagttaatgccatgtaacgccatccggcgttaccgacaggccaaccgggcgcttggacgcacgcgcgcggcggaatgcccgccgactacgcgacgtcagaggggcatgtcatgttcacacgctacgccattcgcacgctgctttgcgttgccgccgtgcccgccatctccgaagagcccgccgcaccaatccatgaccgcgtgtttctgagcaaaaccgagatcgagaccaccttgatcggcaagcccatcgtttcaagcaatctttcgaccggcatggtctcgcgctggcagttctattcggacggccgcgtcgactttgccaaccaaagcgggcccggcaaggcgtcggggaagtggtttctcaaccccgatggctcaatgtgcgtgacgatgatttctcggaccgggtgccgctactggttcaggaacgagaaggacggcgcccttgcgaatgccgataccagggagccgaatgcacctacggtggctgagatacggtttgagtagtagtgcgaggtcgagtggttgggcctgggataggcgaggttttgccagccagttctcccagtcagcctcgggcagaagagagaactcagtcgacgatgcgaccggcaagcggtcatcctcacatggctgcaagcctcaacctgcctgagacctcgcagcaacttcggccataagcctctgcatcacaccgggatcgaaggccaaagcgatgttgatgcagaacgagaatcgaaaccagatcgtgaagaggctgaggtctcccgtgttagccattgcaaagcgatagttaaactggtcgctcaggtcgacggtggctcgacgcaggttggcaaaacctgtgggcactgtgaagatgtcttcggggatcgtcccctcgatctgattgaagttggtgaaccaacgatgccgaattgctgcctcggttggcacaatgcgctcagaatgcttgaagtgcagggccttggcaagcttctccgcaaatactggcactgccaggcgcgcaggctccgggacgctcattagcggcaagtcgctataggtctggccaggatccggcttgagtcccacacgccgcgcgagctcacgctttcgattcgcagtgagttgcattgacctcagcatgccgggcttcaatagcgggcgtgcaagacgctccaattccggttgcgatgacgcagactcggcgtctgcgccggggtgtaggcgagacataagcgcaacccaggattcggctgtcttgctgcctgcgttgcacgtcatacaggctggaaagacgtatccctccggccattgtcggcgagaaaagatcgcgcgcggcgggcaatggtcaaccgtagtagccgcggtgcagccgccacaaaaaatgcactgattcgtcttcgagaatgcgacctcacgggcgctggcctctttagtccgtgcctgccccattacgcggcctatatcggcacgacgctgcctgccggcactcgcctgaggagaaaaactcgatccatcaggttctgaattttctcttcggcgaaagtacgttctgtcatcgttggtctgtctttgaggggcgcttggcaactcagccggtgcatgggtcagtctacggcgaatcggccttcctctgccacgccaccgccgccgcgcaccactcctgcctgcactcagcgcttcgaactaagctgcgccgaccgattgcacgagtatcaggtcgtcagcctcgagtccttctgccgtgaacagttctggagtagcctcctctggaattccttccagcataagcgccgctcttgcttgttgaaaggctcgccgaacagacaagccgaaccccagcgctgagtagaactgcgacgagaagacacgagcagcatcgtctccaattgaggtgttcattccgatcgcagcaggaacatgctcaacgacagcctctgcctgaccgcgggagtaacacgtgttgaagaacaccaactggatatcgtcagacccggccgccatggtctgcacaatcgcctccttcgataccaacttcgcatttccagcgttgtcctgaaagacgatctcgtcttgatccgatccatgcccactgaagtgaacaacggtcggacgtatctcgtttatcgcctgcagcacgtccatgggccgaaccgcccatcgtgacttcaattcgaccgcgtccctatgctgcgactttctgatcatctcctcaatgccacgaacctcttcgtcaagcctcagctgctgctgatcaatcgggttagcagcaagaaaaagcacggtgatccggcgcggtaactgttccagctttttcagcacatccatcgtaagttgatggtgctgacttaccgctcctgccagcgatgccatacgacgcgcattctcctgcgcagcgcgctgctgctcttggcctttccgacgagtttcctgaatctccgcggaggcgagtcgtttgtgcgcatcattcaaccgagtctgctcgcgggcaatcctcgtctcgatatcagccacctttttctgagatcgcgccgcagcctcctcatgctttttcacatcacgaactcgcgattgggccgaggagggactagtcgctcgccgcactaaatcggcagcagtatttgcgcgcttcttctcgtcagccaccttggatgcttctcgagccttttctgtttgcagtcgagcaatctcttgctgatgtttcagcgcgtctcgtcggtagctctctgtcgtcatctctccaagcatagccttggcgtgcgcaggctggcactccccaaacttacgtctcgactgggcgcagtcgttctacgggattgaactagatcgctccggtagggctccacgagacccgctgacgcgcaccaattttgctgccgcctggccgggcgggtagaagatactgaataaaccgccttatggtcgtcgcgcaagcggcaacggtgataaagcccaaaaggcttcgccgccagtctcgtaaggctgcacaatcaggcctgttcagcgcaaaagggcccagagcaatggcactcctcgacaaccttctcaagtacgttagaagcggaaccgcagaaggagaccgaccatttcttggcgagaccttcgtgtcaccgacgcagttcgaccagctttgtgccattgagcctggaagcatgcgccttctcatcggcaataaaggcataggcaagagcgcggtagtcgaatggatcgcaaaggtctcagacaagaaaaaaattccgtgcctcttgatccggccagacaatattatcacgacaccacagccgacttcgtttgatatcggctcattaaagtcctattactatgatgtgctgcttcgcacaattgcgagcaaaattggctccaaccttaaggggtttttaaagggcgatgccgcacgtctttataatgaggcaaagcagcgcggcattgctcagggagacatcattcaaactacattggaactgatttcggcaatctcattgccagtcagcaaggtcaatggagtgcaactagccaaggatctggcagcgtcgaactccgcgcagaatcttacatcggcgattaatcgccagctgctctcttccgggtctgtcttctatttactaattgatgataccgatcaactagctgccccggatcaagctactcacctaaatcggatctggggtttaattctggctgttcgcaggctagcaggcgaatgcatggcagtgcgtccgatcgtgagcttacgtgcaagcgtctggacacggctaaccaccgaaagcctaggccagagggaccagaccgatcacatgcgcggtttagtgattcctctcttggcggacgataaacttatgcaggcgatcattaggcgacgcctggaacgtgctgctgtcgacgccgggtttgcaagaactgacccatatccagttttttttgaaggcaacgaaatgacgcttccgacgagtgacgcgcgtcgatcatggcagtctttcatcacgaaatcagctagagagagaccacgtgatgccattcagcttattaagaacatgatcgatgctgcaaacagcgaatctcatgtaaagattggaagtgctgacgcaaataaggcaatggccttgtactccagcgaacgagtcgatgacgttgtgaacgaattttcaattgactgcaagaacattcgtgaaattattgattcgcttgcagattgtgatttcgactcaaatttcgagtcgattcgccgccatatgagaactgttccaagcattacctctctgagcgtccgcggcacgcaaatgagacctgaagtcgatgatgacgccatcattcttcttgaactgatgcacgaggcaggagttattaacccccgcgtccctgaccgtacgaaagaccgcgattttcgacatatcaattttcacgacgacccctctttcgtaaggacgtcgaattggaatgatatgcaaggggccacctgggaaatccatcccgcatttcgcacctaccttcttggggtcaagcaggcgcgagttaacaggatattgatgccagccacctcaaggcagcgctgaggcgtcggcaaacgcctagcgatgaactcgtccatccaagtgtcgagaccgatacccctatgtgcgcacccgaaagggggaagccctgcgcggagttttttggccccctccaccgaatcccttatagaaagcttgcaagcgaagtgcttagcctcgcaccctgttttcgggatgttgggttttgtgtgggggtagaagcataaaaacggcccaaggccgctagttttctcgctcagtggcggagagtgtgagattcgaactcacggacgatttctcgtcggcagttttcaagactgctggtttaaaccactcacccaactctccggaaccgtcgattttatgctgaccgtgcgccctcaagcctcgggcaggaaaagcgtctgcaggtcgctcagaaaatccagcccgcgttcggtgggccacacgcggtgcaggtcacgggcgatgaggcccttgcgctcggcttcttccatccctttttggatgctggtcatggccagccctgttcgctcgctgaactggggcagcgtgaagccttctttcaggcgcagcgcgttgagcatgaactcgaacggcaggtcggccagcgcgacttcttcgctctgagttactgcggcgcctgcgcgggcgttgtccatgtacaggcgcggttcgcgaaagcgcacctggcgcacgatgcgatgggcaaagctcagcttgctgtgggcgccggcgccaatgccaaggtagtcgccaaactgccagtagttgaggttgtgcgcgcaggtgtggccggcgcgcgcgtaggccgacacctcgtagcgcgacatgccgctggcggcggtgcgctcggtgatgcggtcgagcatggcgtaggccacgtcgtcttcgggcagcgtcggcggaaacttggcgaaccaggtgttgggctcgatggtgaggtggtacaccgagatgtgcggcggcgcgagcgccagcgcctgggtcaggtcggcgtccaggccctcgatcgtctggcccggcagggcgtacatcaggtcgaggttgaaggtgtcgaatgcgctcgcggcttcttcgacggcggcaatggcctgtgcgcgatcgtgcacgcggcccaatgccttcaggtgctcatcattgaagctctgcacaccgaccgacaggcgcgtaacgcccgcactgcggtaggcgcgaaagcggttgcgctcgaaggtgccggggttggcttcgagcgagatctcgcagtcgggcgccagcttgaggcgggcgcgcacgtcgcccagcaggcggtcgatggcctggggcgaaaagaggctgggcgttccgccgccaataaaaatggtgtggacggtgcggccccagatgagcggcagcgcggcatccaggtctgcaatgagcgcgtcgaggtaggctgcctcgggaatgccttcggcctcggcctcgttggtggcgcgccactcgtgcgagttgaagtcgcaataagggcacttgcgcaggcaccagggcaggtgaatgtagagcgacaacggcggcaacgccgcaagctgcagcgggccgggccgcatccagtgcagcacgtcgttggcctgcggcgcgccggtaggctgcgcgggctgaatgggaacgacggtggccatgggtcagaaccagcgttcgcgcatcagggccagcatggcctttgccgcctggccccggtggctgttggcgttttttacctcgggcggcagctgcgcgaaggtcttgccgaagccgggcaaatacatgacgggatcgaagccaaagccgttgtcaccgatgggcgccttcgtgatctcgccgaccacgcggccaacggcgatgaggggctcggggtcgtcgtgcccgcgcagcgcgaccagcgtgctgacgagtgcggcgcgccggttgaccacgccgtcgagctgctcgagcagggccttgacgttgttgccatcgcccttggcgtagccgaactgcgtggcatagaaggcggtgtcgacacccggcaagccgccaaaggcgtcgacgcaaagcccggcgtcatctgcaatggcgggcaggccggttgcggcgctggcatggcgcgccttggccagcgcgttttcgacgaaggtgcgaaacggctcctcggcctcgcccacgcccaatgccgattggggcacgagcgtcacggccaactccgcaaacagctgctggagttcggcaagcttgccggcgttgttggaggccagaaccagtttcatcgccactacttactcatttcgactcgagggactgctgctgcagcacgatcagttcgccgatgcctttctcggccaggccgagcaggatgttcatctcgtcgcgcgagaacgccgcgccttcggcggtgccctgcacttcgacgaaatggccggcaccggtcatgacgacgttcatgtcggtgtcgcaggccgagtcttcggtgtattccaggtcgagcagcggcgtgccgccgacgatgccgaccgaaatggcggccacgtggcccctgatgggcgatgcggggatcgtgccggcggccagcagcttgttgacagcgtcttgcgcggcgacgaatgcgccggtaatggccgcggtgcgggtgccgccatcggcctgcagcacgtcgcagtcgaggtggatggtgcgttcgcccagcgcggccaggtcgaacacggcgcgcatcgagcggccgatgaggcgctggatttcctgcgtgcggccgctttgcttgccgcgtgcggcctcgcggtcgctgcgcgtgtgggtggcgcgcggcagcatgccgtattcggccgtgacccagccttcaccgctgccgcgcttgtgcggtggcacgcgctcctcgaccgaggcggtgcacagcacgcgtgtctggccgaattcgatgagcaccgaaccttcggcgtggatggtgaaaccgcgggtaatgcgcaccgggcgcagctggtcggcggcgcggccggcgcttcgtgtgaaagcagtcatttttgtgagggggtgcgtgggaataaaacggaactcatcggccagccgtgccgcggcgccggcgttgccggcagcgtgggaacagccgccataaaaaggggtgggcggctgcgcaatgcgcggcacgcccgggtatcaaatcttctttgccgcagagcggcgaatggcctcgttgatttcggcaatcgagcgctcgatggcgtcttcgtccatgtcctcgatctcgccgtcggagggcatgccggcctggatggtggacgcaaaaacgccgtcgtcgatggtctcggtggaaacgccgcggtcttcgcgcgtcgaatcgggcatttcccattcgagcgcgatgagcgtcacgttgtcgctgtgggcgccgcccttgcgaagcgccatttcggcaaggtcgggcgccgcatcggacaccggcttgtcggaagacagggtgtgcacgatgacggcatcgtcgagcacgccccacacgccgtccgagcacagcatgatgcggtcgccgcgctgcaattgcagcggggccgaaatatcgaacagcggcgtggtcggcgaacccaggcaggtgagcagcagattgcggttgaccggcatgtccgaaccttgcgggcgcgggcgctcggcgtgcgaatggtcgcgcgtgcgggtcagcaggcggccgtcgcgcaccacgtaaaggcgcgagtcgccgcaatgcatccaggtggccgtggtgccctgcagcagggccgcaacgacggtggtgcgcggcgtgtcgagcatggccttgtggcttgcgtaccgcatgatctgctggtgcgcggccatggccgattcggccaggaaggccttggcgtccttgacggtggggcgcgcttcgcgctggtagagcgccgcaatggtctgcaatgccagctgggccgcaacctcgccctcggggtggccgcccatgccgtcggccagcacgaaaaggcccgactcccgcgtgtagcagtagcccatgcggtcttcgttcttgagacggccgccctttcggctgacctggaataccgagaatttcatgccggacgcgtcgtaggtgccgccgccctgggcagggccttcttgtcgaaggagcggatgttgtcgaatgaaagccgcaccttttcgccaacggtgagcttggtgtagcgccgctcgccttcgcggctcagttctttttgcagcgcaaagaccgattgcggccgcgagagcgggtcgagcgacatgcaccactcgaccacttcgataaggttgtcggagtacacgccacgcagccgcgacagcgacaggctgagccggtctttctcgatgcggcgcggggcgtcgttgggcgggtagccctgcatgcaggcgtaaatgcaggcgccaatggcgtagatgtcggtccaggggcccatcgacgagtcgcgccggtacatctcgggggcggcaaagccgggggtgtacatcggccggatgaagatgccctctttgctgagcacctcgcgggcggcgccaaagtcgatcagcaccgcgcggtcttcgtcggtgacgaagatgttggcgggcttgatgtccaggtgcagcatcttgtactggtgcacgatgcgcaggccccgcagaatttcgtcgaaaagcgaccggatggtcgattcccggaaaaccttgggctttttcaggtcgcgcgcggtcaccacgaagtcctgcagggtcgcgccctccaggtagttcatgaccatgtagacggtctcgttctccctgaaaaagttgagaacgctgaccaccgaggcatgcgagatctgcgcgagcgagcggccttcctcgaaaaagctcttcaggccgagcctgtagagggagagcttttcgggcggaacctcgggcgtgagctcgcccggcccgcgcgtggcgagcgaagacggcaggtattccttgacggcaacctgctgtccgctggggtctatggcgagatagacaacgccaaaaccgcctgcggaaaggcgacgaacgatgcggtaaccgccaatgaccgtatcgggcagcaggggcgaaggcttgacctttgacataatccgggagtttcgcccgaaggcgatggtgcggcaagcgaacgccatgccgacgcctcggtgcatgcaagcaaaaaccacagtgaggcgcaatgccagtttacagcatgaccggctatgccagtggccagaacggccccgttggcagccactccgaagccgaagcacggcctaccgccgcgggacgactcggggtcgagatacgctcggtcaacagccgcttcctcgatctcaccttcaaattgccggaggaactgcgccagcatgaacccgcgctgcgcgagctgctcacgggcaaactcaagcgcggcaaggtcgaagtgcgggccgccatcgagaacaccgcccaggccggcgtcgtcgagccctccgtcaagctgctgcagcggctgaacggcgtgcaggacggcatcagggcctggctgcccggcgcccgcgaattgagcgtggccgacgtgctgcgccttgccggcggcgacagcgccgcccgtggcgactggggcagcgacctgctcgaggtgagcggcaaggcgctggacgccctgatgtccgcccgccagcgcgaaggcgcacggctcgccaagatgctggaggcccatctggcccaattgcgcacgctggtcgaacaggccggcccgctgattccccaactggtcgagcagcagcgcgcacgtttcctggagcgctggcaggaagccatgggcctgaccggcggcaccctgcccgaggcagcccaggaccgggcactgaacgaggccaccgcctttgccattcgtatcgacgtggcggaagagctcacgcgcctcaattcgcacctcgacgaaatcgagcggctgctcaaaaagggcggcgaaatcggcaagcggctggacttcctgatccaggaactgcaccgcgaggccaatacactgggctccaagtcggccgcgctggagctcacccgcattggcgtggacatgaaggtcctgatcgagcagatgcgcgaacaggtacagaacatcgaatgagcgagcgaatggactatccaggcaacatttttgtcgtcgcggcaccaagcggtgccggcaaatcgagcctggtcaaggcgctcatggagctggacacggccgtccagccctcggtttcccacaccacgcggccaccgcgcgggcaggaaaagcacggccgggagtacttttttacctcgccatccgaattcgacgccatgatcgccgccgacggcttcgtggagtgggcccacgtgcacggccaccggtacggcacctccaagaaggccatcgaggagcggatcgcccagggggccgacgtcatcctggagatcgacttccagggcgccatccagatccgcaagacctttgccaacgcggtcatgatcttcatcctgccgcccagctgggaagaattgcgctcgcggctggaacggcgcggcgaagacagcgccgccgtcatcgaactgcgcctcaagaatgccgcggaagaaatggcccgggcgggggaattcgacttcgttataatcaacgagttatttgagcgcgcgcttttcgatctcaaggcgatcgtccacgctcagcggcttcggtattctgcacagcgccgcgcacgtgccgacacattcgccgccctgaacatcccctgatttcctgctcaccccgaccgaaagattctcatcatggcccgcatcaccgtcgaagattgtctgcttcagatccccaaccgcttccagctggttctggccgccacgtaccgtgcgcgcatgctgagccaaggccacgcgcccaagatcgagagcaagaacaagccggccgtgaccgccctgcgcgaaatcgccgaaggcaagatcggcatcgaaatgctcaagaaggtgccgggctgatctgacgcacccctgcaacgaaaaggcaccgcaaagcggtgctttttttacgtctggacgcgtccatacagcggtcacgctaaagtggtagccatgagtgcggttgccaaacatcagtcccatgccccttcgggcacgccaaagccgagcccggcggcgctgaatgcggctgccgcaagctttgccgcactgacggcccggctcgactacctgagccccgaagacaccgagctggtccgccgcgcctaccgctttgccgacgaggcgcacctgggccagctgcgcaacagcggcgaaccgtacatcacccaccccatcgcggtggcggcgcaatgcgccgaatggaagctcgacgcccaggcgctgatggccgccctgctgcacgatgccatcgaggactgcggggttaccaagccggaactgatcgagcgctttggggccccggtggccgagctggtcgacgggctcaccaagctggacaagctgcagttcaatacccgcgaagaaaaccaggccgaatcgttccgcaagatgctgctggccatggcgcgcgacgtgcgcgtcattctggtcaagctggccgaccgcacgcacaacatgcgcacgctcgacgatgcgccgcgcgaaaaatgggcccgcatttcgcgcgaaacgctcgaaatctatgcgcccatcgcgcatcggctgggcctgaaccagacgtatcgcgagctgcaggagctgtcgttccgccacctgaagccctggcgctatgccaccctgtccaaggccgtggccagggcgcgggggcgccgccgcgatctgatccataaggtgcagcgcgaagtcgaaaccgcctttgccaacgccaacatgacgctgcgcatcgcgggacgcgaaaaaacgctctattcgatctaccgcaagatggaagaaaagcacctgagctttgcccaggtgaccgacatctacggctttcgcctgatcgtgccgaacgtgatcgcctgctacaccggccttggcatcctgcaccagatgtacaagccgctgccgggcaagttcaaggaccacatcgccatcgccaagctcaacggctaccagtcgctgcacaccacgctggtgggcccggccggcgtgaacgtggagtttcagctgcgcaccgaggccatgcacgtggtggccgaatccggcgttgcggcgcactggctctacaaggccgcggagccgaatgcggccagcaacgacaggctcggcaccaagtggctgcagtcgttgctcgacatccaggacgaaacgcgcgatgccgccgagttctgggaccacgtcaaggtcgacctctttccggatgcggtgtacgtgttcacgcccaagagccagatcctggccctgccgcgcggcgccacggtggtcgactttgcctacgccatccacagcaacatcggcgaccacacctcggccgcccgcatcaacggcgaccaggtgccgctgcgtaccgagctcaagaacggcgacgtggtcgaggtgattaccgcccccgtatcgacgcccaatccggcctggctcggcttcgtgcgaaccggccgcgcgcgctccaagatccgccactacctgaagaccctggcccatgcggaatccgaaggcctcggcgaaaagctgctggcgcaggcgctgcgcgccgaaggcctcagcaagctgccggccgacgacgccgaacaccaggcactatgggaaaagctgctgcgcttcacgggcaaccgtacccgcgccgaactgctgaccgacatcggcctgggcaagcggattgccagcatcgtggcaaagcgcctggtggccatgctctcagaactgggcgagcggccggatgcgctgctgctgagccgcgaacgcttcatttcgcacgaaaccatctcgcagggggccgtcacgctggacggcagcgagaactcgtcggtccgctttgcgctgtgctgccggcccattccgggcgacgagatcgtcggctatctcgggcatggcgaaggccttgtggtgcacaccgaaagctgcggcgtcggccagcgcctgcgccacaaggacagcgagcgcttcttcgcggtcgaatgggcggacgagcccacccgcgccttcgagaccggcgtggtcatcaccgtgcgcaacgacaagggcgtgctggcccgcgtggccgccaccctggcggacgccgaagccgacatcacgcacgtcgagatggcggacgaaaccccgcaggattcgaccgatctgcgcttcgtgattgccgtgcgcgaccggactcacctggacgccgtcttgcgcgcggcgcggcggaccgcctcggtgctgaccgccgcgcgcacggttcctgcggcctgaaaaaaccgcagcgttgaatggcaacgctacgccggaccgggagccgggtagctgaccgacagcaattcgacctcgtgcgcgccgccgggcgtaacgagcttcaccacgtcgccctcgcgtgacttgagcaacgcccgtgcgatcggggaaatccagctgacctgcgccttggcgctgtcggcttcatcgatgcccaggatcgtcacgctgcgttcgtcgccggtctcgtcgacatagcgcaccgtggcgccaaagaagacttggtcgctgccgtggtgcaccgagggatcggtgacctccgcgatctcgagccgcttggtgagaaagcgaatgcgcctgtcgatttccctgaggcgcttcttgccgtagagatagtcgccgttctccgagcggtcgccgttcttggcggcccaatgcacggcttccaccaccttggggcgctcttcgtccatcaactggagcagttcgtcgcgcagccgggcatagccggccggcgtcatgtagttcttactgccgctgggcagtgcgggggcggtgctgtcgccatcatcgtcgtcgccgccagcgtcggtttccttggtgaacgctttgctcacgatagaagctccaaatccattttcctcaacccaggtccgagcgcttgcagtcgaagaccacgctttgctcgaccgctcgcaggacaggcaccttgttcgcaaaagcgacgcccgcgctgacaaggcgccactcgttcgccttgaacagcttgaaaagatgcgtgacctcggtcccgaccgtgggaatggagttgaaaacatagacgggctccccggactggctctcatccatgctcacaagatcggccctcatcttgcccatggtttccgtgtctttcgttcgggaacgcacgacgtcgaggttgacggtgcgggagtgctcgtcgattgaaatccggcgcacccagttgaaaggcgatgcgggcccattgcttgcgccggggacgcaggtgatggttcctgccgatgccgcgcctgctgctgaagacagcatgagaaattggagtgcaagccgctttgccgaaatgctcatgatgcgttgcgcgttgtatgactgggctgaactttagccccaggcgcatgagcgtgctttctcttcgcgccgtgaccacggctgcactggctgcgatcgcccaaaagaaaatggcctggaagatctaaatcttccaggccattcaagagagtggtgcggctggcaggaattgaacccacgaccccttggttcgtagccaagtactctatccaactgagctacagccgcacagctatcgattatagcatccatttttgcccccggcgagccaggtcagaaaatgaatgccaagtggtaggccgtgatgggcttgaaccatcgaccaacggattatgagtccgctgctctaaccaactgagctaacggcccacgagaggccacgattctattcgcggcgctgcctacttgcggtggctcagcgcattgctgaccagccgggaggtgatgtcgacgatctggatcatgcgctcgtagggcattcgcgtcggcccgatgacgcccagggtgcccaccacctgtccgtcgacttcatagttggcgctgacgatggaaagctcctcgaacggcaccacctggctctcgccgccgatgaaaattcgcacgccttcggccttgctcgacacgtcgagcagccgcatcagttgcgccttttgctcgaacagctcgaacgcacggcgcaaatgactcatgtcgctagaaaaatcggtcacggagagcaggttgcgctcgccggaaatcacgacgtcgtcttcttgcgcctcggtgagcacctcggagctgacattcactgccgcctgcatgagcgctgcaatctcgccacgcagtttttcgacttcggactggagccggtcgcgcacctgctcgatggtcaagcccgcgtagtgggcattgatgtagttcgatgcctccaccaactgcgactgcgaataatcggcctccggaaagatcacccggttctgcacgtcgccgtcgggcgagacgatgatcaccagcagccgccggtccgaaagtttcaggaattcgatctgcttgaacaccgaggcgcgccgcggcgccatgacgacgccgacgaactgcgacaggttggacagcaggttggccgcgttggcaatcaccttctgcggctggtcgggcgcaaggctcggcgcgctcatctgctcgcgctgcgccgtgagcatggtgtcgacgaaaagccgatagccgcgagcagtgggaatacgtccggccgaggtgtgcgggctggcaatcagccccagcgactcgaggtccgacatcacgttgcggatggtcgcgggggacaggtccaacccgggcgcgcgcgacaaagtccgcgacccgaccggctggccttcggcgatgtaacgctcgaccagcgtcttgaggagcaacttggcacggtcgtccagcattgcaagattttagtgttgtaatttgtagatgacttcccgctttcgtcacgtcgcgctgatcggcaaataccaggcttcaggcgcccgggcgcaggcagacgcgcgcgacggcgtcatggaagacatcggcacgttcctggaatcgcaagggtgcgaggtgttcgtagaaaagtccgcggccgacgaagccgatgcggacgcgaacgtcggcggccgctacgaaccgctgagcgtcgaggaaatcggccagcgctgcgatctgggcctggtggtggggggcgacggcaccatgctgggcatcggccggcagctggcgtgctacggcattccgctgatcggcatcaaccgcgggcggctcggtttcatcaccgacattccgctcgacaactaccaggccacgctgatcccgatgctggccggcgagtacgaggaagaccaccgcagcctcatgcatgcgcaggtcatgcgcgacggcgcctcggttttcgatgcgctggcaatgaacgacgtggtggtcaaccgcggcgccacctcgggcatggtcgagctgcgggtttcggtcggccggcatttcgtggccaaccagcgcgccgacggcctgatcatcgcgacgccgacgggctcgacagcctatgcgctgtcggccggcgggccgctgctgcaccccgcggtgccgggctgggtgctggtgcccattgcaccgcacacgctctcgaaccgcccggtgctgctgcccgatgccgacgagatcgtgatcgaactggtggccgggcgcgacgccagcgccaatttcgacatgcagtcgctggcgtcgctcgccatcggcgaccgcgtggtggtgcgccgctccgacttccgggtgcgctttctgcatccgcgcggatggagctatttcgacacgctgcgcaagaaacttcattggaacgaagggggctcctgagatggcgctgcgacgcatcgcactgcgcgacttcgtgatcgtgcgatcactcgaactcgatctatcctctggcttcacggtgctgaccggcgaaaccggcgcgggcaaatccatactgatcgatgcgcttcaactggcgctcggcaaccgcgccgacgcgggcgcagtgcgcgagggcgccgagcggctcgatgtcagcgccgagttcgacgccgatccggcctttgcagcctggctcgacgaaggcggattcgaatccggcgacgccctgctgctgcgccgcaccgtcgacctgcaaggacgcagccgcggctggatcaacgggagcccggccacggccacgcagctgcgggaacttggcgaccgcctgctcgacatccacggccagcatgcctggcagagcctcacgcgtcccgaggccgtgcgcggcctgctcgacgcctatgccggggtgcgcagcgatgcgctggacgcggcttggcaggcatggcgacaagccctctccgcgctcgaccacgcacgctcggcgcaagattcgctgcaacgcgagcgcgaacggctgcaatggcagattgccgaggtgatgaagctggcccccgccgagggcgagtgggaagaactctcgaccaaccatgcgcgcgtctccaacgcgcaggcgctgatcgacgcggcacagggcgccagccaggcgctggaagacgacgacaacggtgccctcgcagcgctgtcgcgcgccgtcaccctgctgcagaactgcgagcacatcgagcctgaattccgcgcccttggcgaggtgctggcctccagcgtggcgcaggcctccgacgccgcgcattcgctgcacgggtacctgcgcgacgccgaagccgatccgcagcgcctggcggaactggacgagcgcatggggctctggatgtcgctggcgcgccgctacaagcgcacgccgggcgacctgccggcgctgctggccggctggcaggccgagctgaaggcgctcgatgcgcaaagcgacctcgaaggcctggagcgcgccgagcaaagcgccgggcaggcctacatgaaggaagccaaggcgctcgccaaatcgcgcaagcaagcggcaccgcgcctggccgaggcggtcacgcgggccatgcaggggcttggcatgcaaggcggccgtttcgaagtcgaactgcagccgctggcacagccgggccgcgctgggctcgaagacgtcgcctttctcgtgagcggccatcccggcagcacgccccgccccatcggcaaggtggcttcaggcggcgagctctcccgcattgccctggccattgcggtgaccacgagccagcttggcgccgcgcagacgctgatcttcgacgaggtcgatgccggcgtcggcggggccgtggccgagaccgtggggcgcctcatgaaacagctcggccgcgaccgccaggtcttggccgtgacccatctgccgcaagtggccgcctgcgccgatcaccacctggtggtggccaagcgccagacggctgcggcgggccaggacggcccgcgcaccgaaagcggcgtttcgcggctcgacgacgacaaccgcgcccgcgagatcgcccgcatgctcggcggcgagaagctttcgcagacttcgctggcgcatgcccgcgaaatgctgggccacaagacttcggcggcgatgtgatggacctcgacctggtgctcatcacgggcatgtccggctcgggcaagtcggtggcgctgcatgcgctggaagacgccggctactactgcgtcgacaacctgccgcccgagttgctgacgcctttcatcgcgctgcagcacgaacagcaggccacgcgcgtcgccattgcgatggacgtgcgcagcggcgtgtcgctgccgatcgtgccgcagcagctcgacgccttgcggaacgacggcgtctcgctgcgatcgctttttctggacgcgaccaccgacgcgttgctgcggcgctattcggagacccgccggcgccatccgctgtcgcgcctcgagggacgcaccgacgctcccgagcaggagcgcgcgctggttcaggccatcgagctcgagcgcgagctgctggccgatttgcgcgacggcgccgacgtgatcgacaccagcctcatccgaccggcccaactgcagagctacatcaaggccctgatctcggcaccgccgagcgcattgacgctggtgttcgagtcgttcgccttcaagcgcggcgtgccgctggacgccgacttcgtattcgacgtgcgcatgctgcccaacccgcactacgtgcccgcattgcgcccgctcacgggccgcgatgcgccggtggtcgaatggctgcgcgagcacgaggacgtggcgcgcatgtacgacgacatcgagcaatttctttcgcgctggctcgatgcgctggcgcgagaccatcgcagctacgtgacggtggccatcggctgcacgggcggccagcaccgctcggtgttcctggtcgagcaattggcgcgtgctttcggaacccgttggggtgccctcaagcggcaccgcgaactcgacgcgacttaagctcgcccccagtcttcgcgcacttcgtgtcgctacgcctaccccctaccgggcgcaacaccagaggcccggcaaagccggttcctcagtgttccacgaaggagccaggacgctagcttgcgctgctctctagaagcagcttgcgcacgggcgccggcaatcccaggcgggcccactcttgcgcacccacccagcgcgcggcatcgccctgcggctggccgctgctgcgaagcagcaccgggtgaaggtgcaggtccttgtgggtcagcacgtgcacgaagggcgacaggtcttgcgtgtggcgctgctcggcgggcggcagcgcggccaacagctcttcgcgggtgtcgaacaccggcaggcaatagagccccgcccagatgccctttgcggggcgcttctccagccatacacggccttctgcatcgcgcgccaacaaggcccagagtgactgggcgctgcgcttcaatttgcgggtcttgacgggatagcgctccggctgcccttctcgcaaccccacgcaggtattggtcaacgggcagatcatgcagctcggcttgcgcggcaggcagaccgtcgcgcccaggtccatcaccccttgcgtatagcttgcgatggcctctttctgttcggccggcggaagcagttgcgtagcctggtcccacagcgcgcgttcctgcgccgacgaagacatgtcgccgccaaagccgagcacgcgcgtcagcacgcgtttcacgttgccgtcgagaatcgcgacccgctcgccaaagcagaaggccgcgatggctgcggcggtggagcggccgatgccgggcaaagtcgtgagctcggcggccgtgcgcggaaattcgccgccgaagcgggccaccacctcttgcgcgcagcggtgcatgttgcgcgcgcggctgtaatagcccagcccgctccagaggccgaacacttcgtcctcggtgccctcggccagggccgacacggtcggaaagcgttcgagaaagcgcgcgaagtatcccagcacagtcgatacctgggtctgctggagcatgacctccgacagccagacccggtagggatcccgcgtgttctgccacggcaactcgctgcggccgtggctgcgttgccagtcgacgatgcgctgggcgaaagccgtgggcacctgcagttccgtggccgcggtggacaccggacgatcaggccgcacgcagttcgccgatggcggcggccgcggcggccggccttccctgttgcgtgatcatcgaagtgaattcctgcagccggacatgcaactcggccaggctgctctcctgcgtggacagctcgagcaggcgctcgtcgaggttgccggccgcactctggatgcgctcgatcgcctcgatgcgcttggtgaagttgcggcggcgctccttcagctgtgcgtcgatctgcgcgctggcgcctttgctccagcgctcgacctcggtcattgcggcttcgttgaccagccgcagccggcttgcgagcgcacgcaccagcttgtcgcaaaaatccgcctgcgccagcttcagcagattgccgacgcccaggtagtgaatgtggctgcgctcgatctggctcagctcctgctcgaagctggtcaggtccggctcggcgggcgcctgcaagttgaagccttgctccgcgttgagctggcggaaggtggcgtgcagcatcgactggatctcggccgtggtcgcctgcacttcgcgcaggttgttgcgcagcgagtcgaaggtttcgccgtacaccttgcgcacgttgaacttgatgcccgggcgcttgagcgcgctcgaaagccgcaccatgtcggccttgagcgcggtgcggccgagcacggcgtacacctcgcgcagcagcttgccctgcaccgagcgcagggccaggatgcgcgtgttgctgccctcgaactccgtctgctcctggtcgatgcgcccacgcatgtggcggatgaccgagatattcttgccgcgcaggccctgcagttccagcgcctgctccgacagatcgcgctggcgcaccttgaggatgcgctcggcctcgacccgcagcgccaccatgcctgcatccacggcaagccgcagcatggtttcgcgcttgcccagcacgccttcggcgagcagcatttcgagtgcaggcaggcggctggcatcgagcagccgcgggtcgcgctggatctttgcctgcaagcccttttgcgccgacaccggcagcacctgcacgagcggaacctcgagaaacttggccgccacttcacgctgccgctcgatctgcatctcgatctgcgcgggcgtgctgagcgagtcccacatggtgtcgatcttgttgagcaccacgaagcgcgtgtcgctgccttcgctttcggtgaccaggtgctcgcgccagatggacaggtcggagcgggtcaccccggtttccgcgcccaggatgaagacgaccgcatgggcctgcgggatcaggctcaccgtgagttcgggttcggcgccgatcgcgttcaggcccggggtgtcgaggatcaccagcccctgctccagcaagggatgcggcatgttcagaatggcatggcgccagcgcggaatctcgacccggccttcggcgtcctgcaccgggttgtcgtccggcgtctcttcgttccagaagcccagcgcgtgcgcctcgtccttgctgacccagcgcacctcggccaccttgcccatggccagggccagttgctcggcgttctccacgtcgatcgcgatttcggtccagcgcgtgggcttttcgcgccagtgcgtgagcgaatgaggctccaggcgcgtttcgatcggcagcagccgcagcttgggggcctgcgcggcgtcatagcccagttcggtcgggcacatcgtcgtgcgccccgcgctggccggcatgatgcgccgcccatagcccgcgaagaagatcgcgttgatcagctccgacttgccgcgcgagaactcggccacgaaggcgaccatgaccttgctgttgcggatctgcagctccaggccgcgcaagcgctcggccacggcctggtcgagcagctcgttttcggtcagccagcgggtcagccactgcaggcgatgcgcaaaattgcttcgccaggcaccgtgctgatcgagttgttgattgaaagagcggctcaaagggaatatgtaagaaacaacttacaaatatagcattgcaagctgtggagcaaccgtttgcaggatattcgaacgcgggcgccgaaacactatttttgacaatttgggcaatagtaagtcgaacgctggccttggcgcagttgccgaatcggcgttgcgcagacccgacaaggctcgcccgcgcggccgtagaccgtcgcttcgagctgaaagtagccgttctgcccgtccacattggagaagtcgcgcagcgtgctgccgcccttctccaccgccctggcgaggatttcgcgcaccgccgcatggagcttggccgcccgcggccggctgatgcgcgcggccgaaagcgtcggccggatgcccgcctggaacagcgcctcggaggcgtagatgttgccgacgcccaccaccacgtcgcccgcgagcagcacctgcttcaccgcggtccggcgcttgcgaaggccggcatggaacgcatccaggtcgaactcgtcgcccagcggctccatgccgaggccgccgagcagcttgatggcccagggcgccgcctcgtcctccacgtagaccacggcgccaaagcggcgcggatcgttgagccgcagcgtgccgcggtcggtgaccaggtcgaagtggtcgtgagcgccaggcgcgggaagcgccgcatcgaagcgcaggctgcccgacatgcccaggtgcagcagcagcagcccgcggtccaggtcgatcagcaggtacttgccgcgccggcgcacttgcagcacccggcgtccggccagcgcttcgggtgcgaccatcagcgcccaccgcaggggcttgccgatgcgggctgcatcgatgcgtgcaccggcgatgcgttcggcaaaaccgcgccgcgtcacttcgacttcgggaagctcaggcatgaaattgaaatctccgggctgcgacgaggccccacgcgatgctcgctcaaaagcttggattattatggttcgatgattccatcgctccgccgacaccgccttgcggcggccgcgtcactcgtcttgctggcttgcgccgttcaagcgcaaacctccgaccccgccgcgcccaagagtccggcccccatcatcgagcggccgacgccatctcggccgggagcaaggcctgccccggcacccgcggcaaagccagccgacgtgaagtccaccagcagcgaagccgccgcacaaccctcggccctgactgcgcaactgttctacgagatcctgatgggcgagctgaccacgcgctccggagatcccggatcgggctatgcgctggtgctcgacgcggcccggcggctgcgcgacggcaagctgttccagcgcgcggtcgaaatcgccctgcaatcgcgctccggtgacgcagcgctggcggcctcccgcgcatggcaggaaacgctgcccaattcgcgcgatgcacgccgcatcgaactgcagatcctgattgcgctcaaccgcatcagtgaaaccgtcgcgccgctgcgcgccgagatcgcggccacgccgcagatcgagcggccgatgctgatggcggtaatcgcccgcaattactcgcgcgcctctgacaagaagctggccgcgtcggtggtcgagcaggcactggtcgacgagctcaagagccccaccaccggtggccttgcctgggcaacggtcggccgcctgcgcctgaatgccggcgacacctccggcgcactggacgccgcgttcaagggccagcagctcgaccccgcctccgacgccccggccgcactggcgctcgagatgatcgaccccggccagccgctcgcagaaccgatcgtcacgcgctatctggccagcaaccccaaggcggcgcccgacctgcgcattgcctacgcccgcgtgctggtcgaaaaccgccgctacaccgattccgccgcgcaattgcaggcgctcaccacggcccggcccgaattggccgagccctggctgctgctcggcagcctccaggcccaggcccggcaggacgcggcggccgaaacgtcgctcaagcgctatgtcgatctggcggccagccagaaagatgcggaagatcgccagcgcggcaccacgcaggcctacctcgttctgtcgcagctggcggaacgccgcaaggacttcacggccgcggaacgatggcttgcacgcgtcgacagcaccgacgaactggttgttgcgcagacgcgccgcgcgggcctgctggcgcgccagggcaagctgcctcaggcacgcgaactcgtgcgcggcctgcccgagcgcacggcagaagacaagaagcagaaattcctcgccgaagtgcagctgctgcgcgacgccaagcaataccaggccgcctacgacatgctggcccaggcgtccgccgctgctcccaacgacagcgacctggtgtacgaccaggccatggtggccgaaaagctgaatcgcctggacgaaatggagcggctgctgcgccggctgatcgagctcaagcccgagaaccagaacgcctacaacgcgctcggctactccttcgccgatcgcaagatccggctcgacgaagcgcgcacgctgatccagaaagccgtgcagctggcacctgaagaccccttcattgccgacagcctgggctgggtggaattccggctgggcaacacgaccgaagccattcgcatcctcgaagcggcctacaagtcccggcccgatccggaaatcggcgcgcattttggcgaagtgctctgggccaccggccagaaggaccgcgcggtcgtcatctggaaggaagccctgctgagcgacgccgaaaacgagacgctgcaggagacgctcaagcgcttgcgggtcaagccgtgacggccatgctttctcccgggcttgatggtggccgccggagcgtgctcgcggcgggcgttgcggcaatgctgctcgcggccggctgcgcgcagctcccgagcgccacgcggccccagggcacggacgcatggagcggccgcatgtcgctgcgcatcgacagccagcctgtgcaaaccttttccgccctgttcgagctgcgtgggtcgcccgagtcgggcgaactctcgctcacgagcccgatcggcagcacgctggcccagttgcactggtcgccgggcgaagccctgctcaagaatggcagcgagatccggcgctacgaatcggtcgatgcactgatcgaagcggccaccggcgccgcgatccccgtgggtgcgcttttcggctggcttgcgggccgcgacgaccgcgtgcccggttggcgcccggacctggggcagatcgccaacggccgcttgcaggctacgcgcgaagcccccagccccacggcagacctgcgcatcgtgttcgaacggtcatgaaggcgatctacgaccttcccgcaccggccaagctcaacctcttcctgcacatcaccggccggcgcgaagacggctaccacctgctgcagtcggtcttcatgctgatcgactggtgcgacacgctccacgtcgagttgcgccacgacggccagttgagccgcgaagacctgacgaccgaactgccgcccgacgaccttgtccttcgcgcggcgcgcgcgctccaggcgcatgccgcgcccggccagggcgcccacatcggcattgccaagcaggtgccggcgcaggccggcatgggcgggggttcttcggacgccgcaacctgcctgctggccctgaaccggctgtggaagctgaacctgccgctgacccgcctggccgaaatcggcgtgaaactgggcgccgacgtgccgtttttcctcggcgggcgcaacgcgtgggtcgagggaatcggcgaaaaaatcagccccgtgaacgtccctccggcacggttcgtggtggtcaagccacccgagggactcgacacccggctaattttttctgcgccggaccttcaacgcgccactcctgttgctataatctcgggctttgctgcagatagcgaacagcttgaagcccaagaccccgaaagcagcgctttcaaggttttcgacttcggccacaacgacctgcagccggttgcccagcggctttgccccgcggtctccgacgccatcgaatggctcggcgcccaaggactgaaagcccggatgaccggctccggaagttcggtattcgcgaaaatgccgcaagggccgcaaaaagcggaactggccgaagccccaacgggctggcaggttcgtcaatgcagcaatttggccgttcatccactttggggatgggcgacctgaagatgatcggactgttaaggtccgatgcgacatatatcggtttgtggtgaaaaccatcgacccgtgtaggggagtcgccaagctggttaaggcactggattttgattccagcatgcaaaggttcgaatcctttctcccctgccaaatttcttcaggctgcggtttaaccgccgcagcgcttcaaactgcggcccaccggccgcagtgcttcttttgcagcccacccgctgcaataattggcggcccctgggtcgccacgactcaaactctttggcggcttcctaaaagccaattcgcactgccgggacgcgctcatgcaggctaatcaccctgatttcatggttttcaccggtaacgccaatcctggcctggccgcggaaatcgcgcacaacctcggcacctcgctgggcgccgcacgcgtgggtcgcttctccgacggcgaagtcaccgtcgagatcaaccagaacgtccgggcgcgcgatgtgttcgtggtgcagtcgacctgcgcaccgaccaacgagaacctgatggaactgctgatcatggtcgacgcgctcaagcgcgcttcggccgagcggatcagcgcagtgattccctattacggctacgcccgccaggaccgccgcccgcgctcgagccgcgtgccgatctcggccaaggtggtggccaacctgcttgaaaccgtgggcgtcgagcgcgtgctcaccatggaccttcacgccgaccagatccagggcttcttcgacattccggtcgacaacatctatgcgtcgccggttctgctgggcgacctgcgccagaagaactacgaagacctgatcgtggtctcgcccgacgtgggcggcgtggtgcgcgcgcgcgcactggccaagcagctgaactgcgacctcgccatcatcgacaagcgccgtccgaaggccaacgtgagcgaggtcatgaacgtgatcggcgagatcgacggccgcaactgcgtgatcatggacgacatgatcgacaccgccggcacgctggtcaaagcggccgaggtgctcaaggagcgcggcgccaagagcgtctacgcctattgcacgcacccgatcttctcgggccctgccatcgagcgcatcacccactccgcgctcgacgaagtggtcgtgaccaacaccattcccctttccgacggcgccctggcgtgcggaaaggtccgccagctctccgtggcaccgctgatcgccgaaacgatccagcgcattgccaagggcgagtcggtgatgagtttgttctcggaccaggacaacctgttctgaccgagcaaaaagcgggcgccaccttcctttttcaggaacggcgtccttgttgaaccggagtcgcactggtcgcggtggactctcacaggagttgttatgaaattcgtcgcttttgagcgcgcaaagcagggcacgggtgcgagccgccgtctccgcatctcgggcaagacgcccggtatcgtctacggtggtgaaggccagccccagctgatcgagctcgatcacaacgcgctgtggcacgccctcaagaaggaagccttccactcgtcgatcctcgaaatggaactcggcagcgccaccagcaaagtgctgctgcgcgacgtgcagtaccacccgttccgccagctggtgcaacacatcgacttccagcgcgtcgatgccaagacccgcctgcacatgaaggtgccgctccacttcaagggtgaagaagagtccgatgccgtcaagctcgaccacaacctcgtgaaccacgtgatgaccgagctcgagatcagctgcctgccggccgacctgcccgagttcatcgagatcgatctctccggcctcaagaagaacgccacgctgcacgtcaacgacatcaagctgcccaagggcgtgaagttcgtgagccacggcaagctgaacccggtcgtcgtgtcggccgtgccgccgctggtcgccgaagagccggcagctgccgctgaaggcgctgcagctcccgaaggcgccgcaccggctgccaacggcaagcctgccgccaagacggcaaagcccgccgcgaagaagtaatttccttcgcgtccctgcaaaaggcccgcctcgtgcgggccttttgctttggggccggcgagataattcccctcatgatcaagctgtttgtcggcctcggtaacccgggtcctgaatacgaagccacccggcacaacgccggcttctggtggatcgacgccctggcgcgcgactggaaactcaacctcgcgcctgagcgcagctatcacggcctcgcggcgcgcgcgaacatcaatgggcaaagcgtctggctcctggagccgcagaccttcatgaacctgtcgggcaaatcggtgggcgcgctcgcgcgattcttcaagattgcgcccgaagaaatcctcgtggtgcacgacgagctcgacgtggtgcccggccaggccaagctcaagttcggcggcagccatgccggccacaacggactgcgcgacatccacgcgcagctgggcactggcgactactggcgcctgcgcctgggcatcggccatcccggcgtgaagtcggaggtcatcaactgggtgctcaagaagccgctgaaggagcagcgcgacgccatcgaagacgccatcgcgcgcaccctgcacgcggcacccgcactggtggcgggcgagatggaaaaagccaccctgatcattcacacgagcaaaccgccccggcccaaaccgccgcggcgagagcccggcgatggaggcgcgcccgccgccccctagtcagccggcccagagcgcgggagagcgagagaaaaagggagagaaaaagaaatgaaaagaaaatcgatcgccggaaaaacggccattgctatctttttggtagcttccggtgctttctgcctgtccgccacggcgcaaggaagggccgaagcctaccgctgcggcaacacctacaccgaccgcccctgcgagggcggaaggcccgtaaaagtcgacgacgtgcgtaccgatgcggaccgccgtgcctcggaggctggcacgcaaagggcggaggcgcgcgccgaccagttggagcgcatcagactgtcggaggaaaaagaagcctacgagcgcagccgaaggtcggcccacgaggcacggcaagccgccatcaacgaacgccggctcgcgtcttccgagcagctggcgcgggcacgggcgcagaaactcagcgccgaaccgcacaagtcgagcgcgcgcttcagcggctcggcgggcggcacgcaggcatctgcccctggcgagggcagcaagaagaaaaagcgaaagccctcgtccgactcaagcgccggttgagggcgcctcggtccgcggctgcggctccgatgcaacggcagcggcggccttggccgcggcgagccgctcgaacttctgccacagcgtctcgcggctttccacgtgctcgggatggatcggaatgcacgcgaccgggcacacctgcacgcactgcggctcgtcgaagtggccgacgcattcggtgcacttgtgcgggtcgatctcgtagaactccgcgcccatgtagattgcatcgttcgggcactcgggctcgcagacatcgcaattgatgcattcgtcggtgatcatgagggccatacccgattatcgcgaacaaggcacgcttgttgcacgagtcgggttatgctgcgccccgccccatgagcctgttcatcctcaagcgcctcgccacgctgatcggtacgctgatcggcgcctcggtcatagtcttcctcgtcctggagatcctgccggggaacgccgcgcagatgctgatgggccccgatgccgcacccgaggccgtggccgccctcgccaccaagctcggcctcgaccagcccgcctggacgcgctactggcactggattgccgggctcctgacgggcaacctgggcgacagctacgcctacagctcgccggtgctcgacctgatcctggaacgcctcgcgcttaccgttcctctggccatgctggcgatggccctcaccgtcgtgattgcgctgctggtgggcgtgaccgccgccgcgcgccacaacaagctcggcgacgtcggcctgatgagcatggcccaggtcggcatcgccattcccaatttctggttcgccatcctgctgatcctggtgttctcggttcagctgcaatggttctcggccggcggcttcgagggttggagcgagggcatcttctcgggcatcaagtcgctgctgctgccggccctgtcgctggcggtggtgcaggccgcgatcctcgcgcgcatcacgcgctcggcggtgctcgaggtgatgcgcgaagacttcgtgcgcaccgcgcgcgccaagggcgtttcgcagcgcgccgtgctctggacccacgtgctgcgcaacgcgatgatccccgtcatcacggtcatgggcatgcagttttccgaactgctggccggcaccatcgtggtggagaacgtgttctacctgccgggcctgggccggctgatcttccaggccatcagcaaccgcgacctgatcgtggtgcgcaactgcgtgatgctgctcgcggcaatggtggttatcgtgaacttcgtggtcgacgtgctttatgccgtgatcgatccgcgcatcaaggcgagcgatatatgagcgccgtgccgggccgccccaagcaagctcgctcccgcctggcgggaaggcgcgcagcgccaagggtgcatcaatgagcgccgtacccgttcccagcgcagcggcgctcacggtgccgggcttctggcggcgcgcgctccggcaccgcagcttcgtgctcggcggcgtgctgacgctgctccttttgctggctgccaccgtctcgctggcgtggacgccctggtcgccctatgagatggacatggccagcaagctgaagccgccgtcgggctcgcactggctgggcaccgacacctacgggcgcgacgtggcttcgctgctgctggtgggcgcgcgggcttccatcctggtgggcgtgatcgcggtcggcatcggcctcgtcgtgggcacggcgctgggcctgctcgccgcggcgcggcgcggctgggtcgaggaagcgatcatgcggctcaccgatttctcgctcgccttcccggccatcctgtcggccatcatgatgacggccgtgttcggcgccggcatcgtcaacgcgatcatcgccatcggcatctacaacatcccgacttttgcgcgcatcacacgggcctcggccaatgccatctggtcgcgcgaatacgtggcggccgcgcgcgcctgcggcaagggttcgttcgccatcacgatgcagcacgtgctgcccaacatctcggccgtgctgatcgtgcagatcacgatccgcttcgcgattgccatcctcgccgaggccgccctctcctacctcggcctgggcacgcagccgccgcagccctcgtggggccgcatgctcagcgaggcgcagaccatgatgttccagtcgcccctgctcgcggtgttccccggcatggcgatcgccatggcggtgctgggcctcaacctgctcggcgacgggctgcgcgatctgctcgacccgcgccttgcgcgcgcccgctaagcgatatgcctcttctcgaagtcaaggacctgcacgtcgaactgcaaacgcagcgcggccccgccgaggccgtgcgcggcatcggcttcacgctcgagcgcggcgaaacgctgggcatcgtcggcgaatcgggctgcggcaagtcgatcacagtgcagtcgctgatgggcctgctgccttccaccgccaaggtcaccggcagcatccgcttcgacgacaccgaactcgtcggccgggacgaaaaagccatgtgccagatccgcggcaaccgcatcggcatgatcttccaggagccgatgacggcgctgaacccggttcacaccatcgcacgccaggtcggcgagccgctgcggctgcaccgcggactcaccggcgccgaagcgcgcaaggaagtgctggcgctgcttgagcgcgtgggccttcccgatgcggcgtcgcggctcgatgcctacccgcaccagttttcgggcggccagcgccagcgcatcggcattgcgatggccctggcctgcggccccgacctgctgattgccgacgaacccaccaccgcgctcgacgtcaccatccagaagcagatcctcgagctcatccagggcctcgtggccgagcgcggcatggcgctgatcctgatctcgcacgacctcggcgtcattgcccagaccgtctcgaaaatgctggtgatgtacggcggcagcgtggtcgagagcggcccgaccgaaaccgtgtttgccgagcgcgcgcatccctacacgcagggcctgttcgcagcgcggccggcgctcggtgcgccgcgcggagttcgcctggccaccatccgcggcagcgtgcccgagctggtcgatctgcctccgggctgcccttttgccggccgctgcaagtacacggtcgatgcctgtcacacgacccggccaccgcccacgatattgcggcacgaccacgccgtgcgctgcatccggctcgaggaaattgccgcggaaggcgccctcgcaacatgagcccccgctcggccgctccgaagggggctcgcaccgcagtgcgaagcacagaggttactcaatgacccagcccaccggcaaccaacccctgctcgaggtgacggacctcgttcgccactacgcactgccgcgcgaaaaactcttcggcccgccgccgaccgtgaaggcgctcaacggcgtcagcttcaaggttgcggccggccgcagcctgggcatcgtcggcgaatcgggctcgggcaagtcgaccatcgctcgcctggtgatggcgctcgacacccccacgtcgggcagcgtgcgcatgctgggccgcgacctgcaccagctgccccgcagcgaactccgggtggcgcggcgcgatttccagatggtgttccaggacccttacggctcgctcgatccgcgccagaccgtggcgcgcatcgtggccgagccgctcgaggcgctggccgaaaccagccgcgccgtgcagcgcgagcgcgcctcggaagccctggccgcggtgggcctgcgcaccaccgacatggacaaatacccgcacgagttctccggcgggcagcgccaacggattgcaattgcgcgcgcgctcatcacgcgccccaagctcatcgtggccgacgaacccgtcagcgcgctcgacgtgtccgtgcaagcgcaggtgctcaacctcatgcaggacctgcagcagcagttcggcatcagctacctgctcatcagccatgacctcgcggtggtgaaccacctgtgcgacgaagtgtgcgtggtgtggaagggcaagatcgtcgaacagggcccgcccggcgagctgttccgcaatgcgcagcatccgtacacgcgcacgctgctcgacgcggtgccgcgcacacccaccggcggcacgctgctggcggcctgagtcctcccggcaggcccatggcctgacctgacatcgaagcttcgcgaggcggctctaggatgagtgggtcataagcatctggttgcgcggccgcccttgtctcgcggaagatgcctgccccctgttccgaggacattgcttcatgctcaaacgacgcaccctgctcgccaccggcgccgcagccctggctcccctcgcgctgccgacggccgcattcgcagagagaaaaaaggacgcgctggtgctggcgctcacgctggagcccacaggcctcgaccccacggccaaggccggtgccgagatcgcggaagtggtgctctacaacgtcttcgaaacgctcaccaagatcgactccgacggcaacgtggcgccgctccttgccgagagctgggaaatctcgcccgacctgaaaacctacaccttcaagctcaggcgcggcatcaggttccagaacggcgagcccttcaatgccaacaccgtgaagttctcgttcgaccgcgccgccgcggccaacagcaccaacaaggacaagcgcactttcaccaacatcggcgcgcaagtggtcgacgagcacaccgtggtgctgatcaacaaggaaatcgaacccgagctgctcttcctgctgggccaggcctcggccatcatggtcgagcccaggagcgtcgacaccaacgccaccaagccggtcggcaccggcccctacaagctcgacaactgggccaagggctcggccatcgtgctcgccaagtgggacggctggcgcaacgccgacgcagtgcgcatccgcaaggcgagcttccgcttcatatccgaacccgctgcgcagaccacggcgctgctctcgggcgacgtcgacctgtttccgcacgcctcggtctcgcgcagcctgccgcagttccagaacgacaagcgctttcaggtggtgttcaacgcctcgcgcggcaagaccatccttgccatcaacaacaggcgcaagccgctcgacgacgtgcgcgtgcgccgcgccattgccgccgcgatcgaccgcaaggccgtgatcgaggccgcggtggacggccgcggcgtagccatcgggagccactacgtgccgggcgcgccgggctacgtcgacaccacgggcatcaacccctacaacgtcgagagggcgaagcagttgctggccgaggcgggcgtgaagacgccgctcgaactcgacttcgtgctgccgccgccgccctatgcgcggcaaggcggcgagctcattgccgctcagctggccaaggtgggcatcgtcgccaagatccagaacgtcgagtgggcgcaatggatcagcggcacatacggcaacaagaactacgatctctcgctgatcctgcacgtcgaacctttcgacctcgtgaactacaccaagcccgagtactactggggctaccagtcggccaggttcaacgagctgttcgacaaggcgcgcaacagcgcacgcaccgctgatcggctgcgctacctcggcgatgcgcagcggctcctggccgaagatgcggccaatgtcttcctgttccagccgcagttcatcacggtggcggcacgcaacctgcgcgggctctggaaagacaccccgatcttcgtcaacgacattgccgccctctcctggagctgagacggcatccgggaacgtcccgaggaaaaaccgcctccgcggcccagcgccaaggcgcccgctgcgagagaatgactttgctgcgcgcgtggcatctttcgtgctgcgtgtccttccttcgtgccgcggcgcctccattcggggcgcggtgcacatggaagcagtcatctcgcactcaccgactttccggagatcacaacgtatgttgaaccgtcgcaccctccttaccaccgccggcgccactgttgcgctggcctctcccattgccggcatggcgcagggacggaaggacgccatcgtgatcggcatggcgctcgagccgccggggctcgatccgaccgccggtgccgcggccgccattgccgaggtcgtgcactacaacatcctcgaaacgctcaccaagatcaacgccgacggcaacgtgacgccgctcctggccgagagctgggaagtctcgcccgacctgaagacctacaccttcaagctcaagcgcggcgtcaagttccagaacggcgaaccgttcaacgccaacaccgtgaaattcgcgttcgaccgcgccggcagcgagaagagcaccaacaaggacaagcgcactttcgcgaacctgagcacgcaggtggtcgacgactacaccgtggtgatcatcaacaaggagatcgaccccgacctgccctttgtgctgggccaggccaccgcggtcatcgtcgagcccaagagcgccgacaccaacgccaccaagccgaccggcaccggcccctacaagttcgacagctgggccaagggctcttcgctcacgctgagcaagtgggacggcttccgcagccccggcactgcgaagatcaacaaggtcacgttccgcttcattgccgacgccgccgcgcaggccgcgtcgctgcttgccggcgacgtcgacgtgttcacgcgcatcggcacgcgcgtggtgccgcagttcaagaacaacccgcagttccagaccatcctggccggctcgcgcgccaagaccatcctgtcgatcaacaacaagaagaagccgctggacgacgtgcgcgtgcgccgcgccatcctcgcggccgtcgaccgcaaggcggtgatcgaaggcgcggccgacggcttcggcgtgcccatcggcagccactacgtgccgggcgccgccggctatgtcgacaccacgggcatcaaccccttcgacatcgagaaagccaagaagctgctcgccgaagccggcgtgaagacgccgctcgaactcaccatgaccctgccgccgccaccctatgcgcgccagggcggcgaggtgatcgtggcccagctggccaagatcggcatcacggtgaaggtgcagaacgtcgaatgggcgcagtggctcagcggcacctacggcaacaaggactacgacctgtcgatcatttcgcacgtcgagcccttcgacctgggcaactacgccaagcccgactactactggggctaccagtcgaaggccttcaacacgctgttcgacaagatcaaggccacgggcaacgccgccgagcgcaacaagctgctcggcgaggcgcagaagatgctggccaccgacgcggccaacggcttcctctaccagccgcagttcccgaccatcgcgaagaagaacgtgaagggcatctggaaggagaacccgatcttcgtgaacgacctctcggccctgtcgtggggatgagcgccgaagtgtcttcttcgctcatcgacctctccgcccaggaactctccaccgcctatcgcgacaagcgcctgtcgccggtcgaagtcacgcaggccgtcatcgctcacatcgagcgctgggagccgcagctgcaggccacctggctcttcaggcccgaagccgcgctcgagcaggcgcgcgcctcggaagcgcgctggcaacgcggcgaagcgctcggcccgctcgacggcgtgccggccaccatcaaggaaaacattgccacccgtggcgacccaatgccggctggcactgcggccgtcgatttgaagccggcagccgccgacgcgccgcctgccgcgcgcctgaaggaagccggcgcggtgatcgttagcaagaccaccatgcctgactacggcatgctgtcttcggggctctcgagttttcacaagctggcgcgcaatccgtgggatctccgcaagacgccgggcggctcgagcgccggagccggtgcggcggctgccgcgggctatggcccgctgcacatcggcaccgacatcggcggttcgctgcgcctgcccgcgagctggtgcggcatcttcacgctcaagccgagcctggggcgcatcccgatcgatccgccttacatgggccgcgccgcagggccaatgacccgcagcgtcggcgatgccgcgctgatgatgcaggtgctctccaagccggacgcacgcgacagcatgagcctgccgccgcaagacatcgattgggccggcttcgatgtgtcgcccgaccatttgcgggggctgcgcatcggcctgctgctggatgcaggatgcggcctcgcggtcgagcccgaaatccaggccgcagtcgagcatgcggcccgtcttttcgaaaaagccggcgcaatcgtcgaaaccatgcagccgttcatgtcgcaagccatgctcgacggcatggaccacctgtggcgcatgcgctcgctggtggacatgaaggcgctgcgcgccgaccagcgcgccaaggtgctgccctacatccgcgaatgggccgagagcgcggccgagttcagcggcgagcacgtgttccgcagcttcagccagttccacgcaacgcgcgtggcggcggtgcaggcgtgtgcgcgcttcgactacgtgatctcgccggtctcgcccaacatgcccgcggccgccgaagcgccttcgccgacgaatgacccattgcggccgctggagcacatcggtttcacggtgccgttcaacatgtcggagcaaccggcttcgtcggtgaactgcgggtactcggcggacggattgccgatcgggctgcagattgcgggccaccgtttcgacgacctcggcgtgctgcgcgtgtcgcgtgcgttcgagcagatccgggagccgcagcggccctggccggtagtgcctcgaggctgagattcatccaggtcgcgatcccgccgacggggtacctttctccgcgaatgtcccccggcctacggcctcctcctttatttcgctgcgcaaggcaccccatcgacgtgctcgttgttcagagcggtggttgatcggcggttcactggcagcgtgccccagtgcacagggcgccgggtgctccccgcagcgaaataaaggaggagccgaaggcgggggacattcgcggaggggagtacccggtggcctttgcacacgccccgaacaacagccccaaacaaaatcactcaagtcgcagcgtagcgccccggcttgtggttgatccacagaaaaagccccatcaccaccgcggccagcaccgaccagcccacgcgctgcggcggaatcacgaacagcgcgagcaacaccaccgtgcagtcgatgccgatctgcaccttgccggcaggccagccgcgtttctcttgcaggtacagcgtcagcaccgtcgcgccgcccaggctcgcgcgatggcgggcaagaaacaggcagccggtgcccagcaacaggccgccgagcacggccgcgaaggccgggtgcagcgattcgatcgagatgtagcgcggcgcccaatcggtcatcaccgacagcagcgcgatggccgagaaggtcttgaccgtgaaggcccggcccatgtggcgccatgcgaaccagtagaacggcaggttcaccaggaagaacagctttccgaagctcacgccggtggcgtagtgcaagaggaatgcgacgccggccgtgccgcccgtgagcaaacctgcctggccgaacagcatcatggcgatggcgacgaacaacgtgcccgaaaaaatggcctgtgcgtcgtcgaaaccggagtggcgcagcagatccggtggggttgtgggttgtggcgcgtccatggcgagcttgacgcaaatcccgcgccaccccgaaacgtcacaccagatgggtcgccagcatctcccgagcccgcgtcacgaattccgtctcgcccctgcggccgggcagcaactggaacgcgacccggggcaacgccggcagcccatgcggcaccgccagccgcgccacgccgtcgcatgttgccgattcgttcaggcaggcgacccccagccccgcacccaatgcagattgcaagcctgccacccccgaagccacgtgtgccagcacatacggcacccgcctccgccgcaacagcgccaccgtgaactgatgcagcgagcatgtgtccggcaaggccagcagccgaaccggctcgccccgcgccagccgcatgcccgtcgcgccgagccacaccagcgattcgcgccggatcaccgacgaggccttcgcgccctgctccgacgccgaagaagaagccccggcgatattcattgccagccccacgtcgaagtctccgcgtgcgtacgcagcccggagcgcgtcgctcttcaggatgctcacgttcaaccgcacctgcggatagctttcgccgaggcgccccagcagccgcgtgagatcgccgggacgaaagtagtcggtcaccgcaagccgaagctcgccctgcaaggtctcgccatgcagatcgcgaaacgcctcgtcgctgagcgcgaggatgcggcgcgcataggccaggagccgcgtgcccgcctcggtcggcgccacgccggccttgctgcgggtgagcagggactgccctgcccgttcctctagcttgcgtatctgctcgctgaccgacgactgcgaaagaaacacgcgcggcgcggccgccgtgaggctgccggcatcgatcaccgcggccagggtgcggagctgttccaggtcgaaggtctgcatgcctatccatctgtttttccgatgttcaacatcatatattcccgcttttccgatggatatggcgtctccacaatacccccatcgttcactcattcatggagttccagatgccgcatatcgttgtccacctctcgggcgagcccgatgcccagctcacgcgcaagaccgtcgacgtggtcgccgagctgacccagagtgcactcggcaagcagttgccggtgatcgccatcacggtgcagtacatcgccgccgacgcatggttcatcggcgggcggtcgctggcctcgctcggcaagtcggcgttccacctcgacatcagcgtcacggacgagaccaacaccaaggcggaaaaggcgcgctacctgcgcgaagtgaatgccgccatggcgcggctgcggcccaacctgcacgaggtgtcgtacatccacgtgatcgatgcgcgcggcgcggcctacggctatggcggcaagacgcaggaataccgccaccagcaagcaggcgtttgaagcccgcggcggggcgtggcaccatggcgccatgccccccgcaaccctgcatgccgacagcttcggcaaccccctcacgctcgacgacgccgccagcctgccgctcgtcgacgacttcgtcatgggcttcgtctcgaccgaagcgcgtgcggtcaacctgcttgcactggccgaccgcgacgcgagccccatcgtgcaggcctattgcgcaacgctgcacctttttgccgaatcgcgcgaggccgcggccaacgcacggcccttcctcgacaaggcgcgcgcaggaatggcgcgcgccacgcagcgcgagcagcgctacgttgcggccatcgaggcctgggctcagggcgacatcgccaaggccatcgccctgcacgcggagcaggcgcgggagcatccgcgcgacctcgtctcggtgaagctcgggcagtaccactgcttcaatgccggcgactgccccggcatgctgcgcctggcgctcgctgcgctaccggccgcgtccgacgtgccctacgtgcacgggatggccgccttcggctacgagcagtgccacctgatgcgcgacgccgaggccagcgcccgccgcgccatcggcatgtgccgcaaggaaccctgggcgcatcacgcgctggcgcatgtgatgctcaccgaaggccggctctccgaagggctggcgttcatgcagggcgtgagcgacagctggaccgggctcaattcgttcatggtcacgcacaactggtggcacgtggcgctgttcctcatcgagctgggtcgcgatgccgaagccctcgcggtgtacgaccgcgaggtgtggggcgtggtgaaggactactcgcaggaccagatcggcgccgtctcgctgctcgcgcgcttcgaactcgcgggcatcgacgtcggtgcgcgatgggacgacgtcagcggctaccttgtgcagcgcaccgccgaccacgtgctgccctttctcgacctgcagtacctgtacggcctagcccgcgcgggccgccccgaggccgatgcgctgctgcgcaacatccaagcccatgcgccacgcgcgccgctctccgcgcgcgccgcctgggagcacgtgtgcgtgccggccgcgcgcggtctcgttgcgcatgcgcgcggcgatttcgcttccgccatcgaagggctgggcatggccttgccgcggctgctcgagattggcggcagccacgcgcagcgcgacctgttcgagcaggtgtacctggacgccctcgtgcgcgccggcagccaggccacgctcacgggtgcacaaggcatcctgcagcagcagcgcaacggccagcccgagtcgttgcgcctgcgccggcaggccagtgccgtctatgcgcggctcgggctcgaacaactggcatcgcggctctgaggggccgggtggaggccatgccttccggtcatggggcgtatcgcaaaaggaattaacggtgcgcgggagtggctcctaaactgcccgactcacatcgctccggatcgctcgccccatgcagaaatcagttgtcgtgctcgccgcgctcgcggccctggcgggtctttcatccgccgccgatgccccggtcgaactcgacctgctgctgcgcggcggcaccgtctacacgggcgactccaacgaacccatcgtgggcgacgtcggcatcctgggtgaccgaatcgtcttcgcgggtccgaaggcgccggcgcaattcagcgcacggcggaccatcgatgccgcgggcatggtcgtggcgccgggcttcgtcgacgcgcacacccacgccgatgccgacctgcattccaccgatccgcagaagcgcctgaacattccctttctcacccagggcgtgaccaccgccgtcatcggcaacgacggctttggcggcttcgacatcgcggcgcagacgaagcggttgcgttcggcgccggtgggcaccaacgtggccatgtacgtgggcttcggcccggtgcgcatcagccagctcggcgaagccaatcgcgcgcccacgcccgagcagctcgacgcgatgcgccagcatgtgagccgggccatgtgcgacggtgcgctgggcctatcgaccggtcttttctatccgccgcagaatttctcgaagaccgaggaggtcatcgagctcgcgaaggtcgcggcccggcacggcgggctctacgacagccacatccgcgacgagtcgatgtacaacatcggactgaaaggcgccatcgaggaagtgatccgcatcggccgcgaagcccgcctgccggtgcacgtggcgcacatcaaggcgctgggtgtggacgtgcagggccagagcggcgacatcatccgccgcatcgagaaggagcgtgccgccgggctcgacatcacggccgaccactatccgtggacggcttcgagcacgcgcttctcggccgcgctggtgccgccatgggccgtcgacggcggccgagaggccatgctcaagcgcttcgacgatgcggcggtgcaggagcgcctgcgaaccggcatgcgggagaacctgcgcctgcgcggcggtcccgagacgatcctgttttcggccggcagcaccaagtatgtcggcaagacgctgaccgacgtggccaaggcctcgaacgccgatccggtggatgccgccattgccgtgctgcgcgacggcgacctgatgatcgcctcgttcaaccagagcgacgacgacgtgcgcgcgttcatgaagcggccatgggtcatgacctcgtccgactcttcgctgggccatccgcgcgcctacggcaccttcgcgcgcaagtacgaccagtacgtggtgaaggaacacgccatctcgctggggcaattcatccgcagcagttcatcgctgacggccgacacgctggggctgaagcagcgcgggcacctgcggccgggctactacgccgatgtggtcgtgttcgaccccgcgcgctatgccgcccgggccacgtacacgcagcctgcgctgctgtccgagggcgtggtcacggtgctggtgaacggccggctcgcagtggatggcggcaagcccaccggcattggcgcggggcaagcgctgctgcgcacgccgaaggccggcagctgcacctgaggaggcgcgcactttttcggcttcagcggctcagttcttctcgagatgccgccgctggtcgtaggtcggctgcggcggcaggtcggcaagatgccgcgtgtcggcccagtcgacgatctcgatcgcatcgggcatggccgggtcggcgatgcggatgcggttgaagcccgcattgggaatgtcgctctggcgcggcccgctgaggctgagcccgcgcgcggtgcgccacaccatgtcgagcacgccgccatgggtgaccacgatcaagtgctgcccgcgatgcgtggcggccagggttccaagcgcggcgacgatgcgcgcatggaactcgcgcgccgattcgccctcgggcatggcgtggtcctcgcgaaactccagccattgctcccaggcgcgcggatgcagcgcctggatctcgtcggcccgcatgccttcgacaatgccgaaatattgctcgcgcaaacccgccgaggtgaccaccggcagcgacagctgcaacgctgcgggcgcggcggtctgctgcgcccgcatgaggtcgctgctgatgatgtgttgcgccgtttcgctcgccagccgcaggccgaggcggcgcgcctgctcatgccccatgtcgttgagcggcacgtccgcatgcccctggaagcgcagttcgcggttccaggcggtttcgccgtggcggatcaggatgagctcggtcgtggaatcggggttgggcgtgggcatggaacgcccattctctactgcgtgcgtgacgcacaggccctcgatggccccatctgttgcatggccgccacctgcagcgggggcggtggggaaagcatgtctgccgggcgccccaaaaacccctcgccgagagacccatgccgctgcgccagatcgctcgatcacgcagaatgggcccatgccgaaccttgtcctgctgcccggcctcgcctgcgacgagcgcctgtgggaagcgcagcttcccgtcctcccccccgcgttcgaagcccgtgtgagcgatgcccacacgcggcacgacaccatcgaggccatggccgcggccgtgctgcgcgaacaccccggtccgctcgtgctctgcggcgcgtcgatgggcggcatgatcgcgatggaagccgcgcggcaagcgcccgagcgcatcgccgggctcgcgctgctgggcaccaatccgcggcccgaggcgcccgaaatgtacgaactgcgcgaaggcgcgatcgaattgttcgagcaaggcgatctgcgcgaggtgatcgaaccgaacatcgtcttcgcttttcatcccgcgcaggccgccgacgaggtgctggtgcagcgctatctcgacatcgtgctggaagccggcgcacagcagctgatccggcagaaccgcgcggtgatgcggcgccccgatgcgcgcgcccacctgcgctcgctgcgcgcgccggtgctgctggtctgcggcgataccgaccggctggcgccgcccgactgcacgcgcgaaatcgcggcgctggtgccgcacgccgaagtggtgtgggtggcccaatgcggccacatgctgaccatggagaagcccgcgttcgtcaacgcggcgctgctctcctggctggctcagtggaactgaccgccggtttcggcaatgtctttttcaacggccagcgcggtggcgaccgcaacgcgcagcgcctcgaccatggcggccagcggcatgctcggcacacccggaaaacgcgccgcctgctcgggcaggtagggaatatggatgaagccgccgcgctgccccgctacggggtgcgttgccatgcggtgcatgagtccgtagaagatgtggttgcagacgaaggtgcccgcggtgttcgacacggacgcgggcacaccggccgcgcgcagatcgcgaaccatggccttgatcggcagtgtcgagaaatacgccgccggcgcaccgggcatcacgggcacgtcgatgggctgccggcccgcgttgtcggcaatgcggccgtcgtcgatgttgatggccacccgctccggcgtgatctcggcgcggccgccagcttggccgatgcacagcaccagctcgggccgcagctcatccatcgcgctcgccagcgcctcgatcgactggccgaaggcgcagggcatctggcgcgcatgcacggtggcgcggccgcacttccagccgtcgagggcgcgcacggtttcccatgaaggattgagggcttcgccgtcgaacggatcgaatccggtcagcaggaccttggttcgctgcgccacggtggaacggcgcgctcaggccaccgcgcgaaccgcgatgccttcttgctgcaggcggtcgcggatgcggcgcgcaaaagccagcgcatgcgcgccgtcgccatgcaggcacacggtctgggcattgaggggtacggtgctgccgtcgatggccgtgaccttgcggtcgcgcaccatcgagagcgtctgggcgagcgactgttcttcgtcttcgatcagcgcgccgggctggctgcgcggcaccaggctgccgtcgggcatgtagccacggtcggcaaacacctcttcgacaggcgtgaggccggcgcggcgcgcggcgtcgatcatgccgctgcccgcgaggccgaaaaacttgagcgagggatcgaagcgccgcaccgcctcgcacagcgcgtcggcgagttcaggctccttcacggcctggttgtagagctggccgtgcgccttcacgtgcgtgagcttgccgccctcggccttgacgatcgcggccagtgcgccgacctggtagagcacgttggcgacgatctcgtcgggcggcaggtgcatggtgctgcggccaaagttttcgcggtcgggaaagctcgggtgggcgccgatggccacgccgtgctcgatggcccagcgcacgcattgccgcatggtcttggcgtcgcccgcatgccagccgcacgcaatgttggccgagctcacgaggccgagcagcgcttcgtcgctgccggcgccttcgccgagatcggcattcaggtcgatttgcataaagcttttttccttcttcgaggcgggcccgcgcctccacgcgcacagtctatgccggtccgctccagcccgcagccgcgagcccttgcgccacttgcgcgagatagcgctgctgctcggcccacgcctccagcgccgcggccatgtcgacctgcaccagccgcaaccggccgtcgagcggcgcctgcgcgagcttccacaggtcggcgcgaatcaccacgccgatgcgcggatagccgccggtggtctgcgcgtcgcccatgaggatgatcggctgccccgaagggggtacctggatggtgccggggatgacgcccgacgagagcatgtcggcactgcgcttgcgcttgagttcggcgcccgcgagccggcttcccatgcggttgctctgcgcggtgatgcgccagcgttcgctccagagttgcgtgtgcgaggctgcggcgaactgatcgaactcagggcccggcagcacgcgcagggcgatggccccatcgctttcgtcgggaccccagtccggtccgcgcaggccgaacggacgccggccgagccgggccgcatcgagcgccgtggcgcccagcgccagccggtcgcccttgcgcagcgcgcgcccctggtggccgccgaagcccgccttcaggtcggtgctgcgcgagccgagcaccggcggcacgtcgatgccgcccgccaccgcgagccagctgcgcaacccggctttcttcacgtcggccgcattggcgcccgcgagcttcagcgtctggcctgccgccaccggcacgctccagcagggccagagcggcgcgccgtccagccgggcgccgaagccgtctcccaccagcgcgatgcgggtggcggtttcgaagcggatctcgcaaccgcccatggtgatctcgagacccgccgccgcgtcggcgttgccgaccagccggttcgccagcgtgagcgccagcacgtcgagcgcgccgcccggacagatgcccaactggcgatgtccgtgccgccccaggtcttgcaccgaggccagcatgccgggcttctggaccagcatcatgtggtctggacgctttcgacgacgaagcgcacgcggtcgcccgggcgcagcagggtgggcggctcggccgagggattgaagagttcgagcgaagtgcggccgatcagctgccagccgcccggcgacaccagcggatagatgccggtctgctcgccgccgatgccgaccgagcgtgccggcaccgcggtgcgcggctcggaccggcgcggcgtggccagctcgggcggcagtccgcccatgaaagcgaagccgggcaggaacccgagcaggtagaccacgtagtcggcctcgctgtggcgccgcaccacttcggcctgcgtgagcccggtgtgagccgcgacgtcggcaagatcgggaccatgctcgccgccgtacgccaccggaatctccaccctccggccctcgatggcggtggccgacagccgcggccaggcctcgttcacgcgcgccatcagcgcatcgatatcgatcgcggtcggatcgaaagtcagcgtgagattgttcatgcccggcagcacctcgcccacgccaggccaccgctgcacctccgcgcccagcgcccagatccgttgctgttgcggcagcgtggccggcggcggcagctcgcacagcagcgccgcgtcgcccagcggatgcaggcgaggcaaaggaggtcggctattcacgaccgaggctgcgcaccttggctgctagctgcttctccacatcgggcgaaacgaacttgtggacctcaccgccgagcatggcgatttcgcgcacgaaggtgctcgagatgaactggtacttgtcgctgggcgtcaggaacacggtctccacgtcgggcatcagcgagcggttcatgcccgcgagctgaaactcgtagtcgaagtcggtcaccgcgcgcaggccgcgcaccatcgccttgccgccgcgcaccacgacgaaatcgcgcagcaagcccgaaaagctctcgaccgtgacctggtcgctgtacggcttcacggcctcgcgcgccatctccatgcgctcctgcagggagaacagcgccttcttgtgatggcccgccgcaaccgcgacgatgaccttcgagaaaagctgggttgcacgccgcaccacgtcctcgtggccgagggtgatgggatcgaaagtgccgggataaaccgcgatcacgttgctggccatggttgcttcttcctcatgcagccggtgcggcttgtccggcggattatgcagtcccgtttgcagcctgccgcagcaggtgcgcatgtaccgcccccgcctttaagtaacgaaaaccaacaaggccggcggcggcaagctcttcgtcgttccagcggcgcggtgcttccaggtaaacggcgcccccggctttcacggcccgtgccgccgccctcagagcaggttcgtagagggcgacattgtcgaaaggcgggtcgagaaacacggcatccaggctgccggcggctgtgcgttcaagcgcggtgagcccgttgccccgctcgatgcgaacggcttcggccgagagcttggtcttggcggcctggagctgcgccaccagcgcggcatcctgctcgcacagcagcacgctcgcggcgccgcgcgaagccgcctccagcccgagcgcccccgtcccggcgaaggcatcgacgcattgccagcccggcagctcgccgccccctgcgccagccatgctcgcgagccagttgaacagcgtttcccgcacgcgatcgggcgtcgggcgcaggcccggcttgtcggccacgggcaggcggctgcgcttccattggccgccgatgatgcgcacctcgcgcggcagcgttttcgaacgcgctggcgagggcgatggagtcggggtggagcgctgggtggctgcggctttcttctgaggcatggggcgagcttaacgccgccgcacgggcccctatgcgcccagaaaagcgcgccgcgccagcagcgcggccagcaccagcatcgtgccgccgatcaacgcatcgagcatctgccaggcgcgcggacgcgcgaacaccggcgccagccatcgcgccccaaagcccagcgccgagaaccacagcgcgcttgccactgccgagcccgcgacgaaccaggccttgagcgagccgccgtactgggcgccggtgctgcccacgagcagcacggtgtccaggtagacatgcgggttcagcaaggtgaagcccgccgcctgcgccagcacggcggttcgcgagagcgatgcgccctgggccgcggcctgcaatgcgccgggctgccgcgaacgccacagcgcgcgcaggccgtacgcgcccaggaacaacgcgccgaggccggccagtgcggtggcgaataccggccgcccgttcagcgcctgcgccatcccggccacgcccgccgcaatcagcaccgcatcgctggcggcgcagaacagcaccaccgcgctcacatgctcgcgccgcaggccctggcgcagcacgtaggcgttttgcgcgccgatggcgacgatgagaaccaggctcatgaagagcccgttgatgaatgcggtggtgatctgttcgtaagccatggcgcaagcttgccgccgcgagccggttaattcaaactaaacttcctaagccatattcagtttttctaatctagcgaggagccatgctcgactacgccgccctgaacgcattggccgccgtggtgcgcgaaggcagcttcgagcgcgcggcccgcgcgctgaacgtcacgccgtcggccgtctcgcaacgcgtgaagctgctcgaagagcgcaccggcggcgcgctgctggtgcgcggccagccctgcgtggccaccgaagccgggcagcagctgtgccgccacatcgagcgcgtgggcatgctggagcacgagttgcgcgacgccctgccctctcttggcatgggcggcgggagcggcagcgcgggcgagcgggtcacggtgcgcgtggcggtgaacgccgacagcctcgccacctggttcatggcggccgctgcggcctttgcacagcaggaagaatcggccctgctcgacctgaccgtggacgaccaggaccacaccgccgagcgcctgcgaagcggcgcggtgctggccgccgtcaccgcgctggcgcagccggtggcgggctgcaacagcgaagcgctgggcaccatgccctacgtggccgccgcaagcccggagttcgttcaccgccatttcgacaagggcgtgggtgcgcgcaccctggccggcgcgcccagcctggtgttcgaccgcaaggaccggctgcaggcgcgctgggtgcggcgcatctgccatcgcagcatcgagacgccgcggcactggctgccatcggcgcatggcttcgtcgaagcggcgcgcgccggcatgggctggggcatgctccccgtgagcctggcggccgatgcgctgcgcacgggcgcgctggtggaactggtgtccggttcggggctgcaggtgccgctctactggcagcaggcacgcgcagcgccgcggctgctcgaacggctcaaggcggcggtgcgcgcagccgcctcgagcggagcgcacgcgctgcgctgaacacgccgcctgctgcctattgcttgccgcccaccaccaccgtcaccatgcggtcgggctgcagcttgcgcgcaaaagcggcgcgaacttcggccgccgtaaccgcgttcatgcgcgcggtccaggtgtcgagatagtccagcggcaggtcgtaccacgcaatattggccacgttgccgatgagcttgcggttgctgtccagcaagagcggaaagccgccaatcaggttgtccttcgcggccttgagctcttcggtggtcggaccttcggccacgaacttcgcgaccacgtcgcgcgaaaccttgacggcctcctcggcctggtcgggccgcgtctggaaaccgacgcggaacgcaccggcatccagccccggcgcaaagccgctgtagacgctgtaggccaggccgcgcttctctctcacttcattggtcaaccgcgagacgaagccaccgccgcccagcacgtagttgccgagcgtgagcgcgaagtgatccgggtccttgcgcgggtagcccggctggccgatgaagacatgggcctgggccgaggcgaacggaatgcgctcgtccttcggggcagcgagtgcggtgaccggtgcgatggcaggcagcggcgtgcaggcctcgggtccgggcagccgcgagagcagcgcggtggccatggcttccgcctcggcgcgggtcacggcgcccacgatgctgagcttggcgcggcacggcacgatgagctgctggtagcgctgccgcatggccgcggtgtcgatccgcgcgagcgtggcttcggtgacttgctgcccgtaggggtggatgccgtagacgccctgcgcgaaggcgcggcccgcgatggtcgccggcttggtgttggcttccttcagcgaggcattgatgcgctcgcgctcgcgctgccagatgtcgtcggggaaggccggctcgccgatctcgcgcgaagccagcgctaccaccttggcccgcagcgcggggtcggacagcgtgcgcagcgagtagctcgcgcgatcggtgccggcgctggcattgaactccgcgcccaggtcggcccaggcttcgcccagcgcgttctcgtcgagtgccggctcgccgttcttgccggcgcgcacgcccttctcgaccatggtcgcggtcgcgctggcaaggcccgcttgcgccgccggatcgcgcctgctgccggcgtcgaaatcgatctgcacgtcgacgatgggcagcgcctgggtcgacaccaggtagatcttggcgccgctcgcaagcgtccagtgctcgatgggcagcgcggcttgcgcggcgttggaacccgccacggcggcaacggcagcgaacagcgcggaacgcaggatttttttcattggggtcattggaatccggcgcccttcagcgcagttcgccctggggcgctgcaaaaccgcggccgcggggtttggattcgagcggcagggggcgcagggtggccacggtgagctggtcgtctccaaagtacttggcggccacggcctgcacctgggatggtgtcacggcctgcagcttcgcgatgatgcgcgcgctggtgtccagcggcagcccctgcacccaattgctgccgagttcgcgggcctgcgccatcaccgaatcgcgcttgtaggtttcgctcgccacccattgcgtcttgacgcgcgcgagttcggcttcgcccacgccttccttggcaacgcgcgccacctgggcccgcagcgcggcctcgaccgcttcggcgctcttgccgttcgccggcacgcccacgagcgtgaacagctgcggcccgcggccggccaggcccgaataggcgctgacggagtcggccacgcggtcggggccctgggtcagcgcgcgatcgagccgcgcgccggtgtagccgtcgagcacggcggagagcacttcgagcgcccacacgtcgctgtcggcggcgtcgatgctctccagctgcggaatgcggaacgcgagcgacacgtaggcctgctcggccggcgccttgaactcgatgcggcggatgccgcgctgtgcgggctcggtgcgcggcttgcgcgcgggcacggcgcgcgcgggaatgccgccgtaatacttctcggccagcgcacgcaccctggccacgtcgacgtcacccaccaccaccacggcggcattggcgggcacgtaccagcggcggaagaaggcgcgggcgtcgtccggcgtcatggcgtccagatcgctcatccagccgaccacggggcggtggtagggcgaggccgtgaagacggccgcattctgctgttcgccgagcaatgcgcgcggctggtcttcggtgcgcaagcggcgttcttccttgaccacttcgatctcgcgcttgaactcgtcgtcggaccactggttgttggcgaagcggtccgattcgagcttcatgacctgctcgaggctggcgaccggaatctgctggtagtagccggtgtagtcgcgcgtggtgaaggcgttttcctgcccgcccagggccgccacgcgacgcgagaactcgccaggcttgatgtccttggtgcccttgaacatcatgtgctcgagcacatgcgccacgcccgaggtgccatcgacctcgtcgaccgagcccacgcgaacccacaacatctgcaccgccgtgggggcgcgcctgtcgggcagcaccagcagcgtcatgccgttggcgagggtgaactgctggggagcgggtgccgtggcggcgagggatgaagcggcgggagccggtgtgggctgggcctgcgcaggcatggtccacggcgccgaaaacgccatcgccagcaccgcaccgaacgcagcacggcgtggcgaggggtgtttcatagaatgggtcggattgtaaaaagctcccgatgttcagtttcttcaagaaaaaaccgcctgccgcatcaccggccgcgccggcgccctccccggccgccgagccggcaccagcccccgagcctgcggccgcgcccgcgcgctcggtgttctcgccgtcgagttggttcggctcgaaacccgccgtggaggaagcgccgcctccgcccgccgcgccggcaccaccacctccagtggcgcctccgccgccaccaccccccgtagccgctcccgctgcgccgatcctcgcgcccacgcccacgcccacgcccacgcccacgcccacgcccacgccagcgcctgcgcctgcacctgcactcgccgaaccggacgagcccctccccgccctcatcaccgaggcagccatggcggccgagcgcaagggctggttcgacaagctcaagacgggcctgcgcaagaccggcaccggcatccaggcggtgttcgtcaacgcgcagatcgacgacgcgctgtacgaggagctcgaatccgccctgctgatggccgacgccggcgtcaaggccaccgaatacctgcttgacgacctgcgcggccgcgtcaagcgccagatggcgaccgacgcggcgcaagtgaagcggctgctggccgacgcgatcaccgacctgctcaagccgctcgagaagccgctggtgatcggccagttcacgccgacggtgatcatggtggccggcgtcaacggcgcgggcaagaccacctccatcggcaagctcaccaagcacctggccaacgagggcgcctcggtgctgctggcggcggccgacaccttccgggcggcggcgcgcgagcagctgctggtctgggccgaccgcaacacggtcgagatcgtgagccaggaaggcggcgacccctccgccgtgagcttcgacgccgtgacggccggcaaggcgcgcggcaaggacgtggtgctggtcgacaccgcgggcaggctgcccacgcagctgcacctgatggacgagctcaagaagatcaagcgcgtcgtcaccaaggccgacgccacggccccgcacgaagtgctgctggtgatcgacggcaacaccgggcagaacgccctgacgcaagtcagggccttcgacgagacgctgggcctcaccggcctggttgtgaccaagctcgacggcacggccaagggcggcgtgctctgcgccattgcgcgcgagcggccggttccggtctacttcatcggcgtgggcgagaagctggaagacctcgagaccttcaacgcacgcgaatttgcgcaggcgctgctgggctgaagtgcagccagcagcgcccaccgccgcttagaagccgcttagaacccaaacagcgagcgggtatcgcagagaaaaccgctgcagttggccggccggacgtagagcgtcctgatctggccgctcggcagcatgtagtcgcccaccagcgcattgcccttggcgccctcggcattcgcttgggcgatgtagtccgcgctgttggccgcggactgcaggttctggtagctgaacgtggccgattgcgacaggtctttctcgtagagcagcttcgtgccgtccgagaagacgtagcccgtcttgaaccggaagccccgggcgccctgggcctcgaactgggccagaaaatcagcgtcgctgccgggctggcccagcgcttcatagccgtaggtcgcgctgccttgcgtgtccttctggtagaccagcaccgtggtcccgccgaccatgtaggcgccgccgacactgtagtagccgttgccgccctgggcgttggtctgcgacagatagccggtgctgtcggcaggtgccgccagcacggcataggtgtaggtcgatgcggagccgttgtccttgcgatagaacgtgcggctctggccgccgaccacgtacggcccgccccacttgaagcctctggcgccctgcgcgttgagctgcgcctcgaggtcagccacggaactggccacgggcagcagctcgaaggaataggtggtctcggcgtccttcacataggcttcgacgacctccacgctggtggggccggtggtgaaggcaaggccgctgaagaagcggaaggcccttgcgccctgcgcattgagccgatcgagaaacgccggagcatctgcggcgggctgcaaggcctcgtatatgaaggtacgcgtagccggggccggggccggagccggggctggagctggggccggagcgggcgatggtgcaggggcgggcgcgggtgctggcgcaggagccggtaccaccggcaagccggcgaaaccaccgccaccactactgcctcctccaccgcaggccgccaaagtcgcggcgagcgccgatatccaaatttttgcttgcatgaaatctctccctgagacgttgacgtgtgtgagaccgcgcaacggtaaaggccggccgataggcacaccagtgccaaaagtcatgaggcgccggcaggcgcgagttcactcagggttcgaaacagcttgccggcatcgaccggcttgaacagcacggcgacgccggacgcgcggacgcgctgcaggcgttcgggcgcggtttcgccagtgaccagcaacaagggcatgccggtgccggcgcgctggcgcaggcgcagaccggcgtcgagcccgtcgttgccctcagccaggcggtagtcgcacaccagcagatcgaagggccgtccctggccctccgcctgcgcaagggctttctccgcgtccgcttcgtcggccacggcgtgcacctcgatggcccaggagcgcagcagctcgctcatggcctcgcggatttccacctcgtcgtcaaccagcagcacgcgcccgggcagtgcctgtgcccctgcagcacggtgccgatgcatctcggcgccttgcaggccagcgccccccagcggcgcggcggcgggcagcaccacgcgaaaatgggtgccccgtcccggacgcgaatgcacctgcaacggatggtccagcaggcgcgacagacgctgcacgatcgacaggccgatacccaggccctgcgagcggtcccggcccgggttgccgacctggtagaactcctcgaagatgcggccgatctgctcgggcgcgatgccgacgccggtgtcgcgcacctcgatccacaccgcattgccgcgtgcacgggccctcacggtcacaccgccgctcaccgtgtacttgagcgcgttgtcgatcaggttggcgagcaggcggtgcaacagctgcggatcgctgcgcacccacaacccgctcgcgcgcactcgcaattgcaattctttctgctcggcctgcggcgagaacatgtggttgagcggcaggaacaacgcgtcgagctgcacctcccgaagctccggcgtgaccacgcccgcgtccagccgcgaaacgtcgagcatggtgtcgagcgacgttcccagtgcgttcaccgcgcgcatcaggcgctccgcgttggcgccttcggggcggccgcgcagttcgttctccagcgcggcgccgaacagcgcaatggcatgcagcggctgccgcaggtcatggctggcgctggccaggaaacgggttttttcttcgctggcacgctcggtggcggcgatctgttccgccagccggacggccaaggcttccttttcgaagcgcagaagcagcgaatccgccagcagcttgtgctcctgcacgcccacgcgcagcatgaggacgagatagatcgtcgaaaaggccgcgaggaagagatggatggcgtcgccctgccacgccagcgcgacgatcagcccgcccatcatcggcagcacgtggccgaacagggcctccttcaggggccgcagcgattgcacggcccgagcgcaattgcccatcatcaccaccatcagcgcggccgtcacaggcaagttgccggcgggcacgaagatccacggcgccagcgcatcggcaaacccgagcagggtcacgatgcgggtgatcttgcgggcccaccgggcactttccgccgcaggttccgccgggctccagcgcggcgtgaagtacatgcccaggtacaacgccagatgcagcacgacaaacggcagcaccatgggatcgcccaactgcaggtacatgaacccaccaagcaccaggacgaaaacgacgcgggccaggaacgtcgcgctgtagttgaaatagatcgaggccacgtgctcgcgcagcacccgctggctcagcggggtttcggccgtgcgcggcgggctcaacgcaggctgctgatcaattgcgcacgcgaacgcacaccgaacagcagcaggatggtcgatacatggttcttcaccgtgccctcgctcaggttcgcgagctgggcgatctccttgttcgccttgccttcgagcacccactgcagcacctgcgtctggcgcggcgtgagttcctgccaggcgctggcgtgggccgattcagcgtagccgccgagcgccttcggcatcgccggagacgaaatttcggtcgactccgcatcgagcaggccgcaggcacggatgaagcccaccacctccttcaagtccgccgacttgggaagaaaagcactggcgcccagggccagcgccccttgggccagcgaggcgttgccggtgcccgaaagcaccacgatgcgggcggacggaaaacgcaatcgaaactcggtcaggccgctcaagccatgcgtatcgggcagtgccagatccagcagcaccaggccgatggactccccatgcgcttcatggagcaccagcgcatcggccacattgccagcttcgaacacctcgatgcccgtgccggacgaagcggcctgtgcctgcaccagcgcgcggacgccgagccgcagcagatcgtggtcgtccaccaccagaattgcggtgggcgggcggagcagcgcgggttccacgctcgaaggcgacgggtgcgatgaagattcgagcggaggggccacgcagtcgatcttagcgatgccccgaacgcgcgacagtgccctaagtcatggcgcgttcatgtccgcgaagaaagttttgctacatttttcatagcacttgccatcgcctgccggcagaggcaccatgcaggaccgccgcaccgaacggcgcttggagacaacatgctgcacaccgccgacgccccgctggcagcgggcgaccgaaaggtcgaccggctgctggcccactatggcgaaagccaccgccacccgaccaacgagctgatccacttcgtcgcgatcccggccatcatgctgagcatcgtcgggctgctgttcgcgctgcacccctgggtggcctacggcttcgtggccgctagcctggtgtactacgccaccttgcgctcccccgtgttcctggccaccatgctcgccgggacggcgctggtactggcgctggttcatgccatgggaggccttgtactgccggtctccgccgccatctttgtcgtggcatggatcttccagttcatcggccacaggatcgaaggcaagaaaccttccttcttcgaagacatccaatatctctgggtggggcccctctttgtactttcgaggctgtttttgcgtctgggtatacgctggtagggctggggtcggacgattccgccggcccgcctcccttccggctgacagctttgcctatcggtgcgatagaaacttagggggaacccttaccttagcactccctctaatcgagtgctaatatgcccaatacaaaggagtttcccctgatgaccatgctgtctggagcctctgccaaccagctcgccgtcgccaatccatggtcgatggtgccgccgctgggcaacctggatgcttatatttcggccgccaaccgcctgccgatgctcacgctcgaagaagagcagggcttcgcacgccgtttgcgcgaccagaacgacctcgaagcggccggtgcgctgatcctctcgcacctgcgcctcgtggtttccatttcccgccagtacctgggctacgggctgccgcacggcgacctgatccaggagggcaatgtcggcctcatgaaggccgtgaagcgtttcgaccccgaccagggcgtgcggctcgtgagctacgccatgcactggatcaaggccgagatccacgagtacatcctgaagaactggcgcatggtcaaggtcgcgacgaccaaggcccagcgcaagctgttcttcaacctgcgctcgatgaagcagggcttcaaggccgattcggccgcggccgacaacggcacgcatcgcgaaacgctgagccccgaagaggtgtcgcaaatggcgacccggctgaacgtcaagcccgaagaagtgctggagatggaaacccgcctgtcgggcggcgacgtgctgctcgatccgggcccgtcggacgacggcgatgaagccttcggcccgatcgcctacctggccgacgccacgcaggaaccgaccgccctgctcgaatcgcagcagcgcgaccggctctcgagcgacggcatcgccaccgcgctcgaagcgctggacgaccgcagccgccgcatagtggaagagcgctggctcaaggtcaacgacgacggctcgggcggcatgacgctgcacgacctggccgcggtgtacggcgtgagcgccgagcgcattcgccagatcgaagtcgcggccatgaagaagatgaagaaggcgctggccgattacgcctgagccctgccgctcttcatccctcaaaaagcccggtcaaccgggctttttcatgcctgtttcgaaagcgttcgcagggcccgtttggcgatgtaccgcgtggccgccgtgtcggattcatcgagccagcgcgtacagagccggtcgacccactccggctgggtcttgctcgcgtcattgagccagttcgccaccgagttctgcacgtagcggttgccgtcggcccgcaaggcctcgatcagcggcaaggcgcgccagggttcggccttgagcgcatcgatctgcgcgcaccacacgccgcgcgggcgcgtgagttcgctggcaaatcggcggatgttcgggtcggcatcggccgtccacggctgcagcagcgccagcgactcgtcgagtgaggcgacgaccgcatcgcgcaccgccatccaggcgatttcgcgcacgccgaagtgcggatcggcggcaaaacgccgcaccgcctccagctgcgccgccagcggcaggcccgacagcgtgacccattgcgcggcccagcaacgcgcggcgtcgctcgcgtgcgtggcaagccggtgggcaacggcatcgcgctcggcatgctgcgccgccaggtcgtaaagcgcgcgtgcaacgtggccgtgccgctgcatcggcttgaacgcgcccagcatggcgagggtgtcggccaggcgttcgctggccggatcgaggccgatgtggcccgccacgctgcgcgcgagctgcggcagttcgagcgccaggaattcgttgaggttgacggtctccagcaagccgtcgttgagcgcgcgcagcacctcgggcggaatgagcgcgatgcggaaggcgcctttgcgcgccttcaggtgatcgacggaagccagggcgacgacggcgtccatgggcgagcgggctgcggccacccgggtcaggtcttgagcagcgccttcacgtccgacaccatgggcgccacgccggcgccatagcgggcgtagagccgcagccggccctgggcgtcgtacacgaagctcgcggccgaatggtccatcgaatagctggtcggggtcttgccctcgaccttcttgaaatagaccttgaagtccttggcggtggtgacgagttggtcggctgagggaatcagcgcgacgaagctcgggtcgaacgcgcccatgtaggccttgagcacttcgggcgtgtcgcgcgccggatcgaccgtgacgaacagcacctgcagcttgtcgccgtcgctgccgagctgctgcttgacctgcgccatttcggtcatggtggtcgggcacacgtcgggacactgggcgtagccgaagaacagcaccaccaccttgcccttgaagtcggccagggtgcggaccttgccgtcggcgtccttcagcgagaagtccttggcgtagtcggcgcccgtgatgtcgaccgcattgaagctgggcctgggctcgctgcaggccgcaacaagccccagcgtggcggcaatgctcgcccatgccgcaccgccggccagtaattgaagggcgtttcgcttgttcatggaagcaggcattcggtcaattcagcgcaggtaatggtcgacgagcaatgccgcgaacagcacgctcaagtgaatcagcgaaaaccggaaggtcttgcgcgccagcgtgtcggagtagttgcgccagagcgcaaaggcatagcccgtgaaaccgatgctcacgcccaccgccaccgccaggtagagccagccgctcatgccgtagatgaaaggcatcaggcaggcggcaaacaggatgaaggtatagagcagcacctgcagtcgcgtgaactcgttgccgtgcgtgacgggcagcatcggcaggccggccttgcggtagtcctcgacgcggtagagcgccagcgcccagaaatgcggcggcgtccacaggaagatgatgaggaacaaaatcagcgcttccggccccacgtcgcccgtcatcgcggcccagcccagcaccggcggcatcgcgcccgaagcgccgccaatcacgatgttctgcggtgtcagcggcttgagaatgacggtgtagatcaccgcataaccgacgaaggtggcaaaagtgagccacatggtgagcgggttgacctggaaccacagcagcgtcgagccggccacgcacagcagggccgaaaacaccagcgcctgcaggtcgctgagctgcccgcgcgccgtggggcgccaggcggtgcgcttcatcttggcgtcgatgcccttctcgaccaggcagttgaacgccgccgccgcccccgccaccagccagatgccgatgcaggccagcacggcgcgctgcacgtcggcccacgagggcaggcccggcacggccagcaccatgccgatgagggcgcagaaaacgatcagctgcaccacgcgcggcttggtcagcgcgtagaactggcgcagcacgttggcggtgcttgtctgctgcacggaaatcggcgtgctcacgcggcggcctccctctggttgttatgtggggcgccgggcgccttgtctctgtcgcgcgcgaccgtggcggccgccccgcggcggctctcgcacagcgcccaggtcagcaccacggccagcgcggcggcgccgccggtgtgcagcaccgcggccacgagcggccagccgagcagcacgttgcccaggccggtggcgagctgcagcagcgccagtcctgcgagccagcgcgcctgcggccgcagcggttcgatgcggcgcagctgccaggcgagcacgcccagcgcggcgaacacggcgtaagccatcagccgatgagcgtagtgaatggcggtgagcgccgaaaagtcgagcggcgcaccgtcaccggtcaggcccagatggcgccagatttcgaagccttgcgcaaaactcatcggcggccaccagctgccctggcaggtcgggaactgggtgcaggccagcacggcatagttggtgctgacccagccgccgagcgcgatctgcagcaggagcagggccgacgtcgcgagcagtccattgcgcagcgccggcgacacggccgtgggcagacggtccgcggcggcctgccggtagcgcaccgcctggatgcacaacagcgccagcagcaccacggcgcccaggaggtgcagcgtgacgatggcgggaaacagcttccaggtcaccgtcagcgcaccgaacgcgccttgcaggcaaacccagaccagcgtgaacgccggccaccaggcgctgagcgtggcgtgctcgccctccgccggcacgggcaggcggcgctggcgccagcgcacgatccaggtggcgcccgcgagcgcgaggatgagcacgccgacgccggtggccaaatagcggtggaccatttcgacccaggccttgctgtgcgtgaccggaccggtcggctgggccgactgcgccatggcgatctcgtggctggcgccgaccgggctcgcgttgccgtagcagcccggccagtcggggcagcccaggcccgaatcggtgagccgcgtgaaagcgccgaacagcgtgaggtcgaaggtgaggaacagcgtcagcacggtgagcgcgtgcagccggcgcgccggcccgccacccgcattgcggcgccacacccacaccagcgggccgagcgcgatcagcacgccggccgccatcagccaggcgatgggggtgaggtcgtagagcgagccggtgtccatcatgcggtctcagcggccaggctcgtcccaggaggcggaggcgcgcagcaggcggtcgaggtcgcgcttggcacggctggcgcccttggcgtccatgcgggccggaaaacgcatcatccagttgcccatggggtcgaccacgaacaggtgctcagccagtccatggcctgctacaggcgcgagccacttggcgagttgctcggcaggcacgcgcagcacggtggcaccatgcaggccgttgtccagccgcggcggaatgggcgccgcgtcgctcacgagccagacgcggtcgagccggtctttctcccggcccaggctttcgcgcaactggcgctgcagatacagctgctgttcgcagagcgcgtcgcaggccgcatcagccaccgcaaccagcagccactgtcccttgagcgtggaaaagtcgaccggcgcgccattgcggtcggtcgcggcaagcacgggcagcgtgcgttgcggatcgatgagttcgccgtaggcgctgcgcccctcgggccggatcacgtagtaggtgaagtacgaggcgatgacgggcgcggcgcacatcagcatcacggcaatcatcttccagcgaccgacgaccgtacggcggccttcggcaccgtcgagcgcctggttgggcgacggcatcgaatgcaccgtcaggcccagcggttcgtcagaggctgcttgcatcgcgtgcgcggcgcctcgagcggcggaagggggcaatgaattgaaaccagacatagaggattaccacgagggccgagagcccgaaccactggaatgcatagccgtagtgcttctccagacccagagcgggggccggccagtcgcgctgcaacccctcggaagcggagccgatctgctgcagcgacacatcggttcgcagcggcagcttggtttcggcgcggaacgcttccaggtcgagattctgccggatgggcgaagaccccgcggattccggtgccgagacggccggcgccggcttgccgagttcgaacaaatggccgggcggcggttcgatcaggcccgtgacttcgacgatgcccggcggggtgtcgaccgcgcccagctgcgtgcggtcattgaaattgcgctgcacccagccgcgctgcaccatcacggcctggtcgctgccttccagggcaaagggcgtcagcacgtagaagcccggcacgccatgcatctgccggttgtccaggtaaacggtttgcgggctcagccagaggccgcgcagccgcaccggccgatgcagttcgccagccggcgcttcgagcgccaggaaatcggcctgggccagcggcggcttctgcttctgcgattcgatctcggcctgcagcgcctccttctgcgccgcgcgcgagagctgccagcggcccagcgacaccgtggcggacacggtcagcacggcggccagcgtgaccagcaggaaacggcctcgcttcggcctcgccctggcggggtgaagaggctctggcgtcactggagcggacgaggcgtgcggccgataatcggagtcatgaaatatttcgtcgccctggctttcgtgggcatcttcgcgagccttgccttcgcgctcttctacatgctgaaagacgggcgcaatggacgcgccaagagcggcggcatggcgcgcgcgctcacctttcggatcggcatctccgtgtttttgttcctctgcatgctgctcgcctggaagttcggctacatccagcccaccgggctcccggtcggcaagtagatggtgctcgttccacgagaaccatgaaaaaggcgcctttcggcgcctttttgtttgcatgccgcggggttcgctcaaagccagtaaaccagcatgtaaaggccgagccacaccacgtcgacgaagtgccagtaccaggccgcgccttcgaagccgaaatggcgttccggcgtgaagtggcccttctgcaggcgcagcgtgatgaacagcagcatcagcatgccgatgaacacgtgcaggccgtggaagccggtcagcatgaagaaggtggagccgtaggcgccggagctgagcttgaggttcaggtcggtgtacaggtggtggtattcgtagccctgcacgcccaggaacagcacgccgagcagcacggtgagccacatgaagcggatggtctgggcacggtggccggcacgcagcgcgtggtgggcaatggtgagcgtgacgcccgagctcagcagcagcgcggtgttgatcgtgggcagccagaacgggccgacggtctggaacggctcgacgatgtcggccggcgagccggtgacgccggcggcaacgctgggccagacggccttgaagtcgggccagagcagcgcgttttcgaggctgccgagcgccggcagcgaatgggtgcgggtccaccacagcgcggtgaagaaagcgccgaagaacatcacttcggagaagatgaaccagctcatgctccaacggaacgagaggtcgatcttgtggccgtactggccgctctcgctctcgccgatggcggtgcggaaccacacgaacagcgtggcgagccatgcgatcatgccggccagcagggaccatgcgccccactggtggccgttgatccattggcccgcgcccagaatcacgaagaacaggccggtcgcggccatgaccgggtaggccgatggccccggcacgaagtagtagggcgtggtgccgtgggtggttgaactcatatcagctcctggctttctttcttctctcgattcgatgggttctggatgtctagcgccgcgtggttcacgcgccgtgcgcaaccacgtagcgcaccagcagcaccaggccgacgatgaaaacgatgaccgccgcaaaagccaccgcgatgatatgcagcggattcagcttggccaggtcgtcctggtaggcgcttttcttgcgcaccccgaagaacgaccagcagacggccttcaccgtgtcccacagcgtggccttgggcggcgtgttcggggcggtcacgaacggggctcatgggcagcattcgaaacggcggccaccggggccgcgggcgtcttgccgcccacctcgaagaaggtgtacgacagcgtgatcgtcttcacgtccttggatatcttggggtcgatcacgaaggccacgggccactgcttcttctcgcccggatcgagcgtgtactggttgaagcagaagcactcgagcttgttgaagtacggcgcggcctgctggggcgcatagcttggaatggcctgcgccgccatgcggcggttctgcacgttctggaactcgtaaatcacggtgttgagctgcccggggtgcacctggatcgtccgttcggcgggcttgaagtcccagagcccgccgcgcacgttggagtcgaactcgaccgtgatggtgcgcgtggtgtcgacctgcgtgttgtcgggcacgcgcacgttcttgccgccgctcgcaccgcccggcacctcgagctcgttgagcgcgaggatgttgatgccggtcatttcgcagatggcgcgatagagcggcaccagggcgtagccgaacgcgaacatgccgcaggtgaccacggccagcttgccgaccatgcggacattggcgcgcttgatgcgttgaccgaggctcatgcgggcggctccgttcgcggctgcttcagcgtccgctgaaccagatcatgcggaccaggaatccgaggaggaacagcacggcgatggaggccagcgtgagccccatgcgtcggttgttccttctttgttcgggcgtggtcattgtggtcatgcgggccggagggcagcaaacgctcagccgatcaccttggtggcggtcgcgtcgagcttgggcgggttctcgaaggtgtggaaaggcgccggcgacggcacttcccactcgaggccttcagcggcttcccaaggcttttgcggtgccttctcgcccttgccgagcatgttcggcagcacgatgaagaagaagaaatagacctgggcaagaccgaatgcgaaggcgccgatcgacgccacggcgttgaagtcggcaaactgcatcgggtagtcggcgtagcggcgcggcatgccggccaggcccagaaagtgcatcgggaagaaggtcacgttgaacgagatcagcgaccaccagaagtggatcttgccgcgcgtttcgtcgtacatcacacccgtccacttgggcgcccagtagtagtagcccgcgaacatggcatagagcgagccggccaccagcacgtagtggaagtgggccaccacatagtaggtgtcctgcagctggatgtcgatcggggcaatggccaggatgaggccggtgaagccgcccatcgtgaacacgaagatgaagccgaccgcaaacagcatcggggtctcgaaggtcatcgagccctgccacatggtggcgatccagttgaagatcttcacggccgtgggcacggcgatcagcatggtcgcgtacatgaagaacagctggcccgtgaccggcatgccggtcgtgaacatgtggtgcgcccagacgatgaacgacaggatcgcgatcgacgaggtggcgtacaccatcgaggcgtagccgaagagccgcttgcgcgagaacgccggcacgatctggctgatgatgccgaaggccggcaagatcatgatgtagacctcggggtggccgaagaaccagaagatgtgctggtacatcaccgggtcgccgccgccggcggggttgaagaagctggtgccgaagtggcggtcggtcagcgtcatggtgatggcgcctgcgagcacgggcatcacggcgatcagcaggtaggcggtgatgagccaggtccagcagaacatcggcatcttcatcagcgtcatgccgggggcgcgcatgttcaggatggtgacgatgatgttgatcgagcccatgatcgacgaggcgcccatgatgtgcatcgcgaagatgccggcgtccatcgaggggcccatctgcagcgtgagcggcgcgtagagcgtccagccggccgccggtgcgccgccgggcatgaagaacgaaccgacgagcatcagcgccgccgggatcagcagccagaagctgaagttgttcatgcgcgcgaacgccatgtcggatgcgccgatctgcagcgggatcatccagttcgcgaagcccacgaacgccggcatgatggcgccgaacaccatgatcaggccgtgcatggtggtgaactggttgaacagctcgggattcaccagttgcaggccgggttggaacagctcggcgcggatcatcagcgcgagcacgccgcccaccatcagcatcgtgaagctgaacagcaggtagagcgtgccgatgtccttgtggttggtggcgaacacccagcggcgccagccggtaggcgctgcgtggtgctcgtcgtgtgcgtggccgtcgtgggcgtgaccgtgggggtcgaggactgcactcatttcgttgttccttgcaatttcttcgtcgcggggcgcttgggctggatcttcacgatcacttgccgcgcaaggccagaacttcggccggctgcaccagctggcccgtcttgttcgaccagctgttcttggtataggtggcgactgccgcgaggtcggtgtcgctcagttgcttccaggagggcatcgcgccattgttctggccgttgagcagcaccagcagctgaatcttgtggtctggatcgaccaccttgggattcgcatcgagcgccttgatcgggcctgcacccttgccgttggcctggtggcaggccgcgcagttggcggcatagaccttctcgccgcgcgtcatcatgtcgggcagggcccagaccttgcccggatcgtcgagcttggccgcggcttccttgcgcttgccatcgacccaggccgtgtagtcggcggccgagaccaccttcacgtggatgggcatgtaggcgtgttccttgccgcagagctcctggcactggccgtagtagtcgcccacggtttcggcgcggaaccaggtgtcgcgcacgaagccgggaaccgcgtcctgcttgatgccgagctgcggcaccgcaaacgcgtggatcacgtcgttggcggtggtgatgatgcggaccttcttctggaccggcaccaccagcgggttgtcgaccttgaagaggtagtcgtcgggcatcgcgcccttggcgccggcgtcggacatggcgcgctgcgagctgtcgagcgtggagatgaaggccaggccctcgccttcgccgttcaggtagtcgtagccccacttccactggtagccggtggtcttgatggtgaggtcggcgttggtggtgtccttctgggccaccagcaccttggtggcgggcagcgccatcacgatcacgatgaggaagggcacgatggtccagatgacctcgaccaccaccgattcatggaagttggccgccttgtggccgaccgacttgcggtgcttccagatcgaatagaacatgaccgcgaacacggcgacgaagatgaccgtgcacaggatcatcatcaccgtgtgcaggaagtgctgttcctgcgcaatcttggtgacaccaagcggaaggttcagctggcgcaccgagggcccgccgggcagatcgttgactgcgtgcgccgcgccgctgaaagccgcgccggccgccagcaacagattcgccggcctgtacttattgcgccaaatgctcttcatcgtgttcacgtttctcaattttttcaacaaacccaaccgtgcagcgccgcgtgagccctcaggcgccacgcaacgccatgcgaatctcgcgcgccagtgcggctcgcaactccgggcgtacatagcgccccaccctgaccgatcgaccctgacccgagacctcgatcagcgaacgatcgccggcctgcggttcgatccgcacctggtgcggtaaaaattccgtgcgctcgtagtctccaccgttctcgagctctaccaccagccgtccgccctgcagcgcgatcctctctccatcggtcgcgtgccgtgcgtacagcatgaacgcgaaacccaccgcagccagctcgagccaggcaaatggcagcaccagcggcgcaccgtgcagccagaagaccgtaccgataccgagcgataccacgcacagcgaggcgtagagccagcccagctggctcggcgtcaccgagcagttccgcttcaggaaccattggatgctctggcctgaaacggtggcaaaacgaaacacggaattcgacacgggcgagttcagcaaatcggtgcgtcgacgaccatccaaccccttgtccccacaggatcggacagacctcgttcgcggaacaacacccgcgagtttcacgcaacggcggattgtagcgggtagacacaggccacaggcggccgcccaccggatgcgcagcttgcgcagcccggcgttcaggcgccgggccggccgcgctggagcatcgagcgcatctcgcgcaacgacaccgcgctctcggccgaaagcgccacgcgcggcgccggcttgaaggcatgcccgtagatgacttcgaaggtcagcgcgatgcgcccgccgccctcttcggccggcgccagttcgggcagcgcatgcttcagcgcctggtgccaagccttgccgcgaagcgccggaaagcgcgccggatgcaggttgcggcccagcgtgcgcagttcggccagtgccgcctcgggcgttgcccaggtaagcacgatgcgttccatgtccatcacgggctcggcgaagccggcatgcaccagcatgtcgccccagtcgtgcatgtcggtgtactcgtggcccgcggccggccagcccaggcgggtgtgcagcgcccgaagctcgcggaccgtgtcggggccgaggcacgagaacatcaggaagccgtccgtcgcgaccaaccggtgccagcgggcgatgagcgcctcggggtcggcggccatgtgcagcgacatgttggcccagagcaggtccacgccgtcttccggcggcgcatcgaagcgcgccttgccgccctgccagcggcgcgcgctccaccagggcgtcgccagtgcctcgctggctgcggcggcaagcgccggctcgggttcgaccacgaagcagccggcctcgcgatagcgcctggccacgagctcgtgcgcctcgaggccgccgcgcaggggcgcccagtcggcccaggtgcggggctgcgccttgatccattggagccggtcttccatgcggcggccgatttcctcgtgcagccagggcgagccggcggtcggcgcgagccggctccagcggtcggccgccgtgggatcgatggtcggcggtcttcttgcggggtcggtggccatggggccgtgagtatattgagcccatgttcagccgttgggccgcccggcctttgacctctcttcttgcacggctgcccagccagtgcgaggtgtgccgcgcctggccgtcgcggcgggtttgcgacgcctgcgtggcccgcttcgcaccgccggccgcacgctgcggaagctgcgccctgcccgttccggacggcgttgtccggtgcggcgaatgcgtgggcgagccgccaccgctggacgcctgccttgcggcatgcagctatgcgtggccgtggcccgactgcatcgcccagttcaaattccgcggcgaggccggctgggccggccccctggccacgctgatgcgcagcgtgccctgggtggaaccggccctggagcagtgcgacaccgtgctgccgatgccgatggcacccgcccggctgcgcgagcgcggcttcaaccaggcggccgaactggcgcgccggctggcgcccgccaagaccgacgcgacgctgctgctgcgcacccgcgacacaccggcgcagatcggcctcgcgcgcgccgagcgccttcgcaacctgcgcggcgccttcgcggtggatccgctgcgcgcgggccagctgcagggctgccgcgtggtgctggtcgacgacgtgatgaccacgggcgcctcgctgttctcggcggccgcggcgctgcggctggccggcgcggcccacgtcacggccgtcgtgttcgcgcgcaccgatccgccgcgttgagcggtgcgcgccgccgcgacaatcggcgcatgttccatatagtcttggtccaccccgaaatcccgccgaacacgggcaacgtgatccgtctcgcggccaacaccggctgcgcgctgcacttggtcgagccgctgggcttctcgatggacgaccgcctgctgcgccgcgccggcctcgactatcacgaatacgccgaggtcaagcgccatgcgagctggcaggccctgctcgacaccgaacagcctgccgccgagcgcatgttcgcactcaccacgcgcggcacgcgcgccgtgcacgacgtgcgcttccagcccagcgactggctggtgttcggttcggagaccagcgggctgccgcctgccgtgcgcgaggccttcgccgagccgcaacgcctgcggctgccgatgcgcgaggggcagcgcagcctgaatctttcgaacgccgtggcagtgaccgtcttcgaggcctggcggcagaacgggttcggctgagcgaacgcgttccagcgccgcggttggctgcaaatatcagcggtagcggcgcaccaccgactcggccacgcaggccggcttggccgcgccttcgagttcgatcgtggcttcccaggtcatctgcaggccgtcgtccgcgatcggctccgccgagagcagcttcatgcgtgcgcgcaggcgcttgcccaccggcacgggcgacatgaagcgcacccggttcagaccgtagttcacgcccatgcgcgactcggccacgtcgaaagcggtttcgtagaagcgcggcagcagcgacagcgtcaggaagccgtgggcgatcggcccgccgaaagggccggccttggcgcgctcgacgtcgacgtggatccactggtggtcgcccgtggcctcggcgaactggttcacctgctcctgcgtgacggtgatccagtcgctcacggcaacttcctggccgacgcaggcggcaagatcctgaagagtctggaatgtctttttggtcatgcggggcattctggtgccaagggcgccggcgcggctgtcgggcttgcgacatgccgggggcccatcagctttccagccattcgcagatcggctgccactgcgccaggtcgcgctggacgcggcccggcgcgatgtcgaacagcgtgagcccgcgcgccgccagctgcacgtagttctgcgtgtcgcgcagttcgcccagcaccggcacgccgaggctagcgatgaactcgttcagccggtcggccgccagggtgcgggcgttcacgcgcatgcccacgaggctgatcctggttttttcggcgcggcgatgctccatcagccggtcgaggaaatcgcgcgtggcgtagatgtcgaagatgctcggctgcagcggcacgatcacccggtcggccagcgccagcacctccttgaagcgccgtccgtgcaggccggccggcgtgtcgagcacggcgtgcgtggtaccgcgcggcggccgcaccacggcactgtcgccggtggcttcccaggtggcgatgggccgcgcctgcggcgggcgcaggccgagccagaggcgcgacgactgctggcggtccacgtcgcccagcatcacggcatggccgcggctcgcaaaatagcccgcaatgttcgtcgcgagtgtcgacttgcccacgccacccttgggattggcgaccagaaccaccggcatgaagttctcctccagaactggaacagccggatggtagtgcctgcctgtccgggcaagagccgatcttgcgctatgttcgcggcatgacgacaacgacatccgccgccggcgcagacggcatctatgtgctcgcggcccatccgcattggcgcgattcccgcgtcaaccggcagctgctggcggccgcgcgcacggtgccaggcgtccaggtgaacgacctgtacggcagctaccccgacttctcgatcgacgtcgaggccgaacaagcccggctcgcaagggccagcctcgtggtgctgctgcacccgatccagtggtactcggcaccgccgctgcaaaagctctggttcgacgacgtgctcagctacggctgggcctatggccacggaggcaccgcgctccagggcaaggactgctggctggtcgccaccaccggcggccccgatgccagctaccacccgcaaagctacaaccgctacttcttcgacgccttcctgccgccctacgagcagaccgccgcgctctgcggcatgcgctttctcccgccgctggtgtttcacggcgcgcgccgcgcgagcgacgccgaggtggcggcgcacgtcgaggtttttgcccagcggctcggcagctatccccagtggccggaactcgaggagctcgacgcctgcgtggcctgccccgttcccgaaaccgatcgcccggcagagcccgacgacgcggacaaggcggcgtccgccgccttccactccgcgacggcccggggcctcgcctccatgtctgccgccaacgaagaaaacgacaacaacgaaaaaggcacggcctgagcatggagcacgcacccgcctggctgacaagcagcctgatctacctgagcgccgccgtcctggtggtgccgctgtccaaggccctgggcctcggctccatcatcggctacctcgtcgccggcatcgccatcggaccgtggggtcttggcctcgtttccagcgtggaagacgtgctgcactttgccgagttcggcgtggtgctgatgctgttcctcgtggggctcgaactcgaacccaagcgcctgtggaacctgcgccggcccatcttcggctggggcgcggcgcaggtgctgagctgcgccgcggtgctgtttgccgtgggctgggccgcgggtgccgaatggcgcgtggcgctggtggcggcgctcggcctcgcactttcgtccacggccatcgcactgcaagtgttcggcgagcgcaacctgctcaggacgccgagcggccaggcgggcttttcgatcctgctgttccaggacgtggcggccatccccatcctcgcgctgctgccgctgctggcgggcgccacggcggccgaacagtcgctcagcgggctcgaccggacactggaagggctgaagatcgtcggcgtgatcgccggcatcatcctcggcggccggttggccttgcgcccgctgctgcgctggatcgcacgcagcgacacgcccgagatcttcaccgccgcgtcgctgctgctggtggtcgccatcgccgcgctgatgcagttcgtgggcctgtcgatggcgctgggcgcctttctggccggcgttctgctggcggaaagcgaataccggcgcgagctcgagaccgacatcgagcccttcaagggcctgctgctcggcctgttcttcatcgccgtgggcatgtcgatcaactttggcgtgctgatcgcgagcccctggctcatggcgatgctggtggtcggcttcatggccatcaagctggcggtgatctacgccctggccaaggccatgggcctcgcctaccaggagcggccggtgttcacgctgctgctggcccagggcggcgagttcgcgttcgtggtgttccaggccgcggggcccgatgtgctgccgcccgagatcacctcgctcctgatcggcgcggtggcactgtcgatgctgctgtcgccgctcgtcctggtgctgctcgacaagttcgtgctgccgcgctacagccgcagcaacggcacgcagatggacgaaatttcggagcagcaggacgccaaggtgctgatctgcggcttcggccgctacggccagatcgtcggccgcatgctgatgtcgcaaggcctgcgcgtcacggtgctcgaccacgacgccgacaccgtcgaaggcctgcgtcagttcggttttcgggtgttctatggcgacgcgacccggctcgatttgctgcgcaccgccggcgccggcacggccaaggccatcgtggtggcggtggacgacatcgagcagtcgctcgagatcgtcgatctcgtgaaggagcactttccgcaggcccgcatcatcgcgcgggcccgcaacgtgacccacctcttccagctgcgcgaccgcggcgtgacggatgtcgaacgcgaggtgttcgaatcgtcgctgcgcagcgcccgctcgacgctcgaagcgctgggctggccggcgcacgaagcgcgcgaaacggcgctgcggttccgccgccggaacctcaagctgagcgacgagatctatccgcactacaaggaccgcgccaagctgatcgccgccaacaaggcgggccgccagcaattcgaggagcagatggcgcgcgaacgcgaagagcggcagcggcgctcgggccgcgattgggaccggctcgacgaaaaggaagaggcggacgcgtagcagcccgccctcttcgtcagccttccagcttcagcagcctgaccgcgttgcctttcaggatgcccggcatcacctcgggcttgaacccggccgcctcgaagtccttcatccagcggtcgggcgtgatcagcgggtagtcgctgccgaacaggatgcggtccttcagcagcgtgttggcgtactgcaccagctgcttcggaaaatacttggggctccagcccgacaggtcgatccacacgttgggcttgtgcgtggccacgctcagcgcctcgtcctgccaggggaagctggggtgcgccatcacgatctgcatgtccgggaagtcgatggccacgtcgtccagatgcatcgggttgctgtattccagcctgaggccgccgccgcagcgcatgcccgagccgatgccgctgtggccggtgtggaagatggccggcagcttgtgctcggcaatcacctcgtagatcggccaggccatcttgtcgtaggggtggaaagcctgcaccgtcgggtggaacttgaagcccttcacgccgtgctcctcgatgagccggcgcgcctcgcgtgcgcccatctttcccttgtgcggatcgatgctcgcgaaggcgatcatcatgtcgctgttctgcttggcggcctcggcgatttcctcgttcggaatgcgccggcggcccatgttcgattcggcgtcgaccatgaacatcaccaggccgattttgcgctcgcggtagtaggccacgctctcggcaatggtcggccgcccgctagagccgaagtatttgtccgcggcgcggtcgtattcctcgccgtagttgtcgaacgggttccagcagctcacttcggcgtgggtgtggatgtcgatggcgatcaggttctggtggtccatgtcgttgtctccagtacgggtaagtccctaggaattggggcgctcaagtgccttgaattgattatttatcataaccataatccaactcacacacgaatgcaatcatgaccaatcccgatctccatctcgacatccgcgacgaagttgccatcgttcgcctgacgcgcggcgccaagcgcaacgcgctttcggacagcctggtcctcgcgctgcgcaacaccttcgagaccctgccgtccacggtgcgcgccgcggtgctcgacggcgaaggcccgcacttctgcgccggcctcgacctgagcgagctgaaagagcgcgacgcgggccagggcatgcagcattcgcggctgtggcacagcgccctcgacctgatccagcacggcccggtgccggtgatcgcggcgctgcacggcgcggtggtcggcggcggcctcgaactggcaagcgcctgccacatccgcgtggccgaccgcagcaccttctatgcgctgcccgaaggctcgcgcggcatcttcgtgggcggtggcggctcggtgcgcattcccaagctgatcggcgtggcccgcatgaccgacatgatgatgaccggccgtgtctacaacgccgaagacggcgagcgcgccaacttcgcgcagtacctggtcgacgagggcacggccttcgacaaggccttcgagctggccaagcgcgtggccaccaacgcgccgctgaccaactatgcactgatgcacgcgctgccgcgcattgccgagcagtcggccgaccacggcttcttcaccgaggcgctgatgtccggcatcgtgcagaacgcgcccgaggccaaggagcgcgtgcgcgatttcctcgaaggccgcggcgcgaaggtgagcaagggatgaccacgatccgataccgtccgctggcgttcggcgtcacgcgcgccgtgctgcgcgacggcgcgccgggcacgcagtacctgcgggccgaaacaccgctcgcgccctaccgcgaccgcatgaccgaccgcctggcgcactgggccgaagcggcacccgaccgcaccttcatcgcccgccgtgaacggctggccgacggcagcaccggcgactggcagcgcgtgagctacgccgaggcactgcagaaggcgcgcagcatcggccaggcgctgctcgaccgcggcctggatgcggagcgcccggtcgcgatcctcagcgaaaacggtatcgaacacgcgctgatggcgctcggctgcctgtatgccggcgtaccgtactgcccggtgtcgccgccctactcggtggtgagccaggacttcgagaaactgcgccacgtgctggacacgctcacgcccggcctggtgtttgccgccgacgccgcgcgcttcggccgcgccattgccgcggcggtgcctgcggaaaccgaagtcgtcatcgccgaaggcaccatcgaaggccgcgccgccacgccgttcgacacgctggccgccacgcccgcaacacccgccatcgatgccgcgatgcgcgccagcggccccgacaccatcaccaagtttctcttcacctcgggctccaccaagatgcccaaggcggtgatcaacacgcaccgcatgtggtgcgccaaccagcagcagctgcgccagtcgattcccgctttgggcgaggagccgccggtgctggtcgactggctgccctggaaccacaccttcggcggcaaccacaacgtgggcatcgtgctggacaacggcggcacgctttacatcgacgacggcaagccgacgccctcgggcatggccgagaccctccgcaacctgcgcgagattgctcccaccatctacttcaacgtgccgaccggcttcgaggccatcgcgcacgccatggagaccgacgcggtgctgcgccgcaacctgctgtcgcgcgtgaagatgttcttctattcaggtgccgcgctgtcgcagcccgtgtgggacagcctgcacaagacgcaggaggccgagatcggcgaacgcatcgtcatgggcaccggcctgggcatgaccgagtccggccccttcgctctctatgtcaccgggcccgaggtgaagtcgggcgacgtgggcctgcccgcggccggcatcgagctcaagctgatcgaggtcgacggcaagaccgaggtgcgctaccgcggccccaacatcacgcccggctactggcgcgcacccgaggccacggccgaagccttcgacgaagagggcttcttctccaccggcgatgcggtgaagtggatcgacgacaacaacatccaccgcggcctgcgcttcgacggccgcattgccgaagacttcaagctcgccaccggcaccttcgtgagcgtgggtccgctgcgcgccaagatcatcacggccggcgcaccctacgtgcaggacgcggtgctgaccggcatcaacctgaaggaagtcggcgcgctggtcttcccgacgcagaaggtgcgacagctggccggcctgccggccgatgcaacgatgcagcaggtgctcgaaagtgcaccggtacaggcgcacttccagcaggtggccaacgaactggcggccatgggcaccggcagcgccaatcgcatcgcgcggctgcacctgatggccgagccgccttcgatcgacaagggcgaagtgaccgacaagggctccatcaaccagcgcgccgtgctcaagcaccgcgccgagatcgtcgaggcgctgcacgccgacaccctgcccttcaccctgaagccccgctgattcatccaggaaaccacacaccatgaagatcgaaggacaagccgcactcgtcaccggcggcgcatcgggcctcggcgaagccaccgcgcgcgaactcgcgcgcctgggcgccaaggtggcggtgctcgaccgcaacgcggcgctcgccgagaaagtcgccgccgagatcggcggcgtcgcttgcgcctgcgacatcaccgacaccgagagcgtcaatgccgcgctcgacaaggccgctgcagcccacggccccgcgcgcatcctgatgaacgtggcgggcatcggcagcgcgaagcgcatcgtcggcaaggatggcaacccggcgccgctcgaagacttcgtgcgcgtggtcaacatcaacctgatcggcggctacaacatggcgcgcctgttcgcggcgcgctgtgccaagctcgacgcgctcgacaacggcgagaagggcgtgatgctcttcaccgcctcggtcgcggccttcgacggccaggtgggccagcaggcctacagcgcctccaagggcggcctggtcggcatgacgctgccgatggcgcgcgatctggcgcagcacgcgattcgcgtgtgcaccgtggcgcccggcctctttgccacgccgcttttgatggaactgcccgaagccgtgcagcaatcgctggccgcgtcgattccgtttccgccgcgcctgggcaagccttcggagtttgccgagctggcctgccacatcgtgaccaacgggcatttgaacggcgaggtgatccgactcgacggcgccctgcgcatggcgccgcgctgattcagtttcagccccaacaaccaggagacaagaccatgaccaacagacgtgaattcgtgaaggccctcggcggcgcagccgcactcggcgccctgtatccgctcggcgcactcgcccaagccgtgcagcaggccaagatctactacggctttccggccggcagcgcaggcgacagcgtggcgcgccgcgtggccgaaaagctcggcgacacgccgtattcgaagatcaacgcagtggtcgagaacaagcccggcgcgggcgggcgcattgcgctcgacacgctcaagacctcgccggctgacggctcggtgctgtgtctcgcgcaggcctccgcgctgtcgacctacccgcacatctacagcaagctcagctacggcatcgccgatttcgcgcccatttcgatcggcgccgtgatgacgcacggcctcgcggtcgggccgatggtgccggccagcgtgaagacgctgaaagactacatcgcctgggccaaggccaaccccggccaggccagctacggctcgccgggcgcgggctccacgccgcacttcctgggtgcgctgctgggcctgaacagcggcaccgacctgcgccatgttccctaccgcggctcgctgccggccatcaacgacgtggtgggcgggcagatcgcctccagcatgacgccggtgggcgactacctgccctttgccaaggccggcaagctgcgcgtgctcgccacctcgggcgcgcaacgcaccgcctacatgcccgacgtgcccaccttcaccgagcagggcttcccggaaatcgtggccgacgaatggttcggcttcttcgcgccagccaagacgcctgccaatgtgattgcggcggcgagcacagcgatccaggccgcgctcaaggacaagaccgtggccgagggcctgctctcggtcgggctgatcgcccacggctcctcgcccgaggacatgaagaaatcgctccaggccgaatacgagcgctggggtccgctggtcaagaagatcggcttcaccgccgagtcctgatacaccgatggattaccggccccgccccgaagaccaccgattcatcctgaacgcggtgctcgacgcaccgtcgacgctgcgcacgctcgcgcccttcgcggaggtcgacgaggcgctgcagggccaggtgctcgatgaagcggcccgcttcgtggccgaggcggtggcgccgtcgaaccgcgacggggacgagatcggctgccgtttcagccagggcgaggtcaccacgccgccgggcttccgcgaggcctaccaggcttttgtcgatggcggctggcccggcttgtcggccgcaccggaagacggcggccagggcctgccgaccgtgctcgaagccatcctctacgaatggctgagcgcggccaaccacggtctcaccatggcgccggggctgttgcacggcgcctatgcctgcctcaagcaccacggcagcgacgagttgcgcgcgcgctatctaccgaagatcgcatcaggcgaatggctcgccaccatgtgcctcaccgaagcccacgcgggcagcgacctgggccaggtgcgcacgcgcgccgtgccgcaggccgacggcagcctgcgcgtgagcggcggcaagatcttcatctccggcggcgaacacgacctgacgccgaacatcgtgcacctggtgctttgccggctgcccgatgcgcccgcggggcccaagggcctgtcgctggtgttggttcccaagctgctgcccgatgacgcgcgcaacgcggtgcactgcgagcgcatcgaggaaaaaatgggcctgcatggcagcccgacctgcgtcatgcgcttcgacgaagccaccggctggctggtcggcgagccgggccgcggcctggccgcgatgttcgtgatgatgaatgcggcgcgcctgcacgtggcgttgcagggcatcggcctgctcgacgctgcctggcagaaggccgacgcctacgcgatggagcgccgccagatgcgggcgcccggcgccgtgccggccagccgcggcggcgaggcggcggacctcatcgccgaacaccccgcgatccgccgcattctcgatacccagcgcgcctgggtcgagggcgcgcgcacgctcgcctaccgcagcgcgctgatgctcgacgtggccgcgcacgacgccgatcccaaggcgcgcgaacgcgcgcagcgctggtgctcgctggtcactccggttctgaaggccgcctgcacgcaccaggcctttcatggcgcgagcgaatgcctccaggtgttcggcggccacggctacgtgcgcgaatggggcatcgagcagatcgtgcgcgacgcacgcgtgacgatgatctacgagggcaccaacgagatccaggccatcgacctgctggtgcgaaaggtactgcccgacaacggcgccggcatgtcagcggtgctgctcgaactgcgcgacacgctcgatgcctcgcgcgaggccgacgccgacgtgcagcgccggctcgcgcagctgcgctacctgggcaccaccatcgcgatggccgcgcatgccaacccggtgctgccatatgaagtggccgacgactacctgcgcgtggtgatgctcacgatgatggcctgggcttgggcgcgcatcgacgcggcgcaagcctcggaggccgagcgtgccgcccgggcaggcccggcggcggccttccggcgctgggtgctgcccgaattcgacatgcggctgggcatcgtcaagcgcgcctgcgaaggtgttgccatgtcgcacgacgccgcaaaatcaccggttgccggcagttaaccgatacacccgcgcggcccggcgcggttacgcttgggaccatgcctcgcccatccaagaacagttctgccaaagcagcgccgccagcggctgccagcaacaagtccgatcggctcgatgcccgtgtgctggaagccctggtcggctacaacgcgcgccgcgcctggctgatcatcacgggggtgtttgccgaacgcatggcgccgtacggtctcaagcagatcgatttctcggtgctctcgctgctggcgcacaacccgggcgccacctcgcgccagctctgcaacacgctcgacatcctgccgcccaacctggtgagcctggtcgccacgctcgacagccgcgggctcatcgagcgccggccacacccgcatgatggccgcgcggtgggactgcatctcaccgaggcgggcgaaaagctgatcggggaggccgagcagacggtcacgcagctcgaggccgatgccagcgcgcggctcacgtcgcgcgagcgcgaaaccctgatccggctgctgcagaagatctatctctagcctcggccctcctggttagaggccgcgctccaccatgtcgatcaggcgctgccccagcgcatgggtggcttctgcatccatgtctctcagcggcccttcgatgatcagcagcgccagcccatgcacggccgaccaggccaagtattcagcgttcggtcgccgcgaagggtcgagcgcacccgcatccacgagccggtcgatcgcgctgccaagcaactcgaacgggtccatgccactcgaccccgcgcgccccggccccacctcgccttgggcgtcttccgacgacacgagaaaagccgttttgaacaaccccggctcggcctgcgcaaaacgcaggtaggcggtgccgatggcccgcacccgcgcccgcgcgaagtcggcgggcggctggtcgcagggcagcaccgccagttctttttccatggccgtggcggccgccgacaacgccgcggcgcgcaccgccagcagcagctcgcgccggcttgcgaaatgccggtacgccgcgttgggcaccacgcccgcacgccgcgtcacttcgcgcagcgccaccgcatcggggccgccgtcgcgagccagttcgatgcccgcgtcgagcagcgcgcggcgcaggtcgccgtggcgatacgtgctgcgggcggcgggcgcgctggggtctggcggaacgatgcgggggctcatcaggtatctccatgtggacagtgtccattatgtctgctattctttgtggacggtgtacacaaactagtaattccgtatgcgcgcaggtctctgcgcatcctttcatcctcagtccaaaggaaacaccatgaaagtccagtcctatctctcgttcgaaggccgctgcgacgaagcgctcgcgttctacaagaaggcgctcggtgccgaagtcgtccaactcatgcgctacagcgaagcgccggcggaagccccttcggacaacgcggatgccagctgcggcggcgccacgcccagccccgacaaagtgatgcacgccgtgctccgcatcggcgaaaccgagctgatggcctccgacggccggtgctcgggccagccggagttcaaggggatcatgctcgcgctcaccgccagcaccgacgccgatgcccgcaagtggttcgacgccctggccgagggcggccaggtgatgcagccgctgatcccgaccttcttcacctccagcttcggcatgctcggcgaccgtttcggcgtgggctggctgctggtggtggcgcccgccaactgaccttcaaccgaccgcccgacacccttgcctccggagtacctccttcatgctcaagaaaattgccctcgtcatcctcgccctgatcgccgtgctgctcatctacggcgcgacacggcccgacaccttccgcgtggaacgcacgatgcgcatccaggcgccggctgcgaagatctttccgctgatcgacgatttccaccgctggggcgcctggtcgccctacgagaagctggaccccggcatgaagcgcgccttcggcggcgcgcccgcgggcaagggcgcgacctacgcctgggaaggcaacgacaaggccggtgcgggccgcatggaaatcaccgattcgacgccctcctcgaagatcgcgatcaagctcgacttcatcaagcccttcgaaggccacaacgtggccgagttcacgctgcagccgcagggcgacgccacgcaggtcacctgggccatgcacggcccgagcccctacgtcgcgaagctcatgggcatcttcttcaacatggaccagatgatcggcaaggacttcgaagcaggtctcgccaatctcaagacggccaccgaaaagtaacccccgaaaggaaacatcatgtctcccatcaacgcttacctcacgttcgacggcaacgctgcagaggccatgcgcttctatgaaaaaacgctcggtggcaccatgcagatgatgatgaccatgggcgaagcccctggcgccgagcagtttccgcctggcgccgaaaagcgcatcatgcatgcggcactggcttacggcgacggcatgctgatggcctcggacaccatgcccggccaaccctacgaaggcatgaagggcttcggcgtggcgctgacgatcgagaccgtagcggaagcgaagcgcgtgttcgacgctttcgccgacggcggcaaggtcacgatgcccttcgacaagaccttctgggtcgaaggcttcggcatggtgaccgaccgcttcggcacgccctggctcatcaacgggggcaagccgctggtctgaccccgcccgtctgattcgcaacctgcaggaatcgctcttcatgaccgacacactcgacaacaaccggaagcgctggctcgcattgatggtgctgtgcctcggcgtgctgatgatcgtgctcgacaccacgatcgtgaacgtcgcgctgccctcgatccgaaccgacctgggcttcaccgagacctcgctggtctgggtggtgaatgcctacatgctgaccttcggcggcttcctgctgctgggcgggcggctgggcgacctgtacggccaccgcaagatcttcttgatcggcctcgtgctgttcacgctcgcctcgctggcctgcggcgttgccaactcgcaggccctgctggtcgcggcacgcgctgtgcaggggctgggcggcgcagtggtctcggcggtggcgctctcgctgatcatgaacatcttcaccgagccggccgaccgtgccaaggcgatgggcgtctacggcttcgtctgcgcgggcggtggcagcatcggcgtgctgctgggcgggctgctcacgagcacgctgagctggcactggatctttctggtcaacctgccaatcggcgtggcggtgtatgcgctgtgcatcgcgctgctgccgtcggcgcgcggccatgcccatggcgagaagctcgacgtggccggcgcggtggccgtcacgctgtcgctgatgctcgcggtgtatgccatcgtcaacggcaacgaagccggctggcagtccacgcagacgctcgggctgctgggcgctgcggcggtgctgatggtgctcttcatcgtgatcgaggccagggtggcgcatccgctgatgccactgggcttgttccggctgcgcagcgtttccgtctccaacgtggtgggcgtgctctgggccgcggccatgttcgcgtggttcttcatttccgcgctctacatgcaactggtgctgggctacacgccgatgcagatcggcctggcgttcctgccggccaacctgatcatggcggtgttctcgctgggcgtgtcggccaggctggtgatgcgcttcggcatccgcaagccgttgtccatcgggctctggctcgcggccatcgggctcgcgctgttcgcgcgggccccggtgaacggcagcttcgcgatcgacgtgctgcccggcatgctgctgctcggcctgggcgccggcatggcgctgaacccgctgctgctcgcggccatgagcgaggtgagccccaccgaatcgggcctggcctccggcgttgtcaacacggccttcatgatgggcggcgcgctgggcctggcggtgctggccagcgccgccgccgcacgcaccgcctcgatggaggcggccggtgcgcagctggcgctcgcgctcgccggtggctacaacctcgcgtttctcatcggtgccgtgttcgcggccgtggcgggattgctcggggccgtgctgcttcgcactgcaggcaacaaaggggccgcgtcatccgctggcacggaaaaccgtgcggcggcatcctgaaggtttgcctggccggcagccgcttttcttgtttttctttccgtttctttcaaggagacttccaatggctcgttatgtcgatggcttcctcgttcccattcccgcgaacaacgtcgaggcctaccgcaagctggcacgcaaggccggcaagatctggatggaatacggcgcgctcgaatacgtggagtgcattggcgacgatgtgaagcccggcaagctcacctcgtttccgcaagccgtgaagcagaaggccgacgaaacggtagcgttctcgtggatcgtctacaagtcgcgcaagcaccgcgacgcggtcaacgccaaggtcatggccgatccgcgcattgccgcgatggatccgaagaccatgcccttcgatgcgaagcggatgatcttcggcggcttcaaatccattgtcgagttctgagctcgccggcctcaggccaggaagccgtcatagacgagcttgaggcccgtgagcagcatgcccaggtacacgaagcgatagaaccacgtcgcattgatgcgccgggcaatgcgaatgcccacccatacgcccagcggcgccagcggcatcagcaccagcgaggtggccatggtgcgaaagtcgatcaggccaagccaggcgtagggaatccatttgctcaggttcaccacgaagaagaaatacgccatcgtggcggtgaacaccaccggcttgagccgcagcggaatcacgtaggcgttgaccggcggaccgccggcgtgggcgatgaagctcgtgaagcccgacaccgccgtgagcgccgcgcccactgcgcgcgaaggcagcgggtcgtcgggcttgggcggaaacaccagccgctgggccagaaacagcaaggtgaacacgccgacgatgcccgccacggtgtgggccgagagcgtgcggaacagcagcgtgccgatcacggtgccgagcagcccgaacggaatcaggaacttgagcagcgcgcggtcgaagtcgttccggaaagccgccaggccgagcaggtccatcaacagcagcagcggcatcaggatggccgccgcctgcggcaccgtgaccgccagcgccatcagcggcaccgcgagcgaaccgaagccggcgccgaaaccgctcttgctgatgccgagcagcagcacagcgggaatggcgaccgcatagaaatgcggatcggtgatgaggggaaagaccatggagaaagaggcggcgcaggcagaaaaaagcccaccgtgtccgtggcgggccgcccgagcgtagcaggatggcgcgggctctgctggcggtcccgcccgacaggccgcgttctccaaaactgtgcgtaaacgcacataccggccgccggggtctccgcacactggaaccgcaaccgtcgcactcccgcggcgacccctccactttccaaggatccgccatgaacaaccaggccgtagccgcccactccgcgcgtgcgccgatcgcaccggcacaggcttcctccctctccccagctacgctggacgactccggcaagctgctgctgcgcgtggtcattggcgtgctcgtgctgctgcacggcatcttcaagatctcggccggcgtcggcttcgtgagcgccatgctggtcaaggccggcctgccgggcgggctcgcctacctggtgtacgtgggcgaaatcgtcgcgccgctgctcatgatcgccggcttctggacccgcgccgccgccggcgtggtcgtcatcaacatgctcgcggcctttggcctggtgcacatggccgacctgttcgcaatgaccaagcaaggcggctgggcgctcgaactgcagggcctgtacctgttcggcgcgctcaccgtggtgctgctgggcgcgggccgcttcagcctcggcggtcttcgcggccgctggaactgatccggctcagccggcgtcgcctctgacctgcgagaccatgcgctcgaggcgggcggcgtcggccaccagcagggccttgccgtccttctgcaacacaccgctgcgcaccagcacgttcagttcgcgggtcacctgctcgcggttggtgctgatctggctggcaagggccgcgtgcttcggcgccggctccagccgcgcctgattgccctccacgccggtcgcgcgcgcaaggcgcagcagttcggcatgcagccggttctgtacgccgagcgtgctcaggtcgatcacgcgttcggaaagctgccgcaccagtgaagccagccgccgcatcacgcgctcggccaccacgggctcctcgcgcagcagggccatgaaggcggtcctgtccaggctggcgagcacgctgggttccagcgtgaccacgtcggccgaacgcggcccgccgtcgatggcggcaatgtcgccaaagtgttcgccggcctccgaatccctgaaagtgacctgccgcccgttggccgaataggtggtcacccgcacccggcccgacaccagcaggaacacgtcgccctgctgctcggcgcgcagcagcagcggcgtgccggcctccacgctgtgccacaggcactgctgcgccagcaggtccaggcgctggtcggagaggccttcgagcagcgcgatgcggcgcagcgcgaggctggagcgaagggtagtgggagatggggccatgcgggtcggtaagggcgcgcgcattatgctcgggtgccgcttcgaacccgttcatggacagacgctccccccacgcccctttttcgctgagaccgccgacacggcgcaatctccgctgggtgagcgggctggtgctgatgggctatgtcacggcgcacctgctgaaccattcgctggggatcttctcctttgcggcggctgaaaccgtgctgcgcggcgtgcagcagttctggcacagcctgccggggacgctgctgctgtacggcgcggctctcacgcacctcgcgctggccgtcgtcgccctgtgggaacggcggaccctgcgcatgccgccgctcgagggcctgcgcgtgctgctgggttttgcgctgccgctgctgctggccacgcacctgacggccatgcgcggcgcctatctcgcctacggtatcgagggctcctacgttcgtgtcgtctgggggctgtggaacctgccgggcgccagcgcgcagttcgccttgatgctcgcggcctggagccacggctgcctgggggtgcacttcgcgttgcgggcgcggcccggctaccgccgcttctcctatctgctgcttgcttttgcggtgatgttgccgctcacggcggcgatgggcttcgtctcgatggggcgcgagttccagtggaccggcgtgccccccgccgtgttgccgacgcccgaacaaggcaaggcactcaaggcggccgagggctgcatcaagtggttctacggcctggcgctgctcgccttgctggtggcccgctggggacgcaacgggttcgcgcgctggtctcgccagccgtccatcgccctgcgctaccccggccggacggtgcatgtgccacgcggctggagcgtgctggaagcgagccgctcgcatggcattgcgcacctgtcggtctgtggcgggcgggcgcgatgttcgacctgccgggtgcgcgtgctcggcccgtcggaacacacggacgcgccgggccgcgacgagcagcgaacgctcgaacgcgtgcgcgcgccgggcgacgtgcggctcgcctgccagctgcgcccgcgaggcgacatcgaggtcacgccgctgtttgcgccgccaccccacggggggcgcccggcgccggtcagcagcttcggccgcgaacgcgacgtggccattctgttcgtggacctgcggcgctggtcgggattgtcggagcggcaatggccgttcgacctggcctatgtgctcgaccgctacttcgccaccgtgggtgcggccgtgcgcgaaagcggcggcgtgccgaaccagttcatcggcgatagcgtgatggcgatcttcgggctcgaaaccgacctgcccaccgcatgccgccaggcgctgcgcgccaccgaactcatcagccagcgcatggatgcgtggagcgaaagcttcgaagcccagttcgggcaacggctggacttcggcatgggcctgcatgccggtcgcgccgcggtgggcgaagtgggttatctcgacaccaccaccttcaccgccatcggcgaagtggtcaacaccgcgagccggctccaggaccacgccaagacggccgcatcgcgactggtggtctcactgttcgcagcgcagcaggccggccttgcgcacacgatggaacaggtcgacatgctgaccgtgcgtggccgctcggaacccctggcggtgatctgttcgcagcctggatcgcccccgcgccctctttcgtgagcaagacgggggctgcgttcagccggcgggccgggccgtgatggtggccgcgcctggcgctttcgagatgtcgtagcgcacgggcagaaagcgctcgatcaccgcgcagttggtgcgcgtgtgctcggtcacttcgctgcacgtgaaggtgccggcgcggccgctttgccatgcggccaggcccagcagcagcgccaactgatcggccaggtgcggccccacggccgcctggcccttctggaactcgcgcagctctttcaccagcgcatgcgccacctgctcggcgctcagcgtcttttcgccgaaggccgtgaagacctcggtgacgtgttcgtaggccagcgtggcgagcagcgcattgcccggcccctcgttctgccgcgccgctcctgtgcgcagctgatcgcccgaccatcccatggcctggcccagcgtttcgagttcgcgcgttgccacgtgccgcgcaagccccggcgccaggcactccgcgtggcccgacagcagcgcgccgcgcgcaacgagatcgaagggccgcagcccgtccgccgcgggcacgatggtcgcttccacttcgccgccgccggcggggtagaaaccgcagcggcgcagcgtcagttgcaggtccgcgcccaggcggcgcaccagcggcgcgaaggcgcgctccagaaaatggaaaggcggcgccatcgggttgtgcgtaccgccgcgcaggtgcaactggctcggtgcgccggccagcagcagcggcggcagcaccgtttgcagaaccagcatgcagctgcccgcgctggcaatcgtgaagcggtactcgcccgcgcgcaccggccggggcacgaagcgcagcgattgcgacccgagctcagcgccttcgaactgcgcattgctgatttcggcagcggcgttgacgcacgcgaggtgctgacgcatcaagcccggcttggcgcggcccgcgcgaatgttgtcgatggcgatgggctggcccgttgccaccgacagggccaggctggtgcgcaggatctggccgccgccttcgccttgggagccgtcgagttcgatcatgggcggcctccttcgtttgcggcagacactgcagcgtcgaagcgcagcaccgtctcgcaaaggaacgcatcgagccccgcttgctcggcctgcggcagcggcgtcaccggctcggccgcattggccgccagctcggtctcgatgaacgcatggatgccgggccagcgcgggctggtcgcggcttcgccggcgcgcatcttcacctcgagcagcgcgttgatctcgtcgatcagcgcggcatcgcgaaccgcgtcgagcgtcttctgcgccaggtcggcgaagcgcatcggcggcacgccgggctgcgtgcggatccagcgcgcggccagcagcgggcgcagcacgtagaggtatttcttgtagcgcacctcgtcggcttgaagatgctcgcggaagttcttcttcgccatcgagctgtagtgatgccagccgcgcgcgttggaaaacaccgcttccgacagcgcgcggaagcgcggcatcgcgaccgcatcctcgcggtacacgatgggcgagcgcagccattcgagcagcgtggggttcgactcgcgcatcaggcccagcgccttgcgcaggtcccagccgttgacgtcgagatcgccgctgatcggcacctcgatcacgtcgcggcgctccgtcaccgtgagataccacggcaggcggttgacgtagatgaagcgcacgtcgtagtcgctgtcgggcgaggcgaaaccccagccgcggctgccggattcgcaggcgaagagcacggtcacgtcgtggcgggcttcgatgtcgcgcaggttctccatgacctgcacgcgcatggcggggtcgatgggatgggcggagcggaggaattcttgagtcgtcatgaaaatagtcttggcgcctgattgttcatttcttcaggcgcgggtcacagtcactttgccagtgctgtcgagttcgaacacatccaggtcgttggccaggaatgcgttgccgcggtagtgggcctgggtctccgccatcagtgccgccatgccctctgctttctggtggcgtgggctcaggtgcgtgagcaccaggttgggcacctgggccgattgcgcaaactcggccagcaggcgcgccgaactgtgcatgggcccgggcccgaccttgtcgagcacttcttgcgtgtaggtggcctcgtgcaccagcagctgcgcgccctggcaggcggcgtgcagcaacgcgggctcggcgttgtcgccccccagcacggcgctggccgtgtcgatctgcgtctccacaaaatcggcgctgcgcagcacccctgcgttgaaaggcacgtcctcgccgttctgcagcgcgcgccatgcgggtcccgccggcaggccggccgcacgcagggcgtcggccttcagccgcgcgcgcagggtttccacctgcacacggtaggcatggctcggcacgcggtgccgcagcacgtggcgctcgatgctgacgcccggtgcttcgtacacgagcgcctgggattcgatatccacatgctcgacctcgtaaggcagatgcaggtcggtcaagcggcgcgtggcctcgaaccactcccacaccggcagcggcgcgatcagcttcagaggcttgctgcgcttgcccatgccggcgcttgcaagcaggcccggcaggccatagcaatggtcgccgtgcacatgcgtgatgcagacggccgccatgtcgtgcagcgagagcgacgtttgctgcagccggtgctgcgtgccttcgccgcaatcgatgagaaaccagtcggcgccgagcacggtttgcaccgcaaggccggacacgttgcgctggcgcgttggcgtgcccgaggacgttcccaggaaagtgagcttcagcattctcgattcgcctccgcatggcgtgccagggcttttgccgcggcgttggccgcttcatattcccagcttccgtaactgcttccacgatctgccgcgaacgcctgcagccgttcgatctgctcggggccgccccaccggcccatgacttcgatggcaaccacgcgcaggctgcgccacttgctctgcaaggcggcctccacctgcgccagcgagccggcggtcggcttctccgttgccaatgcgcgcagccgggccacctcgtcgcccagcaggttggcaccttcgtttcgaagcgccgcatcgcgcagcgcgcggcgggcctgccggcacgcacggcaccgaacggcctggctgtacaccgagccttgcgcaacctcgtgccaccacttctgctgcttggccgtccacacctcttgtgagccgcaatcgcggcaggtgtaggcctgatcgagatagaagtccggcacttcgccgaaggtggtgttgtagtgcgcgaggcgtgacttgtcggccatggccatgcccggcacgagtccgcctgccgacagctgccgggcgtcctgcgttcgcagcttcgccttgaggtcgacggcgcgttcgaggcgacgggccttgatttcggtgcgccgctgtttgttgcttttcatgatggcagtgtcgtgttgttcagatcacgcgaaaggcgcgcaggtggtactcgacctctttcgggaagccgtacggcaaaaggccggacggcctgtttgcaggcagcaattcgaacctgcggctccacagtgcagccaggctggcggcccggtcttgtcgcggctggacatagctgttggccatggccttcccccatgcatcgagctcgatattgatcgcattgcgaagcttgcccgaaggcggttcgccatccagcagcttcatgacgaagagcaggcgatcccatggcgacccgctgccgagcatggcaatgacatccatcgcaagctcccggcgttcgagtcccatgcgcatcagcgcatccgggctcggcaaaggcgcgccgcgccggatgtgatcgattgcgaggcgccgcatctttggcgaaggctcggccgccagtgccatcagttgctcatcgagctcatcgccttgcgccgcggcgagcatcagccaccgcgccaggcgccgcaacggcactgcgggcgactgcgccatcgaacgggcaagaacaatcgcctgcggatcctcgagcaggtgcagcacatgaagcgcggacacggtccaccgcgcttcgcacccgggcctgtccaggatctccttggcgcgcgcggatatctcgtcacgctccgcggccaatgcgcccaccgccagcgaacgcaccgcagcgctcgtgtcgaagcacatgccgcgaagaagtggcctcgcgtcatgcgcctgcaggctcagcagctcacgcaacgccatcatgcgcacacggggcagccgcgaacggctggccgattcgaataccgcacggcggcttgcgagcgcctgcagccggtcggccgcattcaggcaaagcaacgcggtcagcagatcgttcgaacgcacagcccggcacagcaggtcctgcagcgccggctggtcgtgcgttctttgaaggcgcagcgtgaagagccagcgccgcatttcatcgtccagcgccggcgcgtgctgctccagcaggtcgatgttgcgcgccaggaaatcctcgatggcactcctcaggtcgcgcagatcggttcttcgcacgcgatagacaaaagccagctctggcaaggcatgcgcccattgcgcgatgaactcatcgcgcatgagcccggcaagaccttgcatcgccgcacggcgcacctccagaacccagtcgccgacacccaccagcaacaccgggatggcttgcggatcggcccggcggaccagttcgacaacggccgcttcccgctgatagccgtcgcaggagcgggcgagccccatcaaggcacccgcatcgagcgcgcgcatctccagtgccggcagcgcttcggttcttgttttccaccatttcatcgctcttccctttcttcagcgcctacgaattgcgctgcctccatttgccagggcgatgagcttcgccccgggttctatcccttcacgcacaccacctgcttgagcgtgtagaccacctccaccaggtctttctgcgcctccatcaccgcgtcgatgtccttgtaggccatcggaatctcgtcgatcacgtcggcgtccttgcggcattccacgccttcggtggcggcgatctggtcggcaatggtgaagagcttcttcgccttggtgcggctcatgactcggcccgcgccgtggctgcagctcatgaagctctcggggttgccctttccacgcacgatgtagctcttggcacccatgctgccgggaatgatcccgagctcgccggccttggcgctcaccgcgcccttgcgcgtgacgagcacgtcttcgccgaaatgcgtttcgcggctcacgtagttgtgatggcagttcaccgcttccacatgcgcctcgaagggtttggtgatgaccttgcgcgcggccgcgaccacgcgctgcatcatcacttcgcggttggcacgcgcgaacttctgggcccagcccactgcgcgcacgtagtcgccgaagtacttggcgccctcctcgaagtacgccaggtcctgatcgggcaggttgcgctggtgcagttcggcatccttcttcgcgagttcgatgaagtgcgtgccgatggcattccccacgccacgcgaacccgagtgcagcatgaaccacacggcgcccgcttcgtccaggcacacctcgatgaagtggttgccggtacccagcgttcccaggtgcttgtggttgttcgtgttcttgatgcgcgggtagtcctcgcagatcgcgtcgaattcgtccacgagcttggcccaggcggcatcggtctcatcgggcggcgtttcccacgagcccttgtcgcggcccatgcgcttgggattgcttccgtgcggcacggccttttcgatggccgagcgcagcgggcccaggttatcgggcaggtcgcgcgcattgagcgtggtcttgcacgccatcattccgcagccgatgtccacgcccaccgcggccgggatgatggccttgaaggtcgggatcaccgagcccacggtcgcgccgatgccgtagtgcacatcgggcatggccgcgatgtgcttgaacacgatgggcaggcgggcggcgttctcgagctgcttttgcgcttcgtcttccacgggcacgccgttcgtccacatcttgacggggacgccgttggcgacttcgtgcagtttgtagttctgttccatttttctttccctttccgttctatctatctattctttacgactgatggtggacacggcgggattcgaacccgcatcaatacggcgaccatggtgtttgagtccgatggcccagtcgacgattggaaacgcgcgccagtgacagacccgtcatcggagccagcacctgcatcctcaaccttgctcgtcaaccggctttcccgccgcatccggtgctacccggactgccggcaataacaacatttttggcagtggcgctcccttctgtgcctgcgcgcccgaaaacaaaaaaagcagcgacgaaaatcggcgaaacagtcgtgctctaccactgagctacggtcttgcgaccggcgggattcgaacccgcgaccccgagcgttgtaggctgtagttccgccagcattcgctgcaaaaaaacagtgcgacaaggatggcaagacatgcccaccagcgagccggtgttggggttcgacccccgggcgtccagatgtagtcctgcctgcattcgcacaaaaacctcatccccgttcggcgacaaacattcgatgcgaggaagaacatggttggatgtactcgcatctgcattcgccgaacgacgacgttcaatttcttcggatcgggcaccgcgggcaaggcccacggcgccctctcacttttctctcagatcgaagtctcttcgatcactcccacccagtgctcggcgcccaggccacccgcggcatacaccgccagcagcttgaacacttcgtcgctgaagccgccgatgttcagcacatcgtcacgctcctgcgcctgggtggtcgcatagggctggatgtcgatgcacaccatccgcgccttcgggttgcgttgcttgaacgcagcccactcctgcatggtcgcggttccgcggccacgtgcagggtcggcccacgattcgttgtccgacaccagcaccaccagatcggcctgcgccttctccttgttcagcagcgccaagggcgcgctgcacgaggttccgccaccaccgaccgccgccagcttggccgcgttggtcatcaccgaatcacgcggattcagcttcagcgacaccaccttcgtctcgaagggcagcacacgcgcatccgcattgcggcgcagcacggcggcagccaccagcgcggccacgtcgatgcagcgcaccgccgacgttgccgaaccgcggtggcccgtcaccggcgagctcatggagcccgacacgtcggggcacaccaccacgcggccctcgaatgccggcacgttggccagcgcgagttccatcgcgtcctgcagcgcttccttcaccacgtgcggcacctcggcgccggttgcggtgaaggccgccatcagctggtacggcagcacgcgcgccttggccaccgcctgcgggtcacgcagcttg

(The sequence listing continues in the following parts.)